European Patent Application EP 4 803 615 A1 - sequence listing, part 2

SEQ ID NO: 30579 - DNA, 28 bp, synthetic construct
  source 1..28: mol_type = other DNA
ttgaactggctgggaaaaggagggaggg

SEQ ID NO: 30580 - DNA, 28 bp, synthetic construct
  source 1..28: mol_type = other DNA
gctgggaaaaggagggagggtagaaagg

SEQ ID NO: 30581 - DNA, 28 bp, synthetic construct
  source 1..28: mol_type = other DNA
ctgggaaaaggagggagggtagaaaggg

SEQ ID NO: 30582 - DNA, 28 bp, synthetic construct
  source 1..28: mol_type = other DNA
tgggaaaaggagggagggtagaaagggg

SEQ ID NO: 30583 - DNA, 28 bp, synthetic construct
  source 1..28: mol_type = other DNA
gggaaaaggagggagggtagaaaggggg

SEQ ID NO: 30584 - DNA, 28 bp, synthetic construct
  source 1..28: mol_type = other DNA
gagggtagaaagggggccaataccccgg

SEQ ID NO: 30585 - DNA, 28 bp, synthetic construct
  source 1..28: mol_type = other DNA
agaaagggggccaataccccggtcgagg

SEQ ID NO: 30586 - DNA, 28 bp, synthetic construct
  source 1..28: mol_type = other DNA
gaaagggggccaataccccggtcgaggg

SEQ ID NO: 30587 - DNA, 28 bp, synthetic construct
  source 1..28: mol_type = other DNA
agttctcagccctcgaccggggtattgg

SEQ ID NO: 30588 - DNA, 28 bp, synthetic construct
  source 1..28: mol_type = other DNA
taaaacagttctcagccctcgaccgggg

SEQ ID NO: 30589 - DNA, 28 bp, synthetic construct
  source 1..28: mol_type = other DNA
ctaaaacagttctcagccctcgaccggg

SEQ ID NO: 30590 - DNA, 28 bp, synthetic construct
  source 1..28: mol_type = other DNA
tctaaaacagttctcagccctcgaccgg

SEQ ID NO: 30591 - DNA, 28 bp, synthetic construct
  source 1..28: mol_type = other DNA
gtcgagggctgagaactgttttagaagg

SEQ ID NO: 30592 - DNA, 28 bp, synthetic construct
  source 1..28: mol_type = other DNA
gaactgttttagaaggcaacatatttgg

SEQ ID NO: 30593 - DNA, 28 bp, synthetic construct
  source 1..28: mol_type = other DNA
tcagctattatggaagctggctgcaggg

SEQ ID NO: 30594 - DNA, 28 bp, synthetic construct
  source 1..28: mol_type = other DNA
atcagctattatggaagctggctgcagg

SEQ ID NO: 30595 - DNA, 28 bp, synthetic construct
  source 1..28: mol_type = other DNA
ggcaataatcagctattatggaagctgg

SEQ ID NO: 30596 - DNA, 28 bp, synthetic construct
  source 1..28: mol_type = other DNA
acatctgggcaataatcagctattatgg

SEQ ID NO: 30597 - DNA, 28 bp, synthetic construct
  source 1..28: mol_type = other DNA
cctaggagcagctcttttgacatctggg

SEQ ID NO: 30598 - DNA, 28 bp, synthetic construct
  source 1..28: mol_type = other DNA
ccctaggagcagctcttttgacatctgg

SEQ ID NO: 30599 - DNA, 28 bp, synthetic construct
  source 1..28: mol_type = other DNA
ttgtctgatgagcagactgaaccctagg

SEQ ID NO: 30600 - DNA, 28 bp, synthetic construct
  source 1..28: mol_type = other DNA
atttattgaatgtaagtagttgctgagg

SEQ ID NO: 30601 - DNA, 28 bp, synthetic construct
  source 1..28: mol_type = other DNA
tatgcttcactgacattctacaccctgg

SEQ ID NO: 30602 - DNA, 28 bp, synthetic construct
  source 1..28: mol_type = other DNA
atgcttcactgacattctacaccctggg

SEQ ID NO: 30603 - DNA, 28 bp, synthetic construct
  source 1..28: mol_type = other DNA
tctacaccctgggaatgagtgtttctgg

SEQ ID NO: 30604 - DNA, 28 bp, synthetic construct
  source 1..28: mol_type = other DNA
ctacaccctgggaatgagtgtttctggg

SEQ ID NO: 30605 - DNA, 28 bp, synthetic construct
  source 1..28: mol_type = other DNA
acattcccagaaacactcattcccaggg

SEQ ID NO: 30606 - DNA, 28 bp, synthetic construct
  source 1..28: mol_type = other DNA
cacattcccagaaacactcattcccagg

SEQ ID NO: 30607 - DNA, 28 bp, synthetic construct
  source 1..28: mol_type = other DNA
aaaaaaaaaaaaaaaaaaaaaaaaaagg

SEQ ID NO: 30608 - DNA, 28 bp, synthetic construct
  source 1..28: mol_type = other DNA
ttttttttttttttttaacaaaaccagg

SEQ ID NO: 30609 - DNA, 28 bp, synthetic construct
  source 1..28: mol_type = other DNA
tttaacaaaaccaggtttttccctaagg

SEQ ID NO: 30610 - DNA, 28 bp, synthetic construct
  source 1..28: mol_type = other DNA
aaggtgcattccttagggaaaaacctgg

SEQ ID NO: 30611 - DNA, 28 bp, synthetic construct
  source 1..28: mol_type = other DNA
aactttggggaaggtgcattccttaggg

SEQ ID NO: 30612 - DNA, 28 bp, synthetic construct
  source 1..28: mol_type = other DNA
aaactttggggaaggtgcattccttagg

SEQ ID NO: 30613 - DNA, 28 bp, synthetic construct
  source 1..28: mol_type = other DNA
aggaggatgcgggaaactttggggaagg

SEQ ID NO: 30614 - DNA, 28 bp, synthetic construct
  source 1..28: mol_type = other DNA
aggcaggaggatgcgggaaactttgggg

SEQ ID NO: 30615 - DNA, 28 bp, synthetic construct
  source 1..28: mol_type = other DNA
taggcaggaggatgcgggaaactttggg

SEQ ID NO: 30616 - DNA, 28 bp, synthetic construct
  source 1..28: mol_type = other DNA
gtaggcaggaggatgcgggaaactttgg

SEQ ID NO: 30617 - DNA, 28 bp, synthetic construct
  source 1..28: mol_type = other DNA
gtgaattatgtaggcaggaggatgcggg

SEQ ID NO: 30618 - DNA, 28 bp, synthetic construct
  source 1..28: mol_type = other DNA
agtgaattatgtaggcaggaggatgcgg

SEQ ID NO: 30619 - DNA, 28 bp, synthetic construct
  source 1..28: mol_type = other DNA
tatataagtgaattatgtaggcaggagg

SEQ ID NO: 30620 - DNA, 28 bp, synthetic construct
  source 1..28: mol_type = other DNA
gactatataagtgaattatgtaggcagg

SEQ ID NO: 30621 - DNA, 28 bp, synthetic construct
  source 1..28: mol_type = other DNA
tagtgactatataagtgaattatgtagg

SEQ ID NO: 30622 - DNA, 28 bp, synthetic construct
  source 1..28: mol_type = other DNA
gacattaattagattcagaagtctgtgg

SEQ ID NO: 30623 - DNA, 28 bp, synthetic construct
  source 1..28: mol_type = other DNA
agaagtctgtggaaacagcagagctcgg

SEQ ID NO: 30624 - DNA, 28 bp, synthetic construct
  source 1..28: mol_type = other DNA
gtctgtggaaacagcagagctcggcagg

SEQ ID NO: 30625 - DNA, 28 bp, synthetic construct
  source 1..28: mol_type = other DNA
tctgtggaaacagcagagctcggcaggg

SEQ ID NO: 30626 - DNA, 28 bp, synthetic construct
  source 1..28: mol_type = other DNA
aaacagcagagctcggcagggtcagagg

SEQ ID NO: 30627 - DNA, 28 bp, synthetic construct
  source 1..28: mol_type = other DNA
aacagcagagctcggcagggtcagaggg

SEQ ID NO: 30628 - DNA, 28 bp, synthetic construct
  source 1..28: mol_type = other DNA
agctcggcagggtcagagggcaagcagg

SEQ ID NO: 30629 - DNA, 28 bp, synthetic construct
  source 1..28: mol_type = other DNA
gctcggcagggtcagagggcaagcaggg

SEQ ID NO: 30630 - DNA, 28 bp, synthetic construct
  source 1..28: mol_type = other DNA
agggcaagcagggcagagaaaagagagg

SEQ ID NO: 30631 - DNA, 28 bp, synthetic construct
  source 1..28: mol_type = other DNA
gggcaagcagggcagagaaaagagaggg

SEQ ID NO: 30632 - DNA, 28 bp, synthetic construct
  source 1..28: mol_type = other DNA
ggcaagcagggcagagaaaagagagggg

SEQ ID NO: 30633 - DNA, 28 bp, synthetic construct
  source 1..28: mol_type = other DNA
agaaaagagaggggaaaatgagctccgg

SEQ ID NO: 30634 - DNA, 28 bp, synthetic construct
  source 1..28: mol_type = other DNA
gaaaagagaggggaaaatgagctccggg

SEQ ID NO: 30635 - DNA, 28 bp, synthetic construct
  source 1..28: mol_type = other DNA
gagaggggaaaatgagctccgggagagg

SEQ ID NO: 30636 - DNA, 28 bp, synthetic construct
  source 1..28: mol_type = other DNA
agaggggaaaatgagctccgggagaggg

SEQ ID NO: 30637 - DNA, 28 bp, synthetic construct
  source 1..28: mol_type = other DNA
gaggggaaaatgagctccgggagagggg

SEQ ID NO: 30638 - DNA, 28 bp, synthetic construct
  source 1..28: mol_type = other DNA
ggaaaatgagctccgggagaggggaagg

SEQ ID NO: 30639 - DNA, 28 bp, synthetic construct
  source 1..28: mol_type = other DNA
tgagctccgggagaggggaaggaagtgg

SEQ ID NO: 30640 - DNA, 28 bp, synthetic construct
  source 1..28: mol_type = other DNA
gctccgggagaggggaaggaagtggagg

SEQ ID NO: 30641 - DNA, 28 bp, synthetic construct
  source 1..28: mol_type = other DNA
ctccgggagaggggaaggaagtggaggg

SEQ ID NO: 30642 - DNA, 28 bp, synthetic construct
  source 1..28: mol_type = other DNA
ttccctccacttccttcccctctcccgg

SEQ ID NO: 30643 - DNA, 28 bp, synthetic construct
  source 1..28: mol_type = other DNA
atctttgttttgtttggtacttgaaggg

SEQ ID NO: 30644 - DNA, 28 bp, synthetic construct
  source 1..28: mol_type = other DNA
tatctttgttttgtttggtacttgaagg

SEQ ID NO: 30645 - DNA, 28 bp, synthetic construct
  source 1..28: mol_type = other DNA
cttttgaaattatctttgttttgtttgg

SEQ ID NO: 30646 - DNA, 28 bp, synthetic construct
  source 1..28: mol_type = other DNA
aacaaaacaaagataatttcaaaagtgg

SEQ ID NO: 30647 - DNA, 28 bp, synthetic construct
  source 1..28: mol_type = other DNA
tttaattctctaagcagtgttatagtgg

SEQ ID NO: 30648 - DNA, 28 bp, synthetic construct
  source 1..28: mol_type = other DNA
aattgaagagtgctttaaaataaagtgg

SEQ ID NO: 30649 - DNA, 28 bp, synthetic construct
  source 1..28: mol_type = other DNA
gaagagtgctttaaaataaagtggatgg

SEQ ID NO: 30650 - DNA, 28 bp, synthetic construct
  source 1..28: mol_type = other DNA
aagagtgctttaaaataaagtggatggg

SEQ ID NO: 30651 - DNA, 28 bp, synthetic construct
  source 1..28: mol_type = other DNA
agagtgctttaaaataaagtggatgggg

SEQ ID NO: 30652 - DNA, 28 bp, synthetic construct
  source 1..28: mol_type = other DNA
ggatggggcataagcatgtatgtcttgg

SEQ ID NO: 30653 - DNA, 28 bp, synthetic construct
  source 1..28: mol_type = other DNA
tggtgttagttgctccttatacagccgg

SEQ ID NO: 30654 - DNA, 28 bp, synthetic construct
  source 1..28: mol_type = other DNA
ttgctccttatacagccggtactaaagg

SEQ ID NO: 30655 - DNA, 28 bp, synthetic construct
  source 1..28: mol_type = other DNA
tccttatacagccggtactaaaggctgg

SEQ ID NO: 30656 - DNA, 28 bp, synthetic construct
  source 1..28: mol_type = other DNA
accagcctttagtaccggctgtataagg

SEQ ID NO: 30657 - DNA, 28 bp, synthetic construct
  source 1..28: mol_type = other DNA
ttatacagccggtactaaaggctggtgg

SEQ ID NO: 30658 - DNA, 28 bp, synthetic construct
  source 1..28: mol_type = other DNA
tatacagccggtactaaaggctggtggg

SEQ ID NO: 30659 - DNA, 28 bp, synthetic construct
  source 1..28: mol_type = other DNA
agcttcacccaccagcctttagtaccgg

SEQ ID NO: 30660 - DNA, 28 bp, synthetic construct
  source 1..28: mol_type = other DNA
agcttaccacattttaaaaagaaaaagg

SEQ ID NO: 30661 - DNA, 28 bp, synthetic construct
  source 1..28: mol_type = other DNA
taccacattttaaaaagaaaaaggcagg

SEQ ID NO: 30662 - DNA, 28 bp, synthetic construct
  source 1..28: mol_type = other DNA
tgcctgcctttttctttttaaaatgtgg

SEQ ID NO: 30663 - DNA, 28 bp, synthetic construct
  source 1..28: mol_type = other DNA
gcacacatactaaagttgaaaatgcagg

SEQ ID NO: 30664 - DNA, 28 bp, synthetic construct
  source 1..28: mol_type = other DNA
acatactaaagttgaaaatgcaggcagg

SEQ ID NO: 30665 - DNA, 28 bp, synthetic construct
  source 1..28: mol_type = other DNA
actaaagttgaaaatgcaggcaggaagg

SEQ ID NO: 30666 - DNA, 28 bp, synthetic construct
  source 1..28: mol_type = other DNA
gaaggacatttacttttcataaaagcgg

SEQ ID NO: 30667 - DNA, 28 bp, synthetic construct
  source 1..28: mol_type = other DNA
tggcataaaatacatgatctgtgatagg

SEQ ID NO: 30668 - DNA, 28 bp, synthetic construct
  source 1..28: mol_type = other DNA
tattttatgccatgctgaccaatgttgg

SEQ ID NO: 30669 - DNA, 28 bp, synthetic construct
  source 1..28: mol_type = other DNA
attttatgccatgctgaccaatgttggg

SEQ ID NO: 30670 - DNA, 28 bp, synthetic construct
  source 1..28: mol_type = other DNA
ttttatgccatgctgaccaatgttgggg

SEQ ID NO: 30671 - DNA, 28 bp, synthetic construct
  source 1..28: mol_type = other DNA
tttatgccatgctgaccaatgttggggg

SEQ ID NO: 30672 - DNA, 28 bp, synthetic construct
  source 1..28: mol_type = other DNA
gattatcccccaacattggtcagcatgg

SEQ ID NO: 30673 - DNA, 28 bp, synthetic construct
  source 1..28: mol_type = other DNA
aaataatgagattatcccccaacattgg

SEQ ID NO: 30674 - DNA, 28 bp, synthetic construct
  source 1..28: mol_type = other DNA
gtgatatgagaagatcctttgatgctgg

SEQ ID NO: 30675 - DNA, 28 bp, synthetic construct
  source 1..28: mol_type = other DNA
gattggttcttgttaccagcatcaaagg

SEQ ID NO: 30676 - DNA, 28 bp, synthetic construct
  source 1..28: mol_type = other DNA
atattaagatttaagtcaggatgattgg

SEQ ID NO: 30677 - DNA, 28 bp, synthetic construct
  source 1..28: mol_type = other DNA
ctgtggggatattaagatttaagtcagg

SEQ ID NO: 30678 - DNA, 28 bp, synthetic construct
  source 1..28: mol_type = other DNA
ctgacttaaatcttaatatccccacagg

SEQ ID NO: 30679 - DNA, 28 bp, synthetic construct
  source 1..28: mol_type = other DNA
gaagaagcatgacaaagaacctgtgggg

SEQ ID NO: 30680 - DNA, 28 bp, synthetic construct
  source 1..28: mol_type = other DNA
tgaagaagcatgacaaagaacctgtggg

SEQ ID NO: 30681 - DNA, 28 bp, synthetic construct
  source 1..28: mol_type = other DNA
ttgaagaagcatgacaaagaacctgtgg

SEQ ID NO: 30682 - DNA, 28 bp, synthetic construct
  source 1..28: mol_type = other DNA
tgtcatgcttcttcaagatgtgccctgg

SEQ ID NO: 30683 - DNA, 28 bp, synthetic construct
  source 1..28: mol_type = other DNA
gccctggccattcatgcaagtttcaagg

SEQ ID NO: 30684 - DNA, 28 bp, synthetic construct
  source 1..28: mol_type = other DNA
tccttgaaacttgcatgaatggccaggg

SEQ ID NO: 30685 - DNA, 28 bp, synthetic construct
  source 1..28: mol_type = other DNA
gtccttgaaacttgcatgaatggccagg

SEQ ID NO: 30686 - DNA, 28 bp, synthetic construct
  source 1..28: mol_type = other DNA
tcagagtccttgaaacttgcatgaatgg

SEQ ID NO: 30687 - DNA, 28 bp, synthetic construct
  source 1..28: mol_type = other DNA
caaggactctgaatctgttgagaatagg

SEQ ID NO: 30688 - DNA, 28 bp, synthetic construct
  source 1..28: mol_type = other DNA
caaacatgtctatattactgtcaactgg

SEQ ID NO: 30689 - DNA, 28 bp, synthetic construct
  source 1..28: mol_type = other DNA
aaacatgtctatattactgtcaactggg

SEQ ID NO: 30690 - DNA, 28 bp, synthetic construct
  source 1..28: mol_type = other DNA
ctcatgtgcttttgggaggactaaatgg

SEQ ID NO: 30691 - DNA, 28 bp, synthetic construct
  source 1..28: mol_type = other DNA
catttagtcctcccaaaagcacatgagg

SEQ ID NO: 30692 - DNA, 28 bp, synthetic construct
  source 1..28: mol_type = other DNA
gcaacatacctcatgtgcttttgggagg

SEQ ID NO: 30693 - DNA, 28 bp, synthetic construct
  source 1..28: mol_type = other DNA
atggcaacatacctcatgtgcttttggg

SEQ ID NO: 30694 - DNA, 28 bp, synthetic construct
  source 1..28: mol_type = other DNA
aatggcaacatacctcatgtgcttttgg

SEQ ID NO: 30695 - DNA, 28 bp, synthetic construct
  source 1..28: mol_type = other DNA
tatgttgccattgtttttattttgcagg

SEQ ID NO: 30696 - DNA, 28 bp, synthetic construct
  source 1..28: mol_type = other DNA
atactcacctgcaaaataaaaacaatgg

SEQ ID NO: 30697 - DNA, 28 bp, synthetic construct
  source 1..28: mol_type = other DNA
ttttattttgcaggtgagtatgctaagg

SEQ ID NO: 30698 - DNA, 28 bp, synthetic construct
  source 1..28: mol_type = other DNA
tttgcaggtgagtatgctaaggaacagg

SEQ ID NO: 30699 - DNA, 28 bp, synthetic construct
  source 1..28: mol_type = other DNA
caggtaagtgtcacaaacccaagcatgg

SEQ ID NO: 30700 - DNA, 28 bp, synthetic construct
  source 1..28: mol_type = other DNA
gtcacaaacccaagcatggcagatcagg

SEQ ID NO: 30701 - DNA, 28 bp, synthetic construct
  source 1..28: mol_type = other DNA
aacccaagcatggcagatcaggaattgg

SEQ ID NO: 30702 - DNA, 28 bp, synthetic construct
  source 1..28: mol_type = other DNA
taccaattcctgatctgccatgcttggg

SEQ ID NO: 30703 - DNA, 28 bp, synthetic construct
  source 1..28: mol_type = other DNA
ataccaattcctgatctgccatgcttgg

SEQ ID NO: 30704 - DNA, 28 bp, synthetic construct
  source 1..28: mol_type = other DNA
aagcatggcagatcaggaattggtatgg

SEQ ID NO: 30705 - DNA, 28 bp, synthetic construct
  source 1..28: mol_type = other DNA
agatcaggaattggtatggtattactgg

SEQ ID NO: 30706 - DNA, 28 bp, synthetic construct
  source 1..28: mol_type = other DNA
ggcaaaagttgtgggaggtggagtatgg

SEQ ID NO: 30707 - DNA, 28 bp, synthetic construct
  source 1..28: mol_type = other DNA
taattaaggcaaaagttgtgggaggtgg

SEQ ID NO: 30708 - DNA, 28 bp, synthetic construct
  source 1..28: mol_type = other DNA
agataattaaggcaaaagttgtgggagg

SEQ ID NO: 30709 - DNA, 28 bp, synthetic construct
  source 1..28: mol_type = other DNA
tatagataattaaggcaaaagttgtggg

SEQ ID NO: 30710 - DNA, 28 bp, synthetic construct
  source 1..28: mol_type = other DNA
ctatagataattaaggcaaaagttgtgg

SEQ ID NO: 30711 - DNA, 28 bp, synthetic construct
  source 1..28: mol_type = other DNA
cttttgccttaattatctatagcattgg

SEQ ID NO: 30712 - DNA, 28 bp, synthetic construct
  source 1..28: mol_type = other DNA
aatgcgccaatgctatagataattaagg

SEQ ID NO: 30713 - DNA, 28 bp, synthetic construct
  source 1..28: mol_type = other DNA
agcattggcgcattctcatgctcacagg

SEQ ID NO: 30714 - DNA, 28 bp, synthetic construct
  source 1..28: mol_type = other DNA
ataatgaaagtaatacagtcccagtcgg

SEQ ID NO: 30715 - DNA, 28 bp, synthetic construct
  source 1..28: mol_type = other DNA
tgaaagtaatacagtcccagtcggaagg

SEQ ID NO: 30716 - DNA, 28 bp, synthetic construct
  source 1..28: mol_type = other DNA
gagggctctctctcgccttccgactggg

SEQ ID NO: 30717 - DNA, 28 bp, synthetic construct
  source 1..28: mol_type = other DNA
agagggctctctctcgccttccgactgg

SEQ ID NO: 30718 - DNA, 28 bp, synthetic construct
  source 1..28: mol_type = other DNA
caggagaattgcagagaggggtagaggg

SEQ ID NO: 30719 - DNA, 28 bp, synthetic construct
  source 1..28: mol_type = other DNA
gcaggagaattgcagagaggggtagagg

SEQ ID NO: 30720 - DNA, 28 bp, synthetic construct
  source 1..28: mol_type = other DNA
tgggtggcaggagaattgcagagagggg

SEQ ID NO: 30721 - DNA, 28 bp, synthetic construct
  source 1..28: mol_type = other DNA
ctgggtggcaggagaattgcagagaggg

SEQ ID NO: 30722 - DNA, 28 bp, synthetic construct
  source 1..28: mol_type = other DNA
actgggtggcaggagaattgcagagagg

SEQ ID NO: 30723 - DNA, 28 bp, synthetic construct
  source 1..28: mol_type = other DNA
aactcaaggggcaaaactgggtggcagg

SEQ ID NO: 30724 - DNA, 28 bp, synthetic construct
  source 1..28: mol_type = other DNA
gcagaactcaaggggcaaaactgggtgg

SEQ ID NO: 30725 - DNA, 28 bp, synthetic construct
  source 1..28: mol_type = other DNA
atggcagaactcaaggggcaaaactggg

SEQ ID NO: 30726 - DNA, 28 bp, synthetic construct
  source 1..28: mol_type = other DNA
tatggcagaactcaaggggcaaaactgg

SEQ ID NO: 30727 - DNA, 28 bp, synthetic construct
  source 1..28: mol_type = other DNA
aggtgcggttatggcagaactcaagggg

SEQ ID NO: 30728 - DNA, 28 bp, synthetic construct
  source 1..28: mol_type = other DNA
caggtgcggttatggcagaactcaaggg

SEQ ID NO: 30729 - DNA, 28 bp, synthetic construct
  source 1..28: mol_type = other DNA
ccttgagttctgccataaccgcacctgg

SEQ ID NO: 30730 - DNA, 28 bp, synthetic construct
  source 1..28: mol_type = other DNA
ttctgccataaccgcacctggagtgagg

SEQ ID NO: 30731 - DNA, 28 bp, synthetic construct
  source 1..28: mol_type = other DNA
gagcgcctcactccaggtgcggttatgg

SEQ ID NO: 30732 - DNA, 28 bp, synthetic construct
  source 1..28: mol_type = other DNA
gacaaggagcgcctcactccaggtgcgg

SEQ ID NO: 30733 - DNA, 28 bp, synthetic construct
  source 1..28: mol_type = other DNA
ctagagacaaggagcgcctcactccagg

SEQ ID NO: 30734 - DNA, 28 bp, synthetic construct
  source 1..28: mol_type = other DNA
aaggaagacgttgaggctagagacaagg

SEQ ID NO: 30735 - DNA, 28 bp, synthetic construct
  source 1..28: mol_type = other DNA
tctcatgttgcaaaggaagacgttgagg

SEQ ID NO: 30736 - DNA, 28 bp, synthetic construct
  source 1..28: mol_type = other DNA
caacgtcttcctttgcaacatgagaagg

SEQ ID NO: 30737 - DNA, 28 bp, synthetic construct
  source 1..28: mol_type = other DNA
gtcttcctttgcaacatgagaaggctgg

SEQ ID NO: 30738 - DNA, 28 bp, synthetic construct
  source 1..28: mol_type = other DNA
cctttgcaacatgagaaggctggattgg

SEQ ID NO: 30739 - DNA, 28 bp, synthetic construct
  source 1..28: mol_type = other DNA
ctttgcaacatgagaaggctggattggg

SEQ ID NO: 30740 - DNA, 28 bp, synthetic construct
  source 1..28: mol_type = other DNA
gtctctgacagttctgaaatgttagagg

SEQ ID NO: 30741 - DNA, 28 bp, synthetic construct
  source 1..28: mol_type = other DNA
ttgttcttcctgagcactgccagacagg

SEQ ID NO: 30742 - DNA, 28 bp, synthetic construct
  source 1..28: mol_type = other DNA
cagggattcctgtctggcagtgctcagg

SEQ ID NO: 30743 - DNA, 28 bp, synthetic construct
  source 1..28: mol_type = other DNA
ctgagcactgccagacaggaatccctgg

SEQ ID NO: 30744 - DNA, 28 bp, synthetic construct
  source 1..28: mol_type = other DNA
ttgacatactccagggattcctgtctgg

SEQ ID NO: 30745 - DNA, 28 bp, synthetic construct
  source 1..28: mol_type = other DNA
tttatgactctcttgacatactccaggg

SEQ ID NO: 30746 - DNA, 28 bp, synthetic construct
  source 1..28: mol_type = other DNA
gtttatgactctcttgacatactccagg

SEQ ID NO: 30747 - DNA, 28 bp, synthetic construct
  source 1..28: mol_type = other DNA
gagtcataaaccttttcttgtttaaagg

SEQ ID NO: 30748 - DNA, 28 bp, synthetic construct
  source 1..28: mol_type = other DNA
cataaaccttttcttgtttaaaggtagg

SEQ ID NO: 30749 - DNA, 28 bp, synthetic construct
  source 1..28: mol_type = other DNA
ggaggtcctacctttaaacaagaaaagg

SEQ ID NO: 30750 - DNA, 28 bp, synthetic construct
  source 1..28: mol_type = other DNA
ttgtttaaaggtaggacctccttcttgg

SEQ ID NO: 30751 - DNA, 28 bp, synthetic construct
  source 1..28: mol_type = other DNA
ttgagatttgtttaagccaagaaggagg

SEQ ID NO: 30752 - DNA, 28 bp, synthetic construct
  source 1..28: mol_type = other DNA
tccttcttggcttaaacaaatctcaagg

SEQ ID NO: 30753 - DNA, 28 bp, synthetic construct
  source 1..28: mol_type = other DNA
accttgagatttgtttaagccaagaagg

SEQ ID NO: 30754 - DNA, 28 bp, synthetic construct
  source 1..28: mol_type = other DNA
ttggcttaaacaaatctcaaggtgttgg

SEQ ID NO: 30755 - DNA, 28 bp, synthetic construct
  source 1..28: mol_type = other DNA
ctcaaggtgttggtctgcttcaaacagg

SEQ ID NO: 30756 - DNA, 28 bp, synthetic construct
  source 1..28: mol_type = other DNA
gtgctatctgtgaagtattagcagacgg

SEQ ID NO: 30757 - DNA, 28 bp, synthetic construct
  source 1..28: mol_type = other DNA
ctgtgaagtattagcagacggcaagagg

SEQ ID NO: 30758 - DNA, 28 bp, synthetic construct
  source 1..28: mol_type = other DNA
agcagacggcaagaggaatgtgttcagg

SEQ ID NO: 30759 - DNA, 28 bp, synthetic construct
  source 1..28: mol_type = other DNA
cggcaagaggaatgtgttcaggaagagg

SEQ ID NO: 30760 - DNA, 28 bp, synthetic construct
  source 1..28: mol_type = other DNA
tgttcaggaagaggacacttagcttagg

SEQ ID NO: 30761 - DNA, 28 bp, synthetic construct
  source 1..28: mol_type = other DNA
aggaagaggacacttagcttaggtctgg

SEQ ID NO: 30762 - DNA, 28 bp, synthetic construct
  source 1..28: mol_type = other DNA
ggaagaggacacttagcttaggtctggg

SEQ ID NO: 30763 - DNA, 28 bp, synthetic construct
  source 1..28: mol_type = other DNA
gaagaggacacttagcttaggtctgggg

SEQ ID NO: 30764 - DNA, 28 bp, synthetic construct
  source 1..28: mol_type = other DNA
aagaggacacttagcttaggtctggggg

SEQ ID NO: 30765 - DNA, 28 bp, synthetic construct
  source 1..28: mol_type = other DNA
acttagcttaggtctgggggaagcatgg

SEQ ID NO: 30766 - DNA, 28 bp, synthetic construct
  source 1..28: mol_type = other DNA
cttagcttaggtctgggggaagcatggg

SEQ ID NO: 30767 - DNA, 28 bp, synthetic construct
  source 1..28: mol_type = other DNA
ttagcttaggtctgggggaagcatgggg

SEQ ID NO: 30768 - DNA, 28 bp, synthetic construct
  source 1..28: mol_type = other DNA
tggggaagaagtcacaacacaactgtgg

SEQ ID NO: 30769 - DNA, 28 bp, synthetic construct
  source 1..28: mol_type = other DNA
ggggaagaagtcacaacacaactgtggg

SEQ ID NO: 30770 - DNA, 28 bp, synthetic construct
  source 1..28: mol_type = other DNA
aagtcacaacacaactgtgggtgtcagg

SEQ ID NO: 30771 - DNA, 28 bp, synthetic construct
  source 1..28: mol_type = other DNA
actgtgggtgtcaggctcttttctctgg

SEQ ID NO: 30772 - DNA, 28 bp, synthetic construct
  source 1..28: mol_type = other DNA
ctgtgggtgtcaggctcttttctctggg

SEQ ID NO: 30773 - DNA, 28 bp, synthetic construct
  source 1..28: mol_type = other DNA
tgtgggtgtcaggctcttttctctgggg

SEQ ID NO: 30774 - DNA, 28 bp, synthetic construct
  source 1..28: mol_type = other DNA
tggggcaccagagagtattcaagcatgg

SEQ ID NO: 30775 - DNA, 28 bp, synthetic construct
  source 1..28: mol_type = other DNA
caccagagagtattcaagcatggattgg

SEQ ID NO: 30776 - DNA, 28 bp, synthetic construct
  source 1..28: mol_type = other DNA
taccaatccatgcttgaatactctctgg

SEQ ID NO: 30777 - DNA, 28 bp, synthetic construct
  source 1..28: mol_type = other DNA
ggattggtagtccccatgcagccctcgg

SEQ ID NO: 30778 - DNA, 28 bp, synthetic construct
  source 1..28: mol_type = other DNA
ttggtagtccccatgcagccctcggagg

SEQ ID NO: 30779 - DNA, 28 bp, synthetic construct
  source 1..28: mol_type = other DNA
ttcggtttcctccgagggctgcatgggg

SEQ ID NO: 30780 - DNA, 28 bp, synthetic construct
  source 1..28: mol_type = other DNA
cttcggtttcctccgagggctgcatggg

SEQ ID NO: 30781 - DNA, 28 bp, synthetic construct
  source 1..28: mol_type = other DNA
gcttcggtttcctccgagggctgcatgg

SEQ ID NO: 30782 - DNA, 28 bp, synthetic construct
  source 1..28: mol_type = other DNA
catttgcagcttcggtttcctccgaggg

SEQ ID NO: 30783 - DNA, 28 bp, synthetic construct
  source 1..28: mol_type = other DNA
gcatttgcagcttcggtttcctccgagg

SEQ ID NO: 30784 - DNA, 28 bp, synthetic construct
  source 1..28: mol_type = other DNA
accgaagctgcaaatgcagcaattatgg

SEQ ID NO: 30785 - DNA, 28 bp, synthetic construct
  source 1..28: mol_type = other DNA
gccataattgctgcatttgcagcttcgg

SEQ ID NO: 30786 - DNA, 28 bp, synthetic construct
  source 1..28: mol_type = other DNA
gcaattatggcttacagcctgaaaatgg

SEQ ID NO: 30787 - DNA, 28 bp, synthetic construct
  source 1..28: mol_type = other DNA
gcaattttggaatgtcaccattttcagg

SEQ ID NO: 30788 - DNA, 28 bp, synthetic construct
  source 1..28: mol_type = other DNA
gtgacattccaaaattgcatcttaatgg

SEQ ID NO: 30789 - DNA, 28 bp, synthetic construct
  source 1..28: mol_type = other DNA
tgacattccaaaattgcatcttaatggg

SEQ ID NO: 30790 - DNA, 28 bp, synthetic construct
  source 1..28: mol_type = other DNA
tgttttacccattaagatgcaattttgg

SEQ ID NO: 30791 - DNA, 28 bp, synthetic construct
  source 1..28: mol_type = other DNA
aattgcatcttaatgggtaaaacattgg

SEQ ID NO: 30792 - DNA, 28 bp, synthetic construct
  source 1..28: mol_type = other DNA
tgcatcttaatgggtaaaacattggtgg

SEQ ID NO: 30793 - DNA, 28 bp, synthetic construct
  source 1..28: mol_type = other DNA
taatgggtaaaacattggtggagaaagg

SEQ ID NO: 30794 - DNA, 28 bp, synthetic construct
  source 1..28: mol_type = other DNA
aatgggtaaaacattggtggagaaaggg

SEQ ID NO: 30795 - DNA, 28 bp, synthetic construct
  source 1..28: mol_type = other DNA
gaaagggcagcagaagatccccacaagg

SEQ ID NO: 30796 - DNA, 28 bp, synthetic construct
  source 1..28: mol_type = other DNA
gcagaagatccccacaaggtccttcagg

SEQ ID NO: 30797 - DNA, 28 bp, synthetic construct
  source 1..28: mol_type = other DNA
gatccccacaaggtccttcaggtacagg

SEQ ID NO: 30798 - DNA, 28 bp, synthetic construct
  source 1..28: mol_type = other DNA
atgcctgtacctgaaggaccttgtgggg

SEQ ID NO: 30799 - DNA, 28 bp, synthetic construct
  source 1..28: mol_type = other DNA
gatgcctgtacctgaaggaccttgtggg

SEQ ID NO: 30800 - DNA, 28 bp, synthetic construct
  source 1..28: mol_type = other DNA
agatgcctgtacctgaaggaccttgtgg

SEQ ID NO: 30801 - DNA, 28 bp, synthetic construct
  source 1..28: mol_type = other DNA
agcagtgggagatgcctgtacctgaagg

SEQ ID NO: 30802 - DNA, 28 bp, synthetic construct
  source 1..28: mol_type = other DNA
catctcccactgctcagagtcctgctgg

SEQ ID NO: 30803 - DNA, 28 bp, synthetic construct
  source 1..28: mol_type = other DNA
atctcccactgctcagagtcctgctggg

SEQ ID NO: 30804 - DNA, 28 bp, synthetic construct
  source 1..28: mol_type = other DNA
tctcccactgctcagagtcctgctgggg

SEQ ID NO: 30805 - DNA, 28 bp, synthetic construct
  source 1..28: mol_type = other DNA
ctcccactgctcagagtcctgctggggg

SEQ ID NO: 30806 - DNA, 28 bp, synthetic construct
  source 1..28: mol_type = other DNA
gacccccagcaggactctgagcagtggg

SEQ ID NO: 30807 - DNA, 28 bp, synthetic construct
  source 1..28: mol_type = other DNA
ggacccccagcaggactctgagcagtgg

SEQ ID NO: 30808 - DNA, 28 bp, synthetic construct
  source 1..28: mol_type = other DNA
tgtttgggacttggggacccccagcagg

SEQ ID NO: 30809 - DNA, 28 bp, synthetic construct
  source 1..28: mol_type = other DNA
tctgcttcttcttgtttgggacttgggg

SEQ ID NO: 30810 - DNA, 28 bp, synthetic construct
  source 1..28: mol_type = other DNA
ctctgcttcttcttgtttgggacttggg

SEQ ID NO: 30811 - DNA, 28 bp, synthetic construct
  source 1..28: mol_type = other DNA
tctctgcttcttcttgtttgggacttgg

SEQ ID NO: 30812 - DNA, 28 bp, synthetic construct
  source 1..28: mol_type = other DNA
ctctgctctctgcttcttcttgtttggg

SEQ ID NO: 30813 - DNA, 28 bp, synthetic construct
  source 1..28: mol_type = other DNA
actctgctctctgcttcttcttgtttgg

SEQ ID NO: 30814 - DNA, 28 bp, synthetic construct
  source 1..28: mol_type = other DNA
agcagagagcagagttcacctcttcagg

SEQ ID NO: 30815 - DNA, 28 bp, synthetic construct
  source 1..28: mol_type = other DNA
acttgtttatcttaagctcctgaagagg

SEQ ID NO: 30816 - DNA, 28 bp, synthetic construct
  source 1..28: mol_type = other DNA
gataaacaagttcatgcagcagacacgg

SEQ ID NO: 30817 - DNA, 28 bp, synthetic construct
  source 1..28: mol_type = other DNA
aacaagttcatgcagcagacacggctgg

SEQ ID NO: 30818 - DNA, 28 bp, synthetic construct
  source 1..28: mol_type = other DNA
ggacaagtgcagatggatgttgggtggg

SEQ ID NO: 30819 - DNA, 28 bp, synthetic construct
  source 1..28: mol_type = other DNA
aggacaagtgcagatggatgttgggtgg

SEQ ID NO: 30820 - DNA, 28 bp, synthetic construct
  source 1..28: mol_type = other DNA
tcaaggacaagtgcagatggatgttggg

SEQ ID NO: 30821 - DNA, 28 bp, synthetic construct
  source 1..28: mol_type = other DNA
atcaaggacaagtgcagatggatgttgg

SEQ ID NO: 30822 - DNA, 28 bp, synthetic construct
  source 1..28: mol_type = other DNA
ttttgctatcaaggacaagtgcagatgg

SEQ ID NO: 30823 - DNA, 28 bp, synthetic construct
  source 1..28: mol_type = other DNA
tgtccttgatagcaaaacctgagtctgg

SEQ ID NO: 30824 - DNA, 28 bp, synthetic construct
  source 1..28: mol_type = other DNA
aaaccagactcaggttttgctatcaagg

SEQ ID NO: 30825 - DNA, 28 bp, synthetic construct
  source 1..28: mol_type = other DNA
ttgatagcaaaacctgagtctggtttgg

SEQ ID NO: 30826 - DNA, 28 bp, synthetic construct
  source 1..28: mol_type = other DNA
tgatagcaaaacctgagtctggtttggg

SEQ ID NO: 30827 - DNA, 28 bp, synthetic construct
  source 1..28: mol_type = other DNA
gatagcaaaacctgagtctggtttgggg

SEQ ID NO: 30828 - DNA, 28 bp, synthetic construct
  source 1..28: mol_type = other DNA
cttgtgacttccccaaaccagactcagg

SEQ ID NO: 30829 - DNA, 28 bp, synthetic construct
  source 1..28: mol_type = other DNA
actagaaaatacagttatgtcagctggg

SEQ ID NO: 30830 - DNA, 28 bp, synthetic construct
  source 1..28: mol_type = other DNA
gactagaaaatacagttatgtcagctgg

SEQ ID NO: 30831 - DNA, 28 bp, synthetic construct
  source 1..28: mol_type = other DNA
ttctagtctctcttattgcaagaactgg

SEQ ID NO: 30832 - DNA, 28 bp, synthetic construct
  source 1..28: mol_type = other DNA
tctagtctctcttattgcaagaactggg

SEQ ID NO: 30833 - DNA, 28 bp, synthetic construct
  source 1..28: mol_type = other DNA
aagaactgggcatatgacttagttctgg

SEQ ID NO: 30834 - DNA, 28 bp, synthetic construct
  source 1..28: mol_type = other DNA
tgactgacataaacgggtgtcttattgg

SEQ ID NO: 30835 - DNA, 28 bp, synthetic construct
  source 1..28: mol_type = other DNA
aataagacacccgtttatgtcagtcagg

SEQ ID NO: 30836 - DNA, 28 bp, synthetic construct
  source 1..28: mol_type = other DNA
ctgagaaatcctgactgacataaacggg

SEQ ID NO: 30837 - DNA, 28 bp, synthetic construct
  source 1..28: mol_type = other DNA
tctgagaaatcctgactgacataaacgg

SEQ ID NO: 30838 - DNA, 28 bp, synthetic construct
  source 1..28: mol_type = other DNA
agaggaaggggtggtgtctactgcaggg

SEQ ID NO: 30839 - DNA, 28 bp, synthetic construct
  source 1..28: mol_type = other DNA
tagaggaaggggtggtgtctactgcagg

SEQ ID NO: 30840 - DNA, 28 bp, synthetic construct
  source 1..28: mol_type = other DNA
tgcagtagacaccaccccttcctctagg

SEQ ID NO: 30841 - DNA, 28 bp, synthetic construct
  source 1..28: mol_type = other DNA
gaagaaagtgacctagaggaaggggtgg

SEQ ID NO: 30842 - DNA, 28 bp, synthetic construct
  source 1..28: mol_type = other DNA
gaagaagaaagtgacctagaggaagggg

SEQ ID NO: 30843 - DNA, 28 bp, synthetic construct
  source 1..28: mol_type = other DNA
ggaagaagaaagtgacctagaggaaggg

SEQ ID NO: 30844 - DNA, 28 bp, synthetic construct
  source 1..28: mol_type = other DNA
aggaagaagaaagtgacctagaggaagg

SEQ ID NO: 30845 - DNA, 28 bp, synthetic construct
  source 1..28: mol_type = other DNA
ggacaggaagaagaaagtgacctagagg

SEQ ID NO: 30846 - DNA, 28 bp, synthetic construct
  source 1..28: mol_type = other DNA
gtcactttcttcttcctgtccagaaagg

SEQ ID NO: 30847 - DNA, 28 bp, synthetic construct
  source 1..28: mol_type = other DNA
actttcttcttcctgtccagaaaggtgg

SEQ ID NO: 30848 - DNA, 28 bp, synthetic construct
  source 1..28: mol_type = other DNA
tgatggcttctccacctttctggacagg

SEQ ID NO: 30849 - DNA, 28 bp, synthetic construct
  source 1..28: mol_type = other DNA
attgatgatggcttctccacctttctgg

SEQ ID NO: 30850 - DNA, 28 bp, synthetic construct
  source 1..28: mol_type = other DNA
aggtggagaagccatcatcaattttagg

SEQ ID NO: 30851 - DNA, 28 bp, synthetic construct
  source 1..28: mol_type = other DNA
tggcttttgctcctaaaattgatgatgg

SEQ ID NO: 30852 - DNA, 28 bp, synthetic construct
  source 1..28: mol_type = other DNA
aggagcaaaagccacagactaaagttgg

SEQ ID NO: 30853 - DNA, 28 bp, synthetic construct
  source 1..28: mol_type = other DNA
cttcagacttgccaactttagtctgtgg

SEQ ID NO: 30854 - DNA, 28 bp, synthetic construct
  source 1..28: mol_type = other DNA
taaagttggcaagtctgaagttaaaagg

SEQ ID NO: 30855 - DNA, 28 bp, synthetic construct
  source 1..28: mol_type = other DNA
agttggcaagtctgaagttaaaaggagg

SEQ ID NO: 30856 - DNA, 28 bp, synthetic construct
  source 1..28: mol_type = other DNA
gcaagtctgaagttaaaaggaggctagg

SEQ ID NO: 30857 - DNA, 28 bp, synthetic construct
  source 1..28: mol_type = other DNA
gtagggttatatgaagcagtcatcaagg

SEQ ID NO: 30858 - DNA, 28 bp, synthetic construct
  source 1..28: mol_type = other DNA
ctgcttcatataaccctaccatctttgg

SEQ ID NO: 30859 - DNA, 28 bp, synthetic construct
  source 1..28: mol_type = other DNA
tgggtaggatggtccaaagatggtaggg

SEQ ID NO: 30860 - DNA, 28 bp, synthetic construct
  source 1..28: mol_type = other DNA
ctgggtaggatggtccaaagatggtagg

SEQ ID NO: 30861 - DNA, 28 bp, synthetic construct
  source 1..28: mol_type = other DNA
agatctgggtaggatggtccaaagatgg

SEQ ID NO: 30862 - DNA, 28 bp, synthetic construct
  source 1..28: mol_type = other DNA
atctttggaccatcctacccagatctgg

SEQ ID NO: 30863 - DNA, 28 bp, synthetic construct
  source 1..28: mol_type = other DNA
cctaaaagtccagatctgggtaggatgg

SEQ ID NO: 30864 - DNA, 28 bp, synthetic construct
  source 1..28: mol_type = other DNA
tgttcctaaaagtccagatctgggtagg

SEQ ID NO: 30865 - DNA, 28 bp, synthetic construct
  source 1..28: mol_type = other DNA
attttgttcctaaaagtccagatctggg

SEQ ID NO: 30866 - DNA, 28 bp, synthetic construct
  source 1..28: mol_type = other DNA
tattttgttcctaaaagtccagatctgg

SEQ ID NO: 30867 - DNA, 28 bp, synthetic construct
  source 1..28: mol_type = other DNA
tttaggaacaaaataagaccctatgtgg

SEQ ID NO: 30868 - DNA, 28 bp, synthetic construct
  source 1..28: mol_type = other DNA
accctatgtggctaagccactctagcgg

SEQ ID NO: 30869 - DNA, 28 bp, synthetic construct
  source 1..28: mol_type = other DNA
accgctagagtggcttagccacataggg

SEQ ID NO: 30870 - DNA, 28 bp, synthetic construct
  source 1..28: mol_type = other DNA
caccgctagagtggcttagccacatagg

SEQ ID NO: 30871 - DNA, 28 bp, synthetic construct
  source 1..28: mol_type = other DNA
tgcaatattcaaaacaccgctagagtgg

SEQ ID NO: 30872 - DNA, 28 bp, synthetic construct
  source 1..28: mol_type = other DNA
tttaagggactgtgacttctctaatggg

SEQ ID NO: 30873 - DNA, 28 bp, synthetic construct
  source 1..28: mol_type = other DNA
atttaagggactgtgacttctctaatgg

SEQ ID NO: 30874 - DNA, 28 bp, synthetic construct
  source 1..28: mol_type = other DNA
acggcaatgtgcggggcacatttaaggg

SEQ ID NO: 30875 - DNA, 28 bp, synthetic construct
  source 1..28: mol_type = other DNA
cacggcaatgtgcggggcacatttaagg

SEQ ID NO: 30876 - DNA, 28 bp, synthetic construct
  source 1..28: mol_type = other DNA
gccccgcacattgccgtgtatagtcagg

SEQ ID NO: 30877 - DNA, 28 bp, synthetic construct
  source 1..28: mol_type = other DNA
tcctgactatacacggcaatgtgcgggg

SEQ ID NO: 30878 - DNA, 28 bp, synthetic construct
  source 1..28: mol_type = other DNA
gtcctgactatacacggcaatgtgcggg

SEQ ID NO: 30879 - DNA, 28 bp, synthetic construct
  source 1..28: mol_type = other DNA
agtcctgactatacacggcaatgtgcgg

SEQ ID NO: 30880 - DNA, 28 bp, synthetic construct
  source 1..28: mol_type = other DNA
gatatctggtagtcctgactatacacgg

SEQ ID NO: 30881 - DNA, 28 bp, synthetic construct
  source 1..28: mol_type = other DNA
attggggcatataggctgggatatctgg

SEQ ID NO: 30882 - DNA, 28 bp, synthetic construct
  source 1..28: mol_type = other DNA
agatatcccagcctatatgccccaatgg

SEQ ID NO: 30883 - DNA, 28 bp, synthetic construct
  source 1..28: mol_type = other DNA
gatatcccagcctatatgccccaatggg

SEQ ID NO: 30884 - DNA, 28 bp, synthetic construct
  source 1..28: mol_type = other DNA
atatcccagcctatatgccccaatgggg

SEQ ID NO: 30885 - DNA, 28 bp, synthetic construct
  source 1..28: mol_type = other DNA
tatcccagcctatatgccccaatggggg

SEQ ID NO: 30886 - DNA, 28 bp, synthetic construct
  source 1..28: mol_type = other DNA
ctgcccccattggggcatataggctggg

SEQ ID NO: 30887 - DNA, 28 bp, synthetic construct
  source 1..28: mol_type = other DNA
gctgcccccattggggcatataggctgg

SEQ ID NO: 30888 - DNA, 28 bp, synthetic construct
  source 1..28: mol_type = other DNA
cagtgctgcccccattggggcatatagg

SEQ ID NO: 30889 - DNA, 28 bp, synthetic construct
  source 1..28: mol_type = other DNA
ttctttggcagtgctgcccccattgggg

SEQ ID NO: 30890 - DNA, 28 bp, synthetic construct
  source 1..28: mol_type = other DNA
attctttggcagtgctgcccccattggg

SEQ ID NO: 30891 - DNA, 28 bp, synthetic construct
  source 1..28: mol_type = other DNA
aattctttggcagtgctgcccccattgg

SEQ ID NO: 30892 - DNA, 28 bp, synthetic construct
  source 1..28: mol_type = other DNA
tttttgtaaatcacacttaattctttgg

SEQ ID NO: 30893 - DNA, 28 bp, synthetic construct
  source 1..28: mol_type = other DNA
agattacatgtaaggaagtaatcacagg

SEQ ID NO: 30894 - DNA, 28 bp, synthetic construct
  source 1..28: mol_type = other DNA
tcagaagtagtcaagattacatgtaagg

SEQ ID NO: 30895 - DNA, 28 bp, synthetic construct
  source 1..28: mol_type = other DNA
tcttattaattaacttgcttacaattgg

SEQ ID NO: 30896 - DNA, 28 bp, synthetic construct
  source 1..28: mol_type = other DNA
tcaattgtctgaagactgattaatctgg

SEQ ID NO: 30897 - DNA, 28 bp, synthetic construct
  source 1..28: mol_type = other DNA
ataatatggaatattcaaaaaatgctgg

SEQ ID NO: 30898 - DNA, 28 bp, synthetic construct
  source 1..28: mol_type = other DNA
catgaaaataaagaaacaaataatatgg

SEQ ID NO: 30899 - DNA, 28 bp, synthetic construct
  source 1..28: mol_type = other DNA
tttattttcatgttatttgttaacctgg

SEQ ID NO: 30900 - DNA, 28 bp, synthetic construct
  source 1..28: mol_type = other DNA
aatttgtagttggtttcttggaagaagg

SEQ ID NO: 30901 - DNA, 28 bp, synthetic construct
  source 1..28: mol_type = other DNA
atttgtagttggtttcttggaagaaggg

SEQ ID NO: 30902 - DNA, 28 bp, synthetic construct
  source 1..28: mol_type = other DNA
gggagcttcataaagaagctagagctgg

SEQ ID NO: 30903 - DNA, 28 bp, synthetic construct
  source 1..28: mol_type = other DNA
aaagaagctagagctggccacaagaagg

SEQ ID NO: 30904 - DNA, 28 bp, synthetic construct
  source 1..28: mol_type = other DNA
cttgttgtgggcattttccttcttgtgg

SEQ ID NO: 30905 - DNA, 28 bp, synthetic construct
  source 1..28: mol_type = other DNA
agaaggaaaatgcccacaacaagatagg

SEQ ID NO: 30906 - DNA, 28 bp, synthetic construct
  source 1..28: mol_type = other DNA
aggaaaatgcccacaacaagataggagg

SEQ ID NO: 30907 - DNA, 28 bp, synthetic construct
  source 1..28: mol_type = other DNA
aaatgcccacaacaagataggaggcagg

SEQ ID NO: 30908 - DNA, 28 bp, synthetic construct
  source 1..28: mol_type = other DNA
ggtttcctgcctcctatcttgttgtggg

SEQ ID NO: 30909 - DNA, 28 bp, synthetic construct
  source 1..28: mol_type = other DNA
gggtttcctgcctcctatcttgttgtgg

SEQ ID NO: 30910 - DNA, 28 bp, synthetic construct
  source 1..28: mol_type = other DNA
aacaagataggaggcaggaaacccctgg

SEQ ID NO: 30911 - DNA, 28 bp, synthetic construct
  source 1..28: mol_type = other DNA
gcaggtaggtatctttcttttccagggg

SEQ ID NO: 30912 - DNA, 28 bp, synthetic construct
  source 1..28: mol_type = other DNA
agcaggtaggtatctttcttttccaggg

SEQ ID NO: 30913 - DNA, 28 bp, synthetic construct
  source 1..28: mol_type = other DNA
tagcaggtaggtatctttcttttccagg

SEQ ID NO: 30914 - DNA, 28 bp, synthetic construct
  source 1..28: mol_type = other DNA
gaaagatacctacctgctagttctcagg

SEQ ID NO: 30915 - DNA, 28 bp, synthetic construct
  source 1..28: mol_type = other DNA
aaagatacctacctgctagttctcaggg

SEQ ID NO: 30916 - DNA, 28 bp, synthetic construct
  source 1..28: mol_type = other DNA
acctacctgctagttctcagggaagagg

SEQ ID NO: 30917 - DNA, 28 bp, synthetic construct
  source 1..28: mol_type = other DNA
gcctcttccctgagaactagcaggtagg

SEQ ID NO: 30918 - DNA, 28 bp, synthetic construct
  source 1..28: mol_type = other DNA
acctgctagttctcagggaagaggctgg

SEQ ID NO: 30919 - DNA, 28 bp, synthetic construct
  source 1..28: mol_type = other DNA
cccagcctcttccctgagaactagcagg

SEQ ID NO: 30920 - DNA, 28 bp, synthetic construct
  source 1..28: mol_type = other DNA
tagttctcagggaagaggctgggccagg

SEQ ID NO: 30921 - DNA, 28 bp, synthetic construct
  source 1..28: mol_type = other DNA
ctcagggaagaggctgggccaggcatgg

SEQ ID NO: 30922 - DNA, 28 bp, synthetic construct
  source 1..28: mol_type = other DNA
agggaagaggctgggccaggcatggtgg

SEQ ID NO: 30923 - DNA, 28 bp, synthetic construct
  source 1..28: mol_type = other DNA
gattacaggcatgagccaccatgcctgg

SEQ ID NO: 30924 - DNA, 28 bp, synthetic construct
  source 1..28: mol_type = other DNA
atgcctgtaatcccagtactttgagagg

SEQ ID NO: 30925 - DNA, 28 bp, synthetic construct
  source 1..28: mol_type = other DNA
cagcctctcaaagtactgggattacagg

SEQ ID NO: 30926 - DNA, 28 bp, synthetic construct
  source 1..28: mol_type = other DNA
gtaatcccagtactttgagaggctgagg

SEQ ID NO: 30927 - DNA, 28 bp, synthetic construct
  source 1..28: mol_type = other DNA
tcccagtactttgagaggctgaggctgg

SEQ ID NO: 30928 - DNA, 28 bp, synthetic construct
  source 1..28: mol_type = other DNA
tccagcctcagcctctcaaagtactggg

SEQ ID NO: 30929 - DNA, 28 bp, synthetic construct
  source 1..28: mol_type = other DNA
ctccagcctcagcctctcaaagtactgg

SEQ ID NO: 30930 - DNA, 28 bp, synthetic construct
  source 1..28: mol_type = other DNA
cagtactttgagaggctgaggctggagg

SEQ ID NO: 30931 - DNA, 28 bp, synthetic construct
  source 1..28: mol_type = other DNA
ctgaggctggaggatcacttaagccagg

SEQ ID NO: 30932 - DNA, 28 bp, synthetic construct
  source 1..28: mol_type = other DNA
ttaagccaggagttcaagacaagcctgg

SEQ ID NO: 30933 - DNA, 28 bp, synthetic construct
  source 1..28: mol_type = other DNA
taagccaggagttcaagacaagcctggg

SEQ ID NO: 30934 - DNA, 28 bp, synthetic construct
  source 1..28: mol_type = other DNA
gtcgcccaggcttgtcttgaactcctgg

SEQ ID NO: 30935 - DNA, 28 bp, synthetic construct
  source 1..28: mol_type = other DNA
gagttcaagacaagcctgggcgacatgg

SEQ ID NO: 30936 - DNA, 28 bp, synthetic construct
  source 1..28: mol_type = other DNA
gggacagggtctcaccatgtcgcccagg

SEQ ID NO: 30937 - DNA, 28 bp, synthetic construct
  source 1..28: mol_type = other DNA
taattttttattttttgtagggacaggg

SEQ ID NO: 30938 - DNA, 28 bp, synthetic construct
  source 1..28: mol_type = other DNA
ctaattttttattttttgtagggacagg

SEQ ID NO: 30939 - DNA, 28 bp, synthetic construct
  source 1..28: mol_type = other DNA
tccctacaaaaaataaaaaattagctgg

SEQ ID NO: 30940 - DNA, 28 bp, synthetic construct
  source 1..28: mol_type = other DNA
gccagctaattttttattttttgtaggg

SEQ ID NO: 30941 - DNA, 28 bp, synthetic construct
  source 1..28: mol_type = other DNA
ggccagctaattttttattttttgtagg

SEQ ID NO: 30942 - DNA, 28 bp, synthetic construct
  source 1..28: mol_type = other DNA
caaaaaataaaaaattagctggccatgg

SEQ ID NO: 30943 - DNA, 28 bp, synthetic construct
  source 1..28: mol_type = other DNA
aaaataaaaaattagctggccatggtgg

SEQ ID NO: 30944 - DNA, 28 bp, synthetic construct
  source 1..28: mol_type = other DNA
ctgggactacaagtgtgtgccaccatgg

SEQ ID NO: 30945 - DNA, 28 bp, synthetic construct
  source 1..28: mol_type = other DNA
acacttgtagtcccagctactcaagagg

SEQ ID NO: 30946 - DNA, 28 bp, synthetic construct
  source 1..28: mol_type = other DNA
gtagtcccagctactcaagaggctgagg

SEQ ID NO: 30947 - DNA, 28 bp, synthetic construct
  source 1..28: mol_type = other DNA
gtcccagctactcaagaggctgaggtgg

SEQ ID NO: 30948 - DNA, 28 bp, synthetic construct
  source 1..28: mol_type = other DNA
tcccagctactcaagaggctgaggtggg

SEQ ID NO: 30949 - DNA, 28 bp, synthetic construct
  source 1..28: mol_type = other DNA
tcccacctcagcctcttgagtagctggg

SEQ ID NO: 30950 - DNA, 28 bp, synthetic construct
  source 1..28: mol_type = other DNA
ctcccacctcagcctcttgagtagctgg

SEQ ID NO: 30951 - DNA, 28 bp, synthetic construct
  source 1..28: mol_type = other DNA
cagctactcaagaggctgaggtgggagg

SEQ ID NO: 30952 - DNA, 28 bp, synthetic construct
  source 1..28: mol_type = other DNA
gaggatcacttgagctccaaagtcaagg

SEQ ID NO: 30953 - DNA, 28 bp, synthetic construct
  source 1..28: mol_type = other DNA
tcacagctcactgcagccttgactttgg

SEQ ID NO: 30954 - DNA, 28 bp, synthetic construct
  source 1..28: mol_type = other DNA
gaatagatattttagttacgttaagcgg

SEQ ID NO: 30955 - DNA, 28 bp, synthetic construct
  source 1..28: mol_type = other DNA
taaaatatctattctgatgagattctgg

SEQ ID NO: 30956 - DNA, 28 bp, synthetic construct
  source 1..28: mol_type = other DNA
tatgattcgaggggaaaagtcatttggg

SEQ ID NO: 30957 - DNA, 28 bp, synthetic construct
  source 1..28: mol_type = other DNA
ctatgattcgaggggaaaagtcatttgg

SEQ ID NO: 30958 - DNA, 28 bp, synthetic construct
  source 1..28: mol_type = other DNA
caaatgacttttcccctcgaatcatagg

SEQ ID NO: 30959 - DNA, 28 bp, synthetic construct
  source 1..28: mol_type = other DNA
ctgctgcagtttcctatgattcgagggg

SEQ ID NO: 30960 - DNA, 28 bp, synthetic construct
  source 1..28: mol_type = other DNA
tctgctgcagtttcctatgattcgaggg

SEQ ID NO: 30961 - DNA, 28 bp, synthetic construct
  source 1..28: mol_type = other DNA
ctctgctgcagtttcctatgattcgagg

SEQ ID NO: 30962 - DNA, 28 bp, synthetic construct
  source 1..28: mol_type = other DNA
atgtgtacctgcttgccagttactccgg

SEQ ID NO: 30963 - DNA, 28 bp, synthetic construct
  source 1..28: mol_type = other DNA
catcaatccggagtaactggcaagcagg

SEQ ID NO: 30964 - DNA, 28 bp, synthetic construct
  source 1..28: mol_type = other DNA
tcgggaagcatcaatccggagtaactgg

SEQ ID NO: 30965 - DNA, 28 bp, synthetic construct
  source 1..28: mol_type = other DNA
ttgtttacatcgggaagcatcaatccgg

SEQ ID NO: 30966 - DNA, 28 bp, synthetic construct
  source 1..28: mol_type = other DNA
gattgatgcttcccgatgtaaacaatgg

SEQ ID NO: 30967 - DNA, 28 bp, synthetic construct
  source 1..28: mol_type = other DNA
cttacgatcagccattgtttacatcggg

SEQ ID NO: 30968 - DNA, 28 bp, synthetic construct
  source 1..28: mol_type = other DNA
ccttacgatcagccattgtttacatcgg

SEQ ID NO: 30969 - DNA, 28 bp, synthetic construct
  source 1..28: mol_type = other DNA
aaactttctgcaaaacaaaagcgattgg

SEQ ID NO: 30970 - DNA, 28 bp, synthetic construct
  source 1..28: mol_type = other DNA
aactttctgcaaaacaaaagcgattggg

SEQ ID NO: 30971 - DNA, 28 bp, synthetic construct
  source 1..28: mol_type = other DNA
gcaaaacaaaagcgattgggtatttagg

SEQ ID NO: 30972 - DNA, 28 bp, synthetic construct
  source 1..28: mol_type = other DNA
aaaaacatcagtttagtagtttccctgg

SEQ ID NO: 30973 - DNA, 28 bp, synthetic construct
  source 1..28: mol_type = other DNA
acacagagttataggacatttgccaggg

SEQ ID NO: 30974 - DNA, 28 bp, synthetic construct
  source 1..28: mol_type = other DNA
cacacagagttataggacatttgccagg

SEQ ID NO: 30975 - DNA, 28 bp, synthetic construct
  source 1..28: mol_type = other DNA
cacacacacacacacacagagttatagg

SEQ ID NO: 30976 - DNA, 28 bp, synthetic construct
  source 1..28: mol_type = other DNA
agctgtgcccatgctccgctggtcaggg

SEQ ID NO: 30977 - DNA, 28 bp, synthetic construct
  source 1..28: mol_type = other DNA
tagctgtgcccatgctccgctggtcagg

SEQ ID NO: 30978 - DNA, 28 bp, synthetic construct
  source 1..28: mol_type = other DNA
ctaagtagctgtgcccatgctccgctgg

SEQ ID NO: 30979 - DNA, 28 bp, synthetic construct
  source 1..28: mol_type = other DNA
acagctacttagagcgccacccttcagg

SEQ ID NO: 30980 - DNA, 28 bp, synthetic construct
  source 1..28: mol_type = other DNA
agcgccacccttcaggacacaaagtcgg

SEQ ID NO: 30981 - DNA, 28 bp, synthetic construct
  source 1..28: mol_type = other DNA
gcgccacccttcaggacacaaagtcggg

SEQ ID NO: 30982 - DNA, 28 bp, synthetic construct
  source 1..28: mol_type = other DNA
cgccacccttcaggacacaaagtcgggg

SEQ ID NO: 30983 - DNA, 28 bp, synthetic construct
  source 1..28: mol_type = other DNA
agccccgactttgtgtcctgaagggtgg

SEQ ID NO: 30984 - DNA, 28 bp, synthetic construct
  source 1..28: mol_type = other DNA
ggtagccccgactttgtgtcctgaaggg

SEQ ID NO: 30985 - DNA, 28 bp, synthetic construct
  source 1..28: mol_type = other DNA
aggtagccccgactttgtgtcctgaagg

SEQ ID NO: 30986 - DNA, 28 bp, synthetic construct
  source 1..28: mol_type = other DNA
acaaagtcggggctacctctcttccagg

SEQ ID NO: 30987 - DNA, 28 bp, synthetic construct
  source 1..28: mol_type = other DNA
gtcggggctacctctcttccaggcaagg

SEQ ID NO: 30988 - DNA, 28 bp, synthetic construct
  source 1..28: mol_type = other DNA
ctctaggatgccttgcctggaagagagg

SEQ ID NO: 30989 - DNA, 28 bp, synthetic construct
  source 1..28: mol_type = other DNA
ctctcttccaggcaaggcatcctagagg

SEQ ID NO: 30990 - DNA, 28 bp, synthetic construct
  source 1..28: mol_type = other DNA
tctcttccaggcaaggcatcctagaggg

SEQ ID NO: 30991 - DNA, 28 bp, synthetic construct
  source 1..28: mol_type = other DNA
tgcgggccctctaggatgccttgcctgg

SEQ ID NO: 30992 - DNA, 28 bp, synthetic construct
  source 1..28: mol_type = other DNA
aaactggagggtgtgcgggccctctagg

SEQ ID NO: 30993 - DNA, 28 bp, synthetic construct
  source 1..28: mol_type = other DNA
ggtaagatcaaactggagggtgtgcggg

SEQ ID NO: 30994 - DNA, 28 bp, synthetic construct
  source 1..28: mol_type = other DNA
aggtaagatcaaactggagggtgtgcgg

SEQ ID NO: 30995 - DNA, 28 bp, synthetic construct
  source 1..28: mol_type = other DNA
agctgagaggtaagatcaaactggaggg

SEQ ID NO: 30996 - DNA, 28 bp, synthetic construct
  source 1..28: mol_type = other DNA
gagctgagaggtaagatcaaactggagg

SEQ ID NO: 30997 - DNA, 28 bp, synthetic construct
  source 1..28: mol_type = other DNA
cgggagctgagaggtaagatcaaactgg

SEQ ID NO: 30998 - DNA, 28 bp, synthetic construct
  source 1..28: mol_type = other DNA
agaaagaaaaggaacgggagctgagagg

SEQ ID NO: 30999 - DNA, 28 bp, synthetic construct
  source 1..28: mol_type = other DNA
tactggggagagaaagaaaaggaacggg

SEQ ID NO: 31000 - DNA, 28 bp, synthetic construct
  source 1..28: mol_type = other DNA
ttactggggagagaaagaaaaggaacgg

SEQ ID NO: 31001 - DNA, 28 bp, synthetic construct
  source 1..28: mol_type = other DNA
acgacttactggggagagaaagaaaagg

SEQ ID NO: 31002 - DNA, 28 bp, synthetic construct
  source 1..28: mol_type = other DNA
aagaaagacgttcaacgacttactgggg

SEQ ID NO: 31003 - DNA, 28 bp, synthetic construct
  source 1..28: mol_type = other DNA
gaagaaagacgttcaacgacttactggg

SEQ ID NO: 31004 - DNA, 28 bp, synthetic construct
  source 1..28: mol_type = other DNA
agaagaaagacgttcaacgacttactgg

SEQ ID NO: 31005 - DNA, 28 bp, synthetic construct
  source 1..28: mol_type = other DNA
taagtcgttgaacgtctttcttctgagg

SEQ ID NO: 31006 - DNA, 28 bp, synthetic construct
  source 1..28: mol_type = other DNA
aacgtctttcttctgaggctgagcgtgg

SEQ ID NO: 31007 - DNA, 28 bp, synthetic construct
  source 1..28: mol_type = other DNA
gctgagcgtggagctctcttctcgctgg

SEQ ID NO: 31008 - DNA, 28 bp, synthetic construct
  source 1..28: mol_type = other DNA
tcttctcgctggcgagctttctgaatgg

SEQ ID NO: 31009 - DNA, 28 bp, synthetic construct
  source 1..28: mol_type = other DNA
tctgaatggcactttctgtacaaacagg

SEQ ID NO: 31010 - DNA, 28 bp, synthetic construct
  source 1..28: mol_type = other DNA
tctgtacaaacaggaagagcatgtgtgg

SEQ ID NO: 31011 - DNA, 28 bp, synthetic construct
  source 1..28: mol_type = other DNA
atgtgtggtcacaacccaagtgtgcagg

SEQ ID NO: 31012 - DNA, 28 bp, synthetic construct
  source 1..28: mol_type = other DNA
aacccaagtgtgcaggtgttgatagagg

SEQ ID NO: 31013 - DNA, 28 bp, synthetic construct
  source 1..28: mol_type = other DNA
atcctctatcaacacctgcacacttggg

SEQ ID NO: 31014 - DNA, 28 bp, synthetic construct
  source 1..28: mol_type = other DNA
catcctctatcaacacctgcacacttgg

SEQ ID NO: 31015 - DNA, 28 bp, synthetic construct
  source 1..28: mol_type = other DNA
ggtgttgatagaggatgtgaaagtgtgg

SEQ ID NO: 31016 - DNA, 28 bp, synthetic construct
  source 1..28: mol_type = other DNA
gttgatagaggatgtgaaagtgtggagg

SEQ ID NO: 31017 - DNA, 28 bp, synthetic construct
  source 1..28: mol_type = other DNA
cgagtgactaaaccagatacccaaccgg

SEQ ID NO: 31018 - DNA, 28 bp, synthetic construct
  source 1..28: mol_type = other DNA
agtgagagttggccggttgggtatctgg

SEQ ID NO: 31019 - DNA, 28 bp, synthetic construct
  source 1..28: mol_type = other DNA
tacccaaccggccaactctcacttgtgg

SEQ ID NO: 31020 - DNA, 28 bp, synthetic construct
  source 1..28: mol_type = other DNA
tgccacaagtgagagttggccggttggg

SEQ ID NO: 31021 - DNA, 28 bp, synthetic construct
  source 1..28: mol_type = other DNA
ctgccacaagtgagagttggccggttgg

SEQ ID NO: 31022 - DNA, 28 bp, synthetic construct
  source 1..28: mol_type = other DNA
caaccggccaactctcacttgtggcagg

SEQ ID NO: 31023 - DNA, 28 bp, synthetic construct
  source 1..28: mol_type = other DNA
aaccggccaactctcacttgtggcaggg

SEQ ID NO: 31024 - DNA, 28 bp, synthetic construct
  source 1..28: mol_type = other DNA
ggccctgccacaagtgagagttggccgg

SEQ ID NO: 31025 - DNA, 28 bp, synthetic construct
  source 1..28: mol_type = other DNA
gccaactctcacttgtggcagggcctgg

SEQ ID NO: 31026 - DNA, 28 bp, synthetic construct
  source 1..28: mol_type = other DNA
accaggccctgccacaagtgagagttgg

SEQ ID NO: 31027 - DNA, 28 bp, synthetic construct
  source 1..28: mol_type = other DNA
ttgtggcagggcctggtctaccagaagg

SEQ ID NO: 31028 - DNA, 28 bp, synthetic construct
  source 1..28: mol_type = other DNA
ggcagggcctggtctaccagaaggctgg

SEQ ID NO: 31029 - DNA, 28 bp, synthetic construct
  source 1..28: mol_type = other DNA
cctggtctaccagaaggctggaagcagg

SEQ ID NO: 31030 - DNA, 28 bp, synthetic construct
  source 1..28: mol_type = other DNA
taccagaaggctggaagcaggaacctgg

SEQ ID NO: 31031 - DNA, 28 bp, synthetic construct
  source 1..28: mol_type = other DNA
gtccaggttcctgcttccagccttctgg

SEQ ID NO: 31032 - DNA, 28 bp, synthetic construct
  source 1..28: mol_type = other DNA
ggaagcaggaacctggactctactctgg

SEQ ID NO: 31033 - DNA, 28 bp, synthetic construct
  source 1..28: mol_type = other DNA
gaagcaggaacctggactctactctggg

SEQ ID NO: 31034 - DNA, 28 bp, synthetic construct
  source 1..28: mol_type = other DNA
aagcaggaacctggactctactctgggg

SEQ ID NO: 31035 - DNA, 28 bp, synthetic construct
  source 1..28: mol_type = other DNA
agttggtctccccagagtagagtccagg

SEQ ID NO: 31036 - DNA, 28 bp, synthetic construct
  source 1..28: mol_type = other DNA
tggggagaccaactgacaaaagcagagg

SEQ ID NO: 31037 - DNA, 28 bp, synthetic construct
  source 1..28: mol_type = other DNA
gagaccaactgacaaaagcagaggatgg

SEQ ID NO: 31038 - DNA, 28 bp, synthetic construct
  source 1..28: mol_type = other DNA
accaactgacaaaagcagaggatggtgg

SEQ ID NO: 31039 - DNA, 28 bp, synthetic construct
  source 1..28: mol_type = other DNA
gccaccatcctctgcttttgtcagttgg

SEQ ID NO: 31040 - DNA, 28 bp, synthetic construct
  source 1..28: mol_type = other DNA
tgacaaaagcagaggatggtggccctgg

SEQ ID NO: 31041 - DNA, 28 bp, synthetic construct
  source 1..28: mol_type = other DNA
caaaagcagaggatggtggccctggagg

SEQ ID NO: 31042 - DNA, 28 bp, synthetic construct
  source 1..28: mol_type = other DNA
cagaggatggtggccctggaggccaagg

SEQ ID NO: 31043 - DNA, 28 bp, synthetic construct
  source 1..28: mol_type = other DNA
agaggatggtggccctggaggccaaggg

SEQ ID NO: 31044 - DNA, 28 bp, synthetic construct
  source 1..28: mol_type = other DNA
tggtggccctggaggccaagggagaagg

SEQ ID NO: 31045 - DNA, 28 bp, synthetic construct
  source 1..28: mol_type = other DNA
aagagaccttctcccttggcctccaggg

SEQ ID NO: 31046 - DNA, 28 bp, synthetic construct
  source 1..28: mol_type = other DNA
aaagagaccttctcccttggcctccagg

SEQ ID NO: 31047 - DNA, 28 bp, synthetic construct
  source 1..28: mol_type = other DNA
caggagtcaaagagaccttctcccttgg

SEQ ID NO: 31048 - DNA, 28 bp, synthetic construct
  source 1..28: mol_type = other DNA
gggtctgcatagggttagaaagcacagg

SEQ ID NO: 31049 - DNA, 28 bp, synthetic construct
  source 1..28: mol_type = other DNA
tgggattcttttatgggtctgcataggg

SEQ ID NO: 31050 - DNA, 28 bp, synthetic construct
  source 1..28: mol_type = other DNA
ctgggattcttttatgggtctgcatagg

SEQ ID NO: 31051 - DNA, 28 bp, synthetic construct
  source 1..28: mol_type = other DNA
ctatgcagacccataaaagaatcccagg

SEQ ID NO: 31052 - DNA, 28 bp, synthetic construct
  source 1..28: mol_type = other DNA
caaaatgttcctgggattcttttatggg

SEQ ID NO: 31053 - DNA, 28 bp, synthetic construct
  source 1..28: mol_type = other DNA
ccataaaagaatcccaggaacattttgg

SEQ ID NO: 31054 - DNA, 28 bp, synthetic construct
  source 1..28: mol_type = other DNA
atctaagagattccaaaatgttcctggg

SEQ ID NO: 31055 - DNA, 28 bp, synthetic construct
  source 1..28: mol_type = other DNA
tatctaagagattccaaaatgttcctgg

SEQ ID NO: 31056 - DNA, 28 bp, synthetic construct
  source 1..28: mol_type = other DNA
tgattatcaagaatgttgatttcaatgg

SEQ ID NO: 31057 - DNA, 28 bp, synthetic construct
  source 1..28: mol_type = other DNA
gattatcaagaatgttgatttcaatggg

SEQ ID NO: 31058 - DNA, 28 bp, synthetic construct
  source 1..28: mol_type = other DNA
ctgcttaacttgtccaaagctctgctgg

SEQ ID NO: 31059 - DNA, 28 bp, synthetic construct
  source 1..28: mol_type = other DNA
ttgtccaaagctctgctggtttcccagg

SEQ ID NO: 31060 - DNA, 28 bp, synthetic construct
  source 1..28: mol_type = other DNA
acagcctgggaaaccagcagagctttgg

SEQ ID NO: 31061 - DNA, 28 bp, synthetic construct
  source 1..28: mol_type = other DNA
agctctgctggtttcccaggctgtctgg

SEQ ID NO: 31062 - DNA, 28 bp, synthetic construct
  source 1..28: mol_type = other DNA
gctctgctggtttcccaggctgtctggg

SEQ ID NO: 31063 - DNA, 28 bp, synthetic construct
  source 1..28: mol_type = other DNA
gatctcttggaggcccagacagcctggg

SEQ ID NO: 31064 - DNA, 28 bp, synthetic construct
  source 1..28: mol_type = other DNA
tgatctcttggaggcccagacagcctgg

SEQ ID NO: 31065 - DNA, 28 bp, synthetic construct
  source 1..28: mol_type = other DNA
aggctgtctgggcctccaagagatcagg

SEQ ID NO: 31066 - DNA, 28 bp, synthetic construct
  source 1..28: mol_type = other DNA
tgggcctccaagagatcaggaccaaagg

SEQ ID NO: 31067 - DNA, 28 bp, synthetic construct
  source 1..28: mol_type = other DNA
tgagcctttggtcctgatctcttggagg

SEQ ID NO: 31068 - DNA, 28 bp, synthetic construct
  source 1..28: mol_type = other DNA
ggatgagcctttggtcctgatctcttgg

SEQ ID NO: 31069 - DNA, 28 bp, synthetic construct
  source 1..28: mol_type = other DNA
tcaggaccaaaggctcatcctgcattgg

SEQ ID NO: 31070 - DNA, 28 bp, synthetic construct
  source 1..28: mol_type = other DNA
acagttccaatgcaggatgagcctttgg

SEQ ID NO: 31071 - DNA, 28 bp, synthetic construct
  source 1..28: mol_type = other DNA
ggaagacttgtcacagttccaatgcagg

SEQ ID NO: 31072 - DNA, 28 bp, synthetic construct
  source 1..28: mol_type = other DNA
ggtgtagctttgttctagaaaggtctgg

SEQ ID NO: 31073 - DNA, 28 bp, synthetic construct
  source 1..28: mol_type = other DNA
gacctttctagaacaaagctacaccagg

SEQ ID NO: 31074 - DNA, 28 bp, synthetic construct
  source 1..28: mol_type = other DNA
ttcctggtgtagctttgttctagaaagg

SEQ ID NO: 31075 - DNA, 28 bp, synthetic construct
  source 1..28: mol_type = other DNA
agctacaccaggaaagaagagtcttagg

SEQ ID NO: 31076 - DNA, 28 bp, synthetic construct
  source 1..28: mol_type = other DNA
caccaggaaagaagagtcttaggcaagg

SEQ ID NO: 31077 - DNA, 28 bp, synthetic construct
  source 1..28: mol_type = other DNA
ttccttgcctaagactcttctttcctgg

SEQ ID NO: 31078 - DNA, 28 bp, synthetic construct
  source 1..28: mol_type = other DNA
cttaggcaaggaatcagatgtcctaagg

SEQ ID NO: 31079 - DNA, 28 bp, synthetic construct
  source 1..28: mol_type = other DNA
catgtaggtcatgtagagcagccttagg

SEQ ID NO: 31080 - DNA, 28 bp, synthetic construct
  source 1..28: mol_type = other DNA
aggctgctctacatgacctacatgatgg

SEQ ID NO: 31081 - DNA, 28 bp, synthetic construct
  source 1..28: mol_type = other DNA
ggctgctctacatgacctacatgatggg

SEQ ID NO: 31082 - DNA, 28 bp, synthetic construct
  source 1..28: mol_type = other DNA
gatgaggaggtaacacccatcatgtagg

SEQ ID NO: 31083 - DNA, 28 bp, synthetic construct
  source 1..28: mol_type = other DNA
tgggttgactgaatgggagatgaggagg

SEQ ID NO: 31084 - DNA, 28 bp, synthetic construct
  source 1..28: mol_type = other DNA
cctcatctcccattcagtcaacccacgg

SEQ ID NO: 31085 - DNA, 28 bp, synthetic construct
  source 1..28: mol_type = other DNA
ctcatctcccattcagtcaacccacggg

SEQ ID NO: 31086 - DNA, 28 bp, synthetic construct
  source 1..28: mol_type = other DNA
tcccattcagtcaacccacgggcactgg

SEQ ID NO: 31087 - DNA, 28 bp, synthetic construct
  source 1..28: mol_type = other DNA
tccagtgcccgtgggttgactgaatggg

SEQ ID NO: 31088 - DNA, 28 bp, synthetic construct
  source 1..28: mol_type = other DNA
gtccagtgcccgtgggttgactgaatgg

SEQ ID NO: 31089 - DNA, 28 bp, synthetic construct
  source 1..28: mol_type = other DNA
gtcgggcaggaagtccagtgcccgtggg

SEQ ID NO: 31090 - DNA, 28 bp, synthetic construct
  source 1..28: mol_type = other DNA
tgtcgggcaggaagtccagtgcccgtgg

SEQ ID NO: 31091 - DNA, 28 bp, synthetic construct
  source 1..28: mol_type = other DNA
atggggagagggaagggtgtcgggcagg

SEQ ID NO: 31092 - DNA, 28 bp, synthetic construct
  source 1..28: mol_type = other DNA
atgaatggggagagggaagggtgtcggg

SEQ ID NO: 31093 - DNA, 28 bp, synthetic construct
  source 1..28: mol_type = other DNA
catgaatggggagagggaagggtgtcgg

SEQ ID NO: 31094 - DNA, 28 bp, synthetic construct
  source 1..28: mol_type = other DNA
acccttccctctccccattcatgcctgg

SEQ ID NO: 31095 - DNA, 28 bp, synthetic construct
  source 1..28: mol_type = other DNA
tccaggcatgaatggggagagggaaggg

SEQ ID NO: 31096 - DNA, 28 bp, synthetic construct
  source 1..28: mol_type = other DNA
ttccaggcatgaatggggagagggaagg

SEQ ID NO: 31097 - DNA, 28 bp, synthetic construct
  source 1..28: mol_type = other DNA
ataattccaggcatgaatggggagaggg

SEQ ID NO: 31098 - DNA, 28 bp, synthetic construct
  source 1..28: mol_type = other DNA
aataattccaggcatgaatggggagagg

SEQ ID NO: 31099 - DNA, 28 bp, synthetic construct
  source 1..28: mol_type = other DNA
gtgaaaataattccaggcatgaatgggg

SEQ ID NO: 31100 - DNA, 28 bp, synthetic construct
  source 1..28: mol_type = other DNA
agtgaaaataattccaggcatgaatggg

SEQ ID NO: 31101 - DNA, 28 bp, synthetic construct
  source 1..28: mol_type = other DNA
tagtgaaaataattccaggcatgaatgg

SEQ ID NO: 31102 - DNA, 28 bp, synthetic construct
  source 1..28: mol_type = other DNA
tggtgtcattagtgaaaataattccagg

SEQ ID NO: 31103 - DNA, 28 bp, synthetic construct
  source 1..28: mol_type = other DNA
tggaattattttcactaatgacaccagg

SEQ ID NO: 31104 - DNA, 28 bp, synthetic construct
  source 1..28: mol_type = other DNA
ggaattattttcactaatgacaccaggg

SEQ ID NO: 31105 - DNA, 28 bp, synthetic construct
  source 1..28: mol_type = other DNA
actaatgacaccagggattcactaatgg

SEQ ID NO: 31106 - DNA, 28 bp, synthetic construct
  source 1..28: mol_type = other DNA
gaaaaagcatccattagtgaatccctgg

SEQ ID NO: 31107 - DNA, 28 bp, synthetic construct
  source 1..28: mol_type = other DNA
cagttcctgtcctatttgtctccactgg

SEQ ID NO: 31108 - DNA, 28 bp, synthetic construct
  source 1..28: mol_type = other DNA
cactgccagtggagacaaataggacagg

SEQ ID NO: 31109 - DNA, 28 bp, synthetic construct
  source 1..28: mol_type = other DNA
tcaaacactgccagtggagacaaatagg

SEQ ID NO: 31110 - DNA, 28 bp, synthetic construct
  source 1..28: mol_type = other DNA
ctacagggaagtcaaacactgccagtgg

SEQ ID NO: 31111 - DNA, 28 bp, synthetic construct
  source 1..28: mol_type = other DNA
gaggaaagaaatggtcaacactacaggg

SEQ ID NO: 31112 - DNA, 28 bp, synthetic construct
  source 1..28: mol_type = other DNA
ggaggaaagaaatggtcaacactacagg

SEQ ID NO: 31113 - DNA, 28 bp, synthetic construct
  source 1..28: mol_type = other DNA
ggcagaagttctgggaggaaagaaatgg

SEQ ID NO: 31114 - DNA, 28 bp, synthetic construct
  source 1..28: mol_type = other DNA
tttctttcctcccagaacttctgcctgg

SEQ ID NO: 31115 - DNA, 28 bp, synthetic construct
  source 1..28: mol_type = other DNA
ttctttcctcccagaacttctgcctggg

SEQ ID NO: 31116 - DNA, 28 bp, synthetic construct
  source 1..28: mol_type = other DNA
tggcggcccaggcagaagttctgggagg

SEQ ID NO: 31117 - DNA, 28 bp, synthetic construct
  source 1..28: mol_type = other DNA
tcatggcggcccaggcagaagttctggg

SEQ ID NO: 31118 - DNA, 28 bp, synthetic construct
  source 1..28: mol_type = other DNA
gtcatggcggcccaggcagaagttctgg

SEQ ID NO: 31119 - DNA, 28 bp, synthetic construct
  source 1..28: mol_type = other DNA
ggagagtatggagtcatggcggcccagg

SEQ ID NO: 31120 - DNA, 28 bp, synthetic construct
  source 1..28: mol_type = other DNA
gggccgccatgactccatactctcctgg

SEQ ID NO: 31121 - DNA, 28 bp, synthetic construct
  source 1..28: mol_type = other DNA
aaaccaggagagtatggagtcatggcgg

SEQ ID NO: 31122 - DNA, 28 bp, synthetic construct
  source 1..28: mol_type = other DNA
caaaaaccaggagagtatggagtcatgg

SEQ ID NO: 31123 - DNA, 28 bp, synthetic construct
  source 1..28: mol_type = other DNA
actccatactctcctggtttttgtcagg

SEQ ID NO: 31124 - DNA, 28 bp, synthetic construct
  source 1..28: mol_type = other DNA
ccgcctgacaaaaaccaggagagtatgg

SEQ ID NO: 31125 - DNA, 28 bp, synthetic construct
  source 1..28: mol_type = other DNA
tgtgagagaccgcctgacaaaaaccagg

SEQ ID NO: 31126 - DNA, 28 bp, synthetic construct
  source 1..28: mol_type = other DNA
gtttttgtcaggcggtctctcacactgg

SEQ ID NO: 31127 - DNA, 28 bp, synthetic construct
  source 1..28: mol_type = other DNA
ttgtcaggcggtctctcacactggcagg

SEQ ID NO: 31128 - DNA, 28 bp, synthetic construct
  source 1..28: mol_type = other DNA
ctcacactggcaggcttccattctttgg

SEQ ID NO: 31129 - DNA, 28 bp, synthetic construct
  source 1..28: mol_type = other DNA
gagggcgaaaattaagaccaaagaatgg

SEQ ID NO: 31130 - DNA, 28 bp, synthetic construct
  source 1..28: mol_type = other DNA
gaggcggagagtggagcttgcaggaggg

SEQ ID NO: 31131 - DNA, 28 bp, synthetic construct
  source 1..28: mol_type = other DNA
tgaggcggagagtggagcttgcaggagg

SEQ ID NO: 31132 - DNA, 28 bp, synthetic construct
  source 1..28: mol_type = other DNA
ccatgaggcggagagtggagcttgcagg

SEQ ID NO: 31133 - DNA, 28 bp, synthetic construct
  source 1..28: mol_type = other DNA
agaacaggaaccatgaggcggagagtgg

SEQ ID NO: 31134 - DNA, 28 bp, synthetic construct
  source 1..28: mol_type = other DNA
tccgcctcatggttcctgttctccatgg

SEQ ID NO: 31135 - DNA, 28 bp, synthetic construct
  source 1..28: mol_type = other DNA
cccatggagaacaggaaccatgaggcgg

SEQ ID NO: 31136 - DNA, 28 bp, synthetic construct
  source 1..28: mol_type = other DNA
cctcatggttcctgttctccatgggtgg

SEQ ID NO: 31137 - DNA, 28 bp, synthetic construct
  source 1..28: mol_type = other DNA
tgggaagaggccacccatggagaacagg

SEQ ID NO: 31138 - DNA, 28 bp, synthetic construct
  source 1..28: mol_type = other DNA
tctggagctgggaagaggccacccatgg

SEQ ID NO: 31139 - DNA, 28 bp, synthetic construct
  source 1..28: mol_type = other DNA
tgggtggcctcttcccagctccagatgg

SEQ ID NO: 31140 - DNA, 28 bp, synthetic construct
  source 1..28: mol_type = other DNA
gcaagttccatctggagctgggaagagg

SEQ ID NO: 31141 - DNA, 28 bp, synthetic construct
  source 1..28: mol_type = other DNA
ggcttggcaagttccatctggagctggg

SEQ ID NO: 31142 - DNA, 28 bp, synthetic construct
  source 1..28: mol_type = other DNA
gggcttggcaagttccatctggagctgg

SEQ ID NO: 31143 - DNA, 28 bp, synthetic construct
  source 1..28: mol_type = other DNA
ggatgtgggcttggcaagttccatctgg

SEQ ID NO: 31144 - DNA, 28 bp, synthetic construct
  source 1..28: mol_type = other DNA
atgtgtgatgctatggatgtgggcttgg

SEQ ID NO: 31145 - DNA, 28 bp, synthetic construct
  source 1..28: mol_type = other DNA
cagaaatgtgtgatgctatggatgtggg

SEQ ID NO: 31146 - DNA, 28 bp, synthetic construct
  source 1..28: mol_type = other DNA
gcagaaatgtgtgatgctatggatgtgg

SEQ ID NO: 31147 - DNA, 28 bp, synthetic construct
  source 1..28: mol_type = other DNA
agaacagcagaaatgtgtgatgctatgg

SEQ ID NO: 31148 - DNA, 28 bp, synthetic construct
  source 1..28: mol_type = other DNA
gcatcacacatttctgctgttctcctgg

SEQ ID NO: 31149 - DNA, 28 bp, synthetic construct
  source 1..28: mol_type = other DNA
gacgggaggtgctgggggatgttccagg

SEQ ID NO: 31150 - DNA, 28 bp, synthetic construct
  source 1..28: mol_type = other DNA
tggcgagtctgacgggaggtgctggggg

SEQ ID NO: 31151 - DNA, 28 bp, synthetic construct
  source 1..28: mol_type = other DNA
gtggcgagtctgacgggaggtgctgggg

SEQ ID NO: 31152 - DNA, 28 bp, synthetic construct
  source 1..28: mol_type = other DNA
tgtggcgagtctgacgggaggtgctggg

SEQ ID NO: 31153 - DNA, 28 bp, synthetic construct
  source 1..28: mol_type = other DNA
ttgtggcgagtctgacgggaggtgctgg

SEQ ID NO: 31154 - DNA, 28 bp, synthetic construct
  source 1..28: mol_type = other DNA
gtttcattgtggcgagtctgacgggagg

SEQ ID NO: 31155 - DNA, 28 bp, synthetic construct
  source 1..28: mol_type = other DNA
agggtttcattgtggcgagtctgacggg

SEQ ID NO: 31156 - DNA, 28 bp, synthetic construct
  source 1..28: mol_type = other DNA
cagggtttcattgtggcgagtctgacgg

SEQ ID NO: 31157 - DNA, 28 bp, synthetic construct
  source 1..28: mol_type = other DNA
tagaggacagagcagggtttcattgtgg

SEQ ID NO: 31158 - DNA, 28 bp, synthetic construct
  source 1..28: mol_type = other DNA
aatgagtggggtagaggacagagcaggg

SEQ ID NO: 31159 - DNA, 28 bp, synthetic construct
  source 1..28: mol_type = other DNA
taatgagtggggtagaggacagagcagg

SEQ ID NO: 31160 - DNA, 28 bp, synthetic construct
  source 1..28: mol_type = other DNA
acatggtaagtaatgagtggggtagagg

SEQ ID NO: 31161 - DNA, 28 bp, synthetic construct
  source 1..28: mol_type = other DNA
tctaccccactcattacttaccatgtgg

SEQ ID NO: 31162 - DNA, 28 bp, synthetic construct
  source 1..28: mol_type = other DNA
caggccacatggtaagtaatgagtgggg

SEQ ID NO: 31163 - DNA, 28 bp, synthetic construct
  source 1..28: mol_type = other DNA
acaggccacatggtaagtaatgagtggg

SEQ ID NO: 31164 - DNA, 28 bp, synthetic construct
  source 1..28: mol_type = other DNA
cacaggccacatggtaagtaatgagtgg

SEQ ID NO: 31165 - DNA, 28 bp, synthetic construct
  source 1..28: mol_type = other DNA
ggcaggagggaattcacaggccacatgg

SEQ ID NO: 31166 - DNA, 28 bp, synthetic construct
  source 1..28: mol_type = other DNA
tgggacaaggcaggagggaattcacagg

SEQ ID NO: 31167 - DNA, 28 bp, synthetic construct
  source 1..28: mol_type = other DNA
aggagcaagctgggacaaggcaggaggg

SEQ ID NO: 31168 - DNA, 28 bp, synthetic construct
  source 1..28: mol_type = other DNA
gaggagcaagctgggacaaggcaggagg

SEQ ID NO: 31169 - DNA, 28 bp, synthetic construct
  source 1..28: mol_type = other DNA
cctgccttgtcccagcttgctcctcagg

SEQ ID NO: 31170 - DNA, 28 bp, synthetic construct
  source 1..28: mol_type = other DNA
gagacctgaggagcaagctgggacaagg

SEQ ID NO: 31171 - DNA, 28 bp, synthetic construct
  source 1..28: mol_type = other DNA
ggggtagagacctgaggagcaagctggg

SEQ ID NO: 31172 - DNA, 28 bp, synthetic construct
  source 1..28: mol_type = other DNA
gggggtagagacctgaggagcaagctgg

SEQ ID NO: 31173 - DNA, 28 bp, synthetic construct
  source 1..28: mol_type = other DNA
aaactcagaagggggtagagacctgagg

SEQ ID NO: 31174 - DNA, 28 bp, synthetic construct
  source 1..28: mol_type = other DNA
atcagaaggtggtaaactcagaaggggg

SEQ ID NO: 31175 - DNA, 28 bp, synthetic construct
  source 1..28: mol_type = other DNA
gatcagaaggtggtaaactcagaagggg

SEQ ID NO: 31176 - DNA, 28 bp, synthetic construct
  source 1..28: mol_type = other DNA
agatcagaaggtggtaaactcagaaggg

SEQ ID NO: 31177 - DNA, 28 bp, synthetic construct
  source 1..28: mol_type = other DNA
gagatcagaaggtggtaaactcagaagg

SEQ ID NO: 31178 - DNA, 28 bp, synthetic construct
  source 1..28: mol_type = other DNA
agaggcaaagtgagagatcagaaggtgg

SEQ ID NO: 31179 - DNA, 28 bp, synthetic construct
  source 1..28: mol_type = other DNA
agcagaggcaaagtgagagatcagaagg

SEQ ID NO: 31180 - DNA, 28 bp, synthetic construct
  source 1..28: mol_type = other DNA
atctctcactttgcctctgctaatctgg

SEQ ID NO: 31181 - DNA, 28 bp, synthetic construct
  source 1..28: mol_type = other DNA
ttgcctctgctaatctggcttcttcagg

SEQ ID NO: 31182 - DNA, 28 bp, synthetic construct
  source 1..28: mol_type = other DNA
aaacctgaagaagccagattagcagagg

SEQ ID NO: 31183 - DNA, 28 bp, synthetic construct
  source 1..28: mol_type = other DNA
gaccctccattatcctcatccaaacagg

SEQ ID NO: 31184 - DNA, 28 bp, synthetic construct
  source 1..28: mol_type = other DNA
ggcctgtttggatgaggataatggaggg

SEQ ID NO: 31185 - DNA, 28 bp, synthetic construct
  source 1..28: mol_type = other DNA
gggcctgtttggatgaggataatggagg

SEQ ID NO: 31186 - DNA, 28 bp, synthetic construct
  source 1..28: mol_type = other DNA
gacgggcctgtttggatgaggataatgg

SEQ ID NO: 31187 - DNA, 28 bp, synthetic construct
  source 1..28: mol_type = other DNA
ggataaggacgggcctgtttggatgagg

SEQ ID NO: 31188 - DNA, 28 bp, synthetic construct
  source 1..28: mol_type = other DNA
ttctcaggataaggacgggcctgtttgg

SEQ ID NO: 31189 - DNA, 28 bp, synthetic construct
  source 1..28: mol_type = other DNA
aacaggcccgtccttatcctgagaatgg

SEQ ID NO: 31190 - DNA, 28 bp, synthetic construct
  source 1..28: mol_type = other DNA
aggtatccattctcaggataaggacggg

SEQ ID NO: 31191 - DNA, 28 bp, synthetic construct
  source 1..28: mol_type = other DNA
taggtatccattctcaggataaggacgg

SEQ ID NO: 31192 - DNA, 28 bp, synthetic construct
  source 1..28: mol_type = other DNA
tttctaggtatccattctcaggataagg

SEQ ID NO: 31193 - DNA, 28 bp, synthetic construct
  source 1..28: mol_type = other DNA
gggaagtttctaggtatccattctcagg

SEQ ID NO: 31194 - DNA, 28 bp, synthetic construct
  source 1..28: mol_type = other DNA
gataggactgggtggggaagtttctagg

SEQ ID NO: 31195 - DNA, 28 bp, synthetic construct
  source 1..28: mol_type = other DNA
ccagggcttgggataggactgggtgggg

SEQ ID NO: 31196 - DNA, 28 bp, synthetic construct
  source 1..28: mol_type = other DNA
cccagggcttgggataggactgggtggg

SEQ ID NO: 31197 - DNA, 28 bp, synthetic construct
  source 1..28: mol_type = other DNA
tcccagggcttgggataggactgggtgg

SEQ ID NO: 31198 - DNA, 28 bp, synthetic construct
  source 1..28: mol_type = other DNA
atttcccagggcttgggataggactggg

SEQ ID NO: 31199 - DNA, 28 bp, synthetic construct
  source 1..28: mol_type = other DNA
aatttcccagggcttgggataggactgg

SEQ ID NO: 31200 - DNA, 28 bp, synthetic construct
  source 1..28: mol_type = other DNA
gggataatttcccagggcttgggatagg

SEQ ID NO: 31201 - DNA, 28 bp, synthetic construct
  source 1..28: mol_type = other DNA
atactgggataatttcccagggcttggg

SEQ ID NO: 31202 - DNA, 28 bp, synthetic construct
  source 1..28: mol_type = other DNA
aatactgggataatttcccagggcttgg

SEQ ID NO: 31203 - DNA, 28 bp, synthetic construct
  source 1..28: mol_type = other DNA
cagacaatactgggataatttcccaggg

SEQ ID NO: 31204 - DNA, 28 bp, synthetic construct
  source 1..28: mol_type = other DNA
gcagacaatactgggataatttcccagg

SEQ ID NO: 31205 - DNA, 28 bp, synthetic construct
  source 1..28: mol_type = other DNA
ccagggacatgaggcagacaatactggg

SEQ ID NO: 31206 - DNA, 28 bp, synthetic construct
  source 1..28: mol_type = other DNA
gccagggacatgaggcagacaatactgg

SEQ ID NO: 31207 - DNA, 28 bp, synthetic construct
  source 1..28: mol_type = other DNA
tattgtctgcctcatgtccctggcaagg

SEQ ID NO: 31208 - DNA, 28 bp, synthetic construct
  source 1..28: mol_type = other DNA
acgttttctccttgccagggacatgagg

SEQ ID NO: 31209 - DNA, 28 bp, synthetic construct
  source 1..28: mol_type = other DNA
ataaagaaacgttttctccttgccaggg

SEQ ID NO: 31210 - DNA, 28 bp, synthetic construct
  source 1..28: mol_type = other DNA
gataaagaaacgttttctccttgccagg

SEQ ID NO: 31211 - DNA, 28 bp, synthetic construct
  source 1..28: mol_type = other DNA
ctttatcttatacccaaaccagaaatgg

SEQ ID NO: 31212 - DNA, 28 bp, synthetic construct
  source 1..28: mol_type = other DNA
tttatcttatacccaaaccagaaatggg

SEQ ID NO: 31213 - DNA, 28 bp, synthetic construct
  source 1..28: mol_type = other DNA
ttatcttatacccaaaccagaaatgggg

SEQ ID NO: 31214 - DNA, 28 bp, synthetic construct
  source 1..28: mol_type = other DNA
tcttatacccaaaccagaaatggggagg

SEQ ID NO: 31215 - DNA, 28 bp, synthetic construct
  source 1..28: mol_type = other DNA
tgggaagcctccccatttctggtttggg

SEQ ID NO: 31216 - DNA, 28 bp, synthetic construct
  source 1..28: mol_type = other DNA
gtgggaagcctccccatttctggtttgg

SEQ ID NO: 31217 - DNA, 28 bp, synthetic construct
  source 1..28: mol_type = other DNA
agaacgtgggaagcctccccatttctgg

SEQ ID NO: 31218 - DNA, 28 bp, synthetic construct
  source 1..28: mol_type = other DNA
gagtattcagcaaagagaagaacgtggg

SEQ ID NO: 31219 - DNA, 28 bp, synthetic construct
  source 1..28: mol_type = other DNA
agagtattcagcaaagagaagaacgtgg

SEQ ID NO: 31220 - DNA, 28 bp, synthetic construct
  source 1..28: mol_type = other DNA
agaatgggcagggcttggtgatggaagg

SEQ ID NO: 31221 - DNA, 28 bp, synthetic construct
  source 1..28: mol_type = other DNA
aggtagaatgggcagggcttggtgatgg

SEQ ID NO: 31222 - DNA, 28 bp, synthetic construct
  source 1..28: mol_type = other DNA
ctgaagaggtagaatgggcagggcttgg

SEQ ID NO: 31223 - DNA, 28 bp, synthetic construct
  source 1..28: mol_type = other DNA
agtgactgaagaggtagaatgggcaggg

SEQ ID NO: 31224 - DNA, 28 bp, synthetic construct
  source 1..28: mol_type = other DNA
gagtgactgaagaggtagaatgggcagg

SEQ ID NO: 31225 - DNA, 28 bp, synthetic construct
  source 1..28: mol_type = other DNA
tgaggagtgactgaagaggtagaatggg

SEQ ID NO: 31226 - DNA, 28 bp, synthetic construct
  source 1..28: mol_type = other DNA
ctgaggagtgactgaagaggtagaatgg

SEQ ID NO: 31227 - DNA, 28 bp, synthetic construct
  source 1..28: mol_type = other DNA
agaaggatctgaggagtgactgaagagg

SEQ ID NO: 31228 - DNA, 28 bp, synthetic construct
  source 1..28: mol_type = other DNA
agatgcggacgggaagaaggatctgagg

SEQ ID NO: 31229 - DNA, 28 bp, synthetic construct
  source 1..28: mol_type = other DNA
ggctgtggagatgcggacgggaagaagg

SEQ ID NO: 31230 - DNA, 28 bp, synthetic construct
  source 1..28: mol_type = other DNA
agggtgtggctgtggagatgcggacggg

SEQ ID NO: 31231 - DNA, 28 bp, synthetic construct
  source 1..28: mol_type = other DNA
gagggtgtggctgtggagatgcggacgg

SEQ ID NO: 31232 - DNA, 28 bp, synthetic construct
  source 1..28: mol_type = other DNA
gagggagggtgtggctgtggagatgcgg

SEQ ID NO: 31233 - DNA, 28 bp, synthetic construct
  source 1..28: mol_type = other DNA
aggcaatggagggagggtgtggctgtgg

SEQ ID NO: 31234 - DNA, 28 bp, synthetic construct
  source 1..28: mol_type = other DNA
gatgagaggcaatggagggagggtgtgg

SEQ ID NO: 31235 - DNA, 28 bp, synthetic construct
  source 1..28: mol_type = other DNA
gcagtgatgagaggcaatggagggaggg

SEQ ID NO: 31236 - DNA, 28 bp, synthetic construct
  source 1..28: mol_type = other DNA
ggcagtgatgagaggcaatggagggagg

SEQ ID NO: 31237 - DNA, 28 bp, synthetic construct
  source 1..28: mol_type = other DNA
tagggcagtgatgagaggcaatggaggg

SEQ ID NO: 31238 - DNA, 28 bp, synthetic construct
  source 1..28: mol_type = other DNA
ttagggcagtgatgagaggcaatggagg

SEQ ID NO: 31239 - DNA, 28 bp, synthetic construct
  source 1..28: mol_type = other DNA
ggattagggcagtgatgagaggcaatgg

SEQ ID NO: 31240 - DNA, 28 bp, synthetic construct
  source 1..28: mol_type = other DNA
ccttggggattagggcagtgatgagagg

SEQ ID NO: 31241 - DNA, 28 bp, synthetic construct
  source 1..28: mol_type = other DNA
ctctcatcactgccctaatccccaaggg

SEQ ID NO: 31242 - DNA, 28 bp, synthetic construct
  source 1..28: mol_type = other DNA
tctcatcactgccctaatccccaagggg

SEQ ID NO: 31243 - DNA, 28 bp, synthetic construct
  source 1..28: mol_type = other DNA
gggtgcacgtaccccttggggattaggg

SEQ ID NO: 31244 - DNA, 28 bp, synthetic construct
  source 1..28: mol_type = other DNA
tgggtgcacgtaccccttggggattagg

SEQ ID NO: 31245 - DNA, 28 bp, synthetic construct
  source 1..28: mol_type = other DNA
gtgccctgggtgcacgtaccccttgggg

SEQ ID NO: 31246 - DNA, 28 bp, synthetic construct
  source 1..28: mol_type = other DNA
tgtgccctgggtgcacgtaccccttggg

SEQ ID NO: 31247 - DNA, 28 bp, synthetic construct
  source 1..28: mol_type = other DNA
gtgtgccctgggtgcacgtaccccttgg

SEQ ID NO: 31248 - DNA, 28 bp, synthetic construct
  source 1..28: mol_type = other DNA
tgtttaggatttttagagtgctgttggg

SEQ ID NO: 31249 - DNA, 28 bp, synthetic construct
  source 1..28: mol_type = other DNA
atgtttaggatttttagagtgctgttgg

SEQ ID NO: 31250 - DNA, 28 bp, synthetic construct
  source 1..28: mol_type = other DNA
acagcactctaaaaatcctaaacattgg

SEQ ID NO: 31251 - DNA, 28 bp, synthetic construct
  source 1..28: mol_type = other DNA
atgatataacatagcaccaatgtttagg

SEQ ID NO: 31252 - DNA, 28 bp, synthetic construct
  source 1..28: mol_type = other DNA
tatcatgtctagatccaagtatttctgg

SEQ ID NO: 31253 - DNA, 28 bp, synthetic construct
  source 1..28: mol_type = other DNA
ataggaaagctcatccagaaatacttgg

SEQ ID NO: 31254 - DNA, 28 bp, synthetic construct
  source 1..28: mol_type = other DNA
tggatgagctttcctattttaaaaatgg

SEQ ID NO: 31255 - DNA, 28 bp, synthetic construct
  source 1..28: mol_type = other DNA
ggatgagctttcctattttaaaaatggg

SEQ ID NO: 31256 - DNA, 28 bp, synthetic construct
  source 1..28: mol_type = other DNA
tgttttttttacccatttttaaaatagg

SEQ ID NO: 31257 - DNA, 28 bp, synthetic construct
  source 1..28: mol_type = other DNA
acccaagtccctgattcagcttttcagg

SEQ ID NO: 31258 - DNA, 28 bp, synthetic construct
  source 1..28: mol_type = other DNA
gcctgaaaagctgaatcagggacttggg

SEQ ID NO: 31259 - DNA, 28 bp, synthetic construct
  source 1..28: mol_type = other DNA
agcctgaaaagctgaatcagggacttgg

SEQ ID NO: 31260 - DNA, 28 bp, synthetic construct
  source 1..28: mol_type = other DNA
tgatgtagcctgaaaagctgaatcaggg

SEQ ID NO: 31261 - DNA, 28 bp, synthetic construct
  source 1..28: mol_type = other DNA
ttgatgtagcctgaaaagctgaatcagg

SEQ ID NO: 31262 - DNA, 28 bp, synthetic construct
  source 1..28: mol_type = other DNA
gcttttcaggctacatcaatacccctgg

SEQ ID NO: 31263 - DNA, 28 bp, synthetic construct
  source 1..28: mol_type = other DNA
gtcagcatttgtgttgaagcaccagggg

SEQ ID NO: 31264 - DNA, 28 bp, synthetic construct
  source 1..28: mol_type = other DNA
ggtcagcatttgtgttgaagcaccaggg

SEQ ID NO: 31265 - DNA, 28 bp, synthetic construct
  source 1..28: mol_type = other DNA
gggtcagcatttgtgttgaagcaccagg

SEQ ID NO: 31266 - DNA, 28 bp, synthetic construct
  source 1..28: mol_type = other DNA
cacaaatgctgacccttgtactgactgg

SEQ ID NO: 31267 - DNA, 28 bp, synthetic construct
  source 1..28: mol_type = other DNA
gggcactaattgccagtcagtacaaggg

SEQ ID NO: 31268 - DNA, 28 bp, synthetic construct
  source 1..28: mol_type = other DNA
agggcactaattgccagtcagtacaagg

SEQ ID NO: 31269 - DNA, 28 bp, synthetic construct
  source 1..28: mol_type = other DNA
gacattgatctgagggttgaattcaggg

SEQ ID NO: 31270 - DNA, 28 bp, synthetic construct
  source 1..28: mol_type = other DNA
agacattgatctgagggttgaattcagg

SEQ ID NO: 31271 - DNA, 28 bp, synthetic construct
  source 1..28: mol_type = other DNA
accctcagatcaatgtctataaaattgg

SEQ ID NO: 31272 - DNA, 28 bp, synthetic construct
  source 1..28: mol_type = other DNA
gccaattttatagacattgatctgaggg

SEQ ID NO: 31273 - DNA, 28 bp, synthetic construct
  source 1..28: mol_type = other DNA
agccaattttatagacattgatctgagg

SEQ ID NO: 31274 - DNA, 28 bp, synthetic construct
  source 1..28: mol_type = other DNA
caatgtctataaaattggctgtaagagg

SEQ ID NO: 31275 - DNA, 28 bp, synthetic construct
  source 1..28: mol_type = other DNA
tgtctataaaattggctgtaagaggtgg

SEQ ID NO: 31276 - DNA, 28 bp, synthetic construct
  source 1..28: mol_type = other DNA
tcttactcacagtaatgggaatcaaggg

SEQ ID NO: 31277 - DNA, 28 bp, synthetic construct
  source 1..28: mol_type = other DNA
ctcttactcacagtaatgggaatcaagg

SEQ ID NO: 31278 - DNA, 28 bp, synthetic construct
  source 1..28: mol_type = other DNA
gttcacagctcttactcacagtaatggg

SEQ ID NO: 31279 - DNA, 28 bp, synthetic construct
  source 1..28: mol_type = other DNA
ggttcacagctcttactcacagtaatgg

SEQ ID NO: 31280 - DNA, 28 bp, synthetic construct
  source 1..28: mol_type = other DNA
ttttgtgttggctgcaaggggatttagg

SEQ ID NO: 31281 - DNA, 28 bp, synthetic construct
  source 1..28: mol_type = other DNA
gggtaaattttgtgttggctgcaagggg

SEQ ID NO: 31282 - DNA, 28 bp, synthetic construct
  source 1..28: mol_type = other DNA
ggggtaaattttgtgttggctgcaaggg

SEQ ID NO: 31283 - DNA, 28 bp, synthetic construct
  source 1..28: mol_type = other DNA
gggggtaaattttgtgttggctgcaagg

SEQ ID NO: 31284 - DNA, 28 bp, synthetic construct
  source 1..28: mol_type = other DNA
aggcagcagggggtaaattttgtgttgg

SEQ ID NO: 31285 - DNA, 28 bp, synthetic construct
  source 1..28: mol_type = other DNA
acacaaaatttaccccctgctgcctcgg

SEQ ID NO: 31286 - DNA, 28 bp, synthetic construct
  source 1..28: mol_type = other DNA
ttaattggcactccgaggcagcaggggg

SEQ ID NO: 31287 - DNA, 28 bp, synthetic construct
  source 1..28: mol_type = other DNA
tttaattggcactccgaggcagcagggg

SEQ ID NO: 31288 - DNA, 28 bp, synthetic construct
  source 1..28: mol_type = other DNA
ttttaattggcactccgaggcagcaggg

SEQ ID NO: 31289 - DNA, 28 bp, synthetic construct
  source 1..28: mol_type = other DNA
attttaattggcactccgaggcagcagg

SEQ ID NO: 31290 - DNA, 28 bp, synthetic construct
  source 1..28: mol_type = other DNA
ttttattattttaattggcactccgagg

SEQ ID NO: 31291 - DNA, 28 bp, synthetic construct
  source 1..28: mol_type = other DNA
cggttttggtttttattattttaattgg

SEQ ID NO: 31292 - DNA, 28 bp, synthetic construct
  source 1..28: mol_type = other DNA
attaaaataataaaaaccaaaaccgtgg

SEQ ID NO: 31293 - DNA, 28 bp, synthetic construct
  source 1..28: mol_type = other DNA
ttaaaataataaaaaccaaaaccgtggg

SEQ ID NO: 31294 - DNA, 28 bp, synthetic construct
  source 1..28: mol_type = other DNA
aactaattacatctgcccacggttttgg

SEQ ID NO: 31295 - DNA, 28 bp, synthetic construct
  source 1..28: mol_type = other DNA
ttctcaaactaattacatctgcccacgg

SEQ ID NO: 31296 - DNA, 28 bp, synthetic construct
  source 1..28: mol_type = other DNA
tgggcagatgtaattagtttgagaacgg

SEQ ID NO: 31297 - DNA, 28 bp, synthetic construct
  source 1..28: mol_type = other DNA
ggggttaacttgtttgcttggcatgagg

SEQ ID NO: 31298 - DNA, 28 bp, synthetic construct
  source 1..28: mol_type = other DNA
tgccaagcaaacaagttaacccctttgg

SEQ ID NO: 31299 - DNA, 28 bp, synthetic construct
  source 1..28: mol_type = other DNA
caccaaaggggttaacttgtttgcttgg

SEQ ID NO: 31300 - DNA, 28 bp, synthetic construct
  source 1..28: mol_type = other DNA
gattattctgtatatgtcaccaaagggg

SEQ ID NO: 31301 - DNA, 28 bp, synthetic construct
  source 1..28: mol_type = other DNA
agattattctgtatatgtcaccaaaggg

SEQ ID NO: 31302 - DNA, 28 bp, synthetic construct
  source 1..28: mol_type = other DNA
cagattattctgtatatgtcaccaaagg

SEQ ID NO: 31303 - DNA, 28 bp, synthetic construct
  source 1..28: mol_type = other DNA
ctttggtgacatatacagaataatctgg

SEQ ID NO: 31304 - DNA, 28 bp, synthetic construct
  source 1..28: mol_type = other DNA
gacatatacagaataatctggacaaagg

SEQ ID NO: 31305 - DNA, 28 bp, synthetic construct
  source 1..28: mol_type = other DNA
acatatacagaataatctggacaaaggg

SEQ ID NO: 31306 - DNA, 28 bp, synthetic construct
  source 1..28: mol_type = other DNA
ctgaacatttcttgtgctatttgccagg

SEQ ID NO: 31307 - DNA, 28 bp, synthetic construct
  source 1..28: mol_type = other DNA
acagtttttcaatattacaacttcctgg

SEQ ID NO: 31308 - DNA, 28 bp, synthetic construct
  source 1..28: mol_type = other DNA
ttgaaaaactgtgctcttctgagaatgg

SEQ ID NO: 31309 - DNA, 28 bp, synthetic construct
  source 1..28: mol_type = other DNA
tgaaaaactgtgctcttctgagaatggg

SEQ ID NO: 31310 - DNA, 28 bp, synthetic construct
  source 1..28: mol_type = other DNA
gtgctcttctgagaatgggaaaatgagg

SEQ ID NO: 31311 - DNA, 28 bp, synthetic construct
  source 1..28: mol_type = other DNA
aatgggaaaatgaggacataaactctgg

SEQ ID NO: 31312 - DNA, 28 bp, synthetic construct
  source 1..28: mol_type = other DNA
tgaggacataaactctggttccaaatgg

SEQ ID NO: 31313 - DNA, 28 bp, synthetic construct
  source 1..28: mol_type = other DNA
gacataaactctggttccaaatggttgg

SEQ ID NO: 31314 - DNA, 28 bp, synthetic construct
  source 1..28: mol_type = other DNA
cacataaactgcacttccaaccatttgg

SEQ ID NO: 31315 - DNA, 28 bp, synthetic construct
  source 1..28: mol_type = other DNA
caaatggttggaagtgcagtttatgtgg

SEQ ID NO: 31316 - DNA, 28 bp, synthetic construct
  source 1..28: mol_type = other DNA
ggttggaagtgcagtttatgtggtcagg

SEQ ID NO: 31317 - DNA, 28 bp, synthetic construct
  source 1..28: mol_type = other DNA
atcttgaaagtttttttaatgaaagggg

SEQ ID NO: 31318 - DNA, 28 bp, synthetic construct
  source 1..28: mol_type = other DNA
aatcttgaaagtttttttaatgaaaggg

SEQ ID NO: 31319 - DNA, 28 bp, synthetic construct
  source 1..28: mol_type = other DNA
gaatcttgaaagtttttttaatgaaagg

SEQ ID NO: 31320 - DNA, 28 bp, synthetic construct
  source 1..28: mol_type = other DNA
aaaactttcaagattccacttgatccgg

SEQ ID NO: 31321 - DNA, 28 bp, synthetic construct
  source 1..28: mol_type = other DNA
aaactttcaagattccacttgatccggg

SEQ ID NO: 31322 - DNA, 28 bp, synthetic construct
  source 1..28: mol_type = other DNA
cattttcgaagaaacccggatcaagtgg

SEQ ID NO: 31323 - DNA, 28 bp, synthetic construct
  source 1..28: mol_type = other DNA
aaagtaatacattttcgaagaaacccgg

SEQ ID NO: 31324 - DNA, 28 bp, synthetic construct
  source 1..28: mol_type = other DNA
tactttttacaaatataattcttatagg

SEQ ID NO: 31325 - DNA, 28 bp, synthetic construct
  source 1..28: mol_type = other DNA
actttttacaaatataattcttataggg

SEQ ID NO: 31326 - DNA, 28 bp, synthetic construct
  source 1..28: mol_type = other DNA
tagggacagacttcagctgtgtagcagg

SEQ ID NO: 31327 - DNA, 28 bp, synthetic construct
  source 1..28: mol_type = other DNA
gaagagaacgttcttgaaagactgctgg

SEQ ID NO: 31328 - DNA, 28 bp, synthetic construct
  source 1..28: mol_type = other DNA
aagagaacgttcttgaaagactgctggg

SEQ ID NO: 31329 - DNA, 28 bp, synthetic construct
  source 1..28: mol_type = other DNA
actgagcttgatactctttcagaggtgg

SEQ ID NO: 31330 - DNA, 28 bp, synthetic construct
  source 1..28: mol_type = other DNA
acctctgaaagagtatcaagctcagtgg

SEQ ID NO: 31331 - DNA, 28 bp, synthetic construct
  source 1..28: mol_type = other DNA
accactgagcttgatactctttcagagg

SEQ ID NO: 31332 - DNA, 28 bp, synthetic construct
  source 1..28: mol_type = other DNA
ctgaaagagtatcaagctcagtggttgg

SEQ ID NO: 31333 - DNA, 28 bp, synthetic construct
  source 1..28: mol_type = other DNA
gccaagttcctgtcccacccatctctgg

SEQ ID NO: 31334 - DNA, 28 bp, synthetic construct
  source 1..28: mol_type = other DNA
ccaagttcctgtcccacccatctctggg

SEQ ID NO: 31335 - DNA, 28 bp, synthetic construct
  source 1..28: mol_type = other DNA
tcctgtcccacccatctctgggatgagg

SEQ ID NO: 31336 - DNA, 28 bp, synthetic construct
  source 1..28: mol_type = other DNA
tcctcatcccagagatgggtgggacagg

SEQ ID NO: 31337 - DNA, 28 bp, synthetic construct
  source 1..28: mol_type = other DNA
agaactcctcatcccagagatgggtggg

SEQ ID NO: 31338 - DNA, 28 bp, synthetic construct
  source 1..28: mol_type = other DNA
gagaactcctcatcccagagatgggtgg

SEQ ID NO: 31339 - DNA, 28 bp, synthetic construct
  source 1..28: mol_type = other DNA
atggagaactcctcatcccagagatggg

SEQ ID NO: 31340 - DNA, 28 bp, synthetic construct
  source 1..28: mol_type = other DNA
catggagaactcctcatcccagagatgg

SEQ ID NO: 31341 - DNA, 28 bp, synthetic construct
  source 1..28: mol_type = other DNA
catctctgggatgaggagttctccatgg

SEQ ID NO: 31342 - DNA, 28 bp, synthetic construct
  source 1..28: mol_type = other DNA
gagttctccatggtgaccctgagtcagg

SEQ ID NO: 31343 - DNA, 28 bp, synthetic construct
  source 1..28: mol_type = other DNA
gaagaagcctgactcagggtcaccatgg

SEQ ID NO: 31344 - DNA, 28 bp, synthetic construct
  source 1..28: mol_type = other DNA
aggggtgcagaagaagcctgactcaggg

SEQ ID NO: 31345 - DNA, 28 bp, synthetic construct
  source 1..28: mol_type = other DNA
gaggggtgcagaagaagcctgactcagg

SEQ ID NO: 31346 - DNA, 28 bp, synthetic construct
  source 1..28: mol_type = other DNA
caggcttcttctgcacccctctgcctgg

SEQ ID NO: 31347 - DNA, 28 bp, synthetic construct
  source 1..28: mol_type = other DNA
tctgcacccctctgcctggttaatgagg

SEQ ID NO: 31348 - DNA, 28 bp, synthetic construct
  source 1..28: mol_type = other DNA
ttgagtcctcattaaccaggcagagggg

SEQ ID NO: 31349 - DNA, 28 bp, synthetic construct
  source 1..28: mol_type = other DNA
gttgagtcctcattaaccaggcagaggg

SEQ ID NO: 31350 - DNA, 28 bp, synthetic construct
  source 1..28: mol_type = other DNA
agttgagtcctcattaaccaggcagagg

SEQ ID NO: 31351 - DNA, 28 bp, synthetic construct
  source 1..28: mol_type = other DNA
cagttcagttgagtcctcattaaccagg

SEQ ID NO: 31352 - DNA, 28 bp, synthetic construct
  source 1..28: mol_type = other DNA
atgcagaaagggtttgtttgcagatggg

SEQ ID NO: 31353 - DNA, 28 bp, synthetic construct
  source 1..28: mol_type = other DNA
aatgcagaaagggtttgtttgcagatgg

SEQ ID NO: 31354 - DNA, 28 bp, synthetic construct
  source 1..28: mol_type = other DNA
gtgtctagagagaaaaatgcagaaaggg

SEQ ID NO: 31355 - DNA, 28 bp, synthetic construct
  source 1..28: mol_type = other DNA
cgtgtctagagagaaaaatgcagaaagg

SEQ ID NO: 31356 - DNA, 28 bp, synthetic construct
  source 1..28: mol_type = other DNA
ctagacacgagtgagttatgtcagatgg

SEQ ID NO: 31357 - DNA, 28 bp, synthetic construct
  source 1..28: mol_type = other DNA
gagtgagttatgtcagatggtataatgg

SEQ ID NO: 31358 - DNA, 28 bp, synthetic construct
  source 1..28: mol_type = other DNA
agtgagttatgtcagatggtataatggg

SEQ ID NO: 31359 - DNA, 28 bp, synthetic construct
  source 1..28: mol_type = other DNA
agatggtataatgggaaaaagacaaagg

SEQ ID NO: 31360 - DNA, 28 bp, synthetic construct
  source 1..28: mol_type = other DNA
aaaagacaaaggatatttgaatctaagg

SEQ ID NO: 31361 - DNA, 28 bp, synthetic construct
  source 1..28: mol_type = other DNA
caaaggatatttgaatctaaggacatgg

SEQ ID NO: 31362 - DNA, 28 bp, synthetic construct
  source 1..28: mol_type = other DNA
aaaggatatttgaatctaaggacatggg

SEQ ID NO: 31363 - DNA, 28 bp, synthetic construct
  source 1..28: mol_type = other DNA
gatatttgaatctaaggacatgggctgg

SEQ ID NO: 31364 - DNA, 28 bp, synthetic construct
  source 1..28: mol_type = other DNA
tgaatctaaggacatgggctggatcagg

SEQ ID NO: 31365 - DNA, 28 bp, synthetic construct
  source 1..28: mol_type = other DNA
taaggacatgggctggatcaggtgaagg

SEQ ID NO: 31366 - DNA, 28 bp, synthetic construct
  source 1..28: mol_type = other DNA
aaggacatgggctggatcaggtgaaggg

SEQ ID NO: 31367 - DNA, 28 bp, synthetic construct
  source 1..28: mol_type = other DNA
acatgggctggatcaggtgaagggatgg

SEQ ID NO: 31368 - DNA, 28 bp, synthetic construct
  source 1..28: mol_type = other DNA
tgttgctgtttctgcttctttagtttgg

SEQ ID NO: 31369 - DNA, 28 bp, synthetic construct
  source 1..28: mol_type = other DNA
gttgctgtttctgcttctttagtttggg

SEQ ID NO: 31370 - DNA, 28 bp, synthetic construct
  source 1..28: mol_type = other DNA
ttgctgtttctgcttctttagtttgggg

SEQ ID NO: 31371 - DNA, 28 bp, synthetic construct
  source 1..28: mol_type = other DNA
ctgtttctgcttctttagtttggggagg

SEQ ID NO: 31372 - DNA, 28 bp, synthetic construct
  source 1..28: mol_type = other DNA
tttctgcttctttagtttggggaggagg

SEQ ID NO: 31373 - DNA, 28 bp, synthetic construct
  source 1..28: mol_type = other DNA
cttctttagtttggggaggaggataagg

SEQ ID NO: 31374 - DNA, 28 bp, synthetic construct
  source 1..28: mol_type = other DNA
tagtttggggaggaggataaggaaaagg

SEQ ID NO: 31375 - DNA, 28 bp, synthetic construct
  source 1..28: mol_type = other DNA
agtttggggaggaggataaggaaaaggg

SEQ ID NO: 31376 - DNA, 28 bp, synthetic construct
  source 1..28: mol_type = other DNA
tggggaggaggataaggaaaagggttgg

SEQ ID NO: 31377 - DNA, 28 bp, synthetic construct
  source 1..28: mol_type = other DNA
agttaacaaacttaccctcccacatagg

SEQ ID NO: 31378 - DNA, 28 bp, synthetic construct
  source 1..28: mol_type = other DNA
gttaacaaacttaccctcccacataggg

SEQ ID NO: 31379 - DNA, 28 bp, synthetic construct
  source 1..28: mol_type = other DNA
ttaacaaacttaccctcccacatagggg

SEQ ID NO: 31380 - DNA, 28 bp, synthetic construct
  source 1..28: mol_type = other DNA
gacatgaagcatcccctatgtgggaggg

SEQ ID NO: 31381 - DNA, 28 bp, synthetic construct
  source 1..28: mol_type = other DNA
tgacatgaagcatcccctatgtgggagg

SEQ ID NO: 31382 - DNA, 28 bp, synthetic construct
  source 1..28: mol_type = other DNA
gcttgacatgaagcatcccctatgtggg

SEQ ID NO: 31383 - DNA, 28 bp, synthetic construct
  source 1..28: mol_type = other DNA
ggcttgacatgaagcatcccctatgtgg

SEQ ID NO: 31384 - DNA, 28 bp, synthetic construct
  source 1..28: mol_type = other DNA
taggggatgcttcatgtcaagccactgg

SEQ ID NO: 31385 - DNA, 28 bp, synthetic construct
  source 1..28: mol_type = other DNA
aaagaagacggaggcattagaccagtgg

SEQ ID NO: 31386 - DNA, 28 bp, synthetic construct
  source 1..28: mol_type = other DNA
gataattttgaactaaagaagacggagg

SEQ ID NO: 31387 - DNA, 28 bp, synthetic construct
  source 1..28: mol_type = other DNA
taagataattttgaactaaagaagacgg

SEQ ID NO: 31388 - DNA, 28 bp, synthetic construct
  source 1..28: mol_type = other DNA
atggtggaatcatgtttgcaatatttgg

SEQ ID NO: 31389 - DNA, 28 bp, synthetic construct
  source 1..28: mol_type = other DNA
tattgcaaacatgattccaccatgttgg

SEQ ID NO: 31390 - DNA, 28 bp, synthetic construct
  source 1..28: mol_type = other DNA
ctgcacacaactgaaaccaacatggtgg

SEQ ID NO: 31391 - DNA, 28 bp, synthetic construct
  source 1..28: mol_type = other DNA
gaactgcacacaactgaaaccaacatgg

SEQ ID NO: 31392 - DNA, 28 bp, synthetic construct
  source 1..28: mol_type = other DNA
gcagttccctgactgcacacaagtcagg

SEQ ID NO: 31393 - DNA, 28 bp, synthetic construct
  source 1..28: mol_type = other DNA
cagttccctgactgcacacaagtcaggg

SEQ ID NO: 31394 - DNA, 28 bp, synthetic construct
  source 1..28: mol_type = other DNA
tagttccctgacttgtgtgcagtcaggg

SEQ ID NO: 31395 - DNA, 28 bp, synthetic construct
  source 1..28: mol_type = other DNA
ttagttccctgacttgtgtgcagtcagg

SEQ ID NO: 31396 - DNA, 28 bp, synthetic construct
  source 1..28: mol_type = other DNA
tgacactaaagaatgacaagcaaagcgg

SEQ ID NO: 31397 - DNA, 28 bp, synthetic construct
  source 1..28: mol_type = other DNA
agaatgacaagcaaagcggcatcccagg

SEQ ID NO: 31398 - DNA, 28 bp, synthetic construct
  source 1..28: mol_type = other DNA
gaatgacaagcaaagcggcatcccaggg

SEQ ID NO: 31399 - DNA, 28 bp, synthetic construct
  source 1..28: mol_type = other DNA
aagcaaagcggcatcccagggctactgg

SEQ ID NO: 31400 - DNA, 28 bp, synthetic construct
  source 1..28: mol_type = other DNA
ggcatcccagggctactggttgaacagg

SEQ ID NO: 31401 - DNA, 28 bp, synthetic construct
  source 1..28: mol_type = other DNA
gggttcctgttcaaccagtagccctggg

SEQ ID NO: 31402 - DNA, 28 bp, synthetic construct
  source 1..28: mol_type = other DNA
agggttcctgttcaaccagtagccctgg

SEQ ID NO: 31403 - DNA, 28 bp, synthetic construct
  source 1..28: mol_type = other DNA
ggctactggttgaacaggaaccctgtgg

SEQ ID NO: 31404 - DNA, 28 bp, synthetic construct
  source 1..28: mol_type = other DNA
tgagaaggtcatctcaatggccacaggg

SEQ ID NO: 31405 - DNA, 28 bp, synthetic construct
  source 1..28: mol_type = other DNA
ttgagaaggtcatctcaatggccacagg

SEQ ID NO: 31406 - DNA, 28 bp, synthetic construct
  source 1..28: mol_type = other DNA
aggaagcttgagaaggtcatctcaatgg

SEQ ID NO: 31407 - DNA, 28 bp, synthetic construct
  source 1..28: mol_type = other DNA
tgaaggctcaacaggaagcttgagaagg

SEQ ID NO: 31408 - DNA, 28 bp, synthetic construct
  source 1..28: mol_type = other DNA
ctcaagcttcctgttgagccttcactgg

SEQ ID NO: 31409 - DNA, 28 bp, synthetic construct
  source 1..28: mol_type = other DNA
tcaagcttcctgttgagccttcactggg

SEQ ID NO: 31410 - DNA, 28 bp, synthetic construct
  source 1..28: mol_type = other DNA
tcctgttgagccttcactgggacactgg

SEQ ID NO: 31411 - DNA, 28 bp, synthetic construct
  source 1..28: mol_type = other DNA
cctgttgagccttcactgggacactggg

SEQ ID NO: 31412 - DNA, 28 bp, synthetic construct
  source 1..28: mol_type = other DNA
atgcacgctcccagtgtcccagtgaagg

SEQ ID NO: 31413 - DNA, 28 bp, synthetic construct
  source 1..28: mol_type = other DNA
gcgtgtgtgcgtatgtgtatgtatcagg

SEQ ID NO: 31414 - DNA, 28 bp, synthetic construct
  source 1..28: mol_type = other DNA
tcagtatgaagtctgacatttttcatgg

SEQ ID NO: 31415 - DNA, 28 bp, synthetic construct
  source 1..28: mol_type = other DNA
tgtcagacttcatactgataatctgtgg

SEQ ID NO: 31416 - DNA, 28 bp, synthetic construct
  source 1..28: mol_type = other DNA
gtcagacttcatactgataatctgtggg

SEQ ID NO: 31417 - DNA, 28 bp, synthetic construct
  source 1..28: mol_type = other DNA
aaaagcaatctttttgtttcataaatgg

SEQ ID NO: 31418 - DNA, 28 bp, synthetic construct
  source 1..28: mol_type = other DNA
aagattgcttttcgagattataaactgg

SEQ ID NO: 31419 - DNA, 28 bp, synthetic construct
  source 1..28: mol_type = other DNA
agattgcttttcgagattataaactggg

SEQ ID NO: 31420 - DNA, 28 bp, synthetic construct
  source 1..28: mol_type = other DNA
caaaatacgttcaagtcagttgttctgg

SEQ ID NO: 31421 - DNA, 28 bp, synthetic construct
  source 1..28: mol_type = other DNA
tccgtgtaaaaatattcacagaaattgg

SEQ ID NO: 31422 - DNA, 28 bp, synthetic construct
  source 1..28: mol_type = other DNA
accaatttctgtgaatatttttacacgg

SEQ ID NO: 31423 - DNA, 28 bp, synthetic construct
  source 1..28: mol_type = other DNA
gtgtaaaaatattcacagaaattggtgg

SEQ ID NO: 31424 - DNA, 28 bp, synthetic construct
  source 1..28: mol_type = other DNA
taatgtaacatttgcaaccttagaaagg

SEQ ID NO: 31425 - DNA, 28 bp, synthetic construct
  source 1..28: mol_type = other DNA
tggattaaacatgtctgcctttctaagg

SEQ ID NO: 31426 - DNA, 28 bp, synthetic construct
  source 1..28: mol_type = other DNA
tgaaattggaatttataaacggacttgg

SEQ ID NO: 31427 - DNA, 28 bp, synthetic construct
  source 1..28: mol_type = other DNA
tccgtttataaattccaatttcacatgg

SEQ ID NO: 31428 - DNA, 28 bp, synthetic construct
  source 1..28: mol_type = other DNA
tccatgtgaaattggaatttataaacgg

SEQ ID NO: 31429 - DNA, 28 bp, synthetic construct
  source 1..28: mol_type = other DNA
ctgcagtttttaatccatgtgaaattgg

SEQ ID NO: 31430 - DNA, 28 bp, synthetic construct
  source 1..28: mol_type = other DNA
acaataatatcctgtacatgcattaagg

SEQ ID NO: 31431 - DNA, 28 bp, synthetic construct
  source 1..28: mol_type = other DNA
taatatcctgtacatgcattaaggctgg

SEQ ID NO: 31432 - DNA, 28 bp, synthetic construct
  source 1..28: mol_type = other DNA
cagtcaccagccttaatgcatgtacagg

SEQ ID NO: 31433 - DNA, 28 bp, synthetic construct
  source 1..28: mol_type = other DNA
aaggctggtgactgctaaagtctcttgg

SEQ ID NO: 31434 - DNA, 28 bp, synthetic construct
  source 1..28: mol_type = other DNA
aggctggtgactgctaaagtctcttggg

SEQ ID NO: 31435 - DNA, 28 bp, synthetic construct
  source 1..28: mol_type = other DNA
taaagtctcttgggaatctacaaatagg

SEQ ID NO: 31436 - DNA, 28 bp, synthetic construct
  source 1..28: mol_type = other DNA
aaataggaaatcacacgcagattactgg

SEQ ID NO: 31437 - DNA, 28 bp, synthetic construct
  source 1..28: mol_type = other DNA
aataggaaatcacacgcagattactggg

SEQ ID NO: 31438 - DNA, 28 bp, synthetic construct
  source 1..28: mol_type = other DNA
aaaaaatcttgcttttttttttttttgg

SEQ ID NO: 31439 - DNA, 28 bp, synthetic construct
  source 1..28: mol_type = other DNA
gtgatgcagatttcaacagtaactctgg

SEQ ID NO: 31440 - DNA, 28 bp, synthetic construct
  source 1..28: mol_type = other DNA
caaagatgtgattcataaataatgttgg

SEQ ID NO: 31441 - DNA, 28 bp, synthetic construct
  source 1..28: mol_type = other DNA
gagtcactgcgtgttcgcatcaacttgg

SEQ ID NO: 31442 - DNA, 28 bp, synthetic construct
  source 1..28: mol_type = other DNA
cacgcagtgactcatactcaatattagg

SEQ ID NO: 31443 - DNA, 28 bp, synthetic construct
  source 1..28: mol_type = other DNA
atattaggcactagtaatatccttcagg

SEQ ID NO: 31444 - DNA, 28 bp, synthetic construct
  source 1..28: mol_type = other DNA
taacataaaactgtagtacgcctgaagg

SEQ ID NO: 31445 - DNA, 28 bp, synthetic construct
  source 1..28: mol_type = other DNA
ttatacaaactgtgtatattatgtatgg

SEQ ID NO: 31446 - DNA, 28 bp, synthetic construct
  source 1..28: mol_type = other DNA
tatacaaactgtgtatattatgtatggg

SEQ ID NO: 31447 - DNA, 28 bp, synthetic construct
  source 1..28: mol_type = other DNA
atacaaactgtgtatattatgtatgggg

SEQ ID NO: 31448 - DNA, 28 bp, synthetic construct
  source 1..28: mol_type = other DNA
tacacacatcattgttgtacatatgagg

SEQ ID NO: 31449 - DNA, 28 bp, synthetic construct
  source 1..28: mol_type = other DNA
caaattgtgtactagattgaacacatgg

SEQ ID NO: 31450 - DNA, 28 bp, synthetic construct
  source 1..28: mol_type = other DNA
ttccagtacattcctcattagattgtgg

SEQ ID NO: 31451 - DNA, 28 bp, synthetic construct
  source 1..28: mol_type = other DNA
tccagtacattcctcattagattgtggg

SEQ ID NO: 31452 - DNA, 28 bp, synthetic construct
  source 1..28: mol_type = other DNA
acccacaatctaatgaggaatgtactgg

SEQ ID NO: 31453 - DNA, 28 bp, synthetic construct
  source 1..28: mol_type = other DNA
gaaacttgaaacccacaatctaatgagg

SEQ ID NO: 31454 - DNA, 28 bp, synthetic construct
  source 1..28: mol_type = other DNA
tttctggaaacattcaaattgcaaatgg

SEQ ID NO: 31455 - DNA, 28 bp, synthetic construct
  source 1..28: mol_type = other DNA
gaggtttggttaagacagagatttctgg

SEQ ID NO: 31456 - DNA, 28 bp, synthetic construct
  source 1..28: mol_type = other DNA
ctgtcttaaccaaacctctctctccagg

SEQ ID NO: 31457 - DNA, 28 bp, synthetic construct
  source 1..28: mol_type = other DNA
agaatcgtgcctggagagagaggtttgg

SEQ ID NO: 31458 - DNA, 28 bp, synthetic construct
  source 1..28: mol_type = other DNA
tgtgcagaatcgtgcctggagagagagg

SEQ ID NO: 31459 - DNA, 28 bp, synthetic construct
  source 1..28: mol_type = other DNA
tcagactcatgtgcagaatcgtgcctgg

SEQ ID NO: 31460 - DNA, 28 bp, synthetic construct
  source 1..28: mol_type = other DNA
tcatcaaaaatgccaaattttgatcagg

SEQ ID NO: 31461 - DNA, 28 bp, synthetic construct
  source 1..28: mol_type = other DNA
gccaaattttgatcaggaatatacctgg

SEQ ID NO: 31462 - DNA, 28 bp, synthetic construct
  source 1..28: mol_type = other DNA
tccaggtatattcctgatcaaaatttgg

SEQ ID NO: 31463 - DNA, 28 bp, synthetic construct
  source 1..28: mol_type = other DNA
atatacctggactactctctttcaaagg

SEQ ID NO: 31464 - DNA, 28 bp, synthetic construct
  source 1..28: mol_type = other DNA
aattgcctttgaaagagagtagtccagg

SEQ ID NO: 31465 - DNA, 28 bp, synthetic construct
  source 1..28: mol_type = other DNA
caaaggcaattgaacatcgtgataaagg

SEQ ID NO: 31466 - DNA, 28 bp, synthetic construct
  source 1..28: mol_type = other DNA
tcgtgataaaggatagcatctattcagg

SEQ ID NO: 31467 - DNA, 28 bp, synthetic construct
  source 1..28: mol_type = other DNA
taaaggatagcatctattcaggtcatgg

SEQ ID NO: 31468 - DNA, 28 bp, synthetic construct
  source 1..28: mol_type = other DNA
ggatagcatctattcaggtcatggaagg

SEQ ID NO: 31469 - DNA, 28 bp, synthetic construct
  source 1..28: mol_type = other DNA
catctattcaggtcatggaaggatatgg

SEQ ID NO: 31470 - DNA, 28 bp, synthetic construct
  source 1..28: mol_type = other DNA
ggtcagttgaacttgtgttgaactttgg

SEQ ID NO: 31471 - DNA, 28 bp, synthetic construct
  source 1..28: mol_type = other DNA
cagttgaacttgtgttgaactttggagg

SEQ ID NO: 31472 - DNA, 28 bp, synthetic construct
  source 1..28: mol_type = other DNA
atgtacgtcttcaaataaaaagacatgg

SEQ ID NO: 31473 - DNA, 28 bp, synthetic construct
  source 1..28: mol_type = other DNA
ttatttgcttaaatttgagagtctctgg

SEQ ID NO: 31474 - DNA, 28 bp, synthetic construct
  source 1..28: mol_type = other DNA
ttgcttaaatttgagagtctctggaagg

SEQ ID NO: 31475 - DNA, 28 bp, synthetic construct
  source 1..28: mol_type = other DNA
aggatatacatcaaactgtgagcagtgg

SEQ ID NO: 31476 - DNA, 28 bp, synthetic construct
  source 1..28: mol_type = other DNA
tcaaactgtgagcagtggttgtctcagg

SEQ ID NO: 31477 - DNA, 28 bp, synthetic construct
  source 1..28: mol_type = other DNA
gtgagcagtggttgtctcaggcagaagg

SEQ ID NO: 31478 - DNA, 28 bp, synthetic construct
  source 1..28: mol_type = other DNA
tgagcagtggttgtctcaggcagaaggg

SEQ ID NO: 31479 - DNA, 28 bp, synthetic construct
  source 1..28: mol_type = other DNA
gttgtctcaggcagaagggacaaccagg

SEQ ID NO: 31480 - DNA, 28 bp, synthetic construct
  source 1..28: mol_type = other DNA
ttgtctcaggcagaagggacaaccaggg

SEQ ID NO: 31481 - DNA, 28 bp, synthetic construct
  source 1..28: mol_type = other DNA
gtagaaagtagaaagtgtaagtccctgg

SEQ ID NO: 31482 - DNA, 28 bp, synthetic construct
  source 1..28: mol_type = other DNA
cttttctaattagaaaacacaagaaagg

SEQ ID NO: 31483 - DNA, 28 bp, synthetic construct
  source 1..28: mol_type = other DNA
atttcaacttgaaacaaaactaaacagg

SEQ ID NO: 31484 - DNA, 28 bp, synthetic construct
  source 1..28: mol_type = other DNA
aacttgaaacaaaactaaacaggccagg

SEQ ID NO: 31485 - DNA, 28 bp, synthetic construct
  source 1..28: mol_type = other DNA
gaaacaaaactaaacaggccaggcatgg

SEQ ID NO: 31486 - DNA, 28 bp, synthetic construct
  source 1..28: mol_type = other DNA
acaaaactaaacaggccaggcatggtgg

SEQ ID NO: 31487 - DNA, 28 bp, synthetic construct
  source 1..28: mol_type = other DNA
gccaggcatggtggctcatgcactttgg

SEQ ID NO: 31488 - DNA, 28 bp, synthetic construct
  source 1..28: mol_type = other DNA
ccaggcatggtggctcatgcactttggg

SEQ ID NO: 31489 - DNA, 28 bp, synthetic construct
  source 1..28: mol_type = other DNA
ggcatggtggctcatgcactttgggagg

SEQ ID NO: 31490 - DNA, 28 bp, synthetic construct
  source 1..28: mol_type = other DNA
gtggctcatgcactttgggaggccgagg

SEQ ID NO: 31491 - DNA, 28 bp, synthetic construct
  source 1..28: mol_type = other DNA
atgcactttgggaggccgaggccaaagg

SEQ ID NO: 31492 - DNA, 28 bp, synthetic construct
  source 1..28: mol_type = other DNA
ctgggctcaagcgatcctttggcctcgg

SEQ ID NO: 31493 - DNA, 28 bp, synthetic construct
  source 1..28: mol_type = other DNA
cgaggccaaaggatcgcttgagcccagg

SEQ ID NO: 31494 - DNA, 28 bp, synthetic construct
  source 1..28: mol_type = other DNA
aaactcctgggctcaagcgatcctttgg

SEQ ID NO: 31495 - DNA, 28 bp, synthetic construct
  source 1..28: mol_type = other DNA
tgagcccaggagtttgagaccagcctgg

SEQ ID NO: 31496 - DNA, 28 bp, synthetic construct
  source 1..28: mol_type = other DNA
gagcccaggagtttgagaccagcctggg

SEQ ID NO: 31497 - DNA, 28 bp, synthetic construct
  source 1..28: mol_type = other DNA
ttgcccaggctggtctcaaactcctggg

SEQ ID NO: 31498 - DNA, 28 bp, synthetic construct
  source 1..28: mol_type = other DNA
gttgcccaggctggtctcaaactcctgg

SEQ ID NO: 31499 - DNA, 28 bp, synthetic construct
  source 1..28: mol_type = other DNA
gggggtctcactatgttgcccaggctgg

SEQ ID NO: 31500 - DNA, 28 bp, synthetic construct
  source 1..28: mol_type = other DNA
agatgggggtctcactatgttgcccagg

SEQ ID NO: 31501 - DNA, 28 bp, synthetic construct
  source 1..28: mol_type = other DNA
ttctttattttttttgtagagatggggg

SEQ ID NO: 31502 - DNA, 28 bp, synthetic construct
  source 1..28: mol_type = other DNA
tttctttattttttttgtagagatgggg

SEQ ID NO: 31503 - DNA, 28 bp, synthetic construct
  source 1..28: mol_type = other DNA
ttttctttattttttttgtagagatggg

SEQ ID NO: 31504 - DNA, 28 bp, synthetic construct
  source 1..28: mol_type = other DNA
tttttctttattttttttgtagagatgg

SEQ ID NO: 31505 - DNA, 28 bp, synthetic construct
  source 1..28: mol_type = other DNA
caaaaaaaataaagaaaaaattagccgg

SEQ ID NO: 31506 - DNA, 28 bp, synthetic construct
  source 1..28: mol_type = other DNA
aaaaaaaataaagaaaaaattagccggg

SEQ ID NO: 31507 - DNA, 28 bp, synthetic construct
  source 1..28: mol_type = other DNA
aaataaagaaaaaattagccgggtgtgg

SEQ ID NO: 31508 - DNA, 28 bp, synthetic construct
  source 1..28: mol_type = other DNA
taaagaaaaaattagccgggtgtggtgg

SEQ ID NO: 31509 - DNA, 28 bp, synthetic construct
  source 1..28: mol_type = other DNA
gaagataggcacgtgccaccacacccgg

SEQ ID NO: 31510 - DNA, 28 bp, synthetic construct
  source 1..28: mol_type = other DNA
gcacgtgcctatcttcccagctgcttgg

SEQ ID NO: 31511 - DNA, 28 bp, synthetic construct
  source 1..28: mol_type = other DNA
cacgtgcctatcttcccagctgcttggg

SEQ ID NO: 31512 - DNA, 28 bp, synthetic construct
  source 1..28: mol_type = other DNA
gtgcctatcttcccagctgcttgggagg

SEQ ID NO: 31513 - DNA, 28 bp, synthetic construct
  source 1..28: mol_type = other DNA
cagcctcccaagcagctgggaagatagg

SEQ ID NO: 31514 - DNA, 28 bp, synthetic construct
  source 1..28: mol_type = other DNA
atcttcccagctgcttgggaggctgagg

SEQ ID NO: 31515 - DNA, 28 bp, synthetic construct
  source 1..28: mol_type = other DNA
tcccagctgcttgggaggctgaggcagg

SEQ ID NO: 31516 - DNA, 28 bp, synthetic construct
  source 1..28: mol_type = other DNA
tcctgcctcagcctcccaagcagctggg

SEQ ID NO: 31517 - DNA, 28 bp, synthetic construct
  source 1..28: mol_type = other DNA
ctcctgcctcagcctcccaagcagctgg

SEQ ID NO: 31518 - DNA, 28 bp, synthetic construct
  source 1..28: mol_type = other DNA
cagctgcttgggaggctgaggcaggagg

SEQ ID NO: 31519 - DNA, 28 bp, synthetic construct
  source 1..28: mol_type = other DNA
tgaggcaggaggattgcttgagcccagg

SEQ ID NO: 31520 - DNA, 28 bp, synthetic construct
  source 1..28: mol_type = other DNA
aggattgcttgagcccaggagtttgagg

SEQ ID NO: 31521 - DNA, 28 bp, synthetic construct
  source 1..28: mol_type = other DNA
cttgagcccaggagtttgaggctgcagg

SEQ ID NO: 31522 - DNA, 28 bp, synthetic construct
  source 1..28: mol_type = other DNA
ttgagcccaggagtttgaggctgcaggg

SEQ ID NO: 31523 - DNA, 28 bp, synthetic construct
  source 1..28: mol_type = other DNA
tggctccctgcagcctcaaactcctggg

SEQ ID NO: 31524 - DNA, 28 bp, synthetic construct
  source 1..28: mol_type = other DNA
atggctccctgcagcctcaaactcctgg

SEQ ID NO: 31525 - DNA, 28 bp, synthetic construct
  source 1..28: mol_type = other DNA
aagctggaatgcggtggcgcgatcatgg

SEQ ID NO: 31526 - DNA, 28 bp, synthetic construct
  source 1..28: mol_type = other DNA
atgatcgcgccaccgcattccagcttgg

SEQ ID NO: 31527 - DNA, 28 bp, synthetic construct
  source 1..28: mol_type = other DNA
tgatcgcgccaccgcattccagcttggg

SEQ ID NO: 31528 - DNA, 28 bp, synthetic construct
  source 1..28: mol_type = other DNA
ctctgtagcccaagctggaatgcggtgg

SEQ ID NO: 31529 - DNA, 28 bp, synthetic construct
  source 1..28: mol_type = other DNA
tggctctgtagcccaagctggaatgcgg

SEQ ID NO: 31530 - DNA, 28 bp, synthetic construct
  source 1..28: mol_type = other DNA
ccgggtctggctctgtagcccaagctgg

SEQ ID NO: 31531 - DNA, 28 bp, synthetic construct
  source 1..28: mol_type = other DNA
gtttggttggttttgagaccgggtctgg

SEQ ID NO: 31532 - DNA, 28 bp, synthetic construct
  source 1..28: mol_type = other DNA
tgttggtttggttggttttgagaccggg

SEQ ID NO: 31533 - DNA, 28 bp, synthetic construct
  source 1..28: mol_type = other DNA
ttgttggtttggttggttttgagaccgg

SEQ ID NO: 31534 - DNA, 28 bp, synthetic construct
  source 1..28: mol_type = other DNA
ttactgctgttgttgttggtttggttgg

SEQ ID NO: 31535 - DNA, 28 bp, synthetic construct
  source 1..28: mol_type = other DNA
gttgttactgctgttgttgttggtttgg

SEQ ID NO: 31536 - DNA, 28 bp, synthetic construct
  source 1..28: mol_type = other DNA
gttttgttgttactgctgttgttgttgg

SEQ ID NO: 31537 - DNA, 28 bp, synthetic construct
  source 1..28: mol_type = other DNA
agcagtaacaacaaaactaagtaaaagg

SEQ ID NO: 31538 - DNA, 28 bp, synthetic construct
  source 1..28: mol_type = other DNA
atgaatgactttcacaagcaacaattgg

SEQ ID NO: 31539 - DNA, 28 bp, synthetic construct
  source 1..28: mol_type = other DNA
aatgactttcacaagcaacaattggagg

SEQ ID NO: 31540 - DNA, 28 bp, synthetic construct
  source 1..28: mol_type = other DNA
actttcacaagcaacaattggaggatgg

SEQ ID NO: 31541 - DNA, 28 bp, synthetic construct
  source 1..28: mol_type = other DNA
ctgtggggtttggcatgggtgattttgg

SEQ ID NO: 31542 - DNA, 28 bp, synthetic construct
  source 1..28: mol_type = other DNA
cagcagtttctgtggggtttggcatggg

SEQ ID NO: 31543 - DNA, 28 bp, synthetic construct
  source 1..28: mol_type = other DNA
acagcagtttctgtggggtttggcatgg

SEQ ID NO: 31544 - DNA, 28 bp, synthetic construct
  source 1..28: mol_type = other DNA
ttggtacagcagtttctgtggggtttgg

SEQ ID NO: 31545 - DNA, 28 bp, synthetic construct
  source 1..28: mol_type = other DNA
gcacgttggtacagcagtttctgtgggg

SEQ ID NO: 31546 - DNA, 28 bp, synthetic construct
  source 1..28: mol_type = other DNA
agcacgttggtacagcagtttctgtggg

SEQ ID NO: 31547 - DNA, 28 bp, synthetic construct
  source 1..28: mol_type = other DNA
gagcacgttggtacagcagtttctgtgg

SEQ ID NO: 31548 - DNA, 28 bp, synthetic construct
  source 1..28: mol_type = other DNA
tctgtggagcacgtgtggagcacgttgg

SEQ ID NO: 31549 - DNA, 28 bp, synthetic construct
  source 1..28: mol_type = other DNA
tcttgtttcatctgtggagcacgtgtgg

SEQ ID NO: 31550 - DNA, 28 bp, synthetic construct
  source 1..28: mol_type = other DNA
tcttatgactgtcttgtttcatctgtgg

SEQ ID NO: 31551 - DNA, 28 bp, synthetic construct
  source 1..28: mol_type = other DNA
tacacgctctgaccactgcccacaacgg

SEQ ID NO: 31552 - DNA, 28 bp, synthetic construct
  source 1..28: mol_type = other DNA
tcttgaaacttaccgttgtgggcagtgg

SEQ ID NO: 31553 - DNA, 28 bp, synthetic construct
  source 1..28: mol_type = other DNA
aaaacttcttgaaacttaccgttgtggg

SEQ ID NO: 31554 - DNA, 28 bp, synthetic construct
  source 1..28: mol_type = other DNA
gaaaacttcttgaaacttaccgttgtgg

SEQ ID NO: 31555 - DNA, 28 bp, synthetic construct
  source 1..28: mol_type = other DNA
aacggtaagtttcaagaagttttcctgg

SEQ ID NO: 31556 - DNA, 28 bp, synthetic construct
  source 1..28: mol_type = other DNA
acggtaagtttcaagaagttttcctggg

SEQ ID NO: 31557 - DNA, 28 bp, synthetic construct
  source 1..28: mol_type = other DNA
tttcaagaagttttcctgggaaatgtgg

SEQ ID NO: 31558 - DNA, 28 bp, synthetic construct
  source 1..28: mol_type = other DNA
ttcaagaagttttcctgggaaatgtggg

SEQ ID NO: 31559 - DNA, 28 bp, synthetic construct
  source 1..28: mol_type = other DNA
agcactctgatggcccacatttcccagg

SEQ ID NO: 31560 - DNA, 28 bp, synthetic construct
  source 1..28: mol_type = other DNA
cagcagtgttttatcagcactctgatgg

SEQ ID NO: 31561 - DNA, 28 bp, synthetic construct
  source 1..28: mol_type = other DNA
catcagagtgctgataaaacactgctgg

SEQ ID NO: 31562 - DNA, 28 bp, synthetic construct
  source 1..28: mol_type = other DNA
aaacactgctggcccacctgtcaaatgg

SEQ ID NO: 31563 - DNA, 28 bp, synthetic construct
  source 1..28: mol_type = other DNA
aacactgctggcccacctgtcaaatggg

SEQ ID NO: 31564 - DNA, 28 bp, synthetic construct
  source 1..28: mol_type = other DNA
acactgctggcccacctgtcaaatgggg

SEQ ID NO: 31565 - DNA, 28 bp, synthetic construct
  source 1..28: mol_type = other DNA
gcccacctgtcaaatggggcttcacagg

SEQ ID NO: 31566 - DNA, 28 bp, synthetic construct
  source 1..28: mol_type = other DNA
ccctgtgaagccccatttgacaggtggg

SEQ ID NO: 31567 - DNA, 28 bp, synthetic construct
  source 1..28: mol_type = other DNA
tccctgtgaagccccatttgacaggtgg

SEQ ID NO: 31568 - DNA, 28 bp, synthetic construct
  source 1..28: mol_type = other DNA
gcttccctgtgaagccccatttgacagg

SEQ ID NO: 31569 - DNA, 28 bp, synthetic construct
  source 1..28: mol_type = other DNA
gttacaacaaagtctgcaactttcaagg

SEQ ID NO: 31570 - DNA, 28 bp, synthetic construct
  source 1..28: mol_type = other DNA
acaacaaagtctgcaactttcaaggtgg

SEQ ID NO: 31571 - DNA, 28 bp, synthetic construct
  source 1..28: mol_type = other DNA
caacaaagtctgcaactttcaaggtggg

SEQ ID NO: 31572 - DNA, 28 bp, synthetic construct
  source 1..28: mol_type = other DNA
aaagtctgcaactttcaaggtgggcagg

SEQ ID NO: 31573 - DNA, 28 bp, synthetic construct
  source 1..28: mol_type = other DNA
gtgggcaggaccagagaagctctccagg

SEQ ID NO: 31574 - DNA, 28 bp, synthetic construct
  source 1..28: mol_type = other DNA
gaccagagaagctctccaggtatgcagg

SEQ ID NO: 31575 - DNA, 28 bp, synthetic construct
  source 1..28: mol_type = other DNA
atcctgcatacctggagagcttctctgg

SEQ ID NO: 31576 - DNA, 28 bp, synthetic construct
  source 1..28: mol_type = other DNA
ctccaggtatgcaggatagacctccagg

SEQ ID NO: 31577 - DNA, 28 bp, synthetic construct
  source 1..28: mol_type = other DNA
tccaggtatgcaggatagacctccaggg

SEQ ID NO: 31578 - DNA, 28 bp, synthetic construct
  source 1..28: mol_type = other DNA
gccctggaggtctatcctgcatacctgg

SEQ ID NO: 31579 - DNA, 28 bp, synthetic construct
  source 1..28: mol_type = other DNA
caaacacataaagggatggccctggagg

SEQ ID NO: 31580 - DNA, 28 bp, synthetic construct
  source 1..28: mol_type = other DNA
attcaaacacataaagggatggccctgg

SEQ ID NO: 31581 - DNA, 28 bp, synthetic construct
  source 1..28: mol_type = other DNA
tgaaatattcaaacacataaagggatgg

SEQ ID NO: 31582 - DNA, 28 bp, synthetic construct
  source 1..28: mol_type = other DNA
ctgatgaaatattcaaacacataaaggg

SEQ ID NO: 31583 - DNA, 28 bp, synthetic construct
  source 1..28: mol_type = other DNA
cctttatgtgtttgaatatttcatcagg

SEQ ID NO: 31584 - DNA, 28 bp, synthetic construct
  source 1..28: mol_type = other DNA
tatttcatcaggattcttcaagagtagg

SEQ ID NO: 31585 - DNA, 28 bp, synthetic construct
  source 1..28: mol_type = other DNA
tttgagtcatttttttggaggactgagg

SEQ ID NO: 31586 - DNA, 28 bp, synthetic construct
  source 1..28: mol_type = other DNA
aagaaattttgagtcatttttttggagg

SEQ ID NO: 31587 - DNA, 28 bp, synthetic construct
  source 1..28: mol_type = other DNA
cttaagaaattttgagtcatttttttgg

SEQ ID NO: 31588 - DNA, 28 bp, synthetic construct
  source 1..28: mol_type = other DNA
aaaatgactcaaaatttcttaagttagg

SEQ ID NO: 31589 - DNA, 28 bp, synthetic construct
  source 1..28: mol_type = other DNA
taagttaggttcaagtttctgacatagg

SEQ ID NO: 31590 - DNA, 28 bp, synthetic construct
  source 1..28: mol_type = other DNA
ttaggttcaagtttctgacataggatgg

SEQ ID NO: 31591 - DNA, 28 bp, synthetic construct
  source 1..28: mol_type = other DNA
taggttcaagtttctgacataggatggg

SEQ ID NO: 31592 - DNA, 28 bp, synthetic construct
  source 1..28: mol_type = other DNA
gtgaactctgccaaaaattagtgaaagg

SEQ ID NO: 31593 - DNA, 28 bp, synthetic construct
  source 1..28: mol_type = other DNA
tgaactctgccaaaaattagtgaaaggg

SEQ ID NO: 31594 - DNA, 28 bp, synthetic construct
  source 1..28: mol_type = other DNA
ctctgccaaaaattagtgaaagggctgg

SEQ ID NO: 31595 - DNA, 28 bp, synthetic construct
  source 1..28: mol_type = other DNA
tctgccaaaaattagtgaaagggctggg

SEQ ID NO: 31596 - DNA, 28 bp, synthetic construct
  source 1..28: mol_type = other DNA
cacacccagccctttcactaatttttgg

SEQ ID NO: 31597 - DNA, 28 bp, synthetic construct
  source 1..28: mol_type = other DNA
caaaaattagtgaaagggctgggtgtgg

SEQ ID NO: 31598 - DNA, 28 bp, synthetic construct
  source 1..28: mol_type = other DNA
aaattagtgaaagggctgggtgtggtgg

SEQ ID NO: 31599 - DNA, 28 bp, synthetic construct
  source 1..28: mol_type = other DNA
gctcacgcctgtaatcacaacactttgg

SEQ ID NO: 31600 - DNA, 28 bp, synthetic construct
  source 1..28: mol_type = other DNA
ctcacgcctgtaatcacaacactttggg

SEQ ID NO: 31601 - DNA, 28 bp, synthetic construct
  source 1..28: mol_type = other DNA
acgcctgtaatcacaacactttgggagg

SEQ ID NO: 31602 - DNA, 28 bp, synthetic construct
  source 1..28: mol_type = other DNA
cctgtaatcacaacactttgggaggtgg

SEQ ID NO: 31603 - DNA, 28 bp, synthetic construct
  source 1..28: mol_type = other DNA
gtaatcacaacactttgggaggtggagg

SEQ ID NO: 31604 - DNA, 28 bp, synthetic construct
  source 1..28: mol_type = other DNA
atcacaacactttgggaggtggaggcgg

SEQ ID NO: 31605 - DNA, 28 bp, synthetic construct
  source 1..28: mol_type = other DNA
tcacaacactttgggaggtggaggcggg

SEQ ID NO: 31606 - DNA, 28 bp, synthetic construct
  source 1..28: mol_type = other DNA
gaggtggaggcgggtagatcacctgagg

SEQ ID NO: 31607 - DNA, 28 bp, synthetic construct
  source 1..28: mol_type = other DNA
ggaggcgggtagatcacctgaggtcagg

SEQ ID NO: 31608 - DNA, 28 bp, synthetic construct
  source 1..28: mol_type = other DNA
aggctcgtctcaaactcctgacctcagg

SEQ ID NO: 31609 - DNA, 28 bp, synthetic construct
  source 1..28: mol_type = other DNA
tgaggtcaggagtttgagacgagcctgg

SEQ ID NO: 31610 - DNA, 28 bp, synthetic construct
  source 1..28: mol_type = other DNA
gagtttgagacgagcctggccaacatgg

SEQ ID NO: 31611 - DNA, 28 bp, synthetic construct
  source 1..28: mol_type = other DNA
gagactgggtttcaccatgttggccagg

SEQ ID NO: 31612 - DNA, 28 bp, synthetic construct
  source 1..28: mol_type = other DNA
tagtagagactgggtttcaccatgttgg

SEQ ID NO: 31613 - DNA, 28 bp, synthetic construct
  source 1..28: mol_type = other DNA
aatttttgtgtttttagtagagactggg

SEQ ID NO: 31614 - DNA, 28 bp, synthetic construct
  source 1..28: mol_type = other DNA
taatttttgtgtttttagtagagactgg

SEQ ID NO: 31615 - DNA, 28 bp, synthetic construct
  source 1..28: mol_type = other DNA
ctctactaaaaacacaaaaattagctgg

SEQ ID NO: 31616 - DNA, 28 bp, synthetic construct
  source 1..28: mol_type = other DNA
tctactaaaaacacaaaaattagctggg

SEQ ID NO: 31617 - DNA, 28 bp, synthetic construct
  source 1..28: mol_type = other DNA
taaaaacacaaaaattagctgggcatgg

SEQ ID NO: 31618 - DNA, 28 bp, synthetic construct
  source 1..28: mol_type = other DNA
gtgcacacctgtaatcccagctacttgg

SEQ ID NO: 31619 - DNA, 28 bp, synthetic construct
  source 1..28: mol_type = other DNA
tgcacacctgtaatcccagctacttggg

SEQ ID NO: 31620 - DNA, 28 bp, synthetic construct
  source 1..28: mol_type = other DNA
acacctgtaatcccagctacttgggagg

SEQ ID NO: 31621 - DNA, 28 bp, synthetic construct
  source 1..28: mol_type = other DNA
cagcctcccaagtagctgggattacagg

SEQ ID NO: 31622 - DNA, 28 bp, synthetic construct
  source 1..28: mol_type = other DNA
gtaatcccagctacttgggaggctgagg

SEQ ID NO: 31623 - DNA, 28 bp, synthetic construct
  source 1..28: mol_type = other DNA
atcccagctacttgggaggctgaggcgg

SEQ ID NO: 31624 - DNA, 28 bp, synthetic construct
  source 1..28: mol_type = other DNA
tcccagctacttgggaggctgaggcggg

SEQ ID NO: 31625 - DNA, 28 bp, synthetic construct
  source 1..28: mol_type = other DNA
tcccgcctcagcctcccaagtagctggg

SEQ ID NO: 31626 - DNA, 28 bp, synthetic construct
  source 1..28: mol_type = other DNA
gtcccgcctcagcctcccaagtagctgg

SEQ ID NO: 31627 - DNA, 28 bp, synthetic construct
  source 1..28: mol_type = other DNA
tgaggcgggacaatcacttgaacccagg

SEQ ID NO: 31628 - DNA, 28 bp, synthetic construct
  source 1..28: mol_type = other DNA
ggcgggacaatcacttgaacccaggagg

SEQ ID NO: 31629 - DNA, 28 bp, synthetic construct
  source 1..28: mol_type = other DNA
acaatcacttgaacccaggaggcagagg

SEQ ID NO: 31630 - DNA, 28 bp, synthetic construct
  source 1..28: mol_type = other DNA
cggctcactgcatcctctgcctcctggg

SEQ ID NO: 31631 - DNA, 28 bp, synthetic construct
  source 1..28: mol_type = other DNA
tcggctcactgcatcctctgcctcctgg

SEQ ID NO: 31632 - DNA, 28 bp, synthetic construct
  source 1..28: mol_type = other DNA
aggctggagtgcagtggcacgatctcgg

SEQ ID NO: 31633 - DNA, 28 bp, synthetic construct
  source 1..28: mol_type = other DNA
gagatcgtgccactgcactccagcctgg

SEQ ID NO: 31634 - DNA, 28 bp, synthetic construct
  source 1..28: mol_type = other DNA
agatcgtgccactgcactccagcctggg

SEQ ID NO: 31635 - DNA, 28 bp, synthetic construct
  source 1..28: mol_type = other DNA
ctctgttgcccaggctggagtgcagtgg

SEQ ID NO: 31636 - DNA, 28 bp, synthetic construct
  source 1..28: mol_type = other DNA
acgagtttcgctctgttgcccaggctgg

SEQ ID NO: 31637 - DNA, 28 bp, synthetic construct
  source 1..28: mol_type = other DNA
tgagacgagtttcgctctgttgcccagg

SEQ ID NO: 31638 - DNA, 28 bp, synthetic construct
  source 1..28: mol_type = other DNA
aaactcgtctcaaaaaaaaagtgaaagg

SEQ ID NO: 31639 - DNA, 28 bp, synthetic construct
  source 1..28: mol_type = other DNA
aactcgtctcaaaaaaaaagtgaaaggg

SEQ ID NO: 31640 - DNA, 28 bp, synthetic construct
  source 1..28: mol_type = other DNA
aaagggttgtaagaagcaccccagttgg

SEQ ID NO: 31641 - DNA, 28 bp, synthetic construct
  source 1..28: mol_type = other DNA
gcaccccagttggagacatgtaaaatgg

SEQ ID NO: 31642 - DNA, 28 bp, synthetic construct
  source 1..28: mol_type = other DNA
tttccattttacatgtctccaactgggg

SEQ ID NO: 31643 - DNA, 28 bp, synthetic construct
  source 1..28: mol_type = other DNA
atttccattttacatgtctccaactggg

SEQ ID NO: 31644 - DNA, 28 bp, synthetic construct
  source 1..28: mol_type = other DNA
aatttccattttacatgtctccaactgg

SEQ ID NO: 31645 - DNA, 28 bp, synthetic construct
  source 1..28: mol_type = other DNA
tctcttaatatttccaaatgcttgaagg

SEQ ID NO: 31646 - DNA, 28 bp, synthetic construct
  source 1..28: mol_type = other DNA
catttggctttggccttcaagcatttgg

SEQ ID NO: 31647 - DNA, 28 bp, synthetic construct
  source 1..28: mol_type = other DNA
ggcttgtggaatttgcatttggctttgg

SEQ ID NO: 31648 - DNA, 28 bp, synthetic construct
  source 1..28: mol_type = other DNA
aagaagggcttgtggaatttgcatttgg

SEQ ID NO: 31649 - DNA, 28 bp, synthetic construct
  source 1..28: mol_type = other DNA
attaattgaaaataagaagggcttgtgg

SEQ ID NO: 31650 - DNA, 28 bp, synthetic construct
  source 1..28: mol_type = other DNA
atttgaaattaattgaaaataagaaggg

SEQ ID NO: 31651 - DNA, 28 bp, synthetic construct
  source 1..28: mol_type = other DNA
gatttgaaattaattgaaaataagaagg

SEQ ID NO: 31652 - DNA, 28 bp, synthetic construct
  source 1..28: mol_type = other DNA
aattttgaatcagtgctcagagctaagg

SEQ ID NO: 31653 - DNA, 28 bp, synthetic construct
  source 1..28: mol_type = other DNA
tgatcttacttcccacctacagatcagg

SEQ ID NO: 31654 - DNA, 28 bp, synthetic construct
  source 1..28: mol_type = other DNA
atttttgttagcctgatctgtaggtggg

SEQ ID NO: 31655 - DNA, 28 bp, synthetic construct
  source 1..28: mol_type = other DNA
catttttgttagcctgatctgtaggtgg

SEQ ID NO: 31656 - DNA, 28 bp, synthetic construct
  source 1..28: mol_type = other DNA
taacatttttgttagcctgatctgtagg

SEQ ID NO: 31657 - DNA, 28 bp, synthetic construct
  source 1..28: mol_type = other DNA
aacattcactgatattcttacaggttgg

SEQ ID NO: 31658 - DNA, 28 bp, synthetic construct
  source 1..28: mol_type = other DNA
cataaacattcactgatattcttacagg

SEQ ID NO: 31659 - DNA, 28 bp, synthetic construct
  source 1..28: mol_type = other DNA
ctgtaagaatatcagtgaatgtttatgg

SEQ ID NO: 31660 - DNA, 28 bp, synthetic construct
  source 1..28: mol_type = other DNA
ttgtgccgtcatcaccttgaaaaaatgg

SEQ ID NO: 31661 - DNA, 28 bp, synthetic construct
  source 1..28: mol_type = other DNA
gcaatccattttttcaaggtgatgacgg

SEQ ID NO: 31662 - DNA, 28 bp, synthetic construct
  source 1..28: mol_type = other DNA
atatgtggtgcaatccattttttcaagg

SEQ ID NO: 31663 - DNA, 28 bp, synthetic construct
  source 1..28: mol_type = other DNA
tgagaaaggcaggcggtgtaatatgtgg

SEQ ID NO: 31664 - DNA, 28 bp, synthetic construct
  source 1..28: mol_type = other DNA
accgcctgcctttctcagaccgtcctgg

SEQ ID NO: 31665 - DNA, 28 bp, synthetic construct
  source 1..28: mol_type = other DNA
accaggacggtctgagaaaggcaggcgg

SEQ ID NO: 31666 - DNA, 28 bp, synthetic construct
  source 1..28: mol_type = other DNA
tgcaccaggacggtctgagaaaggcagg

SEQ ID NO: 31667 - DNA, 28 bp, synthetic construct
  source 1..28: mol_type = other DNA
aagttgcaccaggacggtctgagaaagg

SEQ ID NO: 31668 - DNA, 28 bp, synthetic construct
  source 1..28: mol_type = other DNA
cttacttgataaagttgcaccaggacgg

SEQ ID NO: 31669 - DNA, 28 bp, synthetic construct
  source 1..28: mol_type = other DNA
tcctggtgcaactttatcaagtaagagg

SEQ ID NO: 31670 - DNA, 28 bp, synthetic construct
  source 1..28: mol_type = other DNA
gcctcttacttgataaagttgcaccagg

SEQ ID NO: 31671 - DNA, 28 bp, synthetic construct
  source 1..28: mol_type = other DNA
caactttatcaagtaagaggccacaagg

SEQ ID NO: 31672 - DNA, 28 bp, synthetic construct
  source 1..28: mol_type = other DNA
gttaaaaacaaaaataatgtccttgtgg

SEQ ID NO: 31673 - DNA, 28 bp, synthetic construct
  source 1..28: mol_type = other DNA
ggacattatttttgtttttaacgtgtgg

SEQ ID NO: 31674 - DNA, 28 bp, synthetic construct
  source 1..28: mol_type = other DNA
tgtggcaagatagaccctctttttcagg

SEQ ID NO: 31675 - DNA, 28 bp, synthetic construct
  source 1..28: mol_type = other DNA
aaaagaaaataactcctgaaaaagaggg

SEQ ID NO: 31676 - DNA, 28 bp, synthetic construct
  source 1..28: mol_type = other DNA
gaaaagaaaataactcctgaaaaagagg

SEQ ID NO: 31677 - DNA, 28 bp, synthetic construct
  source 1..28: mol_type = other DNA
atttagtcatcttgttaaatatatttgg

SEQ ID NO: 31678 - DNA, 28 bp, synthetic construct
  source 1..28: mol_type = other DNA
tatatttaacaagatgactaaatctagg

SEQ ID NO: 31679 - DNA, 28 bp, synthetic construct
  source 1..28: mol_type = other DNA
atatttaacaagatgactaaatctaggg

SEQ ID NO: 31680 - DNA, 28 bp, synthetic construct
  source 1..28: mol_type = other DNA
gaaaacaagagaaaaactcagagcaagg

SEQ ID NO: 31681 - DNA, 28 bp, synthetic construct
  source 1..28: mol_type = other DNA
caaggtgtaaacataccagacacacagg

SEQ ID NO: 31682 - DNA, 28 bp, synthetic construct
  source 1..28: mol_type = other DNA
taaacataccagacacacaggacacagg

SEQ ID NO: 31683 - DNA, 28 bp, synthetic construct
  source 1..28: mol_type = other DNA
taccagacacacaggacacaggaagagg

SEQ ID NO: 31684 - DNA, 28 bp, synthetic construct
  source 1..28: mol_type = other DNA
agcctcttcctgtgtcctgtgtgtctgg

SEQ ID NO: 31685 - DNA, 28 bp, synthetic construct
  source 1..28: mol_type = other DNA
acacacaggacacaggaagaggctctgg

SEQ ID NO: 31686 - DNA, 28 bp, synthetic construct
  source 1..28: mol_type = other DNA
ggctctggttgctgctgccccagaaagg

SEQ ID NO: 31687 - DNA, 28 bp, synthetic construct
  source 1..28: mol_type = other DNA
tgcagaagatcacagttcctttctgggg

SEQ ID NO: 31688 - DNA, 28 bp, synthetic construct
  source 1..28: mol_type = other DNA
atgcagaagatcacagttcctttctggg

SEQ ID NO: 31689 - DNA, 28 bp, synthetic construct
  source 1..28: mol_type = other DNA
aatgcagaagatcacagttcctttctgg

SEQ ID NO: 31690 - DNA, 28 bp, synthetic construct
  source 1..28: mol_type = other DNA
ggcgatttttcaggctttgattagcagg

SEQ ID NO: 31691 - DNA, 28 bp, synthetic construct
  source 1..28: mol_type = other DNA
cgttttgatttgggggcgatttttcagg

SEQ ID NO: 31692 - DNA, 28 bp, synthetic construct
  source 1..28: mol_type = other DNA
tcgcccccaaatcaaaacgcatcaaagg

SEQ ID NO: 31693 - DNA, 28 bp, synthetic construct
  source 1..28: mol_type = other DNA
cgcccccaaatcaaaacgcatcaaaggg

SEQ ID NO: 31694 - DNA, 28 bp, synthetic construct
  source 1..28: mol_type = other DNA
agccctttgatgcgttttgatttggggg

SEQ ID NO: 31695 - DNA, 28 bp, synthetic construct
  source 1..28: mol_type = other DNA
cagccctttgatgcgttttgatttgggg

SEQ ID NO: 31696 - DNA, 28 bp, synthetic construct
  source 1..28: mol_type = other DNA
gcagccctttgatgcgttttgatttggg

SEQ ID NO: 31697 - DNA, 28 bp, synthetic construct
  source 1..28: mol_type = other DNA
tgcagccctttgatgcgttttgatttgg

SEQ ID NO: 31698 - DNA, 28 bp, synthetic construct
  source 1..28: mol_type = other DNA
aaatcaaaacgcatcaaagggctgcagg

SEQ ID NO: 31699 - DNA, 28 bp, synthetic construct
  source 1..28: mol_type = other DNA
gggctgcaggtgcacattctgcatgagg

SEQ ID NO: 31700 - DNA, 28 bp, synthetic construct
  source 1..28: mol_type = other DNA
aggagtgagagaatcagcattatcatgg

SEQ ID NO: 31701 - DNA, 28 bp, synthetic construct
  source 1..28: mol_type = other DNA
ttatcatggcaaatagctctcagcctgg

SEQ ID NO: 31702 - DNA, 28 bp, synthetic construct
  source 1..28: mol_type = other DNA
aaatagctctcagcctggtaagcgaagg

SEQ ID NO: 31703 - DNA, 28 bp, synthetic construct
  source 1..28: mol_type = other DNA
tctcagcctggtaagcgaaggattcagg

SEQ ID NO: 31704 - DNA, 28 bp, synthetic construct
  source 1..28: mol_type = other DNA
taggagcctgaatccttcgcttaccagg

SEQ ID NO: 31705 - DNA, 28 bp, synthetic construct
  source 1..28: mol_type = other DNA
agcgaaggattcaggctcctactgaagg

SEQ ID NO: 31706 - DNA, 28 bp, synthetic construct
  source 1..28: mol_type = other DNA
gcgaaggattcaggctcctactgaaggg

SEQ ID NO: 31707 - DNA, 28 bp, synthetic construct
  source 1..28: mol_type = other DNA
caggctcctactgaagggacaatctagg

SEQ ID NO: 31708 - DNA, 28 bp, synthetic construct
  source 1..28: mol_type = other DNA
cctactgaagggacaatctaggtaatgg

SEQ ID NO: 31709 - DNA, 28 bp, synthetic construct
  source 1..28: mol_type = other DNA
tcttacagattttcttggctaaatgagg

SEQ ID NO: 31710 - DNA, 28 bp, synthetic construct
  source 1..28: mol_type = other DNA
ccaagaaaatctgtaagaaagctattgg

SEQ ID NO: 31711 - DNA, 28 bp, synthetic construct
  source 1..28: mol_type = other DNA
agaaaatctgtaagaaagctattggtgg

SEQ ID NO: 31712 - DNA, 28 bp, synthetic construct
  source 1..28: mol_type = other DNA
tggaaagaaaagacttgaaacagattgg

SEQ ID NO: 31713 - DNA, 28 bp, synthetic construct
  source 1..28: mol_type = other DNA
aacagattggctgacaaatgccatgtgg

SEQ ID NO: 31714 - DNA, 28 bp, synthetic construct
  source 1..28: mol_type = other DNA
gtgactcggtggctgtagagccacatgg

SEQ ID NO: 31715 - DNA, 28 bp, synthetic construct
  source 1..28: mol_type = other DNA
tggctctacagccaccgagtcacagtgg

SEQ ID NO: 31716 - DNA, 28 bp, synthetic construct
  source 1..28: mol_type = other DNA
tctacagccaccgagtcacagtggcagg

SEQ ID NO: 31717 - DNA, 28 bp, synthetic construct
  source 1..28: mol_type = other DNA
tcttcttcctgccactgtgactcggtgg

SEQ ID NO: 31718 - DNA, 28 bp, synthetic construct
  source 1..28: mol_type = other DNA
atttcttcttcctgccactgtgactcgg

SEQ ID NO: 31719 - DNA, 28 bp, synthetic construct
  source 1..28: mol_type = other DNA
cagtggcaggaagaagaaatgcatgtgg

SEQ ID NO: 31720 - DNA, 28 bp, synthetic construct
  source 1..28: mol_type = other DNA
ggcaggaagaagaaatgcatgtggctgg

SEQ ID NO: 31721 - DNA, 28 bp, synthetic construct
  source 1..28: mol_type = other DNA
aggaagaagaaatgcatgtggctggtgg

SEQ ID NO: 31722 - DNA, 28 bp, synthetic construct
  source 1..28: mol_type = other DNA
ggaagaagaaatgcatgtggctggtggg

SEQ ID NO: 31723 - DNA, 28 bp, synthetic construct
  source 1..28: mol_type = other DNA
atgtggctggtgggcttgttatcacagg

SEQ ID NO: 31724 - DNA, 28 bp, synthetic construct
  source 1..28: mol_type = other DNA
aactcctaactgagctccaacacacagg

SEQ ID NO: 31725 - DNA, 28 bp, synthetic construct
  source 1..28: mol_type = other DNA
agtgcctgtgtgttggagctcagttagg

SEQ ID NO: 31726 - DNA, 28 bp, synthetic construct
  source 1..28: mol_type = other DNA
cactaaggtagcagtgcctgtgtgttgg

SEQ ID NO: 31727 - DNA, 28 bp, synthetic construct
  source 1..28: mol_type = other DNA
cgtctttgaaagttaacagacactaagg

SEQ ID NO: 31728 - DNA, 28 bp, synthetic construct
  source 1..28: mol_type = other DNA
atggcactgagatttagcaaaaacgcgg

SEQ ID NO: 31729 - DNA, 28 bp, synthetic construct
  source 1..28: mol_type = other DNA
atctcagtgccatttgcatactacttgg

SEQ ID NO: 31730 - DNA, 28 bp, synthetic construct
  source 1..28: mol_type = other DNA
tcagtgccatttgcatactacttggagg

SEQ ID NO: 31731 - DNA, 28 bp, synthetic construct
  source 1..28: mol_type = other DNA
gtgccatttgcatactacttggaggtgg

SEQ ID NO: 31732 - DNA, 28 bp, synthetic construct
  source 1..28: mol_type = other DNA
tgccatttgcatactacttggaggtggg

SEQ ID NO: 31733 - DNA, 28 bp, synthetic construct
  source 1..28: mol_type = other DNA
gccatttgcatactacttggaggtgggg

SEQ ID NO: 31734 - DNA, 28 bp, synthetic construct
  source 1..28: mol_type = other DNA
gccccacctccaagtagtatgcaaatgg

SEQ ID NO: 31735 - DNA, 28 bp, synthetic construct
  source 1..28: mol_type = other DNA
tttgcatactacttggaggtggggctgg

SEQ ID NO: 31736 - DNA, 28 bp, synthetic construct
  source 1..28: mol_type = other DNA
ttgcatactacttggaggtggggctggg

SEQ ID NO: 31737 - DNA, 28 bp, synthetic construct
  source 1..28: mol_type = other DNA
atactacttggaggtggggctgggaagg

SEQ ID NO: 31738 - DNA, 28 bp, synthetic construct
  source 1..28: mol_type = other DNA
tactacttggaggtggggctgggaaggg

SEQ ID NO: 31739 - DNA, 28 bp, synthetic construct
  source 1..28: mol_type = other DNA
ggctgtgagtgtccatctgtttgcctgg

SEQ ID NO: 31740 - DNA, 28 bp, synthetic construct
  source 1..28: mol_type = other DNA
actaaatgcattccaggcaaacagatgg

SEQ ID NO: 31741 - DNA, 28 bp, synthetic construct
  source 1..28: mol_type = other DNA
ctctattatcaactaaatgcattccagg

SEQ ID NO: 31742 - DNA, 28 bp, synthetic construct
  source 1..28: mol_type = other DNA
gcatttagttgataatagagtcagatgg

SEQ ID NO: 31743 - DNA, 28 bp, synthetic construct
  source 1..28: mol_type = other DNA
catttagttgataatagagtcagatggg

SEQ ID NO: 31744 - DNA, 28 bp, synthetic construct
  source 1..28: mol_type = other DNA
atttagttgataatagagtcagatgggg

SEQ ID NO: 31745 - DNA, 28 bp, synthetic construct
  source 1..28: mol_type = other DNA
tttagttgataatagagtcagatggggg

SEQ ID NO: 31746 - DNA, 28 bp, synthetic construct
  source 1..28: mol_type = other DNA
gttgataatagagtcagatgggggaagg

SEQ ID NO: 31747 - DNA, 28 bp, synthetic construct
  source 1..28: mol_type = other DNA
ttgataatagagtcagatgggggaaggg

SEQ ID NO: 31748 - DNA, 28 bp, synthetic construct
  source 1..28: mol_type = other DNA
gagtcagatgggggaagggaattagagg

SEQ ID NO: 31749 - DNA, 28 bp, synthetic construct
  source 1..28: mol_type = other DNA
gggggaagggaattagaggaagagcagg

SEQ ID NO: 31750 - DNA, 28 bp, synthetic construct
  source 1..28: mol_type = other DNA
ggggaagggaattagaggaagagcaggg

SEQ ID NO: 31751 - DNA, 28 bp, synthetic construct
  source 1..28: mol_type = other DNA
ggaattagaggaagagcagggtatttgg

SEQ ID NO: 31752 - DNA, 28 bp, synthetic construct
  source 1..28: mol_type = other DNA
ggtaacatgcaatctagtaaacttccgg

SEQ ID NO: 31753 - DNA, 28 bp, synthetic construct
  source 1..28: mol_type = other DNA
agtaaacttccggcacaaaaatacctgg

SEQ ID NO: 31754 - DNA, 28 bp, synthetic construct
  source 1..28: mol_type = other DNA
gaaaataagccaggtatttttgtgccgg

SEQ ID NO: 31755 - DNA, 28 bp, synthetic construct
  source 1..28: mol_type = other DNA
ggtaattgaataatgaaaataagccagg

SEQ ID NO: 31756 - DNA, 28 bp, synthetic construct
  source 1..28: mol_type = other DNA
tattttttgattggtatgtattaatggg

SEQ ID NO: 31757 - DNA, 28 bp, synthetic construct
  source 1..28: mol_type = other DNA
ttattttttgattggtatgtattaatgg

SEQ ID NO: 31758 - DNA, 28 bp, synthetic construct
  source 1..28: mol_type = other DNA
taatacataccaatcaaaaaataattgg

SEQ ID NO: 31759 - DNA, 28 bp, synthetic construct
  source 1..28: mol_type = other DNA
aatacataccaatcaaaaaataattggg

SEQ ID NO: 31760 - DNA, 28 bp, synthetic construct
  source 1..28: mol_type = other DNA
atacataccaatcaaaaaataattgggg

SEQ ID NO: 31761 - DNA, 28 bp, synthetic construct
  source 1..28: mol_type = other DNA
tactattccccaattattttttgattgg

SEQ ID NO: 31762 - DNA, 28 bp, synthetic construct
  source 1..28: mol_type = other DNA
tgaaagtaatcaacagtataagagcagg

SEQ ID NO: 31763 - DNA, 28 bp, synthetic construct
  source 1..28: mol_type = other DNA
agtataagagcaggtccatcttcactgg

SEQ ID NO: 31764 - DNA, 28 bp, synthetic construct
  source 1..28: mol_type = other DNA
ccaaaagcttgactgccagtgaagatgg

SEQ ID NO: 31765 - DNA, 28 bp, synthetic construct
  source 1..28: mol_type = other DNA
agcttttggtgtgctgtattgcacctgg

SEQ ID NO: 31766 - DNA, 28 bp, synthetic construct
  source 1..28: mol_type = other DNA
ccaaaatctcatgggttagttaaccagg

SEQ ID NO: 31767 - DNA, 28 bp, synthetic construct
  source 1..28: mol_type = other DNA
ttagaaaattcaaccaaaatctcatggg

SEQ ID NO: 31768 - DNA, 28 bp, synthetic construct
  source 1..28: mol_type = other DNA
cttagaaaattcaaccaaaatctcatgg

SEQ ID NO: 31769 - DNA, 28 bp, synthetic construct
  source 1..28: mol_type = other DNA
tttggttgaattttctaagaagtcacgg

SEQ ID NO: 31770 - DNA, 28 bp, synthetic construct
  source 1..28: mol_type = other DNA
tttctaagaagtcacggtttagcactgg

SEQ ID NO: 31771 - DNA, 28 bp, synthetic construct
  source 1..28: mol_type = other DNA
aagaagtcacggtttagcactggaatgg

SEQ ID NO: 31772 - DNA, 28 bp, synthetic construct
  source 1..28: mol_type = other DNA
gtgtctgtgattgtgtgtgagtgtacgg

SEQ ID NO: 31773 - DNA, 28 bp, synthetic construct
  source 1..28: mol_type = other DNA
aaagtgatcagaggtttctgactagagg

SEQ ID NO: 31774 - DNA, 28 bp, synthetic construct
  source 1..28: mol_type = other DNA
aaacctctgatcactttgtctagcctgg

SEQ ID NO: 31775 - DNA, 28 bp, synthetic construct
  source 1..28: mol_type = other DNA
aacctctgatcactttgtctagcctggg

SEQ ID NO: 31776 - DNA, 28 bp, synthetic construct
  source 1..28: mol_type = other DNA
atcccaggctagacaaagtgatcagagg

SEQ ID NO: 31777 - DNA, 28 bp, synthetic construct
  source 1..28: mol_type = other DNA
gatcactttgtctagcctgggattatgg

SEQ ID NO: 31778 - DNA, 28 bp, synthetic construct
  source 1..28: mol_type = other DNA
ttctttgtctagtttccataatcccagg

SEQ ID NO: 31779 - DNA, 28 bp, synthetic construct
  source 1..28: mol_type = other DNA
tgggattatggaaactagacaaagaagg

SEQ ID NO: 31780 - DNA, 28 bp, synthetic construct
  source 1..28: mol_type = other DNA
agctgtgtatcttacacacatacacagg

SEQ ID NO: 31781 - DNA, 28 bp, synthetic construct
  source 1..28: mol_type = other DNA
tgtgtatcttacacacatacacaggcgg

SEQ ID NO: 31782 - DNA, 28 bp, synthetic construct
  source 1..28: mol_type = other DNA
gcagggcatgtgtgtttgtatgtgtggg

SEQ ID NO: 31783 - DNA, 28 bp, synthetic construct
  source 1..28: mol_type = other DNA
tgcagggcatgtgtgtttgtatgtgtgg

SEQ ID NO: 31784 - DNA, 28 bp, synthetic construct
  source 1..28: mol_type = other DNA
cagcattgaacaatgatcttttgcaggg

SEQ ID NO: 31785 - DNA, 28 bp, synthetic construct
  source 1..28: mol_type = other DNA
tcagcattgaacaatgatcttttgcagg

SEQ ID NO: 31786 - DNA, 28 bp, synthetic construct
  source 1..28: mol_type = other DNA
tgcaaaagatcattgttcaatgctgagg

SEQ ID NO: 31787 - DNA, 28 bp, synthetic construct
  source 1..28: mol_type = other DNA
gttcaccgcagtctgataaatgctgtgg

SEQ ID NO: 31788 - DNA, 28 bp, synthetic construct
  source 1..28: mol_type = other DNA
accgcagtctgataaatgctgtggctgg

SEQ ID NO: 31789 - DNA, 28 bp, synthetic construct
  source 1..28: mol_type = other DNA
ccgcagtctgataaatgctgtggctggg

SEQ ID NO: 31790 - DNA, 28 bp, synthetic construct
  source 1..28: mol_type = other DNA
gtgtccaaaaacgttgagccatctgtgg

SEQ ID NO: 31791 - DNA, 28 bp, synthetic construct
  source 1..28: mol_type = other DNA
gtctccacagatggctcaacgtttttgg

SEQ ID NO: 31792 - DNA, 28 bp, synthetic construct
  source 1..28: mol_type = other DNA
cagagtgggctctggtctccacagatgg

SEQ ID NO: 31793 - DNA, 28 bp, synthetic construct
  source 1..28: mol_type = other DNA
catctgtggagaccagagcccactctgg

SEQ ID NO: 31794 - DNA, 28 bp, synthetic construct
  source 1..28: mol_type = other DNA
ggagaccagagcccactctggccccagg

SEQ ID NO: 31795 - DNA, 28 bp, synthetic construct
  source 1..28: mol_type = other DNA
gagaccagagcccactctggccccaggg

SEQ ID NO: 31796 - DNA, 28 bp, synthetic construct
  source 1..28: mol_type = other DNA
ctcaccctggggccagagtgggctctgg

SEQ ID NO: 31797 - DNA, 28 bp, synthetic construct
  source 1..28: mol_type = other DNA
cagagcccactctggccccagggtgagg

SEQ ID NO: 31798 - DNA, 28 bp, synthetic construct
  source 1..28: mol_type = other DNA
agggacctcaccctggggccagagtggg

SEQ ID NO: 31799 - DNA, 28 bp, synthetic construct
  source 1..28: mol_type = other DNA
tagggacctcaccctggggccagagtgg

SEQ ID NO: 31800 - DNA, 28 bp, synthetic construct
  source 1..28: mol_type = other DNA
ggccccagggtgaggtccctatgacagg

SEQ ID NO: 31801 - DNA, 28 bp, synthetic construct
  source 1..28: mol_type = other DNA
cacctgtcatagggacctcaccctgggg

SEQ ID NO: 31802 - DNA, 28 bp, synthetic construct
  source 1..28: mol_type = other DNA
cccagggtgaggtccctatgacaggtgg

SEQ ID NO: 31803 - DNA, 28 bp, synthetic construct
  source 1..28: mol_type = other DNA
ccagggtgaggtccctatgacaggtggg

SEQ ID NO: 31804 - DNA, 28 bp, synthetic construct
  source 1..28: mol_type = other DNA
tgcggaacagcgcccacctgtcataggg

SEQ ID NO: 31805 - DNA, 28 bp, synthetic construct
  source 1..28: mol_type = other DNA
ctgcggaacagcgcccacctgtcatagg

SEQ ID NO: 31806 - DNA, 28 bp, synthetic construct
  source 1..28: mol_type = other DNA
gtgggcgctgttccgcagccagtgcagg

SEQ ID NO: 31807 - DNA, 28 bp, synthetic construct
  source 1..28: mol_type = other DNA
gttccgcagccagtgcaggccctgttgg

SEQ ID NO: 31808 - DNA, 28 bp, synthetic construct
  source 1..28: mol_type = other DNA
ttccgcagccagtgcaggccctgttggg

SEQ ID NO: 31809 - DNA, 28 bp, synthetic construct
  source 1..28: mol_type = other DNA
ctcccaacagggcctgcactggctgcgg

SEQ ID NO: 31810 - DNA, 28 bp, synthetic construct
  source 1..28: mol_type = other DNA
ccagtgcaggccctgttgggagtactgg

SEQ ID NO: 31811 - DNA, 28 bp, synthetic construct
  source 1..28: mol_type = other DNA
caggccctgttgggagtactggaccagg

SEQ ID NO: 31812 - DNA, 28 bp, synthetic construct
  source 1..28: mol_type = other DNA
agcacctggtccagtactcccaacaggg

SEQ ID NO: 31813 - DNA, 28 bp, synthetic construct
  source 1..28: mol_type = other DNA
gagcacctggtccagtactcccaacagg

SEQ ID NO: 31814 - DNA, 28 bp, synthetic construct
  source 1..28: mol_type = other DNA
gaccaggtgctccatgctgctgtgcagg

SEQ ID NO: 31815 - DNA, 28 bp, synthetic construct
  source 1..28: mol_type = other DNA
accaggtgctccatgctgctgtgcaggg

SEQ ID NO: 31816 - DNA, 28 bp, synthetic construct
  source 1..28: mol_type = other DNA
accctgcacagcagcatggagcacctgg

SEQ ID NO: 31817 - DNA, 28 bp, synthetic construct
  source 1..28: mol_type = other DNA
gctccatgctgctgtgcagggtgaccgg

SEQ ID NO: 31818 - DNA, 28 bp, synthetic construct
  source 1..28: mol_type = other DNA
gggccggtcaccctgcacagcagcatgg

SEQ ID NO: 31819 - DNA, 28 bp, synthetic construct
  source 1..28: mol_type = other DNA
ggtgaccggccccatgagcagatccagg

SEQ ID NO: 31820 - DNA, 28 bp, synthetic construct
  source 1..28: mol_type = other DNA
aacgacctggatctgctcatggggccgg

SEQ ID NO: 31821 - DNA, 28 bp, synthetic construct
  source 1..28: mol_type = other DNA
cttcaacgacctggatctgctcatgggg

SEQ ID NO: 31822 - DNA, 28 bp, synthetic construct
  source 1..28: mol_type = other DNA
tcttcaacgacctggatctgctcatggg

SEQ ID NO: 31823 - DNA, 28 bp, synthetic construct
  source 1..28: mol_type = other DNA
ttcttcaacgacctggatctgctcatgg

SEQ ID NO: 31824 - DNA, 28 bp, synthetic construct
  source 1..28: mol_type = other DNA
cagatccaggtcgttgaagaattctagg

SEQ ID NO: 31825 - DNA, 28 bp, synthetic construct
  source 1..28: mol_type = other DNA
agatccaggtcgttgaagaattctaggg

SEQ ID NO: 31826 - DNA, 28 bp, synthetic construct
  source 1..28: mol_type = other DNA
gatccaggtcgttgaagaattctagggg

SEQ ID NO: 31827 - DNA, 28 bp, synthetic construct
  source 1..28: mol_type = other DNA
atccaggtcgttgaagaattctaggggg

SEQ ID NO: 31828 - DNA, 28 bp, synthetic construct
  source 1..28: mol_type = other DNA
gtccccctagaattcttcaacgacctgg

SEQ ID NO: 31829 - DNA, 28 bp, synthetic construct
  source 1..28: mol_type = other DNA
agttgttaagaatgccacacatgctagg

SEQ ID NO: 31830 - DNA, 28 bp, synthetic construct
  source 1..28: mol_type = other DNA
ctcaggatagcacacctagcatgtgtgg

SEQ ID NO: 31831 - DNA, 28 bp, synthetic construct
  source 1..28: mol_type = other DNA
tgtgctatcctgagcaactgatgtaagg

SEQ ID NO: 31832 - DNA, 28 bp, synthetic construct
  source 1..28: mol_type = other DNA
gaatttttccttacatcagttgctcagg

SEQ ID NO: 31833 - DNA, 28 bp, synthetic construct
  source 1..28: mol_type = other DNA
ctgatgtaaggaaaaattccattcatgg

SEQ ID NO: 31834 - DNA, 28 bp, synthetic construct
  source 1..28: mol_type = other DNA
ccttgatttatatagagaccatgaatgg

SEQ ID NO: 31835 - DNA, 28 bp, synthetic construct
  source 1..28: mol_type = other DNA
aactgtgtgagtatcccagctactcagg

SEQ ID NO: 31836 - DNA, 28 bp, synthetic construct
  source 1..28: mol_type = other DNA
tgtgtgagtatcccagctactcaggagg

SEQ ID NO: 31837 - DNA, 28 bp, synthetic construct
  source 1..28: mol_type = other DNA
agtatcccagctactcaggaggccgagg

SEQ ID NO: 31838 - DNA, 28 bp, synthetic construct
  source 1..28: mol_type = other DNA
ttctgcctcggcctcctgagtagctggg

SEQ ID NO: 31839 - DNA, 28 bp, synthetic construct
  source 1..28: mol_type = other DNA
cttctgcctcggcctcctgagtagctgg

SEQ ID NO: 31840 - DNA, 28 bp, synthetic construct
  source 1..28: mol_type = other DNA
ccgaggcagaagaatcgcttgaacccgg

SEQ ID NO: 31841 - DNA, 28 bp, synthetic construct
  source 1..28: mol_type = other DNA
cgaggcagaagaatcgcttgaacccggg

SEQ ID NO: 31842 - DNA, 28 bp, synthetic construct
  source 1..28: mol_type = other DNA
ggcagaagaatcgcttgaacccgggagg

SEQ ID NO: 31843 - DNA, 28 bp, synthetic construct
  source 1..28: mol_type = other DNA
agaagaatcgcttgaacccgggaggcgg

SEQ ID NO: 31844 - DNA, 28 bp, synthetic construct
  source 1..28: mol_type = other DNA
cttgaacccgggaggcggaagcccctgg

SEQ ID NO: 31845 - DNA, 28 bp, synthetic construct
  source 1..28: mol_type = other DNA
ggggaaccaggggcttccgcctcccggg

SEQ ID NO: 31846 - DNA, 28 bp, synthetic construct
  source 1..28: mol_type = other DNA
cggggaaccaggggcttccgcctcccgg

SEQ ID NO: 31847 - DNA, 28 bp, synthetic construct
  source 1..28: mol_type = other DNA
ggaggcggaagcccctggttccccgtgg

SEQ ID NO: 31848 - DNA, 28 bp, synthetic construct
  source 1..28: mol_type = other DNA
gaggcggaagcccctggttccccgtggg

SEQ ID NO: 31849 - DNA, 28 bp, synthetic construct
  source 1..28: mol_type = other DNA
aggcggaagcccctggttccccgtgggg

SEQ ID NO: 31850 - DNA, 28 bp, synthetic construct
  source 1..28: mol_type = other DNA
gagcgcacaccccacggggaaccagggg

SEQ ID NO: 31851 - DNA, 28 bp, synthetic construct
  source 1..28: mol_type = other DNA
tgagcgcacaccccacggggaaccaggg

SEQ ID NO: 31852 - DNA, 28 bp, synthetic construct
  source 1..28: mol_type = other DNA
gtgagcgcacaccccacggggaaccagg

SEQ ID NO: 31853 - DNA, 28 bp, synthetic construct
  source 1..28: mol_type = other DNA
ttccccgtggggtgtgcgctcacctcgg

SEQ ID NO: 31854 - DNA, 28 bp, synthetic construct
  source 1..28: mol_type = other DNA
aaccgaggtgagcgcacaccccacgggg

SEQ ID NO: 31855 - DNA, 28 bp, synthetic construct
  source 1..28: mol_type = other DNA
aaaccgaggtgagcgcacaccccacggg

SEQ ID NO: 31856 - DNA, 28 bp, synthetic construct
  source 1..28: mol_type = other DNA
aaaaccgaggtgagcgcacaccccacgg

SEQ ID NO: 31857 - DNA, 28 bp, synthetic construct
  source 1..28: mol_type = other DNA
ggtgtgcgctcacctcggttttccttgg

SEQ ID NO: 31858 - DNA, 28 bp, synthetic construct
  source 1..28: mol_type = other DNA
gcgctcacctcggttttccttggccagg

SEQ ID NO: 31859 - DNA, 28 bp, synthetic construct
  source 1..28: mol_type = other DNA
ccgacaacctggccaaggaaaaccgagg

SEQ ID NO: 31860 - DNA, 28 bp, synthetic construct
  source 1..28: mol_type = other DNA
tgggagatggccgacaacctggccaagg

SEQ ID NO: 31861 - DNA, 28 bp, synthetic construct
  source 1..28: mol_type = other DNA
gactactgggagatggccgacaacctgg

SEQ ID NO: 31862 - DNA, 28 bp, synthetic construct
  source 1..28: mol_type = other DNA
ctgcacagctacgactactgggagatgg

SEQ ID NO: 31863 - DNA, 28 bp, synthetic construct
  source 1..28: mol_type = other DNA
catctcccagtagtcgtagctgtgcagg

SEQ ID NO: 31864 - DNA, 28 bp, synthetic construct
  source 1..28: mol_type = other DNA
agcatcctgcacagctacgactactggg

SEQ ID NO: 31865 - DNA, 28 bp, synthetic construct
  source 1..28: mol_type = other DNA
cagcatcctgcacagctacgactactgg

SEQ ID NO: 31866 - DNA, 28 bp, synthetic construct
  source 1..28: mol_type = other DNA
tagtcgtagctgtgcaggatgctgttgg

SEQ ID NO: 31867 - DNA, 28 bp, synthetic construct
  source 1..28: mol_type = other DNA
caggatgctgttggtgatgctgacgtgg

SEQ ID NO: 31868 - DNA, 28 bp, synthetic construct
  source 1..28: mol_type = other DNA
atgctgttggtgatgctgacgtggttgg

SEQ ID NO: 31869 - DNA, 28 bp, synthetic construct
  source 1..28: mol_type = other DNA
gatgctgacgtggttggccgccatctgg

SEQ ID NO: 31870 - DNA, 28 bp, synthetic construct
  source 1..28: mol_type = other DNA
gctgacgtggttggccgccatctggtgg

SEQ ID NO: 31871 - DNA, 28 bp, synthetic construct
  source 1..28: mol_type = other DNA
tggccgccatctggtggatgcgctgtgg

SEQ ID NO: 31872 - DNA, 28 bp, synthetic construct
  source 1..28: mol_type = other DNA
ggccgccatctggtggatgcgctgtggg

SEQ ID NO: 31873 - DNA, 28 bp, synthetic construct
  source 1..28: mol_type = other DNA
atcccacagcgcatccaccagatggcgg

SEQ ID NO: 31874 - DNA, 28 bp, synthetic construct
  source 1..28: mol_type = other DNA
agcatcccacagcgcatccaccagatgg

SEQ ID NO: 31875 - DNA, 28 bp, synthetic construct
  source 1..28: mol_type = other DNA
tggatgcgctgtgggatgctgacgatgg

SEQ ID NO: 31876 - DNA, 28 bp, synthetic construct
  source 1..28: mol_type = other DNA
gctgtgggatgctgacgatggtcgacgg

SEQ ID NO: 31877 - DNA, 28 bp, synthetic construct
  source 1..28: mol_type = other DNA
ctgtgggatgctgacgatggtcgacggg

SEQ ID NO: 31878 - DNA, 28 bp, synthetic construct
  source 1..28: mol_type = other DNA
tgtgggatgctgacgatggtcgacgggg

SEQ ID NO: 31879 - DNA, 28 bp, synthetic construct
  source 1..28: mol_type = other DNA
gatgctgacgatggtcgacggggacagg

SEQ ID NO: 31880 - DNA, 28 bp, synthetic construct
  source 1..28: mol_type = other DNA
atgctgacgatggtcgacggggacaggg

SEQ ID NO: 31881 - DNA, 28 bp, synthetic construct
  source 1..28: mol_type = other DNA
acgatggtcgacggggacagggcgctgg

SEQ ID NO: 31882 - DNA, 28 bp, synthetic construct
  source 1..28: mol_type = other DNA
gtcgacggggacagggcgctggcgttgg

SEQ ID NO: 31883 - DNA, 28 bp, synthetic construct
  source 1..28: mol_type = other DNA
cggggacagggcgctggcgttggagagg

SEQ ID NO: 31884 - DNA, 28 bp, synthetic construct
  source 1..28: mol_type = other DNA
ttggagaggctgccctgagaccccacgg

SEQ ID NO: 31885 - DNA, 28 bp, synthetic construct
  source 1..28: mol_type = other DNA
aggctgccctgagaccccacggagctgg

SEQ ID NO: 31886 - DNA, 28 bp, synthetic construct
  source 1..28: mol_type = other DNA
ctgccctgagaccccacggagctggcgg

SEQ ID NO: 31887 - DNA, 28 bp, synthetic construct
  source 1..28: mol_type = other DNA
tgccctgagaccccacggagctggcggg

SEQ ID NO: 31888 - DNA, 28 bp, synthetic construct
  source 1..28: mol_type = other DNA
ctcccgccagctccgtggggtctcaggg

SEQ ID NO: 31889 - DNA, 28 bp, synthetic construct
  source 1..28: mol_type = other DNA
tctcccgccagctccgtggggtctcagg

SEQ ID NO: 31890 - DNA, 28 bp, synthetic construct
  source 1..28: mol_type = other DNA
tgagaccccacggagctggcgggagagg

SEQ ID NO: 31891 - DNA, 28 bp, synthetic construct
  source 1..28: mol_type = other DNA
gagaccccacggagctggcgggagaggg

SEQ ID NO: 31892 - DNA, 28 bp, synthetic construct
  source 1..28: mol_type = other DNA
agaccccacggagctggcgggagagggg

SEQ ID NO: 31893 - DNA, 28 bp, synthetic construct
  source 1..28: mol_type = other DNA
caacccctctcccgccagctccgtgggg

SEQ ID NO: 31894 - DNA, 28 bp, synthetic construct
  source 1..28: mol_type = other DNA
cccacggagctggcgggagaggggttgg

SEQ ID NO: 31895 - DNA, 28 bp, synthetic construct
  source 1..28: mol_type = other DNA
cccaacccctctcccgccagctccgtgg

SEQ ID NO: 31896 - DNA, 28 bp, synthetic construct
  source 1..28: mol_type = other DNA
ctggcgggagaggggttgggagacatgg

SEQ ID NO: 31897 - DNA, 28 bp, synthetic construct
  source 1..28: mol_type = other DNA
tggcgggagaggggttgggagacatggg

SEQ ID NO: 31898 - DNA, 28 bp, synthetic construct
  source 1..28: mol_type = other DNA
ggcgggagaggggttgggagacatgggg

SEQ ID NO: 31899 - DNA, 28 bp, synthetic construct
  source 1..28: mol_type = other DNA
gcgggagaggggttgggagacatggggg

SEQ ID NO: 31900 - DNA, 28 bp, synthetic construct
  source 1..28: mol_type = other DNA
gagaggggttgggagacatgggggatgg

SEQ ID NO: 31901 - DNA, 28 bp, synthetic construct
  source 1..28: mol_type = other DNA
agaggggttgggagacatgggggatggg

SEQ ID NO: 31902 - DNA, 28 bp, synthetic construct
  source 1..28: mol_type = other DNA
gaggggttgggagacatgggggatgggg

SEQ ID NO: 31903 - DNA, 28 bp, synthetic construct
  source 1..28: mol_type = other DNA
atgggggatggggttccagtgctcctgg

SEQ ID NO: 31904 - DNA, 28 bp, synthetic construct
  source 1..28: mol_type = other DNA
gggatggggttccagtgctcctggaagg

SEQ ID NO: 31905 - DNA, 28 bp, synthetic construct
  source 1..28: mol_type = other DNA
ggatggggttccagtgctcctggaaggg

SEQ ID NO: 31906 - DNA, 28 bp, synthetic construct
  source 1..28: mol_type = other DNA
gatggggttccagtgctcctggaagggg

SEQ ID NO: 31907 - DNA, 28 bp, synthetic construct
  source 1..28: mol_type = other DNA
ggttccagtgctcctggaaggggagagg

SEQ ID NO: 31908 - DNA, 28 bp, synthetic construct
  source 1..28: mol_type = other DNA
tctacctctccccttccaggagcactgg

SEQ ID NO: 31909 - DNA, 28 bp, synthetic construct
  source 1..28: mol_type = other DNA
ctggtttttctacctctccccttccagg

SEQ ID NO: 31910 - DNA, 28 bp, synthetic construct
  source 1..28: mol_type = other DNA
aaggggagaggtagaaaaaccagagtgg

SEQ ID NO: 31911 - DNA, 28 bp, synthetic construct
  source 1..28: mol_type = other DNA
gagaggtagaaaaaccagagtggcgagg

SEQ ID NO: 31912 - DNA, 28 bp, synthetic construct
  source 1..28: mol_type = other DNA
ggtagaaaaaccagagtggcgaggtcgg

SEQ ID NO: 31913 - DNA, 28 bp, synthetic construct
  source 1..28: mol_type = other DNA
gtagaaaaaccagagtggcgaggtcggg

SEQ ID NO: 31914 - DNA, 28 bp, synthetic construct
  source 1..28: mol_type = other DNA
tcgcttgctcccgacctcgccactctgg

SEQ ID NO: 31915 - DNA, 28 bp, synthetic construct
  source 1..28: mol_type = other DNA
agagtggcgaggtcgggagcaagcgagg

SEQ ID NO: 31916 - DNA, 28 bp, synthetic construct
  source 1..28: mol_type = other DNA
tggcgaggtcgggagcaagcgaggcagg

SEQ ID NO: 31917 - DNA, 28 bp, synthetic construct
  source 1..28: mol_type = other DNA
ggcgaggtcgggagcaagcgaggcaggg

SEQ ID NO: 31918 - DNA, 28 bp, synthetic construct
  source 1..28: mol_type = other DNA
gagcaagcgaggcagggcagccccttgg

SEQ ID NO: 31919 - DNA, 28 bp, synthetic construct
  source 1..28: mol_type = other DNA
agcaagcgaggcagggcagccccttggg

SEQ ID NO: 31920 - DNA, 28 bp, synthetic construct
  source 1..28: mol_type = other DNA
gcaagcgaggcagggcagccccttgggg

SEQ ID NO: 31921 - DNA, 28 bp, synthetic construct
  source 1..28: mol_type = other DNA
tgcgctttgctttctgttccccaagggg

SEQ ID NO: 31922 - DNA, 28 bp, synthetic construct
  source 1..28: mol_type = other DNA
ctgcgctttgctttctgttccccaaggg

SEQ ID NO: 31923 - DNA, 28 bp, synthetic construct
  source 1..28: mol_type = other DNA
actgcgctttgctttctgttccccaagg

SEQ ID NO: 31924 - DNA, 28 bp, synthetic construct
  source 1..28: mol_type = other DNA
ttggggaacagaaagcaaagcgcagtgg

SEQ ID NO: 31925 - DNA, 28 bp, synthetic construct
  source 1..28: mol_type = other DNA
cagtggcccagcaccatgcattgtctgg

SEQ ID NO: 31926 - DNA, 28 bp, synthetic construct
  source 1..28: mol_type = other DNA
cgtaagccagacaatgcatggtgctggg

SEQ ID NO: 31927 - DNA, 28 bp, synthetic construct
  source 1..28: mol_type = other DNA
ccgtaagccagacaatgcatggtgctgg

SEQ ID NO: 31928 - DNA, 28 bp, synthetic construct
  source 1..28: mol_type = other DNA
tcaatgccgtaagccagacaatgcatgg

SEQ ID NO: 31929 - DNA, 28 bp, synthetic construct
  source 1..28: mol_type = other DNA
attgtctggcttacggcattgactttgg

SEQ ID NO: 31930 - DNA, 28 bp, synthetic construct
  source 1..28: mol_type = other DNA
ttggaaaagcgaacttactttccactgg

SEQ ID NO: 31931 - DNA, 28 bp, synthetic construct
  source 1..28: mol_type = other DNA
gaacttactttccactggccccccacgg

SEQ ID NO: 31932 - DNA, 28 bp, synthetic construct
  source 1..28: mol_type = other DNA
actttccactggccccccacggagatgg

SEQ ID NO: 31933 - DNA, 28 bp, synthetic construct
  source 1..28: mol_type = other DNA
ctttccactggccccccacggagatggg

SEQ ID NO: 31934 - DNA, 28 bp, synthetic construct
  source 1..28: mol_type = other DNA
tttccactggccccccacggagatgggg

SEQ ID NO: 31935 - DNA, 28 bp, synthetic construct
  source 1..28: mol_type = other DNA
aagccccatctccgtggggggccagtgg

SEQ ID NO: 31936 - DNA, 28 bp, synthetic construct
  source 1..28: mol_type = other DNA
actggccccccacggagatggggcttgg

SEQ ID NO: 31937 - DNA, 28 bp, synthetic construct
  source 1..28: mol_type = other DNA
ctggccccccacggagatggggcttggg

SEQ ID NO: 31938 - DNA, 28 bp, synthetic construct
  source 1..28: mol_type = other DNA
gccccccacggagatggggcttgggcgg

SEQ ID NO: 31939 - DNA, 28 bp, synthetic construct
  source 1..28: mol_type = other DNA
gccgcccaagccccatctccgtgggggg

SEQ ID NO: 31940 - DNA, 28 bp, synthetic construct
  source 1..28: mol_type = other DNA
agccgcccaagccccatctccgtggggg

SEQ ID NO: 31941 - DNA, 28 bp, synthetic construct
  source 1..28: mol_type = other DNA
aagccgcccaagccccatctccgtgggg

SEQ ID NO: 31942 - DNA, 28 bp, synthetic construct
  source 1..28: mol_type = other DNA
aaagccgcccaagccccatctccgtggg

SEQ ID NO: 31943 - DNA, 28 bp, synthetic construct
  source 1..28: mol_type = other DNA
taaagccgcccaagccccatctccgtgg

SEQ ID NO: 31944 - DNA, 28 bp, synthetic construct
  source 1..28: mol_type = other DNA
actgacagtgagtgccatctgcgtgagg

SEQ ID NO: 31945 - DNA, 28 bp, synthetic construct
  source 1..28: mol_type = other DNA
gagtgccatctgcgtgaggtgaaacagg

SEQ ID NO: 31946 - DNA, 28 bp, synthetic construct
  source 1..28: mol_type = other DNA
tgtcacctgtttcacctcacgcagatgg

SEQ ID NO: 31947 - DNA, 28 bp, synthetic construct
  source 1..28: mol_type = other DNA
aaacaggtgacatgaacgtgttttcagg

SEQ ID NO: 31948 - DNA, 28 bp, synthetic construct
  source 1..28: mol_type = other DNA
ttcaggtgactgcagagagaagcaaagg

SEQ ID NO: 31949 - DNA, 28 bp, synthetic construct
  source 1..28: mol_type = other DNA
agagagaagcaaaggcagacactgcagg

SEQ ID NO: 31950 - DNA, 28 bp, synthetic construct
  source 1..28: mol_type = other DNA
agcaaaggcagacactgcaggaaaaagg

SEQ ID NO: 31951 - DNA, 28 bp, synthetic construct
  source 1..28: mol_type = other DNA
taatgcaggtcacctctggtccccaagg

SEQ ID NO: 31952 - DNA, 28 bp, synthetic construct
  source 1..28: mol_type = other DNA
ctttggggttaatgcaggtcacctctgg

SEQ ID NO: 31953 - DNA, 28 bp, synthetic construct
  source 1..28: mol_type = other DNA
gtgacctgcattaaccccaaagcaatgg

SEQ ID NO: 31954 - DNA, 28 bp, synthetic construct
  source 1..28: mol_type = other DNA
gactccattgctttggggttaatgcagg

SEQ ID NO: 31955 - DNA, 28 bp, synthetic construct
  source 1..28: mol_type = other DNA
taaccccaaagcaatggagtctaccagg

SEQ ID NO: 31956 - DNA, 28 bp, synthetic construct
  source 1..28: mol_type = other DNA
gcacctggtagactccattgctttgggg

SEQ ID NO: 31957 - DNA, 28 bp, synthetic construct
  source 1..28: mol_type = other DNA
agcacctggtagactccattgctttggg

SEQ ID NO: 31958 - DNA, 28 bp, synthetic construct
  source 1..28: mol_type = other DNA
aagcacctggtagactccattgctttgg

SEQ ID NO: 31959 - DNA, 28 bp, synthetic construct
  source 1..28: mol_type = other DNA
ctaccaggtgcttcacaaatttgacagg

SEQ ID NO: 31960 - DNA, 28 bp, synthetic construct
  source 1..28: mol_type = other DNA
taccaggtgcttcacaaatttgacaggg

SEQ ID NO: 31961 - DNA, 28 bp, synthetic construct
  source 1..28: mol_type = other DNA
ctccctgtcaaatttgtgaagcacctgg

SEQ ID NO: 31962 - DNA, 28 bp, synthetic construct
  source 1..28: mol_type = other DNA
tttgacagggagacaagtgaaattaagg

SEQ ID NO: 31963 - DNA, 28 bp, synthetic construct
  source 1..28: mol_type = other DNA
tcaaaagcactaatcgactatttcaagg

SEQ ID NO: 31964 - DNA, 28 bp, synthetic construct
  source 1..28: mol_type = other DNA
tagtgcttttgaatactttacagcgtgg

SEQ ID NO: 31965 - DNA, 28 bp, synthetic construct
  source 1..28: mol_type = other DNA
tactggcggatgtttcgactcaaaaggg

SEQ ID NO: 31966 - DNA, 28 bp, synthetic construct
  source 1..28: mol_type = other DNA
gtactggcggatgtttcgactcaaaagg

SEQ ID NO: 31967 - DNA, 28 bp, synthetic construct
  source 1..28: mol_type = other DNA
tttgagtcgaaacatccgccagtacagg

SEQ ID NO: 31968 - DNA, 28 bp, synthetic construct
  source 1..28: mol_type = other DNA
gagtcgaaacatccgccagtacaggagg

SEQ ID NO: 31969 - DNA, 28 bp, synthetic construct
  source 1..28: mol_type = other DNA
agtcgaaacatccgccagtacaggaggg

SEQ ID NO: 31970 - DNA, 28 bp, synthetic construct
  source 1..28: mol_type = other DNA
aaacatccgccagtacaggagggccagg

SEQ ID NO: 31971 - DNA, 28 bp, synthetic construct
  source 1..28: mol_type = other DNA
ccgatgcctggccctcctgtactggcgg

SEQ ID NO: 31972 - DNA, 28 bp, synthetic construct
  source 1..28: mol_type = other DNA
ttaccgatgcctggccctcctgtactgg

SEQ ID NO: 31973 - DNA, 28 bp, synthetic construct
  source 1..28: mol_type = other DNA
aggagggccaggcatcggtaactgcagg

SEQ ID NO: 31974 - DNA, 28 bp, synthetic construct
  source 1..28: mol_type = other DNA
cttttcgcctgcagttaccgatgcctgg

SEQ ID NO: 31975 - DNA, 28 bp, synthetic construct
  source 1..28: mol_type = other DNA
ggtaactgcaggcgaaaagagaaacagg

SEQ ID NO: 31976 - DNA, 28 bp, synthetic construct
  source 1..28: mol_type = other DNA
gcgaaaagagaaacaggcccagaagcgg

SEQ ID NO: 31977 - DNA, 28 bp, synthetic construct
  source 1..28: mol_type = other DNA
gcgcacgacgcactcagccgcttctggg

SEQ ID NO: 31978 - DNA, 28 bp, synthetic construct
  source 1..28: mol_type = other DNA
tgcgcacgacgcactcagccgcttctgg

SEQ ID NO: 31979 - DNA, 28 bp, synthetic construct
  source 1..28: mol_type = other DNA
cttaaacatttttgttgttgttctaagg

SEQ ID NO: 31980 - DNA, 28 bp, synthetic construct
  source 1..28: mol_type = other DNA
caataacaataccttgtttctacatagg

SEQ ID NO: 31981 - DNA, 28 bp, synthetic construct
  source 1..28: mol_type = other DNA
tggggctttgtatgttagaagacattgg

SEQ ID NO: 31982 - DNA, 28 bp, synthetic construct
  source 1..28: mol_type = other DNA
ggggctttgtatgttagaagacattggg

SEQ ID NO: 31983 - DNA, 28 bp, synthetic construct
  source 1..28: mol_type = other DNA
ggcaaacactatgcctttcagcacctgg

SEQ ID NO: 31984 - DNA, 28 bp, synthetic construct
  source 1..28: mol_type = other DNA
catcattggcaaaccaggtgctgaaagg

SEQ ID NO: 31985 - DNA, 28 bp, synthetic construct
  source 1..28: mol_type = other DNA
ctttcagcacctggtttgccaatgatgg

SEQ ID NO: 31986 - DNA, 28 bp, synthetic construct
  source 1..28: mol_type = other DNA
cctggtttgccaatgatggcatgcgagg

SEQ ID NO: 31987 - DNA, 28 bp, synthetic construct
  source 1..28: mol_type = other DNA
gtttgccaatgatggcatgcgaggctgg

SEQ ID NO: 31988 - DNA, 28 bp, synthetic construct
  source 1..28: mol_type = other DNA
tttgccaatgatggcatgcgaggctggg

SEQ ID NO: 31989 - DNA, 28 bp, synthetic construct
  source 1..28: mol_type = other DNA
ttgccaatgatggcatgcgaggctgggg

SEQ ID NO: 31990 - DNA, 28 bp, synthetic construct
  source 1..28: mol_type = other DNA
cagccccagcctcgcatgccatcattgg

SEQ ID NO: 31991 - DNA, 28 bp, synthetic construct
  source 1..28: mol_type = other DNA
gcgaggctggggctgctattctaagcgg

SEQ ID NO: 31992 - DNA, 28 bp, synthetic construct
  source 1..28: mol_type = other DNA
ctggggctgctattctaagcggagatgg

SEQ ID NO: 31993 - DNA, 28 bp, synthetic construct
  source 1..28: mol_type = other DNA
tggggctgctattctaagcggagatggg

SEQ ID NO: 31994 - DNA, 28 bp, synthetic construct
  source 1..28: mol_type = other DNA
agaagacaaacaactggctgcattatgg

SEQ ID NO: 31995 - DNA, 28 bp, synthetic construct
  source 1..28: mol_type = other DNA
ataatgcagccagttgtttgtcttctgg

SEQ ID NO: 31996 - DNA, 28 bp, synthetic construct
  source 1..28: mol_type = other DNA
gcagccagttgtttgtcttctggtgtgg

SEQ ID NO: 31997 - DNA, 28 bp, synthetic construct
  source 1..28: mol_type = other DNA
aatgccacaccagaagacaaacaactgg

SEQ ID NO: 31998 - DNA, 28 bp, synthetic construct
  source 1..28: mol_type = other DNA
agttgtttgtcttctggtgtggcattgg

SEQ ID NO: 31999 - DNA, 28 bp, synthetic construct
  source 1..28: mol_type = other DNA
gttgtttgtcttctggtgtggcattggg

SEQ ID NO: 32000 - DNA, 28 bp, synthetic construct
  source 1..28: mol_type = other DNA
ttgtttgtcttctggtgtggcattgggg

SEQ ID NO: 32001 - DNA, 28 bp, synthetic construct
  source 1..28: mol_type = other DNA
ttctggtgtggcattggggcctgagtgg

SEQ ID NO: 32002 - DNA, 28 bp, synthetic construct
  source 1..28: mol_type = other DNA
tctggtgtggcattggggcctgagtggg

SEQ ID NO: 32003 - DNA, 28 bp, synthetic construct
  source 1..28: mol_type = other DNA
atgctatgagactaaaaacccactcagg

SEQ ID NO: 32004 - DNA, 28 bp, synthetic construct
  source 1..28: mol_type = other DNA
gtctcatagcataccttagaaaaagcgg

SEQ ID NO: 32005 - DNA, 28 bp, synthetic construct
  source 1..28: mol_type = other DNA
tctcatagcataccttagaaaaagcggg

SEQ ID NO: 32006 - DNA, 28 bp, synthetic construct
  source 1..28: mol_type = other DNA
ctcatagcataccttagaaaaagcgggg

SEQ ID NO: 32007 - DNA, 28 bp, synthetic construct
  source 1..28: mol_type = other DNA
atagcataccttagaaaaagcggggagg

SEQ ID NO: 32008 - DNA, 28 bp, synthetic construct
  source 1..28: mol_type = other DNA
gcataccttagaaaaagcggggaggagg

SEQ ID NO: 32009 - DNA, 28 bp, synthetic construct
  source 1..28: mol_type = other DNA
ctattcctcctccccgctttttctaagg

SEQ ID NO: 32010 - DNA, 28 bp, synthetic construct
  source 1..28: mol_type = other DNA
ttttttattaacagaacttctatgatgg

SEQ ID NO: 32011 - DNA, 28 bp, synthetic construct
  source 1..28: mol_type = other DNA
ttttggggggatgaacactggttcctgg

SEQ ID NO: 32012 - DNA, 28 bp, synthetic construct
  source 1..28: mol_type = other DNA
tggggggatgaacactggttcctggtgg

SEQ ID NO: 32013 - DNA, 28 bp, synthetic construct
  source 1..28: mol_type = other DNA
ggggggatgaacactggttcctggtggg

SEQ ID NO: 32014 - DNA, 28 bp, synthetic construct
  source 1..28: mol_type = other DNA
gggggatgaacactggttcctggtgggg

SEQ ID NO: 32015 - DNA, 28 bp, synthetic construct
  source 1..28: mol_type = other DNA
ggggatgaacactggttcctggtggggg

SEQ ID NO: 32016 - DNA, 28 bp, synthetic construct
  source 1..28: mol_type = other DNA
atgaacactggttcctggtgggggatgg

SEQ ID NO: 32017 - DNA, 28 bp, synthetic construct
  source 1..28: mol_type = other DNA
actggttcctggtgggggatggtgcagg

SEQ ID NO: 32018 - DNA, 28 bp, synthetic construct
  source 1..28: mol_type = other DNA
atgtcagcctgcaccatcccccaccagg

SEQ ID NO: 32019 - DNA, 28 bp, synthetic construct
  source 1..28: mol_type = other DNA
gagtgaggaatgtgtggaagcactatgg

SEQ ID NO: 32020 - DNA, 28 bp, synthetic construct
  source 1..28: mol_type = other DNA
gatgaggggaggagtgaggaatgtgtgg

SEQ ID NO: 32021 - DNA, 28 bp, synthetic construct
  source 1..28: mol_type = other DNA
ttcttgctggatgaggggaggagtgagg

SEQ ID NO: 32022 - DNA, 28 bp, synthetic construct
  source 1..28: mol_type = other DNA
cctcccctcatccagcaagaaaacacgg

SEQ ID NO: 32023 - DNA, 28 bp, synthetic construct
  source 1..28: mol_type = other DNA
gcaccgtgttttcttgctggatgagggg

SEQ ID NO: 32024 - DNA, 28 bp, synthetic construct
  source 1..28: mol_type = other DNA
agcaccgtgttttcttgctggatgaggg

SEQ ID NO: 32025 - DNA, 28 bp, synthetic construct
  source 1..28: mol_type = other DNA
aagcaccgtgttttcttgctggatgagg

SEQ ID NO: 32026 - DNA, 28 bp, synthetic construct
  source 1..28: mol_type = other DNA
tcaggtaagcaccgtgttttcttgctgg

SEQ ID NO: 32027 - DNA, 28 bp, synthetic construct
  source 1..28: mol_type = other DNA
gtattcagaaacagtagagctcatcagg

SEQ ID NO: 32028 - DNA, 28 bp, synthetic construct
  source 1..28: mol_type = other DNA
ctactgtttctgaatacatcgtataagg

SEQ ID NO: 32029 - DNA, 28 bp, synthetic construct
  source 1..28: mol_type = other DNA
tctgaatacatcgtataaggagatttgg

SEQ ID NO: 32030 - DNA, 28 bp, synthetic construct
  source 1..28: mol_type = other DNA
atcgtataaggagatttggattccatgg

SEQ ID NO: 32031 - DNA, 28 bp, synthetic construct
  source 1..28: mol_type = other DNA
tcgtataaggagatttggattccatggg

SEQ ID NO: 32032 - DNA, 28 bp, synthetic construct
  source 1..28: mol_type = other DNA
cgtataaggagatttggattccatgggg

SEQ ID NO: 32033 - DNA, 28 bp, synthetic construct
  source 1..28: mol_type = other DNA
ggaaatgcaatggaacaaggccccatgg

SEQ ID NO: 32034 - DNA, 28 bp, synthetic construct
  source 1..28: mol_type = other DNA
tcgagtgtggaaatgcaatggaacaagg

SEQ ID NO: 32035 - DNA, 28 bp, synthetic construct
  source 1..28: mol_type = other DNA
tcgtttatcgagtgtggaaatgcaatgg

SEQ ID NO: 32036 - DNA, 28 bp, synthetic construct
  source 1..28: mol_type = other DNA
aagcagcattgtcgtttatcgagtgtgg

SEQ ID NO: 32037 - DNA, 28 bp, synthetic construct
  source 1..28: mol_type = other DNA
gttgatcaggtggaaaagtttggaaagg

SEQ ID NO: 32038 - DNA, 28 bp, synthetic construct
  source 1..28: mol_type = other DNA
actctgttgatcaggtggaaaagtttgg

SEQ ID NO: 32039 - DNA, 28 bp, synthetic construct
  source 1..28: mol_type = other DNA
cactgtattaactctgttgatcaggtgg

SEQ ID NO: 32040 - DNA, 28 bp, synthetic construct
  source 1..28: mol_type = other DNA
agacactgtattaactctgttgatcagg

SEQ ID NO: 32041 - DNA, 28 bp, synthetic construct
  source 1..28: mol_type = other DNA
ttcctaaacaatagttttttttaaatgg

SEQ ID NO: 32042 - DNA, 28 bp, synthetic construct
  source 1..28: mol_type = other DNA
tgccatttaaaaaaaactattgtttagg

SEQ ID NO: 32043 - DNA, 28 bp, synthetic construct
  source 1..28: mol_type = other DNA
aagtcagagttgggtttctcaaataagg

SEQ ID NO: 32044 - DNA, 28 bp, synthetic construct
  source 1..28: mol_type = other DNA
tcataggattttagaagtcagagttggg

SEQ ID NO: 32045 - DNA, 28 bp, synthetic construct
  source 1..28: mol_type = other DNA
ttcataggattttagaagtcagagttgg

SEQ ID NO: 32046 - DNA, 28 bp, synthetic construct
  source 1..28: mol_type = other DNA
tacaaggatggccgggtctgttcaatgg

SEQ ID NO: 32047 - DNA, 28 bp, synthetic construct
  source 1..28: mol_type = other DNA
tataaaatctattacaaggatggccggg

SEQ ID NO: 32048 - DNA, 28 bp, synthetic construct
  source 1..28: mol_type = other DNA
ttataaaatctattacaaggatggccgg

SEQ ID NO: 32049 - DNA, 28 bp, synthetic construct
  source 1..28: mol_type = other DNA
gtaattataaaatctattacaaggatgg

SEQ ID NO: 32050 - DNA, 28 bp, synthetic construct
  source 1..28: mol_type = other DNA
tggggtaattataaaatctattacaagg

SEQ ID NO: 32051 - DNA, 28 bp, synthetic construct
  source 1..28: mol_type = other DNA
cttcatcactgggacaatatagctgggg

SEQ ID NO: 32052 - DNA, 28 bp, synthetic construct
  source 1..28: mol_type = other DNA
gcttcatcactgggacaatatagctggg

SEQ ID NO: 32053 - DNA, 28 bp, synthetic construct
  source 1..28: mol_type = other DNA
agcttcatcactgggacaatatagctgg

SEQ ID NO: 32054 - DNA, 28 bp, synthetic construct
  source 1..28: mol_type = other DNA
atgtgtgtactgcagcttcatcactggg

SEQ ID NO: 32055 - DNA, 28 bp, synthetic construct
  source 1..28: mol_type = other DNA
tatgtgtgtactgcagcttcatcactgg

SEQ ID NO: 32056 - DNA, 28 bp, synthetic construct
  source 1..28: mol_type = other DNA
atgaagctgcagtacacacataatttgg

SEQ ID NO: 32057 - DNA, 28 bp, synthetic construct
  source 1..28: mol_type = other DNA
cacacataatttggaagaacgtatctgg

SEQ ID NO: 32058 - DNA, 28 bp, synthetic construct
  source 1..28: mol_type = other DNA
ttggaagaacgtatctggaaagaaaagg

SEQ ID NO: 32059 - DNA, 28 bp, synthetic construct
  source 1..28: mol_type = other DNA
tggaagaacgtatctggaaagaaaaggg

SEQ ID NO: 32060 - DNA, 28 bp, synthetic construct
  source 1..28: mol_type = other DNA
cgaatgaagcataaagcagatgcaatgg

SEQ ID NO: 32061 - DNA, 28 bp, synthetic construct
  source 1..28: mol_type = other DNA
cgtttagcttcttgcataaaataatcgg

SEQ ID NO: 32062 - DNA, 28 bp, synthetic construct
  source 1..28: mol_type = other DNA
cttgcataaaataatcggcactgcgagg

SEQ ID NO: 32063 - DNA, 28 bp, synthetic construct
  source 1..28: mol_type = other DNA
aataatcggcactgcgaggcctacaagg

SEQ ID NO: 32064 - DNA, 28 bp, synthetic construct
  source 1..28: mol_type = other DNA
acgtttaatatcattctctccttgtagg

SEQ ID NO: 32065 - DNA, 28 bp, synthetic construct
  source 1..28: mol_type = other DNA
gagagaatgatattaaacgtcattatgg

SEQ ID NO: 32066 - DNA, 28 bp, synthetic construct
  source 1..28: mol_type = other DNA
tattccttcctttcactcaaacttaagg

SEQ ID NO: 32067 - DNA, 28 bp, synthetic construct
  source 1..28: mol_type = other DNA
tgtgccttaagtttgagtgaaaggaagg

SEQ ID NO: 32068 - DNA, 28 bp, synthetic construct
  source 1..28: mol_type = other DNA
aaattgtgccttaagtttgagtgaaagg

SEQ ID NO: 32069 - DNA, 28 bp, synthetic construct
  source 1..28: mol_type = other DNA
cacaatttaaaaactctgcttaatgcgg

SEQ ID NO: 32070 - DNA, 28 bp, synthetic construct
  source 1..28: mol_type = other DNA
ctacagtgcggcctttttttcccctggg

SEQ ID NO: 32071 - DNA, 28 bp, synthetic construct
  source 1..28: mol_type = other DNA
gctacagtgcggcctttttttcccctgg

SEQ ID NO: 32072 - DNA, 28 bp, synthetic construct
  source 1..28: mol_type = other DNA
gaaaaaaaggccgcactgtagctgaagg

SEQ ID NO: 32073 - DNA, 28 bp, synthetic construct
  source 1..28: mol_type = other DNA
aaaaaggccgcactgtagctgaaggtgg

SEQ ID NO: 32074 - DNA, 28 bp, synthetic construct
  source 1..28: mol_type = other DNA
ggtgtggccaccttcagctacagtgcgg

SEQ ID NO: 32075 - DNA, 28 bp, synthetic construct
  source 1..28: mol_type = other DNA
actgtagctgaaggtggccacaccaagg

SEQ ID NO: 32076 - DNA, 28 bp, synthetic construct
  source 1..28: mol_type = other DNA
tggaaggggcatgggcaccttggtgtgg

SEQ ID NO: 32077 - DNA, 28 bp, synthetic construct
  source 1..28: mol_type = other DNA
tcaggtggaaggggcatgggcaccttgg

SEQ ID NO: 32078 - DNA, 28 bp, synthetic construct
  source 1..28: mol_type = other DNA
gaagctgctcaggtggaaggggcatggg

SEQ ID NO: 32079 - DNA, 28 bp, synthetic construct
  source 1..28: mol_type = other DNA
agaagctgctcaggtggaaggggcatgg

SEQ ID NO: 32080 - DNA, 28 bp, synthetic construct
  source 1..28: mol_type = other DNA
agaacagaagctgctcaggtggaagggg

SEQ ID NO: 32081 - DNA, 28 bp, synthetic construct
  source 1..28: mol_type = other DNA
cagaacagaagctgctcaggtggaaggg

SEQ ID NO: 32082 - DNA, 28 bp, synthetic construct
  source 1..28: mol_type = other DNA
acagaacagaagctgctcaggtggaagg

SEQ ID NO: 32083 - DNA, 28 bp, synthetic construct
  source 1..28: mol_type = other DNA
caagacagaacagaagctgctcaggtgg

SEQ ID NO: 32084 - DNA, 28 bp, synthetic construct
  source 1..28: mol_type = other DNA
gggcaagacagaacagaagctgctcagg

SEQ ID NO: 32085 - DNA, 28 bp, synthetic construct
  source 1..28: mol_type = other DNA
ttcagacgcttttaaatgtggtgagggg

SEQ ID NO: 32086 - DNA, 28 bp, synthetic construct
  source 1..28: mol_type = other DNA
gttcagacgcttttaaatgtggtgaggg

SEQ ID NO: 32087 - DNA, 28 bp, synthetic construct
  source 1..28: mol_type = other DNA
agttcagacgcttttaaatgtggtgagg

SEQ ID NO: 32088 - DNA, 28 bp, synthetic construct
  source 1..28: mol_type = other DNA
atgtaagttcagacgcttttaaatgtgg

SEQ ID NO: 32089 - DNA, 28 bp, synthetic construct
  source 1..28: mol_type = other DNA
aagtttctgcctcttgcagtccctgtgg

SEQ ID NO: 32090 - DNA, 28 bp, synthetic construct
  source 1..28: mol_type = other DNA
tgcctcttgcagtccctgtggccgttgg

SEQ ID NO: 32091 - DNA, 28 bp, synthetic construct
  source 1..28: mol_type = other DNA
ctccaacggccacagggactgcaagagg

SEQ ID NO: 32092 - DNA, 28 bp, synthetic construct
  source 1..28: mol_type = other DNA
tgcagtccctgtggccgttggagcctgg

SEQ ID NO: 32093 - DNA, 28 bp, synthetic construct
  source 1..28: mol_type = other DNA
tggtctccaggctccaacggccacaggg

SEQ ID NO: 32094 - DNA, 28 bp, synthetic construct
  source 1..28: mol_type = other DNA
gtggtctccaggctccaacggccacagg

SEQ ID NO: 32095 - DNA, 28 bp, synthetic construct
  source 1..28: mol_type = other DNA
tgtggccgttggagcctggagaccacgg

SEQ ID NO: 32096 - DNA, 28 bp, synthetic construct
  source 1..28: mol_type = other DNA
cgaagccgtggtctccaggctccaacgg

SEQ ID NO: 32097 - DNA, 28 bp, synthetic construct
  source 1..28: mol_type = other DNA
agcctggagaccacggcttcgtctgcgg

SEQ ID NO: 32098 - DNA, 28 bp, synthetic construct
  source 1..28: mol_type = other DNA
ggccgcagacgaagccgtggtctccagg

SEQ ID NO: 32099 - DNA, 28 bp, synthetic construct
  source 1..28: mol_type = other DNA
caagtcacggccgcagacgaagccgtgg

SEQ ID NO: 32100 - DNA, 28 bp, synthetic construct
  source 1..28: mol_type = other DNA
cggcttcgtctgcggccgtgacttgtgg

SEQ ID NO: 32101 - DNA, 28 bp, synthetic construct
  source 1..28: mol_type = other DNA
cttcgtctgcggccgtgacttgtggagg

SEQ ID NO: 32102 - DNA, 28 bp, synthetic construct
  source 1..28: mol_type = other DNA
ttcgtctgcggccgtgacttgtggaggg

SEQ ID NO: 32103 - DNA, 28 bp, synthetic construct
  source 1..28: mol_type = other DNA
tcgtctgcggccgtgacttgtggagggg

SEQ ID NO: 32104 - DNA, 28 bp, synthetic construct
  source 1..28: mol_type = other DNA
tgaaaacattcccctccacaagtcacgg

SEQ ID NO: 32105 - DNA, 28 bp, synthetic construct
  source 1..28: mol_type = other DNA
caaacaacacacatctttgagaaattgg

SEQ ID NO: 32106 - DNA, 28 bp, synthetic construct
  source 1..28: mol_type = other DNA
acacatctttgagaaattggccacctgg

SEQ ID NO: 32107 - DNA, 28 bp, synthetic construct
  source 1..28: mol_type = other DNA
gtgatgggctgctcgcttcaccaggtgg

SEQ ID NO: 32108 - DNA, 28 bp, synthetic construct
  source 1..28: mol_type = other DNA
tatgtgatgggctgctcgcttcaccagg

SEQ ID NO: 32109 - DNA, 28 bp, synthetic construct
  source 1..28: mol_type = other DNA
tattctacgtatgtatgtatgtgatggg

SEQ ID NO: 32110 - DNA, 28 bp, synthetic construct
  source 1..28: mol_type = other DNA
atattctacgtatgtatgtatgtgatgg

SEQ ID NO: 32111 - DNA, 28 bp, synthetic construct
  source 1..28: mol_type = other DNA
catacatacatacgtagaatatctttgg

SEQ ID NO: 32112 - DNA, 28 bp, synthetic construct
  source 1..28: mol_type = other DNA
ctagcacagtctgaacacatgcttgagg

SEQ ID NO: 32113 - DNA, 28 bp, synthetic construct
  source 1..28: mol_type = other DNA
ctcaagcatgtgttcagactgtgctagg

SEQ ID NO: 32114 - DNA, 28 bp, synthetic construct
  source 1..28: mol_type = other DNA
actgtgctaggttagagacagagcttgg

SEQ ID NO: 32115 - DNA, 28 bp, synthetic construct
  source 1..28: mol_type = other DNA
ctgtgctaggttagagacagagcttggg

SEQ ID NO: 32116 - DNA, 28 bp, synthetic construct
  source 1..28: mol_type = other DNA
tgtgctaggttagagacagagcttgggg

SEQ ID NO: 32117 - DNA, 28 bp, synthetic construct
  source 1..28: mol_type = other DNA
gtgctaggttagagacagagcttggggg

SEQ ID NO: 32118 - DNA, 28 bp, synthetic construct
  source 1..28: mol_type = other DNA
agcttgggggtgctcaatttcattttgg

SEQ ID NO: 32119 - DNA, 28 bp, synthetic construct
  source 1..28: mol_type = other DNA
tgctcaatttcattttggttttaattgg

SEQ ID NO: 32120 - DNA, 28 bp, synthetic construct
  source 1..28: mol_type = other DNA
gctcaatttcattttggttttaattggg

SEQ ID NO: 32121 - DNA, 28 bp, synthetic construct
  source 1..28: mol_type = other DNA
atttcattttggttttaattgggaaagg

SEQ ID NO: 32122 - DNA, 28 bp, synthetic construct
  source 1..28: mol_type = other DNA
aaaggaagagcatcaacaaaccgtgagg

SEQ ID NO: 32123 - DNA, 28 bp, synthetic construct
  source 1..28: mol_type = other DNA
aacaaaccgtgaggtctccgccgtgagg

SEQ ID NO: 32124 - DNA, 28 bp, synthetic construct
  source 1..28: mol_type = other DNA
ctgcagcctcacggcggagacctcacgg

SEQ ID NO: 32125 - DNA, 28 bp, synthetic construct
  source 1..28: mol_type = other DNA
gaggtctccgccgtgaggctgcagctgg

SEQ ID NO: 32126 - DNA, 28 bp, synthetic construct
  source 1..28: mol_type = other DNA
ccgccgtgaggctgcagctggctgtcgg

SEQ ID NO: 32127 - DNA, 28 bp, synthetic construct
  source 1..28: mol_type = other DNA
aggccgacagccagctgcagcctcacgg

SEQ ID NO: 32128 - DNA, 28 bp, synthetic construct
  source 1..28: mol_type = other DNA
gaggctgcagctggctgtcggccttagg

SEQ ID NO: 32129 - DNA, 28 bp, synthetic construct
  source 1..28: mol_type = other DNA
tggctgtcggccttaggctttttgctgg

SEQ ID NO: 32130 - DNA, 28 bp, synthetic construct
  source 1..28: mol_type = other DNA
tcggccttaggctttttgctggaagagg

SEQ ID NO: 32131 - DNA, 28 bp, synthetic construct
  source 1..28: mol_type = other DNA
tcagcctcttccagcaaaaagcctaagg

SEQ ID NO: 32132 - DNA, 28 bp, synthetic construct
  source 1..28: mol_type = other DNA
ctgaagtaaacaaactgttgccattagg

SEQ ID NO: 32133 - DNA, 28 bp, synthetic construct
  source 1..28: mol_type = other DNA
agtaaacaaactgttgccattaggtcgg

SEQ ID NO: 32134 - DNA, 28 bp, synthetic construct
  source 1..28: mol_type = other DNA
aacaaactgttgccattaggtcggctgg

SEQ ID NO: 32135 - DNA, 28 bp, synthetic construct
  source 1..28: mol_type = other DNA
acttaacttcttccagccgacctaatgg

SEQ ID NO: 32136 - DNA, 28 bp, synthetic construct
  source 1..28: mol_type = other DNA
cggctggaagaagttaagtcctcgctgg

SEQ ID NO: 32137 - DNA, 28 bp, synthetic construct
  source 1..28: mol_type = other DNA
gcatctaaacacaaatacaccagcgagg

SEQ ID NO: 32138 - DNA, 28 bp, synthetic construct
  source 1..28: mol_type = other DNA
gtatttgtgtttagatgcatcagagagg

SEQ ID NO: 32139 - DNA, 28 bp, synthetic construct
  source 1..28: mol_type = other DNA
tatttgtgtttagatgcatcagagaggg

SEQ ID NO: 32140 - DNA, 28 bp, synthetic construct
  source 1..28: mol_type = other DNA
atttgtgtttagatgcatcagagagggg

SEQ ID NO: 32141 - DNA, 28 bp, synthetic construct
  source 1..28: mol_type = other DNA
ttagatgcatcagagaggggtgagatgg

SEQ ID NO: 32142 - DNA, 28 bp, synthetic construct
  source 1..28: mol_type = other DNA
tagatgcatcagagaggggtgagatggg

SEQ ID NO: 32143 - DNA, 28 bp, synthetic construct
  source 1..28: mol_type = other DNA
aataaataaaaatgaaaaaatgcttcgg

SEQ ID NO: 32144 - DNA, 28 bp, synthetic construct
  source 1..28: mol_type = other DNA
gaagcattttttcatttttatttattgg

SEQ ID NO: 32145 - DNA, 28 bp, synthetic construct
  source 1..28: mol_type = other DNA
tttattggtattgccacactgaaaaagg

SEQ ID NO: 32146 - DNA, 28 bp, synthetic construct
  source 1..28: mol_type = other DNA
attgccacactgaaaaaggaaattacgg

SEQ ID NO: 32147 - DNA, 28 bp, synthetic construct
  source 1..28: mol_type = other DNA
attaccgtaatttcctttttcagtgtgg

SEQ ID NO: 32148 - DNA, 28 bp, synthetic construct
  source 1..28: mol_type = other DNA
acactgaaaaaggaaattacggtaatgg

SEQ ID NO: 32149 - DNA, 28 bp, synthetic construct
  source 1..28: mol_type = other DNA
taatggaatgttacagagtcagcacagg

SEQ ID NO: 32150 - DNA, 28 bp, synthetic construct
  source 1..28: mol_type = other DNA
aatggaatgttacagagtcagcacaggg

SEQ ID NO: 32151 - DNA, 28 bp, synthetic construct
  source 1..28: mol_type = other DNA
aatgttacagagtcagcacagggaaagg

SEQ ID NO: 32152 - DNA, 28 bp, synthetic construct
  source 1..28: mol_type = other DNA
tttcatatgacccaaaccacccaactgg

SEQ ID NO: 32153 - DNA, 28 bp, synthetic construct
  source 1..28: mol_type = other DNA
ttcatatgacccaaaccacccaactggg

SEQ ID NO: 32154 - DNA, 28 bp, synthetic construct
  source 1..28: mol_type = other DNA
cccaaaccacccaactgggacctgttgg

SEQ ID NO: 32155 - DNA, 28 bp, synthetic construct
  source 1..28: mol_type = other DNA
accaacaggtcccagttgggtggtttgg

SEQ ID NO: 32156 - DNA, 28 bp, synthetic construct
  source 1..28: mol_type = other DNA
aaccacccaactgggacctgttggtagg

SEQ ID NO: 32157 - DNA, 28 bp, synthetic construct
  source 1..28: mol_type = other DNA
ctcctaccaacaggtcccagttgggtgg

SEQ ID NO: 32158 - DNA, 28 bp, synthetic construct
  source 1..28: mol_type = other DNA
cttctcctaccaacaggtcccagttggg

SEQ ID NO: 32159 - DNA, 28 bp, synthetic construct
  source 1..28: mol_type = other DNA
gcttctcctaccaacaggtcccagttgg

SEQ ID NO: 32160 - DNA, 28 bp, synthetic construct
  source 1..28: mol_type = other DNA
ggacctgttggtaggagaagcttattgg

SEQ ID NO: 32161 - DNA, 28 bp, synthetic construct
  source 1..28: mol_type = other DNA
gacctgttggtaggagaagcttattggg

SEQ ID NO: 32162 - DNA, 28 bp, synthetic construct
  source 1..28: mol_type = other DNA
ttcccaataagcttctcctaccaacagg

SEQ ID NO: 32163 - DNA, 28 bp, synthetic construct
  source 1..28: mol_type = other DNA
ggctttttgaggactactctggtcaagg

SEQ ID NO: 32164 - DNA, 28 bp, synthetic construct
  source 1..28: mol_type = other DNA
gggtcaggctttttgaggactactctgg

SEQ ID NO: 32165 - DNA, 28 bp, synthetic construct
  source 1..28: mol_type = other DNA
tgttggaggagggtcaggctttttgagg

SEQ ID NO: 32166 - DNA, 28 bp, synthetic construct
  source 1..28: mol_type = other DNA
aagcctgaccctcctccaacatagcagg

SEQ ID NO: 32167 - DNA, 28 bp, synthetic construct
  source 1..28: mol_type = other DNA
tcacctgctatgttggaggagggtcagg

SEQ ID NO: 32168 - DNA, 28 bp, synthetic construct
  source 1..28: mol_type = other DNA
gaaagtcacctgctatgttggaggaggg

SEQ ID NO: 32169 - DNA, 28 bp, synthetic construct
  source 1..28: mol_type = other DNA
tgaaagtcacctgctatgttggaggagg

SEQ ID NO: 32170 - DNA, 28 bp, synthetic construct
  source 1..28: mol_type = other DNA
gtctgaaagtcacctgctatgttggagg

SEQ ID NO: 32171 - DNA, 28 bp, synthetic construct
  source 1..28: mol_type = other DNA
tgggtctgaaagtcacctgctatgttgg

SEQ ID NO: 32172 - DNA, 28 bp, synthetic construct
  source 1..28: mol_type = other DNA
gtggaagtgagctggagagatctctggg

SEQ ID NO: 32173 - DNA, 28 bp, synthetic construct
  source 1..28: mol_type = other DNA
agtggaagtgagctggagagatctctgg

SEQ ID NO: 32174 - DNA, 28 bp, synthetic construct
  source 1..28: mol_type = other DNA
agatctctccagctcacttccactttgg

SEQ ID NO: 32175 - DNA, 28 bp, synthetic construct
  source 1..28: mol_type = other DNA
tctctccagctcacttccactttggagg

SEQ ID NO: 32176 - DNA, 28 bp, synthetic construct
  source 1..28: mol_type = other DNA
ctctccagctcacttccactttggaggg

SEQ ID NO: 32177 - DNA, 28 bp, synthetic construct
  source 1..28: mol_type = other DNA
cattccctccaaagtggaagtgagctgg

SEQ ID NO: 32178 - DNA, 28 bp, synthetic construct
  source 1..28: mol_type = other DNA
acaggtacgtgcattccctccaaagtgg

SEQ ID NO: 32179 - DNA, 28 bp, synthetic construct
  source 1..28: mol_type = other DNA
gtacctgttgatgttcatgttgcagtgg

SEQ ID NO: 32180 - DNA, 28 bp, synthetic construct
  source 1..28: mol_type = other DNA
aaaccactgcaacatgaacatcaacagg

SEQ ID NO: 32181 - DNA, 28 bp, synthetic construct
  source 1..28: mol_type = other DNA
cagtggtttgcagacaaagtattactgg

SEQ ID NO: 32182 - DNA, 28 bp, synthetic construct
  source 1..28: mol_type = other DNA
tggtttgcagacaaagtattactggtgg

SEQ ID NO: 32183 - DNA, 28 bp, synthetic construct
  source 1..28: mol_type = other DNA
tttgcagacaaagtattactggtggagg

SEQ ID NO: 32184 - DNA, 28 bp, synthetic construct
  source 1..28: mol_type = other DNA
gcagacaaagtattactggtggaggtgg

SEQ ID NO: 32185 - DNA, 28 bp, synthetic construct
  source 1..28: mol_type = other DNA
ggagagaaagacagctcttcaagactgg

SEQ ID NO: 32186 - DNA, 28 bp, synthetic construct
  source 1..28: mol_type = other DNA
tcttgaagagctgtctttctctccctgg

SEQ ID NO: 32187 - DNA, 28 bp, synthetic construct
  source 1..28: mol_type = other DNA
cttgaagagctgtctttctctccctggg

SEQ ID NO: 32188 - DNA, 28 bp, synthetic construct
  source 1..28: mol_type = other DNA
actacagggagatcaagaagtcccaggg

SEQ ID NO: 32189 - DNA, 28 bp, synthetic construct
  source 1..28: mol_type = other DNA
gactacagggagatcaagaagtcccagg

SEQ ID NO: 32190 - DNA, 28 bp, synthetic construct
  source 1..28: mol_type = other DNA
cagtgtgacaacgaagacgactacaggg

SEQ ID NO: 32191 - DNA, 28 bp, synthetic construct
  source 1..28: mol_type = other DNA
acagtgtgacaacgaagacgactacagg

SEQ ID NO: 32192 - DNA, 28 bp, synthetic construct
  source 1..28: mol_type = other DNA
tagtcgtcttcgttgtcacactgtatgg

SEQ ID NO: 32193 - DNA, 28 bp, synthetic construct
  source 1..28: mol_type = other DNA
agtcgtcttcgttgtcacactgtatggg

SEQ ID NO: 32194 - DNA, 28 bp, synthetic construct
  source 1..28: mol_type = other DNA
ggaataaactaaagtcaatcagcactgg

SEQ ID NO: 32195 - DNA, 28 bp, synthetic construct
  source 1..28: mol_type = other DNA
aagtcaatcagcactggatttcaagagg

SEQ ID NO: 32196 - DNA, 28 bp, synthetic construct
  source 1..28: mol_type = other DNA
atttcaagaggtattatgagttcccagg

SEQ ID NO: 32197 - DNA, 28 bp, synthetic construct
  source 1..28: mol_type = other DNA
cccaggcaccgacttccacagagcaagg

SEQ ID NO: 32198 - DNA, 28 bp, synthetic construct
  source 1..28: mol_type = other DNA
gccttgctctgtggaagtcggtgcctgg

SEQ ID NO: 32199 - DNA, 28 bp, synthetic construct
  source 1..28: mol_type = other DNA
ccgacttccacagagcaaggcctcctgg

SEQ ID NO: 32200 - DNA, 28 bp, synthetic construct
  source 1..28: mol_type = other DNA
cgacttccacagagcaaggcctcctggg

SEQ ID NO: 32201 - DNA, 28 bp, synthetic construct
  source 1..28: mol_type = other DNA
ggggctcccaggaggccttgctctgtgg

SEQ ID NO: 32202 - DNA, 28 bp, synthetic construct
  source 1..28: mol_type = other DNA
aggcctcctgggagccccactcacctgg

SEQ ID NO: 32203 - DNA, 28 bp, synthetic construct
  source 1..28: mol_type = other DNA
aagccaggtgagtggggctcccaggagg

SEQ ID NO: 32204 - DNA, 28 bp, synthetic construct
  source 1..28: mol_type = other DNA
gggaagccaggtgagtggggctcccagg

SEQ ID NO: 32205 - DNA, 28 bp, synthetic construct
  source 1..28: mol_type = other DNA
gtgcttcggggaagccaggtgagtgggg

SEQ ID NO: 32206 - DNA, 28 bp, synthetic construct
  source 1..28: mol_type = other DNA
tgtgcttcggggaagccaggtgagtggg

SEQ ID NO: 32207 - DNA, 28 bp, synthetic construct
  source 1..28: mol_type = other DNA
ctgtgcttcggggaagccaggtgagtgg

SEQ ID NO: 32208 - DNA, 28 bp, synthetic construct
  source 1..28: mol_type = other DNA
gctgtttgggacggtaggctgccgcagg

SEQ ID NO: 32209 - DNA, 28 bp, synthetic construct
  source 1..28: mol_type = other DNA
gcctaccgtcccaaacagcagcctatgg

SEQ ID NO: 32210 - DNA, 28 bp, synthetic construct
  source 1..28: mol_type = other DNA
cccataggctgctgtttgggacggtagg

SEQ ID NO: 32211 - DNA, 28 bp, synthetic construct
  source 1..28: mol_type = other DNA
agcacccataggctgctgtttgggacgg

SEQ ID NO: 32212 - DNA, 28 bp, synthetic construct
  source 1..28: mol_type = other DNA
atagagcacccataggctgctgtttggg

SEQ ID NO: 32213 - DNA, 28 bp, synthetic construct
  source 1..28: mol_type = other DNA
gatagagcacccataggctgctgtttgg

SEQ ID NO: 32214 - DNA, 28 bp, synthetic construct
  source 1..28: mol_type = other DNA
gtgggtacttggatagagcacccatagg

SEQ ID NO: 32215 - DNA, 28 bp, synthetic construct
  source 1..28: mol_type = other DNA
ggctatctcttaacttgtgggtacttgg

SEQ ID NO: 32216 - DNA, 28 bp, synthetic construct
  source 1..28: mol_type = other DNA
gggaaggggctatctcttaacttgtggg

SEQ ID NO: 32217 - DNA, 28 bp, synthetic construct
  source 1..28: mol_type = other DNA
ggggaaggggctatctcttaacttgtgg

SEQ ID NO: 32218 - DNA, 28 bp, synthetic construct
  source 1..28: mol_type = other DNA
ggggtgcgggggcgtggaggggaagggg

SEQ ID NO: 32219 - DNA, 28 bp, synthetic construct
  source 1..28: mol_type = other DNA
tggggtgcgggggcgtggaggggaaggg

SEQ ID NO: 32220 - DNA, 28 bp, synthetic construct
  source 1..28: mol_type = other DNA
ctggggtgcgggggcgtggaggggaagg

SEQ ID NO: 32221 - DNA, 28 bp, synthetic construct
  source 1..28: mol_type = other DNA
ctgactggggtgcgggggcgtggagggg

SEQ ID NO: 32222 - DNA, 28 bp, synthetic construct
  source 1..28: mol_type = other DNA
gctgactggggtgcgggggcgtggaggg

SEQ ID NO: 32223 - DNA, 28 bp, synthetic construct
  source 1..28: mol_type = other DNA
ggctgactggggtgcgggggcgtggagg

SEQ ID NO: 32224 - DNA, 28 bp, synthetic construct
  source 1..28: mol_type = other DNA
tggggctgactggggtgcgggggcgtgg

SEQ ID NO: 32225 - DNA, 28 bp, synthetic construct
  source 1..28: mol_type = other DNA
acgcccccgcaccccagtcagccccagg

SEQ ID NO: 32226 - DNA, 28 bp, synthetic construct
  source 1..28: mol_type = other DNA
aggcctggggctgactggggtgcggggg

SEQ ID NO: 32227 - DNA, 28 bp, synthetic construct
  source 1..28: mol_type = other DNA
taggcctggggctgactggggtgcgggg

SEQ ID NO: 32228 - DNA, 28 bp, synthetic construct
  source 1..28: mol_type = other DNA
gtaggcctggggctgactggggtgcggg

SEQ ID NO: 32229 - DNA, 28 bp, synthetic construct
  source 1..28: mol_type = other DNA
ggtaggcctggggctgactggggtgcgg

SEQ ID NO: 32230 - DNA, 28 bp, synthetic construct
  source 1..28: mol_type = other DNA
cgcaaggtaggcctggggctgactgggg

SEQ ID NO: 32231 - DNA, 28 bp, synthetic construct
  source 1..28: mol_type = other DNA
acgcaaggtaggcctggggctgactggg

SEQ ID NO: 32232 - DNA, 28 bp, synthetic construct
  source 1..28: mol_type = other DNA
aacgcaaggtaggcctggggctgactgg

SEQ ID NO: 32233 - DNA, 28 bp, synthetic construct
  source 1..28: mol_type = other DNA
caagaggaaacgcaaggtaggcctgggg

SEQ ID NO: 32234 - DNA, 28 bp, synthetic construct
  source 1..28: mol_type = other DNA
cccaggcctaccttgcgtttcctcttgg

SEQ ID NO: 32235 - DNA, 28 bp, synthetic construct
  source 1..28: mol_type = other DNA
tccaagaggaaacgcaaggtaggcctgg

SEQ ID NO: 32236 - DNA, 28 bp, synthetic construct
  source 1..28: mol_type = other DNA
caaaatccaagaggaaacgcaaggtagg

SEQ ID NO: 32237 - DNA, 28 bp, synthetic construct
  source 1..28: mol_type = other DNA
ctaccttgcgtttcctcttggattttgg

SEQ ID NO: 32238 - DNA, 28 bp, synthetic construct
  source 1..28: mol_type = other DNA
ttgccaaaatccaagaggaaacgcaagg

SEQ ID NO: 32239 - DNA, 28 bp, synthetic construct
  source 1..28: mol_type = other DNA
agaaaaggctttgccaaaatccaagagg

SEQ ID NO: 32240 - DNA, 28 bp, synthetic construct
  source 1..28: mol_type = other DNA
tggattttggcaaagccttttctgcagg

SEQ ID NO: 32241 - DNA, 28 bp, synthetic construct
  source 1..28: mol_type = other DNA
aaagccttttctgcaggtgtgtccgagg

SEQ ID NO: 32242 - DNA, 28 bp, synthetic construct
  source 1..28: mol_type = other DNA
cacacctcggacacacctgcagaaaagg

SEQ ID NO: 32243 - DNA, 28 bp, synthetic construct
  source 1..28: mol_type = other DNA
cttttctgcaggtgtgtccgaggtgtgg

SEQ ID NO: 32244 - DNA, 28 bp, synthetic construct
  source 1..28: mol_type = other DNA
tctgcaggtgtgtccgaggtgtggctgg

SEQ ID NO: 32245 - DNA, 28 bp, synthetic construct
  source 1..28: mol_type = other DNA
ctgcaggtgtgtccgaggtgtggctggg

SEQ ID NO: 32246 - DNA, 28 bp, synthetic construct
  source 1..28: mol_type = other DNA
caggtgtgtccgaggtgtggctgggcgg

SEQ ID NO: 32247 - DNA, 28 bp, synthetic construct
  source 1..28: mol_type = other DNA
gagagcgcaccgcccagccacacctcgg

SEQ ID NO: 32248 - DNA, 28 bp, synthetic construct
  source 1..28: mol_type = other DNA
ctgggcggtgcgctctcagagtccttgg

SEQ ID NO: 32249 - DNA, 28 bp, synthetic construct
  source 1..28: mol_type = other DNA
ggcggtgcgctctcagagtccttggtgg

SEQ ID NO: 32250 - DNA, 28 bp, synthetic construct
  source 1..28: mol_type = other DNA
gtgcgctctcagagtccttggtggcagg

SEQ ID NO: 32251 - DNA, 28 bp, synthetic construct
  source 1..28: mol_type = other DNA
tgcgctctcagagtccttggtggcaggg

SEQ ID NO: 32252 - DNA, 28 bp, synthetic construct
  source 1..28: mol_type = other DNA
gcgctctcagagtccttggtggcagggg

SEQ ID NO: 32253 - DNA, 28 bp, synthetic construct
  source 1..28: mol_type = other DNA
ggggtattgagcgcccctgccaccaagg

SEQ ID NO: 32254 - DNA, 28 bp, synthetic construct
  source 1..28: mol_type = other DNA
tggtggcaggggcgctcaatacccctgg

SEQ ID NO: 32255 - DNA, 28 bp, synthetic construct
  source 1..28: mol_type = other DNA
aggggcgctcaatacccctggctcctgg

SEQ ID NO: 32256 - DNA, 28 bp, synthetic construct
  source 1..28: mol_type = other DNA
ggggcgctcaatacccctggctcctggg

SEQ ID NO: 32257 - DNA, 28 bp, synthetic construct
  source 1..28: mol_type = other DNA
gggcgctcaatacccctggctcctgggg

SEQ ID NO: 32258 - DNA, 28 bp, synthetic construct
  source 1..28: mol_type = other DNA
gctcaatacccctggctcctggggcagg

SEQ ID NO: 32259 - DNA, 28 bp, synthetic construct
  source 1..28: mol_type = other DNA
cccctggctcctggggcaggtgttctgg

SEQ ID NO: 32260 - DNA, 28 bp, synthetic construct
  source 1..28: mol_type = other DNA
cccagaacacctgccccaggagccaggg

SEQ ID NO: 32261 - DNA, 28 bp, synthetic construct
  source 1..28: mol_type = other DNA
tcccagaacacctgccccaggagccagg

SEQ ID NO: 32262 - DNA, 28 bp, synthetic construct
  source 1..28: mol_type = other DNA
tcctggggcaggtgttctgggatcctgg

SEQ ID NO: 32263 - DNA, 28 bp, synthetic construct
  source 1..28: mol_type = other DNA
tccaggatcccagaacacctgccccagg

SEQ ID NO: 32264 - DNA, 28 bp, synthetic construct
  source 1..28: mol_type = other DNA
gggcaggtgttctgggatcctggacagg

SEQ ID NO: 32265 - DNA, 28 bp, synthetic construct
  source 1..28: mol_type = other DNA
caggtgttctgggatcctggacaggagg

SEQ ID NO: 32266 - DNA, 28 bp, synthetic construct
  source 1..28: mol_type = other DNA
aggtgttctgggatcctggacaggaggg

SEQ ID NO: 32267 - DNA, 28 bp, synthetic construct
  source 1..28: mol_type = other DNA
ttctgggatcctggacaggagggtcagg

SEQ ID NO: 32268 - DNA, 28 bp, synthetic construct
  source 1..28: mol_type = other DNA
caaaatcgacctgaccctcctgtccagg

SEQ ID NO: 32269 - DNA, 28 bp, synthetic construct
  source 1..28: mol_type = other DNA
gacagtgatgagatcaggtctctctggg

SEQ ID NO: 32270 - DNA, 28 bp, synthetic construct
  source 1..28: mol_type = other DNA
ggacagtgatgagatcaggtctctctgg

SEQ ID NO: 32271 - DNA, 28 bp, synthetic construct
  source 1..28: mol_type = other DNA
acctgatctcatcactgtcctttagagg

SEQ ID NO: 32272 - DNA, 28 bp, synthetic construct
  source 1..28: mol_type = other DNA
cctgatctcatcactgtcctttagaggg

SEQ ID NO: 32273 - DNA, 28 bp, synthetic construct
  source 1..28: mol_type = other DNA
ctgatctcatcactgtcctttagagggg

SEQ ID NO: 32274 - DNA, 28 bp, synthetic construct
  source 1..28: mol_type = other DNA
cggaacgaacttctctcccctctaaagg

SEQ ID NO: 32275 - DNA, 28 bp, synthetic construct
  source 1..28: mol_type = other DNA
ctttagaggggagagaagttcgttccgg

SEQ ID NO: 32276 - DNA, 28 bp, synthetic construct
  source 1..28: mol_type = other DNA
ggggagagaagttcgttccggccaaagg

SEQ ID NO: 32277 - DNA, 28 bp, synthetic construct
  source 1..28: mol_type = other DNA
gggagagaagttcgttccggccaaaggg

SEQ ID NO: 32278 - DNA, 28 bp, synthetic construct
  source 1..28: mol_type = other DNA
ggagagaagttcgttccggccaaagggg

SEQ ID NO: 32279 - DNA, 28 bp, synthetic construct
  source 1..28: mol_type = other DNA
gttctacacactggtcccctttggccgg

SEQ ID NO: 32280 - DNA, 28 bp, synthetic construct
  source 1..28: mol_type = other DNA
agcagttctacacactggtcccctttgg

SEQ ID NO: 32281 - DNA, 28 bp, synthetic construct
  source 1..28: mol_type = other DNA
gagctggaggagcagttctacacactgg

SEQ ID NO: 32282 - DNA, 28 bp, synthetic construct
  source 1..28: mol_type = other DNA
gtgtagaactgctcctccagctccttgg

SEQ ID NO: 32283 - DNA, 28 bp, synthetic construct
  source 1..28: mol_type = other DNA
tcctccagctccttggcgatgtcactgg

SEQ ID NO: 32284 - DNA, 28 bp, synthetic construct
  source 1..28: mol_type = other DNA
accagtgacatcgccaaggagctggagg

SEQ ID NO: 32285 - DNA, 28 bp, synthetic construct
  source 1..28: mol_type = other DNA
tccagctccttggcgatgtcactggtgg

SEQ ID NO: 32286 - DNA, 28 bp, synthetic construct
  source 1..28: mol_type = other DNA
accaccagtgacatcgccaaggagctgg

SEQ ID NO: 32287 - DNA, 28 bp, synthetic construct
  source 1..28: mol_type = other DNA
tccttggcgatgtcactggtggtcctgg

SEQ ID NO: 32288 - DNA, 28 bp, synthetic construct
  source 1..28: mol_type = other DNA
gccaggaccaccagtgacatcgccaagg

SEQ ID NO: 32289 - DNA, 28 bp, synthetic construct
  source 1..28: mol_type = other DNA
atgtcactggtggtcctggcgttgatgg

SEQ ID NO: 32290 - DNA, 28 bp, synthetic construct
  source 1..28: mol_type = other DNA
tggtcctggcgttgatggagcctacagg

SEQ ID NO: 32291 - DNA, 28 bp, synthetic construct
  source 1..28: mol_type = other DNA
ggtcctggcgttgatggagcctacaggg

SEQ ID NO: 32292 - DNA, 28 bp, synthetic construct
  source 1..28: mol_type = other DNA
gtcctggcgttgatggagcctacagggg

SEQ ID NO: 32293 - DNA, 28 bp, synthetic construct
  source 1..28: mol_type = other DNA
ggcccctgtaggctccatcaacgccagg

SEQ ID NO: 32294 - DNA, 28 bp, synthetic construct
  source 1..28: mol_type = other DNA
cgttgatggagcctacaggggccctagg

SEQ ID NO: 32295 - DNA, 28 bp, synthetic construct
  source 1..28: mol_type = other DNA
ggggcagtggtcctagggcccctgtagg

SEQ ID NO: 32296 - DNA, 28 bp, synthetic construct
  source 1..28: mol_type = other DNA
ggggccctaggaccactgcccccgttgg

SEQ ID NO: 32297 - DNA, 28 bp, synthetic construct
  source 1..28: mol_type = other DNA
gctgccaacgggggcagtggtcctaggg

SEQ ID NO: 32298 - DNA, 28 bp, synthetic construct
  source 1..28: mol_type = other DNA
cgctgccaacgggggcagtggtcctagg

SEQ ID NO: 32299 - DNA, 28 bp, synthetic construct
  source 1..28: mol_type = other DNA
ctaggaccactgcccccgttggcagcgg

SEQ ID NO: 32300 - DNA, 28 bp, synthetic construct
  source 1..28: mol_type = other DNA
aggaggccgctgccaacgggggcagtgg

SEQ ID NO: 32301 - DNA, 28 bp, synthetic construct
  source 1..28: mol_type = other DNA
ggctgaaggaggccgctgccaacggggg

SEQ ID NO: 32302 - DNA, 28 bp, synthetic construct
  source 1..28: mol_type = other DNA
aggctgaaggaggccgctgccaacgggg

SEQ ID NO: 32303 - DNA, 28 bp, synthetic construct
  source 1..28: mol_type = other DNA
gaggctgaaggaggccgctgccaacggg

SEQ ID NO: 32304 - DNA, 28 bp, synthetic construct
  source 1..28: mol_type = other DNA
agaggctgaaggaggccgctgccaacgg

SEQ ID NO: 32305 - DNA, 28 bp, synthetic construct
  source 1..28: mol_type = other DNA
gcctccttcagcctctgatcattcccgg

SEQ ID NO: 32306 - DNA, 28 bp, synthetic construct
  source 1..28: mol_type = other DNA
tccgggaatgatcagaggctgaaggagg

SEQ ID NO: 32307 - DNA, 28 bp, synthetic construct
  source 1..28: mol_type = other DNA
tccttcagcctctgatcattcccggagg

SEQ ID NO: 32308 - DNA, 28 bp, synthetic construct
  source 1..28: mol_type = other DNA
tcctccgggaatgatcagaggctgaagg

SEQ ID NO: 32309 - DNA, 28 bp, synthetic construct
  source 1..28: mol_type = other DNA
ttcagcctctgatcattcccggaggagg

SEQ ID NO: 32310 - DNA, 28 bp, synthetic construct
  source 1..28: mol_type = other DNA
ctctgcctcctccgggaatgatcagagg

SEQ ID NO: 32311 - DNA, 28 bp, synthetic construct
  source 1..28: mol_type = other DNA
ctctgatcattcccggaggaggcagagg

SEQ ID NO: 32312 - DNA, 28 bp, synthetic construct
  source 1..28: mol_type = other DNA
ttcccggaggaggcagaggcagccacgg

SEQ ID NO: 32313 - DNA, 28 bp, synthetic construct
  source 1..28: mol_type = other DNA
gaccgtggctgcctctgcctcctccggg

SEQ ID NO: 32314 - DNA, 28 bp, synthetic construct
  source 1..28: mol_type = other DNA
agaccgtggctgcctctgcctcctccgg

SEQ ID NO: 32315 - DNA, 28 bp, synthetic construct
  source 1..28: mol_type = other DNA
gcagaggcagccacggtctgtgctttgg

SEQ ID NO: 32316 - DNA, 28 bp, synthetic construct
  source 1..28: mol_type = other DNA
cagccacggtctgtgctttggacagagg

SEQ ID NO: 32317 - DNA, 28 bp, synthetic construct
  source 1..28: mol_type = other DNA
agccacggtctgtgctttggacagaggg

SEQ ID NO: 32318 - DNA, 28 bp, synthetic construct
  source 1..28: mol_type = other DNA
taccctctgtccaaagcacagaccgtgg

SEQ ID NO: 32319 - DNA, 28 bp, synthetic construct
  source 1..28: mol_type = other DNA
ttggacagagggtactcctcctgctcgg

SEQ ID NO: 32320 - DNA, 28 bp, synthetic construct
  source 1..28: mol_type = other DNA
agggtactcctcctgctcggactccagg

SEQ ID NO: 32321 - DNA, 28 bp, synthetic construct
  source 1..28: mol_type = other DNA
tactcctcctgctcggactccaggtcgg

SEQ ID NO: 32322 - DNA, 28 bp, synthetic construct
  source 1..28: mol_type = other DNA
gactccgacctggagtccgagcaggagg

SEQ ID NO: 32323 - DNA, 28 bp, synthetic construct
  source 1..28: mol_type = other DNA
tcggactccgacctggagtccgagcagg

SEQ ID NO: 32324 - DNA, 28 bp, synthetic construct
  source 1..28: mol_type = other DNA
tgctcggactccaggtcggagtccgagg

SEQ ID NO: 32325 - DNA, 28 bp, synthetic construct
  source 1..28: mol_type = other DNA
tcggactccaggtcggagtccgaggagg

SEQ ID NO: 32326 - DNA, 28 bp, synthetic construct
  source 1..28: mol_type = other DNA
gactccaggtcggagtccgaggaggagg

SEQ ID NO: 32327 - DNA, 28 bp, synthetic construct
  source 1..28: mol_type = other DNA
tcatcctcctcctcggactccgacctgg

SEQ ID NO: 32328 - DNA, 28 bp, synthetic construct
  source 1..28: mol_type = other DNA
gagtcgtcatcttcatcctcctcctcgg

SEQ ID NO: 32329 - DNA, 28 bp, synthetic construct
  source 1..28: mol_type = other DNA
gacgactctgtctcaatgaactccttgg

SEQ ID NO: 32330 - DNA, 28 bp, synthetic construct
  source 1..28: mol_type = other DNA
tctgtctcaatgaactccttggatttgg

SEQ ID NO: 32331 - DNA, 28 bp, synthetic construct
  source 1..28: mol_type = other DNA
ctgtctcaatgaactccttggatttggg

SEQ ID NO: 32332 - DNA, 28 bp, synthetic construct
  source 1..28: mol_type = other DNA
tgtctcaatgaactccttggatttgggg

SEQ ID NO: 32333 - DNA, 28 bp, synthetic construct
  source 1..28: mol_type = other DNA
ctaagcaggatcgtccccaaatccaagg

SEQ ID NO: 32334 - DNA, 28 bp, synthetic construct
  source 1..28: mol_type = other DNA
gacgatcctgcttagcccccgcgtgcgg

SEQ ID NO: 32335 - DNA, 28 bp, synthetic construct
  source 1..28: mol_type = other DNA
gaagcgccgcacgcgggggctaagcagg

SEQ ID NO: 32336 - DNA, 28 bp, synthetic construct
  source 1..28: mol_type = other DNA
agcccccgcgtgcggcgcttctcgcagg

SEQ ID NO: 32337 - DNA, 28 bp, synthetic construct
  source 1..28: mol_type = other DNA
gacctgcgagaagcgccgcacgcggggg

SEQ ID NO: 32338 - DNA, 28 bp, synthetic construct
  source 1..28: mol_type = other DNA
tgacctgcgagaagcgccgcacgcgggg

SEQ ID NO: 32339 - DNA, 28 bp, synthetic construct
  source 1..28: mol_type = other DNA
gtgacctgcgagaagcgccgcacgcggg

SEQ ID NO: 32340 - DNA, 28 bp, synthetic construct
  source 1..28: mol_type = other DNA
cgtgacctgcgagaagcgccgcacgcgg

SEQ ID NO: 32341 - DNA, 28 bp, synthetic construct
  source 1..28: mol_type = other DNA
cgcgtgcggcgcttctcgcaggtcacgg

SEQ ID NO: 32342 - DNA, 28 bp, synthetic construct
  source 1..28: mol_type = other DNA
gtgcggcgcttctcgcaggtcacggagg

SEQ ID NO: 32343 - DNA, 28 bp, synthetic construct
  source 1..28: mol_type = other DNA
ggtcacggaggagcgcagctccttgcgg

SEQ ID NO: 32344 - DNA, 28 bp, synthetic construct
  source 1..28: mol_type = other DNA
cacggaggagcgcagctccttgcggtgg

SEQ ID NO: 32345 - DNA, 28 bp, synthetic construct
  source 1..28: mol_type = other DNA
ggcaacaacagagcgagccaccgcaagg

SEQ ID NO: 32346 - DNA, 28 bp, synthetic construct
  source 1..28: mol_type = other DNA
cggtggctcgctctgttgttgccacagg

SEQ ID NO: 32347 - DNA, 28 bp, synthetic construct
  source 1..28: mol_type = other DNA
ggtggctcgctctgttgttgccacaggg

SEQ ID NO: 32348 - DNA, 28 bp, synthetic construct
  source 1..28: mol_type = other DNA
ctcgctctgttgttgccacagggcctgg

SEQ ID NO: 32349 - DNA, 28 bp, synthetic construct
  source 1..28: mol_type = other DNA
ctgttgttgccacagggcctggttttgg

SEQ ID NO: 32350 - DNA, 28 bp, synthetic construct
  source 1..28: mol_type = other DNA
ttgttgccacagggcctggttttggtgg

SEQ ID NO: 32351 - DNA, 28 bp, synthetic construct
  source 1..28: mol_type = other DNA
tgttgccacagggcctggttttggtggg

SEQ ID NO: 32352 - DNA, 28 bp, synthetic construct
  source 1..28: mol_type = other DNA
cggagcccaccaaaaccaggccctgtgg

SEQ ID NO: 32353 - DNA, 28 bp, synthetic construct
  source 1..28: mol_type = other DNA
cacagggcctggttttggtgggctccgg

SEQ ID NO: 32354 - DNA, 28 bp, synthetic construct
  source 1..28: mol_type = other DNA
acagggcctggttttggtgggctccggg

SEQ ID NO: 32355 - DNA, 28 bp, synthetic construct
  source 1..28: mol_type = other DNA
cagggcctggttttggtgggctccgggg

SEQ ID NO: 32356 - DNA, 28 bp, synthetic construct
  source 1..28: mol_type = other DNA
agggcctggttttggtgggctccggggg

SEQ ID NO: 32357 - DNA, 28 bp, synthetic construct
  source 1..28: mol_type = other DNA
gggcctggttttggtgggctccgggggg

SEQ ID NO: 32358 - DNA, 28 bp, synthetic construct
  source 1..28: mol_type = other DNA
ggtccccccggagcccaccaaaaccagg

SEQ ID NO: 32359 - DNA, 28 bp, synthetic construct
  source 1..28: mol_type = other DNA
ctggggacgagcgtggtggtccccccgg

SEQ ID NO: 32360 - DNA, 28 bp, synthetic construct
  source 1..28: mol_type = other DNA
gcggacgcgctggggacgagcgtggtgg

SEQ ID NO: 32361 - DNA, 28 bp, synthetic construct
  source 1..28: mol_type = other DNA
accacgctcgtccccagcgcgtccgcgg

SEQ ID NO: 32362 - DNA, 28 bp, synthetic construct
  source 1..28: mol_type = other DNA
gccgcggacgcgctggggacgagcgtgg

SEQ ID NO: 32363 - DNA, 28 bp, synthetic construct
  source 1..28: mol_type = other DNA
ctcgtccccagcgcgtccgcggccgcgg

SEQ ID NO: 32364 - DNA, 28 bp, synthetic construct
  source 1..28: mol_type = other DNA
tcgtccccagcgcgtccgcggccgcggg

SEQ ID NO: 32365 - DNA, 28 bp, synthetic construct
  source 1..28: mol_type = other DNA
ggagcccgcggccgcggacgcgctgggg

SEQ ID NO: 32366 - DNA, 28 bp, synthetic construct
  source 1..28: mol_type = other DNA
aggagcccgcggccgcggacgcgctggg

SEQ ID NO: 32367 - DNA, 28 bp, synthetic construct
  source 1..28: mol_type = other DNA
gaggagcccgcggccgcggacgcgctgg

SEQ ID NO: 32368 - DNA, 28 bp, synthetic construct
  source 1..28: mol_type = other DNA
agcgcgtccgcggccgcgggctcctcgg

SEQ ID NO: 32369 - DNA, 28 bp, synthetic construct
  source 1..28: mol_type = other DNA
gcgcgtccgcggccgcgggctcctcggg

SEQ ID NO: 32370 - DNA, 28 bp, synthetic construct
  source 1..28: mol_type = other DNA
gtccgcggccgcgggctcctcgggccgg

SEQ ID NO: 32371 - DNA, 28 bp, synthetic construct
  source 1..28: mol_type = other DNA
caccggcccgaggagcccgcggccgcgg

SEQ ID NO: 32372 - DNA, 28 bp, synthetic construct
  source 1..28: mol_type = other DNA
cgcggccgcgggctcctcgggccggtgg

SEQ ID NO: 32373 - DNA, 28 bp, synthetic construct
  source 1..28: mol_type = other DNA
aactgccaccggcccgaggagcccgcgg

SEQ ID NO: 32374 - DNA, 28 bp, synthetic construct
  source 1..28: mol_type = other DNA
gcgggctcctcgggccggtggcagttgg

SEQ ID NO: 32375 - DNA, 28 bp, synthetic construct
  source 1..28: mol_type = other DNA
gacggcgccaactgccaccggcccgagg

SEQ ID NO: 32376 - DNA, 28 bp, synthetic construct
  source 1..28: mol_type = other DNA
ggccggtggcagttggcgccgtccccgg

SEQ ID NO: 32377 - DNA, 28 bp, synthetic construct
  source 1..28: mol_type = other DNA
agccggggacggcgccaactgccaccgg

SEQ ID NO: 32378 - DNA, 28 bp, synthetic construct
  source 1..28: mol_type = other DNA
tggcagttggcgccgtccccggctgagg

SEQ ID NO: 32379 - DNA, 28 bp, synthetic construct
  source 1..28: mol_type = other DNA
gcgccgtccccggctgaggtcctctcgg

SEQ ID NO: 32380 - DNA, 28 bp, synthetic construct
  source 1..28: mol_type = other DNA
gcaccgagaggacctcagccggggacgg

SEQ ID NO: 32381 - DNA, 28 bp, synthetic construct
  source 1..28: mol_type = other DNA
aggcgcaccgagaggacctcagccgggg

SEQ ID NO: 32382 - DNA, 28 bp, synthetic construct
  source 1..28: mol_type = other DNA
caggcgcaccgagaggacctcagccggg

SEQ ID NO: 32383 - DNA, 28 bp, synthetic construct
  source 1..28: mol_type = other DNA
ccaggcgcaccgagaggacctcagccgg

SEQ ID NO: 32384 - DNA, 28 bp, synthetic construct
  source 1..28: mol_type = other DNA
gctgaggtcctctcggtgcgcctggtgg

SEQ ID NO: 32385 - DNA, 28 bp, synthetic construct
  source 1..28: mol_type = other DNA
ctgaggtcctctcggtgcgcctggtggg

SEQ ID NO: 32386 - DNA, 28 bp, synthetic construct
  source 1..28: mol_type = other DNA
caagaagcccaccaggcgcaccgagagg

SEQ ID NO: 32387 - DNA, 28 bp, synthetic construct
  source 1..28: mol_type = other DNA
gtgcgcctggtgggcttcttgcccgcgg

SEQ ID NO: 32388 - DNA, 28 bp, synthetic construct
  source 1..28: mol_type = other DNA
gaggtccgcgggcaagaagcccaccagg

SEQ ID NO: 32389 - DNA, 28 bp, synthetic construct
  source 1..28: mol_type = other DNA
ggtgggcttcttgcccgcggacctccgg

SEQ ID NO: 32390 - DNA, 28 bp, synthetic construct
  source 1..28: mol_type = other DNA
gtgggcttcttgcccgcggacctccggg

SEQ ID NO: 32391 - DNA, 28 bp, synthetic construct
  source 1..28: mol_type = other DNA
gcttcttgcccgcggacctccgggcagg

SEQ ID NO: 32392 - DNA, 28 bp, synthetic construct
  source 1..28: mol_type = other DNA
ttgcccgcggacctccgggcaggcgcgg

SEQ ID NO: 32393 - DNA, 28 bp, synthetic construct
  source 1..28: mol_type = other DNA
tgcccgcggacctccgggcaggcgcggg

SEQ ID NO: 32394 - DNA, 28 bp, synthetic construct
  source 1..28: mol_type = other DNA
cgcccgcgcctgcccggaggtccgcggg

SEQ ID NO: 32395 - DNA, 28 bp, synthetic construct
  source 1..28: mol_type = other DNA
gcgcccgcgcctgcccggaggtccgcgg

SEQ ID NO: 32396 - DNA, 28 bp, synthetic construct
  source 1..28: mol_type = other DNA
ggagaacgcgcccgcgcctgcccggagg

SEQ ID NO: 32397 - DNA, 28 bp, synthetic construct
  source 1..28: mol_type = other DNA
cgcggagaacgcgcccgcgcctgcccgg

SEQ ID NO: 32398 - DNA, 28 bp, synthetic construct
  source 1..28: mol_type = other DNA
cgggcaggcgcgggcgcgttctccgcgg

SEQ ID NO: 32399 - DNA, 28 bp, synthetic construct
  source 1..28: mol_type = other DNA
gggcaggcgcgggcgcgttctccgcggg

SEQ ID NO: 32400 - DNA, 28 bp, synthetic construct
  source 1..28: mol_type = other DNA
gcgggcgcgttctccgcgggcgcacagg

SEQ ID NO: 32401 - DNA, 28 bp, synthetic construct
  source 1..28: mol_type = other DNA
cgggcgcgttctccgcgggcgcacaggg

SEQ ID NO: 32402 - DNA, 28 bp, synthetic construct
  source 1..28: mol_type = other DNA
ttctccgcgggcgcacagggcactgcgg

SEQ ID NO: 32403 - DNA, 28 bp, synthetic construct
  source 1..28: mol_type = other DNA
tctccgcgggcgcacagggcactgcggg

SEQ ID NO: 32404 - DNA, 28 bp, synthetic construct
  source 1..28: mol_type = other DNA
ccgcgggcgcacagggcactgcgggtgg

SEQ ID NO: 32405 - DNA, 28 bp, synthetic construct
  source 1..28: mol_type = other DNA
cgggcgcacagggcactgcgggtggcgg

SEQ ID NO: 32406 - DNA, 28 bp, synthetic construct
  source 1..28: mol_type = other DNA
gggcgcacagggcactgcgggtggcggg

SEQ ID NO: 32407 - DNA, 28 bp, synthetic construct
  source 1..28: mol_type = other DNA
ggcgcacagggcactgcgggtggcgggg

SEQ ID NO: 32408 - DNA, 28 bp, synthetic construct
  source 1..28: mol_type = other DNA
gcacagggcactgcgggtggcggggcgg

SEQ ID NO: 32409 - DNA, 28 bp, synthetic construct
  source 1..28: mol_type = other DNA
ggcggggcggctgcgctcaccgccacgg

SEQ ID NO: 32410 - DNA, 28 bp, synthetic construct
  source 1..28: mol_type = other DNA
gcggctgcgctcaccgccacggccacgg

SEQ ID NO: 32411 - DNA, 28 bp, synthetic construct
  source 1..28: mol_type = other DNA
gcgctcaccgccacggccacggccgcgg

SEQ ID NO: 32412 - DNA, 28 bp, synthetic construct
  source 1..28: mol_type = other DNA
cgctcaccgccacggccacggccgcggg

SEQ ID NO: 32413 - DNA, 28 bp, synthetic construct
  source 1..28: mol_type = other DNA
tcaccgccacggccacggccgcgggcgg

SEQ ID NO: 32414 - DNA, 28 bp, synthetic construct
  source 1..28: mol_type = other DNA
caccgccacggccacggccgcgggcggg

SEQ ID NO: 32415 - DNA, 28 bp, synthetic construct
  source 1..28: mol_type = other DNA
accgccacggccacggccgcgggcgggg

SEQ ID NO: 32416 - DNA, 28 bp, synthetic construct
  source 1..28: mol_type = other DNA
tccccgcccgcggccgtggccgtggcgg

SEQ ID NO: 32417 - DNA, 28 bp, synthetic construct
  source 1..28: mol_type = other DNA
aagtccccgcccgcggccgtggccgtgg

SEQ ID NO: 32418 - DNA, 28 bp, synthetic construct
  source 1..28: mol_type = other DNA
aagcagaagtccccgcccgcggccgtgg

SEQ ID NO: 32419 - DNA, 28 bp, synthetic construct
  source 1..28: mol_type = other DNA
ggcgtgaagcagaagtccccgcccgcgg

SEQ ID NO: 32420 - DNA, 28 bp, synthetic construct
  source 1..28: mol_type = other DNA
acttctgcttcacgcctttactcccagg

SEQ ID NO: 32421 - DNA, 28 bp, synthetic construct
  source 1..28: mol_type = other DNA
cttctgcttcacgcctttactcccaggg

SEQ ID NO: 32422 - DNA, 28 bp, synthetic construct
  source 1..28: mol_type = other DNA
ttctgcttcacgcctttactcccagggg

SEQ ID NO: 32423 - DNA, 28 bp, synthetic construct
  source 1..28: mol_type = other DNA
acgcctttactcccaggggccttgttgg

SEQ ID NO: 32424 - DNA, 28 bp, synthetic construct
  source 1..28: mol_type = other DNA
cagccaacaaggcccctgggagtaaagg

SEQ ID NO: 32425 - DNA, 28 bp, synthetic construct
  source 1..28: mol_type = other DNA
tcccaggggccttgttggctgtccttgg

SEQ ID NO: 32426 - DNA, 28 bp, synthetic construct
  source 1..28: mol_type = other DNA
gccaaggacagccaacaaggcccctggg

SEQ ID NO: 32427 - DNA, 28 bp, synthetic construct
  source 1..28: mol_type = other DNA
ggccaaggacagccaacaaggcccctgg

SEQ ID NO: 32428 - DNA, 28 bp, synthetic construct
  source 1..28: mol_type = other DNA
gagcaaaggccaaggacagccaacaagg

SEQ ID NO: 32429 - DNA, 28 bp, synthetic construct
  source 1..28: mol_type = other DNA
cacttgcaaggaggagcaaaggccaagg

SEQ ID NO: 32430 - DNA, 28 bp, synthetic construct
  source 1..28: mol_type = other DNA
caagagcacttgcaaggaggagcaaagg

SEQ ID NO: 32431 - DNA, 28 bp, synthetic construct
  source 1..28: mol_type = other DNA
aaggagatcaagagcacttgcaaggagg

SEQ ID NO: 32432 - DNA, 28 bp, synthetic construct
  source 1..28: mol_type = other DNA
gagaaggagatcaagagcacttgcaagg

SEQ ID NO: 32433 - DNA, 28 bp, synthetic construct
  source 1..28: mol_type = other DNA
agtgctcttgatctccttctctctcagg

SEQ ID NO: 32434 - DNA, 28 bp, synthetic construct
  source 1..28: mol_type = other DNA
ctcttgatctccttctctctcaggctgg

SEQ ID NO: 32435 - DNA, 28 bp, synthetic construct
  source 1..28: mol_type = other DNA
tcttgatctccttctctctcaggctggg

SEQ ID NO: 32436 - DNA, 28 bp, synthetic construct
  source 1..28: mol_type = other DNA
gatctccttctctctcaggctgggctgg

SEQ ID NO: 32437 - DNA, 28 bp, synthetic construct
  source 1..28: mol_type = other DNA
gtttgccagcccagcctgagagagaagg

SEQ ID NO: 32438 - DNA, 28 bp, synthetic construct
  source 1..28: mol_type = other DNA
tctctcaggctgggctggcaaacgtcgg

SEQ ID NO: 32439 - DNA, 28 bp, synthetic construct
  source 1..28: mol_type = other DNA
ctctcaggctgggctggcaaacgtcggg

SEQ ID NO: 32440 - DNA, 28 bp, synthetic construct
  source 1..28: mol_type = other DNA
tctcaggctgggctggcaaacgtcgggg

SEQ ID NO: 32441 - DNA, 28 bp, synthetic construct
  source 1..28: mol_type = other DNA
aacgtcggggactttcccacagtcctgg

SEQ ID NO: 32442 - DNA, 28 bp, synthetic construct
  source 1..28: mol_type = other DNA
ggtgaaagaggacgtccaggactgtggg

SEQ ID NO: 32443 - DNA, 28 bp, synthetic construct
  source 1..28: mol_type = other DNA
cggtgaaagaggacgtccaggactgtgg

SEQ ID NO: 32444 - DNA, 28 bp, synthetic construct
  source 1..28: mol_type = other DNA
cacagtcctggacgtcctctttcaccgg

SEQ ID NO: 32445 - DNA, 28 bp, synthetic construct
  source 1..28: mol_type = other DNA
acagtcctggacgtcctctttcaccggg

SEQ ID NO: 32446 - DNA, 28 bp, synthetic construct
  source 1..28: mol_type = other DNA
tacaacccggtgaaagaggacgtccagg

SEQ ID NO: 32447 - DNA, 28 bp, synthetic construct
  source 1..28: mol_type = other DNA
aatcagtactacaacccggtgaaagagg

SEQ ID NO: 32448 - DNA, 28 bp, synthetic construct
  source 1..28: mol_type = other DNA
tcagagagcaatcagtactacaacccgg

SEQ ID NO: 32449 - DNA, 28 bp, synthetic construct
  source 1..28: mol_type = other DNA
gtagtactgattgctctctgacccgtgg

SEQ ID NO: 32450 - DNA, 28 bp, synthetic construct
  source 1..28: mol_type = other DNA
gctctctgacccgtggctttcattttgg

SEQ ID NO: 32451 - DNA, 28 bp, synthetic construct
  source 1..28: mol_type = other DNA
tattctgatccaaaatgaaagccacggg

SEQ ID NO: 32452 - DNA, 28 bp, synthetic construct
  source 1..28: mol_type = other DNA
ctattctgatccaaaatgaaagccacgg

SEQ ID NO: 32453 - DNA, 28 bp, synthetic construct
  source 1..28: mol_type = other DNA
cgtggctttcattttggatcagaatagg

SEQ ID NO: 32454 - DNA, 28 bp, synthetic construct
  source 1..28: mol_type = other DNA
ggctttcattttggatcagaataggagg

SEQ ID NO: 32455 - DNA, 28 bp, synthetic construct
  source 1..28: mol_type = other DNA
attttggatcagaataggaggcttgtgg

SEQ ID NO: 32456 - DNA, 28 bp, synthetic construct
  source 1..28: mol_type = other DNA
ttttggatcagaataggaggcttgtggg

SEQ ID NO: 32457 - DNA, 28 bp, synthetic construct
  source 1..28: mol_type = other DNA
tttggatcagaataggaggcttgtgggg

SEQ ID NO: 32458 - DNA, 28 bp, synthetic construct
  source 1..28: mol_type = other DNA
ctctaacaagtggcagctggataaatgg

SEQ ID NO: 32459 - DNA, 28 bp, synthetic construct
  source 1..28: mol_type = other DNA
catttatccagctgccacttgttagagg

SEQ ID NO: 32460 - DNA, 28 bp, synthetic construct
  source 1..28: mol_type = other DNA
ccggcatcctctaacaagtggcagctgg

SEQ ID NO: 32461 - DNA, 28 bp, synthetic construct
  source 1..28: mol_type = other DNA
ggctgaaccggcatcctctaacaagtgg

SEQ ID NO: 32462 - DNA, 28 bp, synthetic construct
  source 1..28: mol_type = other DNA
ccggttcagcctgaaagcagaaaaccgg

SEQ ID NO: 32463 - DNA, 28 bp, synthetic construct
  source 1..28: mol_type = other DNA
tgtttgtcaccggttttctgctttcagg

SEQ ID NO: 32464 - DNA, 28 bp, synthetic construct
  source 1..28: mol_type = other DNA
taatgaaagatgttttgtttgtcaccgg

SEQ ID NO: 32465 - DNA, 28 bp, synthetic construct
  source 1..28: mol_type = other DNA
tgacaaacaaaacatctttcattacagg

SEQ ID NO: 32466 - DNA, 28 bp, synthetic construct
  source 1..28: mol_type = other DNA
atctttcattacaggctcacttaaaagg

SEQ ID NO: 32467 - DNA, 28 bp, synthetic construct
  source 1..28: mol_type = other DNA
tctttcattacaggctcacttaaaaggg

SEQ ID NO: 32468 - DNA, 28 bp, synthetic construct
  source 1..28: mol_type = other DNA
ctttcattacaggctcacttaaaagggg

SEQ ID NO: 32469 - DNA, 28 bp, synthetic construct
  source 1..28: mol_type = other DNA
attacaggctcacttaaaaggggcctgg

SEQ ID NO: 32470 - DNA, 28 bp, synthetic construct
  source 1..28: mol_type = other DNA
gaagtaagtcaagataaaaacagccagg

SEQ ID NO: 32471 - DNA, 28 bp, synthetic construct
  source 1..28: mol_type = other DNA
tctaagtatatgagcagaaaacgaatgg

SEQ ID NO: 32472 - DNA, 28 bp, synthetic construct
  source 1..28: mol_type = other DNA
ctaagtatatgagcagaaaacgaatggg

SEQ ID NO: 32473 - DNA, 28 bp, synthetic construct
  source 1..28: mol_type = other DNA
gtatatgagcagaaaacgaatgggctgg

SEQ ID NO: 32474 - DNA, 28 bp, synthetic construct
  source 1..28: mol_type = other DNA
agcacctggcttggggtctgcaggaggg

SEQ ID NO: 32475 - DNA, 28 bp, synthetic construct
  source 1..28: mol_type = other DNA
acctggcttggggtctgcaggagggagg

SEQ ID NO: 32476 - DNA, 28 bp, synthetic construct
  source 1..28: mol_type = other DNA
tcctccctcctgcagaccccaagccagg

SEQ ID NO: 32477 - DNA, 28 bp, synthetic construct
  source 1..28: mol_type = other DNA
ggcattgtcactgtcacactgctgcagg

SEQ ID NO: 32478 - DNA, 28 bp, synthetic construct
  source 1..28: mol_type = other DNA
gcagcagtgtgacagtgacaatgcccgg

SEQ ID NO: 32479 - DNA, 28 bp, synthetic construct
  source 1..28: mol_type = other DNA
ctgtctctatgaggatagcaagtccggg

SEQ ID NO: 32480 - DNA, 28 bp, synthetic construct
  source 1..28: mol_type = other DNA
tctgtctctatgaggatagcaagtccgg

SEQ ID NO: 32481 - DNA, 28 bp, synthetic construct
  source 1..28: mol_type = other DNA
cttgctatcctcatagagacagaagtgg

SEQ ID NO: 32482 - DNA, 28 bp, synthetic construct
  source 1..28: mol_type = other DNA
ttgctatcctcatagagacagaagtggg

SEQ ID NO: 32483 - DNA, 28 bp, synthetic construct
  source 1..28: mol_type = other DNA
tcctcatagagacagaagtgggcagagg

SEQ ID NO: 32484 - DNA, 28 bp, synthetic construct
  source 1..28: mol_type = other DNA
tcctctgcccacttctgtctctatgagg

SEQ ID NO: 32485 - DNA, 28 bp, synthetic construct
  source 1..28: mol_type = other DNA
atagagacagaagtgggcagaggagagg

SEQ ID NO: 32486 - DNA, 28 bp, synthetic construct
  source 1..28: mol_type = other DNA
agtgggcagaggagaggcctgagccagg

SEQ ID NO: 32487 - DNA, 28 bp, synthetic construct
  source 1..28: mol_type = other DNA
ggcctgagccaggcagcgcttacctcgg

SEQ ID NO: 32488 - DNA, 28 bp, synthetic construct
  source 1..28: mol_type = other DNA
gcctgagccaggcagcgcttacctcggg

SEQ ID NO: 32489 - DNA, 28 bp, synthetic construct
  source 1..28: mol_type = other DNA
ccccgaggtaagcgctgcctggctcagg

SEQ ID NO: 32490 - DNA, 28 bp, synthetic construct
  source 1..28: mol_type = other DNA
agccaggcagcgcttacctcggggctgg

SEQ ID NO: 32491 - DNA, 28 bp, synthetic construct
  source 1..28: mol_type = other DNA
ctccagccccgaggtaagcgctgcctgg

SEQ ID NO: 32492 - DNA, 28 bp, synthetic construct
  source 1..28: mol_type = other DNA
agcgcttacctcggggctggagaagtgg

SEQ ID NO: 32493 - DNA, 28 bp, synthetic construct
  source 1..28: mol_type = other DNA
gcgcttacctcggggctggagaagtggg

SEQ ID NO: 32494 - DNA, 28 bp, synthetic construct
  source 1..28: mol_type = other DNA
cgcttacctcggggctggagaagtgggg

SEQ ID NO: 32495 - DNA, 28 bp, synthetic construct
  source 1..28: mol_type = other DNA
gcttacctcggggctggagaagtggggg

SEQ ID NO: 32496 - DNA, 28 bp, synthetic construct
  source 1..28: mol_type = other DNA
cttacctcggggctggagaagtgggggg

SEQ ID NO: 32497 - DNA, 28 bp, synthetic construct
  source 1..28: mol_type = other DNA
ttacctcggggctggagaagtggggggg

SEQ ID NO: 32498 - DNA, 28 bp, synthetic construct
  source 1..28: mol_type = other DNA
aagcccccccacttctccagccccgagg

SEQ ID NO: 32499 - DNA, 28 bp, synthetic construct
  source 1..28: mol_type = other DNA
gggggcttgctgccctcactctcgctgg

SEQ ID NO: 32500 - DNA, 28 bp, synthetic construct
  source 1..28: mol_type = other DNA
ccctcactctcgctggagctgctctcgg

SEQ ID NO: 32501 - DNA, 28 bp, synthetic construct
  source 1..28: mol_type = other DNA
accgagagcagctccagcgagagtgagg

SEQ ID NO: 32502 - DNA, 28 bp, synthetic construct
  source 1..28: mol_type = other DNA
ctgctctcggtctccgagtcagatccgg

SEQ ID NO: 32503 - DNA, 28 bp, synthetic construct
  source 1..28: mol_type = other DNA
tcagagagcagctccggatctgactcgg

SEQ ID NO: 32504 - DNA, 28 bp, synthetic construct
  source 1..28: mol_type = other DNA
gatccggagctgctctctgagtcgctgg

SEQ ID NO: 32505 - DNA, 28 bp, synthetic construct
  source 1..28: mol_type = other DNA
cctccagcgactcagagagcagctccgg

SEQ ID NO: 32506 - DNA, 28 bp, synthetic construct
  source 1..28: mol_type = other DNA
agggcagcagcagcagcagcagcagcgg

SEQ ID NO: 32507 - DNA, 28 bp, synthetic construct
  source 1..28: mol_type = other DNA
ctgctgctgctgctgctgcccttgctgg

SEQ ID NO: 32508 - DNA, 28 bp, synthetic construct
  source 1..28: mol_type = other DNA
tgctgctgctgctgcccttgctggaagg

SEQ ID NO: 32509 - DNA, 28 bp, synthetic construct
  source 1..28: mol_type = other DNA
ctgctgcccttgctggaaggcaccgagg

SEQ ID NO: 32510 - DNA, 28 bp, synthetic construct
  source 1..28: mol_type = other DNA
gcagaacctcggtgccttccagcaaggg

SEQ ID NO: 32511 - DNA, 28 bp, synthetic construct
  source 1..28: mol_type = other DNA
tgcagaacctcggtgccttccagcaagg

SEQ ID NO: 32512 - DNA, 28 bp, synthetic construct
  source 1..28: mol_type = other DNA
ctggaaggcaccgaggttctgcagttgg

SEQ ID NO: 32513 - DNA, 28 bp, synthetic construct
  source 1..28: mol_type = other DNA
tggaaggcaccgaggttctgcagttggg

SEQ ID NO: 32514 - DNA, 28 bp, synthetic construct
  source 1..28: mol_type = other DNA
caccgaggttctgcagttgggctgctgg

SEQ ID NO: 32515 - DNA, 28 bp, synthetic construct
  source 1..28: mol_type = other DNA
gtccagcagcccaactgcagaacctcgg

SEQ ID NO: 32516 - DNA, 28 bp, synthetic construct
  source 1..28: mol_type = other DNA
gttctgcagttgggctgctggaccacgg

SEQ ID NO: 32517 - DNA, 28 bp, synthetic construct
  source 1..28: mol_type = other DNA
tggaccacggcgctgccagcccgcgagg

SEQ ID NO: 32518 - DNA, 28 bp, synthetic construct
  source 1..28: mol_type = other DNA
ggggcctcgcgggctggcagcgccgtgg

SEQ ID NO: 32519 - DNA, 28 bp, synthetic construct
  source 1..28: mol_type = other DNA
cggcgctgccagcccgcgaggcccccgg

SEQ ID NO: 32520 - DNA, 28 bp, synthetic construct
  source 1..28: mol_type = other DNA
ggcgctgccagcccgcgaggcccccggg

SEQ ID NO: 32521 - DNA, 28 bp, synthetic construct
  source 1..28: mol_type = other DNA
tctgcttcccgggggcctcgcgggctgg

SEQ ID NO: 32522 - DNA, 28 bp, synthetic construct
  source 1..28: mol_type = other DNA
agcccgcgaggcccccgggaagcagagg

SEQ ID NO: 32523 - DNA, 28 bp, synthetic construct
  source 1..28: mol_type = other DNA
gcccgcgaggcccccgggaagcagaggg

SEQ ID NO: 32524 - DNA, 28 bp, synthetic construct
  source 1..28: mol_type = other DNA
tccctctgcttcccgggggcctcgcggg

SEQ ID NO: 32525 - DNA, 28 bp, synthetic construct
  source 1..28: mol_type = other DNA
ttccctctgcttcccgggggcctcgcgg

SEQ ID NO: 32526 - DNA, 28 bp, synthetic construct
  source 1..28: mol_type = other DNA
gcgaggcccccgggaagcagagggaagg

SEQ ID NO: 32527 - DNA, 28 bp, synthetic construct
  source 1..28: mol_type = other DNA
ggctttccttccctctgcttcccggggg

SEQ ID NO: 32528 - DNA, 28 bp, synthetic construct
  source 1..28: mol_type = other DNA
tggctttccttccctctgcttcccgggg

SEQ ID NO: 32529 - DNA, 28 bp, synthetic construct
  source 1..28: mol_type = other DNA
ttggctttccttccctctgcttcccggg

SEQ ID NO: 32530 - DNA, 28 bp, synthetic construct
  source 1..28: mol_type = other DNA
cttggctttccttccctctgcttcccgg

SEQ ID NO: 32531 - DNA, 28 bp, synthetic construct
  source 1..28: mol_type = other DNA
gggaaggaaagccaagtgagcaaacagg

SEQ ID NO: 32532 - DNA, 28 bp, synthetic construct
  source 1..28: mol_type = other DNA
ggtggtgttttcctgtttgctcacttgg

SEQ ID NO: 32533 - DNA, 28 bp, synthetic construct
  source 1..28: mol_type = other DNA
ctctttagggtgcatgacagcttggtgg

SEQ ID NO: 32534 - DNA, 28 bp, synthetic construct
  source 1..28: mol_type = other DNA
caccaagctgtcatgcaccctaaagagg

SEQ ID NO: 32535 - DNA, 28 bp, synthetic construct
  source 1..28: mol_type = other DNA
accaagctgtcatgcaccctaaagaggg

SEQ ID NO: 32536 - DNA, 28 bp, synthetic construct
  source 1..28: mol_type = other DNA
tccctctttagggtgcatgacagcttgg

SEQ ID NO: 32537 - DNA, 28 bp, synthetic construct
  source 1..28: mol_type = other DNA
aagctgtcatgcaccctaaagagggagg

SEQ ID NO: 32538 - DNA, 28 bp, synthetic construct
  source 1..28: mol_type = other DNA
ctgtcatgcaccctaaagagggaggagg

SEQ ID NO: 32539 - DNA, 28 bp, synthetic construct
  source 1..28: mol_type = other DNA
aggctgcgtgcctcctccctctttaggg

SEQ ID NO: 32540 - DNA, 28 bp, synthetic construct
  source 1..28: mol_type = other DNA
taggctgcgtgcctcctccctctttagg

SEQ ID NO: 32541 - DNA, 28 bp, synthetic construct
  source 1..28: mol_type = other DNA
taacatcccagttcagagatactttagg

SEQ ID NO: 32542 - DNA, 28 bp, synthetic construct
  source 1..28: mol_type = other DNA
aacatcccagttcagagatactttaggg

SEQ ID NO: 32543 - DNA, 28 bp, synthetic construct
  source 1..28: mol_type = other DNA
tttgtccctaaagtatctctgaactggg

SEQ ID NO: 32544 - DNA, 28 bp, synthetic construct
  source 1..28: mol_type = other DNA
ttttgtccctaaagtatctctgaactgg

SEQ ID NO: 32545 - DNA, 28 bp, synthetic construct
  source 1..28: mol_type = other DNA
tttattgtggcatataattcataatcgg

SEQ ID NO: 32546 - DNA, 28 bp, synthetic construct
  source 1..28: mol_type = other DNA
ttatgaattatatgccacaataaatagg

SEQ ID NO: 32547 - DNA, 28 bp, synthetic construct
  source 1..28: mol_type = other DNA
tatgaattatatgccacaataaataggg

SEQ ID NO: 32548 - DNA, 28 bp, synthetic construct
  source 1..28: mol_type = other DNA
atgaaacattgagccctatttattgtgg

SEQ ID NO: 32549 - DNA, 28 bp, synthetic construct
  source 1..28: mol_type = other DNA
caaaatgtacctgtcagagagagcgcgg

SEQ ID NO: 32550 - DNA, 28 bp, synthetic construct
  source 1..28: mol_type = other DNA
aacggctctccgcgctctctctgacagg

SEQ ID NO: 32551 - DNA, 28 bp, synthetic construct
  source 1..28: mol_type = other DNA
gagagccgttctctgagctgcctgctgg

SEQ ID NO: 32552 - DNA, 28 bp, synthetic construct
  source 1..28: mol_type = other DNA
ttcttccagcaggcagctcagagaacgg

SEQ ID NO: 32553 - DNA, 28 bp, synthetic construct
  source 1..28: mol_type = other DNA
ctgagctgcctgctggaagaaagaaagg

SEQ ID NO: 32554 - DNA, 28 bp, synthetic construct
  source 1..28: mol_type = other DNA
tgagctgcctgctggaagaaagaaaggg

SEQ ID NO: 32555 - DNA, 28 bp, synthetic construct
  source 1..28: mol_type = other DNA
atctctgccctttctttcttccagcagg

SEQ ID NO: 32556 - DNA, 28 bp, synthetic construct
  source 1..28: mol_type = other DNA
catggcaaaaatgtgtgtaatgcagggg

SEQ ID NO: 32557 - DNA, 28 bp, synthetic construct
  source 1..28: mol_type = other DNA
acatggcaaaaatgtgtgtaatgcaggg

SEQ ID NO: 32558 - DNA, 28 bp, synthetic construct
  source 1..28: mol_type = other DNA
cacatggcaaaaatgtgtgtaatgcagg

SEQ ID NO: 32559 - DNA, 28 bp, synthetic construct
  source 1..28: mol_type = other DNA
ctgcattacacacatttttgccatgtgg

SEQ ID NO: 32560 - DNA, 28 bp, synthetic construct
  source 1..28: mol_type = other DNA
tgggtattacaaggaagctaagatcagg

SEQ ID NO: 32561 - DNA, 28 bp, synthetic construct
  source 1..28: mol_type = other DNA
ttagcttccttgtaatacccattgctgg

SEQ ID NO: 32562 - DNA, 28 bp, synthetic construct
  source 1..28: mol_type = other DNA
attgagaccagcaatgggtattacaagg

SEQ ID NO: 32563 - DNA, 28 bp, synthetic construct
  source 1..28: mol_type = other DNA
tttttatgatattgagaccagcaatggg

SEQ ID NO: 32564 - DNA, 28 bp, synthetic construct
  source 1..28: mol_type = other DNA
ttttttatgatattgagaccagcaatgg

SEQ ID NO: 32565 - DNA, 28 bp, synthetic construct
  source 1..28: mol_type = other DNA
atatcataaaaaattacagaattcaagg

SEQ ID NO: 32566 - DNA, 28 bp, synthetic construct
  source 1..28: mol_type = other DNA
aaaaaattacagaattcaaggcttaagg

SEQ ID NO: 32567 - DNA, 28 bp, synthetic construct
  source 1..28: mol_type = other DNA
aaaaattacagaattcaaggcttaaggg

SEQ ID NO: 32568 - DNA, 28 bp, synthetic construct
  source 1..28: mol_type = other DNA
agaattcaaggcttaagggaaattatgg

SEQ ID NO: 32569 - DNA, 28 bp, synthetic construct
  source 1..28: mol_type = other DNA
gaattcaaggcttaagggaaattatggg

SEQ ID NO: 32570 - DNA, 28 bp, synthetic construct
  source 1..28: mol_type = other DNA
gctaagtgtgagcttctatgcagttggg

SEQ ID NO: 32571 - DNA, 28 bp, synthetic construct
  source 1..28: mol_type = other DNA
tgctaagtgtgagcttctatgcagttgg

SEQ ID NO: 32572 - DNA, 28 bp, synthetic construct
  source 1..28: mol_type = other DNA
cttagcagacaaaagaccagcagcctgg

SEQ ID NO: 32573 - DNA, 28 bp, synthetic construct
  source 1..28: mol_type = other DNA
gctgaatggtggcactccaggctgctgg

SEQ ID NO: 32574 - DNA, 28 bp, synthetic construct
  source 1..28: mol_type = other DNA
cagcctggagtgccaccattcagcttgg

SEQ ID NO: 32575 - DNA, 28 bp, synthetic construct
  source 1..28: mol_type = other DNA
taaccaagctgaatggtggcactccagg

SEQ ID NO: 32576 - DNA, 28 bp, synthetic construct
  source 1..28: mol_type = other DNA
gccaccattcagcttggttaacacccgg

SEQ ID NO: 32577 - DNA, 28 bp, synthetic construct
  source 1..28: mol_type = other DNA
gccgggtgttaaccaagctgaatggtgg

SEQ ID NO: 32578 - DNA, 28 bp, synthetic construct
  source 1..28: mol_type = other DNA
tgtgccgggtgttaaccaagctgaatgg

SEQ ID NO: 32579 - DNA, 28 bp, synthetic construct
  source 1..28: mol_type = other DNA
tggttaacacccggcacagtccaccagg

SEQ ID NO: 32580 - DNA, 28 bp, synthetic construct
  source 1..28: mol_type = other DNA
taacagttacctggtggactgtgccggg

SEQ ID NO: 32581 - DNA, 28 bp, synthetic construct
  source 1..28: mol_type = other DNA
gtaacagttacctggtggactgtgccgg

SEQ ID NO: 32582 - DNA, 28 bp, synthetic construct
  source 1..28: mol_type = other DNA
ggtgacactggtaacagttacctggtgg

SEQ ID NO: 32583 - DNA, 28 bp, synthetic construct
  source 1..28: mol_type = other DNA
ggaggtgacactggtaacagttacctgg

SEQ ID NO: 32584 - DNA, 28 bp, synthetic construct
  source 1..28: mol_type = other DNA
taactgttaccagtgtcacctccaaagg

SEQ ID NO: 32585 - DNA, 28 bp, synthetic construct
  source 1..28: mol_type = other DNA
tgtcatcatcctttggaggtgacactgg

SEQ ID NO: 32586 - DNA, 28 bp, synthetic construct
  source 1..28: mol_type = other DNA
tctcttttatgtcatcatcctttggagg

SEQ ID NO: 32587 - DNA, 28 bp, synthetic construct
  source 1..28: mol_type = other DNA
gattctcttttatgtcatcatcctttgg

SEQ ID NO: 32588 - DNA, 28 bp, synthetic construct
  source 1..28: mol_type = other DNA
agcagtgatgaagaggagaatgaacagg

SEQ ID NO: 32589 - DNA, 28 bp, synthetic construct
  source 1..28: mol_type = other DNA
ctcctcttcatcactgcttagcttaagg

SEQ ID NO: 32590 - DNA, 28 bp, synthetic construct
  source 1..28: mol_type = other DNA
gaccttaagctaagcagtgatgaagagg

SEQ ID NO: 32591 - DNA, 28 bp, synthetic construct
  source 1..28: mol_type = other DNA
ggtcatcttccagcattctgaaagaagg

SEQ ID NO: 32592 - DNA, 28 bp, synthetic construct
  source 1..28: mol_type = other DNA
ctctttgttccttctttcagaatgctgg

SEQ ID NO: 32593 - DNA, 28 bp, synthetic construct
  source 1..28: mol_type = other DNA
cagcattctgaaagaaggaacaaagagg

SEQ ID NO: 32594 - DNA, 28 bp, synthetic construct
  source 1..28: mol_type = other DNA
aaagaaggaacaaagaggtacaaagagg

SEQ ID NO: 32595 - DNA, 28 bp, synthetic construct
  source 1..28: mol_type = other DNA
ggtacaaagaggtacagatagttagtgg

SEQ ID NO: 32596 - DNA, 28 bp, synthetic construct
  source 1..28: mol_type = other DNA
taataacaacattaaggtgatattttgg

SEQ ID NO: 32597 - DNA, 28 bp, synthetic construct
  source 1..28: mol_type = other DNA
aaatgttgctctaataacaacattaagg

SEQ ID NO: 32598 - DNA, 28 bp, synthetic construct
  source 1..28: mol_type = other DNA
taatgttgttattagagcaacattttgg

SEQ ID NO: 32599 - DNA, 28 bp, synthetic construct
  source 1..28: mol_type = other DNA
tgcataagaaggaaagaaaaaaaatagg

SEQ ID NO: 32600 - DNA, 28 bp, synthetic construct
  source 1..28: mol_type = other DNA
ctttccttcttatgcacttttcctctgg

SEQ ID NO: 32601 - DNA, 28 bp, synthetic construct
  source 1..28: mol_type = other DNA
tgcaccagaggaaaagtgcataagaagg

SEQ ID NO: 32602 - DNA, 28 bp, synthetic construct
  source 1..28: mol_type = other DNA
tatgcacttttcctctggtgcacttagg

SEQ ID NO: 32603 - DNA, 28 bp, synthetic construct
  source 1..28: mol_type = other DNA
gtctactatttcctaagtgcaccagagg

SEQ ID NO: 32604 - DNA, 28 bp, synthetic construct
  source 1..28: mol_type = other DNA
gttgtgagggttaatttttatgatgggg

SEQ ID NO: 32605 - DNA, 28 bp, synthetic construct
  source 1..28: mol_type = other DNA
tgttgtgagggttaatttttatgatggg

SEQ ID NO: 32606 - DNA, 28 bp, synthetic construct
  source 1..28: mol_type = other DNA
ctgttgtgagggttaatttttatgatgg

SEQ ID NO: 32607 - DNA, 28 bp, synthetic construct
  source 1..28: mol_type = other DNA
ccgtcttagctgatgactgttgtgaggg

SEQ ID NO: 32608 - DNA, 28 bp, synthetic construct
  source 1..28: mol_type = other DNA
cctcacaacagtcatcagctaagacggg

SEQ ID NO: 32609 - DNA, 28 bp, synthetic construct
  source 1..28: mol_type = other DNA
agctttcagaagatgctgtgttagcagg

SEQ ID NO: 32610 - DNA, 28 bp, synthetic construct
  source 1..28: mol_type = other DNA
gctttcagaagatgctgtgttagcaggg

SEQ ID NO: 32611 - DNA, 28 bp, synthetic construct
  source 1..28: mol_type = other DNA
tattgtatatttcgaaatagctagaagg

SEQ ID NO: 32612 - DNA, 28 bp, synthetic construct
  source 1..28: mol_type = other DNA
attgtatatttcgaaatagctagaaggg

SEQ ID NO: 32613 - DNA, 28 bp, synthetic construct
  source 1..28: mol_type = other DNA
ttcgaaatagctagaagggaagaattgg

SEQ ID NO: 32614 - DNA, 28 bp, synthetic construct
  source 1..28: mol_type = other DNA
agggaagaattggaatgttcccaacagg

SEQ ID NO: 32615 - DNA, 28 bp, synthetic construct
  source 1..28: mol_type = other DNA
caaatatttatcttttcttcctgttggg

SEQ ID NO: 32616 - DNA, 28 bp, synthetic construct
  source 1..28: mol_type = other DNA
tcaaatatttatcttttcttcctgttgg

SEQ ID NO: 32617 - DNA, 28 bp, synthetic construct
  source 1..28: mol_type = other DNA
aacaggaagaaaagataaatatttgagg

SEQ ID NO: 32618 - DNA, 28 bp, synthetic construct
  source 1..28: mol_type = other DNA
gtgtaatgatcaaatcagggtaactagg

SEQ ID NO: 32619 - DNA, 28 bp, synthetic construct
  source 1..28: mol_type = other DNA
gattcaatgtgtaatgatcaaatcaggg

SEQ ID NO: 32620 - DNA, 28 bp, synthetic construct
  source 1..28: mol_type = other DNA
ggattcaatgtgtaatgatcaaatcagg

SEQ ID NO: 32621 - DNA, 28 bp, synthetic construct
  source 1..28: mol_type = other DNA
caggtacgtgtgatattttgatacaggg

SEQ ID NO: 32622 - DNA, 28 bp, synthetic construct
  source 1..28: mol_type = other DNA
tcaggtacgtgtgatattttgatacagg

SEQ ID NO: 32623 - DNA, 28 bp, synthetic construct
  source 1..28: mol_type = other DNA
catcttcttttttattgctattttcagg

SEQ ID NO: 32624 - DNA, 28 bp, synthetic construct
  source 1..28: mol_type = other DNA
ttttttttttttctctcaaatacatagg

SEQ ID NO: 32625 - DNA, 28 bp, synthetic construct
  source 1..28: mol_type = other DNA
tttttttttttctctcaaatacataggg

SEQ ID NO: 32626 - DNA, 28 bp, synthetic construct
  source 1..28: mol_type = other DNA
ttttttttttctctcaaatacatagggg

SEQ ID NO: 32627 - DNA, 28 bp, synthetic construct
  source 1..28: mol_type = other DNA
ctcaaatacataggggcttttcccctgg

SEQ ID NO: 32628 - DNA, 28 bp, synthetic construct
  source 1..28: mol_type = other DNA
tcaaatacataggggcttttcccctggg

SEQ ID NO: 32629 - DNA, 28 bp, synthetic construct
  source 1..28: mol_type = other DNA
taattgtggaatgcaaactgcccagggg

SEQ ID NO: 32630 - DNA, 28 bp, synthetic construct
  source 1..28: mol_type = other DNA
gtaattgtggaatgcaaactgcccaggg

SEQ ID NO: 32631 - DNA, 28 bp, synthetic construct
  source 1..28: mol_type = other DNA
agtaattgtggaatgcaaactgcccagg

SEQ ID NO: 32632 - DNA, 28 bp, synthetic construct
  source 1..28: mol_type = other DNA
ttggaaaacactaaacaagtaattgtgg

SEQ ID NO: 32633 - DNA, 28 bp, synthetic construct
  source 1..28: mol_type = other DNA
ttagtgttttccaagctcccagtgctgg

SEQ ID NO: 32634 - DNA, 28 bp, synthetic construct
  source 1..28: mol_type = other DNA
tagtgttttccaagctcccagtgctggg

SEQ ID NO: 32635 - DNA, 28 bp, synthetic construct
  source 1..28: mol_type = other DNA
gagacacagcccagcactgggagcttgg

SEQ ID NO: 32636 - DNA, 28 bp, synthetic construct
  source 1..28: mol_type = other DNA
aggcacggagacacagcccagcactggg

SEQ ID NO: 32637 - DNA, 28 bp, synthetic construct
  source 1..28: mol_type = other DNA
caggcacggagacacagcccagcactgg

SEQ ID NO: 32638 - DNA, 28 bp, synthetic construct
  source 1..28: mol_type = other DNA
tgggctgtgtctccgtgcctgccccagg

SEQ ID NO: 32639 - DNA, 28 bp, synthetic construct
  source 1..28: mol_type = other DNA
gggctgtgtctccgtgcctgccccaggg

SEQ ID NO: 32640 - DNA, 28 bp, synthetic construct
  source 1..28: mol_type = other DNA
ggctgtgtctccgtgcctgccccagggg

SEQ ID NO: 32641 - DNA, 28 bp, synthetic construct
  source 1..28: mol_type = other DNA
tccgtgcctgccccaggggctttcatgg

SEQ ID NO: 32642 - DNA, 28 bp, synthetic construct
  source 1..28: mol_type = other DNA
accatgaaagcccctggggcaggcacgg

SEQ ID NO: 32643 - DNA, 28 bp, synthetic construct
  source 1..28: mol_type = other DNA
tctttaccatgaaagcccctggggcagg

SEQ ID NO: 32644 - DNA, 28 bp, synthetic construct
  source 1..28: mol_type = other DNA
tctctctttaccatgaaagcccctgggg

SEQ ID NO: 32645 - DNA, 28 bp, synthetic construct
  source 1..28: mol_type = other DNA
atctctctttaccatgaaagcccctggg

SEQ ID NO: 32646 - DNA, 28 bp, synthetic construct
  source 1..28: mol_type = other DNA
catctctctttaccatgaaagcccctgg

SEQ ID NO: 32647 - DNA, 28 bp, synthetic construct
  source 1..28: mol_type = other DNA
ctcacaactcaagtttatggctttatgg

SEQ ID NO: 32648 - DNA, 28 bp, synthetic construct
  source 1..28: mol_type = other DNA
aagcttcgctcacaactcaagtttatgg

SEQ ID NO: 32649 - DNA, 28 bp, synthetic construct
  source 1..28: mol_type = other DNA
acttgagttgtgagcgaagcttcttagg

SEQ ID NO: 32650 - DNA, 28 bp, synthetic construct
  source 1..28: mol_type = other DNA
ttaggccatccatcagtcaaagagctgg

SEQ ID NO: 32651 - DNA, 28 bp, synthetic construct
  source 1..28: mol_type = other DNA
cttttccagctctttgactgatggatgg

SEQ ID NO: 32652 - DNA, 28 bp, synthetic construct
  source 1..28: mol_type = other DNA
acatcttttccagctctttgactgatgg

SEQ ID NO: 32653 - DNA, 28 bp, synthetic construct
  source 1..28: mol_type = other DNA
atgttgtccccaagatcctacctagtgg

SEQ ID NO: 32654 - DNA, 28 bp, synthetic construct
  source 1..28: mol_type = other DNA
tgttgtccccaagatcctacctagtggg

SEQ ID NO: 32655 - DNA, 28 bp, synthetic construct
  source 1..28: mol_type = other DNA
gttgtccccaagatcctacctagtgggg

SEQ ID NO: 32656 - DNA, 28 bp, synthetic construct
  source 1..28: mol_type = other DNA
gttttccccactaggtaggatcttgggg

SEQ ID NO: 32657 - DNA, 28 bp, synthetic construct
  source 1..28: mol_type = other DNA
ggttttccccactaggtaggatcttggg

SEQ ID NO: 32658 - DNA, 28 bp, synthetic construct
  source 1..28: mol_type = other DNA
tggttttccccactaggtaggatcttgg

SEQ ID NO: 32659 - DNA, 28 bp, synthetic construct
  source 1..28: mol_type = other DNA
tcctacctagtggggaaaaccaagcagg

SEQ ID NO: 32660 - DNA, 28 bp, synthetic construct
  source 1..28: mol_type = other DNA
tcctgcttggttttccccactaggtagg

SEQ ID NO: 32661 - DNA, 28 bp, synthetic construct
  source 1..28: mol_type = other DNA
tacctagtggggaaaaccaagcaggagg

SEQ ID NO: 32662 - DNA, 28 bp, synthetic construct
  source 1..28: mol_type = other DNA
acctagtggggaaaaccaagcaggaggg

SEQ ID NO: 32663 - DNA, 28 bp, synthetic construct
  source 1..28: mol_type = other DNA
gccctcctgcttggttttccccactagg

SEQ ID NO: 32664 - DNA, 28 bp, synthetic construct
  source 1..28: mol_type = other DNA
gcttttcagaaagcgccctcctgcttgg

SEQ ID NO: 32665 - DNA, 28 bp, synthetic construct
  source 1..28: mol_type = other DNA
agggcgctttctgaaaagcctgtgaagg

SEQ ID NO: 32666 - DNA, 28 bp, synthetic construct
  source 1..28: mol_type = other DNA
gggtgggctggggaatcaccttcacagg

SEQ ID NO: 32667 - DNA, 28 bp, synthetic construct
  source 1..28: mol_type = other DNA
gtgaaggtgattccccagcccacccagg

SEQ ID NO: 32668 - DNA, 28 bp, synthetic construct
  source 1..28: mol_type = other DNA
tgaatggggggacctgggtgggctgggg

SEQ ID NO: 32669 - DNA, 28 bp, synthetic construct
  source 1..28: mol_type = other DNA
atgaatggggggacctgggtgggctggg

SEQ ID NO: 32670 - DNA, 28 bp, synthetic construct
  source 1..28: mol_type = other DNA
gatgaatggggggacctgggtgggctgg

SEQ ID NO: 32671 - DNA, 28 bp, synthetic construct
  source 1..28: mol_type = other DNA
tcaggatgaatggggggacctgggtggg

SEQ ID NO: 32672 - DNA, 28 bp, synthetic construct
  source 1..28: mol_type = other DNA
ctcaggatgaatggggggacctgggtgg

SEQ ID NO: 32673 - DNA, 28 bp, synthetic construct
  source 1..28: mol_type = other DNA
cacccaggtccccccattcatcctgagg

SEQ ID NO: 32674 - DNA, 28 bp, synthetic construct
  source 1..28: mol_type = other DNA
ctcctcaggatgaatggggggacctggg

SEQ ID NO: 32675 - DNA, 28 bp, synthetic construct
  source 1..28: mol_type = other DNA
tctcctcaggatgaatggggggacctgg

SEQ ID NO: 32676 - DNA, 28 bp, synthetic construct
  source 1..28: mol_type = other DNA
ccgctgtctcctcaggatgaatgggggg

SEQ ID NO: 32677 - DNA, 28 bp, synthetic construct
  source 1..28: mol_type = other DNA
cccgctgtctcctcaggatgaatggggg

SEQ ID NO: 32678 - DNA, 28 bp, synthetic construct
  source 1..28: mol_type = other DNA
ccccgctgtctcctcaggatgaatgggg

SEQ ID NO: 32679 - DNA, 28 bp, synthetic construct
  source 1..28: mol_type = other DNA
tccccgctgtctcctcaggatgaatggg

SEQ ID NO: 32680 - DNA, 28 bp, synthetic construct
  source 1..28: mol_type = other DNA
ttccccgctgtctcctcaggatgaatgg

SEQ ID NO: 32681 - DNA, 28 bp, synthetic construct
  source 1..28: mol_type = other DNA
cctcgtgcttccccgctgtctcctcagg

SEQ ID NO: 32682 - DNA, 28 bp, synthetic construct
  source 1..28: mol_type = other DNA
tgataacactgtattcttttcagcatgg

SEQ ID NO: 32683 - DNA, 28 bp, synthetic construct
  source 1..28: mol_type = other DNA
gtgctctccacgcagagacgctctgagg

SEQ ID NO: 32684 - DNA, 28 bp, synthetic construct
  source 1..28: mol_type = other DNA
tgctctccacgcagagacgctctgaggg

SEQ ID NO: 32685 - DNA, 28 bp, synthetic construct
  source 1..28: mol_type = other DNA
ccacgcagagacgctctgagggagcagg

SEQ ID NO: 32686 - DNA, 28 bp, synthetic construct
  source 1..28: mol_type = other DNA
cacgcagagacgctctgagggagcaggg

SEQ ID NO: 32687 - DNA, 28 bp, synthetic construct
  source 1..28: mol_type = other DNA
acgcagagacgctctgagggagcagggg

SEQ ID NO: 32688 - DNA, 28 bp, synthetic construct
  source 1..28: mol_type = other DNA
gggagcaggggagagcccacttctgagg

SEQ ID NO: 32689 - DNA, 28 bp, synthetic construct
  source 1..28: mol_type = other DNA
ggagcaggggagagcccacttctgaggg

SEQ ID NO: 32690 - DNA, 28 bp, synthetic construct
  source 1..28: mol_type = other DNA
gggagagcccacttctgagggaccctgg

SEQ ID NO: 32691 - DNA, 28 bp, synthetic construct
  source 1..28: mol_type = other DNA
ggagagcccacttctgagggaccctggg

SEQ ID NO: 32692 - DNA, 28 bp, synthetic construct
  source 1..28: mol_type = other DNA
gagagcccacttctgagggaccctgggg

SEQ ID NO: 32693 - DNA, 28 bp, synthetic construct
  source 1..28: mol_type = other DNA
tggagccccagggtccctcagaagtggg

SEQ ID NO: 32694 - DNA, 28 bp, synthetic construct
  source 1..28: mol_type = other DNA
atggagccccagggtccctcagaagtgg

SEQ ID NO: 32695 - DNA, 28 bp, synthetic construct
  source 1..28: mol_type = other DNA
cttcacactgatgtatggagccccaggg

SEQ ID NO: 32696 - DNA, 28 bp, synthetic construct
  source 1..28: mol_type = other DNA
gcttcacactgatgtatggagccccagg

SEQ ID NO: 32697 - DNA, 28 bp, synthetic construct
  source 1..28: mol_type = other DNA
gctcagcgggcttcacactgatgtatgg

SEQ ID NO: 32698 - DNA, 28 bp, synthetic construct
  source 1..28: mol_type = other DNA
aagcccgctgagcccttgtgctcaaagg

SEQ ID NO: 32699 - DNA, 28 bp, synthetic construct
  source 1..28: mol_type = other DNA
aggcctttgagcacaagggctcagcggg

SEQ ID NO: 32700 - DNA, 28 bp, synthetic construct
  source 1..28: mol_type = other DNA
gaggcctttgagcacaagggctcagcgg

SEQ ID NO: 32701 - DNA, 28 bp, synthetic construct
  source 1..28: mol_type = other DNA
gcttcaatgaggcctttgagcacaaggg

SEQ ID NO: 32702 - DNA, 28 bp, synthetic construct
  source 1..28: mol_type = other DNA
ggcttcaatgaggcctttgagcacaagg

SEQ ID NO: 32703 - DNA, 28 bp, synthetic construct
  source 1..28: mol_type = other DNA
aggcctcattgaagccagcttccaaagg

SEQ ID NO: 32704 - DNA, 28 bp, synthetic construct
  source 1..28: mol_type = other DNA
cagcctttggaagctggcttcaatgagg

SEQ ID NO: 32705 - DNA, 28 bp, synthetic construct
  source 1..28: mol_type = other DNA
attttaggggacagcctttggaagctgg

SEQ ID NO: 32706 - DNA, 28 bp, synthetic construct
  source 1..28: mol_type = other DNA
taggtacattttaggggacagcctttgg

SEQ ID NO: 32707 - DNA, 28 bp, synthetic construct
  source 1..28: mol_type = other DNA
ttaaaggacactaggtacattttagggg

SEQ ID NO: 32708 - DNA, 28 bp, synthetic construct
  source 1..28: mol_type = other DNA
tttaaaggacactaggtacattttaggg

SEQ ID NO: 32709 - DNA, 28 bp, synthetic construct
  source 1..28: mol_type = other DNA
ttttaaaggacactaggtacattttagg

SEQ ID NO: 32710 - DNA, 28 bp, synthetic construct
  source 1..28: mol_type = other DNA
aatgtacctagtgtcctttaaaagccgg

SEQ ID NO: 32711 - DNA, 28 bp, synthetic construct
  source 1..28: mol_type = other DNA
ctacaaccggcttttaaaggacactagg

SEQ ID NO: 32712 - DNA, 28 bp, synthetic construct
  source 1..28: mol_type = other DNA
ctagtgtcctttaaaagccggttgtagg

SEQ ID NO: 32713 - DNA, 28 bp, synthetic construct
  source 1..28: mol_type = other DNA
tgataggcctacaaccggcttttaaagg

SEQ ID NO: 32714 - DNA, 28 bp, synthetic construct
  source 1..28: mol_type = other DNA
catgtatcagtgataggcctacaaccgg

SEQ ID NO: 32715 - DNA, 28 bp, synthetic construct
  source 1..28: mol_type = other DNA
atgttcagaggcatgtatcagtgatagg

SEQ ID NO: 32716 - DNA, 28 bp, synthetic construct
  source 1..28: mol_type = other DNA
ctgatacatgcctctgaacattcgtagg

SEQ ID NO: 32717 - DNA, 28 bp, synthetic construct
  source 1..28: mol_type = other DNA
tgaaatgactcctacgaatgttcagagg

SEQ ID NO: 32718 - DNA, 28 bp, synthetic construct
  source 1..28: mol_type = other DNA
tcgtaggagtcatttcagtcacttttgg

SEQ ID NO: 32719 - DNA, 28 bp, synthetic construct
  source 1..28: mol_type = other DNA
cgtaggagtcatttcagtcacttttggg

SEQ ID NO: 32720 - DNA, 28 bp, synthetic construct
  source 1..28: mol_type = other DNA
gtaggagtcatttcagtcacttttgggg

SEQ ID NO: 32721 - DNA, 28 bp, synthetic construct
  source 1..28: mol_type = other DNA
catttcagtcacttttggggcgaactgg

SEQ ID NO: 32722 - DNA, 28 bp, synthetic construct
  source 1..28: mol_type = other DNA
atttcagtcacttttggggcgaactggg

SEQ ID NO: 32723 - DNA, 28 bp, synthetic construct
  source 1..28: mol_type = other DNA
tttcagtcacttttggggcgaactgggg

SEQ ID NO: 32724 - DNA, 28 bp, synthetic construct
  source 1..28: mol_type = other DNA
ttcagtcacttttggggcgaactggggg

SEQ ID NO: 32725 - DNA, 28 bp, synthetic construct
  source 1..28: mol_type = other DNA
tcagtcacttttggggcgaactgggggg

SEQ ID NO: 32726 - DNA, 28 bp, synthetic construct
  source 1..28: mol_type = other DNA
tggggcgaactggggggtaaagaactgg

SEQ ID NO: 32727 - DNA, 28 bp, synthetic construct
  source 1..28: mol_type = other DNA
gcgaactggggggtaaagaactggcagg

SEQ ID NO: 32728 - DNA, 28 bp, synthetic construct
  source 1..28: mol_type = other DNA
tggggggtaaagaactggcaggataagg

SEQ ID NO: 32729 - DNA, 28 bp, synthetic construct
  source 1..28: mol_type = other DNA
ggtaaagaactggcaggataaggcatgg

SEQ ID NO: 32730 - DNA, 28 bp, synthetic construct
  source 1..28: mol_type = other DNA
gaactggcaggataaggcatggcccagg

SEQ ID NO: 32731 - DNA, 28 bp, synthetic construct
  source 1..28: mol_type = other DNA
tgcatagacaggtggggcagagcctggg

SEQ ID NO: 32732 - DNA, 28 bp, synthetic construct
  source 1..28: mol_type = other DNA
atgcatagacaggtggggcagagcctgg

SEQ ID NO: 32733 - DNA, 28 bp, synthetic construct
  source 1..28: mol_type = other DNA
gctctgccccacctgtctatgcatgtgg

SEQ ID NO: 32734 - DNA, 28 bp, synthetic construct
  source 1..28: mol_type = other DNA
ctctgccccacctgtctatgcatgtggg

SEQ ID NO: 32735 - DNA, 28 bp, synthetic construct
  source 1..28: mol_type = other DNA
tctgccccacctgtctatgcatgtgggg

SEQ ID NO: 32736 - DNA, 28 bp, synthetic construct
  source 1..28: mol_type = other DNA
ctcaccccacatgcatagacaggtgggg

SEQ ID NO: 32737 - DNA, 28 bp, synthetic construct
  source 1..28: mol_type = other DNA
actcaccccacatgcatagacaggtggg

SEQ ID NO: 32738 - DNA, 28 bp, synthetic construct
  source 1..28: mol_type = other DNA
gactcaccccacatgcatagacaggtgg

SEQ ID NO: 32739 - DNA, 28 bp, synthetic construct
  source 1..28: mol_type = other DNA
agcgactcaccccacatgcatagacagg

SEQ ID NO: 32740 - DNA, 28 bp, synthetic construct
  source 1..28: mol_type = other DNA
ctgcacaaatagggaaatggggtcaggg

SEQ ID NO: 32741 - DNA, 28 bp, synthetic construct
  source 1..28: mol_type = other DNA
actgcacaaatagggaaatggggtcagg

SEQ ID NO: 32742 - DNA, 28 bp, synthetic construct
  source 1..28: mol_type = other DNA
acgtcactgcacaaatagggaaatgggg

SEQ ID NO: 32743 - DNA, 28 bp, synthetic construct
  source 1..28: mol_type = other DNA
cacgtcactgcacaaatagggaaatggg

SEQ ID NO: 32744 - DNA, 28 bp, synthetic construct
  source 1..28: mol_type = other DNA
acacgtcactgcacaaatagggaaatgg

SEQ ID NO: 32745 - DNA, 28 bp, synthetic construct
  source 1..28: mol_type = other DNA
tctataacacgtcactgcacaaataggg

SEQ ID NO: 32746 - DNA, 28 bp, synthetic construct
  source 1..28: mol_type = other DNA
ctctataacacgtcactgcacaaatagg

SEQ ID NO: 32747 - DNA, 28 bp, synthetic construct
  source 1..28: mol_type = other DNA
ctatttgtgcagtgacgtgttatagagg

SEQ ID NO: 32748 - DNA, 28 bp, synthetic construct
  source 1..28: mol_type = other DNA
tatttgtgcagtgacgtgttatagaggg

SEQ ID NO: 32749 - DNA, 28 bp, synthetic construct
  source 1..28: mol_type = other DNA
tgacgtgttatagagggcaatcctaagg

SEQ ID NO: 32750 - DNA, 28 bp, synthetic construct
  source 1..28: mol_type = other DNA
ggaatctaaagcaggattcaaccttagg

SEQ ID NO: 32751 - DNA, 28 bp, synthetic construct
  source 1..28: mol_type = other DNA
gtagactcacaacggaatctaaagcagg

SEQ ID NO: 32752 - DNA, 28 bp, synthetic construct
  source 1..28: mol_type = other DNA
gcttcactctccccccatcttccattgg

SEQ ID NO: 32753 - DNA, 28 bp, synthetic construct
  source 1..28: mol_type = other DNA
cattcttattccaatggaagatgggggg

SEQ ID NO: 32754 - DNA, 28 bp, synthetic construct
  source 1..28: mol_type = other DNA
gcattcttattccaatggaagatggggg

SEQ ID NO: 32755 - DNA, 28 bp, synthetic construct
  source 1..28: mol_type = other DNA
agcattcttattccaatggaagatgggg

SEQ ID NO: 32756 - DNA, 28 bp, synthetic construct
  source 1..28: mol_type = other DNA
aagcattcttattccaatggaagatggg

SEQ ID NO: 32757 - DNA, 28 bp, synthetic construct
  source 1..28: mol_type = other DNA
caagcattcttattccaatggaagatgg

SEQ ID NO: 32758 - DNA, 28 bp, synthetic construct
  source 1..28: mol_type = other DNA
cttccattggaataagaatgcttgaagg

SEQ ID NO: 32759 - DNA, 28 bp, synthetic construct
  source 1..28: mol_type = other DNA
ttccattggaataagaatgcttgaaggg

SEQ ID NO: 32760 - DNA, 28 bp, synthetic construct
  source 1..28: mol_type = other DNA
ttcccttcaagcattcttattccaatgg

SEQ ID NO: 32761 - DNA, 28 bp, synthetic construct
  source 1..28: mol_type = other DNA
attggaataagaatgcttgaagggaagg

SEQ ID NO: 32762 - DNA, 28 bp, synthetic construct
  source 1..28: mol_type = other DNA
ttggaataagaatgcttgaagggaaggg

SEQ ID NO: 32763 - DNA, 28 bp, synthetic construct
  source 1..28: mol_type = other DNA
tggaataagaatgcttgaagggaagggg

SEQ ID NO: 32764 - DNA, 28 bp, synthetic construct
  source 1..28: mol_type = other DNA
gaaggggtgtgtttcctcaacgcctagg

SEQ ID NO: 32765 - DNA, 28 bp, synthetic construct
  source 1..28: mol_type = other DNA
gtgtgtttcctcaacgcctaggataagg

SEQ ID NO: 32766 - DNA, 28 bp, synthetic construct
  source 1..28: mol_type = other DNA
ggcttatgccttatcctaggcgttgagg

SEQ ID NO: 32767 - DNA, 28 bp, synthetic construct
  source 1..28: mol_type = other DNA
taatgatgggcttatgccttatcctagg

SEQ ID NO: 32768 - DNA, 28 bp, synthetic construct
  source 1..28: mol_type = other DNA
ataaggcataagcccatcattactaagg

SEQ ID NO: 32769 - DNA, 28 bp, synthetic construct
  source 1..28: mol_type = other DNA
ctcgtggtaattccttagtaatgatggg

SEQ ID NO: 32770 - DNA, 28 bp, synthetic construct
  source 1..28: mol_type = other DNA
cctcgtggtaattccttagtaatgatgg

SEQ ID NO: 32771 - DNA, 28 bp, synthetic construct
  source 1..28: mol_type = other DNA
tactgaagaattctaaaatgcctcgtgg

SEQ ID NO: 32772 - DNA, 28 bp, synthetic construct
  source 1..28: mol_type = other DNA
tcagtagttgttttgagaaaccacaagg

SEQ ID NO: 32773 - DNA, 28 bp, synthetic construct
  source 1..28: mol_type = other DNA
gttttgagaaaccacaaggcagcgctgg

SEQ ID NO: 32774 - DNA, 28 bp, synthetic construct
  source 1..28: mol_type = other DNA
ttttgagaaaccacaaggcagcgctggg

SEQ ID NO: 32775 - DNA, 28 bp, synthetic construct
  source 1..28: mol_type = other DNA
tttgagaaaccacaaggcagcgctgggg

SEQ ID NO: 32776 - DNA, 28 bp, synthetic construct
  source 1..28: mol_type = other DNA
tctcagattccccagcgctgccttgtgg

SEQ ID NO: 32777 - DNA, 28 bp, synthetic construct
  source 1..28: mol_type = other DNA
gagattccagcttgttcttcagccttgg

SEQ ID NO: 32778 - DNA, 28 bp, synthetic construct
  source 1..28: mol_type = other DNA
agattccagcttgttcttcagccttggg

SEQ ID NO: 32779 - DNA, 28 bp, synthetic construct
  source 1..28: mol_type = other DNA
gattccagcttgttcttcagccttgggg

SEQ ID NO: 32780 - DNA, 28 bp, synthetic construct
  source 1..28: mol_type = other DNA
tccagcttgttcttcagccttggggagg

SEQ ID NO: 32781 - DNA, 28 bp, synthetic construct
  source 1..28: mol_type = other DNA
tcctccccaaggctgaagaacaagctgg

SEQ ID NO: 32782 - DNA, 28 bp, synthetic construct
  source 1..28: mol_type = other DNA
cataaaattttctgtttcctccccaagg

SEQ ID NO: 32783 - DNA, 28 bp, synthetic construct
  source 1..28: mol_type = other DNA
tgaatgccacacctttcaagctccctgg

SEQ ID NO: 32784 - DNA, 28 bp, synthetic construct
  source 1..28: mol_type = other DNA
acttctccagggagcttgaaaggtgtgg

SEQ ID NO: 32785 - DNA, 28 bp, synthetic construct
  source 1..28: mol_type = other DNA
tggggacttctccagggagcttgaaagg

SEQ ID NO: 32786 - DNA, 28 bp, synthetic construct
  source 1..28: mol_type = other DNA
tgacgaaagtgtggggacttctccaggg

SEQ ID NO: 32787 - DNA, 28 bp, synthetic construct
  source 1..28: mol_type = other DNA
ttgacgaaagtgtggggacttctccagg

SEQ ID NO: 32788 - DNA, 28 bp, synthetic construct
  source 1..28: mol_type = other DNA
ccccacactttcgtcaagactgcatagg

SEQ ID NO: 32789 - DNA, 28 bp, synthetic construct
  source 1..28: mol_type = other DNA
tcctatgcagtcttgacgaaagtgtggg

SEQ ID NO: 32790 - DNA, 28 bp, synthetic construct
  source 1..28: mol_type = other DNA
atcctatgcagtcttgacgaaagtgtgg

SEQ ID NO: 32791 - DNA, 28 bp, synthetic construct
  source 1..28: mol_type = other DNA
gtcaagactgcataggatagtgtgctgg

SEQ ID NO: 32792 - DNA, 28 bp, synthetic construct
  source 1..28: mol_type = other DNA
tcaagactgcataggatagtgtgctggg

SEQ ID NO: 32793 - DNA, 28 bp, synthetic construct
  source 1..28: mol_type = other DNA
atagtgtgctgggttttctgtctagtgg

SEQ ID NO: 32794 - DNA, 28 bp, synthetic construct
  source 1..28: mol_type = other DNA
ctgggttttctgtctagtggcaacttgg

SEQ ID NO: 32795 - DNA, 28 bp, synthetic construct
  source 1..28: mol_type = other DNA
tgtgatagaaaggagtgcttcaaagggg

SEQ ID NO: 32796 - DNA, 28 bp, synthetic construct
  source 1..28: mol_type = other DNA
ctgtgatagaaaggagtgcttcaaaggg

SEQ ID NO: 32797 - DNA, 28 bp, synthetic construct
  source 1..28: mol_type = other DNA
cctttgaagcactcctttctatcacagg

SEQ ID NO: 32798 - DNA, 28 bp, synthetic construct
  source 1..28: mol_type = other DNA
ctttgaagcactcctttctatcacaggg

SEQ ID NO: 32799 - DNA, 28 bp, synthetic construct
  source 1..28: mol_type = other DNA
tttgaagcactcctttctatcacagggg

SEQ ID NO: 32800 - DNA, 28 bp, synthetic construct
  source 1..28: mol_type = other DNA
aagcactcctttctatcacaggggctgg

SEQ ID NO: 32801 - DNA, 28 bp, synthetic construct
  source 1..28: mol_type = other DNA
cactcctttctatcacaggggctggagg

SEQ ID NO: 32802 - DNA, 28 bp, synthetic construct
  source 1..28: mol_type = other DNA
caggcctccagcccctgtgatagaaagg

SEQ ID NO: 32803 - DNA, 28 bp, synthetic construct
  source 1..28: mol_type = other DNA
ctttctatcacaggggctggaggcctgg

SEQ ID NO: 32804 - DNA, 28 bp, synthetic construct
  source 1..28: mol_type = other DNA
tttctatcacaggggctggaggcctggg

SEQ ID NO: 32805 - DNA, 28 bp, synthetic construct
  source 1..28: mol_type = other DNA
gggattctggggaaatgtagttcccagg

SEQ ID NO: 32806 - DNA, 28 bp, synthetic construct
  source 1..28: mol_type = other DNA
acatttccccagaatccctgccgatagg

SEQ ID NO: 32807 - DNA, 28 bp, synthetic construct
  source 1..28: mol_type = other DNA
catttccccagaatccctgccgataggg

SEQ ID NO: 32808 - DNA, 28 bp, synthetic construct
  source 1..28: mol_type = other DNA
aaaaaccctatcggcagggattctgggg

SEQ ID NO: 32809 - DNA, 28 bp, synthetic construct
  source 1..28: mol_type = other DNA
caaaaaccctatcggcagggattctggg

SEQ ID NO: 32810 - DNA, 28 bp, synthetic construct
  source 1..28: mol_type = other DNA
ccagaatccctgccgatagggtttttgg

SEQ ID NO: 32811 - DNA, 28 bp, synthetic construct
  source 1..28: mol_type = other DNA
catttaaccaaaaaccctatcggcaggg

SEQ ID NO: 32812 - DNA, 28 bp, synthetic construct
  source 1..28: mol_type = other DNA
acatttaaccaaaaaccctatcggcagg

SEQ ID NO: 32813 - DNA, 28 bp, synthetic construct
  source 1..28: mol_type = other DNA
ggcaacatttaaccaaaaaccctatcgg

SEQ ID NO: 32814 - DNA, 28 bp, synthetic construct
  source 1..28: mol_type = other DNA
tttttggttaaatgttgccagtgagagg

SEQ ID NO: 32815 - DNA, 28 bp, synthetic construct
  source 1..28: mol_type = other DNA
tgttgccagtgagaggcacctgaatagg

SEQ ID NO: 32816 - DNA, 28 bp, synthetic construct
  source 1..28: mol_type = other DNA
gttgccagtgagaggcacctgaataggg

SEQ ID NO: 32817 - DNA, 28 bp, synthetic construct
  source 1..28: mol_type = other DNA
caagccctattcaggtgcctctcactgg

SEQ ID NO: 32818 - DNA, 28 bp, synthetic construct
  source 1..28: mol_type = other DNA
cagtgagaggcacctgaatagggcttgg

SEQ ID NO: 32819 - DNA, 28 bp, synthetic construct
  source 1..28: mol_type = other DNA
atctttgattttccaagccctattcagg

SEQ ID NO: 32820 - DNA, 28 bp, synthetic construct
  source 1..28: mol_type = other DNA
attaacagaagcctttactactcccagg

SEQ ID NO: 32821 - DNA, 28 bp, synthetic construct
  source 1..28: mol_type = other DNA
tgcttcactgtcctgggagtagtaaagg

SEQ ID NO: 32822 - DNA, 28 bp, synthetic construct
  source 1..28: mol_type = other DNA
tttactactcccaggacagtgaagcagg

SEQ ID NO: 32823 - DNA, 28 bp, synthetic construct
  source 1..28: mol_type = other DNA
gcttctgcacctgcttcactgtcctggg

SEQ ID NO: 32824 - DNA, 28 bp, synthetic construct
  source 1..28: mol_type = other DNA
agcttctgcacctgcttcactgtcctgg

SEQ ID NO: 32825 - DNA, 28 bp, synthetic construct
  source 1..28: mol_type = other DNA
aagcaggtgcagaagcttcagcagatgg

SEQ ID NO: 32826 - DNA, 28 bp, synthetic construct
  source 1..28: mol_type = other DNA
gaagcttcagcagatggcagatacgagg

SEQ ID NO: 32827 - DNA, 28 bp, synthetic construct
  source 1..28: mol_type = other DNA
gatggcagatacgaggttctgtgagtgg

SEQ ID NO: 32828 - DNA, 28 bp, synthetic construct
  source 1..28: mol_type = other DNA
atacgaggttctgtgagtggcttccagg

SEQ ID NO: 32829 - DNA, 28 bp, synthetic construct
  source 1..28: mol_type = other DNA
caggcattattcacagaagggtgcctgg

SEQ ID NO: 32830 - DNA, 28 bp, synthetic construct
  source 1..28: mol_type = other DNA
gcacccttctgtgaataatgcctgctgg

SEQ ID NO: 32831 - DNA, 28 bp, synthetic construct
  source 1..28: mol_type = other DNA
tctccagcaggcattattcacagaaggg

SEQ ID NO: 32832 - DNA, 28 bp, synthetic construct
  source 1..28: mol_type = other DNA
gtctccagcaggcattattcacagaagg

SEQ ID NO: 32833 - DNA, 28 bp, synthetic construct
  source 1..28: mol_type = other DNA
aacagtaatctcagatgtctccagcagg

SEQ ID NO: 32834 - DNA, 28 bp, synthetic construct
  source 1..28: mol_type = other DNA
ttcttgaaatgactttctgaactgatgg

SEQ ID NO: 32835 - DNA, 28 bp, synthetic construct
  source 1..28: mol_type = other DNA
tctgaactgatggctgatttcctgttgg

SEQ ID NO: 32836 - DNA, 28 bp, synthetic construct
  source 1..28: mol_type = other DNA
tgatttcctgttggtcccccttccctgg

SEQ ID NO: 32837 - DNA, 28 bp, synthetic construct
  source 1..28: mol_type = other DNA
ggagggccagggaagggggaccaacagg

SEQ ID NO: 32838 - DNA, 28 bp, synthetic construct
  source 1..28: mol_type = other DNA
ggtcccccttccctggccctcctgatgg

SEQ ID NO: 32839 - DNA, 28 bp, synthetic construct
  source 1..28: mol_type = other DNA
gtcccccttccctggccctcctgatggg

SEQ ID NO: 32840 - DNA, 28 bp, synthetic construct
  source 1..28: mol_type = other DNA
aacccatcaggagggccagggaaggggg

SEQ ID NO: 32841 - DNA, 28 bp, synthetic construct
  source 1..28: mol_type = other DNA
aaacccatcaggagggccagggaagggg

SEQ ID NO: 32842 - DNA, 28 bp, synthetic construct
  source 1..28: mol_type = other DNA
caaacccatcaggagggccagggaaggg

SEQ ID NO: 32843 - DNA, 28 bp, synthetic construct
  source 1..28: mol_type = other DNA
ccttccctggccctcctgatgggtttgg

SEQ ID NO: 32844 - DNA, 28 bp, synthetic construct
  source 1..28: mol_type = other DNA
ccctggccctcctgatgggtttggaagg

SEQ ID NO: 32845 - DNA, 28 bp, synthetic construct
  source 1..28: mol_type = other DNA
gccttccaaacccatcaggagggccagg

SEQ ID NO: 32846 - DNA, 28 bp, synthetic construct
  source 1..28: mol_type = other DNA
ttagtgccttccaaacccatcaggaggg

SEQ ID NO: 32847 - DNA, 28 bp, synthetic construct
  source 1..28: mol_type = other DNA
attagtgccttccaaacccatcaggagg

SEQ ID NO: 32848 - DNA, 28 bp, synthetic construct
  source 1..28: mol_type = other DNA
ggaattagtgccttccaaacccatcagg

SEQ ID NO: 32849 - DNA, 28 bp, synthetic construct
  source 1..28: mol_type = other DNA
gtatttcaagtagacacttaacataggg

SEQ ID NO: 32850 - DNA, 28 bp, synthetic construct
  source 1..28: mol_type = other DNA
ggtatttcaagtagacacttaacatagg

SEQ ID NO: 32851 - DNA, 28 bp, synthetic construct
  source 1..28: mol_type = other DNA
aagtgtctacttgaaatacctagagtgg

SEQ ID NO: 32852 - DNA, 28 bp, synthetic construct
  source 1..28: mol_type = other DNA
tgatctggagaagagaaaccactctagg

SEQ ID NO: 32853 - DNA, 28 bp, synthetic construct
  source 1..28: mol_type = other DNA
actatacacatcagtcagtttgatctgg

SEQ ID NO: 32854 - DNA, 28 bp, synthetic construct
  source 1..28: mol_type = other DNA
gcatgagctctgcagtcagaaagcctgg

SEQ ID NO: 32855 - DNA, 28 bp, synthetic construct
  source 1..28: mol_type = other DNA
gcatctggatagaaatcaataaaccagg

SEQ ID NO: 32856 - DNA, 28 bp, synthetic construct
  source 1..28: mol_type = other DNA
cacaactagcatgaggtacagcatctgg

SEQ ID NO: 32857 - DNA, 28 bp, synthetic construct
  source 1..28: mol_type = other DNA
tttgcataaggacacaactagcatgagg

SEQ ID NO: 32858 - DNA, 28 bp, synthetic construct
  source 1..28: mol_type = other DNA
agagcaactttaagttctttgcataagg

SEQ ID NO: 32859 - DNA, 28 bp, synthetic construct
  source 1..28: mol_type = other DNA
gccttctgtttcctcatctgtaaaatgg

SEQ ID NO: 32860 - DNA, 28 bp, synthetic construct
  source 1..28: mol_type = other DNA
tccattttacagatgaggaaacagaagg

SEQ ID NO: 32861 - DNA, 28 bp, synthetic construct
  source 1..28: mol_type = other DNA
ctctcgtttttccattttacagatgagg

SEQ ID NO: 32862 - DNA, 28 bp, synthetic construct
  source 1..28: mol_type = other DNA
ggaaaaacgagagtgtttacctcctagg

SEQ ID NO: 32863 - DNA, 28 bp, synthetic construct
  source 1..28: mol_type = other DNA
ctacattttctacaacattcctaggagg

SEQ ID NO: 32864 - DNA, 28 bp, synthetic construct
  source 1..28: mol_type = other DNA
tttctacattttctacaacattcctagg

SEQ ID NO: 32865 - DNA, 28 bp, synthetic construct
  source 1..28: mol_type = other DNA
tgtagaaaacattttatacagtgtctgg

SEQ ID NO: 32866 - DNA, 28 bp, synthetic construct
  source 1..28: mol_type = other DNA
attaataaatattcagtattctaactgg

SEQ ID NO: 32867 - DNA, 28 bp, synthetic construct
  source 1..28: mol_type = other DNA
catagttgttgtcacgagatggaatggg

SEQ ID NO: 32868 - DNA, 28 bp, synthetic construct
  source 1..28: mol_type = other DNA
acatagttgttgtcacgagatggaatgg

SEQ ID NO: 32869 - DNA, 28 bp, synthetic construct
  source 1..28: mol_type = other DNA
ttgtaacatagttgttgtcacgagatgg

SEQ ID NO: 32870 - DNA, 28 bp, synthetic construct
  source 1..28: mol_type = other DNA
aaagaaagaaaaagaaaaggaaaaatgg

SEQ ID NO: 32871 - DNA, 28 bp, synthetic construct
  source 1..28: mol_type = other DNA
tcaaaaaaaaagaaagaaaaagaaaagg

SEQ ID NO: 32872 - DNA, 28 bp, synthetic construct
  source 1..28: mol_type = other DNA
cagagtctcactttgttgcccacgctgg

SEQ ID NO: 32873 - DNA, 28 bp, synthetic construct
  source 1..28: mol_type = other DNA
ctttgttgcccacgctggagtgcagtgg

SEQ ID NO: 32874 - DNA, 28 bp, synthetic construct
  source 1..28: mol_type = other DNA
atatcacaccactgcactccagcgtggg

SEQ ID NO: 32875 - DNA, 28 bp, synthetic construct
  source 1..28: mol_type = other DNA
gatatcacaccactgcactccagcgtgg

SEQ ID NO: 32876 - DNA, 28 bp, synthetic construct
  source 1..28: mol_type = other DNA
cagctcactgcagccttgacctcccagg

SEQ ID NO: 32877 - DNA, 28 bp, synthetic construct
  source 1..28: mol_type = other DNA
aggatcacttgagcctgggaggtcaagg

SEQ ID NO: 32878 - DNA, 28 bp, synthetic construct
  source 1..28: mol_type = other DNA
ggcaggaggatcacttgagcctgggagg

SEQ ID NO: 32879 - DNA, 28 bp, synthetic construct
  source 1..28: mol_type = other DNA
tgaggcaggaggatcacttgagcctggg

SEQ ID NO: 32880 - DNA, 28 bp, synthetic construct
  source 1..28: mol_type = other DNA
ctgaggcaggaggatcacttgagcctgg

SEQ ID NO: 32881 - DNA, 28 bp, synthetic construct
  source 1..28: mol_type = other DNA
cagctacttggggggctgaggcaggagg

SEQ ID NO: 32882 - DNA, 28 bp, synthetic construct
  source 1..28: mol_type = other DNA
ctcctgcctcagccccccaagtagctgg

SEQ ID NO: 32883 - DNA, 28 bp, synthetic construct
  source 1..28: mol_type = other DNA
ttccagctacttggggggctgaggcagg

SEQ ID NO: 32884 - DNA, 28 bp, synthetic construct
  source 1..28: mol_type = other DNA
atagttccagctacttggggggctgagg

SEQ ID NO: 32885 - DNA, 28 bp, synthetic construct
  source 1..28: mol_type = other DNA
cagccccccaagtagctggaactatagg

SEQ ID NO: 32886 - DNA, 28 bp, synthetic construct
  source 1..28: mol_type = other DNA
ccccccaagtagctggaactataggtgg

SEQ ID NO: 32887 - DNA, 28 bp, synthetic construct
  source 1..28: mol_type = other DNA
gccacctatagttccagctacttggggg

SEQ ID NO: 32888 - DNA, 28 bp, synthetic construct
  source 1..28: mol_type = other DNA
ggccacctatagttccagctacttgggg

SEQ ID NO: 32889 - DNA, 28 bp, synthetic construct
  source 1..28: mol_type = other DNA
gggccacctatagttccagctacttggg

SEQ ID NO: 32890 - DNA, 28 bp, synthetic construct
  source 1..28: mol_type = other DNA
tgggccacctatagttccagctacttgg

SEQ ID NO: 32891 - DNA, 28 bp, synthetic construct
  source 1..28: mol_type = other DNA
ggaactataggtggcccaccatgcctgg

SEQ ID NO: 32892 - DNA, 28 bp, synthetic construct
  source 1..28: mol_type = other DNA
cccaccatgcctggctaatttttgtagg

SEQ ID NO: 32893 - DNA, 28 bp, synthetic construct
  source 1..28: mol_type = other DNA
ccctacaaaaattagccaggcatggtgg

SEQ ID NO: 32894 - DNA, 28 bp, synthetic construct
  source 1..28: mol_type = other DNA
cgtccctacaaaaattagccaggcatgg

SEQ ID NO: 32895 - DNA, 28 bp, synthetic construct
  source 1..28: mol_type = other DNA
cctctcgtccctacaaaaattagccagg

SEQ ID NO: 32896 - DNA, 28 bp, synthetic construct
  source 1..28: mol_type = other DNA
gacgagaggttttgttatgttgcccagg

SEQ ID NO: 32897 - DNA, 28 bp, synthetic construct
  source 1..28: mol_type = other DNA
agaggttttgttatgttgcccaggctgg

SEQ ID NO: 32898 - DNA, 28 bp, synthetic construct
  source 1..28: mol_type = other DNA
gttgcccaggctggtctcaaacccctgg

SEQ ID NO: 32899 - DNA, 28 bp, synthetic construct
  source 1..28: mol_type = other DNA
ttgcccaggctggtctcaaacccctggg

SEQ ID NO: 32900 - DNA, 28 bp, synthetic construct
  source 1..28: mol_type = other DNA
gagcccaggggtttgagaccagcctggg

SEQ ID NO: 32901 - DNA, 28 bp, synthetic construct
  source 1..28: mol_type = other DNA
tgagcccaggggtttgagaccagcctgg

SEQ ID NO: 32902 - DNA, 28 bp, synthetic construct
  source 1..28: mol_type = other DNA
aggcaggtggatcacttgagcccagggg

SEQ ID NO: 32903 - DNA, 28 bp, synthetic construct
  source 1..28: mol_type = other DNA
gaggcaggtggatcacttgagcccaggg

SEQ ID NO: 32904 - DNA, 28 bp, synthetic construct
  source 1..28: mol_type = other DNA
tgaggcaggtggatcacttgagcccagg

SEQ ID NO: 32905 - DNA, 28 bp, synthetic construct
  source 1..28: mol_type = other DNA
cagcactttgggaggctgaggcaggtgg

SEQ ID NO: 32906 - DNA, 28 bp, synthetic construct
  source 1..28: mol_type = other DNA
cacctgcctcagcctcccaaagtgctgg

SEQ ID NO: 32907 - DNA, 28 bp, synthetic construct
  source 1..28: mol_type = other DNA
acctgcctcagcctcccaaagtgctggg

SEQ ID NO: 32908 - DNA, 28 bp, synthetic construct
  source 1..28: mol_type = other DNA
tcccagcactttgggaggctgaggcagg

SEQ ID NO: 32909 - DNA, 28 bp, synthetic construct
  source 1..28: mol_type = other DNA
ataatcccagcactttgggaggctgagg

SEQ ID NO: 32910 - DNA, 28 bp, synthetic construct
  source 1..28: mol_type = other DNA
atggctataatcccagcactttgggagg

SEQ ID NO: 32911 - DNA, 28 bp, synthetic construct
  source 1..28: mol_type = other DNA
taaatggctataatcccagcactttggg

SEQ ID NO: 32912 - DNA, 28 bp, synthetic construct
  source 1..28: mol_type = other DNA
gtaaatggctataatcccagcactttgg

SEQ ID NO: 32913 - DNA, 28 bp, synthetic construct
  source 1..28: mol_type = other DNA
tatcttctctgttagagaaagtaaatgg

SEQ ID NO: 32914 - DNA, 28 bp, synthetic construct
  source 1..28: mol_type = other DNA
cgaccacctccgacgagcacattctagg

SEQ ID NO: 32915 - DNA, 28 bp, synthetic construct
  source 1..28: mol_type = other DNA
gcacctagaatgtgctcgtcggaggtgg

SEQ ID NO: 32916 - DNA, 28 bp, synthetic construct
  source 1..28: mol_type = other DNA
ctggcacctagaatgtgctcgtcggagg

SEQ ID NO: 32917 - DNA, 28 bp, synthetic construct
  source 1..28: mol_type = other DNA
tctctggcacctagaatgtgctcgtcgg

SEQ ID NO: 32918 - DNA, 28 bp, synthetic construct
  source 1..28: mol_type = other DNA
gaagacttcttcagttttatatctctgg

SEQ ID NO: 32919 - DNA, 28 bp, synthetic construct
  source 1..28: mol_type = other DNA
ccttttcaagtgtctcactgcttattgg

SEQ ID NO: 32920 - DNA, 28 bp, synthetic construct
  source 1..28: mol_type = other DNA
cttttcaagtgtctcactgcttattggg

SEQ ID NO: 32921 - DNA, 28 bp, synthetic construct
  source 1..28: mol_type = other DNA
gcagaagcagaaaagaaagccagcgagg

SEQ ID NO: 32922 - DNA, 28 bp, synthetic construct
  source 1..28: mol_type = other DNA
aaagccagcgaggtgataaatactatgg

SEQ ID NO: 32923 - DNA, 28 bp, synthetic construct
  source 1..28: mol_type = other DNA
aagccagcgaggtgataaatactatggg

SEQ ID NO: 32924 - DNA, 28 bp, synthetic construct
  source 1..28: mol_type = other DNA
gctcccatagtatttatcacctcgctgg

SEQ ID NO: 32925 - DNA, 28 bp, synthetic construct
  source 1..28: mol_type = other DNA
gggattgtctgacaaggaaaaaagatgg

SEQ ID NO: 32926 - DNA, 28 bp, synthetic construct
  source 1..28: mol_type = other DNA
atcttttttccttgtcagacaatcccgg

SEQ ID NO: 32927 - DNA, 28 bp, synthetic construct
  source 1..28: mol_type = other DNA
ataaaagggccgggattgtctgacaagg

SEQ ID NO: 32928 - DNA, 28 bp, synthetic construct
  source 1..28: mol_type = other DNA
aactacaaggaaaaataaaagggccggg

SEQ ID NO: 32929 - DNA, 28 bp, synthetic construct
  source 1..28: mol_type = other DNA
aaactacaaggaaaaataaaagggccgg

SEQ ID NO: 32930 - DNA, 28 bp, synthetic construct
  source 1..28: mol_type = other DNA
aataaaactacaaggaaaaataaaaggg

SEQ ID NO: 32931 - DNA, 28 bp, synthetic construct
  source 1..28: mol_type = other DNA
gaataaaactacaaggaaaaataaaagg

SEQ ID NO: 32932 - DNA, 28 bp, synthetic construct
  source 1..28: mol_type = other DNA
ctacagactgaagaataaaactacaagg

SEQ ID NO: 32933 - DNA, 28 bp, synthetic construct
  source 1..28: mol_type = other DNA
tttggaaggacactggggaacttgtagg

SEQ ID NO: 32934 - DNA, 28 bp, synthetic construct
  source 1..28: mol_type = other DNA
tgactataaatttggaaggacactgggg

SEQ ID NO: 32935 - DNA, 28 bp, synthetic construct
  source 1..28: mol_type = other DNA
gtgactataaatttggaaggacactggg

SEQ ID NO: 32936 - DNA, 28 bp, synthetic construct
  source 1..28: mol_type = other DNA
cgtgactataaatttggaaggacactgg

SEQ ID NO: 32937 - DNA, 28 bp, synthetic construct
  source 1..28: mol_type = other DNA
gtccttccaaatttatagtcacgtgtgg

SEQ ID NO: 32938 - DNA, 28 bp, synthetic construct
  source 1..28: mol_type = other DNA
tccttccaaatttatagtcacgtgtggg

SEQ ID NO: 32939 - DNA, 28 bp, synthetic construct
  source 1..28: mol_type = other DNA
tcccacacgtgactataaatttggaagg

SEQ ID NO: 32940 - DNA, 28 bp, synthetic construct
  source 1..28: mol_type = other DNA
tgtgtcccacacgtgactataaatttgg

SEQ ID NO: 32941 - DNA, 28 bp, synthetic construct
  source 1..28: mol_type = other DNA
acgtgtgggacacagtccactctacagg

SEQ ID NO: 32942 - DNA, 28 bp, synthetic construct
  source 1..28: mol_type = other DNA
acacagtccactctacaggctctatcgg

SEQ ID NO: 32943 - DNA, 28 bp, synthetic construct
  source 1..28: mol_type = other DNA
gtccactctacaggctctatcggcatgg

SEQ ID NO: 32944 - DNA, 28 bp, synthetic construct
  source 1..28: mol_type = other DNA
gtccatgccgatagagcctgtagagtgg

SEQ ID NO: 32945 - DNA, 28 bp, synthetic construct
  source 1..28: mol_type = other DNA
tacaggctctatcggcatggactgtagg

SEQ ID NO: 32946 - DNA, 28 bp, synthetic construct
  source 1..28: mol_type = other DNA
acaggctctatcggcatggactgtaggg

SEQ ID NO: 32947 - DNA, 28 bp, synthetic construct
  source 1..28: mol_type = other DNA
caggctctatcggcatggactgtagggg

SEQ ID NO: 32948 - DNA, 28 bp, synthetic construct
  source 1..28: mol_type = other DNA
aggctctatcggcatggactgtaggggg

SEQ ID NO: 32949 - DNA, 28 bp, synthetic construct
  source 1..28: mol_type = other DNA
agggggagaatgacccgctttatgttgg

SEQ ID NO: 32950 - DNA, 28 bp, synthetic construct
  source 1..28: mol_type = other DNA
gagctgttgacttccaacataaagcggg

SEQ ID NO: 32951 - DNA, 28 bp, synthetic construct
  source 1..28: mol_type = other DNA
agagctgttgacttccaacataaagcgg

SEQ ID NO: 32952 - DNA, 28 bp, synthetic construct
  source 1..28: mol_type = other DNA
tggaagtcaacagctctgagaattaagg

SEQ ID NO: 32953 - DNA, 28 bp, synthetic construct
  source 1..28: mol_type = other DNA
gagaaagctttaagttatgagtcttagg

SEQ ID NO: 32954 - DNA, 28 bp, synthetic construct
  source 1..28: mol_type = other DNA
gaaggagagactaaatgagcttaggtgg

SEQ ID NO: 32955 - DNA, 28 bp, synthetic construct
  source 1..28: mol_type = other DNA
ggggaaggagagactaaatgagcttagg

SEQ ID NO: 32956 - DNA, 28 bp, synthetic construct
  source 1..28: mol_type = other DNA
agtctctccttccccaaatgtcttgagg

SEQ ID NO: 32957 - DNA, 28 bp, synthetic construct
  source 1..28: mol_type = other DNA
cttttttcctcaagacatttggggaagg

SEQ ID NO: 32958 - DNA, 28 bp, synthetic construct
  source 1..28: mol_type = other DNA
atggcttttttcctcaagacatttgggg

SEQ ID NO: 32959 - DNA, 28 bp, synthetic construct
  source 1..28: mol_type = other DNA
gatggcttttttcctcaagacatttggg

SEQ ID NO: 32960 - DNA, 28 bp, synthetic construct
  source 1..28: mol_type = other DNA
agatggcttttttcctcaagacatttgg

SEQ ID NO: 32961 - DNA, 28 bp, synthetic construct
  source 1..28: mol_type = other DNA
aaaaaagccatctgcctccttgttcagg

SEQ ID NO: 32962 - DNA, 28 bp, synthetic construct
  source 1..28: mol_type = other DNA
tggctgtcctgaacaaggaggcagatgg

SEQ ID NO: 32963 - DNA, 28 bp, synthetic construct
  source 1..28: mol_type = other DNA
tctgcctccttgttcaggacagccatgg

SEQ ID NO: 32964 - DNA, 28 bp, synthetic construct
  source 1..28: mol_type = other DNA
ctgcctccttgttcaggacagccatggg

SEQ ID NO: 32965 - DNA, 28 bp, synthetic construct
  source 1..28: mol_type = other DNA
tgcctccttgttcaggacagccatgggg

SEQ ID NO: 32966 - DNA, 28 bp, synthetic construct
  source 1..28: mol_type = other DNA
gaccccatggctgtcctgaacaaggagg

SEQ ID NO: 32967 - DNA, 28 bp, synthetic construct
  source 1..28: mol_type = other DNA
aatgaccccatggctgtcctgaacaagg

SEQ ID NO: 32968 - DNA, 28 bp, synthetic construct
  source 1..28: mol_type = other DNA
ccatgatgagtcttaaatgaccccatgg

SEQ ID NO: 32969 - DNA, 28 bp, synthetic construct
  source 1..28: mol_type = other DNA
tttaacaaccttatcctacgctgtgtgg

SEQ ID NO: 32970 - DNA, 28 bp, synthetic construct
  source 1..28: mol_type = other DNA
atcttggtccacacagcgtaggataagg

SEQ ID NO: 32971 - DNA, 28 bp, synthetic construct
  source 1..28: mol_type = other DNA
atggtcatcttggtccacacagcgtagg

SEQ ID NO: 32972 - DNA, 28 bp, synthetic construct
  source 1..28: mol_type = other DNA
cgctgtgtggaccaagatgaccatctgg

SEQ ID NO: 32973 - DNA, 28 bp, synthetic construct
  source 1..28: mol_type = other DNA
aatcacaggagccagatggtcatcttgg

SEQ ID NO: 32974 - DNA, 28 bp, synthetic construct
  source 1..28: mol_type = other DNA
gaccatctggctcctgtgattgcagtgg

SEQ ID NO: 32975 - DNA, 28 bp, synthetic construct
  source 1..28: mol_type = other DNA
accatctggctcctgtgattgcagtggg

SEQ ID NO: 32976 - DNA, 28 bp, synthetic construct
  source 1..28: mol_type = other DNA
ccccactgcaatcacaggagccagatgg

SEQ ID NO: 32977 - DNA, 28 bp, synthetic construct
  source 1..28: mol_type = other DNA
acaatgtggtccccactgcaatcacagg

SEQ ID NO: 32978 - DNA, 28 bp, synthetic construct
  source 1..28: mol_type = other DNA
attgcagtggggaccacattgtacctgg

SEQ ID NO: 32979 - DNA, 28 bp, synthetic construct
  source 1..28: mol_type = other DNA
ttgcagtggggaccacattgtacctggg

SEQ ID NO: 32980 - DNA, 28 bp, synthetic construct
  source 1..28: mol_type = other DNA
accacattgtacctgggtattacagagg

SEQ ID NO: 32981 - DNA, 28 bp, synthetic construct
  source 1..28: mol_type = other DNA
acctctgtaatacccaggtacaatgtgg

SEQ ID NO: 32982 - DNA, 28 bp, synthetic construct
  source 1..28: mol_type = other DNA
agatggctgcacctctgtaatacccagg

SEQ ID NO: 32983 - DNA, 28 bp, synthetic construct
  source 1..28: mol_type = other DNA
tggacagctgcagggggaggggagatgg

SEQ ID NO: 32984 - DNA, 28 bp, synthetic construct
  source 1..28: mol_type = other DNA
aggaactggacagctgcagggggagggg

SEQ ID NO: 32985 - DNA, 28 bp, synthetic construct
  source 1..28: mol_type = other DNA
caggaactggacagctgcagggggaggg

SEQ ID NO: 32986 - DNA, 28 bp, synthetic construct
  source 1..28: mol_type = other DNA
ccaggaactggacagctgcagggggagg

SEQ ID NO: 32987 - DNA, 28 bp, synthetic construct
  source 1..28: mol_type = other DNA
tttccaggaactggacagctgcaggggg

SEQ ID NO: 32988 - DNA, 28 bp, synthetic construct
  source 1..28: mol_type = other DNA
ttttccaggaactggacagctgcagggg

SEQ ID NO: 32989 - DNA, 28 bp, synthetic construct
  source 1..28: mol_type = other DNA
gttttccaggaactggacagctgcaggg

SEQ ID NO: 32990 - DNA, 28 bp, synthetic construct
  source 1..28: mol_type = other DNA
cgttttccaggaactggacagctgcagg

SEQ ID NO: 32991 - DNA, 28 bp, synthetic construct
  source 1..28: mol_type = other DNA
tccagttcctggaaaacgtgctcccagg

SEQ ID NO: 32992 - DNA, 28 bp, synthetic construct
  source 1..28: mol_type = other DNA
tcctgggagcacgttttccaggaactgg

SEQ ID NO: 32993 - DNA, 28 bp, synthetic construct
  source 1..28: mol_type = other DNA
tgaaggtcctgggagcacgttttccagg

SEQ ID NO: 32994 - DNA, 28 bp, synthetic construct
  source 1..28: mol_type = other DNA
ctagtcacaagcagctgaaggtcctggg

SEQ ID NO: 32995 - DNA, 28 bp, synthetic construct
  source 1..28: mol_type = other DNA
tctagtcacaagcagctgaaggtcctgg

SEQ ID NO: 32996 - DNA, 28 bp, synthetic construct
  source 1..28: mol_type = other DNA
ggaccttcagctgcttgtgactagatgg

SEQ ID NO: 32997 - DNA, 28 bp, synthetic construct
  source 1..28: mol_type = other DNA
ccttcagctgcttgtgactagatggagg

SEQ ID NO: 32998 - DNA, 28 bp, synthetic construct
  source 1..28: mol_type = other DNA
tgatgtttgtggcagagaggattagtgg

SEQ ID NO: 32999 - DNA, 28 bp, synthetic construct
  source 1..28: mol_type = other DNA
tctgcttatgatgtttgtggcagagagg

SEQ ID NO: 33000 - DNA, 28 bp, synthetic construct
  source 1..28: mol_type = other DNA
ttatacgatctgcttatgatgtttgtgg

SEQ ID NO: 33001 - DNA, 28 bp, synthetic construct
  source 1..28: mol_type = other DNA
ataagcagatcgtataaacgtgaagagg

SEQ ID NO: 33002 - DNA, 28 bp, synthetic construct
  source 1..28: mol_type = other DNA
ctcataggatgctttttctttaatatgg

SEQ ID NO: 33003 - DNA, 28 bp, synthetic construct
  source 1..28: mol_type = other DNA
aaaaagcatcctatgagctatttattgg

SEQ ID NO: 33004 - DNA, 28 bp, synthetic construct
  source 1..28: mol_type = other DNA
agcatcctatgagctatttattggctgg

SEQ ID NO: 33005 - DNA, 28 bp, synthetic construct
  source 1..28: mol_type = other DNA
aatctccagccaataaatagctcatagg

SEQ ID NO: 33006 - DNA, 28 bp, synthetic construct
  source 1..28: mol_type = other DNA
tatgagctatttattggctggagattgg

SEQ ID NO: 33007 - DNA, 28 bp, synthetic construct
  source 1..28: mol_type = other DNA
agattggtagatgatcctcacactaagg

SEQ ID NO: 33008 - DNA, 28 bp, synthetic construct
  source 1..28: mol_type = other DNA
gaattcatggaaatgccttagtgtgagg

SEQ ID NO: 33009 - DNA, 28 bp, synthetic construct
  source 1..28: mol_type = other DNA
tcaaaaaaaaaaaaaaatgaattcatgg

SEQ ID NO: 33010 - DNA, 28 bp, synthetic construct
  source 1..28: mol_type = other DNA
attcatttttttttttttttgagacagg

SEQ ID NO: 33011 - DNA, 28 bp, synthetic construct
  source 1..28: mol_type = other DNA
gagacaggatctcactttgtcatccagg

SEQ ID NO: 33012 - DNA, 28 bp, synthetic construct
  source 1..28: mol_type = other DNA
caggatctcactttgtcatccaggctgg

SEQ ID NO: 33013 - DNA, 28 bp, synthetic construct
  source 1..28: mol_type = other DNA
ctttgtcatccaggctggagtgcagtgg

SEQ ID NO: 33014 - DNA, 28 bp, synthetic construct
  source 1..28: mol_type = other DNA
gtgatcacaccactgcactccagcctgg

SEQ ID NO: 33015 - DNA, 28 bp, synthetic construct
  source 1..28: mol_type = other DNA
acagctcactgtagcctcaacctcctgg

SEQ ID NO: 33016 - DNA, 28 bp, synthetic construct
  source 1..28: mol_type = other DNA
aggatcactggaaaccaggaggttgagg

SEQ ID NO: 33017 - DNA, 28 bp, synthetic construct
  source 1..28: mol_type = other DNA
ggtgggaggatcactggaaaccaggagg

SEQ ID NO: 33018 - DNA, 28 bp, synthetic construct
  source 1..28: mol_type = other DNA
cgaggtgggaggatcactggaaaccagg

SEQ ID NO: 33019 - DNA, 28 bp, synthetic construct
  source 1..28: mol_type = other DNA
ctggtttccagtgatcctcccacctcgg

SEQ ID NO: 33020 - DNA, 28 bp, synthetic construct
  source 1..28: mol_type = other DNA
tgggaggccgaggtgggaggatcactgg

SEQ ID NO: 33021 - DNA, 28 bp, synthetic construct
  source 1..28: mol_type = other DNA
cagcactttgggaggccgaggtgggagg

SEQ ID NO: 33022 - DNA, 28 bp, synthetic construct
  source 1..28: mol_type = other DNA
tcgcagcactttgggaggccgaggtggg

SEQ ID NO: 33023 - DNA, 28 bp, synthetic construct
  source 1..28: mol_type = other DNA
atcgcagcactttgggaggccgaggtgg

SEQ ID NO: 33024 - DNA, 28 bp, synthetic construct
  source 1..28: mol_type = other DNA
gtaatcgcagcactttgggaggccgagg

SEQ ID NO: 33025 - DNA, 28 bp, synthetic construct
  source 1..28: mol_type = other DNA
cggcctcccaaagtgctgcgattacagg

SEQ ID NO: 33026 - DNA, 28 bp, synthetic construct
  source 1..28: mol_type = other DNA
aggcctgtaatcgcagcactttgggagg

SEQ ID NO: 33027 - DNA, 28 bp, synthetic construct
  source 1..28: mol_type = other DNA
ctcaggcctgtaatcgcagcactttggg

SEQ ID NO: 33028 - DNA, 28 bp, synthetic construct
  source 1..28: mol_type = other DNA
gctcaggcctgtaatcgcagcactttgg

SEQ ID NO: 33029 - DNA, 28 bp, synthetic construct
  source 1..28: mol_type = other DNA
attcatgggctgggcacggtggctcagg

SEQ ID NO: 33030 - DNA, 28 bp, synthetic construct
  source 1..28: mol_type = other DNA
agctgaattcatgggctgggcacggtgg

SEQ ID NO: 33031 - DNA, 28 bp, synthetic construct
  source 1..28: mol_type = other DNA
taaagctgaattcatgggctgggcacgg

SEQ ID NO: 33032 - DNA, 28 bp, synthetic construct
  source 1..28: mol_type = other DNA
agtattaaagctgaattcatgggctggg

SEQ ID NO: 33033 - DNA, 28 bp, synthetic construct
  source 1..28: mol_type = other DNA
tagtattaaagctgaattcatgggctgg

SEQ ID NO: 33034 - DNA, 28 bp, synthetic construct
  source 1..28: mol_type = other DNA
gtggtagtattaaagctgaattcatggg

SEQ ID NO: 33035 - DNA, 28 bp, synthetic construct
  source 1..28: mol_type = other DNA
agtggtagtattaaagctgaattcatgg

SEQ ID NO: 33036 - DNA, 28 bp, synthetic construct
  source 1..28: mol_type = other DNA
gaaaatatgcaaagtgctgcaaaagtgg

SEQ ID NO: 33037 - DNA, 28 bp, synthetic construct
  source 1..28: mol_type = other DNA
ggattcattttataatgaaaaattctgg

SEQ ID NO: 33038 - DNA, 28 bp, synthetic construct
  source 1..28: mol_type = other DNA
gaatttttcattataaaatgaatccagg

SEQ ID NO: 33039 - DNA, 28 bp, synthetic construct
  source 1..28: mol_type = other DNA
tttttcattataaaatgaatccaggtgg

SEQ ID NO: 33040 - DNA, 28 bp, synthetic construct
  source 1..28: mol_type = other DNA
atttgatttctatattcaaaccacctgg

SEQ ID NO: 33041 - DNA, 28 bp, synthetic construct
  source 1..28: mol_type = other DNA
atctcaaaaaaactcactatataccagg

SEQ ID NO: 33042 - DNA, 28 bp, synthetic construct
  source 1..28: mol_type = other DNA
aaaaaaagaaagaaagaaaaagtcctgg

SEQ ID NO: 33043 - DNA, 28 bp, synthetic construct
  source 1..28: mol_type = other DNA
tttctttctttcttttttttttttttgg

SEQ ID NO: 33044 - DNA, 28 bp, synthetic construct
  source 1..28: mol_type = other DNA
gagactgagtcttgctttattgcccagg

SEQ ID NO: 33045 - DNA, 28 bp, synthetic construct
  source 1..28: mol_type = other DNA
gagtcttgctttattgcccaggctgagg

SEQ ID NO: 33046 - DNA, 28 bp, synthetic construct
  source 1..28: mol_type = other DNA
ctttattgcccaggctgaggtgcagtgg

SEQ ID NO: 33047 - DNA, 28 bp, synthetic construct
  source 1..28: mol_type = other DNA
agatagcaccactgcacctcagcctggg

SEQ ID NO: 33048 - DNA, 28 bp, synthetic construct
  source 1..28: mol_type = other DNA
aagatagcaccactgcacctcagcctgg

SEQ ID NO: 33049 - DNA, 28 bp, synthetic construct
  source 1..28: mol_type = other DNA
aggctgaggtgcagtggtgctatcttgg

SEQ ID NO: 33050 - DNA, 28 bp, synthetic construct
  source 1..28: mol_type = other DNA
acttgaacatgggaggcggaggttgtgg

SEQ ID NO: 33051 - DNA, 28 bp, synthetic construct
  source 1..28: mol_type = other DNA
agagtcacttgaacatgggaggcggagg

SEQ ID NO: 33052 - DNA, 28 bp, synthetic construct
  source 1..28: mol_type = other DNA
acgagagtcacttgaacatgggaggcgg

SEQ ID NO: 33053 - DNA, 28 bp, synthetic construct
  source 1..28: mol_type = other DNA
agcacgagagtcacttgaacatgggagg

SEQ ID NO: 33054 - DNA, 28 bp, synthetic construct
  source 1..28: mol_type = other DNA
tgaagcacgagagtcacttgaacatggg

SEQ ID NO: 33055 - DNA, 28 bp, synthetic construct
  source 1..28: mol_type = other DNA
ctgaagcacgagagtcacttgaacatgg

SEQ ID NO: 33056 - DNA, 28 bp, synthetic construct
  source 1..28: mol_type = other DNA
ctcgtgcttcagcctcccaagtagctgg

SEQ ID NO: 33057 - DNA, 28 bp, synthetic construct
  source 1..28: mol_type = other DNA
tcgtgcttcagcctcccaagtagctggg

SEQ ID NO: 33058 - DNA, 28 bp, synthetic construct
  source 1..28: mol_type = other DNA
cagcctcccaagtagctgggattacagg

SEQ ID NO: 33059 - DNA, 28 bp, synthetic construct
  source 1..28: mol_type = other DNA
gcacctgtaatcccagctacttgggagg

SEQ ID NO: 33060 - DNA, 28 bp, synthetic construct
  source 1..28: mol_type = other DNA
cgggcacctgtaatcccagctacttggg

SEQ ID NO: 33061 - DNA, 28 bp, synthetic construct
  source 1..28: mol_type = other DNA
gcgggcacctgtaatcccagctacttgg

SEQ ID NO: 33062 - DNA, 28 bp, synthetic construct
  source 1..28: mol_type = other DNA
gattacaggtgcccgccaccacacctgg

SEQ ID NO: 33063 - DNA, 28 bp, synthetic construct
  source 1..28: mol_type = other DNA
acaaaaattagccaggtgtggtggcggg

SEQ ID NO: 33064 - DNA, 28 bp, synthetic construct
  source 1..28: mol_type = other DNA
tacaaaaattagccaggtgtggtggcgg

SEQ ID NO: 33065 - DNA, 28 bp, synthetic construct
  source 1..28: mol_type = other DNA
aattacaaaaattagccaggtgtggtgg

SEQ ID NO: 33066 - DNA, 28 bp, synthetic construct
  source 1..28: mol_type = other DNA
taaaattacaaaaattagccaggtgtgg

SEQ ID NO: 33067 - DNA, 28 bp, synthetic construct
  source 1..28: mol_type = other DNA
tctattaaaattacaaaaattagccagg

SEQ ID NO: 33068 - DNA, 28 bp, synthetic construct
  source 1..28: mol_type = other DNA
taatttttgtaattttaatagagaccgg

SEQ ID NO: 33069 - DNA, 28 bp, synthetic construct
  source 1..28: mol_type = other DNA
ttttaatagagaccggttttcaccatgg

SEQ ID NO: 33070 - DNA, 28 bp, synthetic construct
  source 1..28: mol_type = other DNA
atagagaccggttttcaccatggtgtgg

SEQ ID NO: 33071 - DNA, 28 bp, synthetic construct
  source 1..28: mol_type = other DNA
gaccggttttcaccatggtgtggccagg

SEQ ID NO: 33072 - DNA, 28 bp, synthetic construct
  source 1..28: mol_type = other DNA
agcctggccacaccatggtgaaaaccgg

SEQ ID NO: 33073 - DNA, 28 bp, synthetic construct
  source 1..28: mol_type = other DNA
ggttttcaccatggtgtggccaggctgg

SEQ ID NO: 33074 - DNA, 28 bp, synthetic construct
  source 1..28: mol_type = other DNA
gtttgagaccagcctggccacaccatgg

SEQ ID NO: 33075 - DNA, 28 bp, synthetic construct
  source 1..28: mol_type = other DNA
tgaggtcagtagtttgagaccagcctgg

SEQ ID NO: 33076 - DNA, 28 bp, synthetic construct
  source 1..28: mol_type = other DNA
gagtctgaggcaggcagatcacttgagg

SEQ ID NO: 33077 - DNA, 28 bp, synthetic construct
  source 1..28: mol_type = other DNA
tgcctgcctcagactcccaaagtgctgg

SEQ ID NO: 33078 - DNA, 28 bp, synthetic construct
  source 1..28: mol_type = other DNA
gcctgcctcagactcccaaagtgctggg

SEQ ID NO: 33079 - DNA, 28 bp, synthetic construct
  source 1..28: mol_type = other DNA
tcccagcactttgggagtctgaggcagg

SEQ ID NO: 33080 - DNA, 28 bp, synthetic construct
  source 1..28: mol_type = other DNA
gtaatcccagcactttgggagtctgagg

SEQ ID NO: 33081 - DNA, 28 bp, synthetic construct
  source 1..28: mol_type = other DNA
cagactcccaaagtgctgggattacagg

SEQ ID NO: 33082 - DNA, 28 bp, synthetic construct
  source 1..28: mol_type = other DNA
ctcaggcctgtaatcccagcactttggg

SEQ ID NO: 33083 - DNA, 28 bp, synthetic construct
  source 1..28: mol_type = other DNA
gctcaggcctgtaatcccagcactttgg

SEQ ID NO: 33084 - DNA, 28 bp, synthetic construct
  source 1..28: mol_type = other DNA
ggattacaggcctgagccacccccctgg

SEQ ID NO: 33085 - DNA, 28 bp, synthetic construct
  source 1..28: mol_type = other DNA
aaaagaaaggccaggggggtggctcagg

SEQ ID NO: 33086 - DNA, 28 bp, synthetic construct
  source 1..28: mol_type = other DNA
ttttaaaaaagaaaggccaggggggtgg

SEQ ID NO: 33087 - DNA, 28 bp, synthetic construct
  source 1..28: mol_type = other DNA
tatttttaaaaaagaaaggccagggggg

SEQ ID NO: 33088 - DNA, 28 bp, synthetic construct
  source 1..28: mol_type = other DNA
ctatttttaaaaaagaaaggccaggggg

SEQ ID NO: 33089 - DNA, 28 bp, synthetic construct
  source 1..28: mol_type = other DNA
tctatttttaaaaaagaaaggccagggg

SEQ ID NO: 33090 - DNA, 28 bp, synthetic construct
  source 1..28: mol_type = other DNA
ctctatttttaaaaaagaaaggccaggg

SEQ ID NO: 33091 - DNA, 28 bp, synthetic construct
  source 1..28: mol_type = other DNA
actctatttttaaaaaagaaaggccagg

SEQ ID NO: 33092 - DNA, 28 bp, synthetic construct
  source 1..28: mol_type = other DNA
tttcaactctatttttaaaaaagaaagg

SEQ ID NO: 33093 - DNA, 28 bp, synthetic construct
  source 1..28: mol_type = other DNA
ttttttaaaaatagagttgaaaattagg

SEQ ID NO: 33094 - DNA, 28 bp, synthetic construct
  source 1..28: mol_type = other DNA
atggatttagaactctcaatatacttgg

SEQ ID NO: 33095 - DNA, 28 bp, synthetic construct
  source 1..28: mol_type = other DNA
tattgagagttctaaatccattgtcagg

SEQ ID NO: 33096 - DNA, 28 bp, synthetic construct
  source 1..28: mol_type = other DNA
aaatccattgtcaggtacatacaactgg

SEQ ID NO: 33097 - DNA, 28 bp, synthetic construct
  source 1..28: mol_type = other DNA
aaagccagttgtatgtacctgacaatgg

SEQ ID NO: 33098 - DNA, 28 bp, synthetic construct
  source 1..28: mol_type = other DNA
agagaggcatgttggcagggtaatcagg

SEQ ID NO: 33099 - DNA, 28 bp, synthetic construct
  source 1..28: mol_type = other DNA
tggtgtatagagaggcatgttggcaggg

SEQ ID NO: 33100 - DNA, 28 bp, synthetic construct
  source 1..28: mol_type = other DNA
ttggtgtatagagaggcatgttggcagg

SEQ ID NO: 33101 - DNA, 28 bp, synthetic construct
  source 1..28: mol_type = other DNA
gtaattggtgtatagagaggcatgttgg

SEQ ID NO: 33102 - DNA, 28 bp, synthetic construct
  source 1..28: mol_type = other DNA
agtagaatgtaattggtgtatagagagg

SEQ ID NO: 33103 - DNA, 28 bp, synthetic construct
  source 1..28: mol_type = other DNA
tctctatacaccaattacattctactgg

SEQ ID NO: 33104 - DNA, 28 bp, synthetic construct
  source 1..28: mol_type = other DNA
ctctatacaccaattacattctactggg

SEQ ID NO: 33105 - DNA, 28 bp, synthetic construct
  source 1..28: mol_type = other DNA
tgaacaactcccagtagaatgtaattgg

SEQ ID NO: 33106 - DNA, 28 bp, synthetic construct
  source 1..28: mol_type = other DNA
attctactgggagttgttcaactcatgg

SEQ ID NO: 33107 - DNA, 28 bp, synthetic construct
  source 1..28: mol_type = other DNA
tggatatggcaaggcttaatttacatgg

SEQ ID NO: 33108 - DNA, 28 bp, synthetic construct
  source 1..28: mol_type = other DNA
agccttgccatatccattgcagaagagg

SEQ ID NO: 33109 - DNA, 28 bp, synthetic construct
  source 1..28: mol_type = other DNA
gccttgccatatccattgcagaagaggg

SEQ ID NO: 33110 - DNA, 28 bp, synthetic construct
  source 1..28: mol_type = other DNA
ccttgccatatccattgcagaagagggg

SEQ ID NO: 33111 - DNA, 28 bp, synthetic construct
  source 1..28: mol_type = other DNA
atgcacccctcttctgcaatggatatgg

SEQ ID NO: 33112 - DNA, 28 bp, synthetic construct
  source 1..28: mol_type = other DNA
cagtaaatgcacccctcttctgcaatgg

SEQ ID NO: 33113 - DNA, 28 bp, synthetic construct
  source 1..28: mol_type = other DNA
cattgcagaagaggggtgcatttactgg

SEQ ID NO: 33114 - DNA, 28 bp, synthetic construct
  source 1..28: mol_type = other DNA
attgcagaagaggggtgcatttactggg

SEQ ID NO: 33115 - DNA, 28 bp, synthetic construct
  source 1..28: mol_type = other DNA
cagaagaggggtgcatttactgggttgg

SEQ ID NO: 33116 - DNA, 28 bp, synthetic construct
  source 1..28: mol_type = other DNA
aggggtgcatttactgggttggaagtgg

SEQ ID NO: 33117 - DNA, 28 bp, synthetic construct
  source 1..28: mol_type = other DNA
ttactgggttggaagtggtgtcaccagg

SEQ ID NO: 33118 - DNA, 28 bp, synthetic construct
  source 1..28: mol_type = other DNA
gaagtggtgtcaccaggaccagtcaagg

SEQ ID NO: 33119 - DNA, 28 bp, synthetic construct
  source 1..28: mol_type = other DNA
cttaaggagtggccttgactggtcctgg

SEQ ID NO: 33120 - DNA, 28 bp, synthetic construct
  source 1..28: mol_type = other DNA
accagtcaaggccactccttaagaaagg

SEQ ID NO: 33121 - DNA, 28 bp, synthetic construct
  source 1..28: mol_type = other DNA
acctttcttaaggagtggccttgactgg

SEQ ID NO: 33122 - DNA, 28 bp, synthetic construct
  source 1..28: mol_type = other DNA
gaaatgctgaacctttcttaaggagtgg

SEQ ID NO: 33123 - DNA, 28 bp, synthetic construct
  source 1..28: mol_type = other DNA
atgacgaaatgctgaacctttcttaagg

SEQ ID NO: 33124 - DNA, 28 bp, synthetic construct
  source 1..28: mol_type = other DNA
ttaagaaaggttcagcatttcgtcatgg

SEQ ID NO: 33125 - DNA, 28 bp, synthetic construct
  source 1..28: mol_type = other DNA
cagcatttcgtcatggttttatatcagg

SEQ ID NO: 33126 - DNA, 28 bp, synthetic construct
  source 1..28: mol_type = other DNA
gtttaaaaagttaggaaggcaacaaagg

SEQ ID NO: 33127 - DNA, 28 bp, synthetic construct
  source 1..28: mol_type = other DNA
gatgaatatgtttaaaaagttaggaagg

SEQ ID NO: 33128 - DNA, 28 bp, synthetic construct
  source 1..28: mol_type = other DNA
aatagatgaatatgtttaaaaagttagg

SEQ ID NO: 33129 - DNA, 28 bp, synthetic construct
  source 1..28: mol_type = other DNA
catattcatctatttctctttcagctgg

SEQ ID NO: 33130 - DNA, 28 bp, synthetic construct
  source 1..28: mol_type = other DNA
aaaaattcctgtgaaaaactctaagtgg

SEQ ID NO: 33131 - DNA, 28 bp, synthetic construct
  source 1..28: mol_type = other DNA
aaaattcctgtgaaaaactctaagtggg

SEQ ID NO: 33132 - DNA, 28 bp, synthetic construct
  source 1..28: mol_type = other DNA
tacattcccacttagagtttttcacagg

SEQ ID NO: 33133 - DNA, 28 bp, synthetic construct
  source 1..28: mol_type = other DNA
aagtgggaatgtacacttctgagatagg

SEQ ID NO: 33134 - DNA, 28 bp, synthetic construct
  source 1..28: mol_type = other DNA
ctgcttagtgcttaagaaaataaccagg

SEQ ID NO: 33135 - DNA, 28 bp, synthetic construct
  source 1..28: mol_type = other DNA
gtaactaaatagatcgttattttcctgg

SEQ ID NO: 33136 - DNA, 28 bp, synthetic construct
  source 1..28: mol_type = other DNA
ataacgatctatttagttactatcctgg

SEQ ID NO: 33137 - DNA, 28 bp, synthetic construct
  source 1..28: mol_type = other DNA
tatttagttactatcctggaagtcatgg

SEQ ID NO: 33138 - DNA, 28 bp, synthetic construct
  source 1..28: mol_type = other DNA
tagcagtatggacaccatgacttccagg

SEQ ID NO: 33139 - DNA, 28 bp, synthetic construct
  source 1..28: mol_type = other DNA
agtcatggtgtccatactgctaaagtgg

SEQ ID NO: 33140 - DNA, 28 bp, synthetic construct
  source 1..28: mol_type = other DNA
gtcatggtgtccatactgctaaagtggg

SEQ ID NO: 33141 - DNA, 28 bp, synthetic construct
  source 1..28: mol_type = other DNA
agtgaatagacccactttagcagtatgg

SEQ ID NO: 33142 - DNA, 28 bp, synthetic construct
  source 1..28: mol_type = other DNA
ctgctaaagtgggtctattcactgatgg

SEQ ID NO: 33143 - DNA, 28 bp, synthetic construct
  source 1..28: mol_type = other DNA
ctaaagtgggtctattcactgatggagg

SEQ ID NO: 33144 - DNA, 28 bp, synthetic construct
  source 1..28: mol_type = other DNA
gtgggtctattcactgatggaggacagg

SEQ ID NO: 33145 - DNA, 28 bp, synthetic construct
  source 1..28: mol_type = other DNA
attcactgatggaggacaggagagtagg

SEQ ID NO: 33146 - DNA, 28 bp, synthetic construct
  source 1..28: mol_type = other DNA
ttcactgatggaggacaggagagtaggg

SEQ ID NO: 33147 - DNA, 28 bp, synthetic construct
  source 1..28: mol_type = other DNA
caggagagtagggataaaaacagacagg

SEQ ID NO: 33148 - DNA, 28 bp, synthetic construct
  source 1..28: mol_type = other DNA
gtagggataaaaacagacaggatccagg

SEQ ID NO: 33149 - DNA, 28 bp, synthetic construct
  source 1..28: mol_type = other DNA
ggataaaaacagacaggatccaggccgg

SEQ ID NO: 33150 - DNA, 28 bp, synthetic construct
  source 1..28: mol_type = other DNA
gataaaaacagacaggatccaggccggg

SEQ ID NO: 33151 - DNA, 28 bp, synthetic construct
  source 1..28: mol_type = other DNA
aaacagacaggatccaggccgggcatgg

SEQ ID NO: 33152 - DNA, 28 bp, synthetic construct
  source 1..28: mol_type = other DNA
cagacaggatccaggccgggcatggtgg

SEQ ID NO: 33153 - DNA, 28 bp, synthetic construct
  source 1..28: mol_type = other DNA
caggtttgagccaccatgcccggcctgg

SEQ ID NO: 33154 - DNA, 28 bp, synthetic construct
  source 1..28: mol_type = other DNA
gattacaggtttgagccaccatgcccgg

SEQ ID NO: 33155 - DNA, 28 bp, synthetic construct
  source 1..28: mol_type = other DNA
ggtggctcaaacctgtaatcccagtagg

SEQ ID NO: 33156 - DNA, 28 bp, synthetic construct
  source 1..28: mol_type = other DNA
tcaaacctgtaatcccagtaggctgtgg

SEQ ID NO: 33157 - DNA, 28 bp, synthetic construct
  source 1..28: mol_type = other DNA
caaacctgtaatcccagtaggctgtggg

SEQ ID NO: 33158 - DNA, 28 bp, synthetic construct
  source 1..28: mol_type = other DNA
acctgtaatcccagtaggctgtgggagg

SEQ ID NO: 33159 - DNA, 28 bp, synthetic construct
  source 1..28: mol_type = other DNA
gcctcccacagcctactgggattacagg

SEQ ID NO: 33160 - DNA, 28 bp, synthetic construct
  source 1..28: mol_type = other DNA
tgtaatcccagtaggctgtgggaggcgg

SEQ ID NO: 33161 - DNA, 28 bp, synthetic construct
  source 1..28: mol_type = other DNA
aatcccagtaggctgtgggaggcggagg

SEQ ID NO: 33162 - DNA, 28 bp, synthetic construct
  source 1..28: mol_type = other DNA
cccagtaggctgtgggaggcggaggcgg

SEQ ID NO: 33163 - DNA, 28 bp, synthetic construct
  source 1..28: mol_type = other DNA
cccgcctccgcctcccacagcctactgg

SEQ ID NO: 33164 - DNA, 28 bp, synthetic construct
  source 1..28: mol_type = other DNA
gtaggctgtgggaggcggaggcgggcgg

SEQ ID NO: 33165 - DNA, 28 bp, synthetic construct
  source 1..28: mol_type = other DNA
gggaggcggaggcgggcggatcatgagg

SEQ ID NO: 33166 - DNA, 28 bp, synthetic construct
  source 1..28: mol_type = other DNA
gcggaggcgggcggatcatgaggtcagg

SEQ ID NO: 33167 - DNA, 28 bp, synthetic construct
  source 1..28: mol_type = other DNA
tgaggtcaggagatcgagaccatcctgg

SEQ ID NO: 33168 - DNA, 28 bp, synthetic construct
  source 1..28: mol_type = other DNA
cagggtttcactgtgttagccaggatgg

SEQ ID NO: 33169 - DNA, 28 bp, synthetic construct
  source 1..28: mol_type = other DNA
gagacagggtttcactgtgttagccagg

SEQ ID NO: 33170 - DNA, 28 bp, synthetic construct
  source 1..28: mol_type = other DNA
tttttttgtatttttagtggagacaggg

SEQ ID NO: 33171 - DNA, 28 bp, synthetic construct
  source 1..28: mol_type = other DNA
ttttttttgtatttttagtggagacagg

SEQ ID NO: 33172 - DNA, 28 bp, synthetic construct
  source 1..28: mol_type = other DNA
cggctaattttttttgtatttttagtgg

SEQ ID NO: 33173 - DNA, 28 bp, synthetic construct
  source 1..28: mol_type = other DNA
cactaaaaatacaaaaaaaattagccgg

SEQ ID NO: 33174 - DNA, 28 bp, synthetic construct
  source 1..28: mol_type = other DNA
actaaaaatacaaaaaaaattagccggg

SEQ ID NO: 33175 - DNA, 28 bp, synthetic construct
  source 1..28: mol_type = other DNA
aaatacaaaaaaaattagccgggcttgg

SEQ ID NO: 33176 - DNA, 28 bp, synthetic construct
  source 1..28: mol_type = other DNA
tacaaaaaaaattagccgggcttggtgg

SEQ ID NO: 33177 - DNA, 28 bp, synthetic construct
  source 1..28: mol_type = other DNA
aaaaaaaattagccgggcttggtggtgg

SEQ ID NO: 33178 - DNA, 28 bp, synthetic construct
  source 1..28: mol_type = other DNA
aaaaaaattagccgggcttggtggtggg

SEQ ID NO: 33179 - DNA, 28 bp, synthetic construct
  source 1..28: mol_type = other DNA
agccgggcttggtggtgggtgcctgtgg

SEQ ID NO: 33180 - DNA, 28 bp, synthetic construct
  source 1..28: mol_type = other DNA
gaccacaggcacccaccaccaagcccgg

SEQ ID NO: 33181 - DNA, 28 bp, synthetic construct
  source 1..28: mol_type = other DNA
tgggtgcctgtggtcccagctactcagg

SEQ ID NO: 33182 - DNA, 28 bp, synthetic construct
  source 1..28: mol_type = other DNA
gtgcctgtggtcccagctactcaggagg

SEQ ID NO: 33183 - DNA, 28 bp, synthetic construct
  source 1..28: mol_type = other DNA
cagcctcctgagtagctgggaccacagg

SEQ ID NO: 33184 - DNA, 28 bp, synthetic construct
  source 1..28: mol_type = other DNA
tcccagctactcaggaggctgaagcagg

SEQ ID NO: 33185 - DNA, 28 bp, synthetic construct
  source 1..28: mol_type = other DNA
tcctgcttcagcctcctgagtagctggg

SEQ ID NO: 33186 - DNA, 28 bp, synthetic construct
  source 1..28: mol_type = other DNA
ctcctgcttcagcctcctgagtagctgg

SEQ ID NO: 33187 - DNA, 28 bp, synthetic construct
  source 1..28: mol_type = other DNA
tactcaggaggctgaagcaggagaatgg

SEQ ID NO: 33188 - DNA, 28 bp, synthetic construct
  source 1..28: mol_type = other DNA
tgaagcaggagaatggcatgaacccagg

SEQ ID NO: 33189 - DNA, 28 bp, synthetic construct
  source 1..28: mol_type = other DNA
agcaggagaatggcatgaacccaggagg

SEQ ID NO: 33190 - DNA, 28 bp, synthetic construct
  source 1..28: mol_type = other DNA
aggagaatggcatgaacccaggaggtgg

SEQ ID NO: 33191 - DNA, 28 bp, synthetic construct
  source 1..28: mol_type = other DNA
agaatggcatgaacccaggaggtggagg

SEQ ID NO: 33192 - DNA, 28 bp, synthetic construct
  source 1..28: mol_type = other DNA
cggctcatagcaacctccacctcctggg

SEQ ID NO: 33193 - DNA, 28 bp, synthetic construct
  source 1..28: mol_type = other DNA
tcggctcatagcaacctccacctcctgg

SEQ ID NO: 33194 - DNA, 28 bp, synthetic construct
  source 1..28: mol_type = other DNA
aggctggagtgcagtggcgcaatctcgg

SEQ ID NO: 33195 - DNA, 28 bp, synthetic construct
  source 1..28: mol_type = other DNA
gagattgcgccactgcactccagcctgg

SEQ ID NO: 33196 - DNA, 28 bp, synthetic construct
  source 1..28: mol_type = other DNA
agattgcgccactgcactccagcctggg

SEQ ID NO: 33197 - DNA, 28 bp, synthetic construct
  source 1..28: mol_type = other DNA
ctgtgtcgcccaggctggagtgcagtgg

SEQ ID NO: 33198 - DNA, 28 bp, synthetic construct
  source 1..28: mol_type = other DNA
tggagtctcgctgtgtcgcccaggctgg

SEQ ID NO: 33199 - DNA, 28 bp, synthetic construct
  source 1..28: mol_type = other DNA
tagatggagtctcgctgtgtcgcccagg

SEQ ID NO: 33200 - DNA, 28 bp, synthetic construct
  source 1..28: mol_type = other DNA
actccatctaaaaaagaaagcagacagg

SEQ ID NO: 33201 - DNA, 28 bp, synthetic construct
  source 1..28: mol_type = other DNA
gatcctgtctgctttcttttttagatgg

SEQ ID NO: 33202 - DNA, 28 bp, synthetic construct
  source 1..28: mol_type = other DNA
aaagtcagaaagtctgcattggactggg

SEQ ID NO: 33203 - DNA, 28 bp, synthetic construct
  source 1..28: mol_type = other DNA
gaaagtcagaaagtctgcattggactgg

SEQ ID NO: 33204 - DNA, 28 bp, synthetic construct
  source 1..28: mol_type = other DNA
aataggaaagtcagaaagtctgcattgg

SEQ ID NO: 33205 - DNA, 28 bp, synthetic construct
  source 1..28: mol_type = other DNA
tcaggactcttgactcatctaaaatagg

SEQ ID NO: 33206 - DNA, 28 bp, synthetic construct
  source 1..28: mol_type = other DNA
gtcattttaattgaaactgtggatcagg

SEQ ID NO: 33207 - DNA, 28 bp, synthetic construct
  source 1..28: mol_type = other DNA
ctttctgtcattttaattgaaactgtgg

SEQ ID NO: 33208 - DNA, 28 bp, synthetic construct
  source 1..28: mol_type = other DNA
gagccaacaccaaataacactgtgaagg

SEQ ID NO: 33209 - DNA, 28 bp, synthetic construct
  source 1..28: mol_type = other DNA
cttccttcacagtgttatttggtgttgg

SEQ ID NO: 33210 - DNA, 28 bp, synthetic construct
  source 1..28: mol_type = other DNA
actcaacttccttcacagtgttatttgg

SEQ ID NO: 33211 - DNA, 28 bp, synthetic construct
  source 1..28: mol_type = other DNA
tacctttgaaaacccctaccacttcagg

SEQ ID NO: 33212 - DNA, 28 bp, synthetic construct
  source 1..28: mol_type = other DNA
cacctgaagtggtaggggttttcaaagg

SEQ ID NO: 33213 - DNA, 28 bp, synthetic construct
  source 1..28: mol_type = other DNA
agggagtgtgcacctgaagtggtagggg

SEQ ID NO: 33214 - DNA, 28 bp, synthetic construct
  source 1..28: mol_type = other DNA
gagggagtgtgcacctgaagtggtaggg

SEQ ID NO: 33215 - DNA, 28 bp, synthetic construct
  source 1..28: mol_type = other DNA
agagggagtgtgcacctgaagtggtagg

SEQ ID NO: 33216 - DNA, 28 bp, synthetic construct
  source 1..28: mol_type = other DNA
ctggagagggagtgtgcacctgaagtgg

SEQ ID NO: 33217 - DNA, 28 bp, synthetic construct
  source 1..28: mol_type = other DNA
cacttcaggtgcacactccctctccagg

SEQ ID NO: 33218 - DNA, 28 bp, synthetic construct
  source 1..28: mol_type = other DNA
tacatgggagtatgagtcctggagaggg

SEQ ID NO: 33219 - DNA, 28 bp, synthetic construct
  source 1..28: mol_type = other DNA
ctacatgggagtatgagtcctggagagg

SEQ ID NO: 33220 - DNA, 28 bp, synthetic construct
  source 1..28: mol_type = other DNA
atagtctacatgggagtatgagtcctgg

SEQ ID NO: 33221 - DNA, 28 bp, synthetic construct
  source 1..28: mol_type = other DNA
ttggtcagaaaggaatagtctacatggg

SEQ ID NO: 33222 - DNA, 28 bp, synthetic construct
  source 1..28: mol_type = other DNA
cttggtcagaaaggaatagtctacatgg

SEQ ID NO: 33223 - DNA, 28 bp, synthetic construct
  source 1..28: mol_type = other DNA
catgtagactattcctttctgaccaagg

SEQ ID NO: 33224 - DNA, 28 bp, synthetic construct
  source 1..28: mol_type = other DNA
gactattcctttctgaccaaggaactgg

SEQ ID NO: 33225 - DNA, 28 bp, synthetic construct
  source 1..28: mol_type = other DNA
aatagctccagttccttggtcagaaagg

SEQ ID NO: 33226 - DNA, 28 bp, synthetic construct
  source 1..28: mol_type = other DNA
gaccaaggaactggagctattctcatgg

SEQ ID NO: 33227 - DNA, 28 bp, synthetic construct
  source 1..28: mol_type = other DNA
gaccatgagaatagctccagttccttgg

SEQ ID NO: 33228 - DNA, 28 bp, synthetic construct
  source 1..28: mol_type = other DNA
aggaactggagctattctcatggtctgg

SEQ ID NO: 33229 - DNA, 28 bp, synthetic construct
  source 1..28: mol_type = other DNA
ctggagctattctcatggtctggaatgg

SEQ ID NO: 33230 - DNA, 28 bp, synthetic construct
  source 1..28: mol_type = other DNA
tggagctattctcatggtctggaatggg

SEQ ID NO: 33231 - DNA, 28 bp, synthetic construct
  source 1..28: mol_type = other DNA
aaacactttagcaagtaggcaggaaagg

SEQ ID NO: 33232 - DNA, 28 bp, synthetic construct
  source 1..28: mol_type = other DNA
aagagaaacactttagcaagtaggcagg

SEQ ID NO: 33233 - DNA, 28 bp, synthetic construct
  source 1..28: mol_type = other DNA
tgagaagagaaacactttagcaagtagg

SEQ ID NO: 33234 - DNA, 28 bp, synthetic construct
  source 1..28: mol_type = other DNA
tttctcttctcagtcccataccctttgg

SEQ ID NO: 33235 - DNA, 28 bp, synthetic construct
  source 1..28: mol_type = other DNA
ggctcacaactaatccaaagggtatggg

SEQ ID NO: 33236 - DNA, 28 bp, synthetic construct
  source 1..28: mol_type = other DNA
tggctcacaactaatccaaagggtatgg

SEQ ID NO: 33237 - DNA, 28 bp, synthetic construct
  source 1..28: mol_type = other DNA
atggctggctcacaactaatccaaaggg

SEQ ID NO: 33238 - DNA, 28 bp, synthetic construct
  source 1..28: mol_type = other DNA
tatggctggctcacaactaatccaaagg

SEQ ID NO: 33239 - DNA, 28 bp, synthetic construct
  source 1..28: mol_type = other DNA
ccagccatattgcatattgaagagttgg

SEQ ID NO: 33240 - DNA, 28 bp, synthetic construct
  source 1..28: mol_type = other DNA
cttaccaactcttcaatatgcaatatgg

SEQ ID NO: 33241 - DNA, 28 bp, synthetic construct
  source 1..28: mol_type = other DNA
ttggtaagatttgactccttctaacagg

SEQ ID NO: 33242 - DNA, 28 bp, synthetic construct
  source 1..28: mol_type = other DNA
caatagagcttgggaacctgttagaagg

SEQ ID NO: 33243 - DNA, 28 bp, synthetic construct
  source 1..28: mol_type = other DNA
ttgcaattacaggtcaatagagcttggg

SEQ ID NO: 33244 - DNA, 28 bp, synthetic construct
  source 1..28: mol_type = other DNA
tttgcaattacaggtcaatagagcttgg

SEQ ID NO: 33245 - DNA, 28 bp, synthetic construct
  source 1..28: mol_type = other DNA
tttatttgtatttttttgcaattacagg

SEQ ID NO: 33246 - DNA, 28 bp, synthetic construct
  source 1..28: mol_type = other DNA
aaccccaacagcaacaaagatcctgagg

SEQ ID NO: 33247 - DNA, 28 bp, synthetic construct
  source 1..28: mol_type = other DNA
accccaacagcaacaaagatcctgaggg

SEQ ID NO: 33248 - DNA, 28 bp, synthetic construct
  source 1..28: mol_type = other DNA
tccctcaggatctttgttgctgttgggg

SEQ ID NO: 33249 - DNA, 28 bp, synthetic construct
  source 1..28: mol_type = other DNA
ctccctcaggatctttgttgctgttggg

SEQ ID NO: 33250 - DNA, 28 bp, synthetic construct
  source 1..28: mol_type = other DNA
actccctcaggatctttgttgctgttgg

SEQ ID NO: 33251 - DNA, 28 bp, synthetic construct
  source 1..28: mol_type = other DNA
aaagatcctgagggagtgacattaatgg

SEQ ID NO: 33252 - DNA, 28 bp, synthetic construct
  source 1..28: mol_type = other DNA
attctaccattaatgtcactccctcagg

SEQ ID NO: 33253 - DNA, 28 bp, synthetic construct
  source 1..28: mol_type = other DNA
agtgacattaatggtagaatttttaagg

SEQ ID NO: 33254 - DNA, 28 bp, synthetic construct
  source 1..28: mol_type = other DNA
taatggtagaatttttaaggtacagcgg

SEQ ID NO: 33255 - DNA, 28 bp, synthetic construct
  source 1..28: mol_type = other DNA
ttaaggtacagcggtagcccccaaatgg

SEQ ID NO: 33256 - DNA, 28 bp, synthetic construct
  source 1..28: mol_type = other DNA
taaggtacagcggtagcccccaaatggg

SEQ ID NO: 33257 - DNA, 28 bp, synthetic construct
  source 1..28: mol_type = other DNA
gacgaaggaaaaatggcccatttggggg

SEQ ID NO: 33258 - DNA, 28 bp, synthetic construct
  source 1..28: mol_type = other DNA
agacgaaggaaaaatggcccatttgggg

SEQ ID NO: 33259 - DNA, 28 bp, synthetic construct
  source 1..28: mol_type = other DNA
tagacgaaggaaaaatggcccatttggg

SEQ ID NO: 33260 - DNA, 28 bp, synthetic construct
  source 1..28: mol_type = other DNA
ttagacgaaggaaaaatggcccatttgg

SEQ ID NO: 33261 - DNA, 28 bp, synthetic construct
  source 1..28: mol_type = other DNA
gcaataagattagacgaaggaaaaatgg

SEQ ID NO: 33262 - DNA, 28 bp, synthetic construct
  source 1..28: mol_type = other DNA
ttttccttcgtctaatcttattgcatgg

SEQ ID NO: 33263 - DNA, 28 bp, synthetic construct
  source 1..28: mol_type = other DNA
tttgccatgcaataagattagacgaagg

SEQ ID NO: 33264 - DNA, 28 bp, synthetic construct
  source 1..28: mol_type = other DNA
ttgcatggcaaatatagacagcagcagg

SEQ ID NO: 33265 - DNA, 28 bp, synthetic construct
  source 1..28: mol_type = other DNA
agcaggcattcctgactgagaaccctgg

SEQ ID NO: 33266 - DNA, 28 bp, synthetic construct
  source 1..28: mol_type = other DNA
cattcctgactgagaaccctggtgatgg

SEQ ID NO: 33267 - DNA, 28 bp, synthetic construct
  source 1..28: mol_type = other DNA
caggccatcaccagggttctcagtcagg

SEQ ID NO: 33268 - DNA, 28 bp, synthetic construct
  source 1..28: mol_type = other DNA
actgagaaccctggtgatggcctgatgg

SEQ ID NO: 33269 - DNA, 28 bp, synthetic construct
  source 1..28: mol_type = other DNA
ctctgcttccatcaggccatcaccaggg

SEQ ID NO: 33270 - DNA, 28 bp, synthetic construct
  source 1..28: mol_type = other DNA
tctctgcttccatcaggccatcaccagg

SEQ ID NO: 33271 - DNA, 28 bp, synthetic construct
  source 1..28: mol_type = other DNA
agacagtctcatctctgcttccatcagg

SEQ ID NO: 33272 - DNA, 28 bp, synthetic construct
  source 1..28: mol_type = other DNA
gagatgagactgtctgatccactccagg

SEQ ID NO: 33273 - DNA, 28 bp, synthetic construct
  source 1..28: mol_type = other DNA
actgtctgatccactccaggcagcatgg

SEQ ID NO: 33274 - DNA, 28 bp, synthetic construct
  source 1..28: mol_type = other DNA
ccactccaggcagcatggtccctaaagg

SEQ ID NO: 33275 - DNA, 28 bp, synthetic construct
  source 1..28: mol_type = other DNA
cactccaggcagcatggtccctaaaggg

SEQ ID NO: 33276 - DNA, 28 bp, synthetic construct
  source 1..28: mol_type = other DNA
agggccctttagggaccatgctgcctgg

SEQ ID NO: 33277 - DNA, 28 bp, synthetic construct
  source 1..28: mol_type = other DNA
tggtccctaaagggccctctacagctgg

SEQ ID NO: 33278 - DNA, 28 bp, synthetic construct
  source 1..28: mol_type = other DNA
ggtccctaaagggccctctacagctggg

SEQ ID NO: 33279 - DNA, 28 bp, synthetic construct
  source 1..28: mol_type = other DNA
gctcccagctgtagagggccctttaggg

SEQ ID NO: 33280 - DNA, 28 bp, synthetic construct
  source 1..28: mol_type = other DNA
ggctcccagctgtagagggccctttagg

SEQ ID NO: 33281 - DNA, 28 bp, synthetic construct
  source 1..28: mol_type = other DNA
aacagggtaggctcccagctgtagaggg

SEQ ID NO: 33282 - DNA, 28 bp, synthetic construct
  source 1..28: mol_type = other DNA
gaacagggtaggctcccagctgtagagg

SEQ ID NO: 33283 - DNA, 28 bp, synthetic construct
  source 1..28: mol_type = other DNA
atgtgctgttattacagaacagggtagg

SEQ ID NO: 33284 - DNA, 28 bp, synthetic construct
  source 1..28: mol_type = other DNA
gctgatgtgctgttattacagaacaggg

SEQ ID NO: 33285 - DNA, 28 bp, synthetic construct
  source 1..28: mol_type = other DNA
tgctgatgtgctgttattacagaacagg

SEQ ID NO: 33286 - DNA, 28 bp, synthetic construct
  source 1..28: mol_type = other DNA
agcacatcagcaacctctatcattgtgg

SEQ ID NO: 33287 - DNA, 28 bp, synthetic construct
  source 1..28: mol_type = other DNA
tcagcaacctctatcattgtggcaatgg

SEQ ID NO: 33288 - DNA, 28 bp, synthetic construct
  source 1..28: mol_type = other DNA
ttgattaccattgccacaatgatagagg

SEQ ID NO: 33289 - DNA, 28 bp, synthetic construct
  source 1..28: mol_type = other DNA
atttcattgattgcctttatgtgccagg

SEQ ID NO: 33290 - DNA, 28 bp, synthetic construct
  source 1..28: mol_type = other DNA
ggctggcaacatgcctggcacataaagg

SEQ ID NO: 33291 - DNA, 28 bp, synthetic construct
  source 1..28: mol_type = other DNA
ggtttgcattggctggcaacatgcctgg

SEQ ID NO: 33292 - DNA, 28 bp, synthetic construct
  source 1..28: mol_type = other DNA
ttattcatcattggtttgcattggctgg

SEQ ID NO: 33293 - DNA, 28 bp, synthetic construct
  source 1..28: mol_type = other DNA
tttcttattcatcattggtttgcattgg

SEQ ID NO: 33294 - DNA, 28 bp, synthetic construct
  source 1..28: mol_type = other DNA
atgcaaaccaatgatgaataagaaatgg

SEQ ID NO: 33295 - DNA, 28 bp, synthetic construct
  source 1..28: mol_type = other DNA
ggaggaaccatttcttattcatcattgg

SEQ ID NO: 33296 - DNA, 28 bp, synthetic construct
  source 1..28: mol_type = other DNA
atgaataagaaatggttcctcccttagg

SEQ ID NO: 33297 - DNA, 28 bp, synthetic construct
  source 1..28: mol_type = other DNA
tgaataagaaatggttcctcccttaggg

SEQ ID NO: 33298 - DNA, 28 bp, synthetic construct
  source 1..28: mol_type = other DNA
gttcctcccttagggagctccagtctgg

SEQ ID NO: 33299 - DNA, 28 bp, synthetic construct
  source 1..28: mol_type = other DNA
cttccagactggagctccctaagggagg

SEQ ID NO: 33300 - DNA, 28 bp, synthetic construct
  source 1..28: mol_type = other DNA
ctcccttagggagctccagtctggaagg

SEQ ID NO: 33301 - DNA, 28 bp, synthetic construct
  source 1..28: mol_type = other DNA
tcccttagggagctccagtctggaaggg

SEQ ID NO: 33302 - DNA, 28 bp, synthetic construct
  source 1..28: mol_type = other DNA
tcccttccagactggagctccctaaggg

SEQ ID NO: 33303 - DNA, 28 bp, synthetic construct
  source 1..28: mol_type = other DNA
ttcccttccagactggagctccctaagg

SEQ ID NO: 33304 - DNA, 28 bp, synthetic construct
  source 1..28: mol_type = other DNA
ggagctccagtctggaagggaactcagg

SEQ ID NO: 33305 - DNA, 28 bp, synthetic construct
  source 1..28: mol_type = other DNA
agtgagcctgagttcccttccagactgg

SEQ ID NO: 33306 - DNA, 28 bp, synthetic construct
  source 1..28: mol_type = other DNA
tcaggctcactgaattttcttatccagg

SEQ ID NO: 33307 - DNA, 28 bp, synthetic construct
  source 1..28: mol_type = other DNA
tcttatccaggcaacaaactgtcccagg

SEQ ID NO: 33308 - DNA, 28 bp, synthetic construct
  source 1..28: mol_type = other DNA
aaagatcctgggacagtttgttgcctgg

SEQ ID NO: 33309 - DNA, 28 bp, synthetic construct
  source 1..28: mol_type = other DNA
ctcaggaaactgtttaaaagatcctggg

SEQ ID NO: 33310 - DNA, 28 bp, synthetic construct
  source 1..28: mol_type = other DNA
actcaggaaactgtttaaaagatcctgg

SEQ ID NO: 33311 - DNA, 28 bp, synthetic construct
  source 1..28: mol_type = other DNA
ttaatgttacatactcattgcactcagg

SEQ ID NO: 33312 - DNA, 28 bp, synthetic construct
  source 1..28: mol_type = other DNA
taacattaaactcagaacaaagagaagg

SEQ ID NO: 33313 - DNA, 28 bp, synthetic construct
  source 1..28: mol_type = other DNA
aaactcagaacaaagagaaggatctagg

SEQ ID NO: 33314 - DNA, 28 bp, synthetic construct
  source 1..28: mol_type = other DNA
ggatctaggaatgcaatttcctatgtgg

SEQ ID NO: 33315 - DNA, 28 bp, synthetic construct
  source 1..28: mol_type = other DNA
gtaggaacacatctcttggccacatagg

SEQ ID NO: 33316 - DNA, 28 bp, synthetic construct
  source 1..28: mol_type = other DNA
acgtttgtggtaggaacacatctcttgg

SEQ ID NO: 33317 - DNA, 28 bp, synthetic construct
  source 1..28: mol_type = other DNA
tgtgttcctaccacaaacgtattcctgg

SEQ ID NO: 33318 - DNA, 28 bp, synthetic construct
  source 1..28: mol_type = other DNA
cagaagccaggaatacgtttgtggtagg

SEQ ID NO: 33319 - DNA, 28 bp, synthetic construct
  source 1..28: mol_type = other DNA
accacaaacgtattcctggcttctgagg

SEQ ID NO: 33320 - DNA, 28 bp, synthetic construct
  source 1..28: mol_type = other DNA
gcctcagaagccaggaatacgtttgtgg

SEQ ID NO: 33321 - DNA, 28 bp, synthetic construct
  source 1..28: mol_type = other DNA
caatgatcaaagtgcctcagaagccagg

SEQ ID NO: 33322 - DNA, 28 bp, synthetic construct
  source 1..28: mol_type = other DNA
tatttactattaaaaatggctgcatggg

SEQ ID NO: 33323 - DNA, 28 bp, synthetic construct
  source 1..28: mol_type = other DNA
ctatttactattaaaaatggctgcatgg

SEQ ID NO: 33324 - DNA, 28 bp, synthetic construct
  source 1..28: mol_type = other DNA
atatttagctatttactattaaaaatgg

SEQ ID NO: 33325 - DNA, 28 bp, synthetic construct
  source 1..28: mol_type = other DNA
agtaaatagctaaatattcagaaatagg

SEQ ID NO: 33326 - DNA, 28 bp, synthetic construct
  source 1..28: mol_type = other DNA
gcacttcacaattatttatttgatttgg

SEQ ID NO: 33327 - DNA, 28 bp, synthetic construct
  source 1..28: mol_type = other DNA
cacttcacaattatttatttgatttggg

SEQ ID NO: 33328 - DNA, 28 bp, synthetic construct
  source 1..28: mol_type = other DNA
ttatttatttgatttgggtagtgtcagg

SEQ ID NO: 33329 - DNA, 28 bp, synthetic construct
  source 1..28: mol_type = other DNA
tatttgatttgggtagtgtcaggctagg

SEQ ID NO: 33330 - DNA, 28 bp, synthetic construct
  source 1..28: mol_type = other DNA
atttgatttgggtagtgtcaggctaggg

SEQ ID NO: 33331 - DNA, 28 bp, synthetic construct
  source 1..28: mol_type = other DNA
agtgtcaggctagggaaacactaccagg

SEQ ID NO: 33332 - DNA, 28 bp, synthetic construct
  source 1..28: mol_type = other DNA
catttctcttcttgtcttggtgtcctgg

SEQ ID NO: 33333 - DNA, 28 bp, synthetic construct
  source 1..28: mol_type = other DNA
caccaagacaagaagagaaatgtcccgg

SEQ ID NO: 33334 - DNA, 28 bp, synthetic construct
  source 1..28: mol_type = other DNA
taccgggacatttctcttcttgtcttgg

SEQ ID NO: 33335 - DNA, 28 bp, synthetic construct
  source 1..28: mol_type = other DNA
agacaagaagagaaatgtcccggtatgg

SEQ ID NO: 33336 - DNA, 28 bp, synthetic construct
  source 1..28: mol_type = other DNA
aagaagagaaatgtcccggtatggcagg

SEQ ID NO: 33337 - DNA, 28 bp, synthetic construct
  source 1..28: mol_type = other DNA
agaagagaaatgtcccggtatggcaggg

SEQ ID NO: 33338 - DNA, 28 bp, synthetic construct
  source 1..28: mol_type = other DNA
gaagagaaatgtcccggtatggcagggg

SEQ ID NO: 33339 - DNA, 28 bp, synthetic construct
  source 1..28: mol_type = other DNA
gtcccggtatggcaggggccagatgcgg

SEQ ID NO: 33340 - DNA, 28 bp, synthetic construct
  source 1..28: mol_type = other DNA
tcccggtatggcaggggccagatgcggg

SEQ ID NO: 33341 - DNA, 28 bp, synthetic construct
  source 1..28: mol_type = other DNA
tcccgcatctggcccctgccataccggg

SEQ ID NO: 33342 - DNA, 28 bp, synthetic construct
  source 1..28: mol_type = other DNA
ctcccgcatctggcccctgccataccgg

SEQ ID NO: 33343 - DNA, 28 bp, synthetic construct
  source 1..28: mol_type = other DNA
tatggcaggggccagatgcgggagaagg

SEQ ID NO: 33344 - DNA, 28 bp, synthetic construct
  source 1..28: mol_type = other DNA
ggcaggggccagatgcgggagaaggagg

SEQ ID NO: 33345 - DNA, 28 bp, synthetic construct
  source 1..28: mol_type = other DNA
aaactggtcctccttctcccgcatctgg

SEQ ID NO: 33346 - DNA, 28 bp, synthetic construct
  source 1..28: mol_type = other DNA
gaggaccagttttatcaaatgagccagg

SEQ ID NO: 33347 - DNA, 28 bp, synthetic construct
  source 1..28: mol_type = other DNA
gaccagttttatcaaatgagccaggtgg

SEQ ID NO: 33348 - DNA, 28 bp, synthetic construct
  source 1..28: mol_type = other DNA
accagttttatcaaatgagccaggtggg

SEQ ID NO: 33349 - DNA, 28 bp, synthetic construct
  source 1..28: mol_type = other DNA
acccacctggctcatttgataaaactgg

SEQ ID NO: 33350 - DNA, 28 bp, synthetic construct
  source 1..28: mol_type = other DNA
tttatcaaatgagccaggtgggtaatgg

SEQ ID NO: 33351 - DNA, 28 bp, synthetic construct
  source 1..28: mol_type = other DNA
ttatcaaatgagccaggtgggtaatggg

SEQ ID NO: 33352 - DNA, 28 bp, synthetic construct
  source 1..28: mol_type = other DNA
gagccaggtgggtaatgggagtgagtgg

SEQ ID NO: 33353 - DNA, 28 bp, synthetic construct
  source 1..28: mol_type = other DNA
agccaggtgggtaatgggagtgagtggg

SEQ ID NO: 33354 - DNA, 28 bp, synthetic construct
  source 1..28: mol_type = other DNA
ctcccactcactcccattacccacctgg

SEQ ID NO: 33355 - DNA, 28 bp, synthetic construct
  source 1..28: mol_type = other DNA
gggagtgagtgggagcttcaagtcatgg

SEQ ID NO: 33356 - DNA, 28 bp, synthetic construct
  source 1..28: mol_type = other DNA
ggagcttcaagtcatggagaacagacgg

SEQ ID NO: 33357 - DNA, 28 bp, synthetic construct
  source 1..28: mol_type = other DNA
gacggagtgttctaagaactcagcgagg

SEQ ID NO: 33358 - DNA, 28 bp, synthetic construct
  source 1..28: mol_type = other DNA
cagcgaggacactcttcaagccacgagg

SEQ ID NO: 33359 - DNA, 28 bp, synthetic construct
  source 1..28: mol_type = other DNA
ctagagttctaggagctcagcctcgtgg

SEQ ID NO: 33360 - DNA, 28 bp, synthetic construct
  source 1..28: mol_type = other DNA
cacgaggctgagctcctagaactctagg

SEQ ID NO: 33361 - DNA, 28 bp, synthetic construct
  source 1..28: mol_type = other DNA
ctgagctcctagaactctaggagacagg

SEQ ID NO: 33362 - DNA, 28 bp, synthetic construct
  source 1..28: mol_type = other DNA
tctagctcctgtctcctagagttctagg

SEQ ID NO: 33363 - DNA, 28 bp, synthetic construct
  source 1..28: mol_type = other DNA
tagaactctaggagacaggagctagagg

SEQ ID NO: 33364 - DNA, 28 bp, synthetic construct
  source 1..28: mol_type = other DNA
ctctaggagacaggagctagaggagagg

SEQ ID NO: 33365 - DNA, 28 bp, synthetic construct
  source 1..28: mol_type = other DNA
taggagacaggagctagaggagaggtgg

SEQ ID NO: 33366 - DNA, 28 bp, synthetic construct
  source 1..28: mol_type = other DNA
aggagacaggagctagaggagaggtggg

SEQ ID NO: 33367 - DNA, 28 bp, synthetic construct
  source 1..28: mol_type = other DNA
agctagaggagaggtgggctctcactgg

SEQ ID NO: 33368 - DNA, 28 bp, synthetic construct
  source 1..28: mol_type = other DNA
ggagaggtgggctctcactggcctgtgg

SEQ ID NO: 33369 - DNA, 28 bp, synthetic construct
  source 1..28: mol_type = other DNA
gctctcactggcctgtggaataaagagg

SEQ ID NO: 33370 - DNA, 28 bp, synthetic construct
  source 1..28: mol_type = other DNA
aggttcatcagcctctttattccacagg

SEQ ID NO: 33371 - DNA, 28 bp, synthetic construct
  source 1..28: mol_type = other DNA
agaggctgatgaaccttcccaagcgagg

SEQ ID NO: 33372 - DNA, 28 bp, synthetic construct
  source 1..28: mol_type = other DNA
gaggctgatgaaccttcccaagcgaggg

SEQ ID NO: 33373 - DNA, 28 bp, synthetic construct
  source 1..28: mol_type = other DNA
ctgcttatgagaccctcgcttgggaagg

SEQ ID NO: 33374 - DNA, 28 bp, synthetic construct
  source 1..28: mol_type = other DNA
cttcccaagcgagggtctcataagcagg

SEQ ID NO: 33375 - DNA, 28 bp, synthetic construct
  source 1..28: mol_type = other DNA
ttcccaagcgagggtctcataagcaggg

SEQ ID NO: 33376 - DNA, 28 bp, synthetic construct
  source 1..28: mol_type = other DNA
ctccctgcttatgagaccctcgcttggg

SEQ ID NO: 33377 - DNA, 28 bp, synthetic construct
  source 1..28: mol_type = other DNA
cctccctgcttatgagaccctcgcttgg

SEQ ID NO: 33378 - DNA, 28 bp, synthetic construct
  source 1..28: mol_type = other DNA
ggtctcataagcagggaggaaagtatgg

SEQ ID NO: 33379 - DNA, 28 bp, synthetic construct
  source 1..28: mol_type = other DNA
gtctcataagcagggaggaaagtatggg

SEQ ID NO: 33380 - DNA, 28 bp, synthetic construct
  source 1..28: mol_type = other DNA
tctcataagcagggaggaaagtatgggg

SEQ ID NO: 33381 - DNA, 28 bp, synthetic construct
  source 1..28: mol_type = other DNA
gcagggaggaaagtatggggcttagagg

SEQ ID NO: 33382 - DNA, 28 bp, synthetic construct
  source 1..28: mol_type = other DNA
cagggaggaaagtatggggcttagaggg

SEQ ID NO: 33383 - DNA, 28 bp, synthetic construct
  source 1..28: mol_type = other DNA
aagtatggggcttagagggagaatcagg

SEQ ID NO: 33384 - DNA, 28 bp, synthetic construct
  source 1..28: mol_type = other DNA
atggggcttagagggagaatcaggctgg

SEQ ID NO: 33385 - DNA, 28 bp, synthetic construct
  source 1..28: mol_type = other DNA
gggcttagagggagaatcaggctggtgg

SEQ ID NO: 33386 - DNA, 28 bp, synthetic construct
  source 1..28: mol_type = other DNA
atatttataaataacaacagctgactgg

SEQ ID NO: 33387 - DNA, 28 bp, synthetic construct
  source 1..28: mol_type = other DNA
cagaaaagttaccaagagaacacagagg

SEQ ID NO: 33388 - DNA, 28 bp, synthetic construct
  source 1..28: mol_type = other DNA
agaaaagttaccaagagaacacagaggg

SEQ ID NO: 33389 - DNA, 28 bp, synthetic construct
  source 1..28: mol_type = other DNA
tattcgagaaccctctgtgttctcttgg

SEQ ID NO: 33390 - DNA, 28 bp, synthetic construct
  source 1..28: mol_type = other DNA
tccgtgtccagttttccttgtccttagg

SEQ ID NO: 33391 - DNA, 28 bp, synthetic construct
  source 1..28: mol_type = other DNA
tcctaaggacaaggaaaactggacacgg

SEQ ID NO: 33392 - DNA, 28 bp, synthetic construct
  source 1..28: mol_type = other DNA
gtgagatcctaaggacaaggaaaactgg

SEQ ID NO: 33393 - DNA, 28 bp, synthetic construct
  source 1..28: mol_type = other DNA
attctgctgtgagatcctaaggacaagg

SEQ ID NO: 33394 - DNA, 28 bp, synthetic construct
  source 1..28: mol_type = other DNA
ggtatcattctgctgtgagatcctaagg

SEQ ID NO: 33395 - DNA, 28 bp, synthetic construct
  source 1..28: mol_type = other DNA
aatataggtgtattcattgtgacaaagg

SEQ ID NO: 33396 - DNA, 28 bp, synthetic construct
  source 1..28: mol_type = other DNA
tggacttacgttatcatagcaatatagg

SEQ ID NO: 33397 - DNA, 28 bp, synthetic construct
  source 1..28: mol_type = other DNA
tatgataacgtaagtccatttgaaatgg

SEQ ID NO: 33398 - DNA, 28 bp, synthetic construct
  source 1..28: mol_type = other DNA
ggtgacagcaagactccatttcaaatgg

SEQ ID NO: 33399 - DNA, 28 bp, synthetic construct
  source 1..28: mol_type = other DNA
ttgaaatggagtcttgctgtcacccagg

SEQ ID NO: 33400 - DNA, 28 bp, synthetic construct
  source 1..28: mol_type = other DNA
aatggagtcttgctgtcacccaggctgg

SEQ ID NO: 33401 - DNA, 28 bp, synthetic construct
  source 1..28: mol_type = other DNA
tgctgtcacccaggctggagtgcagcgg

SEQ ID NO: 33402 - DNA, 28 bp, synthetic construct
  source 1..28: mol_type = other DNA
agatcacgccgctgcactccagcctggg

SEQ ID NO: 33403 - DNA, 28 bp, synthetic construct
  source 1..28: mol_type = other DNA
gagatcacgccgctgcactccagcctgg

SEQ ID NO: 33404 - DNA, 28 bp, synthetic construct
  source 1..28: mol_type = other DNA
cagcttactgcgacctccgcctcccagg

SEQ ID NO: 33405 - DNA, 28 bp, synthetic construct
  source 1..28: mol_type = other DNA
agaacagcttgaacctgggaggcggagg

SEQ ID NO: 33406 - DNA, 28 bp, synthetic construct
  source 1..28: mol_type = other DNA
aggagaacagcttgaacctgggaggcgg

SEQ ID NO: 33407 - DNA, 28 bp, synthetic construct
  source 1..28: mol_type = other DNA
ggcaggagaacagcttgaacctgggagg

SEQ ID NO: 33408 - DNA, 28 bp, synthetic construct
  source 1..28: mol_type = other DNA
tgaggcaggagaacagcttgaacctggg

SEQ ID NO: 33409 - DNA, 28 bp, synthetic construct
  source 1..28: mol_type = other DNA
ctgaggcaggagaacagcttgaacctgg

SEQ ID NO: 33410 - DNA, 28 bp, synthetic construct
  source 1..28: mol_type = other DNA
ctcctgcctcagcttcctgagtagctgg

SEQ ID NO: 33411 - DNA, 28 bp, synthetic construct
  source 1..28: mol_type = other DNA
ttccagctactcaggaagctgaggcagg

SEQ ID NO: 33412 - DNA, 28 bp, synthetic construct
  source 1..28: mol_type = other DNA
gtagttccagctactcaggaagctgagg

SEQ ID NO: 33413 - DNA, 28 bp, synthetic construct
  source 1..28: mol_type = other DNA
cagcttcctgagtagctggaactacagg

SEQ ID NO: 33414 - DNA, 28 bp, synthetic construct
  source 1..28: mol_type = other DNA
cgggcacctgtagttccagctactcagg

SEQ ID NO: 33415 - DNA, 28 bp, synthetic construct
  source 1..28: mol_type = other DNA
aactacaggtgcccgccaccacgcccgg

SEQ ID NO: 33416 - DNA, 28 bp, synthetic construct
  source 1..28: mol_type = other DNA
caaaaaattagccgggcgtggtggcggg

SEQ ID NO: 33417 - DNA, 28 bp, synthetic construct
  source 1..28: mol_type = other DNA
acaaaaaattagccgggcgtggtggcgg

SEQ ID NO: 33418 - DNA, 28 bp, synthetic construct
  source 1..28: mol_type = other DNA
aatacaaaaaattagccgggcgtggtgg

SEQ ID NO: 33419 - DNA, 28 bp, synthetic construct
  source 1..28: mol_type = other DNA
aaaaatacaaaaaattagccgggcgtgg

SEQ ID NO: 33420 - DNA, 28 bp, synthetic construct
  source 1..28: mol_type = other DNA
ctactaaaaatacaaaaaattagccggg

SEQ ID NO: 33421 - DNA, 28 bp, synthetic construct
  source 1..28: mol_type = other DNA
tctactaaaaatacaaaaaattagccgg

SEQ ID NO: 33422 - DNA, 28 bp, synthetic construct
  source 1..28: mol_type = other DNA
aattttttgtatttttagtagagacagg

SEQ ID NO: 33423 - DNA, 28 bp, synthetic construct
  source 1..28: mol_type = other DNA
attttttgtatttttagtagagacaggg

SEQ ID NO: 33424 - DNA, 28 bp, synthetic construct
  source 1..28: mol_type = other DNA
gagacagggtttcaccatgttagccagg

SEQ ID NO: 33425 - DNA, 28 bp, synthetic construct
  source 1..28: mol_type = other DNA
cagggtttcaccatgttagccaggatgg

SEQ ID NO: 33426 - DNA, 28 bp, synthetic construct
  source 1..28: mol_type = other DNA
gagatcaagaccatcctggctaacatgg

SEQ ID NO: 33427 - DNA, 28 bp, synthetic construct
  source 1..28: mol_type = other DNA
cgaggtcaggagatcaagaccatcctgg

SEQ ID NO: 33428 - DNA, 28 bp, synthetic construct
  source 1..28: mol_type = other DNA
tcctgacctcgtgatccgcccgcctcgg

SEQ ID NO: 33429 - DNA, 28 bp, synthetic construct
  source 1..28: mol_type = other DNA
gccgaggcgggcggatcacgaggtcagg

SEQ ID NO: 33430 - DNA, 28 bp, synthetic construct
  source 1..28: mol_type = other DNA
gggaggccgaggcgggcggatcacgagg

SEQ ID NO: 33431 - DNA, 28 bp, synthetic construct
  source 1..28: mol_type = other DNA
cagcattttgggaggccgaggcgggcgg

SEQ ID NO: 33432 - DNA, 28 bp, synthetic construct
  source 1..28: mol_type = other DNA
cgcccgcctcggcctcccaaaatgctgg

SEQ ID NO: 33433 - DNA, 28 bp, synthetic construct
  source 1..28: mol_type = other DNA
gcccgcctcggcctcccaaaatgctggg

SEQ ID NO: 33434 - DNA, 28 bp, synthetic construct
  source 1..28: mol_type = other DNA
tcccagcattttgggaggccgaggcggg

SEQ ID NO: 33435 - DNA, 28 bp, synthetic construct
  source 1..28: mol_type = other DNA
atcccagcattttgggaggccgaggcgg

SEQ ID NO: 33436 - DNA, 28 bp, synthetic construct
  source 1..28: mol_type = other DNA
gtaatcccagcattttgggaggccgagg

SEQ ID NO: 33437 - DNA, 28 bp, synthetic construct
  source 1..28: mol_type = other DNA
cggcctcccaaaatgctgggattacagg

SEQ ID NO: 33438 - DNA, 28 bp, synthetic construct
  source 1..28: mol_type = other DNA
acacctgtaatcccagcattttgggagg

SEQ ID NO: 33439 - DNA, 28 bp, synthetic construct
  source 1..28: mol_type = other DNA
ctcacacctgtaatcccagcattttggg

SEQ ID NO: 33440 - DNA, 28 bp, synthetic construct
  source 1..28: mol_type = other DNA
gctcacacctgtaatcccagcattttgg

SEQ ID NO: 33441 - DNA, 28 bp, synthetic construct
  source 1..28: mol_type = other DNA
gattacaggtgtgagccactgcgcccgg

SEQ ID NO: 33442 - DNA, 28 bp, synthetic construct
  source 1..28: mol_type = other DNA
aataaatgactggggccgggcgcagtgg

SEQ ID NO: 33443 - DNA, 28 bp, synthetic construct
  source 1..28: mol_type = other DNA
ctgatagaaataaatgactggggccggg

SEQ ID NO: 33444 - DNA, 28 bp, synthetic construct
  source 1..28: mol_type = other DNA
actgatagaaataaatgactggggccgg

SEQ ID NO: 33445 - DNA, 28 bp, synthetic construct
  source 1..28: mol_type = other DNA
ccatactgatagaaataaatgactgggg

SEQ ID NO: 33446 - DNA, 28 bp, synthetic construct
  source 1..28: mol_type = other DNA
tccatactgatagaaataaatgactggg

SEQ ID NO: 33447 - DNA, 28 bp, synthetic construct
  source 1..28: mol_type = other DNA
gtccatactgatagaaataaatgactgg

SEQ ID NO: 33448 - DNA, 28 bp, synthetic construct
  source 1..28: mol_type = other DNA
tggactcttgcatgctttcttgctttgg

SEQ ID NO: 33449 - DNA, 28 bp, synthetic construct
  source 1..28: mol_type = other DNA
tgattcaggaacagttgactagtattgg

SEQ ID NO: 33450 - DNA, 28 bp, synthetic construct
  source 1..28: mol_type = other DNA
gtcaactgttcctgaatcacatataagg

SEQ ID NO: 33451 - DNA, 28 bp, synthetic construct
  source 1..28: mol_type = other DNA
tagtgtagtaccttatatgtgattcagg

SEQ ID NO: 33452 - DNA, 28 bp, synthetic construct
  source 1..28: mol_type = other DNA
tcacatataaggtactacactatagtgg

SEQ ID NO: 33453 - DNA, 28 bp, synthetic construct
  source 1..28: mol_type = other DNA
ataaggtactacactatagtggtgcagg

SEQ ID NO: 33454 - DNA, 28 bp, synthetic construct
  source 1..28: mol_type = other DNA
tgcaggcactctgtacatacagcaaagg

SEQ ID NO: 33455 - DNA, 28 bp, synthetic construct
  source 1..28: mol_type = other DNA
gcaggcactctgtacatacagcaaaggg

SEQ ID NO: 33456 - DNA, 28 bp, synthetic construct
  source 1..28: mol_type = other DNA
caggcactctgtacatacagcaaagggg

SEQ ID NO: 33457 - DNA, 28 bp, synthetic construct
  source 1..28: mol_type = other DNA
gggcagaattaccatgtgctgcccatgg

SEQ ID NO: 33458 - DNA, 28 bp, synthetic construct
  source 1..28: mol_type = other DNA
taccatgtgctgcccatggtagtgatgg

SEQ ID NO: 33459 - DNA, 28 bp, synthetic construct
  source 1..28: mol_type = other DNA
gtccatcactaccatgggcagcacatgg

SEQ ID NO: 33460 - DNA, 28 bp, synthetic construct
  source 1..28: mol_type = other DNA
tttgatttgtgtccatcactaccatggg

SEQ ID NO: 33461 - DNA, 28 bp, synthetic construct
  source 1..28: mol_type = other DNA
ctttgatttgtgtccatcactaccatgg

SEQ ID NO: 33462 - DNA, 28 bp, synthetic construct
  source 1..28: mol_type = other DNA
catggtagtgatggacacaaatcaaagg

SEQ ID NO: 33463 - DNA, 28 bp, synthetic construct
  source 1..28: mol_type = other DNA
aaggcttatcattacctgtgcaaagtgg

SEQ ID NO: 33464 - DNA, 28 bp, synthetic construct
  source 1..28: mol_type = other DNA
tacctgtgcaaagtggttaaaattctgg

SEQ ID NO: 33465 - DNA, 28 bp, synthetic construct
  source 1..28: mol_type = other DNA
ggccagaattttaaccactttgcacagg

SEQ ID NO: 33466 - DNA, 28 bp, synthetic construct
  source 1..28: mol_type = other DNA
attgttgggactgaaaatgtctttttgg

SEQ ID NO: 33467 - DNA, 28 bp, synthetic construct
  source 1..28: mol_type = other DNA
tggtcaagcatctgattgcattgttggg

SEQ ID NO: 33468 - DNA, 28 bp, synthetic construct
  source 1..28: mol_type = other DNA
ctggtcaagcatctgattgcattgttgg

SEQ ID NO: 33469 - DNA, 28 bp, synthetic construct
  source 1..28: mol_type = other DNA
aatttggaaagtatactgcttttgctgg

SEQ ID NO: 33470 - DNA, 28 bp, synthetic construct
  source 1..28: mol_type = other DNA
aaaagcagtatactttccaaattatagg

SEQ ID NO: 33471 - DNA, 28 bp, synthetic construct
  source 1..28: mol_type = other DNA
tgtggatatgcagatacctataatttgg

SEQ ID NO: 33472 - DNA, 28 bp, synthetic construct
  source 1..28: mol_type = other DNA
atccacacatataccttaaaactactgg

SEQ ID NO: 33473 - DNA, 28 bp, synthetic construct
  source 1..28: mol_type = other DNA
tccacacatataccttaaaactactggg

SEQ ID NO: 33474 - DNA, 28 bp, synthetic construct
  source 1..28: mol_type = other DNA
ccacacatataccttaaaactactgggg

SEQ ID NO: 33475 - DNA, 28 bp, synthetic construct
  source 1..28: mol_type = other DNA
cacacatataccttaaaactactggggg

SEQ ID NO: 33476 - DNA, 28 bp, synthetic construct
  source 1..28: mol_type = other DNA
caattgaatgcccccagtagttttaagg

SEQ ID NO: 33477 - DNA, 28 bp, synthetic construct
  source 1..28: mol_type = other DNA
gggggcattcaattgccaaatcaaatgg

SEQ ID NO: 33478 - DNA, 28 bp, synthetic construct
  source 1..28: mol_type = other DNA
caattgccaaatcaaatggacaccttgg

SEQ ID NO: 33479 - DNA, 28 bp, synthetic construct
  source 1..28: mol_type = other DNA
aggagaccaaggtgtccatttgatttgg

SEQ ID NO: 33480 - DNA, 28 bp, synthetic construct
  source 1..28: mol_type = other DNA
gacaccttggtctccttgtcttgcttgg

SEQ ID NO: 33481 - DNA, 28 bp, synthetic construct
  source 1..28: mol_type = other DNA
gtgaccaagcaagacaaggagaccaagg

SEQ ID NO: 33482 - DNA, 28 bp, synthetic construct
  source 1..28: mol_type = other DNA
taaatcagagtgaccaagcaagacaagg

SEQ ID NO: 33483 - DNA, 28 bp, synthetic construct
  source 1..28: mol_type = other DNA
aagctgcacaagaacagctcaatgaagg

SEQ ID NO: 33484 - DNA, 28 bp, synthetic construct
  source 1..28: mol_type = other DNA
tcttgtgcagcttctctgattctcgagg

SEQ ID NO: 33485 - DNA, 28 bp, synthetic construct
  source 1..28: mol_type = other DNA
ttcctttgatgattctacccctttctgg

SEQ ID NO: 33486 - DNA, 28 bp, synthetic construct
  source 1..28: mol_type = other DNA
ggccagaaaggggtagaatcatcaaagg

SEQ ID NO: 33487 - DNA, 28 bp, synthetic construct
  source 1..28: mol_type = other DNA
gcagctctgaagggtggccagaaagggg

SEQ ID NO: 33488 - DNA, 28 bp, synthetic construct
  source 1..28: mol_type = other DNA
agcagctctgaagggtggccagaaaggg

SEQ ID NO: 33489 - DNA, 28 bp, synthetic construct
  source 1..28: mol_type = other DNA
cagcagctctgaagggtggccagaaagg

SEQ ID NO: 33490 - DNA, 28 bp, synthetic construct
  source 1..28: mol_type = other DNA
ctagggtgacagcagctctgaagggtgg

SEQ ID NO: 33491 - DNA, 28 bp, synthetic construct
  source 1..28: mol_type = other DNA
cacccttcagagctgctgtcaccctagg

SEQ ID NO: 33492 - DNA, 28 bp, synthetic construct
  source 1..28: mol_type = other DNA
atcctagggtgacagcagctctgaaggg

SEQ ID NO: 33493 - DNA, 28 bp, synthetic construct
  source 1..28: mol_type = other DNA
gatcctagggtgacagcagctctgaagg

SEQ ID NO: 33494 - DNA, 28 bp, synthetic construct
  source 1..28: mol_type = other DNA
agaagaaaactgaggctggatcctaggg

SEQ ID NO: 33495 - DNA, 28 bp, synthetic construct
  source 1..28: mol_type = other DNA
cagaagaaaactgaggctggatcctagg

SEQ ID NO: 33496 - DNA, 28 bp, synthetic construct
  source 1..28: mol_type = other DNA
aggatccagcctcagttttcttctgagg

SEQ ID NO: 33497 - DNA, 28 bp, synthetic construct
  source 1..28: mol_type = other DNA
agagacctcagaagaaaactgaggctgg

SEQ ID NO: 33498 - DNA, 28 bp, synthetic construct
  source 1..28: mol_type = other DNA
catgagagacctcagaagaaaactgagg

SEQ ID NO: 33499 - DNA, 28 bp, synthetic construct
  source 1..28: mol_type = other DNA
tggatgtcatggttgggagtggatgagg

SEQ ID NO: 33500 - DNA, 28 bp, synthetic construct
  source 1..28: mol_type = other DNA
cagtcatggatgtcatggttgggagtgg

SEQ ID NO: 33501 - DNA, 28 bp, synthetic construct
  source 1..28: mol_type = other DNA
ggaagcagtcatggatgtcatggttggg

SEQ ID NO: 33502 - DNA, 28 bp, synthetic construct
  source 1..28: mol_type = other DNA
aggaagcagtcatggatgtcatggttgg

SEQ ID NO: 33503 - DNA, 28 bp, synthetic construct
  source 1..28: mol_type = other DNA
ttggaggaagcagtcatggatgtcatgg

SEQ ID NO: 33504 - DNA, 28 bp, synthetic construct
  source 1..28: mol_type = other DNA
gggtggcacttggaggaagcagtcatgg

SEQ ID NO: 33505 - DNA, 28 bp, synthetic construct
  source 1..28: mol_type = other DNA
tgcttcctccaagtgccaccccctcagg

SEQ ID NO: 33506 - DNA, 28 bp, synthetic construct
  source 1..28: mol_type = other DNA
agtggcctgagggggtggcacttggagg

SEQ ID NO: 33507 - DNA, 28 bp, synthetic construct
  source 1..28: mol_type = other DNA
cgcagtggcctgagggggtggcacttgg

SEQ ID NO: 33508 - DNA, 28 bp, synthetic construct
  source 1..28: mol_type = other DNA
tgccaccccctcaggccactgcgcctgg

SEQ ID NO: 33509 - DNA, 28 bp, synthetic construct
  source 1..28: mol_type = other DNA
gccaccccctcaggccactgcgcctggg

SEQ ID NO: 33510 - DNA, 28 bp, synthetic construct
  source 1..28: mol_type = other DNA
gcccaggcgcagtggcctgagggggtgg

SEQ ID NO: 33511 - DNA, 28 bp, synthetic construct
  source 1..28: mol_type = other DNA
gatgcccaggcgcagtggcctgaggggg

SEQ ID NO: 33512 - DNA, 28 bp, synthetic construct
  source 1..28: mol_type = other DNA
agatgcccaggcgcagtggcctgagggg

SEQ ID NO: 33513 - DNA, 28 bp, synthetic construct
  source 1..28: mol_type = other DNA
gagatgcccaggcgcagtggcctgaggg

SEQ ID NO: 33514 - DNA, 28 bp, synthetic construct
  source 1..28: mol_type = other DNA
agagatgcccaggcgcagtggcctgagg

SEQ ID NO: 33515 - DNA, 28 bp, synthetic construct
  source 1..28: mol_type = other DNA
acagtgcagagatgcccaggcgcagtgg

SEQ ID NO: 33516 - DNA, 28 bp, synthetic construct
  source 1..28: mol_type = other DNA
actgcgcctgggcatctctgcactgtgg

SEQ ID NO: 33517 - DNA, 28 bp, synthetic construct
  source 1..28: mol_type = other DNA
aggaagccacagtgcagagatgcccagg

SEQ ID NO: 33518 - DNA, 28 bp, synthetic construct
  source 1..28: mol_type = other DNA
tgggcatctctgcactgtggcttcctgg

SEQ ID NO: 33519 - DNA, 28 bp, synthetic construct
  source 1..28: mol_type = other DNA
gcatctctgcactgtggcttcctggagg

SEQ ID NO: 33520 - DNA, 28 bp, synthetic construct
  source 1..28: mol_type = other DNA
agataaaatatgagctcgagcctccagg

SEQ ID NO: 33521 - DNA, 28 bp, synthetic construct
  source 1..28: mol_type = other DNA
aggctcgagctcatattttatctcacgg

SEQ ID NO: 33522 - DNA, 28 bp, synthetic construct
  source 1..28: mol_type = other DNA
ggctcgagctcatattttatctcacggg

SEQ ID NO: 33523 - DNA, 28 bp, synthetic construct
  source 1..28: mol_type = other DNA
tatctcacgggcatcttcagcatctagg

SEQ ID NO: 33524 - DNA, 28 bp, synthetic construct
  source 1..28: mol_type = other DNA
catcttcagcatctaggaaaatgcccgg

SEQ ID NO: 33525 - DNA, 28 bp, synthetic construct
  source 1..28: mol_type = other DNA
atgtattgtgtggtgattgcatgccggg

SEQ ID NO: 33526 - DNA, 28 bp, synthetic construct
  source 1..28: mol_type = other DNA
catgtattgtgtggtgattgcatgccgg

SEQ ID NO: 33527 - DNA, 28 bp, synthetic construct
  source 1..28: mol_type = other DNA
attggctcaacaaacatgtattgtgtgg

SEQ ID NO: 33528 - DNA, 28 bp, synthetic construct
  source 1..28: mol_type = other DNA
ttgagccaataagttaatccctacttgg

SEQ ID NO: 33529 - DNA, 28 bp, synthetic construct
  source 1..28: mol_type = other DNA
cacatccaagtagggattaacttattgg

SEQ ID NO: 33530 - DNA, 28 bp, synthetic construct
  source 1..28: mol_type = other DNA
gtcaaggtggaggcacatccaagtaggg

SEQ ID NO: 33531 - DNA, 28 bp, synthetic construct
  source 1..28: mol_type = other DNA
agtcaaggtggaggcacatccaagtagg

SEQ ID NO: 33532 - DNA, 28 bp, synthetic construct
  source 1..28: mol_type = other DNA
tacttggatgtgcctccaccttgactgg

SEQ ID NO: 33533 - DNA, 28 bp, synthetic construct
  source 1..28: mol_type = other DNA
tctggtttgaggccagtcaaggtggagg

SEQ ID NO: 33534 - DNA, 28 bp, synthetic construct
  source 1..28: mol_type = other DNA
ggttctggtttgaggccagtcaaggtgg

SEQ ID NO: 33535 - DNA, 28 bp, synthetic construct
  source 1..28: mol_type = other DNA
ataggttctggtttgaggccagtcaagg

SEQ ID NO: 33536 - DNA, 28 bp, synthetic construct
  source 1..28: mol_type = other DNA
tggggaggtaataggttctggtttgagg

SEQ ID NO: 33537 - DNA, 28 bp, synthetic construct
  source 1..28: mol_type = other DNA
aaccagaacctattacctccccacctgg

SEQ ID NO: 33538 - DNA, 28 bp, synthetic construct
  source 1..28: mol_type = other DNA
ttccaggtggggaggtaataggttctgg

SEQ ID NO: 33539 - DNA, 28 bp, synthetic construct
  source 1..28: mol_type = other DNA
gttggattccaggtggggaggtaatagg

SEQ ID NO: 33540 - DNA, 28 bp, synthetic construct
  source 1..28: mol_type = other DNA
ggtgctcgttggattccaggtggggagg

SEQ ID NO: 33541 - DNA, 28 bp, synthetic construct
  source 1..28: mol_type = other DNA
gtgggtgctcgttggattccaggtgggg

SEQ ID NO: 33542 - DNA, 28 bp, synthetic construct
  source 1..28: mol_type = other DNA
ggtgggtgctcgttggattccaggtggg

SEQ ID NO: 33543 - DNA, 28 bp, synthetic construct
  source 1..28: mol_type = other DNA
aggtgggtgctcgttggattccaggtgg

SEQ ID NO: 33544 - DNA, 28 bp, synthetic construct
  source 1..28: mol_type = other DNA
acctggaatccaacgagcacccacctgg

SEQ ID NO: 33545 - DNA, 28 bp, synthetic construct
  source 1..28: mol_type = other DNA
accaggtgggtgctcgttggattccagg

SEQ ID NO: 33546 - DNA, 28 bp, synthetic construct
  source 1..28: mol_type = other DNA
tgcagaggaccaggtgggtgctcgttgg

SEQ ID NO: 33547 - DNA, 28 bp, synthetic construct
  source 1..28: mol_type = other DNA
gagcacccacctggtcctctgcacgtgg

SEQ ID NO: 33548 - DNA, 28 bp, synthetic construct
  source 1..28: mol_type = other DNA
agcacccacctggtcctctgcacgtggg

SEQ ID NO: 33549 - DNA, 28 bp, synthetic construct
  source 1..28: mol_type = other DNA
aaaacccacgtgcagaggaccaggtggg

SEQ ID NO: 33550 - DNA, 28 bp, synthetic construct
  source 1..28: mol_type = other DNA
caaaacccacgtgcagaggaccaggtgg

SEQ ID NO: 33551 - DNA, 28 bp, synthetic construct
  source 1..28: mol_type = other DNA
agtcaaaacccacgtgcagaggaccagg

SEQ ID NO: 33552 - DNA, 28 bp, synthetic construct
  source 1..28: mol_type = other DNA
agaggaagtcaaaacccacgtgcagagg

SEQ ID NO: 33553 - DNA, 28 bp, synthetic construct
  source 1..28: mol_type = other DNA
tttgttgtctgtagggaggagagagagg

SEQ ID NO: 33554 - DNA, 28 bp, synthetic construct
  source 1..28: mol_type = other DNA
gctaggagttttgttgtctgtagggagg

SEQ ID NO: 33555 - DNA, 28 bp, synthetic construct
  source 1..28: mol_type = other DNA
actgctaggagttttgttgtctgtaggg

SEQ ID NO: 33556 - DNA, 28 bp, synthetic construct
  source 1..28: mol_type = other DNA
cactgctaggagttttgttgtctgtagg

SEQ ID NO: 33557 - DNA, 28 bp, synthetic construct
  source 1..28: mol_type = other DNA
cttgagaaataagatggacactgctagg

SEQ ID NO: 33558 - DNA, 28 bp, synthetic construct
  source 1..28: mol_type = other DNA
tccatcttatttctcaagcttttcttgg

SEQ ID NO: 33559 - DNA, 28 bp, synthetic construct
  source 1..28: mol_type = other DNA
tccaagaaaagcttgagaaataagatgg

SEQ ID NO: 33560 - DNA, 28 bp, synthetic construct
  source 1..28: mol_type = other DNA
agcgtcacaagggatggagaaagggagg

SEQ ID NO: 33561 - DNA, 28 bp, synthetic construct
  source 1..28: mol_type = other DNA
agcagcgtcacaagggatggagaaaggg

SEQ ID NO: 33562 - DNA, 28 bp, synthetic construct
  source 1..28: mol_type = other DNA
aagcagcgtcacaagggatggagaaagg

SEQ ID NO: 33563 - DNA, 28 bp, synthetic construct
  source 1..28: mol_type = other DNA
ttctccatcccttgtgacgctgcttcgg

SEQ ID NO: 33564 - DNA, 28 bp, synthetic construct
  source 1..28: mol_type = other DNA
taaaccgaagcagcgtcacaagggatgg

SEQ ID NO: 33565 - DNA, 28 bp, synthetic construct
  source 1..28: mol_type = other DNA
aatgtaaaccgaagcagcgtcacaaggg

SEQ ID NO: 33566 - DNA, 28 bp, synthetic construct
  source 1..28: mol_type = other DNA
aaatgtaaaccgaagcagcgtcacaagg

SEQ ID NO: 33567 - DNA, 28 bp, synthetic construct
  source 1..28: mol_type = other DNA
cttcggtttacatttcatttctcactgg

SEQ ID NO: 33568 - DNA, 28 bp, synthetic construct
  source 1..28: mol_type = other DNA
aactcctctcttcagtcccttctccagg

SEQ ID NO: 33569 - DNA, 28 bp, synthetic construct
  source 1..28: mol_type = other DNA
agagcctggagaagggactgaagagagg

SEQ ID NO: 33570 - DNA, 28 bp, synthetic construct
  source 1..28: mol_type = other DNA
aaggtgggaaatagagcctggagaaggg

SEQ ID NO: 33571 - DNA, 28 bp, synthetic construct
  source 1..28: mol_type = other DNA
caaggtgggaaatagagcctggagaagg

SEQ ID NO: 33572 - DNA, 28 bp, synthetic construct
  source 1..28: mol_type = other DNA
ctgcagcaaggtgggaaatagagcctgg

SEQ ID NO: 33573 - DNA, 28 bp, synthetic construct
  source 1..28: mol_type = other DNA
aatcatagggggactgcagcaaggtggg

SEQ ID NO: 33574 - DNA, 28 bp, synthetic construct
  source 1..28: mol_type = other DNA
aaatcatagggggactgcagcaaggtgg

SEQ ID NO: 33575 - DNA, 28 bp, synthetic construct
  source 1..28: mol_type = other DNA
tttaaatcatagggggactgcagcaagg

SEQ ID NO: 33576 - DNA, 28 bp, synthetic construct
  source 1..28: mol_type = other DNA
cagtgttaggaatttaaatcataggggg

SEQ ID NO: 33577 - DNA, 28 bp, synthetic construct
  source 1..28: mol_type = other DNA
ccagtgttaggaatttaaatcatagggg

SEQ ID NO: 33578 - DNA, 28 bp, synthetic construct
  source 1..28: mol_type = other DNA
gccagtgttaggaatttaaatcataggg

SEQ ID NO: 33579 - DNA, 28 bp, synthetic construct
  source 1..28: mol_type = other DNA
agccagtgttaggaatttaaatcatagg

SEQ ID NO: 33580 - DNA, 28 bp, synthetic construct
  source 1..28: mol_type = other DNA
aaattcctaacactggctgcttcttagg

SEQ ID NO: 33581 - DNA, 28 bp, synthetic construct
  source 1..28: mol_type = other DNA
aattcctaacactggctgcttcttaggg

SEQ ID NO: 33582 - DNA, 28 bp, synthetic construct
  source 1..28: mol_type = other DNA
tctaccctaagaagcagccagtgttagg

SEQ ID NO: 33583 - DNA, 28 bp, synthetic construct
  source 1..28: mol_type = other DNA
cactggctgcttcttagggtagacaagg

SEQ ID NO: 33584 - DNA, 28 bp, synthetic construct
  source 1..28: mol_type = other DNA
ttcttagggtagacaaggctcttcatgg

SEQ ID NO: 33585 - DNA, 28 bp, synthetic construct
  source 1..28: mol_type = other DNA
tagggtagacaaggctcttcatggttgg

SEQ ID NO: 33586 - DNA, 28 bp, synthetic construct
  source 1..28: mol_type = other DNA
gcctcagctgactgcagctgctgcctgg

SEQ ID NO: 33587 - DNA, 28 bp, synthetic construct
  source 1..28: mol_type = other DNA
accaggcagcagctgcagtcagctgagg

SEQ ID NO: 33588 - DNA, 28 bp, synthetic construct
  source 1..28: mol_type = other DNA
agtattgagttacagggctgggaccagg

SEQ ID NO: 33589 - DNA, 28 bp, synthetic construct
  source 1..28: mol_type = other DNA
tggtcccagccctgtaactcaatactgg

SEQ ID NO: 33590 - DNA, 28 bp, synthetic construct
  source 1..28: mol_type = other DNA
cattccagtattgagttacagggctggg

SEQ ID NO: 33591 - DNA, 28 bp, synthetic construct
  source 1..28: mol_type = other DNA
tcattccagtattgagttacagggctgg

SEQ ID NO: 33592 - DNA, 28 bp, synthetic construct
  source 1..28: mol_type = other DNA
tgcatcattccagtattgagttacaggg

SEQ ID NO: 33593 - DNA, 28 bp, synthetic construct
  source 1..28: mol_type = other DNA
ttgcatcattccagtattgagttacagg

SEQ ID NO: 33594 - DNA, 28 bp, synthetic construct
  source 1..28: mol_type = other DNA
tttatagttccacttctctgagtctcgg

SEQ ID NO: 33595 - DNA, 28 bp, synthetic construct
  source 1..28: mol_type = other DNA
agttccacttctctgagtctcggcctgg

SEQ ID NO: 33596 - DNA, 28 bp, synthetic construct
  source 1..28: mol_type = other DNA
gttccacttctctgagtctcggcctggg

SEQ ID NO: 33597 - DNA, 28 bp, synthetic construct
  source 1..28: mol_type = other DNA
cagcccaggccgagactcagagaagtgg

SEQ ID NO: 33598 - DNA, 28 bp, synthetic construct
  source 1..28: mol_type = other DNA
gggcatcaggcaggaagggcagcccagg

SEQ ID NO: 33599 - DNA, 28 bp, synthetic construct
  source 1..28: mol_type = other DNA
cagggagaagggcatcaggcaggaaggg

SEQ ID NO: 33600 - DNA, 28 bp, synthetic construct
  source 1..28: mol_type = other DNA
acagggagaagggcatcaggcaggaagg

SEQ ID NO: 33601 - DNA, 28 bp, synthetic construct
  source 1..28: mol_type = other DNA
gagaacagggagaagggcatcaggcagg

SEQ ID NO: 33602 - DNA, 28 bp, synthetic construct
  source 1..28: mol_type = other DNA
aaatgagaacagggagaagggcatcagg

SEQ ID NO: 33603 - DNA, 28 bp, synthetic construct
  source 1..28: mol_type = other DNA
gagtaataaatgagaacagggagaaggg

SEQ ID NO: 33604 - DNA, 28 bp, synthetic construct
  source 1..28: mol_type = other DNA
tgagtaataaatgagaacagggagaagg

SEQ ID NO: 33605 - DNA, 28 bp, synthetic construct
  source 1..28: mol_type = other DNA
gaggagtgagtaataaatgagaacaggg

SEQ ID NO: 33606 - DNA, 28 bp, synthetic construct
  source 1..28: mol_type = other DNA
tgaggagtgagtaataaatgagaacagg

SEQ ID NO: 33607 - DNA, 28 bp, synthetic construct
  source 1..28: mol_type = other DNA
actcactcctcaaagaccaccccaaagg

SEQ ID NO: 33608 - DNA, 28 bp, synthetic construct
  source 1..28: mol_type = other DNA
ctcactcctcaaagaccaccccaaaggg

SEQ ID NO: 33609 - DNA, 28 bp, synthetic construct
  source 1..28: mol_type = other DNA
gctgtgccctttggggtggtctttgagg

SEQ ID NO: 33610 - DNA, 28 bp, synthetic construct
  source 1..28: mol_type = other DNA
gaccaccccaaagggcacagctttttgg

SEQ ID NO: 33611 - DNA, 28 bp, synthetic construct
  source 1..28: mol_type = other DNA
caccaaaaagctgtgccctttggggtgg

SEQ ID NO: 33612 - DNA, 28 bp, synthetic construct
  source 1..28: mol_type = other DNA
gagcaccaaaaagctgtgccctttgggg

SEQ ID NO: 33613 - DNA, 28 bp, synthetic construct
  source 1..28: mol_type = other DNA
tgagcaccaaaaagctgtgccctttggg

SEQ ID NO: 33614 - DNA, 28 bp, synthetic construct
  source 1..28: mol_type = other DNA
ctgagcaccaaaaagctgtgccctttgg

SEQ ID NO: 33615 - DNA, 28 bp, synthetic construct
  source 1..28: mol_type = other DNA
gggtacagcagagggtaattcaataagg

SEQ ID NO: 33616 - DNA, 28 bp, synthetic construct
  source 1..28: mol_type = other DNA
cactaatagacatgggtacagcagaggg

SEQ ID NO: 33617 - DNA, 28 bp, synthetic construct
  source 1..28: mol_type = other DNA
gcactaatagacatgggtacagcagagg

SEQ ID NO: 33618 - DNA, 28 bp, synthetic construct
  source 1..28: mol_type = other DNA
gagtggcaagtgcactaatagacatggg

SEQ ID NO: 33619 - DNA, 28 bp, synthetic construct
  source 1..28: mol_type = other DNA
ggagtggcaagtgcactaatagacatgg

SEQ ID NO: 33620 - DNA, 28 bp, synthetic construct
  source 1..28: mol_type = other DNA
tattagtgcacttgccactccacactgg

SEQ ID NO: 33621 - DNA, 28 bp, synthetic construct
  source 1..28: mol_type = other DNA
gaagactaatcattccagtgtggagtgg

SEQ ID NO: 33622 - DNA, 28 bp, synthetic construct
  source 1..28: mol_type = other DNA
gacatgaagactaatcattccagtgtgg

SEQ ID NO: 33623 - DNA, 28 bp, synthetic construct
  source 1..28: mol_type = other DNA
actgtcaactgagaagcacatgagtagg

SEQ ID NO: 33624 - DNA, 28 bp, synthetic construct
  source 1..28: mol_type = other DNA
ggcactggagatacagaaaggagtaagg

SEQ ID NO: 33625 - DNA, 28 bp, synthetic construct
  source 1..28: mol_type = other DNA
actcctttctgtatctccagtgccttgg

SEQ ID NO: 33626 - DNA, 28 bp, synthetic construct
  source 1..28: mol_type = other DNA
tctccaaggcactggagatacagaaagg

SEQ ID NO: 33627 - DNA, 28 bp, synthetic construct
  source 1..28: mol_type = other DNA
tgtatctccagtgccttggagacacagg

SEQ ID NO: 33628 - DNA, 28 bp, synthetic construct
  source 1..28: mol_type = other DNA
ataaatacctgtgtctccaaggcactgg

SEQ ID NO: 33629 - DNA, 28 bp, synthetic construct
  source 1..28: mol_type = other DNA
aattaaataaatacctgtgtctccaagg

SEQ ID NO: 33630 - DNA, 28 bp, synthetic construct
  source 1..28: mol_type = other DNA
aaaagagcattcaccccttcaaaatagg

SEQ ID NO: 33631 - DNA, 28 bp, synthetic construct
  source 1..28: mol_type = other DNA
gcaggtcttgtctcctattttgaagggg

SEQ ID NO: 33632 - DNA, 28 bp, synthetic construct
  source 1..28: mol_type = other DNA
tgcaggtcttgtctcctattttgaaggg

SEQ ID NO: 33633 - DNA, 28 bp, synthetic construct
  source 1..28: mol_type = other DNA
ttgcaggtcttgtctcctattttgaagg

SEQ ID NO: 33634 - DNA, 28 bp, synthetic construct
  source 1..28: mol_type = other DNA
gtcgtggatcgactgtgctctttgcagg

SEQ ID NO: 33635 - DNA, 28 bp, synthetic construct
  source 1..28: mol_type = other DNA
agcacagtcgatccacgactccaaatgg

SEQ ID NO: 33636 - DNA, 28 bp, synthetic construct
  source 1..28: mol_type = other DNA
agtcgatccacgactccaaatggaatgg

SEQ ID NO: 33637 - DNA, 28 bp, synthetic construct
  source 1..28: mol_type = other DNA
atgtattccattccatttggagtcgtgg

SEQ ID NO: 33638 - DNA, 28 bp, synthetic construct
  source 1..28: mol_type = other DNA
tattttaaatgtattccattccatttgg

SEQ ID NO: 33639 - DNA, 28 bp, synthetic construct
  source 1..28: mol_type = other DNA
gaatggaatacatttaaaatacatctgg

SEQ ID NO: 33640 - DNA, 28 bp, synthetic construct
  source 1..28: mol_type = other DNA
gaatacatttaaaatacatctggagtgg

SEQ ID NO: 33641 - DNA, 28 bp, synthetic construct
  source 1..28: mol_type = other DNA
aatacatttaaaatacatctggagtggg

SEQ ID NO: 33642 - DNA, 28 bp, synthetic construct
  source 1..28: mol_type = other DNA
gcttactttaaaaaacaacacttagagg

SEQ ID NO: 33643 - DNA, 28 bp, synthetic construct
  source 1..28: mol_type = other DNA
tttaaaaaacaacacttagaggccaagg

SEQ ID NO: 33644 - DNA, 28 bp, synthetic construct
  source 1..28: mol_type = other DNA
aaaaacaacacttagaggccaaggcagg

SEQ ID NO: 33645 - DNA, 28 bp, synthetic construct
  source 1..28: mol_type = other DNA
aacaacacttagaggccaaggcaggtgg

SEQ ID NO: 33646 - DNA, 28 bp, synthetic construct
  source 1..28: mol_type = other DNA
gaggccaaggcaggtggatcacctgagg

SEQ ID NO: 33647 - DNA, 28 bp, synthetic construct
  source 1..28: mol_type = other DNA
ctgacctcaggtgatccacctgccttgg

SEQ ID NO: 33648 - DNA, 28 bp, synthetic construct
  source 1..28: mol_type = other DNA
caaggcaggtggatcacctgaggtcagg

SEQ ID NO: 33649 - DNA, 28 bp, synthetic construct
  source 1..28: mol_type = other DNA
atgctggtctcgaactcctgacctcagg

SEQ ID NO: 33650 - DNA, 28 bp, synthetic construct
  source 1..28: mol_type = other DNA
gagttcgagaccagcatgaccaatatgg

SEQ ID NO: 33651 - DNA, 28 bp, synthetic construct
  source 1..28: mol_type = other DNA
tggggtctcaccatattggtcatgctgg

SEQ ID NO: 33652 - DNA, 28 bp, synthetic construct
  source 1..28: mol_type = other DNA
tggtagagatggggtctcaccatattgg

SEQ ID NO: 33653 - DNA, 28 bp, synthetic construct
  source 1..28: mol_type = other DNA
aatttttgtatttttggtagagatgggg

SEQ ID NO: 33654 - DNA, 28 bp, synthetic construct
  source 1..28: mol_type = other DNA
taatttttgtatttttggtagagatggg

SEQ ID NO: 33655 - DNA, 28 bp, synthetic construct
  source 1..28: mol_type = other DNA
ctaatttttgtatttttggtagagatgg

SEQ ID NO: 33656 - DNA, 28 bp, synthetic construct
  source 1..28: mol_type = other DNA
ctctaccaaaaatacaaaaattagctgg

SEQ ID NO: 33657 - DNA, 28 bp, synthetic construct
  source 1..28: mol_type = other DNA
tctaccaaaaatacaaaaattagctggg

SEQ ID NO: 33658 - DNA, 28 bp, synthetic construct
  source 1..28: mol_type = other DNA
catgcccagctaatttttgtatttttgg

SEQ ID NO: 33659 - DNA, 28 bp, synthetic construct
  source 1..28: mol_type = other DNA
aaatacaaaaattagctgggcatgatgg

SEQ ID NO: 33660 - DNA, 28 bp, synthetic construct
  source 1..28: mol_type = other DNA
gtatgtgcctgtagtcccagctacttgg

SEQ ID NO: 33661 - DNA, 28 bp, synthetic construct
  source 1..28: mol_type = other DNA
tatgtgcctgtagtcccagctacttggg

SEQ ID NO: 33662 - DNA, 28 bp, synthetic construct
  source 1..28: mol_type = other DNA
gtgcctgtagtcccagctacttgggagg

SEQ ID NO: 33663 - DNA, 28 bp, synthetic construct
  source 1..28: mol_type = other DNA
cagcctcccaagtagctgggactacagg

SEQ ID NO: 33664 - DNA, 28 bp, synthetic construct
  source 1..28: mol_type = other DNA
ctgtagtcccagctacttgggaggctgg

SEQ ID NO: 33665 - DNA, 28 bp, synthetic construct
  source 1..28: mol_type = other DNA
tgtagtcccagctacttgggaggctggg

SEQ ID NO: 33666 - DNA, 28 bp, synthetic construct
  source 1..28: mol_type = other DNA
tcccagctacttgggaggctgggacagg

SEQ ID NO: 33667 - DNA, 28 bp, synthetic construct
  source 1..28: mol_type = other DNA
tcctgtcccagcctcccaagtagctggg

SEQ ID NO: 33668 - DNA, 28 bp, synthetic construct
  source 1..28: mol_type = other DNA
ctcctgtcccagcctcccaagtagctgg

SEQ ID NO: 33669 - DNA, 28 bp, synthetic construct
  source 1..28: mol_type = other DNA
ctgggacaggagaattgcttgaacctgg

SEQ ID NO: 33670 - DNA, 28 bp, synthetic construct
  source 1..28: mol_type = other DNA
tgggacaggagaattgcttgaacctggg

SEQ ID NO: 33671 - DNA, 28 bp, synthetic construct
  source 1..28: mol_type = other DNA
gacaggagaattgcttgaacctgggagg

SEQ ID NO: 33672 - DNA, 28 bp, synthetic construct
  source 1..28: mol_type = other DNA
aggagaattgcttgaacctgggaggtgg

SEQ ID NO: 33673 - DNA, 28 bp, synthetic construct
  source 1..28: mol_type = other DNA
agaattgcttgaacctgggaggtggagg

SEQ ID NO: 33674 - DNA, 28 bp, synthetic construct
  source 1..28: mol_type = other DNA
cggctcactgcaacctccacctcccagg

SEQ ID NO: 33675 - DNA, 28 bp, synthetic construct
  source 1..28: mol_type = other DNA
aggctggagtgcagtcgtgtgatctcgg

SEQ ID NO: 33676 - DNA, 28 bp, synthetic construct
  source 1..28: mol_type = other DNA
gagatcacacgactgcactccagcctgg

SEQ ID NO: 33677 - DNA, 28 bp, synthetic construct
  source 1..28: mol_type = other DNA
agatcacacgactgcactccagcctggg

SEQ ID NO: 33678 - DNA, 28 bp, synthetic construct
  source 1..28: mol_type = other DNA
cagagtctcgctctgtcacccaggctgg

SEQ ID NO: 33679 - DNA, 28 bp, synthetic construct
  source 1..28: mol_type = other DNA
gagacagagtctcgctctgtcacccagg

SEQ ID NO: 33680 - DNA, 28 bp, synthetic construct
  source 1..28: mol_type = other DNA
ttgtggggtttttttgggggtggggggg

SEQ ID NO: 33681 - DNA, 28 bp, synthetic construct
  source 1..28: mol_type = other DNA
gttgtggggtttttttgggggtgggggg

SEQ ID NO: 33682 - DNA, 28 bp, synthetic construct
  source 1..28: mol_type = other DNA
tgttgtggggtttttttgggggtggggg

SEQ ID NO: 33683 - DNA, 28 bp, synthetic construct
  source 1..28: mol_type = other DNA
gtgttgtggggtttttttgggggtgggg

SEQ ID NO: 33684 - DNA, 28 bp, synthetic construct
  source 1..28: mol_type = other DNA
ggtgttgtggggtttttttgggggtggg

SEQ ID NO: 33685 - DNA, 28 bp, synthetic construct
  source 1..28: mol_type = other DNA
aggtgttgtggggtttttttgggggtgg

SEQ ID NO: 33686 - DNA, 28 bp, synthetic construct
  source 1..28: mol_type = other DNA
tttaggtgttgtggggtttttttggggg

SEQ ID NO: 33687 - DNA, 28 bp, synthetic construct
  source 1..28: mol_type = other DNA
atttaggtgttgtggggtttttttgggg

SEQ ID NO: 33688 - DNA, 28 bp, synthetic construct
  source 1..28: mol_type = other DNA
aatttaggtgttgtggggtttttttggg

SEQ ID NO: 33689 - DNA, 28 bp, synthetic construct
  source 1..28: mol_type = other DNA
aaatttaggtgttgtggggtttttttgg

SEQ ID NO: 33690 - DNA, 28 bp, synthetic construct
  source 1..28: mol_type = other DNA
ggttattataaatttaggtgttgtgggg

SEQ ID NO: 33691 - DNA, 28 bp, synthetic construct
  source 1..28: mol_type = other DNA
tggttattataaatttaggtgttgtggg

SEQ ID NO: 33692 - DNA, 28 bp, synthetic construct
  source 1..28: mol_type = other DNA
gtggttattataaatttaggtgttgtgg

SEQ ID NO: 33693 - DNA, 28 bp, synthetic construct
  source 1..28: mol_type = other DNA
taaagattgtggttattataaatttagg

SEQ ID NO: 33694 - DNA, 28 bp, synthetic construct
  source 1..28: mol_type = other DNA
ataataataataataataaagattgtgg

SEQ ID NO: 33695 - DNA, 28 bp, synthetic construct
  source 1..28: mol_type = other DNA
ttgagacagtctcgctctgtcgcccagg

SEQ ID NO: 33696 - DNA, 28 bp, synthetic construct
  source 1..28: mol_type = other DNA
gacagtctcgctctgtcgcccaggctgg

SEQ ID NO: 33697 - DNA, 28 bp, synthetic construct
  source 1..28: mol_type = other DNA
ctctgtcgcccaggctggagtgcagtgg

SEQ ID NO: 33698 - DNA, 28 bp, synthetic construct
  source 1..28: mol_type = other DNA
agatcgcgccactgcactccagcctggg

SEQ ID NO: 33699 - DNA, 28 bp, synthetic construct
  source 1..28: mol_type = other DNA
gagatcgcgccactgcactccagcctgg

SEQ ID NO: 33700 - DNA, 28 bp, synthetic construct
  source 1..28: mol_type = other DNA
aggctggagtgcagtggcgcgatctcgg

SEQ ID NO: 33701 - DNA, 28 bp, synthetic construct
  source 1..28: mol_type = other DNA
tcggctcactgcaagctccgcctcccgg

SEQ ID NO: 33702 - DNA, 28 bp, synthetic construct
  source 1..28: mol_type = other DNA
cggctcactgcaagctccgcctcccggg

SEQ ID NO: 33703 - DNA, 28 bp, synthetic construct
  source 1..28: mol_type = other DNA
aggaaaatggcgtgaacccgggaggcgg

SEQ ID NO: 33704 - DNA, 28 bp, synthetic construct
  source 1..28: mol_type = other DNA
ggcaggaaaatggcgtgaacccgggagg

SEQ ID NO: 33705 - DNA, 28 bp, synthetic construct
  source 1..28: mol_type = other DNA
tgaggcaggaaaatggcgtgaacccggg

SEQ ID NO: 33706 - DNA, 28 bp, synthetic construct
  source 1..28: mol_type = other DNA
ctgaggcaggaaaatggcgtgaacccgg

SEQ ID NO: 33707 - DNA, 28 bp, synthetic construct
  source 1..28: mol_type = other DNA
tactcgggaggctgaggcaggaaaatgg

SEQ ID NO: 33708 - DNA, 28 bp, synthetic construct
  source 1..28: mol_type = other DNA
ttcctgcctcagcctcccgagtagctgg

SEQ ID NO: 33709 - DNA, 28 bp, synthetic construct
  source 1..28: mol_type = other DNA
tcctgcctcagcctcccgagtagctggg

SEQ ID NO: 33710 - DNA, 28 bp, synthetic construct
  source 1..28: mol_type = other DNA
tcccagctactcgggaggctgaggcagg

SEQ ID NO: 33711 - DNA, 28 bp, synthetic construct
  source 1..28: mol_type = other DNA
gtagtcccagctactcgggaggctgagg

SEQ ID NO: 33712 - DNA, 28 bp, synthetic construct
  source 1..28: mol_type = other DNA
cagcctcccgagtagctgggactacagg

SEQ ID NO: 33713 - DNA, 28 bp, synthetic construct
  source 1..28: mol_type = other DNA
gtgcctgtagtcccagctactcgggagg

SEQ ID NO: 33714 - DNA, 28 bp, synthetic construct
  source 1..28: mol_type = other DNA
cgggtgcctgtagtcccagctactcggg

SEQ ID NO: 33715 - DNA, 28 bp, synthetic construct
  source 1..28: mol_type = other DNA
gcgggtgcctgtagtcccagctactcgg

SEQ ID NO: 33716 - DNA, 28 bp, synthetic construct
  source 1..28: mol_type = other DNA
gactacaggcacccgccaccacgcccgg

SEQ ID NO: 33717 - DNA, 28 bp, synthetic construct
  source 1..28: mol_type = other DNA
aaaaaaattagccgggcgtggtggcggg

SEQ ID NO: 33718 - DNA, 28 bp, synthetic construct
  source 1..28: mol_type = other DNA
caaaaaaattagccgggcgtggtggcgg

SEQ ID NO: 33719 - DNA, 28 bp, synthetic construct
  source 1..28: mol_type = other DNA
atacaaaaaaattagccgggcgtggtgg

SEQ ID NO: 33720 - DNA, 28 bp, synthetic construct
  source 1..28: mol_type = other DNA
aaaatacaaaaaaattagccgggcgtgg

SEQ ID NO: 33721 - DNA, 28 bp, synthetic construct
  source 1..28: mol_type = other DNA
tactaaaaatacaaaaaaattagccggg

SEQ ID NO: 33722 - DNA, 28 bp, synthetic construct
  source 1..28: mol_type = other DNA
ctactaaaaatacaaaaaaattagccgg

SEQ ID NO: 33723 - DNA, 28 bp, synthetic construct
  source 1..28: mol_type = other DNA
aatttttttgtatttttagtagagatgg

SEQ ID NO: 33724 - DNA, 28 bp, synthetic construct
  source 1..28: mol_type = other DNA
atttttttgtatttttagtagagatggg

SEQ ID NO: 33725 - DNA, 28 bp, synthetic construct
  source 1..28: mol_type = other DNA
tttttttgtatttttagtagagatgggg

SEQ ID NO: 33726 - DNA, 28 bp, synthetic construct
  source 1..28: mol_type = other DNA
gagatggggtttcaccgtgttagccagg

SEQ ID NO: 33727 - DNA, 28 bp, synthetic construct
  source 1..28: mol_type = other DNA
tggggtttcaccgtgttagccaggatgg

SEQ ID NO: 33728 - DNA, 28 bp, synthetic construct
  source 1..28: mol_type = other DNA
gagatcgagaccatcctggctaacacgg

SEQ ID NO: 33729 - DNA, 28 bp, synthetic construct
  source 1..28: mol_type = other DNA
cgaggtcaggagatcgagaccatcctgg

SEQ ID NO: 33730 - DNA, 28 bp, synthetic construct
  source 1..28: mol_type = other DNA
tcctgacctcgtgatccgcccgcctcgg

SEQ ID NO: 33731 - DNA, 28 bp, synthetic construct
  source 1..28: mol_type = other DNA
gccgaggcgggcggatcacgaggtcagg

SEQ ID NO: 33732 - DNA, 28 bp, synthetic construct
  source 1..28: mol_type = other DNA
gggaggccgaggcgggcggatcacgagg

SEQ ID NO: 33733 - DNA, 28 bp, synthetic construct
  source 1..28: mol_type = other DNA
cagcactttgggaggccgaggcgggcgg

SEQ ID NO: 33734 - DNA, 28 bp, synthetic construct
  source 1..28: mol_type = other DNA
cgcccgcctcggcctcccaaagtgctgg

SEQ ID NO: 33735 - DNA, 28 bp, synthetic construct
  source 1..28: mol_type = other DNA
gcccgcctcggcctcccaaagtgctggg

SEQ ID NO: 33736 - DNA, 28 bp, synthetic construct
  source 1..28: mol_type = other DNA
tcccagcactttgggaggccgaggcggg

SEQ ID NO: 33737 - DNA, 28 bp, synthetic construct
  source 1..28: mol_type = other DNA
atcccagcactttgggaggccgaggcgg

SEQ ID NO: 33738 - DNA, 28 bp, synthetic construct
  source 1..28: mol_type = other DNA
gtaatcccagcactttgggaggccgagg

SEQ ID NO: 33739 - DNA, 28 bp, synthetic construct
  source 1..28: mol_type = other DNA
cggcctcccaaagtgctgggattacagg

SEQ ID NO: 33740 - DNA, 28 bp, synthetic construct
  source 1..28: mol_type = other DNA
acgcctgtaatcccagcactttgggagg

SEQ ID NO: 33741 - DNA, 28 bp, synthetic construct
  source 1..28: mol_type = other DNA
ctcacgcctgtaatcccagcactttggg

SEQ ID NO: 33742 - DNA, 28 bp, synthetic construct
  source 1..28: mol_type = other DNA
gctcacgcctgtaatcccagcactttgg

SEQ ID NO: 33743 - DNA, 28 bp, synthetic construct
  source 1..28: mol_type = other DNA
gattacaggcgtgagccaccacgctcgg

SEQ ID NO: 33744 - DNA, 28 bp, synthetic construct
  source 1..28: mol_type = other DNA
gattgtggttattggccgagcgtggtgg

SEQ ID NO: 33745 - DNA, 28 bp, synthetic construct
  source 1..28: mol_type = other DNA
aaagattgtggttattggccgagcgtgg

SEQ ID NO: 33746 - DNA, 28 bp, synthetic construct
  source 1..28: mol_type = other DNA
aatgaactttaaagattgtggttattgg

SEQ ID NO: 33747 - DNA, 28 bp, synthetic construct
  source 1..28: mol_type = other DNA
aatagacaatgaactttaaagattgtgg

SEQ ID NO: 33748 - DNA, 28 bp, synthetic construct
  source 1..28: mol_type = other DNA
cattgtctattaactttaaaaacaaagg

SEQ ID NO: 33749 - DNA, 28 bp, synthetic construct
  source 1..28: mol_type = other DNA
tctattaactttaaaaacaaaggaatgg

SEQ ID NO: 33750 - DNA, 28 bp, synthetic construct
  source 1..28: mol_type = other DNA
ttaactttaaaaacaaaggaatggttgg

SEQ ID NO: 33751 - DNA, 28 bp, synthetic construct
  source 1..28: mol_type = other DNA
taactttaaaaacaaaggaatggttggg

SEQ ID NO: 33752 - DNA, 28 bp, synthetic construct
  source 1..28: mol_type = other DNA
aatggttgggcagatttgtctattatgg

SEQ ID NO: 33753 - DNA, 28 bp, synthetic construct
  source 1..28: mol_type = other DNA
tctattatggaatcagaccagcagcagg

SEQ ID NO: 33754 - DNA, 28 bp, synthetic construct
  source 1..28: mol_type = other DNA
ttatggaatcagaccagcagcaggaagg

SEQ ID NO: 33755 - DNA, 28 bp, synthetic construct
  source 1..28: mol_type = other DNA
tatggaatcagaccagcagcaggaaggg

SEQ ID NO: 33756 - DNA, 28 bp, synthetic construct
  source 1..28: mol_type = other DNA
agaccagcagcaggaagggctcaattgg

SEQ ID NO: 33757 - DNA, 28 bp, synthetic construct
  source 1..28: mol_type = other DNA
tttccaattgagcccttcctgctgctgg

SEQ ID NO: 33758 - DNA, 28 bp, synthetic construct
  source 1..28: mol_type = other DNA
caattggaaagtgctgagaatcccacgg

SEQ ID NO: 33759 - DNA, 28 bp, synthetic construct
  source 1..28: mol_type = other DNA
gtgctgagaatcccacggcttcgatcgg

SEQ ID NO: 33760 - DNA, 28 bp, synthetic construct
  source 1..28: mol_type = other DNA
aatcccacggcttcgatcggttgtatgg

SEQ ID NO: 33761 - DNA, 28 bp, synthetic construct
  source 1..28: mol_type = other DNA
atcccacggcttcgatcggttgtatggg

SEQ ID NO: 33762 - DNA, 28 bp, synthetic construct
  source 1..28: mol_type = other DNA
cacccatacaaccgatcgaagccgtggg

SEQ ID NO: 33763 - DNA, 28 bp, synthetic construct
  source 1..28: mol_type = other DNA
gcacccatacaaccgatcgaagccgtgg

SEQ ID NO: 33764 - DNA, 28 bp, synthetic construct
  source 1..28: mol_type = other DNA
taaaaagtcgtacatggattctaacagg

SEQ ID NO: 33765 - DNA, 28 bp, synthetic construct
  source 1..28: mol_type = other DNA
gaagctctggctaaaaagtcgtacatgg

SEQ ID NO: 33766 - DNA, 28 bp, synthetic construct
  source 1..28: mol_type = other DNA
gtctgattttttctgggagaagctctgg

SEQ ID NO: 33767 - DNA, 28 bp, synthetic construct
  source 1..28: mol_type = other DNA
atttgtgaaaagtctgattttttctggg

SEQ ID NO: 33768 - DNA, 28 bp, synthetic construct
  source 1..28: mol_type = other DNA
tatttgtgaaaagtctgattttttctgg

SEQ ID NO: 33769 - DNA, 28 bp, synthetic construct
  source 1..28: mol_type = other DNA
aatcagacttttcacaaatatattttgg

SEQ ID NO: 33770 - DNA, 28 bp, synthetic construct
  source 1..28: mol_type = other DNA
ttttggttaaaagtatactaacccaagg

SEQ ID NO: 33771 - DNA, 28 bp, synthetic construct
  source 1..28: mol_type = other DNA
ttgaaaaaaaaaaaattcttaccttggg

SEQ ID NO: 33772 - DNA, 28 bp, synthetic construct
  source 1..28: mol_type = other DNA
tttgaaaaaaaaaaaattcttaccttgg

SEQ ID NO: 33773 - DNA, 28 bp, synthetic construct
  source 1..28: mol_type = other DNA
tgtgtattttgaagagtttatactcagg

SEQ ID NO: 33774 - DNA, 28 bp, synthetic construct
  source 1..28: mol_type = other DNA
ttgaagagtttatactcaggcatagtgg

SEQ ID NO: 33775 - DNA, 28 bp, synthetic construct
  source 1..28: mol_type = other DNA
tggagatcccttctttctgttttcttgg

SEQ ID NO: 33776 - DNA, 28 bp, synthetic construct
  source 1..28: mol_type = other DNA
agatcccttctttctgttttcttggtgg

SEQ ID NO: 33777 - DNA, 28 bp, synthetic construct
  source 1..28: mol_type = other DNA
gatcccttctttctgttttcttggtggg

SEQ ID NO: 33778 - DNA, 28 bp, synthetic construct
  source 1..28: mol_type = other DNA
tttcccaccaagaaaacagaaagaaggg

SEQ ID NO: 33779 - DNA, 28 bp, synthetic construct
  source 1..28: mol_type = other DNA
ctttcccaccaagaaaacagaaagaagg

SEQ ID NO: 33780 - DNA, 28 bp, synthetic construct
  source 1..28: mol_type = other DNA
cttctttctgttttcttggtgggaaagg

SEQ ID NO: 33781 - DNA, 28 bp, synthetic construct
  source 1..28: mol_type = other DNA
cttggtgggaaaggcagaagcagagagg

SEQ ID NO: 33782 - DNA, 28 bp, synthetic construct
  source 1..28: mol_type = other DNA
tgggaaaggcagaagcagagaggtcagg

SEQ ID NO: 33783 - DNA, 28 bp, synthetic construct
  source 1..28: mol_type = other DNA
ggcagaagcagagaggtcaggagaaagg

SEQ ID NO: 33784 - DNA, 28 bp, synthetic construct
  source 1..28: mol_type = other DNA
agcagagaggtcaggagaaaggagatgg

SEQ ID NO: 33785 - DNA, 28 bp, synthetic construct
  source 1..28: mol_type = other DNA
gcagagaggtcaggagaaaggagatggg

SEQ ID NO: 33786 - DNA, 28 bp, synthetic construct
  source 1..28: mol_type = other DNA
cagagaggtcaggagaaaggagatgggg

SEQ ID NO: 33787 - DNA, 28 bp, synthetic construct
  source 1..28: mol_type = other DNA
gaggtcaggagaaaggagatggggacgg

SEQ ID NO: 33788 - DNA, 28 bp, synthetic construct
  source 1..28: mol_type = other DNA
aaggagatggggacggataacagcatgg

SEQ ID NO: 33789 - DNA, 28 bp, synthetic construct
  source 1..28: mol_type = other DNA
gagatggggacggataacagcatggtgg

SEQ ID NO: 33790 - DNA, 28 bp, synthetic construct
  source 1..28: mol_type = other DNA
agatggggacggataacagcatggtggg

SEQ ID NO: 33791 - DNA, 28 bp, synthetic construct
  source 1..28: mol_type = other DNA
ggataacagcatggtgggcagtgccagg

SEQ ID NO: 33792 - DNA, 28 bp, synthetic construct
  source 1..28: mol_type = other DNA
gcatggtgggcagtgccaggcatgctgg

SEQ ID NO: 33793 - DNA, 28 bp, synthetic construct
  source 1..28: mol_type = other DNA
catggtgggcagtgccaggcatgctggg

SEQ ID NO: 33794 - DNA, 28 bp, synthetic construct
  source 1..28: mol_type = other DNA
caaacagaaacacacccagcatgcctgg

SEQ ID NO: 33795 - DNA, 28 bp, synthetic construct
  source 1..28: mol_type = other DNA
tgggtgtgtttctgtttgaatgtccagg

SEQ ID NO: 33796 - DNA, 28 bp, synthetic construct
  source 1..28: mol_type = other DNA
tgtttgaatgtccaggctgtgacaaagg

SEQ ID NO: 33797 - DNA, 28 bp, synthetic construct
  source 1..28: mol_type = other DNA
gtttgaatgtccaggctgtgacaaaggg

SEQ ID NO: 33798 - DNA, 28 bp, synthetic construct
  source 1..28: mol_type = other DNA
gtccaggctgtgacaaagggaagtaagg

SEQ ID NO: 33799 - DNA, 28 bp, synthetic construct
  source 1..28: mol_type = other DNA
ttccttacttccctttgtcacagcctgg

SEQ ID NO: 33800 - DNA, 28 bp, synthetic construct
  source 1..28: mol_type = other DNA
acaaagggaagtaaggaatgcatgttgg

SEQ ID NO: 33801 - DNA, 28 bp, synthetic construct
  source 1..28: mol_type = other DNA
aagggaagtaaggaatgcatgttggagg

SEQ ID NO: 33802 - DNA, 28 bp, synthetic construct
  source 1..28: mol_type = other DNA
agggaagtaaggaatgcatgttggaggg

SEQ ID NO: 33803 - DNA, 28 bp, synthetic construct
  source 1..28: mol_type = other DNA
ctagacatgagggcaaatgagaaatggg

SEQ ID NO: 33804 - DNA, 28 bp, synthetic construct
  source 1..28: mol_type = other DNA
cctagacatgagggcaaatgagaaatgg

SEQ ID NO: 33805 - DNA, 28 bp, synthetic construct
  source 1..28: mol_type = other DNA
catttctcatttgccctcatgtctaggg

SEQ ID NO: 33806 - DNA, 28 bp, synthetic construct
  source 1..28: mol_type = other DNA
atttgccctcatgtctagggcccagagg

SEQ ID NO: 33807 - DNA, 28 bp, synthetic construct
  source 1..28: mol_type = other DNA
ctggtcctctgggccctagacatgaggg

SEQ ID NO: 33808 - DNA, 28 bp, synthetic construct
  source 1..28: mol_type = other DNA
actggtcctctgggccctagacatgagg

SEQ ID NO: 33809 - DNA, 28 bp, synthetic construct
  source 1..28: mol_type = other DNA
ctagggcccagaggaccagtcacttagg

SEQ ID NO: 33810 - DNA, 28 bp, synthetic construct
  source 1..28: mol_type = other DNA
agctgtcctaagtgactggtcctctggg

SEQ ID NO: 33811 - DNA, 28 bp, synthetic construct
  source 1..28: mol_type = other DNA
cagctgtcctaagtgactggtcctctgg

SEQ ID NO: 33812 - DNA, 28 bp, synthetic construct
  source 1..28: mol_type = other DNA
cttggcttcagctgtcctaagtgactgg

SEQ ID NO: 33813 - DNA, 28 bp, synthetic construct
  source 1..28: mol_type = other DNA
gaagccaagcaactgttgacatttctgg

SEQ ID NO: 33814 - DNA, 28 bp, synthetic construct
  source 1..28: mol_type = other DNA
aaggccagaaatgtcaacagttgcttgg

SEQ ID NO: 33815 - DNA, 28 bp, synthetic construct
  source 1..28: mol_type = other DNA
ttttggtgagggagaagaggagacaagg

SEQ ID NO: 33816 - DNA, 28 bp, synthetic construct
  source 1..28: mol_type = other DNA
taatatcattttggtgagggagaagagg

SEQ ID NO: 33817 - DNA, 28 bp, synthetic construct
  source 1..28: mol_type = other DNA
tctccctcaccaaaatgatattagctgg

SEQ ID NO: 33818 - DNA, 28 bp, synthetic construct
  source 1..28: mol_type = other DNA
ctccctcaccaaaatgatattagctggg

SEQ ID NO: 33819 - DNA, 28 bp, synthetic construct
  source 1..28: mol_type = other DNA
gtcccagctaatatcattttggtgaggg

SEQ ID NO: 33820 - DNA, 28 bp, synthetic construct
  source 1..28: mol_type = other DNA
agtcccagctaatatcattttggtgagg

SEQ ID NO: 33821 - DNA, 28 bp, synthetic construct
  source 1..28: mol_type = other DNA
gaggaagtcccagctaatatcattttgg

SEQ ID NO: 33822 - DNA, 28 bp, synthetic construct
  source 1..28: mol_type = other DNA
gggaatgcattgtggataggaggtgagg

SEQ ID NO: 33823 - DNA, 28 bp, synthetic construct
  source 1..28: mol_type = other DNA
gaacagggaatgcattgtggataggagg

SEQ ID NO: 33824 - DNA, 28 bp, synthetic construct
  source 1..28: mol_type = other DNA
ctggaacagggaatgcattgtggatagg

SEQ ID NO: 33825 - DNA, 28 bp, synthetic construct
  source 1..28: mol_type = other DNA
attcagcagacagcacaagcctcaaagg

SEQ ID NO: 33826 - DNA, 28 bp, synthetic construct
  source 1..28: mol_type = other DNA
tacattctggggaatatggcctttgagg

SEQ ID NO: 33827 - DNA, 28 bp, synthetic construct
  source 1..28: mol_type = other DNA
taggatgattacattctggggaatatgg

SEQ ID NO: 33828 - DNA, 28 bp, synthetic construct
  source 1..28: mol_type = other DNA
tcaaaagtaggatgattacattctgggg

SEQ ID NO: 33829 - DNA, 28 bp, synthetic construct
  source 1..28: mol_type = other DNA
ttcaaaagtaggatgattacattctggg

SEQ ID NO: 33830 - DNA, 28 bp, synthetic construct
  source 1..28: mol_type = other DNA
tttcaaaagtaggatgattacattctgg

SEQ ID NO: 33831 - DNA, 28 bp, synthetic construct
  source 1..28: mol_type = other DNA
attatatcttcggtatttcaaaagtagg

SEQ ID NO: 33832 - DNA, 28 bp, synthetic construct
  source 1..28: mol_type = other DNA
tattttcattgtactattatatcttcgg

SEQ ID NO: 33833 - DNA, 28 bp, synthetic construct
  source 1..28: mol_type = other DNA
aatgaaaatattcttaccccgatgaagg

SEQ ID NO: 33834 - DNA, 28 bp, synthetic construct
  source 1..28: mol_type = other DNA
aaaatattcttaccccgatgaaggctgg

SEQ ID NO: 33835 - DNA, 28 bp, synthetic construct
  source 1..28: mol_type = other DNA
ccccgatgaaggctggctccagttgtgg

SEQ ID NO: 33836 - DNA, 28 bp, synthetic construct
  source 1..28: mol_type = other DNA
gccacaactggagccagccttcatcggg

SEQ ID NO: 33837 - DNA, 28 bp, synthetic construct
  source 1..28: mol_type = other DNA
agccacaactggagccagccttcatcgg

SEQ ID NO: 33838 - DNA, 28 bp, synthetic construct
  source 1..28: mol_type = other DNA
agtttttgacttgctaagccacaactgg

SEQ ID NO: 33839 - DNA, 28 bp, synthetic construct
  source 1..28: mol_type = other DNA
ctttggaattttaggatgttgttacagg

SEQ ID NO: 33840 - DNA, 28 bp, synthetic construct
  source 1..28: mol_type = other DNA
ctgtaacaacatcctaaaattccaaagg

SEQ ID NO: 33841 - DNA, 28 bp, synthetic construct
  source 1..28: mol_type = other DNA
ggggaagaataacctttggaattttagg

SEQ ID NO: 33842 - DNA, 28 bp, synthetic construct
  source 1..28: mol_type = other DNA
actgtggatggggaagaataacctttgg

SEQ ID NO: 33843 - DNA, 28 bp, synthetic construct
  source 1..28: mol_type = other DNA
ggagatggctttttaactgtggatgggg

SEQ ID NO: 33844 - DNA, 28 bp, synthetic construct
  source 1..28: mol_type = other DNA
aggagatggctttttaactgtggatggg

SEQ ID NO: 33845 - DNA, 28 bp, synthetic construct
  source 1..28: mol_type = other DNA
taggagatggctttttaactgtggatgg

SEQ ID NO: 33846 - DNA, 28 bp, synthetic construct
  source 1..28: mol_type = other DNA
tctgtaggagatggctttttaactgtgg

SEQ ID NO: 33847 - DNA, 28 bp, synthetic construct
  source 1..28: mol_type = other DNA
agatatgacactgttctgtaggagatgg

SEQ ID NO: 33848 - DNA, 28 bp, synthetic construct
  source 1..28: mol_type = other DNA
tgtcacagatatgacactgttctgtagg

SEQ ID NO: 33849 - DNA, 28 bp, synthetic construct
  source 1..28: mol_type = other DNA
atatctgtgacatgtccaagattaaagg

SEQ ID NO: 33850 - DNA, 28 bp, synthetic construct
  source 1..28: mol_type = other DNA
agcaagaaggctcttcctttaatcttgg

SEQ ID NO: 33851 - DNA, 28 bp, synthetic construct
  source 1..28: mol_type = other DNA
gccttcttgcttttagtaatttgtctgg

SEQ ID NO: 33852 - DNA, 28 bp, synthetic construct
  source 1..28: mol_type = other DNA
accagacaaattactaaaagcaagaagg

SEQ ID NO: 33853 - DNA, 28 bp, synthetic construct
  source 1..28: mol_type = other DNA
ttaaaaaagccatcttcatgcttcatgg

SEQ ID NO: 33854 - DNA, 28 bp, synthetic construct
  source 1..28: mol_type = other DNA
taaaaaagccatcttcatgcttcatggg

SEQ ID NO: 33855 - DNA, 28 bp, synthetic construct
  source 1..28: mol_type = other DNA
acatttctcccatgaagcatgaagatgg

SEQ ID NO: 33856 - DNA, 28 bp, synthetic construct
  source 1..28: mol_type = other DNA
ggagaaatgtgtgatttttaaacagagg

SEQ ID NO: 33857 - DNA, 28 bp, synthetic construct
  source 1..28: mol_type = other DNA
aaattatctgatacttgatacgaagagg

SEQ ID NO: 33858 - DNA, 28 bp, synthetic construct
  source 1..28: mol_type = other DNA
gataatttttttgcatttcagcacgagg

SEQ ID NO: 33859 - DNA, 28 bp, synthetic construct
  source 1..28: mol_type = other DNA
tttcagcacgaggcaaacaaacaaaagg

SEQ ID NO: 33860 - DNA, 28 bp, synthetic construct
  source 1..28: mol_type = other DNA
ttactaagacgcgtttgaaacttcgtgg

SEQ ID NO: 33861 - DNA, 28 bp, synthetic construct
  source 1..28: mol_type = other DNA
cgtcttagtaacataaactgaagttagg

SEQ ID NO: 33862 - DNA, 28 bp, synthetic construct
  source 1..28: mol_type = other DNA
tactttggtaattcaatatcaaagaagg

SEQ ID NO: 33863 - DNA, 28 bp, synthetic construct
  source 1..28: mol_type = other DNA
ggatttttttttcagcgagatactttgg

SEQ ID NO: 33864 - DNA, 28 bp, synthetic construct
  source 1..28: mol_type = other DNA
cacaacttgtttattaattgcaaggggg

SEQ ID NO: 33865 - DNA, 28 bp, synthetic construct
  source 1..28: mol_type = other DNA
ccacaacttgtttattaattgcaagggg

SEQ ID NO: 33866 - DNA, 28 bp, synthetic construct
  source 1..28: mol_type = other DNA
accacaacttgtttattaattgcaaggg

SEQ ID NO: 33867 - DNA, 28 bp, synthetic construct
  source 1..28: mol_type = other DNA
taccacaacttgtttattaattgcaagg

SEQ ID NO: 33868 - DNA, 28 bp, synthetic construct
  source 1..28: mol_type = other DNA
tttggaatgtgaagattcttagctttgg

SEQ ID NO: 33869 - DNA, 28 bp, synthetic construct
  source 1..28: mol_type = other DNA
ttcacattccaaatctttccattcctgg

SEQ ID NO: 33870 - DNA, 28 bp, synthetic construct
  source 1..28: mol_type = other DNA
aagctcttccaggaatggaaagatttgg

SEQ ID NO: 33871 - DNA, 28 bp, synthetic construct
  source 1..28: mol_type = other DNA
aatctttccattcctggaagagctttgg

SEQ ID NO: 33872 - DNA, 28 bp, synthetic construct
  source 1..28: mol_type = other DNA
ctaaataccaaagctcttccaggaatgg

SEQ ID NO: 33873 - DNA, 28 bp, synthetic construct
  source 1..28: mol_type = other DNA
aacatctaaataccaaagctcttccagg

SEQ ID NO: 33874 - DNA, 28 bp, synthetic construct
  source 1..28: mol_type = other DNA
agagctttggtatttagatgttaatagg

SEQ ID NO: 33875 - DNA, 28 bp, synthetic construct
  source 1..28: mol_type = other DNA
aaaaaaagaaaaaaaaaaaaaaggcagg

SEQ ID NO: 33876 - DNA, 28 bp, synthetic construct
  source 1..28: mol_type = other DNA
tgccttttttttttttttctttttttgg

SEQ ID NO: 33877 - DNA, 28 bp, synthetic construct
  source 1..28: mol_type = other DNA
ggccaaaaaaagaaaaaaaaaaaaaagg

SEQ ID NO: 33878 - DNA, 28 bp, synthetic construct
  source 1..28: mol_type = other DNA
ttttttctttttttggccaatcttcagg

SEQ ID NO: 33879 - DNA, 28 bp, synthetic construct
  source 1..28: mol_type = other DNA
ttcacagactctttagcctgaagattgg

SEQ ID NO: 33880 - DNA, 28 bp, synthetic construct
  source 1..28: mol_type = other DNA
ttttccatcctatgacctcagttttagg

SEQ ID NO: 33881 - DNA, 28 bp, synthetic construct
  source 1..28: mol_type = other DNA
aaatcctaaaactgaggtcataggatgg

SEQ ID NO: 33882 - DNA, 28 bp, synthetic construct
  source 1..28: mol_type = other DNA
aaagaaatcctaaaactgaggtcatagg

SEQ ID NO: 33883 - DNA, 28 bp, synthetic construct
  source 1..28: mol_type = other DNA
ttgcaagaaagaaatcctaaaactgagg

SEQ ID NO: 33884 - DNA, 28 bp, synthetic construct
  source 1..28: mol_type = other DNA
tctttcttgcaaaatttagttattttgg

SEQ ID NO: 33885 - DNA, 28 bp, synthetic construct
  source 1..28: mol_type = other DNA
tcttgcaaaatttagttattttggttgg

SEQ ID NO: 33886 - DNA, 28 bp, synthetic construct
  source 1..28: mol_type = other DNA
ggagaaagaaaataagaatgaattctgg

SEQ ID NO: 33887 - DNA, 28 bp, synthetic construct
  source 1..28: mol_type = other DNA
ttcattcttattttctttctccttctgg

SEQ ID NO: 33888 - DNA, 28 bp, synthetic construct
  source 1..28: mol_type = other DNA
gggggtaaagggagaaagtaccagaagg

SEQ ID NO: 33889 - DNA, 28 bp, synthetic construct
  source 1..28: mol_type = other DNA
agggagagaaacagaagggggtaaaggg

SEQ ID NO: 33890 - DNA, 28 bp, synthetic construct
  source 1..28: mol_type = other DNA
aagggagagaaacagaagggggtaaagg

SEQ ID NO: 33891 - DNA, 28 bp, synthetic construct
  source 1..28: mol_type = other DNA
gtgaagaagggagagaaacagaaggggg

SEQ ID NO: 33892 - DNA, 28 bp, synthetic construct
  source 1..28: mol_type = other DNA
ggtgaagaagggagagaaacagaagggg

SEQ ID NO: 33893 - DNA, 28 bp, synthetic construct
  source 1..28: mol_type = other DNA
aggtgaagaagggagagaaacagaaggg

SEQ ID NO: 33894 - DNA, 28 bp, synthetic construct
  source 1..28: mol_type = other DNA
taggtgaagaagggagagaaacagaagg

SEQ ID NO: 33895 - DNA, 28 bp, synthetic construct
  source 1..28: mol_type = other DNA
agaataatacaagataggtgaagaaggg

SEQ ID NO: 33896 - DNA, 28 bp, synthetic construct
  source 1..28: mol_type = other DNA
gagaataatacaagataggtgaagaagg

SEQ ID NO: 33897 - DNA, 28 bp, synthetic construct
  source 1..28: mol_type = other DNA
ttcaattcagagaataatacaagatagg

SEQ ID NO: 33898 - DNA, 28 bp, synthetic construct
  source 1..28: mol_type = other DNA
tgaattgaattaagaatttaaagtccgg

SEQ ID NO: 33899 - DNA, 28 bp, synthetic construct
  source 1..28: mol_type = other DNA
ttgaattaagaatttaaagtccggttgg

SEQ ID NO: 33900 - DNA, 28 bp, synthetic construct
  source 1..28: mol_type = other DNA
aattaagaatttaaagtccggttggtgg

SEQ ID NO: 33901 - DNA, 28 bp, synthetic construct
  source 1..28: mol_type = other DNA
agaatttaaagtccggttggtggactgg

SEQ ID NO: 33902 - DNA, 28 bp, synthetic construct
  source 1..28: mol_type = other DNA
agagactgtagtccagtccaccaaccgg

SEQ ID NO: 33903 - DNA, 28 bp, synthetic construct
  source 1..28: mol_type = other DNA
actggactacagtctctatgatgtttgg

SEQ ID NO: 33904 - DNA, 28 bp, synthetic construct
  source 1..28: mol_type = other DNA
gactacagtctctatgatgtttggtagg

SEQ ID NO: 33905 - DNA, 28 bp, synthetic construct
  source 1..28: mol_type = other DNA
actacagtctctatgatgtttggtaggg

SEQ ID NO: 33906 - DNA, 28 bp, synthetic construct
  source 1..28: mol_type = other DNA
tgttagaattagcaaatgaaaatacagg

SEQ ID NO: 33907 - DNA, 28 bp, synthetic construct
  source 1..28: mol_type = other DNA
ggatgcctagttaaatttgaatttcagg

SEQ ID NO: 33908 - DNA, 28 bp, synthetic construct
  source 1..28: mol_type = other DNA
gtttacctgaaattcaaatttaactagg

SEQ ID NO: 33909 - DNA, 28 bp, synthetic construct
  source 1..28: mol_type = other DNA
tgtaaatgtgtctcatgcaatatttggg

SEQ ID NO: 33910 - DNA, 28 bp, synthetic construct
  source 1..28: mol_type = other DNA
gtgtaaatgtgtctcatgcaatatttgg

SEQ ID NO: 33911 - DNA, 28 bp, synthetic construct
  source 1..28: mol_type = other DNA
ctacaaattattttcaagtattgcatgg

SEQ ID NO: 33912 - DNA, 28 bp, synthetic construct
  source 1..28: mol_type = other DNA
tacaaattattttcaagtattgcatggg

SEQ ID NO: 33913 - DNA, 28 bp, synthetic construct
  source 1..28: mol_type = other DNA
tgtttatctgaaattcaaatttaactgg

SEQ ID NO: 33914 - DNA, 28 bp, synthetic construct
  source 1..28: mol_type = other DNA
gtttatctgaaattcaaatttaactggg

SEQ ID NO: 33915 - DNA, 28 bp, synthetic construct
  source 1..28: mol_type = other DNA
ttaactgggcgtcttatattttatctgg

SEQ ID NO: 33916 - DNA, 28 bp, synthetic construct
  source 1..28: mol_type = other DNA
tatattttatctggcaacactactttgg

SEQ ID NO: 33917 - DNA, 28 bp, synthetic construct
  source 1..28: mol_type = other DNA
attttatctggcaacactactttggagg

SEQ ID NO: 33918 - DNA, 28 bp, synthetic construct
  source 1..28: mol_type = other DNA
tggcaacactactttggaggttcaatgg

SEQ ID NO: 33919 - DNA, 28 bp, synthetic construct
  source 1..28: mol_type = other DNA
aacactactttggaggttcaatggaagg

SEQ ID NO: 33920 - DNA, 28 bp, synthetic construct
  source 1..28: mol_type = other DNA
acactactttggaggttcaatggaaggg

SEQ ID NO: 33921 - DNA, 28 bp, synthetic construct
  source 1..28: mol_type = other DNA
atggaagggattttaaaaaaaacaaagg

SEQ ID NO: 33922 - DNA, 28 bp, synthetic construct
  source 1..28: mol_type = other DNA
aacaaaggcatccatttacaactcctgg

SEQ ID NO: 33923 - DNA, 28 bp, synthetic construct
  source 1..28: mol_type = other DNA
tttctcttcttccaggagttgtaaatgg

SEQ ID NO: 33924 - DNA, 28 bp, synthetic construct
  source 1..28: mol_type = other DNA
taggagtggaaatttctcttcttccagg

SEQ ID NO: 33925 - DNA, 28 bp, synthetic construct
  source 1..28: mol_type = other DNA
caaaaagcgttcaagaggataggagtgg

SEQ ID NO: 33926 - DNA, 28 bp, synthetic construct
  source 1..28: mol_type = other DNA
ctagacaaaaagcgttcaagaggatagg

SEQ ID NO: 33927 - DNA, 28 bp, synthetic construct
  source 1..28: mol_type = other DNA
tacatctagacaaaaagcgttcaagagg

SEQ ID NO: 33928 - DNA, 28 bp, synthetic construct
  source 1..28: mol_type = other DNA
actgggtcaaaaataaactaaaatgagg

SEQ ID NO: 33929 - DNA, 28 bp, synthetic construct
  source 1..28: mol_type = other DNA
tgtggagcttttagtacaacttactggg

SEQ ID NO: 33930 - DNA, 28 bp, synthetic construct
  source 1..28: mol_type = other DNA
ctgtggagcttttagtacaacttactgg

SEQ ID NO: 33931 - DNA, 28 bp, synthetic construct
  source 1..28: mol_type = other DNA
taatataaggatgtgacatgctctgtgg

SEQ ID NO: 33932 - DNA, 28 bp, synthetic construct
  source 1..28: mol_type = other DNA
tccttatattaaagaagtccatcccagg

SEQ ID NO: 33933 - DNA, 28 bp, synthetic construct
  source 1..28: mol_type = other DNA
acctgggatggacttctttaatataagg

SEQ ID NO: 33934 - DNA, 28 bp, synthetic construct
  source 1..28: mol_type = other DNA
attaaagaagtccatcccaggtttcagg

SEQ ID NO: 33935 - DNA, 28 bp, synthetic construct
  source 1..28: mol_type = other DNA
tccatcccaggtttcaggtctcactcgg

SEQ ID NO: 33936 - DNA, 28 bp, synthetic construct
  source 1..28: mol_type = other DNA
accgagtgagacctgaaacctgggatgg

SEQ ID NO: 33937 - DNA, 28 bp, synthetic construct
  source 1..28: mol_type = other DNA
tgacaccgagtgagacctgaaacctggg

SEQ ID NO: 33938 - DNA, 28 bp, synthetic construct
  source 1..28: mol_type = other DNA
ctgacaccgagtgagacctgaaacctgg

SEQ ID NO: 33939 - DNA, 28 bp, synthetic construct
  source 1..28: mol_type = other DNA
caggtttcaggtctcactcggtgtcagg

SEQ ID NO: 33940 - DNA, 28 bp, synthetic construct
  source 1..28: mol_type = other DNA
ttcaggtctcactcggtgtcaggccagg

SEQ ID NO: 33941 - DNA, 28 bp, synthetic construct
  source 1..28: mol_type = other DNA
caggccaggccagagcttgcaaaattgg

SEQ ID NO: 33942 - DNA, 28 bp, synthetic construct
  source 1..28: mol_type = other DNA
gggaccaattttgcaagctctggcctgg

SEQ ID NO: 33943 - DNA, 28 bp, synthetic construct
  source 1..28: mol_type = other DNA
cctgggggaccaattttgcaagctctgg

SEQ ID NO: 33944 - DNA, 28 bp, synthetic construct
  source 1..28: mol_type = other DNA
tgcaaaattggtcccccaggcaacatgg

SEQ ID NO: 33945 - DNA, 28 bp, synthetic construct
  source 1..28: mol_type = other DNA
gcaaaattggtcccccaggcaacatggg

SEQ ID NO: 33946 - DNA, 28 bp, synthetic construct
  source 1..28: mol_type = other DNA
tggtcccccaggcaacatgggaccttgg

SEQ ID NO: 33947 - DNA, 28 bp, synthetic construct
  source 1..28: mol_type = other DNA
tgcgccaaggtcccatgttgcctggggg

SEQ ID NO: 33948 - DNA, 28 bp, synthetic construct
  source 1..28: mol_type = other DNA
ctgcgccaaggtcccatgttgcctgggg

SEQ ID NO: 33949 - DNA, 28 bp, synthetic construct
  source 1..28: mol_type = other DNA
actgcgccaaggtcccatgttgcctggg

SEQ ID NO: 33950 - DNA, 28 bp, synthetic construct
  source 1..28: mol_type = other DNA
tactgcgccaaggtcccatgttgcctgg

SEQ ID NO: 33951 - DNA, 28 bp, synthetic construct
  source 1..28: mol_type = other DNA
tttgcattgttctgttactgcgccaagg

SEQ ID NO: 33952 - DNA, 28 bp, synthetic construct
  source 1..28: mol_type = other DNA
agattttgaaggaaaaaattaaaactgg

SEQ ID NO: 33953 - DNA, 28 bp, synthetic construct
  source 1..28: mol_type = other DNA
actaaatttggtgttcagattttgaagg

SEQ ID NO: 33954 - DNA, 28 bp, synthetic construct
  source 1..28: mol_type = other DNA
tgaacaccaaatttagtacttttgaagg

SEQ ID NO: 33955 - DNA, 28 bp, synthetic construct
  source 1..28: mol_type = other DNA
tcagtgccttcaaaagtactaaatttgg

SEQ ID NO: 33956 - DNA, 28 bp, synthetic construct
  source 1..28: mol_type = other DNA
agttttctctcctcagtgctcactttgg

SEQ ID NO: 33957 - DNA, 28 bp, synthetic construct
  source 1..28: mol_type = other DNA
gttttctctcctcagtgctcactttggg

SEQ ID NO: 33958 - DNA, 28 bp, synthetic construct
  source 1..28: mol_type = other DNA
ttttctctcctcagtgctcactttgggg

SEQ ID NO: 33959 - DNA, 28 bp, synthetic construct
  source 1..28: mol_type = other DNA
ctaaattgccccaaagtgagcactgagg

SEQ ID NO: 33960 - DNA, 28 bp, synthetic construct
  source 1..28: mol_type = other DNA
tttcaacattcatgtgaattctattggg

SEQ ID NO: 33961 - DNA, 28 bp, synthetic construct
  source 1..28: mol_type = other DNA
atttcaacattcatgtgaattctattgg

SEQ ID NO: 33962 - DNA, 28 bp, synthetic construct
  source 1..28: mol_type = other DNA
gaaatgtaataaaatgatcactttttgg

SEQ ID NO: 33963 - DNA, 28 bp, synthetic construct
  source 1..28: mol_type = other DNA
aaatgtaataaaatgatcactttttggg

SEQ ID NO: 33964 - DNA, 28 bp, synthetic construct
  source 1..28: mol_type = other DNA
atgatcactttttgggcattttgaaagg

SEQ ID NO: 33965 - DNA, 28 bp, synthetic construct
  source 1..28: mol_type = other DNA
tgatcactttttgggcattttgaaaggg

SEQ ID NO: 33966 - DNA, 28 bp, synthetic construct
  source 1..28: mol_type = other DNA
tcttaattacattaattattaattcagg

SEQ ID NO: 33967 - DNA, 28 bp, synthetic construct
  source 1..28: mol_type = other DNA
tatttctgaacatctaaagaaacccagg

SEQ ID NO: 33968 - DNA, 28 bp, synthetic construct
  source 1..28: mol_type = other DNA
ttctgaacatctaaagaaacccaggagg

SEQ ID NO: 33969 - DNA, 28 bp, synthetic construct
  source 1..28: mol_type = other DNA
tctgaacatctaaagaaacccaggaggg

SEQ ID NO: 33970 - DNA, 28 bp, synthetic construct
  source 1..28: mol_type = other DNA
ttttggaattatgtgtcgccctcctggg

SEQ ID NO: 33971 - DNA, 28 bp, synthetic construct
  source 1..28: mol_type = other DNA
attttggaattatgtgtcgccctcctgg

SEQ ID NO: 33972 - DNA, 28 bp, synthetic construct
  source 1..28: mol_type = other DNA
gtctctaaataagagaacggcattttgg

SEQ ID NO: 33973 - DNA, 28 bp, synthetic construct
  source 1..28: mol_type = other DNA
atcaatgtgtctctaaataagagaacgg

SEQ ID NO: 33974 - DNA, 28 bp, synthetic construct
  source 1..28: mol_type = other DNA
agagacacattgatattcagtattttgg

SEQ ID NO: 33975 - DNA, 28 bp, synthetic construct
  source 1..28: mol_type = other DNA
ctattttgaagtttaatagctgaaatgg

SEQ ID NO: 33976 - DNA, 28 bp, synthetic construct
  source 1..28: mol_type = other DNA
ttttgaagtttaatagctgaaatggagg

SEQ ID NO: 33977 - DNA, 28 bp, synthetic construct
  source 1..28: mol_type = other DNA
gaggctgtactttaaattcttaaactgg

SEQ ID NO: 33978 - DNA, 28 bp, synthetic construct
  source 1..28: mol_type = other DNA
ttcaattcaaagaataatacaagatagg

SEQ ID NO: 33979 - DNA, 28 bp, synthetic construct
  source 1..28: mol_type = other DNA
aagaataatacaagataggtgaagaagg

SEQ ID NO: 33980 - DNA, 28 bp, synthetic construct
  source 1..28: mol_type = other DNA
taggtgaagaaggaagagaaacagaagg

SEQ ID NO: 33981 - DNA, 28 bp, synthetic construct
  source 1..28: mol_type = other DNA
aggtgaagaaggaagagaaacagaaggg

SEQ ID NO: 33982 - DNA, 28 bp, synthetic construct
  source 1..28: mol_type = other DNA
ggtgaagaaggaagagaaacagaagggg

SEQ ID NO: 33983 - DNA, 28 bp, synthetic construct
  source 1..28: mol_type = other DNA
gtgaagaaggaagagaaacagaaggggg

SEQ ID NO: 33984 - DNA, 28 bp, synthetic construct
  source 1..28: mol_type = other DNA
aaggaagagaaacagaagggggtaaagg

SEQ ID NO: 33985 - DNA, 28 bp, synthetic construct
  source 1..28: mol_type = other DNA
aggaagagaaacagaagggggtaaaggg

SEQ ID NO: 33986 - DNA, 28 bp, synthetic construct
  source 1..28: mol_type = other DNA
gggggtaaagggagaaagtaccagaagg

SEQ ID NO: 33987 - DNA, 28 bp, synthetic construct
  source 1..28: mol_type = other DNA
tgtgtgattattttgtttctccttctgg

SEQ ID NO: 33988 - DNA, 28 bp, synthetic construct
  source 1..28: mol_type = other DNA
aataatgatgatggaaggaagcccatgg

SEQ ID NO: 33989 - DNA, 28 bp, synthetic construct
  source 1..28: mol_type = other DNA
ttgtaatagtaataatgatgatggaagg

SEQ ID NO: 33990 - DNA, 28 bp, synthetic construct
  source 1..28: mol_type = other DNA
tatcttgtaatagtaataatgatgatgg

SEQ ID NO: 33991 - DNA, 28 bp, synthetic construct
  source 1..28: mol_type = other DNA
gatacttgcactatctcattttatgagg

SEQ ID NO: 33992 - DNA, 28 bp, synthetic construct
  source 1..28: mol_type = other DNA
cattttatgaggcatatttaagaacagg

SEQ ID NO: 33993 - DNA, 28 bp, synthetic construct
  source 1..28: mol_type = other DNA
acgatgtattcgatgtgccattgtctgg

SEQ ID NO: 33994 - DNA, 28 bp, synthetic construct
  source 1..28: mol_type = other DNA
tcgatgtgccattgtctggactctctgg

SEQ ID NO: 33995 - DNA, 28 bp, synthetic construct
  source 1..28: mol_type = other DNA
atgcagagccagagagtccagacaatgg

SEQ ID NO: 33996 - DNA, 28 bp, synthetic construct
  source 1..28: mol_type = other DNA
gctctgcatcacctttctcttaaaaagg

SEQ ID NO: 33997 - DNA, 28 bp, synthetic construct
  source 1..28: mol_type = other DNA
tttttctgcttcctttttaagagaaagg

SEQ ID NO: 33998 - DNA, 28 bp, synthetic construct
  source 1..28: mol_type = other DNA
cttaaagactgtaagactcatatgtcgg

SEQ ID NO: 33999 - DNA, 28 bp, synthetic construct
  source 1..28: mol_type = other DNA
ttttgaaagattgttaataggagcatgg

SEQ ID NO: 34000 - DNA, 28 bp, synthetic construct
  source 1..28: mol_type = other DNA
ctacacattttgaaagattgttaatagg

SEQ ID NO: 34001 - DNA, 28 bp, synthetic construct
  source 1..28: mol_type = other DNA
ttaacaatctttcaaaatgtgtagcagg

SEQ ID NO: 34002 - DNA, 28 bp, synthetic construct
  source 1..28: mol_type = other DNA
acaatctttcaaaatgtgtagcaggagg

SEQ ID NO: 34003 - DNA, 28 bp, synthetic construct
  source 1..28: mol_type = other DNA
ttcaaagaaattcactaaaaaactgggg

SEQ ID NO: 34004 - DNA, 28 bp, synthetic construct
  source 1..28: mol_type = other DNA
tttcaaagaaattcactaaaaaactggg

SEQ ID NO: 34005 - DNA, 28 bp, synthetic construct
  source 1..28: mol_type = other DNA
gtttcaaagaaattcactaaaaaactgg

SEQ ID NO: 34006 - DNA, 28 bp, synthetic construct
  source 1..28: mol_type = other DNA
ggaggatgagcacacattggacagtagg

SEQ ID NO: 34007 - DNA, 28 bp, synthetic construct
  source 1..28: mol_type = other DNA
aaggggagggaggatgagcacacattgg

SEQ ID NO: 34008 - DNA, 28 bp, synthetic construct
  source 1..28: mol_type = other DNA
gggggcagagggcagaaggggagggagg

SEQ ID NO: 34009 - DNA, 28 bp, synthetic construct
  source 1..28: mol_type = other DNA
ggtgggggcagagggcagaaggggaggg

SEQ ID NO: 34010 - DNA, 28 bp, synthetic construct
  source 1..28: mol_type = other DNA
gggtgggggcagagggcagaaggggagg

SEQ ID NO: 34011 - DNA, 28 bp, synthetic construct
  source 1..28: mol_type = other DNA
agggggtgggggcagagggcagaagggg

SEQ ID NO: 34012 - DNA, 28 bp, synthetic construct
  source 1..28: mol_type = other DNA
cagggggtgggggcagagggcagaaggg

SEQ ID NO: 34013 - DNA, 28 bp, synthetic construct
  source 1..28: mol_type = other DNA
gcagggggtgggggcagagggcagaagg

SEQ ID NO: 34014 - DNA, 28 bp, synthetic construct
  source 1..28: mol_type = other DNA
ctggggagcagggggtgggggcagaggg

SEQ ID NO: 34015 - DNA, 28 bp, synthetic construct
  source 1..28: mol_type = other DNA
tctggggagcagggggtgggggcagagg

SEQ ID NO: 34016 - DNA, 28 bp, synthetic construct
  source 1..28: mol_type = other DNA
gtttcatctggggagcagggggtggggg

SEQ ID NO: 34017 - DNA, 28 bp, synthetic construct
  source 1..28: mol_type = other DNA
agtttcatctggggagcagggggtgggg

SEQ ID NO: 34018 - DNA, 28 bp, synthetic construct
  source 1..28: mol_type = other DNA
gagtttcatctggggagcagggggtggg

SEQ ID NO: 34019 - DNA, 28 bp, synthetic construct
  source 1..28: mol_type = other DNA
ggagtttcatctggggagcagggggtgg

SEQ ID NO: 34020 - DNA, 28 bp, synthetic construct
  source 1..28: mol_type = other DNA
tctggagtttcatctggggagcaggggg

SEQ ID NO: 34021 - DNA, 28 bp, synthetic construct
  source 1..28: mol_type = other DNA
ctctggagtttcatctggggagcagggg

SEQ ID NO: 34022 - DNA, 28 bp, synthetic construct
  source 1..28: mol_type = other DNA
gctctggagtttcatctggggagcaggg

SEQ ID NO: 34023 - DNA, 28 bp, synthetic construct
  source 1..28: mol_type = other DNA
cgctctggagtttcatctggggagcagg

SEQ ID NO: 34024 - DNA, 28 bp, synthetic construct
  source 1..28: mol_type = other DNA
agacttcgctctggagtttcatctgggg

SEQ ID NO: 34025 - DNA, 28 bp, synthetic construct
  source 1..28: mol_type = other DNA
aagacttcgctctggagtttcatctggg

SEQ ID NO: 34026 - DNA, 28 bp, synthetic construct
  source 1..28: mol_type = other DNA
aaagacttcgctctggagtttcatctgg

SEQ ID NO: 34027 - DNA, 28 bp, synthetic construct
  source 1..28: mol_type = other DNA
actccagagcgaagtctttcttacttgg

SEQ ID NO: 34028 - DNA, 28 bp, synthetic construct
  source 1..28: mol_type = other DNA
aatccaagtaagaaagacttcgctctgg

SEQ ID NO: 34029 - DNA, 28 bp, synthetic construct
  source 1..28: mol_type = other DNA
ttcttacttggattattgtgtccagagg

SEQ ID NO: 34030 - DNA, 28 bp, synthetic construct
  source 1..28: mol_type = other DNA
ttcaggactctcagcttgtatcctctgg

SEQ ID NO: 34031 - DNA, 28 bp, synthetic construct
  source 1..28: mol_type = other DNA
attaattgatatttcttgttctttcagg

SEQ ID NO: 34032 - DNA, 28 bp, synthetic construct
  source 1..28: mol_type = other DNA
tttaaacatgatctcatgtttaacttgg

SEQ ID NO: 34033 - DNA, 28 bp, synthetic construct
  source 1..28: mol_type = other DNA
ttaaacatgagatcatgtttaaaactgg

SEQ ID NO: 34034 - DNA, 28 bp, synthetic construct
  source 1..28: mol_type = other DNA
ctgatagagattgagagcaatgaatcgg

SEQ ID NO: 34035 - DNA, 28 bp, synthetic construct
  source 1..28: mol_type = other DNA
tttcttctgtaaatattcctgccagagg

SEQ ID NO: 34036 - DNA, 28 bp, synthetic construct
  source 1..28: mol_type = other DNA
atatttacagaagaaaagacaatcacgg

SEQ ID NO: 34037 - DNA, 28 bp, synthetic construct
  source 1..28: mol_type = other DNA
tatttacagaagaaaagacaatcacggg

SEQ ID NO: 34038 - DNA, 28 bp, synthetic construct
  source 1..28: mol_type = other DNA
catgcaggcatttctagtgggcagtggg

SEQ ID NO: 34039 - DNA, 28 bp, synthetic construct
  source 1..28: mol_type = other DNA
tcatgcaggcatttctagtgggcagtgg

SEQ ID NO: 34040 - DNA, 28 bp, synthetic construct
  source 1..28: mol_type = other DNA
tttcactcatgcaggcatttctagtggg

SEQ ID NO: 34041 - DNA, 28 bp, synthetic construct
  source 1..28: mol_type = other DNA
gtttcactcatgcaggcatttctagtgg

SEQ ID NO: 34042 - DNA, 28 bp, synthetic construct
  source 1..28: mol_type = other DNA
caggaggaatatgtttcactcatgcagg

SEQ ID NO: 34043 - DNA, 28 bp, synthetic construct
  source 1..28: mol_type = other DNA
gcatgagtgaaacatattcctcctgagg

SEQ ID NO: 34044 - DNA, 28 bp, synthetic construct
  source 1..28: mol_type = other DNA
catgagtgaaacatattcctcctgaggg

SEQ ID NO: 34045 - DNA, 28 bp, synthetic construct
  source 1..28: mol_type = other DNA
aaggtgagatcttgcatccctcaggagg

SEQ ID NO: 34046 - DNA, 28 bp, synthetic construct
  source 1..28: mol_type = other DNA
aataaggtgagatcttgcatccctcagg

SEQ ID NO: 34047 - DNA, 28 bp, synthetic construct
  source 1..28: mol_type = other DNA
gagggatgcaagatctcaccttatttgg

SEQ ID NO: 34048 - DNA, 28 bp, synthetic construct
  source 1..28: mol_type = other DNA
tgcaagatctcaccttatttggaaatgg

SEQ ID NO: 34049 - DNA, 28 bp, synthetic construct
  source 1..28: mol_type = other DNA
ctcaccttatttggaaatggaaatttgg

SEQ ID NO: 34050 - DNA, 28 bp, synthetic construct
  source 1..28: mol_type = other DNA
ccaaccaaatttccatttccaaataagg

SEQ ID NO: 34051 - DNA, 28 bp, synthetic construct
  source 1..28: mol_type = other DNA
gaaatttggttggttccactttgccagg

SEQ ID NO: 34052 - DNA, 28 bp, synthetic construct
  source 1..28: mol_type = other DNA
tctgctattcaagcacctggcaaagtgg

SEQ ID NO: 34053 - DNA, 28 bp, synthetic construct
  source 1..28: mol_type = other DNA
tgccaggtgcttgaatagcagaaagtgg

SEQ ID NO: 34054 - DNA, 28 bp, synthetic construct
  source 1..28: mol_type = other DNA
caccactttctgctattcaagcacctgg

SEQ ID NO: 34055 - DNA, 28 bp, synthetic construct
  source 1..28: mol_type = other DNA
caggtgcttgaatagcagaaagtggtgg

SEQ ID NO: 34056 - DNA, 28 bp, synthetic construct
  source 1..28: mol_type = other DNA
tgaatagcagaaagtggtggaagccagg

SEQ ID NO: 34057 - DNA, 28 bp, synthetic construct
  source 1..28: mol_type = other DNA
tggtggaagccaggtcatctcctgaagg

SEQ ID NO: 34058 - DNA, 28 bp, synthetic construct
  source 1..28: mol_type = other DNA
ggaagccaggtcatctcctgaaggacgg

SEQ ID NO: 34059 - DNA, 28 bp, synthetic construct
  source 1..28: mol_type = other DNA
gaagccaggtcatctcctgaaggacggg

SEQ ID NO: 34060 - DNA, 28 bp, synthetic construct
  source 1..28: mol_type = other DNA
ttatcccgtccttcaggagatgacctgg

SEQ ID NO: 34061 - DNA, 28 bp, synthetic construct
  source 1..28: mol_type = other DNA
attgtttgtttttatcccgtccttcagg

SEQ ID NO: 34062 - DNA, 28 bp, synthetic construct
  source 1..28: mol_type = other DNA
tgatacagacagtatttaaaatcagcgg

SEQ ID NO: 34063 - DNA, 28 bp, synthetic construct
  source 1..28: mol_type = other DNA
gcggtatgtaaagcagctgtacaagtgg

SEQ ID NO: 34064 - DNA, 28 bp, synthetic construct
  source 1..28: mol_type = other DNA
cggtatgtaaagcagctgtacaagtggg

SEQ ID NO: 34065 - DNA, 28 bp, synthetic construct
  source 1..28: mol_type = other DNA
gcagctgtacaagtgggccttcataagg

SEQ ID NO: 34066 - DNA, 28 bp, synthetic construct
  source 1..28: mol_type = other DNA
ctgtacaagtgggccttcataaggcagg

SEQ ID NO: 34067 - DNA, 28 bp, synthetic construct
  source 1..28: mol_type = other DNA
tgtacaagtgggccttcataaggcaggg

SEQ ID NO: 34068 - DNA, 28 bp, synthetic construct
  source 1..28: mol_type = other DNA
caagtgggccttcataaggcagggaagg

SEQ ID NO: 34069 - DNA, 28 bp, synthetic construct
  source 1..28: mol_type = other DNA
aagtgggccttcataaggcagggaaggg

SEQ ID NO: 34070 - DNA, 28 bp, synthetic construct
  source 1..28: mol_type = other DNA
tttttaacccttccctgccttatgaagg

SEQ ID NO: 34071 - DNA, 28 bp, synthetic construct
  source 1..28: mol_type = other DNA
cagggaagggttaaaaaatgtacaaagg

SEQ ID NO: 34072 - DNA, 28 bp, synthetic construct
  source 1..28: mol_type = other DNA
aaggtaaatgtcaaaccacagactatgg

SEQ ID NO: 34073 - DNA, 28 bp, synthetic construct
  source 1..28: mol_type = other DNA
aggtaaatgtcaaaccacagactatggg

SEQ ID NO: 34074 - DNA, 28 bp, synthetic construct
  source 1..28: mol_type = other DNA
ccacagactatgggctcctttatcatgg

SEQ ID NO: 34075 - DNA, 28 bp, synthetic construct
  source 1..28: mol_type = other DNA
atgggctcctttatcatggagccgcagg

SEQ ID NO: 34076 - DNA, 28 bp, synthetic construct
  source 1..28: mol_type = other DNA
aaggaaacctgcggctccatgataaagg

SEQ ID NO: 34077 - DNA, 28 bp, synthetic construct
  source 1..28: mol_type = other DNA
agactctaaatagaaaggaaacctgcgg

SEQ ID NO: 34078 - DNA, 28 bp, synthetic construct
  source 1..28: mol_type = other DNA
tgtgggacatagactctaaatagaaagg

SEQ ID NO: 34079 - DNA, 28 bp, synthetic construct
  source 1..28: mol_type = other DNA
tctttaaacagtcttatcaatctgtggg

SEQ ID NO: 34080 - DNA, 28 bp, synthetic construct
  source 1..28: mol_type = other DNA
ttctttaaacagtcttatcaatctgtgg

SEQ ID NO: 34081 - DNA, 28 bp, synthetic construct
  source 1..28: mol_type = other DNA
agactgtttaaagaataatcttacccgg

SEQ ID NO: 34082 - DNA, 28 bp, synthetic construct
  source 1..28: mol_type = other DNA
aacagctgtgttgaagaaataatccggg

SEQ ID NO: 34083 - DNA, 28 bp, synthetic construct
  source 1..28: mol_type = other DNA
caacagctgtgttgaagaaataatccgg

SEQ ID NO: 34084 - DNA, 28 bp, synthetic construct
  source 1..28: mol_type = other DNA
cggattatttcttcaacacagctgttgg

SEQ ID NO: 34085 - DNA, 28 bp, synthetic construct
  source 1..28: mol_type = other DNA
ttctttgctttcaggagagtagatctgg

SEQ ID NO: 34086 - DNA, 28 bp, synthetic construct
  source 1..28: mol_type = other DNA
gcttaatttttttttctttgctttcagg

SEQ ID NO: 34087 - DNA, 28 bp, synthetic construct
  source 1..28: mol_type = other DNA
gcaaagaaaaaaaaattaagcctgatgg

SEQ ID NO: 34088 - DNA, 28 bp, synthetic construct
  source 1..28: mol_type = other DNA
tgtgtggtcatcaatctattccatcagg

SEQ ID NO: 34089 - DNA, 28 bp, synthetic construct
  source 1..28: mol_type = other DNA
ttgatgaccacacagaagacatgcaagg

SEQ ID NO: 34090 - DNA, 28 bp, synthetic construct
  source 1..28: mol_type = other DNA
tttggaaccttgcatgtcttctgtgtgg

SEQ ID NO: 34091 - DNA, 28 bp, synthetic construct
  source 1..28: mol_type = other DNA
atttttttgttgggggggactaatttgg

SEQ ID NO: 34092 - DNA, 28 bp, synthetic construct
  source 1..28: mol_type = other DNA
aactcgctgaatttttttgttggggggg

SEQ ID NO: 34093 - DNA, 28 bp, synthetic construct
  source 1..28: mol_type = other DNA
taactcgctgaatttttttgttgggggg

SEQ ID NO: 34094 - DNA, 28 bp, synthetic construct
  source 1..28: mol_type = other DNA
gtaactcgctgaatttttttgttggggg

SEQ ID NO: 34095 - DNA, 28 bp, synthetic construct
  source 1..28: mol_type = other DNA
tgtaactcgctgaatttttttgttgggg

SEQ ID NO: 34096 - DNA, 28 bp, synthetic construct
  source 1..28: mol_type = other DNA
ctgtaactcgctgaatttttttgttggg

SEQ ID NO: 34097 - DNA, 28 bp, synthetic construct
  source 1..28: mol_type = other DNA
cctgtaactcgctgaatttttttgttgg

SEQ ID NO: 34098 - DNA, 28 bp, synthetic construct
  source 1..28: mol_type = other DNA
aaaaaattcagcgagttacaggttgagg

SEQ ID NO: 34099 - DNA, 28 bp, synthetic construct
  source 1..28: mol_type = other DNA
aaaaattcagcgagttacaggttgaggg

SEQ ID NO: 34100 - DNA, 28 bp, synthetic construct
  source 1..28: mol_type = other DNA
aaaattcagcgagttacaggttgagggg

SEQ ID NO: 34101 - DNA, 28 bp, synthetic construct
  source 1..28: mol_type = other DNA
cctaagtggccagtgacaaggagctggg

SEQ ID NO: 34102 - DNA, 28 bp, synthetic construct
  source 1..28: mol_type = other DNA
gacaaggagctgggagcttgccctgagg

SEQ ID NO: 34103 - DNA, 28 bp, synthetic construct
  source 1..28: mol_type = other DNA
acaaggagctgggagcttgccctgaggg

SEQ ID NO: 34104 - DNA, 28 bp, synthetic construct
  source 1..28: mol_type = other DNA
gctgggagcttgccctgagggcagcagg

SEQ ID NO: 34105 - DNA, 28 bp, synthetic construct
  source 1..28: mol_type = other DNA
gggagcttgccctgagggcagcaggagg

SEQ ID NO: 34106 - DNA, 28 bp, synthetic construct
  source 1..28: mol_type = other DNA
ttgccctgagggcagcaggaggccatgg

SEQ ID NO: 34107 - DNA, 28 bp, synthetic construct
  source 1..28: mol_type = other DNA
tgccctgagggcagcaggaggccatggg

SEQ ID NO: 34108 - DNA, 28 bp, synthetic construct
  source 1..28: mol_type = other DNA
tgcccatggcctcctgctgccctcaggg

SEQ ID NO: 34109 - DNA, 28 bp, synthetic construct
  source 1..28: mol_type = other DNA
ttgcccatggcctcctgctgccctcagg

SEQ ID NO: 34110 - DNA, 28 bp, synthetic construct
  source 1..28: mol_type = other DNA
gcaggaggccatgggcaagcagagaagg

SEQ ID NO: 34111 - DNA, 28 bp, synthetic construct
  source 1..28: mol_type = other DNA
caggaggccatgggcaagcagagaaggg

SEQ ID NO: 34112 - DNA, 28 bp, synthetic construct
  source 1..28: mol_type = other DNA
ggccatgggcaagcagagaagggacagg

SEQ ID NO: 34113 - DNA, 28 bp, synthetic construct
  source 1..28: mol_type = other DNA
gccatgggcaagcagagaagggacaggg

SEQ ID NO: 34114 - DNA, 28 bp, synthetic construct
  source 1..28: mol_type = other DNA
accctgtcccttctctgcttgcccatgg

SEQ ID NO: 34115 - DNA, 28 bp, synthetic construct
  source 1..28: mol_type = other DNA
tgggcaagcagagaagggacagggtagg

SEQ ID NO: 34116 - DNA, 28 bp, synthetic construct
  source 1..28: mol_type = other DNA
gatttgactttcagaaacagtcctctgg

SEQ ID NO: 34117 - DNA, 28 bp, synthetic construct
  source 1..28: mol_type = other DNA
cagaaacagtcctctggttgctaaatgg

SEQ ID NO: 34118 - DNA, 28 bp, synthetic construct
  source 1..28: mol_type = other DNA
agaaacagtcctctggttgctaaatggg

SEQ ID NO: 34119 - DNA, 28 bp, synthetic construct
  source 1..28: mol_type = other DNA
gtcctctggttgctaaatgggagaaagg

SEQ ID NO: 34120 - DNA, 28 bp, synthetic construct
  source 1..28: mol_type = other DNA
ctcctttctcccatttagcaaccagagg

SEQ ID NO: 34121 - DNA, 28 bp, synthetic construct
  source 1..28: mol_type = other DNA
aaatgggagaaaggagtgacagtagagg

SEQ ID NO: 34122 - DNA, 28 bp, synthetic construct
  source 1..28: mol_type = other DNA
gggagaaaggagtgacagtagaggcagg

SEQ ID NO: 34123 - DNA, 28 bp, synthetic construct
  source 1..28: mol_type = other DNA
aaggagtgacagtagaggcaggagaagg

SEQ ID NO: 34124 - DNA, 28 bp, synthetic construct
  source 1..28: mol_type = other DNA
agtgacagtagaggcaggagaaggcagg

SEQ ID NO: 34125 - DNA, 28 bp, synthetic construct
  source 1..28: mol_type = other DNA
agaggcaggagaaggcaggatcagacgg

SEQ ID NO: 34126 - DNA, 28 bp, synthetic construct
  source 1..28: mol_type = other DNA
gaggcaggagaaggcaggatcagacggg

SEQ ID NO: 34127 - DNA, 28 bp, synthetic construct
  source 1..28: mol_type = other DNA
aggcaggagaaggcaggatcagacgggg

SEQ ID NO: 34128 - DNA, 28 bp, synthetic construct
  source 1..28: mol_type = other DNA
ggcaggagaaggcaggatcagacggggg

SEQ ID NO: 34129 - DNA, 28 bp, synthetic construct
  source 1..28: mol_type = other DNA
agaaggcaggatcagacgggggtgctgg

SEQ ID NO: 34130 - DNA, 28 bp, synthetic construct
  source 1..28: mol_type = other DNA
gaaggcaggatcagacgggggtgctggg

SEQ ID NO: 34131 - DNA, 28 bp, synthetic construct
  source 1..28: mol_type = other DNA
gcaggatcagacgggggtgctgggaagg

SEQ ID NO: 34132 - DNA, 28 bp, synthetic construct
  source 1..28: mol_type = other DNA
caggatcagacgggggtgctgggaaggg

SEQ ID NO: 34133 - DNA, 28 bp, synthetic construct
  source 1..28: mol_type = other DNA
aggatcagacgggggtgctgggaagggg

SEQ ID NO: 34134 - DNA, 28 bp, synthetic construct
  source 1..28: mol_type = other DNA
tcagacgggggtgctgggaaggggcagg

SEQ ID NO: 34135 - DNA, 28 bp, synthetic construct
  source 1..28: mol_type = other DNA
ggaaggggcaggtagaagagacatcagg

SEQ ID NO: 34136 - DNA, 28 bp, synthetic construct
  source 1..28: mol_type = other DNA
aggggcaggtagaagagacatcaggagg

SEQ ID NO: 34137 - DNA, 28 bp, synthetic construct
  source 1..28: mol_type = other DNA
agagacatcaggaggccaaacagatagg

SEQ ID NO: 34138 - DNA, 28 bp, synthetic construct
  source 1..28: mol_type = other DNA
ggtgcatcataaagtcctatctgtttgg

SEQ ID NO: 34139 - DNA, 28 bp, synthetic construct
  source 1..28: mol_type = other DNA
cagataggactttatgatgcaccgtagg

SEQ ID NO: 34140 - DNA, 28 bp, synthetic construct
  source 1..28: mol_type = other DNA
ctgtgtttgggtactggtatacctacgg

SEQ ID NO: 34141 - DNA, 28 bp, synthetic construct
  source 1..28: mol_type = other DNA
cgtaggtataccagtacccaaacacagg

SEQ ID NO: 34142 - DNA, 28 bp, synthetic construct
  source 1..28: mol_type = other DNA
aggtataccagtacccaaacacaggtgg

SEQ ID NO: 34143 - DNA, 28 bp, synthetic construct
  source 1..28: mol_type = other DNA
ctcttggccacctgtgtttgggtactgg

SEQ ID NO: 34144 - DNA, 28 bp, synthetic construct
  source 1..28: mol_type = other DNA
cctctgctcttggccacctgtgtttggg

SEQ ID NO: 34145 - DNA, 28 bp, synthetic construct
  source 1..28: mol_type = other DNA
ccctctgctcttggccacctgtgtttgg

SEQ ID NO: 34146 - DNA, 28 bp, synthetic construct
  source 1..28: mol_type = other DNA
ggctgggcgtctatccctctgctcttgg

SEQ ID NO: 34147 - DNA, 28 bp, synthetic construct
  source 1..28: mol_type = other DNA
cctggatgtctgtgaggaggaggctggg

SEQ ID NO: 34148 - DNA, 28 bp, synthetic construct
  source 1..28: mol_type = other DNA
gcctggatgtctgtgaggaggaggctgg

SEQ ID NO: 34149 - DNA, 28 bp, synthetic construct
  source 1..28: mol_type = other DNA
gcatgcctggatgtctgtgaggaggagg

SEQ ID NO: 34150 - DNA, 28 bp, synthetic construct
  source 1..28: mol_type = other DNA
tctgcatgcctggatgtctgtgaggagg

SEQ ID NO: 34151 - DNA, 28 bp, synthetic construct
  source 1..28: mol_type = other DNA
ggctctgcatgcctggatgtctgtgagg

SEQ ID NO: 34152 - DNA, 28 bp, synthetic construct
  source 1..28: mol_type = other DNA
tggcacgtggagggctctgcatgcctgg

SEQ ID NO: 34153 - DNA, 28 bp, synthetic construct
  source 1..28: mol_type = other DNA
agagccctccacgtgccaaacacacagg

SEQ ID NO: 34154 - DNA, 28 bp, synthetic construct
  source 1..28: mol_type = other DNA
gagccctccacgtgccaaacacacaggg

SEQ ID NO: 34155 - DNA, 28 bp, synthetic construct
  source 1..28: mol_type = other DNA
cggccctgtgtgtttggcacgtggaggg

SEQ ID NO: 34156 - DNA, 28 bp, synthetic construct
  source 1..28: mol_type = other DNA
tcggccctgtgtgtttggcacgtggagg

SEQ ID NO: 34157 - DNA, 28 bp, synthetic construct
  source 1..28: mol_type = other DNA
tccacgtgccaaacacacagggccgagg

SEQ ID NO: 34158 - DNA, 28 bp, synthetic construct
  source 1..28: mol_type = other DNA
tcctcggccctgtgtgtttggcacgtgg

SEQ ID NO: 34159 - DNA, 28 bp, synthetic construct
  source 1..28: mol_type = other DNA
gtgccaaacacacagggccgaggaatgg

SEQ ID NO: 34160 - DNA, 28 bp, synthetic construct
  source 1..28: mol_type = other DNA
cttccattcctcggccctgtgtgtttgg

SEQ ID NO: 34161 - DNA, 28 bp, synthetic construct
  source 1..28: mol_type = other DNA
tcggctctgctgcacttccattcctcgg

SEQ ID NO: 34162 - DNA, 28 bp, synthetic construct
  source 1..28: mol_type = other DNA
tggaagtgcagcagagccgatacgcagg

SEQ ID NO: 34163 - DNA, 28 bp, synthetic construct
  source 1..28: mol_type = other DNA
tattgcagatctgctgcctgcgtatcgg

SEQ ID NO: 34164 - DNA, 28 bp, synthetic construct
  source 1..28: mol_type = other DNA
cgcaggcagcagatctgcaataaccagg

SEQ ID NO: 34165 - DNA, 28 bp, synthetic construct
  source 1..28: mol_type = other DNA
aaccaggacacacagtcccaccagaagg

SEQ ID NO: 34166 - DNA, 28 bp, synthetic construct
  source 1..28: mol_type = other DNA
ctccttctggtgggactgtgtgtcctgg

SEQ ID NO: 34167 - DNA, 28 bp, synthetic construct
  source 1..28: mol_type = other DNA
cagtcccaccagaaggagagagcagtgg

SEQ ID NO: 34168 - DNA, 28 bp, synthetic construct
  source 1..28: mol_type = other DNA
cattccactgctctctccttctggtggg

SEQ ID NO: 34169 - DNA, 28 bp, synthetic construct
  source 1..28: mol_type = other DNA
tcattccactgctctctccttctggtgg

SEQ ID NO: 34170 - DNA, 28 bp, synthetic construct
  source 1..28: mol_type = other DNA
tgatcattccactgctctctccttctgg

SEQ ID NO: 34171 - DNA, 28 bp, synthetic construct
  source 1..28: mol_type = other DNA
agaaggagagagcagtggaatgatcagg

SEQ ID NO: 34172 - DNA, 28 bp, synthetic construct
  source 1..28: mol_type = other DNA
gaaggagagagcagtggaatgatcaggg

SEQ ID NO: 34173 - DNA, 28 bp, synthetic construct
  source 1..28: mol_type = other DNA
agggctcactgcagcctcgatctcttgg

SEQ ID NO: 34174 - DNA, 28 bp, synthetic construct
  source 1..28: mol_type = other DNA
aggaacgcttgagtccaagagatcgagg

SEQ ID NO: 34175 - DNA, 28 bp, synthetic construct
  source 1..28: mol_type = other DNA
cagctactagggaggctggagtgagagg

SEQ ID NO: 34176 - DNA, 28 bp, synthetic construct
  source 1..28: mol_type = other DNA
ctctcactccagcctccctagtagctgg

SEQ ID NO: 34177 - DNA, 28 bp, synthetic construct
  source 1..28: mol_type = other DNA
tctcactccagcctccctagtagctggg

SEQ ID NO: 34178 - DNA, 28 bp, synthetic construct
  source 1..28: mol_type = other DNA
ctgtggtcccagctactagggaggctgg

SEQ ID NO: 34179 - DNA, 28 bp, synthetic construct
  source 1..28: mol_type = other DNA
cagcctccctagtagctgggaccacagg

SEQ ID NO: 34180 - DNA, 28 bp, synthetic construct
  source 1..28: mol_type = other DNA
gtgcctgtggtcccagctactagggagg

SEQ ID NO: 34181 - DNA, 28 bp, synthetic construct
  source 1..28: mol_type = other DNA
cgtgtgcctgtggtcccagctactaggg

SEQ ID NO: 34182 - DNA, 28 bp, synthetic construct
  source 1..28: mol_type = other DNA
gcgtgtgcctgtggtcccagctactagg

SEQ ID NO: 34183 - DNA, 28 bp, synthetic construct
  source 1..28: mol_type = other DNA
gaccacaggcacacgccatgatacctgg

SEQ ID NO: 34184 - DNA, 28 bp, synthetic construct
  source 1..28: mol_type = other DNA
aaccaggtatcatggcgtgtgcctgtgg

SEQ ID NO: 34185 - DNA, 28 bp, synthetic construct
  source 1..28: mol_type = other DNA
aaaattaaaacttaaccaggtatcatgg

SEQ ID NO: 34186 - DNA, 28 bp, synthetic construct
  source 1..28: mol_type = other DNA
gaagtttaaaaattaaaacttaaccagg

SEQ ID NO: 34187 - DNA, 28 bp, synthetic construct
  source 1..28: mol_type = other DNA
ttaatttttaaacttcttgtagagatgg

SEQ ID NO: 34188 - DNA, 28 bp, synthetic construct
  source 1..28: mol_type = other DNA
taatttttaaacttcttgtagagatggg

SEQ ID NO: 34189 - DNA, 28 bp, synthetic construct
  source 1..28: mol_type = other DNA
aatttttaaacttcttgtagagatgggg

SEQ ID NO: 34190 - DNA, 28 bp, synthetic construct
  source 1..28: mol_type = other DNA
atttttaaacttcttgtagagatggggg

SEQ ID NO: 34191 - DNA, 28 bp, synthetic construct
  source 1..28: mol_type = other DNA
gggggtctcagtgcattgaccagtctgg

SEQ ID NO: 34192 - DNA, 28 bp, synthetic construct
  source 1..28: mol_type = other DNA
attgaccagtctggtctcgaactcctgg

SEQ ID NO: 34193 - DNA, 28 bp, synthetic construct
  source 1..28: mol_type = other DNA
ttgaccagtctggtctcgaactcctggg

SEQ ID NO: 34194 - DNA, 28 bp, synthetic construct
  source 1..28: mol_type = other DNA
tgagcccaggagttcgagaccagactgg

SEQ ID NO: 34195 - DNA, 28 bp, synthetic construct
  source 1..28: mol_type = other DNA
caaggtgggaggatcgcttgagcccagg

SEQ ID NO: 34196 - DNA, 28 bp, synthetic construct
  source 1..28: mol_type = other DNA
ctgggctcaagcgatcctcccaccttgg

SEQ ID NO: 34197 - DNA, 28 bp, synthetic construct
  source 1..28: mol_type = other DNA
cagcactttgggaggccaaggtgggagg

SEQ ID NO: 34198 - DNA, 28 bp, synthetic construct
  source 1..28: mol_type = other DNA
ctcccaccttggcctcccaaagtgctgg

SEQ ID NO: 34199 - DNA, 28 bp, synthetic construct
  source 1..28: mol_type = other DNA
tcccaccttggcctcccaaagtgctggg

SEQ ID NO: 34200 - DNA, 28 bp, synthetic construct
  source 1..28: mol_type = other DNA
tcccagcactttgggaggccaaggtggg

SEQ ID NO: 34201 - DNA, 28 bp, synthetic construct
  source 1..28: mol_type = other DNA
atcccagcactttgggaggccaaggtgg

SEQ ID NO: 34202 - DNA, 28 bp, synthetic construct
  source 1..28: mol_type = other DNA
gtaatcccagcactttgggaggccaagg

SEQ ID NO: 34203 - DNA, 28 bp, synthetic construct
  source 1..28: mol_type = other DNA
tggcctcccaaagtgctgggattacagg

SEQ ID NO: 34204 - DNA, 28 bp, synthetic construct
  source 1..28: mol_type = other DNA
actcctgtaatcccagcactttgggagg

SEQ ID NO: 34205 - DNA, 28 bp, synthetic construct
  source 1..28: mol_type = other DNA
ctcactcctgtaatcccagcactttggg

SEQ ID NO: 34206 - DNA, 28 bp, synthetic construct
  source 1..28: mol_type = other DNA
actcactcctgtaatcccagcactttgg

SEQ ID NO: 34207 - DNA, 28 bp, synthetic construct
  source 1..28: mol_type = other DNA
gattacaggagtgagttactgtgcccgg

SEQ ID NO: 34208 - DNA, 28 bp, synthetic construct
  source 1..28: mol_type = other DNA
atgggaataagaatagttgttggccggg

SEQ ID NO: 34209 - DNA, 28 bp, synthetic construct
  source 1..28: mol_type = other DNA
aatgggaataagaatagttgttggccgg

SEQ ID NO: 34210 - DNA, 28 bp, synthetic construct
  source 1..28: mol_type = other DNA
gtaaaatgggaataagaatagttgttgg

SEQ ID NO: 34211 - DNA, 28 bp, synthetic construct
  source 1..28: mol_type = other DNA
actattcttattcccattttacagatgg

SEQ ID NO: 34212 - DNA, 28 bp, synthetic construct
  source 1..28: mol_type = other DNA
tcccattttacagatggacaaactgagg

SEQ ID NO: 34213 - DNA, 28 bp, synthetic construct
  source 1..28: mol_type = other DNA
gcctcagtttgtccatctgtaaaatggg

SEQ ID NO: 34214 - DNA, 28 bp, synthetic construct
  source 1..28: mol_type = other DNA
agcctcagtttgtccatctgtaaaatgg

SEQ ID NO: 34215 - DNA, 28 bp, synthetic construct
  source 1..28: mol_type = other DNA
tttacagatggacaaactgaggctcagg

SEQ ID NO: 34216 - DNA, 28 bp, synthetic construct
  source 1..28: mol_type = other DNA
acagatggacaaactgaggctcaggagg

SEQ ID NO: 34217 - DNA, 28 bp, synthetic construct
  source 1..28: mol_type = other DNA
taactgtgggctacaggcaagtgactgg

SEQ ID NO: 34218 - DNA, 28 bp, synthetic construct
  source 1..28: mol_type = other DNA
tcacttgcctgtagcccacagttagtgg

SEQ ID NO: 34219 - DNA, 28 bp, synthetic construct
  source 1..28: mol_type = other DNA
agtgctaccactaactgtgggctacagg

SEQ ID NO: 34220 - DNA, 28 bp, synthetic construct
  source 1..28: mol_type = other DNA
tgtagcccacagttagtggtagcactgg

SEQ ID NO: 34221 - DNA, 28 bp, synthetic construct
  source 1..28: mol_type = other DNA
gtagcccacagttagtggtagcactggg

SEQ ID NO: 34222 - DNA, 28 bp, synthetic construct
  source 1..28: mol_type = other DNA
gaatcccagtgctaccactaactgtggg

SEQ ID NO: 34223 - DNA, 28 bp, synthetic construct
  source 1..28: mol_type = other DNA
ggaatcccagtgctaccactaactgtgg

SEQ ID NO: 34224 - DNA, 28 bp, synthetic construct
  source 1..28: mol_type = other DNA
tagtggtagcactgggattccaacttgg

SEQ ID NO: 34225 - DNA, 28 bp, synthetic construct
  source 1..28: mol_type = other DNA
agtggtagcactgggattccaacttggg

SEQ ID NO: 34226 - DNA, 28 bp, synthetic construct
  source 1..28: mol_type = other DNA
caggcgacatgaaggggacccaagttgg

SEQ ID NO: 34227 - DNA, 28 bp, synthetic construct
  source 1..28: mol_type = other DNA
gggtccccttcatgtcgcctgtatttgg

SEQ ID NO: 34228 - DNA, 28 bp, synthetic construct
  source 1..28: mol_type = other DNA
gacaccaaatacaggcgacatgaagggg

SEQ ID NO: 34229 - DNA, 28 bp, synthetic construct
  source 1..28: mol_type = other DNA
ggacaccaaatacaggcgacatgaaggg

SEQ ID NO: 34230 - DNA, 28 bp, synthetic construct
  source 1..28: mol_type = other DNA
gggacaccaaatacaggcgacatgaagg

SEQ ID NO: 34231 - DNA, 28 bp, synthetic construct
  source 1..28: mol_type = other DNA
gtcgcctgtatttggtgtcccatttagg

SEQ ID NO: 34232 - DNA, 28 bp, synthetic construct
  source 1..28: mol_type = other DNA
gacgcctaaatgggacaccaaatacagg

SEQ ID NO: 34233 - DNA, 28 bp, synthetic construct
  source 1..28: mol_type = other DNA
tggtgtcccatttaggcgtccatgcagg

SEQ ID NO: 34234 - DNA, 28 bp, synthetic construct
  source 1..28: mol_type = other DNA
ccaaaacctgcatggacgcctaaatggg

SEQ ID NO: 34235 - DNA, 28 bp, synthetic construct
  source 1..28: mol_type = other DNA
gccaaaacctgcatggacgcctaaatgg

SEQ ID NO: 34236 - DNA, 28 bp, synthetic construct
  source 1..28: mol_type = other DNA
atcttcagacacgccaaaacctgcatgg

SEQ ID NO: 34237 - DNA, 28 bp, synthetic construct
  source 1..28: mol_type = other DNA
tgtctccccaagtaagtgtcccccatgg

SEQ ID NO: 34238 - DNA, 28 bp, synthetic construct
  source 1..28: mol_type = other DNA
ggcatccatgggggacacttacttgggg

SEQ ID NO: 34239 - DNA, 28 bp, synthetic construct
  source 1..28: mol_type = other DNA
gggcatccatgggggacacttacttggg

SEQ ID NO: 34240 - DNA, 28 bp, synthetic construct
  source 1..28: mol_type = other DNA
tgggcatccatgggggacacttacttgg

SEQ ID NO: 34241 - DNA, 28 bp, synthetic construct
  source 1..28: mol_type = other DNA
gacacggctgggtgggcatccatggggg

SEQ ID NO: 34242 - DNA, 28 bp, synthetic construct
  source 1..28: mol_type = other DNA
ggacacggctgggtgggcatccatgggg

SEQ ID NO: 34243 - DNA, 28 bp, synthetic construct
  source 1..28: mol_type = other DNA
aggacacggctgggtgggcatccatggg

SEQ ID NO: 34244 - DNA, 28 bp, synthetic construct
  source 1..28: mol_type = other DNA
gaggacacggctgggtgggcatccatgg

SEQ ID NO: 34245 - DNA, 28 bp, synthetic construct
  source 1..28: mol_type = other DNA
cagagacaggaggacacggctgggtggg

SEQ ID NO: 34246 - DNA, 28 bp, synthetic construct
  source 1..28: mol_type = other DNA
tcagagacaggaggacacggctgggtgg

SEQ ID NO: 34247 - DNA, 28 bp, synthetic construct
  source 1..28: mol_type = other DNA
acccagccgtgtcctcctgtctctgagg

SEQ ID NO: 34248 - DNA, 28 bp, synthetic construct
  source 1..28: mol_type = other DNA
acctcagagacaggaggacacggctggg

SEQ ID NO: 34249 - DNA, 28 bp, synthetic construct
  source 1..28: mol_type = other DNA
aacctcagagacaggaggacacggctgg

SEQ ID NO: 34250 - DNA, 28 bp, synthetic construct
  source 1..28: mol_type = other DNA
gagaaacctcagagacaggaggacacgg

SEQ ID NO: 34251 - DNA, 28 bp, synthetic construct
  source 1..28: mol_type = other DNA
gtcctcctgtctctgaggtttctccagg

SEQ ID NO: 34252 - DNA, 28 bp, synthetic construct
  source 1..28: mol_type = other DNA
ttcctggagaaacctcagagacaggagg

SEQ ID NO: 34253 - DNA, 28 bp, synthetic construct
  source 1..28: mol_type = other DNA
cgattcctggagaaacctcagagacagg

SEQ ID NO: 34254 - DNA, 28 bp, synthetic construct
  source 1..28: mol_type = other DNA
gaggtttctccaggaatcgagctcctgg

SEQ ID NO: 34255 - DNA, 28 bp, synthetic construct
  source 1..28: mol_type = other DNA
ttctccaggaatcgagctcctggcctgg

SEQ ID NO: 34256 - DNA, 28 bp, synthetic construct
  source 1..28: mol_type = other DNA
caagccaggccaggagctcgattcctgg

SEQ ID NO: 34257 - DNA, 28 bp, synthetic construct
  source 1..28: mol_type = other DNA
cagacacactcagacaagccaggccagg

SEQ ID NO: 34258 - DNA, 28 bp, synthetic construct
  source 1..28: mol_type = other DNA
ggcctggcttgtctgagtgtgtctgtgg

SEQ ID NO: 34259 - DNA, 28 bp, synthetic construct
  source 1..28: mol_type = other DNA
gcctggcttgtctgagtgtgtctgtggg

SEQ ID NO: 34260 - DNA, 28 bp, synthetic construct
  source 1..28: mol_type = other DNA
gcccacagacacactcagacaagccagg

SEQ ID NO: 34261 - DNA, 28 bp, synthetic construct
  source 1..28: mol_type = other DNA
ggccagtagcatgcccctgcccgtctgg

SEQ ID NO: 34262 - DNA, 28 bp, synthetic construct
  source 1..28: mol_type = other DNA
gccagtagcatgcccctgcccgtctggg

SEQ ID NO: 34263 - DNA, 28 bp, synthetic construct
  source 1..28: mol_type = other DNA
acccagacgggcaggggcatgctactgg

SEQ ID NO: 34264 - DNA, 28 bp, synthetic construct
  source 1..28: mol_type = other DNA
cacgcagagggacccagacgggcagggg

SEQ ID NO: 34265 - DNA, 28 bp, synthetic construct
  source 1..28: mol_type = other DNA
acacgcagagggacccagacgggcaggg

SEQ ID NO: 34266 - DNA, 28 bp, synthetic construct
  source 1..28: mol_type = other DNA
gacacgcagagggacccagacgggcagg

SEQ ID NO: 34267 - DNA, 28 bp, synthetic construct
  source 1..28: mol_type = other DNA
cagagacacgcagagggacccagacggg

SEQ ID NO: 34268 - DNA, 28 bp, synthetic construct
  source 1..28: mol_type = other DNA
gcagagacacgcagagggacccagacgg

SEQ ID NO: 34269 - DNA, 28 bp, synthetic construct
  source 1..28: mol_type = other DNA
gctaggacaagcagagacacgcagaggg

SEQ ID NO: 34270 - DNA, 28 bp, synthetic construct
  source 1..28: mol_type = other DNA
ggctaggacaagcagagacacgcagagg

SEQ ID NO: 34271 - DNA, 28 bp, synthetic construct
  source 1..28: mol_type = other DNA
tagacgtcactgacacacacaggctagg

SEQ ID NO: 34272 - DNA, 28 bp, synthetic construct
  source 1..28: mol_type = other DNA
actcttagacgtcactgacacacacagg

SEQ ID NO: 34273 - DNA, 28 bp, synthetic construct
  source 1..28: mol_type = other DNA
gtgtgtgtgtgtgtgtccttgtccgagg

SEQ ID NO: 34274 - DNA, 28 bp, synthetic construct
  source 1..28: mol_type = other DNA
ccttgtccgaggagccgagagagtgagg

SEQ ID NO: 34275 - DNA, 28 bp, synthetic construct
  source 1..28: mol_type = other DNA
cttgtccgaggagccgagagagtgaggg

SEQ ID NO: 34276 - DNA, 28 bp, synthetic construct
  source 1..28: mol_type = other DNA
ttgtccgaggagccgagagagtgagggg

SEQ ID NO: 34277 - DNA, 28 bp, synthetic construct
  source 1..28: mol_type = other DNA
tgtccgaggagccgagagagtgaggggg

SEQ ID NO: 34278 - DNA, 28 bp, synthetic construct
  source 1..28: mol_type = other DNA
attccccctcactctctcggctcctcgg

SEQ ID NO: 34279 - DNA, 28 bp, synthetic construct
  source 1..28: mol_type = other DNA
gagccgagagagtgagggggaatgaagg

SEQ ID NO: 34280 - DNA, 28 bp, synthetic construct
  source 1..28: mol_type = other DNA
agccgagagagtgagggggaatgaaggg

SEQ ID NO: 34281 - DNA, 28 bp, synthetic construct
  source 1..28: mol_type = other DNA
ggcccttcattccccctcactctctcgg

SEQ ID NO: 34282 - DNA, 28 bp, synthetic construct
  source 1..28: mol_type = other DNA
gagagtgagggggaatgaagggccaagg

SEQ ID NO: 34283 - DNA, 28 bp, synthetic construct
  source 1..28: mol_type = other DNA
agtgagggggaatgaagggccaaggagg

SEQ ID NO: 34284 - DNA, 28 bp, synthetic construct
  source 1..28: mol_type = other DNA
gggggaatgaagggccaaggaggcctgg

SEQ ID NO: 34285 - DNA, 28 bp, synthetic construct
  source 1..28: mol_type = other DNA
gaatgaagggccaaggaggcctggctgg

SEQ ID NO: 34286 - DNA, 28 bp, synthetic construct
  source 1..28: mol_type = other DNA
aatgaagggccaaggaggcctggctggg

SEQ ID NO: 34287 - DNA, 28 bp, synthetic construct
  source 1..28: mol_type = other DNA
atgaagggccaaggaggcctggctgggg

SEQ ID NO: 34288 - DNA, 28 bp, synthetic construct
  source 1..28: mol_type = other DNA
agggccaaggaggcctggctggggctgg

SEQ ID NO: 34289 - DNA, 28 bp, synthetic construct
  source 1..28: mol_type = other DNA
gggccaaggaggcctggctggggctggg

SEQ ID NO: 34290 - DNA, 28 bp, synthetic construct
  source 1..28: mol_type = other DNA
cagcccagccccagccaggcctccttgg

SEQ ID NO: 34291 - DNA, 28 bp, synthetic construct
  source 1..28: mol_type = other DNA
caaggaggcctggctggggctgggctgg

SEQ ID NO: 34292 - DNA, 28 bp, synthetic construct
  source 1..28: mol_type = other DNA
aaggaggcctggctggggctgggctggg

SEQ ID NO: 34293 - DNA, 28 bp, synthetic construct
  source 1..28: mol_type = other DNA
aggaggcctggctggggctgggctgggg

SEQ ID NO: 34294 - DNA, 28 bp, synthetic construct
  source 1..28: mol_type = other DNA
ggaggcctggctggggctgggctggggg

SEQ ID NO: 34295 - DNA, 28 bp, synthetic construct
  source 1..28: mol_type = other DNA
ggcctggctggggctgggctgggggtgg

SEQ ID NO: 34296 - DNA, 28 bp, synthetic construct
  source 1..28: mol_type = other DNA
ctccacccccagcccagccccagccagg

SEQ ID NO: 34297 - DNA, 28 bp, synthetic construct
  source 1..28: mol_type = other DNA
ctggctggggctgggctgggggtggagg

SEQ ID NO: 34298 - DNA, 28 bp, synthetic construct
  source 1..28: mol_type = other DNA
gctggggctgggctgggggtggaggcgg

SEQ ID NO: 34299 - DNA, 28 bp, synthetic construct
  source 1..28: mol_type = other DNA
ctggggctgggctgggggtggaggcggg

SEQ ID NO: 34300 - DNA, 28 bp, synthetic construct
  source 1..28: mol_type = other DNA
tggggctgggctgggggtggaggcgggg

SEQ ID NO: 34301 - DNA, 28 bp, synthetic construct
  source 1..28: mol_type = other DNA
ctgggctgggggtggaggcggggagagg

SEQ ID NO: 34302 - DNA, 28 bp, synthetic construct
  source 1..28: mol_type = other DNA
tgggctgggggtggaggcggggagaggg

SEQ ID NO: 34303 - DNA, 28 bp, synthetic construct
  source 1..28: mol_type = other DNA
gggctgggggtggaggcggggagagggg

SEQ ID NO: 34304 - DNA, 28 bp, synthetic construct
  source 1..28: mol_type = other DNA
ggtggaggcggggagaggggcgtcacgg

SEQ ID NO: 34305 - DNA, 28 bp, synthetic construct
  source 1..28: mol_type = other DNA
gaggggcgtcacggcctgagctgagagg

SEQ ID NO: 34306 - DNA, 28 bp, synthetic construct
  source 1..28: mol_type = other DNA
aggggcgtcacggcctgagctgagaggg

SEQ ID NO: 34307 - DNA, 28 bp, synthetic construct
  source 1..28: mol_type = other DNA
ggggcgtcacggcctgagctgagagggg

SEQ ID NO: 34308 - DNA, 28 bp, synthetic construct
  source 1..28: mol_type = other DNA
gtcacggcctgagctgagaggggagtgg

SEQ ID NO: 34309 - DNA, 28 bp, synthetic construct
  source 1..28: mol_type = other DNA
cagaactccactcccctctcagctcagg

SEQ ID NO: 34310 - DNA, 28 bp, synthetic construct
  source 1..28: mol_type = other DNA
ctgagctgagaggggagtggagttctgg

SEQ ID NO: 34311 - DNA, 28 bp, synthetic construct
  source 1..28: mol_type = other DNA
agctgagaggggagtggagttctggagg

SEQ ID NO: 34312 - DNA, 28 bp, synthetic construct
  source 1..28: mol_type = other DNA
aatgtttaccagacacagagcccagagg

SEQ ID NO: 34313 - DNA, 28 bp, synthetic construct
  source 1..28: mol_type = other DNA
atgtttaccagacacagagcccagaggg

SEQ ID NO: 34314 - DNA, 28 bp, synthetic construct
  source 1..28: mol_type = other DNA
gcgctgtccctctgggctctgtgtctgg

SEQ ID NO: 34315 - DNA, 28 bp, synthetic construct
  source 1..28: mol_type = other DNA
gcccagagggacagcgcccagagcccgg

SEQ ID NO: 34316 - DNA, 28 bp, synthetic construct
  source 1..28: mol_type = other DNA
tccgggctctgggcgctgtccctctggg

SEQ ID NO: 34317 - DNA, 28 bp, synthetic construct
  source 1..28: mol_type = other DNA
atccgggctctgggcgctgtccctctgg

SEQ ID NO: 34318 - DNA, 28 bp, synthetic construct
  source 1..28: mol_type = other DNA
cgcccagagcccggatagagagacacgg

SEQ ID NO: 34319 - DNA, 28 bp, synthetic construct
  source 1..28: mol_type = other DNA
ggccgtgtctctctatccgggctctggg

SEQ ID NO: 34320 - DNA, 28 bp, synthetic construct
  source 1..28: mol_type = other DNA
aggccgtgtctctctatccgggctctgg

SEQ ID NO: 34321 - DNA, 28 bp, synthetic construct
  source 1..28: mol_type = other DNA
ccagtgaggccgtgtctctctatccggg

SEQ ID NO: 34322 - DNA, 28 bp, synthetic construct
  source 1..28: mol_type = other DNA
gccagtgaggccgtgtctctctatccgg

SEQ ID NO: 34323 - DNA, 28 bp, synthetic construct
  source 1..28: mol_type = other DNA
tagagagacacggcctcactggctcagg

SEQ ID NO: 34324 - DNA, 28 bp, synthetic construct
  source 1..28: mol_type = other DNA
agacacggcctcactggctcaggacagg

SEQ ID NO: 34325 - DNA, 28 bp, synthetic construct
  source 1..28: mol_type = other DNA
gacacggcctcactggctcaggacaggg

SEQ ID NO: 34326 - DNA, 28 bp, synthetic construct
  source 1..28: mol_type = other DNA
acacggcctcactggctcaggacagggg

SEQ ID NO: 34327 - DNA, 28 bp, synthetic construct
  source 1..28: mol_type = other DNA
cacggcctcactggctcaggacaggggg

SEQ ID NO: 34328 - DNA, 28 bp, synthetic construct
  source 1..28: mol_type = other DNA
ctgtgccccctgtcctgagccagtgagg

SEQ ID NO: 34329 - DNA, 28 bp, synthetic construct
  source 1..28: mol_type = other DNA
gctcaggacagggggcacagccaccagg

SEQ ID NO: 34330 - DNA, 28 bp, synthetic construct
  source 1..28: mol_type = other DNA
ctcaggacagggggcacagccaccaggg

SEQ ID NO: 34331 - DNA, 28 bp, synthetic construct
  source 1..28: mol_type = other DNA
ctgaggagggggaaggggaccctggtgg

SEQ ID NO: 34332 - DNA, 28 bp, synthetic construct
  source 1..28: mol_type = other DNA
gagctgaggagggggaaggggaccctgg

SEQ ID NO: 34333 - DNA, 28 bp, synthetic construct
  source 1..28: mol_type = other DNA
agggagggagctgaggagggggaagggg

SEQ ID NO: 34334 - DNA, 28 bp, synthetic construct
  source 1..28: mol_type = other DNA
cagggagggagctgaggagggggaaggg

SEQ ID NO: 34335 - DNA, 28 bp, synthetic construct
  source 1..28: mol_type = other DNA
ccagggagggagctgaggagggggaagg

SEQ ID NO: 34336 - DNA, 28 bp, synthetic construct
  source 1..28: mol_type = other DNA
ggggccagggagggagctgaggaggggg

SEQ ID NO: 34337 - DNA, 28 bp, synthetic construct
  source 1..28: mol_type = other DNA
aggggccagggagggagctgaggagggg

SEQ ID NO: 34338 - DNA, 28 bp, synthetic construct
  source 1..28: mol_type = other DNA
aaggggccagggagggagctgaggaggg

SEQ ID NO: 34339 - DNA, 28 bp, synthetic construct
  source 1..28: mol_type = other DNA
aaaggggccagggagggagctgaggagg

SEQ ID NO: 34340 - DNA, 28 bp, synthetic construct
  source 1..28: mol_type = other DNA
cttaaaggggccagggagggagctgagg

SEQ ID NO: 34341 - DNA, 28 bp, synthetic construct
  source 1..28: mol_type = other DNA
agctctttcttaaaggggccagggaggg

SEQ ID NO: 34342 - DNA, 28 bp, synthetic construct
  source 1..28: mol_type = other DNA
cagctctttcttaaaggggccagggagg

SEQ ID NO: 34343 - DNA, 28 bp, synthetic construct
  source 1..28: mol_type = other DNA
gatcagctctttcttaaaggggccaggg

SEQ ID NO: 34344 - DNA, 28 bp, synthetic construct
  source 1..28: mol_type = other DNA
ggatcagctctttcttaaaggggccagg

SEQ ID NO: 34345 - DNA, 28 bp, synthetic construct
  source 1..28: mol_type = other DNA
ggagaggatcagctctttcttaaagggg

SEQ ID NO: 34346 - DNA, 28 bp, synthetic construct
  source 1..28: mol_type = other DNA
aggagaggatcagctctttcttaaaggg

SEQ ID NO: 34347 - DNA, 28 bp, synthetic construct
  source 1..28: mol_type = other DNA
gaggagaggatcagctctttcttaaagg

SEQ ID NO: 34348 - DNA, 28 bp, synthetic construct
  source 1..28: mol_type = other DNA
atcaggggttaactcaagagaggagagg

SEQ ID NO: 34349 - DNA, 28 bp, synthetic construct
  source 1..28: mol_type = other DNA
ggacaatcaggggttaactcaagagagg

SEQ ID NO: 34350 - DNA, 28 bp, synthetic construct
  source 1..28: mol_type = other DNA
ctcttgagttaacccctgattgtccagg

SEQ ID NO: 34351 - DNA, 28 bp, synthetic construct
  source 1..28: mol_type = other DNA
ttgagttaacccctgattgtccaggtgg

SEQ ID NO: 34352 - DNA, 28 bp, synthetic construct
  source 1..28: mol_type = other DNA
aacccctgattgtccaggtggcccctgg

SEQ ID NO: 34353 - DNA, 28 bp, synthetic construct
  source 1..28: mol_type = other DNA
acccctgattgtccaggtggcccctggg

SEQ ID NO: 34354 - DNA, 28 bp, synthetic construct
  source 1..28: mol_type = other DNA
gcccaggggccacctggacaatcagggg

SEQ ID NO: 34355 - DNA, 28 bp, synthetic construct
  source 1..28: mol_type = other DNA
agcccaggggccacctggacaatcaggg

SEQ ID NO: 34356 - DNA, 28 bp, synthetic construct
  source 1..28: mol_type = other DNA
gagcccaggggccacctggacaatcagg

SEQ ID NO: 34357 - DNA, 28 bp, synthetic construct
  source 1..28: mol_type = other DNA
gattgtccaggtggcccctgggctctgg

SEQ ID NO: 34358 - DNA, 28 bp, synthetic construct
  source 1..28: mol_type = other DNA
ccaggtggcccctgggctctggccctgg

SEQ ID NO: 34359 - DNA, 28 bp, synthetic construct
  source 1..28: mol_type = other DNA
ggtggcccctgggctctggccctggtgg

SEQ ID NO: 34360 - DNA, 28 bp, synthetic construct
  source 1..28: mol_type = other DNA
gtggcccctgggctctggccctggtggg

SEQ ID NO: 34361 - DNA, 28 bp, synthetic construct
  source 1..28: mol_type = other DNA
gcccctgggctctggccctggtgggcgg

SEQ ID NO: 34362 - DNA, 28 bp, synthetic construct
  source 1..28: mol_type = other DNA
tccgcccaccagggccagagcccagggg

SEQ ID NO: 34363 - DNA, 28 bp, synthetic construct
  source 1..28: mol_type = other DNA
ctccgcccaccagggccagagcccaggg

SEQ ID NO: 34364 - DNA, 28 bp, synthetic construct
  source 1..28: mol_type = other DNA
cctgggctctggccctggtgggcggagg

SEQ ID NO: 34365 - DNA, 28 bp, synthetic construct
  source 1..28: mol_type = other DNA
ctctggccctggtgggcggaggcaaagg

SEQ ID NO: 34366 - DNA, 28 bp, synthetic construct
  source 1..28: mol_type = other DNA
tctggccctggtgggcggaggcaaaggg

SEQ ID NO: 34367 - DNA, 28 bp, synthetic construct
  source 1..28: mol_type = other DNA
ctggccctggtgggcggaggcaaagggg

SEQ ID NO: 34368 - DNA, 28 bp, synthetic construct
  source 1..28: mol_type = other DNA
tggccctggtgggcggaggcaaaggggg

SEQ ID NO: 34369 - DNA, 28 bp, synthetic construct
  source 1..28: mol_type = other DNA
gctccccctttgcctccgcccaccaggg

SEQ ID NO: 34370 - DNA, 28 bp, synthetic construct
  source 1..28: mol_type = other DNA
ggctccccctttgcctccgcccaccagg

SEQ ID NO: 34371 - DNA, 28 bp, synthetic construct
  source 1..28: mol_type = other DNA
ggtgggcggaggcaaagggggagccagg

SEQ ID NO: 34372 - DNA, 28 bp, synthetic construct
  source 1..28: mol_type = other DNA
gtgggcggaggcaaagggggagccaggg

SEQ ID NO: 34373 - DNA, 28 bp, synthetic construct
  source 1..28: mol_type = other DNA
tgggcggaggcaaagggggagccagggg

SEQ ID NO: 34374 - DNA, 28 bp, synthetic construct
  source 1..28: mol_type = other DNA
gcggaggcaaagggggagccaggggcgg

SEQ ID NO: 34375 - DNA, 28 bp, synthetic construct
  source 1..28: mol_type = other DNA
caaagggggagccaggggcggagaaagg

SEQ ID NO: 34376 - DNA, 28 bp, synthetic construct
  source 1..28: mol_type = other DNA
aaagggggagccaggggcggagaaaggg

SEQ ID NO: 34377 - DNA, 28 bp, synthetic construct
  source 1..28: mol_type = other DNA
acttgggcaaccctttctccgcccctgg

SEQ ID NO: 34378 - DNA, 28 bp, synthetic construct
  source 1..28: mol_type = other DNA
gggcggagaaagggttgcccaagtctgg

SEQ ID NO: 34379 - DNA, 28 bp, synthetic construct
  source 1..28: mol_type = other DNA
ggcggagaaagggttgcccaagtctggg

SEQ ID NO: 34380 - DNA, 28 bp, synthetic construct
  source 1..28: mol_type = other DNA
aaagggttgcccaagtctgggagtgagg

SEQ ID NO: 34381 - DNA, 28 bp, synthetic construct
  source 1..28: mol_type = other DNA
aagggttgcccaagtctgggagtgaggg

SEQ ID NO: 34382 - DNA, 28 bp, synthetic construct
  source 1..28: mol_type = other DNA
gttgcccaagtctgggagtgagggaagg

SEQ ID NO: 34383 - DNA, 28 bp, synthetic construct
  source 1..28: mol_type = other DNA
gcccaagtctgggagtgagggaaggagg

SEQ ID NO: 34384 - DNA, 28 bp, synthetic construct
  source 1..28: mol_type = other DNA
gcctccttccctcactcccagacttggg

SEQ ID NO: 34385 - DNA, 28 bp, synthetic construct
  source 1..28: mol_type = other DNA
tgcctccttccctcactcccagacttgg

SEQ ID NO: 34386 - DNA, 28 bp, synthetic construct
  source 1..28: mol_type = other DNA
aagtctgggagtgagggaaggaggcagg

SEQ ID NO: 34387 - DNA, 28 bp, synthetic construct
  source 1..28: mol_type = other DNA
agtctgggagtgagggaaggaggcaggg

SEQ ID NO: 34388 - DNA, 28 bp, synthetic construct
  source 1..28: mol_type = other DNA
gtctgggagtgagggaaggaggcagggg

SEQ ID NO: 34389 - DNA, 28 bp, synthetic construct
  source 1..28: mol_type = other DNA
agggaaggaggcaggggtgctgagaagg

SEQ ID NO: 34390 - DNA, 28 bp, synthetic construct
  source 1..28: mol_type = other DNA
gaaggaggcaggggtgctgagaaggcgg

SEQ ID NO: 34391 - DNA, 28 bp, synthetic construct
  source 1..28: mol_type = other DNA
gcaggggtgctgagaaggcggctgctgg

SEQ ID NO: 34392 - DNA, 28 bp, synthetic construct
  source 1..28: mol_type = other DNA
caggggtgctgagaaggcggctgctggg

SEQ ID NO: 34393 - DNA, 28 bp, synthetic construct
  source 1..28: mol_type = other DNA
tgagaaggcggctgctgggcagagccgg

SEQ ID NO: 34394 - DNA, 28 bp, synthetic construct
  source 1..28: mol_type = other DNA
gaaggcggctgctgggcagagccggtgg

SEQ ID NO: 34395 - DNA, 28 bp, synthetic construct
  source 1..28: mol_type = other DNA
cggctgctgggcagagccggtggcaagg

SEQ ID NO: 34396 - DNA, 28 bp, synthetic construct
  source 1..28: mol_type = other DNA
ggctgctgggcagagccggtggcaaggg

SEQ ID NO: 34397 - DNA, 28 bp, synthetic construct
  source 1..28: mol_type = other DNA
cagcggcaggggaggcccttgccaccgg

SEQ ID NO: 34398 - DNA, 28 bp, synthetic construct
  source 1..28: mol_type = other DNA
caagggcctcccctgccgctgtgccagg

SEQ ID NO: 34399 - DNA, 28 bp, synthetic construct
  source 1..28: mol_type = other DNA
ggcctcccctgccgctgtgccaggcagg

SEQ ID NO: 34400 - DNA, 28 bp, synthetic construct
  source 1..28: mol_type = other DNA
tgcctgcctggcacagcggcaggggagg

SEQ ID NO: 34401 - DNA, 28 bp, synthetic construct
  source 1..28: mol_type = other DNA
cactgcctgcctggcacagcggcagggg

SEQ ID NO: 34402 - DNA, 28 bp, synthetic construct
  source 1..28: mol_type = other DNA
gcactgcctgcctggcacagcggcaggg

SEQ ID NO: 34403 - DNA, 28 bp, synthetic construct
  source 1..28: mol_type = other DNA
ggcactgcctgcctggcacagcggcagg

SEQ ID NO: 34404 - DNA, 28 bp, synthetic construct
  source 1..28: mol_type = other DNA
atttggcactgcctgcctggcacagcgg

SEQ ID NO: 34405 - DNA, 28 bp, synthetic construct
  source 1..28: mol_type = other DNA
tgtgccaggcaggcagtgccaaatccgg

SEQ ID NO: 34406 - DNA, 28 bp, synthetic construct
  source 1..28: mol_type = other DNA
gtgccaggcaggcagtgccaaatccggg

SEQ ID NO: 34407 - DNA, 28 bp, synthetic construct
  source 1..28: mol_type = other DNA
tgccaggcaggcagtgccaaatccgggg

SEQ ID NO: 34408 - DNA, 28 bp, synthetic construct
  source 1..28: mol_type = other DNA
ctccccggatttggcactgcctgcctgg

SEQ ID NO: 34409 - DNA, 28 bp, synthetic construct
  source 1..28: mol_type = other DNA
caggcagtgccaaatccggggagcctgg

SEQ ID NO: 34410 - DNA, 28 bp, synthetic construct
  source 1..28: mol_type = other DNA
gtgccaaatccggggagcctggagctgg

SEQ ID NO: 34411 - DNA, 28 bp, synthetic construct
  source 1..28: mol_type = other DNA
tgccaaatccggggagcctggagctggg

SEQ ID NO: 34412 - DNA, 28 bp, synthetic construct
  source 1..28: mol_type = other DNA
gccaaatccggggagcctggagctgggg

SEQ ID NO: 34413 - DNA, 28 bp, synthetic construct
  source 1..28: mol_type = other DNA
cccccagctccaggctccccggatttgg

SEQ ID NO: 34414 - DNA, 28 bp, synthetic construct
  source 1..28: mol_type = other DNA
caaatccggggagcctggagctgggggg

SEQ ID NO: 34415 - DNA, 28 bp, synthetic construct
  source 1..28: mol_type = other DNA
atccggggagcctggagctggggggagg

SEQ ID NO: 34416 - DNA, 28 bp, synthetic construct
  source 1..28: mol_type = other DNA
tccggggagcctggagctggggggaggg

SEQ ID NO: 34417 - DNA, 28 bp, synthetic construct
  source 1..28: mol_type = other DNA
gccctccccccagctccaggctccccgg

SEQ ID NO: 34418 - DNA, 28 bp, synthetic construct
  source 1..28: mol_type = other DNA
gggagcctggagctggggggagggccgg

SEQ ID NO: 34419 - DNA, 28 bp, synthetic construct
  source 1..28: mol_type = other DNA
ggagcctggagctggggggagggccggg

SEQ ID NO: 34420 - DNA, 28 bp, synthetic construct
  source 1..28: mol_type = other DNA
gagcctggagctggggggagggccgggg

SEQ ID NO: 34421 - DNA, 28 bp, synthetic construct
  source 1..28: mol_type = other DNA
tgtccccggccctccccccagctccagg

SEQ ID NO: 34422 - DNA, 28 bp, synthetic construct
  source 1..28: mol_type = other DNA
gctggggggagggccggggacagcccgg

SEQ ID NO: 34423 - DNA, 28 bp, synthetic construct
  source 1..28: mol_type = other DNA
ggagggggcagggccgggctgtccccgg

SEQ ID NO: 34424 - DNA, 28 bp, synthetic construct
  source 1..28: mol_type = other DNA
agcccggccctgccccctcccccgctgg

SEQ ID NO: 34425 - DNA, 28 bp, synthetic construct
  source 1..28: mol_type = other DNA
gcccggccctgccccctcccccgctggg

SEQ ID NO: 34426 - DNA, 28 bp, synthetic construct
  source 1..28: mol_type = other DNA
tcccagcgggggagggggcagggccggg

SEQ ID NO: 34427 - DNA, 28 bp, synthetic construct
  source 1..28: mol_type = other DNA
ctcccagcgggggagggggcagggccgg

SEQ ID NO: 34428 - DNA, 28 bp, synthetic construct
  source 1..28: mol_type = other DNA
tgggctcccagcgggggagggggcaggg

SEQ ID NO: 34429 - DNA, 28 bp, synthetic construct
  source 1..28: mol_type = other DNA
ttgggctcccagcgggggagggggcagg

SEQ ID NO: 34430 - DNA, 28 bp, synthetic construct
  source 1..28: mol_type = other DNA
gttgttgggctcccagcgggggaggggg

SEQ ID NO: 34431 - DNA, 28 bp, synthetic construct
  source 1..28: mol_type = other DNA
agttgttgggctcccagcgggggagggg

SEQ ID NO: 34432 - DNA, 28 bp, synthetic construct
  source 1..28: mol_type = other DNA
aagttgttgggctcccagcgggggaggg

SEQ ID NO: 34433 - DNA, 28 bp, synthetic construct
  source 1..28: mol_type = other DNA
gaagttgttgggctcccagcgggggagg

SEQ ID NO: 34434 - DNA, 28 bp, synthetic construct
  source 1..28: mol_type = other DNA
tcagaagttgttgggctcccagcggggg

SEQ ID NO: 34435 - DNA, 28 bp, synthetic construct
  source 1..28: mol_type = other DNA
ctcagaagttgttgggctcccagcgggg

SEQ ID NO: 34436 - DNA, 28 bp, synthetic construct
  source 1..28: mol_type = other DNA
cctcagaagttgttgggctcccagcggg

SEQ ID NO: 34437 - DNA, 28 bp, synthetic construct
  source 1..28: mol_type = other DNA
tcctcagaagttgttgggctcccagcgg

SEQ ID NO: 34438 - DNA, 28 bp, synthetic construct
  source 1..28: mol_type = other DNA
agcccaacaacttctgaggaaagtttgg

SEQ ID NO: 34439 - DNA, 28 bp, synthetic construct
  source 1..28: mol_type = other DNA
tgccaaactttcctcagaagttgttggg

SEQ ID NO: 34440 - DNA, 28 bp, synthetic construct
  source 1..28: mol_type = other DNA
gtgccaaactttcctcagaagttgttgg

SEQ ID NO: 34441 - DNA, 28 bp, synthetic construct
  source 1..28: mol_type = other DNA
acttctgaggaaagtttggcacccatgg

SEQ ID NO: 34442 - DNA, 28 bp, synthetic construct
  source 1..28: mol_type = other DNA
tgaggaaagtttggcacccatggcgtgg

SEQ ID NO: 34443 - DNA, 28 bp, synthetic construct
  source 1..28: mol_type = other DNA
ggaaagtttggcacccatggcgtggcgg

SEQ ID NO: 34444 - DNA, 28 bp, synthetic construct
  source 1..28: mol_type = other DNA
ggcacccatggcgtggcggtgccccagg

SEQ ID NO: 34445 - DNA, 28 bp, synthetic construct
  source 1..28: mol_type = other DNA
ccatcctggggcaccgccacgccatggg

SEQ ID NO: 34446 - DNA, 28 bp, synthetic construct
  source 1..28: mol_type = other DNA
cccatcctggggcaccgccacgccatgg

SEQ ID NO: 34447 - DNA, 28 bp, synthetic construct
  source 1..28: mol_type = other DNA
ggcgtggcggtgccccaggatgggcagg

SEQ ID NO: 34448 - DNA, 28 bp, synthetic construct
  source 1..28: mol_type = other DNA
gcgtggcggtgccccaggatgggcaggg

SEQ ID NO: 34449 - DNA, 28 bp, synthetic construct
  source 1..28: mol_type = other DNA
tgccccaggatgggcagggtcccgctgg

SEQ ID NO: 34450 - DNA, 28 bp, synthetic construct
  source 1..28: mol_type = other DNA
ggccagcgggaccctgcccatcctgggg

SEQ ID NO: 34451 - DNA, 28 bp, synthetic construct
  source 1..28: mol_type = other DNA
aggccagcgggaccctgcccatcctggg

SEQ ID NO: 34452 - DNA, 28 bp, synthetic construct
  source 1..28: mol_type = other DNA
caggccagcgggaccctgcccatcctgg

SEQ ID NO: 34453 - DNA, 28 bp, synthetic construct
  source 1..28: mol_type = other DNA
caggatgggcagggtcccgctggcctgg

SEQ ID NO: 34454 - DNA, 28 bp, synthetic construct
  source 1..28: mol_type = other DNA
ggcagggtcccgctggcctggtgcttgg

SEQ ID NO: 34455 - DNA, 28 bp, synthetic construct
  source 1..28: mol_type = other DNA
gcacagcgccaagcaccaggccagcggg

SEQ ID NO: 34456 - DNA, 28 bp, synthetic construct
  source 1..28: mol_type = other DNA
cgcacagcgccaagcaccaggccagcgg

SEQ ID NO: 34457 - DNA, 28 bp, synthetic construct
  source 1..28: mol_type = other DNA
cgctggcctggtgcttggcgctgtgcgg

SEQ ID NO: 34458 - DNA, 28 bp, synthetic construct
  source 1..28: mol_type = other DNA
ggcctggtgcttggcgctgtgcggctgg

SEQ ID NO: 34459 - DNA, 28 bp, synthetic construct
  source 1..28: mol_type = other DNA
gcctggtgcttggcgctgtgcggctggg

SEQ ID NO: 34460 - DNA, 28 bp, synthetic construct
  source 1..28: mol_type = other DNA
gcccagccgcacagcgccaagcaccagg

SEQ ID NO: 34461 - DNA, 28 bp, synthetic construct
  source 1..28: mol_type = other DNA
ttggcgctgtgcggctgggcgtgcatgg

SEQ ID NO: 34462 - DNA, 28 bp, synthetic construct
  source 1..28: mol_type = other DNA
gtgcggctgggcgtgcatggcccccagg

SEQ ID NO: 34463 - DNA, 28 bp, synthetic construct
  source 1..28: mol_type = other DNA
tgcggctgggcgtgcatggcccccaggg

SEQ ID NO: 34464 - DNA, 28 bp, synthetic construct
  source 1..28: mol_type = other DNA
gcggctgggcgtgcatggcccccagggg

SEQ ID NO: 34465 - DNA, 28 bp, synthetic construct
  source 1..28: mol_type = other DNA
gtgcatggcccccaggggtgagtgatgg

SEQ ID NO: 34466 - DNA, 28 bp, synthetic construct
  source 1..28: mol_type = other DNA
tgcatggcccccaggggtgagtgatggg

SEQ ID NO: 34467 - DNA, 28 bp, synthetic construct
  source 1..28: mol_type = other DNA
gcatggcccccaggggtgagtgatgggg

SEQ ID NO: 34468 - DNA, 28 bp, synthetic construct
  source 1..28: mol_type = other DNA
catggcccccaggggtgagtgatggggg

SEQ ID NO: 34469 - DNA, 28 bp, synthetic construct
  source 1..28: mol_type = other DNA
aggagcccccatcactcacccctggggg

SEQ ID NO: 34470 - DNA, 28 bp, synthetic construct
  source 1..28: mol_type = other DNA
aaggagcccccatcactcacccctgggg

SEQ ID NO: 34471 - DNA, 28 bp, synthetic construct
  source 1..28: mol_type = other DNA
caaggagcccccatcactcacccctggg

SEQ ID NO: 34472 - DNA, 28 bp, synthetic construct
  source 1..28: mol_type = other DNA
ccaaggagcccccatcactcacccctgg

SEQ ID NO: 34473 - DNA, 28 bp, synthetic construct
  source 1..28: mol_type = other DNA
caggggtgagtgatgggggctccttggg

SEQ ID NO: 34474 - DNA, 28 bp, synthetic construct
  source 1..28: mol_type = other DNA
aggggtgagtgatgggggctccttgggg

SEQ ID NO: 34475 - DNA, 28 bp, synthetic construct
  source 1..28: mol_type = other DNA
gtgagtgatgggggctccttggggcagg

SEQ ID NO: 34476 - DNA, 28 bp, synthetic construct
  source 1..28: mol_type = other DNA
tgagtgatgggggctccttggggcaggg

SEQ ID NO: 34477 - DNA, 28 bp, synthetic construct
  source 1..28: mol_type = other DNA
gggctccttggggcagggatcccctcgg

SEQ ID NO: 34478 - DNA, 28 bp, synthetic construct
  source 1..28: mol_type = other DNA
ctccttggggcagggatcccctcggagg

SEQ ID NO: 34479 - DNA, 28 bp, synthetic construct
  source 1..28: mol_type = other DNA
tccttggggcagggatcccctcggaggg

SEQ ID NO: 34480 - DNA, 28 bp, synthetic construct
  source 1..28: mol_type = other DNA
ccttggggcagggatcccctcggagggg

SEQ ID NO: 34481 - DNA, 28 bp, synthetic construct
  source 1..28: mol_type = other DNA
ggggcagggatcccctcggaggggctgg

SEQ ID NO: 34482 - DNA, 28 bp, synthetic construct
  source 1..28: mol_type = other DNA
gggcagggatcccctcggaggggctggg

SEQ ID NO: 34483 - DNA, 28 bp, synthetic construct
  source 1..28: mol_type = other DNA
ggcagggatcccctcggaggggctgggg

SEQ ID NO: 34484 - DNA, 28 bp, synthetic construct
  source 1..28: mol_type = other DNA
gggatcccctcggaggggctggggcagg

SEQ ID NO: 34485 - DNA, 28 bp, synthetic construct
  source 1..28: mol_type = other DNA
ggatcccctcggaggggctggggcaggg

SEQ ID NO: 34486 - DNA, 28 bp, synthetic construct
  source 1..28: mol_type = other DNA
gatcccctcggaggggctggggcagggg

SEQ ID NO: 34487 - DNA, 28 bp, synthetic construct
  source 1..28: mol_type = other DNA
ctacccctgccccagcccctccgagggg

SEQ ID NO: 34488 - DNA, 28 bp, synthetic construct
  source 1..28: mol_type = other DNA
cctacccctgccccagcccctccgaggg

SEQ ID NO: 34489 - DNA, 28 bp, synthetic construct
  source 1..28: mol_type = other DNA
tcctacccctgccccagcccctccgagg

SEQ ID NO: 34490 - DNA, 28 bp, synthetic construct
  source 1..28: mol_type = other DNA
tcggaggggctggggcaggggtaggagg

SEQ ID NO: 34491 - DNA, 28 bp, synthetic construct
  source 1..28: mol_type = other DNA
gaggggctggggcaggggtaggaggtgg

SEQ ID NO: 34492 - DNA, 28 bp, synthetic construct
  source 1..28: mol_type = other DNA
aggggctggggcaggggtaggaggtggg

SEQ ID NO: 34493 - DNA, 28 bp, synthetic construct
  source 1..28: mol_type = other DNA
ggggctggggcaggggtaggaggtgggg

SEQ ID NO: 34494 - DNA, 28 bp, synthetic construct
  source 1..28: mol_type = other DNA
gggctggggcaggggtaggaggtggggg

SEQ ID NO: 34495 - DNA, 28 bp, synthetic construct
  source 1..28: mol_type = other DNA
ggcaggggtaggaggtgggggatgatgg

SEQ ID NO: 34496 - DNA, 28 bp, synthetic construct
  source 1..28: mol_type = other DNA
ggggtaggaggtgggggatgatggcagg

SEQ ID NO: 34497 - DNA, 28 bp, synthetic construct
  source 1..28: mol_type = other DNA
aggaggtgggggatgatggcaggtgtgg

SEQ ID NO: 34498 - DNA, 28 bp, synthetic construct
  source 1..28: mol_type = other DNA
ggaggtgggggatgatggcaggtgtggg

SEQ ID NO: 34499 - DNA, 28 bp, synthetic construct
  source 1..28: mol_type = other DNA
gaggtgggggatgatggcaggtgtgggg

SEQ ID NO: 34500 - DNA, 28 bp, synthetic construct
  source 1..28: mol_type = other DNA
aggtgggggatgatggcaggtgtggggg

SEQ ID NO: 34501 - DNA, 28 bp, synthetic construct
  source 1..28: mol_type = other DNA
ggtgggggatgatggcaggtgtgggggg

SEQ ID NO: 34502 - DNA, 28 bp, synthetic construct
  source 1..28: mol_type = other DNA
gggatgatggcaggtgtggggggcctgg

SEQ ID NO: 34503 - DNA, 28 bp, synthetic construct
  source 1..28: mol_type = other DNA
ggatgatggcaggtgtggggggcctggg

SEQ ID NO: 34504 - DNA, 28 bp, synthetic construct
  source 1..28: mol_type = other DNA
gatggcaggtgtggggggcctgggctgg

SEQ ID NO: 34505 - DNA, 28 bp, synthetic construct
  source 1..28: mol_type = other DNA
aggtgtggggggcctgggctggcttagg

SEQ ID NO: 34506 - DNA, 28 bp, synthetic construct
  source 1..28: mol_type = other DNA
ggtgtggggggcctgggctggcttaggg

SEQ ID NO: 34507 - DNA, 28 bp, synthetic construct
  source 1..28: mol_type = other DNA
cctgggctggcttagggagtttccttgg

SEQ ID NO: 34508 - DNA, 28 bp, synthetic construct
  source 1..28: mol_type = other DNA
ctgggctggcttagggagtttccttggg

SEQ ID NO: 34509 - DNA, 28 bp, synthetic construct
  source 1..28: mol_type = other DNA
caactatgtcggcctaagggcctggcgg

SEQ ID NO: 34510 - DNA, 28 bp, synthetic construct
  source 1..28: mol_type = other DNA
aactatgtcggcctaagggcctggcggg

SEQ ID NO: 34511 - DNA, 28 bp, synthetic construct
  source 1..28: mol_type = other DNA
actatgtcggcctaagggcctggcgggg

SEQ ID NO: 34512 - DNA, 28 bp, synthetic construct
  source 1..28: mol_type = other DNA
tcggcctaagggcctggcggggtcctgg

SEQ ID NO: 34513 - DNA, 28 bp, synthetic construct
  source 1..28: mol_type = other DNA
gcggccaggaccccgccaggcccttagg

SEQ ID NO: 34514 - DNA, 28 bp, synthetic construct
  source 1..28: mol_type = other DNA
aagggcctggcggggtcctggccgccgg

SEQ ID NO: 34515 - DNA, 28 bp, synthetic construct
  source 1..28: mol_type = other DNA
ggcctggcggggtcctggccgccggtgg

SEQ ID NO: 34516 - DNA, 28 bp, synthetic construct
  source 1..28: mol_type = other DNA
gcctggcggggtcctggccgccggtggg

SEQ ID NO: 34517 - DNA, 28 bp, synthetic construct
  source 1..28: mol_type = other DNA
gcccaccggcggccaggaccccgccagg

SEQ ID NO: 34518 - DNA, 28 bp, synthetic construct
  source 1..28: mol_type = other DNA
ggcggggtcctggccgccggtgggcagg

SEQ ID NO: 34519 - DNA, 28 bp, synthetic construct
  source 1..28: mol_type = other DNA
ggtcctggccgccggtgggcaggcaagg

SEQ ID NO: 34520 - DNA, 28 bp, synthetic construct
  source 1..28: mol_type = other DNA
tgtccttgcctgcccaccggcggccagg

SEQ ID NO: 34521 - DNA, 28 bp, synthetic construct
  source 1..28: mol_type = other DNA
tggccgccggtgggcaggcaaggacagg

SEQ ID NO: 34522 - DNA, 28 bp, synthetic construct
  source 1..28: mol_type = other DNA
ggccgccggtgggcaggcaaggacaggg

SEQ ID NO: 34523 - DNA, 28 bp, synthetic construct
  source 1..28: mol_type = other DNA
caccctgtccttgcctgcccaccggcgg

SEQ ID NO: 34524 - DNA, 28 bp, synthetic construct
  source 1..28: mol_type = other DNA
cgccggtgggcaggcaaggacagggtgg

SEQ ID NO: 34525 - DNA, 28 bp, synthetic construct
  source 1..28: mol_type = other DNA
ttccaccctgtccttgcctgcccaccgg

SEQ ID NO: 34526 - DNA, 28 bp, synthetic construct
  source 1..28: mol_type = other DNA
ggcaggcaaggacagggtggaactgagg

SEQ ID NO: 34527 - DNA, 28 bp, synthetic construct
  source 1..28: mol_type = other DNA
gcaggcaaggacagggtggaactgaggg

SEQ ID NO: 34528 - DNA, 28 bp, synthetic construct
  source 1..28: mol_type = other DNA
gcaaggacagggtggaactgagggccgg

SEQ ID NO: 34529 - DNA, 28 bp, synthetic construct
  source 1..28: mol_type = other DNA
ggacagggtggaactgagggccggaagg

SEQ ID NO: 34530 - DNA, 28 bp, synthetic construct
  source 1..28: mol_type = other DNA
ggtggaactgagggccggaaggagctgg

SEQ ID NO: 34531 - DNA, 28 bp, synthetic construct
  source 1..28: mol_type = other DNA
gtggaactgagggccggaaggagctggg

SEQ ID NO: 34532 - DNA, 28 bp, synthetic construct
  source 1..28: mol_type = other DNA
tggaactgagggccggaaggagctgggg

SEQ ID NO: 34533 - DNA, 28 bp, synthetic construct
  source 1..28: mol_type = other DNA
ggaactgagggccggaaggagctggggg

SEQ ID NO: 34534 - DNA, 28 bp, synthetic construct
  source 1..28: mol_type = other DNA
gaactgagggccggaaggagctgggggg

SEQ ID NO: 34535 - DNA, 28 bp, synthetic construct
  source 1..28: mol_type = other DNA
agcttaggaaccccccagctccttccgg

SEQ ID NO: 34536 - DNA, 28 bp, synthetic construct
  source 1..28: mol_type = other DNA
gaggggagatgggaagagttagcttagg

SEQ ID NO: 34537 - DNA, 28 bp, synthetic construct
  source 1..28: mol_type = other DNA
agctaactcttcccatctcccctccagg

SEQ ID NO: 34538 - DNA, 28 bp, synthetic construct
  source 1..28: mol_type = other DNA
cttcccatctcccctccaggcacgcagg

SEQ ID NO: 34539 - DNA, 28 bp, synthetic construct
  source 1..28: mol_type = other DNA
cagcctgcgtgcctggaggggagatggg

SEQ ID NO: 34540 - DNA, 28 bp, synthetic construct
  source 1..28: mol_type = other DNA
tcagcctgcgtgcctggaggggagatgg

SEQ ID NO: 34541 - DNA, 28 bp, synthetic construct
  source 1..28: mol_type = other DNA
ctttcttcagcctgcgtgcctggagggg

SEQ ID NO: 34542 - DNA, 28 bp, synthetic construct
  source 1..28: mol_type = other DNA
actttcttcagcctgcgtgcctggaggg

SEQ ID NO: 34543 - DNA, 28 bp, synthetic construct
  source 1..28: mol_type = other DNA
gactttcttcagcctgcgtgcctggagg

SEQ ID NO: 34544 - DNA, 28 bp, synthetic construct
  source 1..28: mol_type = other DNA
agggactttcttcagcctgcgtgcctgg

SEQ ID NO: 34545 - DNA, 28 bp, synthetic construct
  source 1..28: mol_type = other DNA
acgcaggctgaagaaagtcccttcgtgg

SEQ ID NO: 34546 - DNA, 28 bp, synthetic construct
  source 1..28: mol_type = other DNA
cgcaggctgaagaaagtcccttcgtggg

SEQ ID NO: 34547 - DNA, 28 bp, synthetic construct
  source 1..28: mol_type = other DNA
aagaaagtcccttcgtgggcaacccagg

SEQ ID NO: 34548 - DNA, 28 bp, synthetic construct
  source 1..28: mol_type = other DNA
agaaagtcccttcgtgggcaacccaggg

SEQ ID NO: 34549 - DNA, 28 bp, synthetic construct
  source 1..28: mol_type = other DNA
tgatattccctgggttgcccacgaaggg

SEQ ID NO: 34550 - DNA, 28 bp, synthetic construct
  source 1..28: mol_type = other DNA
gtgatattccctgggttgcccacgaagg

SEQ ID NO: 34551 - DNA, 28 bp, synthetic construct
  source 1..28: mol_type = other DNA
tcgtgggcaacccagggaatatcacagg

SEQ ID NO: 34552 - DNA, 28 bp, synthetic construct
  source 1..28: mol_type = other DNA
caacccagggaatatcacaggtgcccgg

SEQ ID NO: 34553 - DNA, 28 bp, synthetic construct
  source 1..28: mol_type = other DNA
aacccagggaatatcacaggtgcccggg

SEQ ID NO: 34554 - DNA, 28 bp, synthetic construct
  source 1..28: mol_type = other DNA
acccagggaatatcacaggtgcccgggg

SEQ ID NO: 34555 - DNA, 28 bp, synthetic construct
  source 1..28: mol_type = other DNA
tccccgggcacctgtgatattccctggg

SEQ ID NO: 34556 - DNA, 28 bp, synthetic construct
  source 1..28: mol_type = other DNA
gtccccgggcacctgtgatattccctgg

SEQ ID NO: 34557 - DNA, 28 bp, synthetic construct
  source 1..28: mol_type = other DNA
aatatcacaggtgcccggggactcacgg

SEQ ID NO: 34558 - DNA, 28 bp, synthetic construct
  source 1..28: mol_type = other DNA
atatcacaggtgcccggggactcacggg

SEQ ID NO: 34559 - DNA, 28 bp, synthetic construct
  source 1..28: mol_type = other DNA
tgcccggggactcacgggcacccttcgg

SEQ ID NO: 34560 - DNA, 28 bp, synthetic construct
  source 1..28: mol_type = other DNA
caccgaagggtgcccgtgagtccccggg

SEQ ID NO: 34561 - DNA, 28 bp, synthetic construct
  source 1..28: mol_type = other DNA
acaccgaagggtgcccgtgagtccccgg

SEQ ID NO: 34562 - DNA, 28 bp, synthetic construct
  source 1..28: mol_type = other DNA
acgggcacccttcggtgtcagctccagg

SEQ ID NO: 34563 - DNA, 28 bp, synthetic construct
  source 1..28: mol_type = other DNA
acccttcggtgtcagctccaggttcagg

SEQ ID NO: 34564 - DNA, 28 bp, synthetic construct
  source 1..28: mol_type = other DNA
cccttcggtgtcagctccaggttcaggg

SEQ ID NO: 34565 - DNA, 28 bp, synthetic construct
  source 1..28: mol_type = other DNA
tccctgaacctggagctgacaccgaagg

SEQ ID NO: 34566 - DNA, 28 bp, synthetic construct
  source 1..28: mol_type = other DNA
ctccaggttcagggagagccccccgagg

SEQ ID NO: 34567 - DNA, 28 bp, synthetic construct
  source 1..28: mol_type = other DNA
tacctcggggggctctccctgaacctgg

SEQ ID NO: 34568 - DNA, 28 bp, synthetic construct
  source 1..28: mol_type = other DNA
tcagggagagccccccgaggtacattgg

SEQ ID NO: 34569 - DNA, 28 bp, synthetic construct
  source 1..28: mol_type = other DNA
agagccccccgaggtacattggcttcgg

SEQ ID NO: 34570 - DNA, 28 bp, synthetic construct
  source 1..28: mol_type = other DNA
gagccccccgaggtacattggcttcggg

SEQ ID NO: 34571 - DNA, 28 bp, synthetic construct
  source 1..28: mol_type = other DNA
catcccgaagccaatgtacctcgggggg

SEQ ID NO: 34572 - DNA, 28 bp, synthetic construct
  source 1..28: mol_type = other DNA
cccccgaggtacattggcttcgggatgg

SEQ ID NO: 34573 - DNA, 28 bp, synthetic construct
  source 1..28: mol_type = other DNA
tccatcccgaagccaatgtacctcgggg

SEQ ID NO: 34574 - DNA, 28 bp, synthetic construct
  source 1..28: mol_type = other DNA
gtccatcccgaagccaatgtacctcggg

SEQ ID NO: 34575 - DNA, 28 bp, synthetic construct
  source 1..28: mol_type = other DNA
tgtccatcccgaagccaatgtacctcgg

SEQ ID NO: 34576 - DNA, 28 bp, synthetic construct
  source 1..28: mol_type = other DNA
cattggcttcgggatggacagatcctgg

SEQ ID NO: 34577 - DNA, 28 bp, synthetic construct
  source 1..28: mol_type = other DNA
cgggatggacagatcctggagctcgcgg

SEQ ID NO: 34578 - DNA, 28 bp, synthetic construct
  source 1..28: mol_type = other DNA
ggtctgggtgctgtccgcgagctccagg

SEQ ID NO: 34579 - DNA, 28 bp, synthetic construct
  source 1..28: mol_type = other DNA
gagctcgcggacagcacccagacccagg

SEQ ID NO: 34580 - DNA, 28 bp, synthetic construct
  source 1..28: mol_type = other DNA
gacagcacccagacccaggtgcccctgg

SEQ ID NO: 34581 - DNA, 28 bp, synthetic construct
  source 1..28: mol_type = other DNA
acagcacccagacccaggtgcccctggg

SEQ ID NO: 34582 - DNA, 28 bp, synthetic construct
  source 1..28: mol_type = other DNA
acccagacccaggtgcccctgggtgagg

SEQ ID NO: 34583 - DNA, 28 bp, synthetic construct
  source 1..28: mol_type = other DNA
tcctcacccaggggcacctgggtctggg

SEQ ID NO: 34584 - DNA, 28 bp, synthetic construct
  source 1..28: mol_type = other DNA
atcctcacccaggggcacctgggtctgg

SEQ ID NO: 34585 - DNA, 28 bp, synthetic construct
  source 1..28: mol_type = other DNA
tgttcatcctcacccaggggcacctggg

SEQ ID NO: 34586 - DNA, 28 bp, synthetic construct
  source 1..28: mol_type = other DNA
ctgttcatcctcacccaggggcacctgg

SEQ ID NO: 34587 - DNA, 28 bp, synthetic construct
  source 1..28: mol_type = other DNA
caggtgcccctgggtgaggatgaacagg

SEQ ID NO: 34588 - DNA, 28 bp, synthetic construct
  source 1..28: mol_type = other DNA
agtcatcctgttcatcctcacccagggg

SEQ ID NO: 34589 - DNA, 28 bp, synthetic construct
  source 1..28: mol_type = other DNA
cagtcatcctgttcatcctcacccaggg

SEQ ID NO: 34590 - DNA, 28 bp, synthetic construct
  source 1..28: mol_type = other DNA
cctgggtgaggatgaacaggatgactgg

SEQ ID NO: 34591 - DNA, 28 bp, synthetic construct
  source 1..28: mol_type = other DNA
gaggatgaacaggatgactggatagtgg

SEQ ID NO: 34592 - DNA, 28 bp, synthetic construct
  source 1..28: mol_type = other DNA
tgactggatagtggtcagccagctcagg

SEQ ID NO: 34593 - DNA, 28 bp, synthetic construct
  source 1..28: mol_type = other DNA
atagtggtcagccagctcaggtgtgtgg

SEQ ID NO: 34594 - DNA, 28 bp, synthetic construct
  source 1..28: mol_type = other DNA
cggggatgtggccacacacctgagctgg

SEQ ID NO: 34595 - DNA, 28 bp, synthetic construct
  source 1..28: mol_type = other DNA
gaggtgggagtgggattcggggatgtgg

SEQ ID NO: 34596 - DNA, 28 bp, synthetic construct
  source 1..28: mol_type = other DNA
gtgacggaggtgggagtgggattcgggg

SEQ ID NO: 34597 - DNA, 28 bp, synthetic construct
  source 1..28: mol_type = other DNA
tgtgacggaggtgggagtgggattcggg

SEQ ID NO: 34598 - DNA, 28 bp, synthetic construct
  source 1..28: mol_type = other DNA
gtgtgacggaggtgggagtgggattcgg

SEQ ID NO: 34599 - DNA, 28 bp, synthetic construct
  source 1..28: mol_type = other DNA
tcccactcccacctccgtcacacagagg

SEQ ID NO: 34600 - DNA, 28 bp, synthetic construct
  source 1..28: mol_type = other DNA
cccactcccacctccgtcacacagaggg

SEQ ID NO: 34601 - DNA, 28 bp, synthetic construct
  source 1..28: mol_type = other DNA
gccctctgtgtgacggaggtgggagtgg

SEQ ID NO: 34602 - DNA, 28 bp, synthetic construct
  source 1..28: mol_type = other DNA
tttctgccctctgtgtgacggaggtggg

SEQ ID NO: 34603 - DNA, 28 bp, synthetic construct
  source 1..28: mol_type = other DNA
ctttctgccctctgtgtgacggaggtgg

SEQ ID NO: 34604 - DNA, 28 bp, synthetic construct
  source 1..28: mol_type = other DNA
gggctttctgccctctgtgtgacggagg

SEQ ID NO: 34605 - DNA, 28 bp, synthetic construct
  source 1..28: mol_type = other DNA
ggtgggctttctgccctctgtgtgacgg

SEQ ID NO: 34606 - DNA, 28 bp, synthetic construct
  source 1..28: mol_type = other DNA
tcacacagagggcagaaagcccacctgg

SEQ ID NO: 34607 - DNA, 28 bp, synthetic construct
  source 1..28: mol_type = other DNA
cacacagagggcagaaagcccacctggg

SEQ ID NO: 34608 - DNA, 28 bp, synthetic construct
  source 1..28: mol_type = other DNA
acagagggcagaaagcccacctgggtgg

SEQ ID NO: 34609 - DNA, 28 bp, synthetic construct
  source 1..28: mol_type = other DNA
cagagggcagaaagcccacctgggtggg

SEQ ID NO: 34610 - DNA, 28 bp, synthetic construct
  source 1..28: mol_type = other DNA
gtcaaactggggttcccacccaggtggg

SEQ ID NO: 34611 - DNA, 28 bp, synthetic construct
  source 1..28: mol_type = other DNA
ggtcaaactggggttcccacccaggtgg

SEQ ID NO: 34612 - DNA, 28 bp, synthetic construct
  source 1..28: mol_type = other DNA
agtggtcaaactggggttcccacccagg

SEQ ID NO: 34613 - DNA, 28 bp, synthetic construct
  source 1..28: mol_type = other DNA
gcacggctgacaagtggtcaaactgggg

SEQ ID NO: 34614 - DNA, 28 bp, synthetic construct
  source 1..28: mol_type = other DNA
cgcacggctgacaagtggtcaaactggg

SEQ ID NO: 34615 - DNA, 28 bp, synthetic construct
  source 1..28: mol_type = other DNA
ccagtttgaccacttgtcagccgtgcgg

SEQ ID NO: 34616 - DNA, 28 bp, synthetic construct
  source 1..28: mol_type = other DNA
tgctcaaagccgcacggctgacaagtgg

SEQ ID NO: 34617 - DNA, 28 bp, synthetic construct
  source 1..28: mol_type = other DNA
cagccgtgcggctttgagcatgtgatgg

SEQ ID NO: 34618 - DNA, 28 bp, synthetic construct
  source 1..28: mol_type = other DNA
gttccatcacatgctcaaagccgcacgg

SEQ ID NO: 34619 - DNA, 28 bp, synthetic construct
  source 1..28: mol_type = other DNA
tcgtggttgtcatgagcttccagactgg

SEQ ID NO: 34620 - DNA, 28 bp, synthetic construct
  source 1..28: mol_type = other DNA
cagaacggaaagagggtgtccagtctgg

SEQ ID NO: 34621 - DNA, 28 bp, synthetic construct
  source 1..28: mol_type = other DNA
gagggggtctgtcagaacggaaagaggg

SEQ ID NO: 34622 - DNA, 28 bp, synthetic construct
  source 1..28: mol_type = other DNA
ggagggggtctgtcagaacggaaagagg

SEQ ID NO: 34623 - DNA, 28 bp, synthetic construct
  source 1..28: mol_type = other DNA
gacactgggagggggtctgtcagaacgg

SEQ ID NO: 34624 - DNA, 28 bp, synthetic construct
  source 1..28: mol_type = other DNA
agggtcagagctggacactgggaggggg

SEQ ID NO: 34625 - DNA, 28 bp, synthetic construct
  source 1..28: mol_type = other DNA
cagggtcagagctggacactgggagggg

SEQ ID NO: 34626 - DNA, 28 bp, synthetic construct
  source 1..28: mol_type = other DNA
tcagggtcagagctggacactgggaggg

SEQ ID NO: 34627 - DNA, 28 bp, synthetic construct
  source 1..28: mol_type = other DNA
ttcagggtcagagctggacactgggagg

SEQ ID NO: 34628 - DNA, 28 bp, synthetic construct
  source 1..28: mol_type = other DNA
aggttcagggtcagagctggacactggg

SEQ ID NO: 34629 - DNA, 28 bp, synthetic construct
  source 1..28: mol_type = other DNA
gaggttcagggtcagagctggacactgg

SEQ ID NO: 34630 - DNA, 28 bp, synthetic construct
  source 1..28: mol_type = other DNA
agacagagaggttcagggtcagagctgg

SEQ ID NO: 34631 - DNA, 28 bp, synthetic construct
  source 1..28: mol_type = other DNA
gcaagaggagagacagagaggttcaggg

SEQ ID NO: 34632 - DNA, 28 bp, synthetic construct
  source 1..28: mol_type = other DNA
ggcaagaggagagacagagaggttcagg

SEQ ID NO: 34633 - DNA, 28 bp, synthetic construct
  source 1..28: mol_type = other DNA
tgacagggcaagaggagagacagagagg

SEQ ID NO: 34634 - DNA, 28 bp, synthetic construct
  source 1..28: mol_type = other DNA
agggaggtgattctgacagggcaagagg

SEQ ID NO: 34635 - DNA, 28 bp, synthetic construct
  source 1..28: mol_type = other DNA
aagctgcagggaggtgattctgacaggg

SEQ ID NO: 34636 - DNA, 28 bp, synthetic construct
  source 1..28: mol_type = other DNA
aaagctgcagggaggtgattctgacagg

SEQ ID NO: 34637 - DNA, 28 bp, synthetic construct
  source 1..28: mol_type = other DNA
atcacctccctgcagctttccgacacgg

SEQ ID NO: 34638 - DNA, 28 bp, synthetic construct
  source 1..28: mol_type = other DNA
tcacctccctgcagctttccgacacggg

SEQ ID NO: 34639 - DNA, 28 bp, synthetic construct
  source 1..28: mol_type = other DNA
tgtcccgtgtcggaaagctgcagggagg

SEQ ID NO: 34640 - DNA, 28 bp, synthetic construct
  source 1..28: mol_type = other DNA
tactgtcccgtgtcggaaagctgcaggg

SEQ ID NO: 34641 - DNA, 28 bp, synthetic construct
  source 1..28: mol_type = other DNA
gtactgtcccgtgtcggaaagctgcagg

SEQ ID NO: 34642 - DNA, 28 bp, synthetic construct
  source 1..28: mol_type = other DNA
tccgacacgggacagtaccagtgtttgg

SEQ ID NO: 34643 - DNA, 28 bp, synthetic construct
  source 1..28: mol_type = other DNA
accaaacactggtactgtcccgtgtcgg

SEQ ID NO: 34644 - DNA, 28 bp, synthetic construct
  source 1..28: mol_type = other DNA
ggacagtaccagtgtttggtgtttctgg

SEQ ID NO: 34645 - DNA, 28 bp, synthetic construct
  source 1..28: mol_type = other DNA
gacagtaccagtgtttggtgtttctggg

SEQ ID NO: 34646 - DNA, 28 bp, synthetic construct
  source 1..28: mol_type = other DNA
ctgatgtcccagaaacaccaaacactgg

SEQ ID NO: 34647 - DNA, 28 bp, synthetic construct
  source 1..28: mol_type = other DNA
gacatcagaccttcgtgtcccagcctgg

SEQ ID NO: 34648 - DNA, 28 bp, synthetic construct
  source 1..28: mol_type = other DNA
ccaacatagccaggctgggacacgaagg

SEQ ID NO: 34649 - DNA, 28 bp, synthetic construct
  source 1..28: mol_type = other DNA
cttcgtgtcccagcctggctatgttggg

SEQ ID NO: 34650 - DNA, 28 bp, synthetic construct
  source 1..28: mol_type = other DNA
gtgtcccagcctggctatgttgggctgg

SEQ ID NO: 34651 - DNA, 28 bp, synthetic construct
  source 1..28: mol_type = other DNA
tcccagcctggctatgttgggctggagg

SEQ ID NO: 34652 - DNA, 28 bp, synthetic construct
  source 1..28: mol_type = other DNA
ccctccagcccaacatagccaggctggg

SEQ ID NO: 34653 - DNA, 28 bp, synthetic construct
  source 1..28: mol_type = other DNA
accctccagcccaacatagccaggctgg

SEQ ID NO: 34654 - DNA, 28 bp, synthetic construct
  source 1..28: mol_type = other DNA
gctcaccctccagcccaacatagccagg

SEQ ID NO: 34655 - DNA, 28 bp, synthetic construct
  source 1..28: mol_type = other DNA
ctatgttgggctggagggtgagctctgg

SEQ ID NO: 34656 - DNA, 28 bp, synthetic construct
  source 1..28: mol_type = other DNA
tatgttgggctggagggtgagctctggg

SEQ ID NO: 34657 - DNA, 28 bp, synthetic construct
  source 1..28: mol_type = other DNA
atgttgggctggagggtgagctctgggg

SEQ ID NO: 34658 - DNA, 28 bp, synthetic construct
  source 1..28: mol_type = other DNA
gggctggagggtgagctctggggtcagg

SEQ ID NO: 34659 - DNA, 28 bp, synthetic construct
  source 1..28: mol_type = other DNA
ggctggagggtgagctctggggtcaggg

SEQ ID NO: 34660 - DNA, 28 bp, synthetic construct
  source 1..28: mol_type = other DNA
gctggagggtgagctctggggtcagggg

SEQ ID NO: 34661 - DNA, 28 bp, synthetic construct
  source 1..28: mol_type = other DNA
gtgagctctggggtcaggggtcctgagg

SEQ ID NO: 34662 - DNA, 28 bp, synthetic construct
  source 1..28: mol_type = other DNA
tgagctctggggtcaggggtcctgaggg

SEQ ID NO: 34663 - DNA, 28 bp, synthetic construct
  source 1..28: mol_type = other DNA
gagctctggggtcaggggtcctgagggg

SEQ ID NO: 34664 - DNA, 28 bp, synthetic construct
  source 1..28: mol_type = other DNA
ggggtcaggggtcctgaggggtcagagg

SEQ ID NO: 34665 - DNA, 28 bp, synthetic construct
  source 1..28: mol_type = other DNA
gggtcctgaggggtcagaggacatgtgg

SEQ ID NO: 34666 - DNA, 28 bp, synthetic construct
  source 1..28: mol_type = other DNA
agcgccacatgtcctctgacccctcagg

SEQ ID NO: 34667 - DNA, 28 bp, synthetic construct
  source 1..28: mol_type = other DNA
gggtcagaggacatgtggcgctcatagg

SEQ ID NO: 34668 - DNA, 28 bp, synthetic construct
  source 1..28: mol_type = other DNA
gaggacatgtggcgctcataggttgtgg

SEQ ID NO: 34669 - DNA, 28 bp, synthetic construct
  source 1..28: mol_type = other DNA
aggacatgtggcgctcataggttgtggg

SEQ ID NO: 34670 - DNA, 28 bp, synthetic construct
  source 1..28: mol_type = other DNA
tggcgctcataggttgtgggaagtcagg

SEQ ID NO: 34671 - DNA, 28 bp, synthetic construct
  source 1..28: mol_type = other DNA
aggttgtgggaagtcaggaatcctgagg

SEQ ID NO: 34672 - DNA, 28 bp, synthetic construct
  source 1..28: mol_type = other DNA
ggttgtgggaagtcaggaatcctgaggg

SEQ ID NO: 34673 - DNA, 28 bp, synthetic construct
  source 1..28: mol_type = other DNA
gttgtgggaagtcaggaatcctgagggg

SEQ ID NO: 34674 - DNA, 28 bp, synthetic construct
  source 1..28: mol_type = other DNA
ggaagtcaggaatcctgaggggtcaagg

SEQ ID NO: 34675 - DNA, 28 bp, synthetic construct
  source 1..28: mol_type = other DNA
aggaatcctgaggggtcaaggtcaaagg

SEQ ID NO: 34676 - DNA, 28 bp, synthetic construct
  source 1..28: mol_type = other DNA
ggaatcctgaggggtcaaggtcaaaggg

SEQ ID NO: 34677 - DNA, 28 bp, synthetic construct
  source 1..28: mol_type = other DNA
cagcaccctttgaccttgacccctcagg

SEQ ID NO: 34678 - DNA, 28 bp, synthetic construct
  source 1..28: mol_type = other DNA
ctgaggggtcaaggtcaaagggtgctgg

SEQ ID NO: 34679 - DNA, 28 bp, synthetic construct
  source 1..28: mol_type = other DNA
aggggtcaaggtcaaagggtgctggagg

SEQ ID NO: 34680 - DNA, 28 bp, synthetic construct
  source 1..28: mol_type = other DNA
aaggtcaaagggtgctggaggattcagg

SEQ ID NO: 34681 - DNA, 28 bp, synthetic construct
  source 1..28: mol_type = other DNA
agataaggcaagtcaatgaccctgcagg

SEQ ID NO: 34682 - DNA, 28 bp, synthetic construct
  source 1..28: mol_type = other DNA
gataaggcaagtcaatgaccctgcaggg

SEQ ID NO: 34683 - DNA, 28 bp, synthetic construct
  source 1..28: mol_type = other DNA
aaggcaagtcaatgaccctgcagggtgg

SEQ ID NO: 34684 - DNA, 28 bp, synthetic construct
  source 1..28: mol_type = other DNA
aggcaagtcaatgaccctgcagggtggg

SEQ ID NO: 34685 - DNA, 28 bp, synthetic construct
  source 1..28: mol_type = other DNA
ctttgggcagcaaacccaccctgcaggg

SEQ ID NO: 34686 - DNA, 28 bp, synthetic construct
  source 1..28: mol_type = other DNA
gctttgggcagcaaacccaccctgcagg

SEQ ID NO: 34687 - DNA, 28 bp, synthetic construct
  source 1..28: mol_type = other DNA
ctgcccaaagcctacagcatcctagtgg

SEQ ID NO: 34688 - DNA, 28 bp, synthetic construct
  source 1..28: mol_type = other DNA
tcaccactaggatgctgtaggctttggg

SEQ ID NO: 34689 - DNA, 28 bp, synthetic construct
  source 1..28: mol_type = other DNA
ctcaccactaggatgctgtaggctttgg

SEQ ID NO: 34690 - DNA, 28 bp, synthetic construct
  source 1..28: mol_type = other DNA
gcctacagcatcctagtggtgagtcagg

SEQ ID NO: 34691 - DNA, 28 bp, synthetic construct
  source 1..28: mol_type = other DNA
gcctgactcaccactaggatgctgtagg

SEQ ID NO: 34692 - DNA, 28 bp, synthetic construct
  source 1..28: mol_type = other DNA
catcctagtggtgagtcaggcatcttgg

SEQ ID NO: 34693 - DNA, 28 bp, synthetic construct
  source 1..28: mol_type = other DNA
atcctagtggtgagtcaggcatcttggg

SEQ ID NO: 34694 - DNA, 28 bp, synthetic construct
  source 1..28: mol_type = other DNA
tcctagtggtgagtcaggcatcttgggg

SEQ ID NO: 34695 - DNA, 28 bp, synthetic construct
  source 1..28: mol_type = other DNA
gccccaagatgcctgactcaccactagg

SEQ ID NO: 34696 - DNA, 28 bp, synthetic construct
  source 1..28: mol_type = other DNA
tgagtcaggcatcttggggcctcagagg

SEQ ID NO: 34697 - DNA, 28 bp, synthetic construct
  source 1..28: mol_type = other DNA
gagtcaggcatcttggggcctcagaggg

SEQ ID NO: 34698 - DNA, 28 bp, synthetic construct
  source 1..28: mol_type = other DNA
agtggtagaggctggggtccctctgagg

SEQ ID NO: 34699 - DNA, 28 bp, synthetic construct
  source 1..28: mol_type = other DNA
gcggggtgggcagtggtagaggctgggg

SEQ ID NO: 34700 - DNA, 28 bp, synthetic construct
  source 1..28: mol_type = other DNA
agcggggtgggcagtggtagaggctggg

SEQ ID NO: 34701 - DNA, 28 bp, synthetic construct
  source 1..28: mol_type = other DNA
tagcggggtgggcagtggtagaggctgg

SEQ ID NO: 34702 - DNA, 28 bp, synthetic construct
  source 1..28: mol_type = other DNA
agcctctaccactgcccaccccgctagg

SEQ ID NO: 34703 - DNA, 28 bp, synthetic construct
  source 1..28: mol_type = other DNA
agcctagcggggtgggcagtggtagagg

SEQ ID NO: 34704 - DNA, 28 bp, synthetic construct
  source 1..28: mol_type = other DNA
aaggcaagcctagcggggtgggcagtgg

SEQ ID NO: 34705 - DNA, 28 bp, synthetic construct
  source 1..28: mol_type = other DNA
ggaagtaaggcaagcctagcggggtggg

SEQ ID NO: 34706 - DNA, 28 bp, synthetic construct
  source 1..28: mol_type = other DNA
aggaagtaaggcaagcctagcggggtgg

SEQ ID NO: 34707 - DNA, 28 bp, synthetic construct
  source 1..28: mol_type = other DNA
accccgctaggcttgccttacttcctgg

SEQ ID NO: 34708 - DNA, 28 bp, synthetic construct
  source 1..28: mol_type = other DNA
tccaggaagtaaggcaagcctagcgggg

SEQ ID NO: 34709 - DNA, 28 bp, synthetic construct
  source 1..28: mol_type = other DNA
ctccaggaagtaaggcaagcctagcggg

SEQ ID NO: 34710 - DNA, 28 bp, synthetic construct
  source 1..28: mol_type = other DNA
cctccaggaagtaaggcaagcctagcgg

SEQ ID NO: 34711 - DNA, 28 bp, synthetic construct
  source 1..28: mol_type = other DNA
tgtcttcgggctcctccaggaagtaagg

SEQ ID NO: 34712 - DNA, 28 bp, synthetic construct
  source 1..28: mol_type = other DNA
ttacttcctggaggagcccgaagacagg

SEQ ID NO: 34713 - DNA, 28 bp, synthetic construct
  source 1..28: mol_type = other DNA
cacagtcctgtcttcgggctcctccagg

SEQ ID NO: 34714 - DNA, 28 bp, synthetic construct
  source 1..28: mol_type = other DNA
ctggaggagcccgaagacaggactgtgg

SEQ ID NO: 34715 - DNA, 28 bp, synthetic construct
  source 1..28: mol_type = other DNA
tgttggcggccacagtcctgtcttcggg

SEQ ID NO: 34716 - DNA, 28 bp, synthetic construct
  source 1..28: mol_type = other DNA
gtgttggcggccacagtcctgtcttcgg

SEQ ID NO: 34717 - DNA, 28 bp, synthetic construct
  source 1..28: mol_type = other DNA
cagctcaggttgaagggggtgttggcgg

SEQ ID NO: 34718 - DNA, 28 bp, synthetic construct
  source 1..28: mol_type = other DNA
tggcagctcaggttgaagggggtgttgg

SEQ ID NO: 34719 - DNA, 28 bp, synthetic construct
  source 1..28: mol_type = other DNA
tgagcttggcagctcaggttgaaggggg

SEQ ID NO: 34720 - DNA, 28 bp, synthetic construct
  source 1..28: mol_type = other DNA
ctgagcttggcagctcaggttgaagggg

SEQ ID NO: 34721 - DNA, 28 bp, synthetic construct
  source 1..28: mol_type = other DNA
cccttcaacctgagctgccaagctcagg

SEQ ID NO: 34722 - DNA, 28 bp, synthetic construct
  source 1..28: mol_type = other DNA
ccctgagcttggcagctcaggttgaagg

SEQ ID NO: 34723 - DNA, 28 bp, synthetic construct
  source 1..28: mol_type = other DNA
tgggggtccctgagcttggcagctcagg

SEQ ID NO: 34724 - DNA, 28 bp, synthetic construct
  source 1..28: mol_type = other DNA
cacgggctctgggggtccctgagcttgg

SEQ ID NO: 34725 - DNA, 28 bp, synthetic construct
  source 1..28: mol_type = other DNA
caagctcagggacccccagagcccgtgg

SEQ ID NO: 34726 - DNA, 28 bp, synthetic construct
  source 1..28: mol_type = other DNA
acccccagagcccgtggacctactctgg

SEQ ID NO: 34727 - DNA, 28 bp, synthetic construct
  source 1..28: mol_type = other DNA
gccagagtaggtccacgggctctggggg

SEQ ID NO: 34728 - DNA, 28 bp, synthetic construct
  source 1..28: mol_type = other DNA
agccagagtaggtccacgggctctgggg

SEQ ID NO: 34729 - DNA, 28 bp, synthetic construct
  source 1..28: mol_type = other DNA
gagccagagtaggtccacgggctctggg

SEQ ID NO: 34730 - DNA, 28 bp, synthetic construct
  source 1..28: mol_type = other DNA
ggagccagagtaggtccacgggctctgg

SEQ ID NO: 34731 - DNA, 28 bp, synthetic construct
  source 1..28: mol_type = other DNA
gagcccgtggacctactctggctccagg

SEQ ID NO: 34732 - DNA, 28 bp, synthetic construct
  source 1..28: mol_type = other DNA
catcctggagccagagtaggtccacggg

SEQ ID NO: 34733 - DNA, 28 bp, synthetic construct
  source 1..28: mol_type = other DNA
gcatcctggagccagagtaggtccacgg

SEQ ID NO: 34734 - DNA, 28 bp, synthetic construct
  source 1..28: mol_type = other DNA
ggggacagcatcctggagccagagtagg

SEQ ID NO: 34735 - DNA, 28 bp, synthetic construct
  source 1..28: mol_type = other DNA
ctctggctccaggatgctgtccccctgg

SEQ ID NO: 34736 - DNA, 28 bp, synthetic construct
  source 1..28: mol_type = other DNA
ctccaggatgctgtccccctggccacgg

SEQ ID NO: 34737 - DNA, 28 bp, synthetic construct
  source 1..28: mol_type = other DNA
agccgtggccagggggacagcatcctgg

SEQ ID NO: 34738 - DNA, 28 bp, synthetic construct
  source 1..28: mol_type = other DNA
atgctgtccccctggccacggctccagg

SEQ ID NO: 34739 - DNA, 28 bp, synthetic construct
  source 1..28: mol_type = other DNA
tccccctggccacggctccaggtcacgg

SEQ ID NO: 34740 - DNA, 28 bp, synthetic construct
  source 1..28: mol_type = other DNA
gccgtgacctggagccgtggccaggggg

SEQ ID NO: 34741 - DNA, 28 bp, synthetic construct
  source 1..28: mol_type = other DNA
ggccgtgacctggagccgtggccagggg

SEQ ID NO: 34742 - DNA, 28 bp, synthetic construct
  source 1..28: mol_type = other DNA
gggccgtgacctggagccgtggccaggg

SEQ ID NO: 34743 - DNA, 28 bp, synthetic construct
  source 1..28: mol_type = other DNA
ggggccgtgacctggagccgtggccagg

SEQ ID NO: 34744 - DNA, 28 bp, synthetic construct
  source 1..28: mol_type = other DNA
cgctgggggccgtgacctggagccgtgg

SEQ ID NO: 34745 - DNA, 28 bp, synthetic construct
  source 1..28: mol_type = other DNA
gcaggctgcgctgggggccgtgacctgg

SEQ ID NO: 34746 - DNA, 28 bp, synthetic construct
  source 1..28: mol_type = other DNA
gcccccagcgcagcctgcatgttccagg

SEQ ID NO: 34747 - DNA, 28 bp, synthetic construct
  source 1..28: mol_type = other DNA
acctggaacatgcaggctgcgctggggg

SEQ ID NO: 34748 - DNA, 28 bp, synthetic construct
  source 1..28: mol_type = other DNA
cacctggaacatgcaggctgcgctgggg

SEQ ID NO: 34749 - DNA, 28 bp, synthetic construct
  source 1..28: mol_type = other DNA
tcacctggaacatgcaggctgcgctggg

SEQ ID NO: 34750 - DNA, 28 bp, synthetic construct
  source 1..28: mol_type = other DNA
ctcacctggaacatgcaggctgcgctgg

SEQ ID NO: 34751 - DNA, 28 bp, synthetic construct
  source 1..28: mol_type = other DNA
gcagcctgcatgttccaggtgagtccgg

SEQ ID NO: 34752 - DNA, 28 bp, synthetic construct
  source 1..28: mol_type = other DNA
cagcctgcatgttccaggtgagtccggg

SEQ ID NO: 34753 - DNA, 28 bp, synthetic construct
  source 1..28: mol_type = other DNA
agcctgcatgttccaggtgagtccgggg

SEQ ID NO: 34754 - DNA, 28 bp, synthetic construct
  source 1..28: mol_type = other DNA
atccccggactcacctggaacatgcagg

SEQ ID NO: 34755 - DNA, 28 bp, synthetic construct
  source 1..28: mol_type = other DNA
catgttccaggtgagtccggggatgtgg

SEQ ID NO: 34756 - DNA, 28 bp, synthetic construct
  source 1..28: mol_type = other DNA
atgttccaggtgagtccggggatgtggg

SEQ ID NO: 34757 - DNA, 28 bp, synthetic construct
  source 1..28: mol_type = other DNA
gctgacccacatccccggactcacctgg

SEQ ID NO: 34758 - DNA, 28 bp, synthetic construct
  source 1..28: mol_type = other DNA
cctattcggagctgacccacatccccgg

SEQ ID NO: 34759 - DNA, 28 bp, synthetic construct
  source 1..28: mol_type = other DNA
cggggatgtgggtcagctccgaataggg

SEQ ID NO: 34760 - DNA, 28 bp, synthetic construct
  source 1..28: mol_type = other DNA
ggggatgtgggtcagctccgaatagggg

SEQ ID NO: 34761 - DNA, 28 bp, synthetic construct
  source 1..28: mol_type = other DNA
gggatgtgggtcagctccgaataggggg

SEQ ID NO: 34762 - DNA, 28 bp, synthetic construct
  source 1..28: mol_type = other DNA
tgtgggtcagctccgaatagggggccgg

SEQ ID NO: 34763 - DNA, 28 bp, synthetic construct
  source 1..28: mol_type = other DNA
gtgggtcagctccgaatagggggccggg

SEQ ID NO: 34764 - DNA, 28 bp, synthetic construct
  source 1..28: mol_type = other DNA
gtcagctccgaatagggggccgggcagg

SEQ ID NO: 34765 - DNA, 28 bp, synthetic construct
  source 1..28: mol_type = other DNA
tcagctccgaatagggggccgggcaggg

SEQ ID NO: 34766 - DNA, 28 bp, synthetic construct
  source 1..28: mol_type = other DNA
cttcagccctgcccggccccctattcgg

SEQ ID NO: 34767 - DNA, 28 bp, synthetic construct
  source 1..28: mol_type = other DNA
tagggggccgggcagggctgaagtcagg

SEQ ID NO: 34768 - DNA, 28 bp, synthetic construct
  source 1..28: mol_type = other DNA
ccgggcagggctgaagtcaggagcaagg

SEQ ID NO: 34769 - DNA, 28 bp, synthetic construct
  source 1..28: mol_type = other DNA
cgggcagggctgaagtcaggagcaaggg

SEQ ID NO: 34770 - DNA, 28 bp, synthetic construct
  source 1..28: mol_type = other DNA
gaaggacagtcagacactcacgcagagg

SEQ ID NO: 34771 - DNA, 28 bp, synthetic construct
  source 1..28: mol_type = other DNA
agagagacagacagtgagggacagaagg

SEQ ID NO: 34772 - DNA, 28 bp, synthetic construct
  source 1..28: mol_type = other DNA
cgaggccggtggatcacttgaggtcagg

SEQ ID NO: 34773 - DNA, 28 bp, synthetic construct
  source 1..28: mol_type = other DNA
ctgacctcaagtgatccaccggcctcgg

SEQ ID NO: 34774 - DNA, 28 bp, synthetic construct
  source 1..28: mol_type = other DNA
gaggccgaggccggtggatcacttgagg

SEQ ID NO: 34775 - DNA, 28 bp, synthetic construct
  source 1..28: mol_type = other DNA
cagtactttgggaggccgaggccggtgg

SEQ ID NO: 34776 - DNA, 28 bp, synthetic construct
  source 1..28: mol_type = other DNA
caccggcctcggcctcccaaagtactgg

SEQ ID NO: 34777 - DNA, 28 bp, synthetic construct
  source 1..28: mol_type = other DNA
accggcctcggcctcccaaagtactggg

SEQ ID NO: 34778 - DNA, 28 bp, synthetic construct
  source 1..28: mol_type = other DNA
tcccagtactttgggaggccgaggccgg

SEQ ID NO: 34779 - DNA, 28 bp, synthetic construct
  source 1..28: mol_type = other DNA
gtaatcccagtactttgggaggccgagg

SEQ ID NO: 34780 - DNA, 28 bp, synthetic construct
  source 1..28: mol_type = other DNA
cggcctcccaaagtactgggattacagg

SEQ ID NO: 34781 - DNA, 28 bp, synthetic construct
  source 1..28: mol_type = other DNA
acgcctgtaatcccagtactttgggagg

SEQ ID NO: 34782 - DNA, 28 bp, synthetic construct
  source 1..28: mol_type = other DNA
ctcacgcctgtaatcccagtactttggg

SEQ ID NO: 34783 - DNA, 28 bp, synthetic construct
  source 1..28: mol_type = other DNA
gctcacgcctgtaatcccagtactttgg

SEQ ID NO: 34784 - DNA, 28 bp, synthetic construct
  source 1..28: mol_type = other DNA
aaaaacacatttgcgctgggtgcggtgg

SEQ ID NO: 34785 - DNA, 28 bp, synthetic construct
  source 1..28: mol_type = other DNA
tacaaaaacacatttgcgctgggtgcgg

SEQ ID NO: 34786 - DNA, 28 bp, synthetic construct
  source 1..28: mol_type = other DNA
actgatacaaaaacacatttgcgctggg

SEQ ID NO: 34787 - DNA, 28 bp, synthetic construct
  source 1..28: mol_type = other DNA
gactgatacaaaaacacatttgcgctgg

SEQ ID NO: 34788 - DNA, 28 bp, synthetic construct
  source 1..28: mol_type = other DNA
atgtgtttttgtatcagtctgtgtctgg

SEQ ID NO: 34789 - DNA, 28 bp, synthetic construct
  source 1..28: mol_type = other DNA
tgtgtttttgtatcagtctgtgtctggg

SEQ ID NO: 34790 - DNA, 28 bp, synthetic construct
  source 1..28: mol_type = other DNA
tctgtgtctgggtgaacatgaaacctgg

SEQ ID NO: 34791 - DNA, 28 bp, synthetic construct
  source 1..28: mol_type = other DNA
ctgtgtctgggtgaacatgaaacctggg

SEQ ID NO: 34792 - DNA, 28 bp, synthetic construct
  source 1..28: mol_type = other DNA
ccataagatggagctggatgcgcccagg

SEQ ID NO: 34793 - DNA, 28 bp, synthetic construct
  source 1..28: mol_type = other DNA
atccagctccatcttatggcgtagatgg

SEQ ID NO: 34794 - DNA, 28 bp, synthetic construct
  source 1..28: mol_type = other DNA
ctccatctacgccataagatggagctgg

SEQ ID NO: 34795 - DNA, 28 bp, synthetic construct
  source 1..28: mol_type = other DNA
cagctccatcttatggcgtagatggagg

SEQ ID NO: 34796 - DNA, 28 bp, synthetic construct
  source 1..28: mol_type = other DNA
ccatcttatggcgtagatggaggcttgg

SEQ ID NO: 34797 - DNA, 28 bp, synthetic construct
  source 1..28: mol_type = other DNA
tggcgtagatggaggcttggctgtgagg

SEQ ID NO: 34798 - DNA, 28 bp, synthetic construct
  source 1..28: mol_type = other DNA
aggcttggctgtgaggtgtacgcgtcgg

SEQ ID NO: 34799 - DNA, 28 bp, synthetic construct
  source 1..28: mol_type = other DNA
cgcgtcggtgtgtctgtgtctgagcagg

SEQ ID NO: 34800 - DNA, 28 bp, synthetic construct
  source 1..28: mol_type = other DNA
gtcaaaatgacccttcattgtgtcctgg

SEQ ID NO: 34801 - DNA, 28 bp, synthetic construct
  source 1..28: mol_type = other DNA
tagatacacaccaggacacaatgaaggg

SEQ ID NO: 34802 - DNA, 28 bp, synthetic construct
  source 1..28: mol_type = other DNA
atagatacacaccaggacacaatgaagg

SEQ ID NO: 34803 - DNA, 28 bp, synthetic construct
  source 1..28: mol_type = other DNA
tgaggtggacagatagatacacaccagg

SEQ ID NO: 34804 - DNA, 28 bp, synthetic construct
  source 1..28: mol_type = other DNA
cgtaacagcgtacatggagttgaggtgg

SEQ ID NO: 34805 - DNA, 28 bp, synthetic construct
  source 1..28: mol_type = other DNA
ccacgtaacagcgtacatggagttgagg

SEQ ID NO: 34806 - DNA, 28 bp, synthetic construct
  source 1..28: mol_type = other DNA
gacacacaccacgtaacagcgtacatgg

SEQ ID NO: 34807 - DNA, 28 bp, synthetic construct
  source 1..28: mol_type = other DNA
acgtggtgtgtgtctctgaatatacagg

SEQ ID NO: 34808 - DNA, 28 bp, synthetic construct
  source 1..28: mol_type = other DNA
cgtggtgtgtgtctctgaatatacaggg

SEQ ID NO: 34809 - DNA, 28 bp, synthetic construct
  source 1..28: mol_type = other DNA
gggacatttaagtttctgtgtgtgttgg

SEQ ID NO: 34810 - DNA, 28 bp, synthetic construct
  source 1..28: mol_type = other DNA
cagcctagatgtacattgcgtcgctagg

SEQ ID NO: 34811 - DNA, 28 bp, synthetic construct
  source 1..28: mol_type = other DNA
acacctagcgacgcaatgtacatctagg

SEQ ID NO: 34812 - DNA, 28 bp, synthetic construct
  source 1..28: mol_type = other DNA
gtgtgtttatgtgtttgtcccacgttgg

SEQ ID NO: 34813 - DNA, 28 bp, synthetic construct
  source 1..28: mol_type = other DNA
gacatgtatgcatacaagccaacgtggg

SEQ ID NO: 34814 - DNA, 28 bp, synthetic construct
  source 1..28: mol_type = other DNA
agacatgtatgcatacaagccaacgtgg

SEQ ID NO: 34815 - DNA, 28 bp, synthetic construct
  source 1..28: mol_type = other DNA
agcccgcgtgtatatgtgtgagtcacgg

SEQ ID NO: 34816 - DNA, 28 bp, synthetic construct
  source 1..28: mol_type = other DNA
caccgtgactcacacatatacacgcggg

SEQ ID NO: 34817 - DNA, 28 bp, synthetic construct
  source 1..28: mol_type = other DNA
acaccgtgactcacacatatacacgcgg

SEQ ID NO: 34818 - DNA, 28 bp, synthetic construct
  source 1..28: mol_type = other DNA
aagttaacggcacacagatatgcaaggg

SEQ ID NO: 34819 - DNA, 28 bp, synthetic construct
  source 1..28: mol_type = other DNA
taagttaacggcacacagatatgcaagg

SEQ ID NO: 34820 - DNA, 28 bp, synthetic construct
  source 1..28: mol_type = other DNA
gaagacgcagcgcttggtaagttaacgg

SEQ ID NO: 34821 - DNA, 28 bp, synthetic construct
  source 1..28: mol_type = other DNA
ttattagcacagaagacgcagcgcttgg

SEQ ID NO: 34822 - DNA, 28 bp, synthetic construct
  source 1..28: mol_type = other DNA
caatgaatcacacttaaacacacagggg

SEQ ID NO: 34823 - DNA, 28 bp, synthetic construct
  source 1..28: mol_type = other DNA
acaatgaatcacacttaaacacacaggg

SEQ ID NO: 34824 - DNA, 28 bp, synthetic construct
  source 1..28: mol_type = other DNA
cacaatgaatcacacttaaacacacagg

SEQ ID NO: 34825 - DNA, 28 bp, synthetic construct
  source 1..28: mol_type = other DNA
gtgtgattcattgtgagtgtgtgtgtgg

SEQ ID NO: 34826 - DNA, 28 bp, synthetic construct
  source 1..28: mol_type = other DNA
tgtgattcattgtgagtgtgtgtgtggg

SEQ ID NO: 34827 - DNA, 28 bp, synthetic construct
  source 1..28: mol_type = other DNA
gtgattcattgtgagtgtgtgtgtgggg

SEQ ID NO: 34828 - DNA, 28 bp, synthetic construct
  source 1..28: mol_type = other DNA
tgattcattgtgagtgtgtgtgtggggg

SEQ ID NO: 34829 - DNA, 28 bp, synthetic construct
  source 1..28: mol_type = other DNA
gattcattgtgagtgtgtgtgtgggggg

SEQ ID NO: 34830 - DNA, 28 bp, synthetic construct
  source 1..28: mol_type = other DNA
attcattgtgagtgtgtgtgtggggggg

SEQ ID NO: 34831 - DNA, 28 bp, synthetic construct
  source 1..28: mol_type = other DNA
gtgtgtgggggggtttgctgtgtgaagg

SEQ ID NO: 34832 - DNA, 28 bp, synthetic construct
  source 1..28: mol_type = other DNA
agatagagggacagacgcacacaaacgg

SEQ ID NO: 34833 - DNA, 28 bp, synthetic construct
  source 1..28: mol_type = other DNA
gtgcgtctgtccctctatctgactcagg

SEQ ID NO: 34834 - DNA, 28 bp, synthetic construct
  source 1..28: mol_type = other DNA
tgcgtctgtccctctatctgactcaggg

SEQ ID NO: 34835 - DNA, 28 bp, synthetic construct
  source 1..28: mol_type = other DNA
aggggcacgccctgagtcagatagaggg

SEQ ID NO: 34836 - DNA, 28 bp, synthetic construct
  source 1..28: mol_type = other DNA
gaggggcacgccctgagtcagatagagg

SEQ ID NO: 34837 - DNA, 28 bp, synthetic construct
  source 1..28: mol_type = other DNA
agaatgagagggatggaaggaggagggg

SEQ ID NO: 34838 - DNA, 28 bp, synthetic construct
  source 1..28: mol_type = other DNA
gagaatgagagggatggaaggaggaggg

SEQ ID NO: 34839 - DNA, 28 bp, synthetic construct
  source 1..28: mol_type = other DNA
agagaatgagagggatggaaggaggagg

SEQ ID NO: 34840 - DNA, 28 bp, synthetic construct
  source 1..28: mol_type = other DNA
tcctccttccatccctctcattctctgg

SEQ ID NO: 34841 - DNA, 28 bp, synthetic construct
  source 1..28: mol_type = other DNA
tccagagaatgagagggatggaaggagg

SEQ ID NO: 34842 - DNA, 28 bp, synthetic construct
  source 1..28: mol_type = other DNA
ttttccagagaatgagagggatggaagg

SEQ ID NO: 34843 - DNA, 28 bp, synthetic construct
  source 1..28: mol_type = other DNA
cagcttttccagagaatgagagggatgg

SEQ ID NO: 34844 - DNA, 28 bp, synthetic construct
  source 1..28: mol_type = other DNA
catccctctcattctctggaaaagctgg

SEQ ID NO: 34845 - DNA, 28 bp, synthetic construct
  source 1..28: mol_type = other DNA
atccctctcattctctggaaaagctggg

SEQ ID NO: 34846 - DNA, 28 bp, synthetic construct
  source 1..28: mol_type = other DNA
tccctctcattctctggaaaagctgggg

SEQ ID NO: 34847 - DNA, 28 bp, synthetic construct
  source 1..28: mol_type = other DNA
gccccagcttttccagagaatgagaggg

SEQ ID NO: 34848 - DNA, 28 bp, synthetic construct
  source 1..28: mol_type = other DNA
cgccccagcttttccagagaatgagagg

SEQ ID NO: 34849 - DNA, 28 bp, synthetic construct
  source 1..28: mol_type = other DNA
ctctcattctctggaaaagctggggcgg

SEQ ID NO: 34850 - DNA, 28 bp, synthetic construct
  source 1..28: mol_type = other DNA
ctctggaaaagctggggcggagagcagg

SEQ ID NO: 34851 - DNA, 28 bp, synthetic construct
  source 1..28: mol_type = other DNA
tctggaaaagctggggcggagagcaggg

SEQ ID NO: 34852 - DNA, 28 bp, synthetic construct
  source 1..28: mol_type = other DNA
ctggaaaagctggggcggagagcagggg

SEQ ID NO: 34853 - DNA, 28 bp, synthetic construct
  source 1..28: mol_type = other DNA
aagctggggcggagagcaggggttgtgg

SEQ ID NO: 34854 - DNA, 28 bp, synthetic construct
  source 1..28: mol_type = other DNA
agctggggcggagagcaggggttgtggg

SEQ ID NO: 34855 - DNA, 28 bp, synthetic construct
  source 1..28: mol_type = other DNA
gctggggcggagagcaggggttgtgggg

SEQ ID NO: 34856 - DNA, 28 bp, synthetic construct
  source 1..28: mol_type = other DNA
ctggggcggagagcaggggttgtggggg

SEQ ID NO: 34857 - DNA, 28 bp, synthetic construct
  source 1..28: mol_type = other DNA
tggggcggagagcaggggttgtgggggg

SEQ ID NO: 34858 - DNA, 28 bp, synthetic construct
  source 1..28: mol_type = other DNA
gcggagagcaggggttgtggggggatgg

SEQ ID NO: 34859 - DNA, 28 bp, synthetic construct
  source 1..28: mol_type = other DNA
gagcaggggttgtggggggatggtcagg

SEQ ID NO: 34860 - DNA, 28 bp, synthetic construct
  source 1..28: mol_type = other DNA
gttgtggggggatggtcaggacatctgg

SEQ ID NO: 34861 - DNA, 28 bp, synthetic construct
  source 1..28: mol_type = other DNA
ggtcaggacatctggaaagcacatctgg

SEQ ID NO: 34862 - DNA, 28 bp, synthetic construct
  source 1..28: mol_type = other DNA
gacatctggaaagcacatctggaatcgg

SEQ ID NO: 34863 - DNA, 28 bp, synthetic construct
  source 1..28: mol_type = other DNA
gaatcggcctgctcctgtcgtcttgcgg

SEQ ID NO: 34864 - DNA, 28 bp, synthetic construct
  source 1..28: mol_type = other DNA
tgctttaccgcaagacgacaggagcagg

SEQ ID NO: 34865 - DNA, 28 bp, synthetic construct
  source 1..28: mol_type = other DNA
ggttcttgctttaccgcaagacgacagg

SEQ ID NO: 34866 - DNA, 28 bp, synthetic construct
  source 1..28: mol_type = other DNA
gtcttgcggtaaagcaagaaccttctgg

SEQ ID NO: 34867 - DNA, 28 bp, synthetic construct
  source 1..28: mol_type = other DNA
ttgcggtaaagcaagaaccttctggagg

SEQ ID NO: 34868 - DNA, 28 bp, synthetic construct
  source 1..28: mol_type = other DNA
tgcggtaaagcaagaaccttctggaggg

SEQ ID NO: 34869 - DNA, 28 bp, synthetic construct
  source 1..28: mol_type = other DNA
gcggtaaagcaagaaccttctggagggg

SEQ ID NO: 34870 - DNA, 28 bp, synthetic construct
  source 1..28: mol_type = other DNA
taaagcaagaaccttctggaggggaagg

SEQ ID NO: 34871 - DNA, 28 bp, synthetic construct
  source 1..28: mol_type = other DNA
aaagcaagaaccttctggaggggaaggg

SEQ ID NO: 34872 - DNA, 28 bp, synthetic construct
  source 1..28: mol_type = other DNA
aagcaagaaccttctggaggggaagggg

SEQ ID NO: 34873 - DNA, 28 bp, synthetic construct
  source 1..28: mol_type = other DNA
gaactgggaccccttcccctccagaagg

SEQ ID NO: 34874 - DNA, 28 bp, synthetic construct
  source 1..28: mol_type = other DNA
ttgagtgaaggggacaggaggaactggg

SEQ ID NO: 34875 - DNA, 28 bp, synthetic construct
  source 1..28: mol_type = other DNA
cttgagtgaaggggacaggaggaactgg

SEQ ID NO: 34876 - DNA, 28 bp, synthetic construct
  source 1..28: mol_type = other DNA
cagttcctcctgtccccttcactcaagg

SEQ ID NO: 34877 - DNA, 28 bp, synthetic construct
  source 1..28: mol_type = other DNA
cctcctgtccccttcactcaaggtgcgg

SEQ ID NO: 34878 - DNA, 28 bp, synthetic construct
  source 1..28: mol_type = other DNA
cggccgcaccttgagtgaaggggacagg

SEQ ID NO: 34879 - DNA, 28 bp, synthetic construct
  source 1..28: mol_type = other DNA
tccccttcactcaaggtgcggccgttgg

SEQ ID NO: 34880 - DNA, 28 bp, synthetic construct
  source 1..28: mol_type = other DNA
ccccttcactcaaggtgcggccgttggg

SEQ ID NO: 34881 - DNA, 28 bp, synthetic construct
  source 1..28: mol_type = other DNA
ccccaacggccgcaccttgagtgaaggg

SEQ ID NO: 34882 - DNA, 28 bp, synthetic construct
  source 1..28: mol_type = other DNA
gccccaacggccgcaccttgagtgaagg

SEQ ID NO: 34883 - DNA, 28 bp, synthetic construct
  source 1..28: mol_type = other DNA
cactcaaggtgcggccgttggggcctgg

SEQ ID NO: 34884 - DNA, 28 bp, synthetic construct
  source 1..28: mol_type = other DNA
actcaaggtgcggccgttggggcctggg

SEQ ID NO: 34885 - DNA, 28 bp, synthetic construct
  source 1..28: mol_type = other DNA
aaggtgcggccgttggggcctgggaagg

SEQ ID NO: 34886 - DNA, 28 bp, synthetic construct
  source 1..28: mol_type = other DNA
aggtgcggccgttggggcctgggaaggg

SEQ ID NO: 34887 - DNA, 28 bp, synthetic construct
  source 1..28: mol_type = other DNA
ggtgcggccgttggggcctgggaagggg

SEQ ID NO: 34888 - DNA, 28 bp, synthetic construct
  source 1..28: mol_type = other DNA
gtgcggccgttggggcctgggaaggggg

SEQ ID NO: 34889 - DNA, 28 bp, synthetic construct
  source 1..28: mol_type = other DNA
cgggatcccccttcccaggccccaacgg

SEQ ID NO: 34890 - DNA, 28 bp, synthetic construct
  source 1..28: mol_type = other DNA
cgttggggcctgggaagggggatcccgg

SEQ ID NO: 34891 - DNA, 28 bp, synthetic construct
  source 1..28: mol_type = other DNA
ggcctgggaagggggatcccggctctgg

SEQ ID NO: 34892 - DNA, 28 bp, synthetic construct
  source 1..28: mol_type = other DNA
agccagagccgggatcccccttcccagg

SEQ ID NO: 34893 - DNA, 28 bp, synthetic construct
  source 1..28: mol_type = other DNA
gcttcgggggcgcggagccagagccggg

SEQ ID NO: 34894 - DNA, 28 bp, synthetic construct
  source 1..28: mol_type = other DNA
ggcttcgggggcgcggagccagagccgg

SEQ ID NO: 34895 - DNA, 28 bp, synthetic construct
  source 1..28: mol_type = other DNA
ggctctggctccgcgcccccgaagccgg

SEQ ID NO: 34896 - DNA, 28 bp, synthetic construct
  source 1..28: mol_type = other DNA
ctggctccgcgcccccgaagccggccgg

SEQ ID NO: 34897 - DNA, 28 bp, synthetic construct
  source 1..28: mol_type = other DNA
gcgcttccggccggcttcgggggcgcgg

SEQ ID NO: 34898 - DNA, 28 bp, synthetic construct
  source 1..28: mol_type = other DNA
cgcccccgaagccggccggaagcgctgg

SEQ ID NO: 34899 - DNA, 28 bp, synthetic construct
  source 1..28: mol_type = other DNA
gcccccgaagccggccggaagcgctggg

SEQ ID NO: 34900 - DNA, 28 bp, synthetic construct
  source 1..28: mol_type = other DNA
ccccagcgcttccggccggcttcggggg

SEQ ID NO: 34901 - DNA, 28 bp, synthetic construct
  source 1..28: mol_type = other DNA
accccagcgcttccggccggcttcgggg

SEQ ID NO: 34902 - DNA, 28 bp, synthetic construct
  source 1..28: mol_type = other DNA
caccccagcgcttccggccggcttcggg

SEQ ID NO: 34903 - DNA, 28 bp, synthetic construct
  source 1..28: mol_type = other DNA
ccaccccagcgcttccggccggcttcgg

SEQ ID NO: 34904 - DNA, 28 bp, synthetic construct
  source 1..28: mol_type = other DNA
cgaagccggccggaagcgctggggtggg

SEQ ID NO: 34905 - DNA, 28 bp, synthetic construct
  source 1..28: mol_type = other DNA
gaagccggccggaagcgctggggtgggg

SEQ ID NO: 34906 - DNA, 28 bp, synthetic construct
  source 1..28: mol_type = other DNA
gccggccggaagcgctggggtggggagg

SEQ ID NO: 34907 - DNA, 28 bp, synthetic construct
  source 1..28: mol_type = other DNA
acctccccaccccagcgcttccggccgg

SEQ ID NO: 34908 - DNA, 28 bp, synthetic construct
  source 1..28: mol_type = other DNA
gggcacctccccaccccagcgcttccgg

SEQ ID NO: 34909 - DNA, 28 bp, synthetic construct
  source 1..28: mol_type = other DNA
aagcgctggggtggggaggtgcccccgg

SEQ ID NO: 34910 - DNA, 28 bp, synthetic construct
  source 1..28: mol_type = other DNA
ggggaggtgcccccggtgactcacgcgg

SEQ ID NO: 34911 - DNA, 28 bp, synthetic construct
  source 1..28: mol_type = other DNA
gggaggtgcccccggtgactcacgcggg

SEQ ID NO: 34912 - DNA, 28 bp, synthetic construct
  source 1..28: mol_type = other DNA
ggaggtgcccccggtgactcacgcgggg

SEQ ID NO: 34913 - DNA, 28 bp, synthetic construct
  source 1..28: mol_type = other DNA
gaggtgcccccggtgactcacgcggggg

SEQ ID NO: 34914 - DNA, 28 bp, synthetic construct
  source 1..28: mol_type = other DNA
tgcccccggtgactcacgcgggggcagg

SEQ ID NO: 34915 - DNA, 28 bp, synthetic construct
  source 1..28: mol_type = other DNA
ttcctgcccccgcgtgagtcaccggggg

SEQ ID NO: 34916 - DNA, 28 bp, synthetic construct
  source 1..28: mol_type = other DNA
attcctgcccccgcgtgagtcaccgggg

SEQ ID NO: 34917 - DNA, 28 bp, synthetic construct
  source 1..28: mol_type = other DNA
cattcctgcccccgcgtgagtcaccggg

SEQ ID NO: 34918 - DNA, 28 bp, synthetic construct
  source 1..28: mol_type = other DNA
gcattcctgcccccgcgtgagtcaccgg

SEQ ID NO: 34919 - DNA, 28 bp, synthetic construct
  source 1..28: mol_type = other DNA
gactcacgcgggggcaggaatgctgcgg

SEQ ID NO: 34920 - DNA, 28 bp, synthetic construct
  source 1..28: mol_type = other DNA
cacgcgggggcaggaatgctgcggtcgg

SEQ ID NO: 34921 - DNA, 28 bp, synthetic construct
  source 1..28: mol_type = other DNA
gggggcaggaatgctgcggtcggaacgg

SEQ ID NO: 34922 - DNA, 28 bp, synthetic construct
  source 1..28: mol_type = other DNA
ggggcaggaatgctgcggtcggaacggg

SEQ ID NO: 34923 - DNA, 28 bp, synthetic construct
  source 1..28: mol_type = other DNA
ggaatgctgcggtcggaacgggacccgg

SEQ ID NO: 34924 - DNA, 28 bp, synthetic construct
  source 1..28: mol_type = other DNA
ggggctggaggtgggttctggagccggg

SEQ ID NO: 34925 - DNA, 28 bp, synthetic construct
  source 1..28: mol_type = other DNA
tggggctggaggtgggttctggagccgg

SEQ ID NO: 34926 - DNA, 28 bp, synthetic construct
  source 1..28: mol_type = other DNA
ggctccagaacccacctccagccccagg

SEQ ID NO: 34927 - DNA, 28 bp, synthetic construct
  source 1..28: mol_type = other DNA
gctccagaacccacctccagccccaggg

SEQ ID NO: 34928 - DNA, 28 bp, synthetic construct
  source 1..28: mol_type = other DNA
aagccctggggctggaggtgggttctgg

SEQ ID NO: 34929 - DNA, 28 bp, synthetic construct
  source 1..28: mol_type = other DNA
ccggagaagccctggggctggaggtggg

SEQ ID NO: 34930 - DNA, 28 bp, synthetic construct
  source 1..28: mol_type = other DNA
gccggagaagccctggggctggaggtgg

SEQ ID NO: 34931 - DNA, 28 bp, synthetic construct
  source 1..28: mol_type = other DNA
ccggccggagaagccctggggctggagg

SEQ ID NO: 34932 - DNA, 28 bp, synthetic construct
  source 1..28: mol_type = other DNA
ccagccccagggcttctccggccggcgg

SEQ ID NO: 34933 - DNA, 28 bp, synthetic construct
  source 1..28: mol_type = other DNA
ggcgccgccggccggagaagccctgggg

SEQ ID NO: 34934 - DNA, 28 bp, synthetic construct
  source 1..28: mol_type = other DNA
tggcgccgccggccggagaagccctggg

SEQ ID NO: 34935 - DNA, 28 bp, synthetic construct
  source 1..28: mol_type = other DNA
ctggcgccgccggccggagaagccctgg

SEQ ID NO: 34936 - DNA, 28 bp, synthetic construct
  source 1..28: mol_type = other DNA
gcgcgcgggagctggcgccgccggccgg

SEQ ID NO: 34937 - DNA, 28 bp, synthetic construct
  source 1..28: mol_type = other DNA
gtcagcgcgcgggagctggcgccgccgg

SEQ ID NO: 34938 - DNA, 28 bp, synthetic construct
  source 1..28: mol_type = other DNA
ggcgccagctcccgcgcgctgaccctgg

SEQ ID NO: 34939 - DNA, 28 bp, synthetic construct
  source 1..28: mol_type = other DNA
gccagctcccgcgcgctgaccctggcgg

SEQ ID NO: 34940 - DNA, 28 bp, synthetic construct
  source 1..28: mol_type = other DNA
ccagctcccgcgcgctgaccctggcggg

SEQ ID NO: 34941 - DNA, 28 bp, synthetic construct
  source 1..28: mol_type = other DNA
cagctcccgcgcgctgaccctggcgggg

SEQ ID NO: 34942 - DNA, 28 bp, synthetic construct
  source 1..28: mol_type = other DNA
tggggccccgccagggtcagcgcgcggg

SEQ ID NO: 34943 - DNA, 28 bp, synthetic construct
  source 1..28: mol_type = other DNA
gtggggccccgccagggtcagcgcgcgg

SEQ ID NO: 34944 - DNA, 28 bp, synthetic construct
  source 1..28: mol_type = other DNA
tgaccctggcggggccccacgtgccagg

SEQ ID NO: 34945 - DNA, 28 bp, synthetic construct
  source 1..28: mol_type = other DNA
ccctggcggggccccacgtgccaggtgg

SEQ ID NO: 34946 - DNA, 28 bp, synthetic construct
  source 1..28: mol_type = other DNA
gccacctggcacgtggggccccgccagg

SEQ ID NO: 34947 - DNA, 28 bp, synthetic construct
  source 1..28: mol_type = other DNA
ggcggggccccacgtgccaggtggctgg

SEQ ID NO: 34948 - DNA, 28 bp, synthetic construct
  source 1..28: mol_type = other DNA
gtcgggtccagccacctggcacgtgggg

SEQ ID NO: 34949 - DNA, 28 bp, synthetic construct
  source 1..28: mol_type = other DNA
ggtcgggtccagccacctggcacgtggg

SEQ ID NO: 34950 - DNA, 28 bp, synthetic construct
  source 1..28: mol_type = other DNA
gggtcgggtccagccacctggcacgtgg

SEQ ID NO: 34951 - DNA, 28 bp, synthetic construct
  source 1..28: mol_type = other DNA
cgtgccaggtggctggacccgacccagg

SEQ ID NO: 34952 - DNA, 28 bp, synthetic construct
  source 1..28: mol_type = other DNA
ggagcctgggtcgggtccagccacctgg

SEQ ID NO: 34953 - DNA, 28 bp, synthetic construct
  source 1..28: mol_type = other DNA
cgagtgggggcggggagcctgggtcggg

SEQ ID NO: 34954 - DNA, 28 bp, synthetic construct
  source 1..28: mol_type = other DNA
ccgacccaggctccccgcccccactcgg

SEQ ID NO: 34955 - DNA, 28 bp, synthetic construct
  source 1..28: mol_type = other DNA
cgacccaggctccccgcccccactcggg

SEQ ID NO: 34956 - DNA, 28 bp, synthetic construct
  source 1..28: mol_type = other DNA
cggcccgagtgggggcggggagcctggg

SEQ ID NO: 34957 - DNA, 28 bp, synthetic construct
  source 1..28: mol_type = other DNA
gcggcccgagtgggggcggggagcctgg

SEQ ID NO: 34958 - DNA, 28 bp, synthetic construct
  source 1..28: mol_type = other DNA
cgggcgggcggcccgagtgggggcgggg

SEQ ID NO: 34959 - DNA, 28 bp, synthetic construct
  source 1..28: mol_type = other DNA
ccgggcgggcggcccgagtgggggcggg

SEQ ID NO: 34960 - DNA, 28 bp, synthetic construct
  source 1..28: mol_type = other DNA
cccgggcgggcggcccgagtgggggcgg

SEQ ID NO: 34961 - DNA, 28 bp, synthetic construct
  source 1..28: mol_type = other DNA
agtcccgggcgggcggcccgagtggggg

SEQ ID NO: 34962 - DNA, 28 bp, synthetic construct
  source 1..28: mol_type = other DNA
cagtcccgggcgggcggcccgagtgggg

SEQ ID NO: 34963 - DNA, 28 bp, synthetic construct
  source 1..28: mol_type = other DNA
acagtcccgggcgggcggcccgagtggg

SEQ ID NO: 34964 - DNA, 28 bp, synthetic construct
  source 1..28: mol_type = other DNA
tacagtcccgggcgggcggcccgagtgg

SEQ ID NO: 34965 - DNA, 28 bp, synthetic construct
  source 1..28: mol_type = other DNA
gagaaacagtacagtcccgggcgggcgg

SEQ ID NO: 34966 - DNA, 28 bp, synthetic construct
  source 1..28: mol_type = other DNA
gaggagaaacagtacagtcccgggcggg

SEQ ID NO: 34967 - DNA, 28 bp, synthetic construct
  source 1..28: mol_type = other DNA
ggaggagaaacagtacagtcccgggcgg

SEQ ID NO: 34968 - DNA, 28 bp, synthetic construct
  source 1..28: mol_type = other DNA
gcccgggactgtactgtttctcctccgg

SEQ ID NO: 34969 - DNA, 28 bp, synthetic construct
  source 1..28: mol_type = other DNA
cccgggactgtactgtttctcctccggg

SEQ ID NO: 34970 - DNA, 28 bp, synthetic construct
  source 1..28: mol_type = other DNA
gcccggaggagaaacagtacagtcccgg

SEQ ID NO: 34971 - DNA, 28 bp, synthetic construct
  source 1..28: mol_type = other DNA
gggactgtactgtttctcctccgggcgg

SEQ ID NO: 34972 - DNA, 28 bp, synthetic construct
  source 1..28: mol_type = other DNA
tgtactgtttctcctccgggcggcgcgg

SEQ ID NO: 34973 - DNA, 28 bp, synthetic construct
  source 1..28: mol_type = other DNA
gtactgtttctcctccgggcggcgcggg

SEQ ID NO: 34974 - DNA, 28 bp, synthetic construct
  source 1..28: mol_type = other DNA
tactgtttctcctccgggcggcgcgggg

SEQ ID NO: 34975 - DNA, 28 bp, synthetic construct
  source 1..28: mol_type = other DNA
actgtttctcctccgggcggcgcggggg

SEQ ID NO: 34976 - DNA, 28 bp, synthetic construct
  source 1..28: mol_type = other DNA
tctcctccgggcggcgcgggggctgcgg

SEQ ID NO: 34977 - DNA, 28 bp, synthetic construct
  source 1..28: mol_type = other DNA
ctcctccgggcggcgcgggggctgcggg

SEQ ID NO: 34978 - DNA, 28 bp, synthetic construct
  source 1..28: mol_type = other DNA
cgcccgcagcccccgcgccgcccggagg

SEQ ID NO: 34979 - DNA, 28 bp, synthetic construct
  source 1..28: mol_type = other DNA
ccgggcggcgcgggggctgcgggcgcgg

SEQ ID NO: 34980 - DNA, 28 bp, synthetic construct
  source 1..28: mol_type = other DNA
cgggcggcgcgggggctgcgggcgcggg

SEQ ID NO: 34981 - DNA, 28 bp, synthetic construct
  source 1..28: mol_type = other DNA
gggcggcgcgggggctgcgggcgcgggg

SEQ ID NO: 34982 - DNA, 28 bp, synthetic construct
  source 1..28: mol_type = other DNA
cgggggctgcgggcgcggggccttcagg

SEQ ID NO: 34983 - DNA, 28 bp, synthetic construct
  source 1..28: mol_type = other DNA
gggggctgcgggcgcggggccttcaggg

SEQ ID NO: 34984 - DNA, 28 bp, synthetic construct
  source 1..28: mol_type = other DNA
ctgcgggcgcggggccttcagggcgcgg

SEQ ID NO: 34985 - DNA, 28 bp, synthetic construct
  source 1..28: mol_type = other DNA
cgggcgcggggccttcagggcgcggagg

SEQ ID NO: 34986 - DNA, 28 bp, synthetic construct
  source 1..28: mol_type = other DNA
cggggccttcagggcgcggaggctgcgg

SEQ ID NO: 34987 - DNA, 28 bp, synthetic construct
  source 1..28: mol_type = other DNA
ggggccttcagggcgcggaggctgcggg

SEQ ID NO: 34988 - DNA, 28 bp, synthetic construct
  source 1..28: mol_type = other DNA
cgctcccgcagcctccgcgccctgaagg

SEQ ID NO: 34989 - DNA, 28 bp, synthetic construct
  source 1..28: mol_type = other DNA
cttcagggcgcggaggctgcgggagcgg

SEQ ID NO: 34990 - DNA, 28 bp, synthetic construct
  source 1..28: mol_type = other DNA
ttcagggcgcggaggctgcgggagcggg

SEQ ID NO: 34991 - DNA, 28 bp, synthetic construct
  source 1..28: mol_type = other DNA
gcgggagcgggcacctgaccttgtctgg

SEQ ID NO: 34992 - DNA, 28 bp, synthetic construct
  source 1..28: mol_type = other DNA
cgggagcgggcacctgaccttgtctggg

SEQ ID NO: 34993 - DNA, 28 bp, synthetic construct
  source 1..28: mol_type = other DNA
gcgggcacctgaccttgtctgggaacgg

SEQ ID NO: 34994 - DNA, 28 bp, synthetic construct
  source 1..28: mol_type = other DNA
taggtggccgttcccagacaaggtcagg

SEQ ID NO: 34995 - DNA, 28 bp, synthetic construct
  source 1..28: mol_type = other DNA
tgaccttgtctgggaacggccacctagg

SEQ ID NO: 34996 - DNA, 28 bp, synthetic construct
  source 1..28: mol_type = other DNA
cttcctaggtggccgttcccagacaagg

SEQ ID NO: 34997 - DNA, 28 bp, synthetic construct
  source 1..28: mol_type = other DNA
acggccacctaggaagccgcgactgagg

SEQ ID NO: 34998 - DNA, 28 bp, synthetic construct
  source 1..28: mol_type = other DNA
agctcctcagtcgcggcttcctaggtgg

SEQ ID NO: 34999 - DNA, 28 bp, synthetic construct
  source 1..28: mol_type = other DNA
gggagctcctcagtcgcggcttcctagg

SEQ ID NO: 35000 - DNA, 28 bp, synthetic construct
  source 1..28: mol_type = other DNA
ggagggtaggggagctcctcagtcgcgg

SEQ ID NO: 35001 - DNA, 28 bp, synthetic construct
  source 1..28: mol_type = other DNA
aggagctcccctaccctcccctttccgg

SEQ ID NO: 35002 - DNA, 28 bp, synthetic construct
  source 1..28: mol_type = other DNA
gcagaggccggaaaggggagggtagggg

SEQ ID NO: 35003 - DNA, 28 bp, synthetic construct
  source 1..28: mol_type = other DNA
tgcagaggccggaaaggggagggtaggg

SEQ ID NO: 35004 - DNA, 28 bp, synthetic construct
  source 1..28: mol_type = other DNA
ctgcagaggccggaaaggggagggtagg

SEQ ID NO: 35005 - DNA, 28 bp, synthetic construct
  source 1..28: mol_type = other DNA
aagtctgcagaggccggaaaggggaggg

SEQ ID NO: 35006 - DNA, 28 bp, synthetic construct
  source 1..28: mol_type = other DNA
aaagtctgcagaggccggaaaggggagg

SEQ ID NO: 35007 - DNA, 28 bp, synthetic construct
  source 1..28: mol_type = other DNA
tgcaaagtctgcagaggccggaaagggg

SEQ ID NO: 35008 - DNA, 28 bp, synthetic construct
  source 1..28: mol_type = other DNA
gtgcaaagtctgcagaggccggaaaggg

SEQ ID NO: 35009 - DNA, 28 bp, synthetic construct
  source 1..28: mol_type = other DNA
ggtgcaaagtctgcagaggccggaaagg

SEQ ID NO: 35010 - DNA, 28 bp, synthetic construct
  source 1..28: mol_type = other DNA
ggaatggtgcaaagtctgcagaggccgg

SEQ ID NO: 35011 - DNA, 28 bp, synthetic construct
  source 1..28: mol_type = other DNA
gagtggaatggtgcaaagtctgcagagg

SEQ ID NO: 35012 - DNA, 28 bp, synthetic construct
  source 1..28: mol_type = other DNA
tgcaccattccactccctccgctgacgg

SEQ ID NO: 35013 - DNA, 28 bp, synthetic construct
  source 1..28: mol_type = other DNA
ttctccgtcagcggagggagtggaatgg

SEQ ID NO: 35014 - DNA, 28 bp, synthetic construct
  source 1..28: mol_type = other DNA
tccactccctccgctgacggagaaaagg

SEQ ID NO: 35015 - DNA, 28 bp, synthetic construct
  source 1..28: mol_type = other DNA
tccttttctccgtcagcggagggagtgg

SEQ ID NO: 35016 - DNA, 28 bp, synthetic construct
  source 1..28: mol_type = other DNA
aagtttccttttctccgtcagcggaggg

SEQ ID NO: 35017 - DNA, 28 bp, synthetic construct
  source 1..28: mol_type = other DNA
aaagtttccttttctccgtcagcggagg

SEQ ID NO: 35018 - DNA, 28 bp, synthetic construct
  source 1..28: mol_type = other DNA
cacaaagtttccttttctccgtcagcgg

SEQ ID NO: 35019 - DNA, 28 bp, synthetic construct
  source 1..28: mol_type = other DNA
cggagaaaaggaaactttgtgtctgcgg

SEQ ID NO: 35020 - DNA, 28 bp, synthetic construct
  source 1..28: mol_type = other DNA
gaaaaggaaactttgtgtctgcggatgg

SEQ ID NO: 35021 - DNA, 28 bp, synthetic construct
  source 1..28: mol_type = other DNA
ggatggagagcctcccttgccaacgcgg

SEQ ID NO: 35022 - DNA, 28 bp, synthetic construct
  source 1..28: mol_type = other DNA
tggagagcctcccttgccaacgcggtgg

SEQ ID NO: 35023 - DNA, 28 bp, synthetic construct
  source 1..28: mol_type = other DNA
ggagagcctcccttgccaacgcggtggg

SEQ ID NO: 35024 - DNA, 28 bp, synthetic construct
  source 1..28: mol_type = other DNA
tctgttcccaccgcgttggcaagggagg

SEQ ID NO: 35025 - DNA, 28 bp, synthetic construct
  source 1..28: mol_type = other DNA
tcccttgccaacgcggtgggaacagagg

SEQ ID NO: 35026 - DNA, 28 bp, synthetic construct
  source 1..28: mol_type = other DNA
gcctctgttcccaccgcgttggcaaggg

SEQ ID NO: 35027 - DNA, 28 bp, synthetic construct
  source 1..28: mol_type = other DNA
cgcctctgttcccaccgcgttggcaagg

SEQ ID NO: 35028 - DNA, 28 bp, synthetic construct
  source 1..28: mol_type = other DNA
gtgtacgcctctgttcccaccgcgttgg

SEQ ID NO: 35029 - DNA, 28 bp, synthetic construct
  source 1..28: mol_type = other DNA
cggtgggaacagaggcgtacacgcacgg

SEQ ID NO: 35030 - DNA, 28 bp, synthetic construct
  source 1..28: mol_type = other DNA
gtacacaccatccacagatacacgcagg

SEQ ID NO: 35031 - DNA, 28 bp, synthetic construct
  source 1..28: mol_type = other DNA
tacacaccatccacagatacacgcaggg

SEQ ID NO: 35032 - DNA, 28 bp, synthetic construct
  source 1..28: mol_type = other DNA
ttgtgaccctgcgtgtatctgtggatgg

SEQ ID NO: 35033 - DNA, 28 bp, synthetic construct
  source 1..28: mol_type = other DNA
atgtttgtgaccctgcgtgtatctgtgg

SEQ ID NO: 35034 - DNA, 28 bp, synthetic construct
  source 1..28: mol_type = other DNA
tgcatctgtgtttgtgtttctgagctgg

SEQ ID NO: 35035 - DNA, 28 bp, synthetic construct
  source 1..28: mol_type = other DNA
gaactgcagtcgcacttacaagacttgg

SEQ ID NO: 35036 - DNA, 28 bp, synthetic construct
  source 1..28: mol_type = other DNA
agtcgcacttacaagacttggtcccagg

SEQ ID NO: 35037 - DNA, 28 bp, synthetic construct
  source 1..28: mol_type = other DNA
gtcgcacttacaagacttggtcccaggg

SEQ ID NO: 35038 - DNA, 28 bp, synthetic construct
  source 1..28: mol_type = other DNA
cacttacaagacttggtcccagggccgg

SEQ ID NO: 35039 - DNA, 28 bp, synthetic construct
  source 1..28: mol_type = other DNA
acttacaagacttggtcccagggccggg

SEQ ID NO: 35040 - DNA, 28 bp, synthetic construct
  source 1..28: mol_type = other DNA
cttggtcccagggccgggcaccgagtgg

SEQ ID NO: 35041 - DNA, 28 bp, synthetic construct
  source 1..28: mol_type = other DNA
gcagagccactcggtgcccggccctggg

SEQ ID NO: 35042 - DNA, 28 bp, synthetic construct
  source 1..28: mol_type = other DNA
ggcagagccactcggtgcccggccctgg

SEQ ID NO: 35043 - DNA, 28 bp, synthetic construct
  source 1..28: mol_type = other DNA
atcgcaggcagagccactcggtgcccgg

SEQ ID NO: 35044 - DNA, 28 bp, synthetic construct
  source 1..28: mol_type = other DNA
gtgctggatcgcaggcagagccactcgg

SEQ ID NO: 35045 - DNA, 28 bp, synthetic construct
  source 1..28: mol_type = other DNA
tggctctgcctgcgatccagcactttgg

SEQ ID NO: 35046 - DNA, 28 bp, synthetic construct
  source 1..28: mol_type = other DNA
ggctctgcctgcgatccagcactttggg

SEQ ID NO: 35047 - DNA, 28 bp, synthetic construct
  source 1..28: mol_type = other DNA
tctgcctgcgatccagcactttgggagg

SEQ ID NO: 35048 - DNA, 28 bp, synthetic construct
  source 1..28: mol_type = other DNA
tcggcctcccaaagtgctggatcgcagg

SEQ ID NO: 35049 - DNA, 28 bp, synthetic construct
  source 1..28: mol_type = other DNA
tgcgatccagcactttgggaggccgagg

SEQ ID NO: 35050 - DNA, 28 bp, synthetic construct
  source 1..28: mol_type = other DNA
gatccagcactttgggaggccgaggcgg

SEQ ID NO: 35051 - DNA, 28 bp, synthetic construct
  source 1..28: mol_type = other DNA
atccagcactttgggaggccgaggcggg

SEQ ID NO: 35052 - DNA, 28 bp, synthetic construct
  source 1..28: mol_type = other DNA
ctcccgcctcggcctcccaaagtgctgg

SEQ ID NO: 35053 - DNA, 28 bp, synthetic construct
  source 1..28: mol_type = other DNA
cagcactttgggaggccgaggcgggagg

SEQ ID NO: 35054 - DNA, 28 bp, synthetic construct
  source 1..28: mol_type = other DNA
gggaggccgaggcgggaggatcgcttgg

SEQ ID NO: 35055 - DNA, 28 bp, synthetic construct
  source 1..28: mol_type = other DNA
ggaggccgaggcgggaggatcgcttggg

SEQ ID NO: 35056 - DNA, 28 bp, synthetic construct
  source 1..28: mol_type = other DNA
gaggccgaggcgggaggatcgcttgggg

SEQ ID NO: 35057 - DNA, 28 bp, synthetic construct
  source 1..28: mol_type = other DNA
ctggccccaagcgatcctcccgcctcgg

SEQ ID NO: 35058 - DNA, 28 bp, synthetic construct
  source 1..28: mol_type = other DNA
tggggccagaagtttgagagcagcctgg

SEQ ID NO: 35059 - DNA, 28 bp, synthetic construct
  source 1..28: mol_type = other DNA
ggggccagaagtttgagagcagcctggg

SEQ ID NO: 35060 - DNA, 28 bp, synthetic construct
  source 1..28: mol_type = other DNA
gttgcccaggctgctctcaaacttctgg

SEQ ID NO: 35061 - DNA, 28 bp, synthetic construct
  source 1..28: mol_type = other DNA
aagtttgagagcagcctgggcaacgtgg

SEQ ID NO: 35062 - DNA, 28 bp, synthetic construct
  source 1..28: mol_type = other DNA
agaggagagtctcaccacgttgcccagg

SEQ ID NO: 35063 - DNA, 28 bp, synthetic construct
  source 1..28: mol_type = other DNA
ttttcaatttttttttgtagagaagagg

SEQ ID NO: 35064 - DNA, 28 bp, synthetic construct
  source 1..28: mol_type = other DNA
aaaaaattgaaaagttagccaagtgtgg

SEQ ID NO: 35065 - DNA, 28 bp, synthetic construct
  source 1..28: mol_type = other DNA
aaattgaaaagttagccaagtgtggtgg

SEQ ID NO: 35066 - DNA, 28 bp, synthetic construct
  source 1..28: mol_type = other DNA
tgggactacaggcggccaccacacttgg

SEQ ID NO: 35067 - DNA, 28 bp, synthetic construct
  source 1..28: mol_type = other DNA
gtggccgcctgtagtcccagctgcttgg

SEQ ID NO: 35068 - DNA, 28 bp, synthetic construct
  source 1..28: mol_type = other DNA
tggccgcctgtagtcccagctgcttggg

SEQ ID NO: 35069 - DNA, 28 bp, synthetic construct
  source 1..28: mol_type = other DNA
cctcccaagcagctgggactacaggcgg

SEQ ID NO: 35070 - DNA, 28 bp, synthetic construct
  source 1..28: mol_type = other DNA
catcctcccaagcagctgggactacagg

SEQ ID NO: 35071 - DNA, 28 bp, synthetic construct
  source 1..28: mol_type = other DNA
tcccagctgcttgggaggatgagacagg

SEQ ID NO: 35072 - DNA, 28 bp, synthetic construct
  source 1..28: mol_type = other DNA
tcctgtctcatcctcccaagcagctggg

SEQ ID NO: 35073 - DNA, 28 bp, synthetic construct
  source 1..28: mol_type = other DNA
ctcctgtctcatcctcccaagcagctgg

SEQ ID NO: 35074 - DNA, 28 bp, synthetic construct
  source 1..28: mol_type = other DNA
cagctgcttgggaggatgagacaggagg

SEQ ID NO: 35075 - DNA, 28 bp, synthetic construct
  source 1..28: mol_type = other DNA
tgagacaggaggatcgcttgagccctgg

SEQ ID NO: 35076 - DNA, 28 bp, synthetic construct
  source 1..28: mol_type = other DNA
gacaggaggatcgcttgagccctggagg

SEQ ID NO: 35077 - DNA, 28 bp, synthetic construct
  source 1..28: mol_type = other DNA
aggatcgcttgagccctggaggtcaagg

SEQ ID NO: 35078 - DNA, 28 bp, synthetic construct
  source 1..28: mol_type = other DNA
gtgcctgtgtgggctgcactgcccctgg

SEQ ID NO: 35079 - DNA, 28 bp, synthetic construct
  source 1..28: mol_type = other DNA
tgaccaggggcagtgcagcccacacagg

SEQ ID NO: 35080 - DNA, 28 bp, synthetic construct
  source 1..28: mol_type = other DNA
tgtgtgggctgcactgcccctggtcagg

SEQ ID NO: 35081 - DNA, 28 bp, synthetic construct
  source 1..28: mol_type = other DNA
tgggctgcactgcccctggtcaggcagg

SEQ ID NO: 35082 - DNA, 28 bp, synthetic construct
  source 1..28: mol_type = other DNA
gcactgcccctggtcaggcaggccatgg

SEQ ID NO: 35083 - DNA, 28 bp, synthetic construct
  source 1..28: mol_type = other DNA
tgcccctggtcaggcaggccatggtagg

SEQ ID NO: 35084 - DNA, 28 bp, synthetic construct
  source 1..28: mol_type = other DNA
ctcctaccatggcctgcctgaccagggg

SEQ ID NO: 35085 - DNA, 28 bp, synthetic construct
  source 1..28: mol_type = other DNA
actcctaccatggcctgcctgaccaggg

SEQ ID NO: 35086 - DNA, 28 bp, synthetic construct
  source 1..28: mol_type = other DNA
cactcctaccatggcctgcctgaccagg

SEQ ID NO: 35087 - DNA, 28 bp, synthetic construct
  source 1..28: mol_type = other DNA
ctggtcaggcaggccatggtaggagtgg

SEQ ID NO: 35088 - DNA, 28 bp, synthetic construct
  source 1..28: mol_type = other DNA
caggcaggccatggtaggagtggcccgg

SEQ ID NO: 35089 - DNA, 28 bp, synthetic construct
  source 1..28: mol_type = other DNA
aggccatggtaggagtggcccggcatgg

SEQ ID NO: 35090 - DNA, 28 bp, synthetic construct
  source 1..28: mol_type = other DNA
gggccatgccgggccactcctaccatgg

SEQ ID NO: 35091 - DNA, 28 bp, synthetic construct
  source 1..28: mol_type = other DNA
tggtaggagtggcccggcatggccccgg

SEQ ID NO: 35092 - DNA, 28 bp, synthetic construct
  source 1..28: mol_type = other DNA
gcaggaagggctccggggccatgccggg

SEQ ID NO: 35093 - DNA, 28 bp, synthetic construct
  source 1..28: mol_type = other DNA
ggcaggaagggctccggggccatgccgg

SEQ ID NO: 35094 - DNA, 28 bp, synthetic construct
  source 1..28: mol_type = other DNA
tcagagaggggcaggaagggctccgggg

SEQ ID NO: 35095 - DNA, 28 bp, synthetic construct
  source 1..28: mol_type = other DNA
atcagagaggggcaggaagggctccggg

SEQ ID NO: 35096 - DNA, 28 bp, synthetic construct
  source 1..28: mol_type = other DNA
tatcagagaggggcaggaagggctccgg

SEQ ID NO: 35097 - DNA, 28 bp, synthetic construct
  source 1..28: mol_type = other DNA
agcccttcctgcccctctctgatattgg

SEQ ID NO: 35098 - DNA, 28 bp, synthetic construct
  source 1..28: mol_type = other DNA
gtccaatatcagagaggggcaggaaggg

SEQ ID NO: 35099 - DNA, 28 bp, synthetic construct
  source 1..28: mol_type = other DNA
ggtccaatatcagagaggggcaggaagg

SEQ ID NO: 35100 - DNA, 28 bp, synthetic construct
  source 1..28: mol_type = other DNA
gaagggtccaatatcagagaggggcagg

SEQ ID NO: 35101 - DNA, 28 bp, synthetic construct
  source 1..28: mol_type = other DNA
gagggaagggtccaatatcagagagggg

SEQ ID NO: 35102 - DNA, 28 bp, synthetic construct
  source 1..28: mol_type = other DNA
tgagggaagggtccaatatcagagaggg

SEQ ID NO: 35103 - DNA, 28 bp, synthetic construct
  source 1..28: mol_type = other DNA
atgagggaagggtccaatatcagagagg

SEQ ID NO: 35104 - DNA, 28 bp, synthetic construct
  source 1..28: mol_type = other DNA
ggacccttccctcatatgactccctagg

SEQ ID NO: 35105 - DNA, 28 bp, synthetic construct
  source 1..28: mol_type = other DNA
gacccttccctcatatgactccctaggg

SEQ ID NO: 35106 - DNA, 28 bp, synthetic construct
  source 1..28: mol_type = other DNA
agccctagggagtcatatgagggaaggg

SEQ ID NO: 35107 - DNA, 28 bp, synthetic construct
  source 1..28: mol_type = other DNA
cagccctagggagtcatatgagggaagg

SEQ ID NO: 35108 - DNA, 28 bp, synthetic construct
  source 1..28: mol_type = other DNA
tgttcagccctagggagtcatatgaggg

SEQ ID NO: 35109 - DNA, 28 bp, synthetic construct
  source 1..28: mol_type = other DNA
ttgttcagccctagggagtcatatgagg

SEQ ID NO: 35110 - DNA, 28 bp, synthetic construct
  source 1..28: mol_type = other DNA
aaagaggatgtcttgttcagccctaggg

SEQ ID NO: 35111 - DNA, 28 bp, synthetic construct
  source 1..28: mol_type = other DNA
gaaagaggatgtcttgttcagccctagg

SEQ ID NO: 35112 - DNA, 28 bp, synthetic construct
  source 1..28: mol_type = other DNA
gcgttatgggcttcgcaggagaaagagg

SEQ ID NO: 35113 - DNA, 28 bp, synthetic construct
  source 1..28: mol_type = other DNA
ttctcctgcgaagcccataacgccaagg

SEQ ID NO: 35114 - DNA, 28 bp, synthetic construct
  source 1..28: mol_type = other DNA
tctcctgcgaagcccataacgccaaggg

SEQ ID NO: 35115 - DNA, 28 bp, synthetic construct
  source 1..28: mol_type = other DNA
ctcctgcgaagcccataacgccaagggg

SEQ ID NO: 35116 - DNA, 28 bp, synthetic construct
  source 1..28: mol_type = other DNA
tcctgcgaagcccataacgccaaggggg

SEQ ID NO: 35117 - DNA, 28 bp, synthetic construct
  source 1..28: mol_type = other DNA
acccccttggcgttatgggcttcgcagg

SEQ ID NO: 35118 - DNA, 28 bp, synthetic construct
  source 1..28: mol_type = other DNA
gatgtggtgacccccttggcgttatggg

SEQ ID NO: 35119 - DNA, 28 bp, synthetic construct
  source 1..28: mol_type = other DNA
ggatgtggtgacccccttggcgttatgg

SEQ ID NO: 35120 - DNA, 28 bp, synthetic construct
  source 1..28: mol_type = other DNA
gctgtgcgggatgtggtgacccccttgg

SEQ ID NO: 35121 - DNA, 28 bp, synthetic construct
  source 1..28: mol_type = other DNA
ccacatcccgcacagccaccatcacagg

SEQ ID NO: 35122 - DNA, 28 bp, synthetic construct
  source 1..28: mol_type = other DNA
ctgtcacctgtgatggtggctgtgcggg

SEQ ID NO: 35123 - DNA, 28 bp, synthetic construct
  source 1..28: mol_type = other DNA
tctgtcacctgtgatggtggctgtgcgg

SEQ ID NO: 35124 - DNA, 28 bp, synthetic construct
  source 1..28: mol_type = other DNA
cagccaccatcacaggtgacagagttgg

SEQ ID NO: 35125 - DNA, 28 bp, synthetic construct
  source 1..28: mol_type = other DNA
agccaccatcacaggtgacagagttggg

SEQ ID NO: 35126 - DNA, 28 bp, synthetic construct
  source 1..28: mol_type = other DNA
ctcccaactctgtcacctgtgatggtgg

SEQ ID NO: 35127 - DNA, 28 bp, synthetic construct
  source 1..28: mol_type = other DNA
caccatcacaggtgacagagttgggagg

SEQ ID NO: 35128 - DNA, 28 bp, synthetic construct
  source 1..28: mol_type = other DNA
cacctcccaactctgtcacctgtgatgg

SEQ ID NO: 35129 - DNA, 28 bp, synthetic construct
  source 1..28: mol_type = other DNA
catcacaggtgacagagttgggaggtgg

SEQ ID NO: 35130 - DNA, 28 bp, synthetic construct
  source 1..28: mol_type = other DNA
atcacaggtgacagagttgggaggtggg

SEQ ID NO: 35131 - DNA, 28 bp, synthetic construct
  source 1..28: mol_type = other DNA
tcacaggtgacagagttgggaggtgggg

SEQ ID NO: 35132 - DNA, 28 bp, synthetic construct
  source 1..28: mol_type = other DNA
gtgacagagttgggaggtggggagctgg

SEQ ID NO: 35133 - DNA, 28 bp, synthetic construct
  source 1..28: mol_type = other DNA
tgacagagttgggaggtggggagctggg

SEQ ID NO: 35134 - DNA, 28 bp, synthetic construct
  source 1..28: mol_type = other DNA
tgggaggtggggagctgggcgtcagagg

SEQ ID NO: 35135 - DNA, 28 bp, synthetic construct
  source 1..28: mol_type = other DNA
gggaggtggggagctgggcgtcagaggg

SEQ ID NO: 35136 - DNA, 28 bp, synthetic construct
  source 1..28: mol_type = other DNA
aggtggggagctgggcgtcagagggtgg

SEQ ID NO: 35137 - DNA, 28 bp, synthetic construct
  source 1..28: mol_type = other DNA
ggtggggagctgggcgtcagagggtggg

SEQ ID NO: 35138 - DNA, 28 bp, synthetic construct
  source 1..28: mol_type = other DNA
gtggggagctgggcgtcagagggtgggg

SEQ ID NO: 35139 - DNA, 28 bp, synthetic construct
  source 1..28: mol_type = other DNA
gagctgggcgtcagagggtggggtttgg

SEQ ID NO: 35140 - DNA, 28 bp, synthetic construct
  source 1..28: mol_type = other DNA
agctgggcgtcagagggtggggtttggg

SEQ ID NO: 35141 - DNA, 28 bp, synthetic construct
  source 1..28: mol_type = other DNA
ggcgtcagagggtggggtttgggtccgg

SEQ ID NO: 35142 - DNA, 28 bp, synthetic construct
  source 1..28: mol_type = other DNA
gcgtcagagggtggggtttgggtccggg

SEQ ID NO: 35143 - DNA, 28 bp, synthetic construct
  source 1..28: mol_type = other DNA
cgtcagagggtggggtttgggtccgggg

SEQ ID NO: 35144 - DNA, 28 bp, synthetic construct
  source 1..28: mol_type = other DNA
gtggggtttgggtccggggtcagagtgg

SEQ ID NO: 35145 - DNA, 28 bp, synthetic construct
  source 1..28: mol_type = other DNA
tggggtttgggtccggggtcagagtggg

SEQ ID NO: 35146 - DNA, 28 bp, synthetic construct
  source 1..28: mol_type = other DNA
ggggtttgggtccggggtcagagtgggg

SEQ ID NO: 35147 - DNA, 28 bp, synthetic construct
  source 1..28: mol_type = other DNA
gggtttgggtccggggtcagagtggggg

SEQ ID NO: 35148 - DNA, 28 bp, synthetic construct
  source 1..28: mol_type = other DNA
ctgctctctgcccccactctgaccccgg

SEQ ID NO: 35149 - DNA, 28 bp, synthetic construct
  source 1..28: mol_type = other DNA
cggggtcagagtgggggcagagagcagg

SEQ ID NO: 35150 - DNA, 28 bp, synthetic construct
  source 1..28: mol_type = other DNA
ggggtcagagtgggggcagagagcaggg

SEQ ID NO: 35151 - DNA, 28 bp, synthetic construct
  source 1..28: mol_type = other DNA
tcagagtgggggcagagagcagggtagg

SEQ ID NO: 35152 - DNA, 28 bp, synthetic construct
  source 1..28: mol_type = other DNA
cagagtgggggcagagagcagggtaggg

SEQ ID NO: 35153 - DNA, 28 bp, synthetic construct
  source 1..28: mol_type = other DNA
gagcagggtagggagctttgagcaaagg

SEQ ID NO: 35154 - DNA, 28 bp, synthetic construct
  source 1..28: mol_type = other DNA
agggagctttgagcaaaggctccccagg

SEQ ID NO: 35155 - DNA, 28 bp, synthetic construct
  source 1..28: mol_type = other DNA
gggagctttgagcaaaggctccccaggg

SEQ ID NO: 35156 - DNA, 28 bp, synthetic construct
  source 1..28: mol_type = other DNA
ggacaaacgggagagattgaccctgggg

SEQ ID NO: 35157 - DNA, 28 bp, synthetic construct
  source 1..28: mol_type = other DNA
tggacaaacgggagagattgaccctggg

SEQ ID NO: 35158 - DNA, 28 bp, synthetic construct
  source 1..28: mol_type = other DNA
gtggacaaacgggagagattgaccctgg

SEQ ID NO: 35159 - DNA, 28 bp, synthetic construct
  source 1..28: mol_type = other DNA
tgctgggggagcactgtggacaaacggg

SEQ ID NO: 35160 - DNA, 28 bp, synthetic construct
  source 1..28: mol_type = other DNA
ctgctgggggagcactgtggacaaacgg

SEQ ID NO: 35161 - DNA, 28 bp, synthetic construct
  source 1..28: mol_type = other DNA
ttacggggctgctgggggagcactgtgg

SEQ ID NO: 35162 - DNA, 28 bp, synthetic construct
  source 1..28: mol_type = other DNA
caggtggaggttacggggctgctggggg

SEQ ID NO: 35163 - DNA, 28 bp, synthetic construct
  source 1..28: mol_type = other DNA
ccccagcagccccgtaacctccacctgg

SEQ ID NO: 35164 - DNA, 28 bp, synthetic construct
  source 1..28: mol_type = other DNA
accaggtggaggttacggggctgctggg

SEQ ID NO: 35165 - DNA, 28 bp, synthetic construct
  source 1..28: mol_type = other DNA
gaccaggtggaggttacggggctgctgg

SEQ ID NO: 35166 - DNA, 28 bp, synthetic construct
  source 1..28: mol_type = other DNA
ggcgggagaccaggtggaggttacgggg

SEQ ID NO: 35167 - DNA, 28 bp, synthetic construct
  source 1..28: mol_type = other DNA
tggcgggagaccaggtggaggttacggg

SEQ ID NO: 35168 - DNA, 28 bp, synthetic construct
  source 1..28: mol_type = other DNA
ttggcgggagaccaggtggaggttacgg

SEQ ID NO: 35169 - DNA, 28 bp, synthetic construct
  source 1..28: mol_type = other DNA
cgtgggttggcgggagaccaggtggagg

SEQ ID NO: 35170 - DNA, 28 bp, synthetic construct
  source 1..28: mol_type = other DNA
ctccacctggtctcccgccaacccacgg

SEQ ID NO: 35171 - DNA, 28 bp, synthetic construct
  source 1..28: mol_type = other DNA
ctccgtgggttggcgggagaccaggtgg

SEQ ID NO: 35172 - DNA, 28 bp, synthetic construct
  source 1..28: mol_type = other DNA
cagctccgtgggttggcgggagaccagg

SEQ ID NO: 35173 - DNA, 28 bp, synthetic construct
  source 1..28: mol_type = other DNA
ctggtctcccgccaacccacggagctgg

SEQ ID NO: 35174 - DNA, 28 bp, synthetic construct
  source 1..28: mol_type = other DNA
gtctcccgccaacccacggagctggagg

SEQ ID NO: 35175 - DNA, 28 bp, synthetic construct
  source 1..28: mol_type = other DNA
tcccgccaacccacggagctggaggtgg

SEQ ID NO: 35176 - DNA, 28 bp, synthetic construct
  source 1..28: mol_type = other DNA
gccacctccagctccgtgggttggcggg

SEQ ID NO: 35177 - DNA, 28 bp, synthetic construct
  source 1..28: mol_type = other DNA
agccacctccagctccgtgggttggcgg

SEQ ID NO: 35178 - DNA, 28 bp, synthetic construct
  source 1..28: mol_type = other DNA
ccaacccacggagctggaggtggcttgg

SEQ ID NO: 35179 - DNA, 28 bp, synthetic construct
  source 1..28: mol_type = other DNA
gagtccaagccacctccagctccgtggg

SEQ ID NO: 35180 - DNA, 28 bp, synthetic construct
  source 1..28: mol_type = other DNA
ggagtccaagccacctccagctccgtgg

SEQ ID NO: 35181 - DNA, 28 bp, synthetic construct
  source 1..28: mol_type = other DNA
cggagctggaggtggcttggactccagg

SEQ ID NO: 35182 - DNA, 28 bp, synthetic construct
  source 1..28: mol_type = other DNA
aggtggcttggactccaggcctgagcgg

SEQ ID NO: 35183 - DNA, 28 bp, synthetic construct
  source 1..28: mol_type = other DNA
tcagggggtagatgccgctcaggcctgg

SEQ ID NO: 35184 - DNA, 28 bp, synthetic construct
  source 1..28: mol_type = other DNA
gtgggtcagggggtagatgccgctcagg

SEQ ID NO: 35185 - DNA, 28 bp, synthetic construct
  source 1..28: mol_type = other DNA
taccccctgacccactgcaccctgcagg

SEQ ID NO: 35186 - DNA, 28 bp, synthetic construct
  source 1..28: mol_type = other DNA
cacctgcagggtgcagtgggtcaggggg

SEQ ID NO: 35187 - DNA, 28 bp, synthetic construct
  source 1..28: mol_type = other DNA
tcacctgcagggtgcagtgggtcagggg

SEQ ID NO: 35188 - DNA, 28 bp, synthetic construct
  source 1..28: mol_type = other DNA
ctcacctgcagggtgcagtgggtcaggg

SEQ ID NO: 35189 - DNA, 28 bp, synthetic construct
  source 1..28: mol_type = other DNA
tctcacctgcagggtgcagtgggtcagg

SEQ ID NO: 35190 - DNA, 28 bp, synthetic construct
  source 1..28: mol_type = other DNA
gggagtctcacctgcagggtgcagtggg

SEQ ID NO: 35191 - DNA, 28 bp, synthetic construct
  source 1..28: mol_type = other DNA
tgggagtctcacctgcagggtgcagtgg

SEQ ID NO: 35192 - DNA, 28 bp, synthetic construct
  source 1..28: mol_type = other DNA
accctgcaggtgagactcccaaacttgg

SEQ ID NO: 35193 - DNA, 28 bp, synthetic construct
  source 1..28: mol_type = other DNA
accaagtttgggagtctcacctgcaggg

SEQ ID NO: 35194 - DNA, 28 bp, synthetic construct
  source 1..28: mol_type = other DNA
aaccaagtttgggagtctcacctgcagg

SEQ ID NO: 35195 - DNA, 28 bp, synthetic construct
  source 1..28: mol_type = other DNA
cccaaacttggttcatttcagtctcagg

SEQ ID NO: 35196 - DNA, 28 bp, synthetic construct
  source 1..28: mol_type = other DNA
gcctgagactgaaatgaaccaagtttgg

SEQ ID NO: 35197 - DNA, 28 bp, synthetic construct
  source 1..28: mol_type = other DNA
gggggttgtggatgtgggtggaaggagg

SEQ ID NO: 35198 - DNA, 28 bp, synthetic construct
  source 1..28: mol_type = other DNA
gatgggggttgtggatgtgggtggaagg

SEQ ID NO: 35199 - DNA, 28 bp, synthetic construct
  source 1..28: mol_type = other DNA
agaggatgggggttgtggatgtgggtgg

SEQ ID NO: 35200 - DNA, 28 bp, synthetic construct
  source 1..28: mol_type = other DNA
gggagaggatgggggttgtggatgtggg

SEQ ID NO: 35201 - DNA, 28 bp, synthetic construct
  source 1..28: mol_type = other DNA
agggagaggatgggggttgtggatgtgg

SEQ ID NO: 35202 - DNA, 28 bp, synthetic construct
  source 1..28: mol_type = other DNA
acatccacaacccccatcctctccctgg

SEQ ID NO: 35203 - DNA, 28 bp, synthetic construct
  source 1..28: mol_type = other DNA
catccacaacccccatcctctccctggg

SEQ ID NO: 35204 - DNA, 28 bp, synthetic construct
  source 1..28: mol_type = other DNA
gttcccagggagaggatgggggttgtgg

SEQ ID NO: 35205 - DNA, 28 bp, synthetic construct
  source 1..28: mol_type = other DNA
tggtgggttcccagggagaggatggggg

SEQ ID NO: 35206 - DNA, 28 bp, synthetic construct
  source 1..28: mol_type = other DNA
gtggtgggttcccagggagaggatgggg

SEQ ID NO: 35207 - DNA, 28 bp, synthetic construct
  source 1..28: mol_type = other DNA
agtggtgggttcccagggagaggatggg

SEQ ID NO: 35208 - DNA, 28 bp, synthetic construct
  source 1..28: mol_type = other DNA
aagtggtgggttcccagggagaggatgg

SEQ ID NO: 35209 - DNA, 28 bp, synthetic construct
  source 1..28: mol_type = other DNA
cgagaagtggtgggttcccagggagagg

SEQ ID NO: 35210 - DNA, 28 bp, synthetic construct
  source 1..28: mol_type = other DNA
ctctccctgggaacccaccacttctcgg

SEQ ID NO: 35211 - DNA, 28 bp, synthetic construct
  source 1..28: mol_type = other DNA
gtggccgagaagtggtgggttcccaggg

SEQ ID NO: 35212 - DNA, 28 bp, synthetic construct
  source 1..28: mol_type = other DNA
agtggccgagaagtggtgggttcccagg

SEQ ID NO: 35213 - DNA, 28 bp, synthetic construct
  source 1..28: mol_type = other DNA
ttctcaacagtggccgagaagtggtggg

SEQ ID NO: 35214 - DNA, 28 bp, synthetic construct
  source 1..28: mol_type = other DNA
cttctcaacagtggccgagaagtggtgg

SEQ ID NO: 35215 - DNA, 28 bp, synthetic construct
  source 1..28: mol_type = other DNA
ctgcttctcaacagtggccgagaagtgg

SEQ ID NO: 35216 - DNA, 28 bp, synthetic construct
  source 1..28: mol_type = other DNA
gccactgttgagaagcagtagagcctgg

SEQ ID NO: 35217 - DNA, 28 bp, synthetic construct
  source 1..28: mol_type = other DNA
ccactgttgagaagcagtagagcctggg

SEQ ID NO: 35218 - DNA, 28 bp, synthetic construct
  source 1..28: mol_type = other DNA
cactgttgagaagcagtagagcctgggg

SEQ ID NO: 35219 - DNA, 28 bp, synthetic construct
  source 1..28: mol_type = other DNA
actgttgagaagcagtagagcctggggg

SEQ ID NO: 35220 - DNA, 28 bp, synthetic construct
  source 1..28: mol_type = other DNA
ctgttgagaagcagtagagcctgggggg

SEQ ID NO: 35221 - DNA, 28 bp, synthetic construct
  source 1..28: mol_type = other DNA
ctggtgtgactacacaacttttcaaggg

SEQ ID NO: 35222 - DNA, 28 bp, synthetic construct
  source 1..28: mol_type = other DNA
tctggtgtgactacacaacttttcaagg

SEQ ID NO: 35223 - DNA, 28 bp, synthetic construct
  source 1..28: mol_type = other DNA
tgtagtcacaccagaccaccaccactgg

SEQ ID NO: 35224 - DNA, 28 bp, synthetic construct
  source 1..28: mol_type = other DNA
gtagtcacaccagaccaccaccactggg

SEQ ID NO: 35225 - DNA, 28 bp, synthetic construct
  source 1..28: mol_type = other DNA
cacacagctcccagtggtggtggtctgg

SEQ ID NO: 35226 - DNA, 28 bp, synthetic construct
  source 1..28: mol_type = other DNA
atggtcacacagctcccagtggtggtgg

SEQ ID NO: 35227 - DNA, 28 bp, synthetic construct
  source 1..28: mol_type = other DNA
gagatggtcacacagctcccagtggtgg

SEQ ID NO: 35228 - DNA, 28 bp, synthetic construct
  source 1..28: mol_type = other DNA
cacgagatggtcacacagctcccagtgg

SEQ ID NO: 35229 - DNA, 28 bp, synthetic construct
  source 1..28: mol_type = other DNA
tgtgtgaccatctcgtgtgattgcttgg

SEQ ID NO: 35230 - DNA, 28 bp, synthetic construct
  source 1..28: mol_type = other DNA
gggacagccaagcaatcacacgagatgg

SEQ ID NO: 35231 - DNA, 28 bp, synthetic construct
  source 1..28: mol_type = other DNA
tgaggagaggcaagggtgtgaggacggg

SEQ ID NO: 35232 - DNA, 28 bp, synthetic construct
  source 1..28: mol_type = other DNA
ctgaggagaggcaagggtgtgaggacgg

SEQ ID NO: 35233 - DNA, 28 bp, synthetic construct
  source 1..28: mol_type = other DNA
cgtcctcacacccttgcctctcctcagg

SEQ ID NO: 35234 - DNA, 28 bp, synthetic construct
  source 1..28: mol_type = other DNA
cagcctgaggagaggcaagggtgtgagg

SEQ ID NO: 35235 - DNA, 28 bp, synthetic construct
  source 1..28: mol_type = other DNA
gacagcacagcctgaggagaggcaaggg

SEQ ID NO: 35236 - DNA, 28 bp, synthetic construct
  source 1..28: mol_type = other DNA
tgacagcacagcctgaggagaggcaagg

SEQ ID NO: 35237 - DNA, 28 bp, synthetic construct
  source 1..28: mol_type = other DNA
tcgtctgacagcacagcctgaggagagg

SEQ ID NO: 35238 - DNA, 28 bp, synthetic construct
  source 1..28: mol_type = other DNA
ctcctcaggctgtgctgtcagacgatgg

SEQ ID NO: 35239 - DNA, 28 bp, synthetic construct
  source 1..28: mol_type = other DNA
tcctcaggctgtgctgtcagacgatggg

SEQ ID NO: 35240 - DNA, 28 bp, synthetic construct
  source 1..28: mol_type = other DNA
tcccatcgtctgacagcacagcctgagg

SEQ ID NO: 35241 - DNA, 28 bp, synthetic construct
  source 1..28: mol_type = other DNA
caggctgtgctgtcagacgatgggatgg

SEQ ID NO: 35242 - DNA, 28 bp, synthetic construct
  source 1..28: mol_type = other DNA
aggctgtgctgtcagacgatgggatggg

SEQ ID NO: 35243 - DNA, 28 bp, synthetic construct
  source 1..28: mol_type = other DNA
ctgtcagacgatgggatgggcatccagg

SEQ ID NO: 35244 - DNA, 28 bp, synthetic construct
  source 1..28: mol_type = other DNA
tcagacgatgggatgggcatccaggcgg

SEQ ID NO: 35245 - DNA, 28 bp, synthetic construct
  source 1..28: mol_type = other DNA
cagacgatgggatgggcatccaggcggg

SEQ ID NO: 35246 - DNA, 28 bp, synthetic construct
  source 1..28: mol_type = other DNA
ctctggggggtctggttctcccgcctgg

SEQ ID NO: 35247 - DNA, 28 bp, synthetic construct
  source 1..28: mol_type = other DNA
caggcgggagaaccagaccccccagagg

SEQ ID NO: 35248 - DNA, 28 bp, synthetic construct
  source 1..28: mol_type = other DNA
aggtgaggggctcctctggggggtctgg

SEQ ID NO: 35249 - DNA, 28 bp, synthetic construct
  source 1..28: mol_type = other DNA
ttgcgaggtgaggggctcctctgggggg

SEQ ID NO: 35250 - DNA, 28 bp, synthetic construct
  source 1..28: mol_type = other DNA
cttgcgaggtgaggggctcctctggggg

SEQ ID NO: 35251 - DNA, 28 bp, synthetic construct
  source 1..28: mol_type = other DNA
gcttgcgaggtgaggggctcctctgggg

SEQ ID NO: 35252 - DNA, 28 bp, synthetic construct
  source 1..28: mol_type = other DNA
tgcttgcgaggtgaggggctcctctggg

SEQ ID NO: 35253 - DNA, 28 bp, synthetic construct
  source 1..28: mol_type = other DNA
atgcttgcgaggtgaggggctcctctgg

SEQ ID NO: 35254 - DNA, 28 bp, synthetic construct
  source 1..28: mol_type = other DNA
ggggcacggatgcttgcgaggtgagggg

SEQ ID NO: 35255 - DNA, 28 bp, synthetic construct
  source 1..28: mol_type = other DNA
gggggcacggatgcttgcgaggtgaggg

SEQ ID NO: 35256 - DNA, 28 bp, synthetic construct
  source 1..28: mol_type = other DNA
ggggggcacggatgcttgcgaggtgagg

SEQ ID NO: 35257 - DNA, 28 bp, synthetic construct
  source 1..28: mol_type = other DNA
tgatgggggggcacggatgcttgcgagg

SEQ ID NO: 35258 - DNA, 28 bp, synthetic construct
  source 1..28: mol_type = other DNA
agcatccgtgcccccccatcagcttcgg

SEQ ID NO: 35259 - DNA, 28 bp, synthetic construct
  source 1..28: mol_type = other DNA
cctagccgaagctgatgggggggcacgg

SEQ ID NO: 35260 - DNA, 28 bp, synthetic construct
  source 1..28: mol_type = other DNA
ggctgcctagccgaagctgatggggggg

SEQ ID NO: 35261 - DNA, 28 bp, synthetic construct
  source 1..28: mol_type = other DNA
aggctgcctagccgaagctgatgggggg

SEQ ID NO: 35262 - DNA, 28 bp, synthetic construct
  source 1..28: mol_type = other DNA
gaggctgcctagccgaagctgatggggg

SEQ ID NO: 35263 - DNA, 28 bp, synthetic construct
  source 1..28: mol_type = other DNA
ggaggctgcctagccgaagctgatgggg

SEQ ID NO: 35264 - DNA, 28 bp, synthetic construct
  source 1..28: mol_type = other DNA
tggaggctgcctagccgaagctgatggg

SEQ ID NO: 35265 - DNA, 28 bp, synthetic construct
  source 1..28: mol_type = other DNA
atggaggctgcctagccgaagctgatgg

SEQ ID NO: 35266 - DNA, 28 bp, synthetic construct
  source 1..28: mol_type = other DNA
gatgtgataaggggtgtgaggatggagg

SEQ ID NO: 35267 - DNA, 28 bp, synthetic construct
  source 1..28: mol_type = other DNA
gcggatgtgataaggggtgtgaggatgg

SEQ ID NO: 35268 - DNA, 28 bp, synthetic construct
  source 1..28: mol_type = other DNA
cctcacaccccttatcacatccgcgtgg

SEQ ID NO: 35269 - DNA, 28 bp, synthetic construct
  source 1..28: mol_type = other DNA
gtgcatgccacgcggatgtgataagggg

SEQ ID NO: 35270 - DNA, 28 bp, synthetic construct
  source 1..28: mol_type = other DNA
ggtgcatgccacgcggatgtgataaggg

SEQ ID NO: 35271 - DNA, 28 bp, synthetic construct
  source 1..28: mol_type = other DNA
tggtgcatgccacgcggatgtgataagg

SEQ ID NO: 35272 - DNA, 28 bp, synthetic construct
  source 1..28: mol_type = other DNA
atccgcgtggcatgcaccagcagccagg

SEQ ID NO: 35273 - DNA, 28 bp, synthetic construct
  source 1..28: mol_type = other DNA
tccgcgtggcatgcaccagcagccaggg

SEQ ID NO: 35274 - DNA, 28 bp, synthetic construct
  source 1..28: mol_type = other DNA
gccctggctgctggtgcatgccacgcgg

SEQ ID NO: 35275 - DNA, 28 bp, synthetic construct
  source 1..28: mol_type = other DNA
caccagcagccagggcccctcatcctgg

SEQ ID NO: 35276 - DNA, 28 bp, synthetic construct
  source 1..28: mol_type = other DNA
gtccaggatgaggggccctggctgctgg

SEQ ID NO: 35277 - DNA, 28 bp, synthetic construct
  source 1..28: mol_type = other DNA
ccagtgggtccaggatgaggggccctgg

SEQ ID NO: 35278 - DNA, 28 bp, synthetic construct
  source 1..28: mol_type = other DNA
aggaagccagtgggtccaggatgagggg

SEQ ID NO: 35279 - DNA, 28 bp, synthetic construct
  source 1..28: mol_type = other DNA
caggaagccagtgggtccaggatgaggg

SEQ ID NO: 35280 - DNA, 28 bp, synthetic construct
  source 1..28: mol_type = other DNA
acaggaagccagtgggtccaggatgagg

SEQ ID NO: 35281 - DNA, 28 bp, synthetic construct
  source 1..28: mol_type = other DNA
tcatcctggacccactggcttcctgtgg

SEQ ID NO: 35282 - DNA, 28 bp, synthetic construct
  source 1..28: mol_type = other DNA
gtctccacaggaagccagtgggtccagg

SEQ ID NO: 35283 - DNA, 28 bp, synthetic construct
  source 1..28: mol_type = other DNA
acccactggcttcctgtggagacgccgg

SEQ ID NO: 35284 - DNA, 28 bp, synthetic construct
  source 1..28: mol_type = other DNA
tccggcgtctccacaggaagccagtggg

SEQ ID NO: 35285 - DNA, 28 bp, synthetic construct
  source 1..28: mol_type = other DNA
ctccggcgtctccacaggaagccagtgg

SEQ ID NO: 35286 - DNA, 28 bp, synthetic construct
  source 1..28: mol_type = other DNA
cactggcttcctgtggagacgccggagg

SEQ ID NO: 35287 - DNA, 28 bp, synthetic construct
  source 1..28: mol_type = other DNA
actggcttcctgtggagacgccggaggg

SEQ ID NO: 35288 - DNA, 28 bp, synthetic construct
  source 1..28: mol_type = other DNA
ggcttcctgtggagacgccggagggagg

SEQ ID NO: 35289 - DNA, 28 bp, synthetic construct
  source 1..28: mol_type = other DNA
tcttacctccctccggcgtctccacagg

SEQ ID NO: 35290 - DNA, 28 bp, synthetic construct
  source 1..28: mol_type = other DNA
gtggagacgccggagggaggtaagaagg

SEQ ID NO: 35291 - DNA, 28 bp, synthetic construct
  source 1..28: mol_type = other DNA
tggagacgccggagggaggtaagaaggg

SEQ ID NO: 35292 - DNA, 28 bp, synthetic construct
  source 1..28: mol_type = other DNA
gacgccggagggaggtaagaagggttgg

SEQ ID NO: 35293 - DNA, 28 bp, synthetic construct
  source 1..28: mol_type = other DNA
acgccggagggaggtaagaagggttggg

SEQ ID NO: 35294 - DNA, 28 bp, synthetic construct
  source 1..28: mol_type = other DNA
cgccggagggaggtaagaagggttgggg

SEQ ID NO: 35295 - DNA, 28 bp, synthetic construct
  source 1..28: mol_type = other DNA
ctccccaacccttcttacctccctccgg

SEQ ID NO: 35296 - DNA, 28 bp, synthetic construct
  source 1..28: mol_type = other DNA
cggagggaggtaagaagggttggggagg

SEQ ID NO: 35297 - DNA, 28 bp, synthetic construct
  source 1..28: mol_type = other DNA
ggagggaggtaagaagggttggggaggg

SEQ ID NO: 35298 - DNA, 28 bp, synthetic construct
  source 1..28: mol_type = other DNA
gagggacacgtcaccactgccccaccgg

SEQ ID NO: 35299 - DNA, 28 bp, synthetic construct
  source 1..28: mol_type = other DNA
atataagcaaggtccggtggggcagtgg

SEQ ID NO: 35300 - DNA, 28 bp, synthetic construct
  source 1..28: mol_type = other DNA
gcactgatataagcaaggtccggtgggg

SEQ ID NO: 35301 - DNA, 28 bp, synthetic construct
  source 1..28: mol_type = other DNA
ggcactgatataagcaaggtccggtggg

SEQ ID NO: 35302 - DNA, 28 bp, synthetic construct
  source 1..28: mol_type = other DNA
tggcactgatataagcaaggtccggtgg

SEQ ID NO: 35303 - DNA, 28 bp, synthetic construct
  source 1..28: mol_type = other DNA
gggtggcactgatataagcaaggtccgg

SEQ ID NO: 35304 - DNA, 28 bp, synthetic construct
  source 1..28: mol_type = other DNA
aatgggggtggcactgatataagcaagg

SEQ ID NO: 35305 - DNA, 28 bp, synthetic construct
  source 1..28: mol_type = other DNA
aaggagtgaaaggggacaatgggggtgg

SEQ ID NO: 35306 - DNA, 28 bp, synthetic construct
  source 1..28: mol_type = other DNA
gtaaaggagtgaaaggggacaatggggg

SEQ ID NO: 35307 - DNA, 28 bp, synthetic construct
  source 1..28: mol_type = other DNA
ggtaaaggagtgaaaggggacaatgggg

SEQ ID NO: 35308 - DNA, 28 bp, synthetic construct
  source 1..28: mol_type = other DNA
gggtaaaggagtgaaaggggacaatggg

SEQ ID NO: 35309 - DNA, 28 bp, synthetic construct
  source 1..28: mol_type = other DNA
ggggtaaaggagtgaaaggggacaatgg

SEQ ID NO: 35310 - DNA, 28 bp, synthetic construct
  source 1..28: mol_type = other DNA
tcccctttcactcctttacccctcatgg

SEQ ID NO: 35311 - DNA, 28 bp, synthetic construct
  source 1..28: mol_type = other DNA
gccatgaggggtaaaggagtgaaagggg

SEQ ID NO: 35312 - DNA, 28 bp, synthetic construct
  source 1..28: mol_type = other DNA
ggccatgaggggtaaaggagtgaaaggg

SEQ ID NO: 35313 - DNA, 28 bp, synthetic construct
  source 1..28: mol_type = other DNA
aggccatgaggggtaaaggagtgaaagg

SEQ ID NO: 35314 - DNA, 28 bp, synthetic construct
  source 1..28: mol_type = other DNA
aggagattgaggccatgaggggtaaagg

SEQ ID NO: 35315 - DNA, 28 bp, synthetic construct
  source 1..28: mol_type = other DNA
atgggaaggagattgaggccatgagggg

SEQ ID NO: 35316 - DNA, 28 bp, synthetic construct
  source 1..28: mol_type = other DNA
gatgggaaggagattgaggccatgaggg

SEQ ID NO: 35317 - DNA, 28 bp, synthetic construct
  source 1..28: mol_type = other DNA
ggatgggaaggagattgaggccatgagg

SEQ ID NO: 35318 - DNA, 28 bp, synthetic construct
  source 1..28: mol_type = other DNA
gggcacacacgtgggcaactcgtgcagg

SEQ ID NO: 35319 - DNA, 28 bp, synthetic construct
  source 1..28: mol_type = other DNA
cacgagttgcccacgtgtgtgcccttgg

SEQ ID NO: 35320 - DNA, 28 bp, synthetic construct
  source 1..28: mol_type = other DNA
tgcagggtgccaagggcacacacgtggg

SEQ ID NO: 35321 - DNA, 28 bp, synthetic construct
  source 1..28: mol_type = other DNA
gtgcagggtgccaagggcacacacgtgg

SEQ ID NO: 35322 - DNA, 28 bp, synthetic construct
  source 1..28: mol_type = other DNA
ccaggaagtgggtgcagggtgccaaggg

SEQ ID NO: 35323 - DNA, 28 bp, synthetic construct
  source 1..28: mol_type = other DNA
cccaggaagtgggtgcagggtgccaagg

SEQ ID NO: 35324 - DNA, 28 bp, synthetic construct
  source 1..28: mol_type = other DNA
caccctgcacccacttcctgggaacagg

SEQ ID NO: 35325 - DNA, 28 bp, synthetic construct
  source 1..28: mol_type = other DNA
accctgcacccacttcctgggaacaggg

SEQ ID NO: 35326 - DNA, 28 bp, synthetic construct
  source 1..28: mol_type = other DNA
cccctgttcccaggaagtgggtgcaggg

SEQ ID NO: 35327 - DNA, 28 bp, synthetic construct
  source 1..28: mol_type = other DNA
tcccctgttcccaggaagtgggtgcagg

SEQ ID NO: 35328 - DNA, 28 bp, synthetic construct
  source 1..28: mol_type = other DNA
tgcacccacttcctgggaacaggggagg

SEQ ID NO: 35329 - DNA, 28 bp, synthetic construct
  source 1..28: mol_type = other DNA
gcacccacttcctgggaacaggggaggg

SEQ ID NO: 35330 - DNA, 28 bp, synthetic construct
  source 1..28: mol_type = other DNA
cacccacttcctgggaacaggggagggg

SEQ ID NO: 35331 - DNA, 28 bp, synthetic construct
  source 1..28: mol_type = other DNA
acccacttcctgggaacaggggaggggg

SEQ ID NO: 35332 - DNA, 28 bp, synthetic construct
  source 1..28: mol_type = other DNA
accccctcccctgttcccaggaagtggg

SEQ ID NO: 35333 - DNA, 28 bp, synthetic construct
  source 1..28: mol_type = other DNA
gaccccctcccctgttcccaggaagtgg

SEQ ID NO: 35334 - DNA, 28 bp, synthetic construct
  source 1..28: mol_type = other DNA
cttcctgggaacaggggagggggtcagg

SEQ ID NO: 35335 - DNA, 28 bp, synthetic construct
  source 1..28: mol_type = other DNA
cttcctgaccccctcccctgttcccagg

SEQ ID NO: 35336 - DNA, 28 bp, synthetic construct
  source 1..28: mol_type = other DNA
gggaacaggggagggggtcaggaagagg

SEQ ID NO: 35337 - DNA, 28 bp, synthetic construct
  source 1..28: mol_type = other DNA
aacaggggagggggtcaggaagaggtgg

SEQ ID NO: 35338 - DNA, 28 bp, synthetic construct
  source 1..28: mol_type = other DNA
acaggggagggggtcaggaagaggtggg

SEQ ID NO: 35339 - DNA, 28 bp, synthetic construct
  source 1..28: mol_type = other DNA
caggggagggggtcaggaagaggtgggg

SEQ ID NO: 35340 - DNA, 28 bp, synthetic construct
  source 1..28: mol_type = other DNA
aggggagggggtcaggaagaggtggggg

SEQ ID NO: 35341 - DNA, 28 bp, synthetic construct
  source 1..28: mol_type = other DNA
ctggaggacagggaagaggggaagctgg

SEQ ID NO: 35342 - DNA, 28 bp, synthetic construct
  source 1..28: mol_type = other DNA
aggggcactggaggacagggaagagggg

SEQ ID NO: 35343 - DNA, 28 bp, synthetic construct
  source 1..28: mol_type = other DNA
caggggcactggaggacagggaagaggg

SEQ ID NO: 35344 - DNA, 28 bp, synthetic construct
  source 1..28: mol_type = other DNA
ccaggggcactggaggacagggaagagg

SEQ ID NO: 35345 - DNA, 28 bp, synthetic construct
  source 1..28: mol_type = other DNA
ctcttccctgtcctccagtgcccctggg

SEQ ID NO: 35346 - DNA, 28 bp, synthetic construct
  source 1..28: mol_type = other DNA
gggggcccaggggcactggaggacaggg

SEQ ID NO: 35347 - DNA, 28 bp, synthetic construct
  source 1..28: mol_type = other DNA
ggggggcccaggggcactggaggacagg

SEQ ID NO: 35348 - DNA, 28 bp, synthetic construct
  source 1..28: mol_type = other DNA
tctcaggggggcccaggggcactggagg

SEQ ID NO: 35349 - DNA, 28 bp, synthetic construct
  source 1..28: mol_type = other DNA
tgttctcaggggggcccaggggcactgg

SEQ ID NO: 35350 - DNA, 28 bp, synthetic construct
  source 1..28: mol_type = other DNA
cactaatgttctcaggggggcccagggg

SEQ ID NO: 35351 - DNA, 28 bp, synthetic construct
  source 1..28: mol_type = other DNA
gcactaatgttctcaggggggcccaggg

SEQ ID NO: 35352 - DNA, 28 bp, synthetic construct
  source 1..28: mol_type = other DNA
agcactaatgttctcaggggggcccagg

SEQ ID NO: 35353 - DNA, 28 bp, synthetic construct
  source 1..28: mol_type = other DNA
cccccctgagaacattagtgctacgcgg

SEQ ID NO: 35354 - DNA, 28 bp, synthetic construct
  source 1..28: mol_type = other DNA
tccgcgtagcactaatgttctcaggggg

SEQ ID NO: 35355 - DNA, 28 bp, synthetic construct
  source 1..28: mol_type = other DNA
ttccgcgtagcactaatgttctcagggg

SEQ ID NO: 35356 - DNA, 28 bp, synthetic construct
  source 1..28: mol_type = other DNA
attccgcgtagcactaatgttctcaggg

SEQ ID NO: 35357 - DNA, 28 bp, synthetic construct
  source 1..28: mol_type = other DNA
cattccgcgtagcactaatgttctcagg

SEQ ID NO: 35358 - DNA, 28 bp, synthetic construct
  source 1..28: mol_type = other DNA
ctgagaacattagtgctacgcggaatgg

SEQ ID NO: 35359 - DNA, 28 bp, synthetic construct
  source 1..28: mol_type = other DNA
tgagaacattagtgctacgcggaatggg

SEQ ID NO: 35360 - DNA, 28 bp, synthetic construct
  source 1..28: mol_type = other DNA
attagtgctacgcggaatgggagccagg

SEQ ID NO: 35361 - DNA, 28 bp, synthetic construct
  source 1..28: mol_type = other DNA
gaatgggagccaggccttcgtgcattgg

SEQ ID NO: 35362 - DNA, 28 bp, synthetic construct
  source 1..28: mol_type = other DNA
gggctcttgccaatgcacgaaggcctgg

SEQ ID NO: 35363 - DNA, 28 bp, synthetic construct
  source 1..28: mol_type = other DNA
ggccttcgtgcattggcaagagccccgg

SEQ ID NO: 35364 - DNA, 28 bp, synthetic construct
  source 1..28: mol_type = other DNA
gccttcgtgcattggcaagagccccggg

SEQ ID NO: 35365 - DNA, 28 bp, synthetic construct
  source 1..28: mol_type = other DNA
gcccggggctcttgccaatgcacgaagg

SEQ ID NO: 35366 - DNA, 28 bp, synthetic construct
  source 1..28: mol_type = other DNA
tggcaagagccccgggcgcccctgcagg

SEQ ID NO: 35367 - DNA, 28 bp, synthetic construct
  source 1..28: mol_type = other DNA
ggcaagagccccgggcgcccctgcaggg

SEQ ID NO: 35368 - DNA, 28 bp, synthetic construct
  source 1..28: mol_type = other DNA
acagggtaccctgcaggggcgcccgggg

SEQ ID NO: 35369 - DNA, 28 bp, synthetic construct
  source 1..28: mol_type = other DNA
aacagggtaccctgcaggggcgcccggg

SEQ ID NO: 35370 - DNA, 28 bp, synthetic construct
  source 1..28: mol_type = other DNA
taacagggtaccctgcaggggcgcccgg

SEQ ID NO: 35371 - DNA, 28 bp, synthetic construct
  source 1..28: mol_type = other DNA
gggcgcccctgcagggtaccctgttagg

SEQ ID NO: 35372 - DNA, 28 bp, synthetic construct
  source 1..28: mol_type = other DNA
ggcgcccctgcagggtaccctgttaggg

SEQ ID NO: 35373 - DNA, 28 bp, synthetic construct
  source 1..28: mol_type = other DNA
ggtaccctaacagggtaccctgcagggg

SEQ ID NO: 35374 - DNA, 28 bp, synthetic construct
  source 1..28: mol_type = other DNA
cggtaccctaacagggtaccctgcaggg

SEQ ID NO: 35375 - DNA, 28 bp, synthetic construct
  source 1..28: mol_type = other DNA
cctgcagggtaccctgttagggtaccgg

SEQ ID NO: 35376 - DNA, 28 bp, synthetic construct
  source 1..28: mol_type = other DNA
cagggtaccctgttagggtaccggctgg

SEQ ID NO: 35377 - DNA, 28 bp, synthetic construct
  source 1..28: mol_type = other DNA
tgatacgccagccggtaccctaacaggg

SEQ ID NO: 35378 - DNA, 28 bp, synthetic construct
  source 1..28: mol_type = other DNA
ttgatacgccagccggtaccctaacagg

SEQ ID NO: 35379 - DNA, 28 bp, synthetic construct
  source 1..28: mol_type = other DNA
tgttagggtaccggctggcgtatcaagg

SEQ ID NO: 35380 - DNA, 28 bp, synthetic construct
  source 1..28: mol_type = other DNA
gggtaccggctggcgtatcaaggccagg

SEQ ID NO: 35381 - DNA, 28 bp, synthetic construct
  source 1..28: mol_type = other DNA
ggtgtcctggccttgatacgccagccgg

SEQ ID NO: 35382 - DNA, 28 bp, synthetic construct
  source 1..28: mol_type = other DNA
gcgtatcaaggccaggacaccccagagg

SEQ ID NO: 35383 - DNA, 28 bp, synthetic construct
  source 1..28: mol_type = other DNA
tatcaaggccaggacaccccagaggtgg

SEQ ID NO: 35384 - DNA, 28 bp, synthetic construct
  source 1..28: mol_type = other DNA
atcaaggccaggacaccccagaggtggg

SEQ ID NO: 35385 - DNA, 28 bp, synthetic construct
  source 1..28: mol_type = other DNA
agcagcacccacctctggggtgtcctgg

SEQ ID NO: 35386 - DNA, 28 bp, synthetic construct
  source 1..28: mol_type = other DNA
aggacaccccagaggtgggtgctgctgg

SEQ ID NO: 35387 - DNA, 28 bp, synthetic construct
  source 1..28: mol_type = other DNA
acaccccagaggtgggtgctgctggtgg

SEQ ID NO: 35388 - DNA, 28 bp, synthetic construct
  source 1..28: mol_type = other DNA
caccccagaggtgggtgctgctggtggg

SEQ ID NO: 35389 - DNA, 28 bp, synthetic construct
  source 1..28: mol_type = other DNA
atcccaccagcagcacccacctctgggg

SEQ ID NO: 35390 - DNA, 28 bp, synthetic construct
  source 1..28: mol_type = other DNA
aatcccaccagcagcacccacctctggg

SEQ ID NO: 35391 - DNA, 28 bp, synthetic construct
  source 1..28: mol_type = other DNA
caatcccaccagcagcacccacctctgg

SEQ ID NO: 35392 - DNA, 28 bp, synthetic construct
  source 1..28: mol_type = other DNA
cagaggtgggtgctgctggtgggattgg

SEQ ID NO: 35393 - DNA, 28 bp, synthetic construct
  source 1..28: mol_type = other DNA
gtgggtgctgctggtgggattggagtgg

SEQ ID NO: 35394 - DNA, 28 bp, synthetic construct
  source 1..28: mol_type = other DNA
tgctgctggtgggattggagtggagtgg

SEQ ID NO: 35395 - DNA, 28 bp, synthetic construct
  source 1..28: mol_type = other DNA
ctggtgggattggagtggagtggcttgg

SEQ ID NO: 35396 - DNA, 28 bp, synthetic construct
  source 1..28: mol_type = other DNA
tggtgggattggagtggagtggcttggg

SEQ ID NO: 35397 - DNA, 28 bp, synthetic construct
  source 1..28: mol_type = other DNA
ggtgggattggagtggagtggcttgggg

SEQ ID NO: 35398 - DNA, 28 bp, synthetic construct
  source 1..28: mol_type = other DNA
gggattggagtggagtggcttggggagg

SEQ ID NO: 35399 - DNA, 28 bp, synthetic construct
  source 1..28: mol_type = other DNA
attggagtggagtggcttggggaggagg

SEQ ID NO: 35400 - DNA, 28 bp, synthetic construct
  source 1..28: mol_type = other DNA
ttggagtggagtggcttggggaggaggg

SEQ ID NO: 35401 - DNA, 28 bp, synthetic construct
  source 1..28: mol_type = other DNA
gagtggagtggcttggggaggagggagg

SEQ ID NO: 35402 - DNA, 28 bp, synthetic construct
  source 1..28: mol_type = other DNA
tggggaggagggaggagaacatatcagg

SEQ ID NO: 35403 - DNA, 28 bp, synthetic construct
  source 1..28: mol_type = other DNA
ggggaggagggaggagaacatatcaggg

SEQ ID NO: 35404 - DNA, 28 bp, synthetic construct
  source 1..28: mol_type = other DNA
gagaacatatcagggcagacatagatgg

SEQ ID NO: 35405 - DNA, 28 bp, synthetic construct
  source 1..28: mol_type = other DNA
tcagggcagacatagatggttgtgaagg

SEQ ID NO: 35406 - DNA, 28 bp, synthetic construct
  source 1..28: mol_type = other DNA
ggcagacatagatggttgtgaaggttgg

SEQ ID NO: 35407 - DNA, 28 bp, synthetic construct
  source 1..28: mol_type = other DNA
gcagacatagatggttgtgaaggttggg

SEQ ID NO: 35408 - DNA, 28 bp, synthetic construct
  source 1..28: mol_type = other DNA
ggtagtacacaattgctctatgcctagg

SEQ ID NO: 35409 - DNA, 28 bp, synthetic construct
  source 1..28: mol_type = other DNA
gtagtacacaattgctctatgcctaggg

SEQ ID NO: 35410 - DNA, 28 bp, synthetic construct
  source 1..28: mol_type = other DNA
tagtacacaattgctctatgcctagggg

SEQ ID NO: 35411 - DNA, 28 bp, synthetic construct
  source 1..28: mol_type = other DNA
agtacacaattgctctatgcctaggggg

SEQ ID NO: 35412 - DNA, 28 bp, synthetic construct
  source 1..28: mol_type = other DNA
aggaaggatgaggagttggaggatgggg

SEQ ID NO: 35413 - DNA, 28 bp, synthetic construct
  source 1..28: mol_type = other DNA
tggggagagcgttttgagaaagagatgg

SEQ ID NO: 35414 - DNA, 28 bp, synthetic construct
  source 1..28: mol_type = other DNA
ggggagagcgttttgagaaagagatggg

SEQ ID NO: 35415 - DNA, 28 bp, synthetic construct
  source 1..28: mol_type = other DNA
gggagagcgttttgagaaagagatgggg

SEQ ID NO: 35416 - DNA, 28 bp, synthetic construct
  source 1..28: mol_type = other DNA
gatggggcattgagcccgagagtgaagg

SEQ ID NO: 35417 - DNA, 28 bp, synthetic construct
  source 1..28: mol_type = other DNA
agcccgagagtgaaggcttaacagctgg

SEQ ID NO: 35418 - DNA, 28 bp, synthetic construct
  source 1..28: mol_type = other DNA
gcccgagagtgaaggcttaacagctggg

SEQ ID NO: 35419 - DNA, 28 bp, synthetic construct
  source 1..28: mol_type = other DNA
ccccagctgttaagccttcactctcggg

SEQ ID NO: 35420 - DNA, 28 bp, synthetic construct
  source 1..28: mol_type = other DNA
ccgagagtgaaggcttaacagctggggg

SEQ ID NO: 35421 - DNA, 28 bp, synthetic construct
  source 1..28: mol_type = other DNA
cgagagtgaaggcttaacagctgggggg

SEQ ID NO: 35422 - DNA, 28 bp, synthetic construct
  source 1..28: mol_type = other DNA
gtgaaggcttaacagctggggggtaagg

SEQ ID NO: 35423 - DNA, 28 bp, synthetic construct
  source 1..28: mol_type = other DNA
taaggttctaccctgatgccacttctgg

SEQ ID NO: 35424 - DNA, 28 bp, synthetic construct
  source 1..28: mol_type = other DNA
ccctgatgccacttctggacctcctagg

SEQ ID NO: 35425 - DNA, 28 bp, synthetic construct
  source 1..28: mol_type = other DNA
acctaggaggtccagaagtggcatcagg

SEQ ID NO: 35426 - DNA, 28 bp, synthetic construct
  source 1..28: mol_type = other DNA
cattagcacctaggaggtccagaagtgg

SEQ ID NO: 35427 - DNA, 28 bp, synthetic construct
  source 1..28: mol_type = other DNA
cacttctggacctcctaggtgctaatgg

SEQ ID NO: 35428 - DNA, 28 bp, synthetic construct
  source 1..28: mol_type = other DNA
ggacctcctaggtgctaatggacatagg

SEQ ID NO: 35429 - DNA, 28 bp, synthetic construct
  source 1..28: mol_type = other DNA
gacctcctaggtgctaatggacataggg

SEQ ID NO: 35430 - DNA, 28 bp, synthetic construct
  source 1..28: mol_type = other DNA
agccctatgtccattagcacctaggagg

SEQ ID NO: 35431 - DNA, 28 bp, synthetic construct
  source 1..28: mol_type = other DNA
cttagccctatgtccattagcacctagg

SEQ ID NO: 35432 - DNA, 28 bp, synthetic construct
  source 1..28: mol_type = other DNA
ctaggtgctaatggacatagggctaagg

SEQ ID NO: 35433 - DNA, 28 bp, synthetic construct
  source 1..28: mol_type = other DNA
ctaatggacatagggctaaggcaagagg

SEQ ID NO: 35434 - DNA, 28 bp, synthetic construct
  source 1..28: mol_type = other DNA
atagggctaaggcaagaggtgaccctgg

SEQ ID NO: 35435 - DNA, 28 bp, synthetic construct
  source 1..28: mol_type = other DNA
aggcaagaggtgaccctggagctgcagg

SEQ ID NO: 35436 - DNA, 28 bp, synthetic construct
  source 1..28: mol_type = other DNA
ggcaagaggtgaccctggagctgcaggg

SEQ ID NO: 35437 - DNA, 28 bp, synthetic construct
  source 1..28: mol_type = other DNA
gcaagaggtgaccctggagctgcagggg

SEQ ID NO: 35438 - DNA, 28 bp, synthetic construct
  source 1..28: mol_type = other DNA
caagaggtgaccctggagctgcaggggg

SEQ ID NO: 35439 - DNA, 28 bp, synthetic construct
  source 1..28: mol_type = other DNA
aggtgaccctggagctgcagggggacgg

SEQ ID NO: 35440 - DNA, 28 bp, synthetic construct
  source 1..28: mol_type = other DNA
ggtgaccctggagctgcagggggacggg

SEQ ID NO: 35441 - DNA, 28 bp, synthetic construct
  source 1..28: mol_type = other DNA
acagacccgtccccctgcagctccaggg

SEQ ID NO: 35442 - DNA, 28 bp, synthetic construct
  source 1..28: mol_type = other DNA
cacagacccgtccccctgcagctccagg

SEQ ID NO: 35443 - DNA, 28 bp, synthetic construct
  source 1..28: mol_type = other DNA
tctgtgtccaatctgacagtgtgtgtgg

SEQ ID NO: 35444 - DNA, 28 bp, synthetic construct
  source 1..28: mol_type = other DNA
taggctgccacacacactgtcagattgg

SEQ ID NO: 35445 - DNA, 28 bp, synthetic construct
  source 1..28: mol_type = other DNA
tgtgtgtggcagcctacactgctgctgg

SEQ ID NO: 35446 - DNA, 28 bp, synthetic construct
  source 1..28: mol_type = other DNA
gtgtgtggcagcctacactgctgctggg

SEQ ID NO: 35447 - DNA, 28 bp, synthetic construct
  source 1..28: mol_type = other DNA
tgtgtggcagcctacactgctgctgggg

SEQ ID NO: 35448 - DNA, 28 bp, synthetic construct
  source 1..28: mol_type = other DNA
tggcagcctacactgctgctggggatgg

SEQ ID NO: 35449 - DNA, 28 bp, synthetic construct
  source 1..28: mol_type = other DNA
cagggtccatccccagcagcagtgtagg

SEQ ID NO: 35450 - DNA, 28 bp, synthetic construct
  source 1..28: mol_type = other DNA
ctacactgctgctggggatggaccctgg

SEQ ID NO: 35451 - DNA, 28 bp, synthetic construct
  source 1..28: mol_type = other DNA
ggaccctggagcctcccagtacccctgg

SEQ ID NO: 35452 - DNA, 28 bp, synthetic construct
  source 1..28: mol_type = other DNA
ccctggagcctcccagtacccctggagg

SEQ ID NO: 35453 - DNA, 28 bp, synthetic construct
  source 1..28: mol_type = other DNA
gcctccaggggtactgggaggctccagg

SEQ ID NO: 35454 - DNA, 28 bp, synthetic construct
  source 1..28: mol_type = other DNA
gagcctcccagtacccctggaggcctgg

SEQ ID NO: 35455 - DNA, 28 bp, synthetic construct
  source 1..28: mol_type = other DNA
gcgccaggcctccaggggtactgggagg

SEQ ID NO: 35456 - DNA, 28 bp, synthetic construct
  source 1..28: mol_type = other DNA
tgggcgccaggcctccaggggtactggg

SEQ ID NO: 35457 - DNA, 28 bp, synthetic construct
  source 1..28: mol_type = other DNA
ctgggcgccaggcctccaggggtactgg

SEQ ID NO: 35458 - DNA, 28 bp, synthetic construct
  source 1..28: mol_type = other DNA
cagtacccctggaggcctggcgcccagg

SEQ ID NO: 35459 - DNA, 28 bp, synthetic construct
  source 1..28: mol_type = other DNA
acttacctgggcgccaggcctccagggg

SEQ ID NO: 35460 - DNA, 28 bp, synthetic construct
  source 1..28: mol_type = other DNA
gacttacctgggcgccaggcctccaggg

SEQ ID NO: 35461 - DNA, 28 bp, synthetic construct
  source 1..28: mol_type = other DNA
ggacttacctgggcgccaggcctccagg

SEQ ID NO: 35462 - DNA, 28 bp, synthetic construct
  source 1..28: mol_type = other DNA
atggctttggacttacctgggcgccagg

SEQ ID NO: 35463 - DNA, 28 bp, synthetic construct
  source 1..28: mol_type = other DNA
gttgggcatggctttggacttacctggg

SEQ ID NO: 35464 - DNA, 28 bp, synthetic construct
  source 1..28: mol_type = other DNA
ggttgggcatggctttggacttacctgg

SEQ ID NO: 35465 - DNA, 28 bp, synthetic construct
  source 1..28: mol_type = other DNA
ggttgaagcaggttgggcatggctttgg

SEQ ID NO: 35466 - DNA, 28 bp, synthetic construct
  source 1..28: mol_type = other DNA
agacagggttgaagcaggttgggcatgg

SEQ ID NO: 35467 - DNA, 28 bp, synthetic construct
  source 1..28: mol_type = other DNA
gggagagacagggttgaagcaggttggg

SEQ ID NO: 35468 - DNA, 28 bp, synthetic construct
  source 1..28: mol_type = other DNA
agggagagacagggttgaagcaggttgg

SEQ ID NO: 35469 - DNA, 28 bp, synthetic construct
  source 1..28: mol_type = other DNA
tgtcagggagagacagggttgaagcagg

SEQ ID NO: 35470 - DNA, 28 bp, synthetic construct
  source 1..28: mol_type = other DNA
aagtcagggctgtcagggagagacaggg

SEQ ID NO: 35471 - DNA, 28 bp, synthetic construct
  source 1..28: mol_type = other DNA
taagtcagggctgtcagggagagacagg

SEQ ID NO: 35472 - DNA, 28 bp, synthetic construct
  source 1..28: mol_type = other DNA
tacaaggagtaagtcagggctgtcaggg

SEQ ID NO: 35473 - DNA, 28 bp, synthetic construct
  source 1..28: mol_type = other DNA
gtacaaggagtaagtcagggctgtcagg

SEQ ID NO: 35474 - DNA, 28 bp, synthetic construct
  source 1..28: mol_type = other DNA
actgaaaggtacaaggagtaagtcaggg

SEQ ID NO: 35475 - DNA, 28 bp, synthetic construct
  source 1..28: mol_type = other DNA
cactgaaaggtacaaggagtaagtcagg

SEQ ID NO: 35476 - DNA, 28 bp, synthetic construct
  source 1..28: mol_type = other DNA
agttgcggtaacactgaaaggtacaagg

SEQ ID NO: 35477 - DNA, 28 bp, synthetic construct
  source 1..28: mol_type = other DNA
gtacctttcagtgttaccgcaacttagg

SEQ ID NO: 35478 - DNA, 28 bp, synthetic construct
  source 1..28: mol_type = other DNA
gggcctaagttgcggtaacactgaaagg

SEQ ID NO: 35479 - DNA, 28 bp, synthetic construct
  source 1..28: mol_type = other DNA
cagggtaggaacagggcctaagttgcgg

SEQ ID NO: 35480 - DNA, 28 bp, synthetic construct
  source 1..28: mol_type = other DNA
ctcagtaaggctcagggtaggaacaggg

SEQ ID NO: 35481 - DNA, 28 bp, synthetic construct
  source 1..28: mol_type = other DNA
tctcagtaaggctcagggtaggaacagg

SEQ ID NO: 35482 - DNA, 28 bp, synthetic construct
  source 1..28: mol_type = other DNA
gggtgtggcacgagtaagggagtgaagg

SEQ ID NO: 35483 - DNA, 28 bp, synthetic construct
  source 1..28: mol_type = other DNA
gggagtgagggtgtggcacgagtaaggg

SEQ ID NO: 35484 - DNA, 28 bp, synthetic construct
  source 1..28: mol_type = other DNA
agggagtgagggtgtggcacgagtaagg

SEQ ID NO: 35485 - DNA, 28 bp, synthetic construct
  source 1..28: mol_type = other DNA
tggcacgggtaagggagtgagggtgtgg

SEQ ID NO: 35486 - DNA, 28 bp, synthetic construct
  source 1..28: mol_type = other DNA
gggtgtggcacgggtaagggagtgaggg

SEQ ID NO: 35487 - DNA, 28 bp, synthetic construct
  source 1..28: mol_type = other DNA
agggtgtggcacgggtaagggagtgagg

SEQ ID NO: 35488 - DNA, 28 bp, synthetic construct
  source 1..28: mol_type = other DNA
gggagtaagggtgtggcacgggtaaggg

SEQ ID NO: 35489 - DNA, 28 bp, synthetic construct
  source 1..28: mol_type = other DNA
agggagtaagggtgtggcacgggtaagg

SEQ ID NO: 35490 - DNA, 28 bp, synthetic construct
  source 1..28: mol_type = other DNA
gggtaagggagtaagggtgtggcacggg

SEQ ID NO: 35491 - DNA, 28 bp, synthetic construct
  source 1..28: mol_type = other DNA
cgggtaagggagtaagggtgtggcacgg

SEQ ID NO: 35492 - DNA, 28 bp, synthetic construct
  source 1..28: mol_type = other DNA
tggcacgggtaagggagtaagggtgtgg

SEQ ID NO: 35493 - DNA, 28 bp, synthetic construct
  source 1..28: mol_type = other DNA
tggcgtggcacgggtaagggagtaaggg

SEQ ID NO: 35494 - DNA, 28 bp, synthetic construct
  source 1..28: mol_type = other DNA
ctggcgtggcacgggtaagggagtaagg

SEQ ID NO: 35495 - DNA, 28 bp, synthetic construct
  source 1..28: mol_type = other DNA
gacaagactggcgtggcacgggtaaggg

SEQ ID NO: 35496 - DNA, 28 bp, synthetic construct
  source 1..28: mol_type = other DNA
ggacaagactggcgtggcacgggtaagg

SEQ ID NO: 35497 - DNA, 28 bp, synthetic construct
  source 1..28: mol_type = other DNA
agagaggacaagactggcgtggcacggg

SEQ ID NO: 35498 - DNA, 28 bp, synthetic construct
  source 1..28: mol_type = other DNA
cagagaggacaagactggcgtggcacgg

SEQ ID NO: 35499 - DNA, 28 bp, synthetic construct
  source 1..28: mol_type = other DNA
gtgctcagagaggacaagactggcgtgg

SEQ ID NO: 35500 - DNA, 28 bp, synthetic construct
  source 1..28: mol_type = other DNA
gagatgtgctcagagaggacaagactgg

SEQ ID NO: 35501 - DNA, 28 bp, synthetic construct
  source 1..28: mol_type = other DNA
ggacagagaggagatgtgctcagagagg

SEQ ID NO: 35502 - DNA, 28 bp, synthetic construct
  source 1..28: mol_type = other DNA
tctcctctctgtcctttcttctcacagg

SEQ ID NO: 35503 - DNA, 28 bp, synthetic construct
  source 1..28: mol_type = other DNA
ctcctctctgtcctttcttctcacaggg

SEQ ID NO: 35504 - DNA, 28 bp, synthetic construct
  source 1..28: mol_type = other DNA
tgccctgtgagaagaaaggacagagagg

SEQ ID NO: 35505 - DNA, 28 bp, synthetic construct
  source 1..28: mol_type = other DNA
ggctgtgcttgccctgtgagaagaaagg

SEQ ID NO: 35506 - DNA, 28 bp, synthetic construct
  source 1..28: mol_type = other DNA
gggcaagcacagccagtccaccagctgg

SEQ ID NO: 35507 - DNA, 28 bp, synthetic construct
  source 1..28: mol_type = other DNA
ggcaagcacagccagtccaccagctggg

SEQ ID NO: 35508 - DNA, 28 bp, synthetic construct
  source 1..28: mol_type = other DNA
gcacagccagtccaccagctgggtaagg

SEQ ID NO: 35509 - DNA, 28 bp, synthetic construct
  source 1..28: mol_type = other DNA
cacagccagtccaccagctgggtaaggg

SEQ ID NO: 35510 - DNA, 28 bp, synthetic construct
  source 1..28: mol_type = other DNA
ggaagcccttacccagctggtggactgg

SEQ ID NO: 35511 - DNA, 28 bp, synthetic construct
  source 1..28: mol_type = other DNA
ggtgtggaagcccttacccagctggtgg

SEQ ID NO: 35512 - DNA, 28 bp, synthetic construct
  source 1..28: mol_type = other DNA
tggggtgtggaagcccttacccagctgg

SEQ ID NO: 35513 - DNA, 28 bp, synthetic construct
  source 1..28: mol_type = other DNA
gggtagggaaggaggagatggggtgtgg

SEQ ID NO: 35514 - DNA, 28 bp, synthetic construct
  source 1..28: mol_type = other DNA
gttgagggtagggaaggaggagatgggg

SEQ ID NO: 35515 - DNA, 28 bp, synthetic construct
  source 1..28: mol_type = other DNA
tgttgagggtagggaaggaggagatggg

SEQ ID NO: 35516 - DNA, 28 bp, synthetic construct
  source 1..28: mol_type = other DNA
gtgttgagggtagggaaggaggagatgg

SEQ ID NO: 35517 - DNA, 28 bp, synthetic construct
  source 1..28: mol_type = other DNA
cactaggtgttgagggtagggaaggagg

SEQ ID NO: 35518 - DNA, 28 bp, synthetic construct
  source 1..28: mol_type = other DNA
ctccttccctaccctcaacacctagtgg

SEQ ID NO: 35519 - DNA, 28 bp, synthetic construct
  source 1..28: mol_type = other DNA
tccttccctaccctcaacacctagtggg

SEQ ID NO: 35520 - DNA, 28 bp, synthetic construct
  source 1..28: mol_type = other DNA
ccttccctaccctcaacacctagtgggg

SEQ ID NO: 35521 - DNA, 28 bp, synthetic construct
  source 1..28: mol_type = other DNA
cttccctaccctcaacacctagtggggg

SEQ ID NO: 35522 - DNA, 28 bp, synthetic construct
  source 1..28: mol_type = other DNA
gtgcccccactaggtgttgagggtaggg

SEQ ID NO: 35523 - DNA, 28 bp, synthetic construct
  source 1..28: mol_type = other DNA
agtgcccccactaggtgttgagggtagg

SEQ ID NO: 35524 - DNA, 28 bp, synthetic construct
  source 1..28: mol_type = other DNA
tgacagtgcccccactaggtgttgaggg

SEQ ID NO: 35525 - DNA, 28 bp, synthetic construct
  source 1..28: mol_type = other DNA
gtgacagtgcccccactaggtgttgagg

SEQ ID NO: 35526 - DNA, 28 bp, synthetic construct
  source 1..28: mol_type = other DNA
tatgcatggtgacagtgcccccactagg

SEQ ID NO: 35527 - DNA, 28 bp, synthetic construct
  source 1..28: mol_type = other DNA
gaaagggatgtgcaatgagtatgcatgg

SEQ ID NO: 35528 - DNA, 28 bp, synthetic construct
  source 1..28: mol_type = other DNA
agtgatgagttagagaaacatgaaaggg

SEQ ID NO: 35529 - DNA, 28 bp, synthetic construct
  source 1..28: mol_type = other DNA
gagtgatgagttagagaaacatgaaagg

SEQ ID NO: 35530 - DNA, 28 bp, synthetic construct
  source 1..28: mol_type = other DNA
ggcaaagatgtgcacatacttgatgagg

SEQ ID NO: 35531 - DNA, 28 bp, synthetic construct
  source 1..28: mol_type = other DNA
atcaagtatgtgcacatctttgccgagg

SEQ ID NO: 35532 - DNA, 28 bp, synthetic construct
  source 1..28: mol_type = other DNA
gatgtgggagggaggcagaaggcctcgg

SEQ ID NO: 35533 - DNA, 28 bp, synthetic construct
  source 1..28: mol_type = other DNA
aggggtgatgtgggagggaggcagaagg

SEQ ID NO: 35534 - DNA, 28 bp, synthetic construct
  source 1..28: mol_type = other DNA
ctgcctccctcccacatcacccctttgg

SEQ ID NO: 35535 - DNA, 28 bp, synthetic construct
  source 1..28: mol_type = other DNA
tgcctccctcccacatcacccctttggg

SEQ ID NO: 35536 - DNA, 28 bp, synthetic construct
  source 1..28: mol_type = other DNA
gacccaaaggggtgatgtgggagggagg

SEQ ID NO: 35537 - DNA, 28 bp, synthetic construct
  source 1..28: mol_type = other DNA
tgggacccaaaggggtgatgtgggaggg

SEQ ID NO: 35538 - DNA, 28 bp, synthetic construct
  source 1..28: mol_type = other DNA
ctgggacccaaaggggtgatgtgggagg

SEQ ID NO: 35539 - DNA, 28 bp, synthetic construct
  source 1..28: mol_type = other DNA
tctctgggacccaaaggggtgatgtggg

SEQ ID NO: 35540 - DNA, 28 bp, synthetic construct
  source 1..28: mol_type = other DNA
ctctctgggacccaaaggggtgatgtgg

SEQ ID NO: 35541 - DNA, 28 bp, synthetic construct
  source 1..28: mol_type = other DNA
atcacccctttgggtcccagagagctgg

SEQ ID NO: 35542 - DNA, 28 bp, synthetic construct
  source 1..28: mol_type = other DNA
ggatccagctctctgggacccaaagggg

SEQ ID NO: 35543 - DNA, 28 bp, synthetic construct
  source 1..28: mol_type = other DNA
tggatccagctctctgggacccaaaggg

SEQ ID NO: 35544 - DNA, 28 bp, synthetic construct
  source 1..28: mol_type = other DNA
ttggatccagctctctgggacccaaagg

SEQ ID NO: 35545 - DNA, 28 bp, synthetic construct
  source 1..28: mol_type = other DNA
tttgggtcccagagagctggatccaagg

SEQ ID NO: 35546 - DNA, 28 bp, synthetic construct
  source 1..28: mol_type = other DNA
gatgaagccttggatccagctctctggg

SEQ ID NO: 35547 - DNA, 28 bp, synthetic construct
  source 1..28: mol_type = other DNA
ggatgaagccttggatccagctctctgg

SEQ ID NO: 35548 - DNA, 28 bp, synthetic construct
  source 1..28: mol_type = other DNA
gaggaacaggtcatggatgaagccttgg

SEQ ID NO: 35549 - DNA, 28 bp, synthetic construct
  source 1..28: mol_type = other DNA
atcagggggtatgaggaacaggtcatgg

SEQ ID NO: 35550 - DNA, 28 bp, synthetic construct
  source 1..28: mol_type = other DNA
ttcactatcagggggtatgaggaacagg

SEQ ID NO: 35551 - DNA, 28 bp, synthetic construct
  source 1..28: mol_type = other DNA
tgttcctcataccccctgatagtgaagg

SEQ ID NO: 35552 - DNA, 28 bp, synthetic construct
  source 1..28: mol_type = other DNA
ggttccttcactatcagggggtatgagg

SEQ ID NO: 35553 - DNA, 28 bp, synthetic construct
  source 1..28: mol_type = other DNA
agttgaaggttccttcactatcaggggg

SEQ ID NO: 35554 - DNA, 28 bp, synthetic construct
  source 1..28: mol_type = other DNA
gagttgaaggttccttcactatcagggg

SEQ ID NO: 35555 - DNA, 28 bp, synthetic construct
  source 1..28: mol_type = other DNA
ggagttgaaggttccttcactatcaggg

SEQ ID NO: 35556 - DNA, 28 bp, synthetic construct
  source 1..28: mol_type = other DNA
aggagttgaaggttccttcactatcagg

SEQ ID NO: 35557 - DNA, 28 bp, synthetic construct
  source 1..28: mol_type = other DNA
ggaaccttcaactcctgccttctcgtgg

SEQ ID NO: 35558 - DNA, 28 bp, synthetic construct
  source 1..28: mol_type = other DNA
agggccacgagaaggcaggagttgaagg

SEQ ID NO: 35559 - DNA, 28 bp, synthetic construct
  source 1..28: mol_type = other DNA
ttcaactcctgccttctcgtggccctgg

SEQ ID NO: 35560 - DNA, 28 bp, synthetic construct
  source 1..28: mol_type = other DNA
aactcctgccttctcgtggccctggtgg

SEQ ID NO: 35561 - DNA, 28 bp, synthetic construct
  source 1..28: mol_type = other DNA
cataccaccagggccacgagaaggcagg

SEQ ID NO: 35562 - DNA, 28 bp, synthetic construct
  source 1..28: mol_type = other DNA
agtacataccaccagggccacgagaagg

SEQ ID NO: 35563 - DNA, 28 bp, synthetic construct
  source 1..28: mol_type = other DNA
cgtggccctggtggtatgtactgctagg

SEQ ID NO: 35564 - DNA, 28 bp, synthetic construct
  source 1..28: mol_type = other DNA
ctgctcctagcagtacataccaccaggg

SEQ ID NO: 35565 - DNA, 28 bp, synthetic construct
  source 1..28: mol_type = other DNA
actgctcctagcagtacataccaccagg

SEQ ID NO: 35566 - DNA, 28 bp, synthetic construct
  source 1..28: mol_type = other DNA
tggtatgtactgctaggagcagtcgtgg

SEQ ID NO: 35567 - DNA, 28 bp, synthetic construct
  source 1..28: mol_type = other DNA
gtggccgctgcctgtgtcctcatcttgg

SEQ ID NO: 35568 - DNA, 28 bp, synthetic construct
  source 1..28: mol_type = other DNA
agagccaagatgaggacacaggcagcgg

SEQ ID NO: 35569 - DNA, 28 bp, synthetic construct
  source 1..28: mol_type = other DNA
aggaagagagccaagatgaggacacagg

SEQ ID NO: 35570 - DNA, 28 bp, synthetic construct
  source 1..28: mol_type = other DNA
gtggacaaggaagagagccaagatgagg

SEQ ID NO: 35571 - DNA, 28 bp, synthetic construct
  source 1..28: mol_type = other DNA
catcttggctctcttccttgtccaccgg

SEQ ID NO: 35572 - DNA, 28 bp, synthetic construct
  source 1..28: mol_type = other DNA
ctcttccttgtccaccggcgaaagaagg

SEQ ID NO: 35573 - DNA, 28 bp, synthetic construct
  source 1..28: mol_type = other DNA
ggtctccttctttcgccggtggacaagg

SEQ ID NO: 35574 - DNA, 28 bp, synthetic construct
  source 1..28: mol_type = other DNA
ataacgggtctccttctttcgccggtgg

SEQ ID NO: 35575 - DNA, 28 bp, synthetic construct
  source 1..28: mol_type = other DNA
accggcgaaagaaggagacccgttatgg

SEQ ID NO: 35576 - DNA, 28 bp, synthetic construct
  source 1..28: mol_type = other DNA
ccggcgaaagaaggagacccgttatggg

SEQ ID NO: 35577 - DNA, 28 bp, synthetic construct
  source 1..28: mol_type = other DNA
agaaggagacccgttatgggtgagttgg

SEQ ID NO: 35578 - DNA, 28 bp, synthetic construct
  source 1..28: mol_type = other DNA
catgtggttccaactcacccataacggg

SEQ ID NO: 35579 - DNA, 28 bp, synthetic construct
  source 1..28: mol_type = other DNA
ccgttatgggtgagttggaaccacatgg

SEQ ID NO: 35580 - DNA, 28 bp, synthetic construct
  source 1..28: mol_type = other DNA
cgttatgggtgagttggaaccacatggg

SEQ ID NO: 35581 - DNA, 28 bp, synthetic construct
  source 1..28: mol_type = other DNA
gttatgggtgagttggaaccacatgggg

SEQ ID NO: 35582 - DNA, 28 bp, synthetic construct
  source 1..28: mol_type = other DNA
atgggtgagttggaaccacatggggagg

SEQ ID NO: 35583 - DNA, 28 bp, synthetic construct
  source 1..28: mol_type = other DNA
gttggaaccacatggggaggctgtgtgg

SEQ ID NO: 35584 - DNA, 28 bp, synthetic construct
  source 1..28: mol_type = other DNA
aaccacatggggaggctgtgtggcctgg

SEQ ID NO: 35585 - DNA, 28 bp, synthetic construct
  source 1..28: mol_type = other DNA
accacatggggaggctgtgtggcctggg

SEQ ID NO: 35586 - DNA, 28 bp, synthetic construct
  source 1..28: mol_type = other DNA
tcccaggccacacagcctccccatgtgg

SEQ ID NO: 35587 - DNA, 28 bp, synthetic construct
  source 1..28: mol_type = other DNA
catggggaggctgtgtggcctgggatgg

SEQ ID NO: 35588 - DNA, 28 bp, synthetic construct
  source 1..28: mol_type = other DNA
ggaggctgtgtggcctgggatggagagg

SEQ ID NO: 35589 - DNA, 28 bp, synthetic construct
  source 1..28: mol_type = other DNA
gctgtgtggcctgggatggagaggctgg

SEQ ID NO: 35590 - DNA, 28 bp, synthetic construct
  source 1..28: mol_type = other DNA
gtgtggcctgggatggagaggctggagg

SEQ ID NO: 35591 - DNA, 28 bp, synthetic construct
  source 1..28: mol_type = other DNA
ggcctgggatggagaggctggaggcagg

SEQ ID NO: 35592 - DNA, 28 bp, synthetic construct
  source 1..28: mol_type = other DNA
gcctgggatggagaggctggaggcaggg

SEQ ID NO: 35593 - DNA, 28 bp, synthetic construct
  source 1..28: mol_type = other DNA
tccctgcctccagcctctccatcccagg

SEQ ID NO: 35594 - DNA, 28 bp, synthetic construct
  source 1..28: mol_type = other DNA
tgggatggagaggctggaggcagggagg

SEQ ID NO: 35595 - DNA, 28 bp, synthetic construct
  source 1..28: mol_type = other DNA
gaggctggaggcagggaggccagtgagg

SEQ ID NO: 35596 - DNA, 28 bp, synthetic construct
  source 1..28: mol_type = other DNA
gctggaggcagggaggccagtgaggagg

SEQ ID NO: 35597 - DNA, 28 bp, synthetic construct
  source 1..28: mol_type = other DNA
gaggcagggaggccagtgaggaggctgg

SEQ ID NO: 35598 - DNA, 28 bp, synthetic construct
  source 1..28: mol_type = other DNA
gggaggccagtgaggaggctggtgcagg

SEQ ID NO: 35599 - DNA, 28 bp, synthetic construct
  source 1..28: mol_type = other DNA
aggccagtgaggaggctggtgcaggagg

SEQ ID NO: 35600 - DNA, 28 bp, synthetic construct
  source 1..28: mol_type = other DNA
actcctcctgcaccagcctcctcactgg

SEQ ID NO: 35601 - DNA, 28 bp, synthetic construct
  source 1..28: mol_type = other DNA
ggagtgatgactaagaatcagaatgagg

SEQ ID NO: 35602 - DNA, 28 bp, synthetic construct
  source 1..28: mol_type = other DNA
gagtgatgactaagaatcagaatgaggg

SEQ ID NO: 35603 - DNA, 28 bp, synthetic construct
  source 1..28: mol_type = other DNA
atgactaagaatcagaatgagggcaagg

SEQ ID NO: 35604 - DNA, 28 bp, synthetic construct
  source 1..28: mol_type = other DNA
tgactaagaatcagaatgagggcaaggg

SEQ ID NO: 35605 - DNA, 28 bp, synthetic construct
  source 1..28: mol_type = other DNA
ctcagcaaatgttagcacagagggcagg

SEQ ID NO: 35606 - DNA, 28 bp, synthetic construct
  source 1..28: mol_type = other DNA
gcaaatgttagcacagagggcaggcagg

SEQ ID NO: 35607 - DNA, 28 bp, synthetic construct
  source 1..28: mol_type = other DNA
caaatgttagcacagagggcaggcaggg

SEQ ID NO: 35608 - DNA, 28 bp, synthetic construct
  source 1..28: mol_type = other DNA
tagcacagagggcaggcagggcttgagg

SEQ ID NO: 35609 - DNA, 28 bp, synthetic construct
  source 1..28: mol_type = other DNA
gggcaggcagggcttgaggctgagatgg

SEQ ID NO: 35610 - DNA, 28 bp, synthetic construct
  source 1..28: mol_type = other DNA
gctgagatggtgcttgctcaactgctgg

SEQ ID NO: 35611 - DNA, 28 bp, synthetic construct
  source 1..28: mol_type = other DNA
gtgcttgctcaactgctggttgagtagg

SEQ ID NO: 35612 - DNA, 28 bp, synthetic construct
  source 1..28: mol_type = other DNA
tgcttgctcaactgctggttgagtaggg

SEQ ID NO: 35613 - DNA, 28 bp, synthetic construct
  source 1..28: mol_type = other DNA
gcttgctcaactgctggttgagtagggg

SEQ ID NO: 35614 - DNA, 28 bp, synthetic construct
  source 1..28: mol_type = other DNA
cttgctcaactgctggttgagtaggggg

SEQ ID NO: 35615 - DNA, 28 bp, synthetic construct
  source 1..28: mol_type = other DNA
tgctggttgagtagggggttccacatgg

SEQ ID NO: 35616 - DNA, 28 bp, synthetic construct
  source 1..28: mol_type = other DNA
taggtgagggcagggaaaaaccatgtgg

SEQ ID NO: 35617 - DNA, 28 bp, synthetic construct
  source 1..28: mol_type = other DNA
gggggagggggagtaggtgagggcaggg

SEQ ID NO: 35618 - DNA, 28 bp, synthetic construct
  source 1..28: mol_type = other DNA
ggggggagggggagtaggtgagggcagg

SEQ ID NO: 35619 - DNA, 28 bp, synthetic construct
  source 1..28: mol_type = other DNA
tctgggggggagggggagtaggtgaggg

SEQ ID NO: 35620 - DNA, 28 bp, synthetic construct
  source 1..28: mol_type = other DNA
ctctgggggggagggggagtaggtgagg

SEQ ID NO: 35621 - DNA, 28 bp, synthetic construct
  source 1..28: mol_type = other DNA
cacttctctgggggggagggggagtagg

SEQ ID NO: 35622 - DNA, 28 bp, synthetic construct
  source 1..28: mol_type = other DNA
ttcaaacacttctctgggggggaggggg

SEQ ID NO: 35623 - DNA, 28 bp, synthetic construct
  source 1..28: mol_type = other DNA
gttcaaacacttctctgggggggagggg

SEQ ID NO: 35624 - DNA, 28 bp, synthetic construct
  source 1..28: mol_type = other DNA
ggttcaaacacttctctgggggggaggg

SEQ ID NO: 35625 - DNA, 28 bp, synthetic construct
  source 1..28: mol_type = other DNA
tggttcaaacacttctctgggggggagg

SEQ ID NO: 35626 - DNA, 28 bp, synthetic construct
  source 1..28: mol_type = other DNA
tgttggttcaaacacttctctggggggg

SEQ ID NO: 35627 - DNA, 28 bp, synthetic construct
  source 1..28: mol_type = other DNA
ctgttggttcaaacacttctctgggggg

SEQ ID NO: 35628 - DNA, 28 bp, synthetic construct
  source 1..28: mol_type = other DNA
actgttggttcaaacacttctctggggg

SEQ ID NO: 35629 - DNA, 28 bp, synthetic construct
  source 1..28: mol_type = other DNA
cactgttggttcaaacacttctctgggg

SEQ ID NO: 35630 - DNA, 28 bp, synthetic construct
  source 1..28: mol_type = other DNA
ccactgttggttcaaacacttctctggg

SEQ ID NO: 35631 - DNA, 28 bp, synthetic construct
  source 1..28: mol_type = other DNA
tccactgttggttcaaacacttctctgg

SEQ ID NO: 35632 - DNA, 28 bp, synthetic construct
  source 1..28: mol_type = other DNA
aagtgtttgaaccaacagtggaaagagg

SEQ ID NO: 35633 - DNA, 28 bp, synthetic construct
  source 1..28: mol_type = other DNA
gaaccaacagtggaaagaggtgaactgg

SEQ ID NO: 35634 - DNA, 28 bp, synthetic construct
  source 1..28: mol_type = other DNA
ctaccagttcacctctttccactgttgg

SEQ ID NO: 35635 - DNA, 28 bp, synthetic construct
  source 1..28: mol_type = other DNA
agtggaaagaggtgaactggtagtcagg

SEQ ID NO: 35636 - DNA, 28 bp, synthetic construct
  source 1..28: mol_type = other DNA
ccgcgtgcgcaagtcctacagtcgtcgg

SEQ ID NO: 35637 - DNA, 28 bp, synthetic construct
  source 1..28: mol_type = other DNA
gtagcttcagtggtccgacgactgtagg

SEQ ID NO: 35638 - DNA, 28 bp, synthetic construct
  source 1..28: mol_type = other DNA
agggttcacttacaggtagcttcagtgg

SEQ ID NO: 35639 - DNA, 28 bp, synthetic construct
  source 1..28: mol_type = other DNA
gcagtggggcatagggttcacttacagg

SEQ ID NO: 35640 - DNA, 28 bp, synthetic construct
  source 1..28: mol_type = other DNA
aagtgaaccctatgccccactgccctgg

SEQ ID NO: 35641 - DNA, 28 bp, synthetic construct
  source 1..28: mol_type = other DNA
aaccctatgccccactgccctggcctgg

SEQ ID NO: 35642 - DNA, 28 bp, synthetic construct
  source 1..28: mol_type = other DNA
atccaggccagggcagtggggcataggg

SEQ ID NO: 35643 - DNA, 28 bp, synthetic construct
  source 1..28: mol_type = other DNA
gatccaggccagggcagtggggcatagg

SEQ ID NO: 35644 - DNA, 28 bp, synthetic construct
  source 1..28: mol_type = other DNA
cctttagatccaggccagggcagtgggg

SEQ ID NO: 35645 - DNA, 28 bp, synthetic construct
  source 1..28: mol_type = other DNA
gcctttagatccaggccagggcagtggg

SEQ ID NO: 35646 - DNA, 28 bp, synthetic construct
  source 1..28: mol_type = other DNA
agcctttagatccaggccagggcagtgg

SEQ ID NO: 35647 - DNA, 28 bp, synthetic construct
  source 1..28: mol_type = other DNA
ctctacagcctttagatccaggccaggg

SEQ ID NO: 35648 - DNA, 28 bp, synthetic construct
  source 1..28: mol_type = other DNA
tctctacagcctttagatccaggccagg

SEQ ID NO: 35649 - DNA, 28 bp, synthetic construct
  source 1..28: mol_type = other DNA
cagattctctacagcctttagatccagg

SEQ ID NO: 35650 - DNA, 28 bp, synthetic construct
  source 1..28: mol_type = other DNA
ctggatctaaaggctgtagagaatctgg

SEQ ID NO: 35651 - DNA, 28 bp, synthetic construct
  source 1..28: mol_type = other DNA
aaaggctgtagagaatctggcctgctgg

SEQ ID NO: 35652 - DNA, 28 bp, synthetic construct
  source 1..28: mol_type = other DNA
aaggctgtagagaatctggcctgctggg

SEQ ID NO: 35653 - DNA, 28 bp, synthetic construct
  source 1..28: mol_type = other DNA
gctcacacatgtacagaagcccagcagg

SEQ ID NO: 35654 - DNA, 28 bp, synthetic construct
  source 1..28: mol_type = other DNA
acatgtgtgagccaaaagtttctaaagg

SEQ ID NO: 35655 - DNA, 28 bp, synthetic construct
  source 1..28: mol_type = other DNA
gtgagccaaaagtttctaaaggccttgg

SEQ ID NO: 35656 - DNA, 28 bp, synthetic construct
  source 1..28: mol_type = other DNA
tgagccaaaagtttctaaaggccttggg

SEQ ID NO: 35657 - DNA, 28 bp, synthetic construct
  source 1..28: mol_type = other DNA
gtatcccaaggcctttagaaacttttgg

SEQ ID NO: 35658 - DNA, 28 bp, synthetic construct
  source 1..28: mol_type = other DNA
cagaagtatgtcagtgtttcaacaatgg

SEQ ID NO: 35659 - DNA, 28 bp, synthetic construct
  source 1..28: mol_type = other DNA
gtttcaacaatggatctatccctactgg

SEQ ID NO: 35660 - DNA, 28 bp, synthetic construct
  source 1..28: mol_type = other DNA
tcaacaatggatctatccctactggtgg

SEQ ID NO: 35661 - DNA, 28 bp, synthetic construct
  source 1..28: mol_type = other DNA
caacaatggatctatccctactggtggg

SEQ ID NO: 35662 - DNA, 28 bp, synthetic construct
  source 1..28: mol_type = other DNA
ttcaggtgacattcacccaccagtaggg

SEQ ID NO: 35663 - DNA, 28 bp, synthetic construct
  source 1..28: mol_type = other DNA
attcaggtgacattcacccaccagtagg

SEQ ID NO: 35664 - DNA, 28 bp, synthetic construct
  source 1..28: mol_type = other DNA
gagtcatggagcagggctgacattcagg

SEQ ID NO: 35665 - DNA, 28 bp, synthetic construct
  source 1..28: mol_type = other DNA
ttggggtggacagagtcatggagcaggg

SEQ ID NO: 35666 - DNA, 28 bp, synthetic construct
  source 1..28: mol_type = other DNA
gttggggtggacagagtcatggagcagg

SEQ ID NO: 35667 - DNA, 28 bp, synthetic construct
  source 1..28: mol_type = other DNA
tgcaaggttggggtggacagagtcatgg

SEQ ID NO: 35668 - DNA, 28 bp, synthetic construct
  source 1..28: mol_type = other DNA
ctgttcactgcatgcaaggttggggtgg

SEQ ID NO: 35669 - DNA, 28 bp, synthetic construct
  source 1..28: mol_type = other DNA
aggctgttcactgcatgcaaggttgggg

SEQ ID NO: 35670 - DNA, 28 bp, synthetic construct
  source 1..28: mol_type = other DNA
caggctgttcactgcatgcaaggttggg

SEQ ID NO: 35671 - DNA, 28 bp, synthetic construct
  source 1..28: mol_type = other DNA
ccaaccttgcatgcagtgaacagcctgg

SEQ ID NO: 35672 - DNA, 28 bp, synthetic construct
  source 1..28: mol_type = other DNA
caaccttgcatgcagtgaacagcctggg

SEQ ID NO: 35673 - DNA, 28 bp, synthetic construct
  source 1..28: mol_type = other DNA
atgcccaggctgttcactgcatgcaagg

SEQ ID NO: 35674 - DNA, 28 bp, synthetic construct
  source 1..28: mol_type = other DNA
agcctgggcatcagtgaagagctgaagg

SEQ ID NO: 35675 - DNA, 28 bp, synthetic construct
  source 1..28: mol_type = other DNA
ctccttcagctcttcactgatgcccagg

SEQ ID NO: 35676 - DNA, 28 bp, synthetic construct
  source 1..28: mol_type = other DNA
cagtgaagagctgaaggagaagctgcgg

SEQ ID NO: 35677 - DNA, 28 bp, synthetic construct
  source 1..28: mol_type = other DNA
agtgaagagctgaaggagaagctgcggg

SEQ ID NO: 35678 - DNA, 28 bp, synthetic construct
  source 1..28: mol_type = other DNA
ctgaaggagaagctgcgggatgtgatgg

SEQ ID NO: 35679 - DNA, 28 bp, synthetic construct
  source 1..28: mol_type = other DNA
aaggagaagctgcgggatgtgatggtgg

SEQ ID NO: 35680 - DNA, 28 bp, synthetic construct
  source 1..28: mol_type = other DNA
gaagctgcgggatgtgatggtggaccgg

SEQ ID NO: 35681 - DNA, 28 bp, synthetic construct
  source 1..28: mol_type = other DNA
cgggatgtgatggtggaccggcacaagg

SEQ ID NO: 35682 - DNA, 28 bp, synthetic construct
  source 1..28: mol_type = other DNA
gatgtgatggtggaccggcacaaggtgg

SEQ ID NO: 35683 - DNA, 28 bp, synthetic construct
  source 1..28: mol_type = other DNA
atggtggaccggcacaaggtggccctgg

SEQ ID NO: 35684 - DNA, 28 bp, synthetic construct
  source 1..28: mol_type = other DNA
tggtggaccggcacaaggtggccctggg

SEQ ID NO: 35685 - DNA, 28 bp, synthetic construct
  source 1..28: mol_type = other DNA
ggtggaccggcacaaggtggccctgggg

SEQ ID NO: 35686 - DNA, 28 bp, synthetic construct
  source 1..28: mol_type = other DNA
agtcttccccagggccaccttgtgccgg

SEQ ID NO: 35687 - DNA, 28 bp, synthetic construct
  source 1..28: mol_type = other DNA
cacaaggtggccctggggaagactctgg

SEQ ID NO: 35688 - DNA, 28 bp, synthetic construct
  source 1..28: mol_type = other DNA
acaaggtggccctggggaagactctggg

SEQ ID NO: 35689 - DNA, 28 bp, synthetic construct
  source 1..28: mol_type = other DNA
gtggccctggggaagactctgggagagg

SEQ ID NO: 35690 - DNA, 28 bp, synthetic construct
  source 1..28: mol_type = other DNA
tggccctggggaagactctgggagaggg

SEQ ID NO: 35691 - DNA, 28 bp, synthetic construct
  source 1..28: mol_type = other DNA
tcaccctctcccagagtcttccccaggg

SEQ ID NO: 35692 - DNA, 28 bp, synthetic construct
  source 1..28: mol_type = other DNA
ctcaccctctcccagagtcttccccagg

SEQ ID NO: 35693 - DNA, 28 bp, synthetic construct
  source 1..28: mol_type = other DNA
agactctgggagagggtgagtcccccgg

SEQ ID NO: 35694 - DNA, 28 bp, synthetic construct
  source 1..28: mol_type = other DNA
cagaaggatgtgtgtatgctgccggggg

SEQ ID NO: 35695 - DNA, 28 bp, synthetic construct
  source 1..28: mol_type = other DNA
tcagaaggatgtgtgtatgctgccgggg

SEQ ID NO: 35696 - DNA, 28 bp, synthetic construct
  source 1..28: mol_type = other DNA
ttcagaaggatgtgtgtatgctgccggg

SEQ ID NO: 35697 - DNA, 28 bp, synthetic construct
  source 1..28: mol_type = other DNA
gttcagaaggatgtgtgtatgctgccgg

SEQ ID NO: 35698 - DNA, 28 bp, synthetic construct
  source 1..28: mol_type = other DNA
aagtgcaggatctcagaagttcagaagg

SEQ ID NO: 35699 - DNA, 28 bp, synthetic construct
  source 1..28: mol_type = other DNA
tagttgggtgggagtgtggaagtgcagg

SEQ ID NO: 35700 - DNA, 28 bp, synthetic construct
  source 1..28: mol_type = other DNA
cacttccacactcccacccaactatagg

SEQ ID NO: 35701 - DNA, 28 bp, synthetic construct
  source 1..28: mol_type = other DNA
tatttcctatagttgggtgggagtgtgg

SEQ ID NO: 35702 - DNA, 28 bp, synthetic construct
  source 1..28: mol_type = other DNA
gggactgtatttcctatagttgggtggg

SEQ ID NO: 35703 - DNA, 28 bp, synthetic construct
  source 1..28: mol_type = other DNA
ggggactgtatttcctatagttgggtgg

SEQ ID NO: 35704 - DNA, 28 bp, synthetic construct
  source 1..28: mol_type = other DNA
cgtggggactgtatttcctatagttggg

SEQ ID NO: 35705 - DNA, 28 bp, synthetic construct
  source 1..28: mol_type = other DNA
ccaactataggaaatacagtccccacgg

SEQ ID NO: 35706 - DNA, 28 bp, synthetic construct
  source 1..28: mol_type = other DNA
caactataggaaatacagtccccacggg

SEQ ID NO: 35707 - DNA, 28 bp, synthetic construct
  source 1..28: mol_type = other DNA
aaatacagtccccacgggccctctgagg

SEQ ID NO: 35708 - DNA, 28 bp, synthetic construct
  source 1..28: mol_type = other DNA
agacactgacctcagagggcccgtgggg

SEQ ID NO: 35709 - DNA, 28 bp, synthetic construct
  source 1..28: mol_type = other DNA
gagacactgacctcagagggcccgtggg

SEQ ID NO: 35710 - DNA, 28 bp, synthetic construct
  source 1..28: mol_type = other DNA
ggagacactgacctcagagggcccgtgg

SEQ ID NO: 35711 - DNA, 28 bp, synthetic construct
  source 1..28: mol_type = other DNA
gccctctgaggtcagtgtctccctctgg

SEQ ID NO: 35712 - DNA, 28 bp, synthetic construct
  source 1..28: mol_type = other DNA
gccagagggagacactgacctcagaggg

SEQ ID NO: 35713 - DNA, 28 bp, synthetic construct
  source 1..28: mol_type = other DNA
ggccagagggagacactgacctcagagg

SEQ ID NO: 35714 - DNA, 28 bp, synthetic construct
  source 1..28: mol_type = other DNA
tcagtgtctccctctggccccccacagg

SEQ ID NO: 35715 - DNA, 28 bp, synthetic construct
  source 1..28: mol_type = other DNA
ccctctggccccccacaggagagtttgg

SEQ ID NO: 35716 - DNA, 28 bp, synthetic construct
  source 1..28: mol_type = other DNA
tccaaactctcctgtggggggccagagg

SEQ ID NO: 35717 - DNA, 28 bp, synthetic construct
  source 1..28: mol_type = other DNA
tcacagctccaaactctcctgtgggggg

SEQ ID NO: 35718 - DNA, 28 bp, synthetic construct
  source 1..28: mol_type = other DNA
atcacagctccaaactctcctgtggggg

SEQ ID NO: 35719 - DNA, 28 bp, synthetic construct
  source 1..28: mol_type = other DNA
catcacagctccaaactctcctgtgggg

SEQ ID NO: 35720 - DNA, 28 bp, synthetic construct
  source 1..28: mol_type = other DNA
ccatcacagctccaaactctcctgtggg

SEQ ID NO: 35721 - DNA, 28 bp, synthetic construct
  source 1..28: mol_type = other DNA
tccatcacagctccaaactctcctgtgg

SEQ ID NO: 35722 - DNA, 28 bp, synthetic construct
  source 1..28: mol_type = other DNA
caggagagtttggagctgtgatggaagg

SEQ ID NO: 35723 - DNA, 28 bp, synthetic construct
  source 1..28: mol_type = other DNA
gctgtgatggaaggccagctcaaccagg

SEQ ID NO: 35724 - DNA, 28 bp, synthetic construct
  source 1..28: mol_type = other DNA
gaggatggagtcgtcctggttgagctgg

SEQ ID NO: 35725 - DNA, 28 bp, synthetic construct
  source 1..28: mol_type = other DNA
ctcaaccaggacgactccatcctcaagg

SEQ ID NO: 35726 - DNA, 28 bp, synthetic construct
  source 1..28: mol_type = other DNA
aaccaggacgactccatcctcaaggtgg

SEQ ID NO: 35727 - DNA, 28 bp, synthetic construct
  source 1..28: mol_type = other DNA
agccaccttgaggatggagtcgtcctgg

SEQ ID NO: 35728 - DNA, 28 bp, synthetic construct
  source 1..28: mol_type = other DNA
atcgtcttcacagccaccttgaggatgg

SEQ ID NO: 35729 - DNA, 28 bp, synthetic construct
  source 1..28: mol_type = other DNA
cttcatcgtcttcacagccaccttgagg

SEQ ID NO: 35730 - DNA, 28 bp, synthetic construct
  source 1..28: mol_type = other DNA
aagagtgagttacgtgcacatgtgtagg

SEQ ID NO: 35731 - DNA, 28 bp, synthetic construct
  source 1..28: mol_type = other DNA
ctcaggggcatagggaaggagctggggg

SEQ ID NO: 35732 - DNA, 28 bp, synthetic construct
  source 1..28: mol_type = other DNA
tctcaggggcatagggaaggagctgggg

SEQ ID NO: 35733 - DNA, 28 bp, synthetic construct
  source 1..28: mol_type = other DNA
gtctcaggggcatagggaaggagctggg

SEQ ID NO: 35734 - DNA, 28 bp, synthetic construct
  source 1..28: mol_type = other DNA
tgtctcaggggcatagggaaggagctgg

SEQ ID NO: 35735 - DNA, 28 bp, synthetic construct
  source 1..28: mol_type = other DNA
ctcttctgtctcaggggcatagggaagg

SEQ ID NO: 35736 - DNA, 28 bp, synthetic construct
  source 1..28: mol_type = other DNA
tgctctcttctgtctcaggggcataggg

SEQ ID NO: 35737 - DNA, 28 bp, synthetic construct
  source 1..28: mol_type = other DNA
ttgctctcttctgtctcaggggcatagg

SEQ ID NO: 35738 - DNA, 28 bp, synthetic construct
  source 1..28: mol_type = other DNA
acttgcttgctctcttctgtctcagggg

SEQ ID NO: 35739 - DNA, 28 bp, synthetic construct
  source 1..28: mol_type = other DNA
aacttgcttgctctcttctgtctcaggg

SEQ ID NO: 35740 - DNA, 28 bp, synthetic construct
  source 1..28: mol_type = other DNA
taacttgcttgctctcttctgtctcagg

SEQ ID NO: 35741 - DNA, 28 bp, synthetic construct
  source 1..28: mol_type = other DNA
caagttagccatagcttagaacttctgg

SEQ ID NO: 35742 - DNA, 28 bp, synthetic construct
  source 1..28: mol_type = other DNA
tggaaacaccagaagttctaagctatgg

SEQ ID NO: 35743 - DNA, 28 bp, synthetic construct
  source 1..28: mol_type = other DNA
cttagaacttctggtgtttccagatagg

SEQ ID NO: 35744 - DNA, 28 bp, synthetic construct
  source 1..28: mol_type = other DNA
acttctggtgtttccagataggcaatgg

SEQ ID NO: 35745 - DNA, 28 bp, synthetic construct
  source 1..28: mol_type = other DNA
gtgatgatgatgatgatgatgatgatgg

SEQ ID NO: 35746 - DNA, 28 bp, synthetic construct
  source 1..28: mol_type = other DNA
gatgatgatgatgatgatgatggagtgg

SEQ ID NO: 35747 - DNA, 28 bp, synthetic construct
  source 1..28: mol_type = other DNA
gatgatgatgatgatgatggagtggagg

SEQ ID NO: 35748 - DNA, 28 bp, synthetic construct
  source 1..28: mol_type = other DNA
gatgatgatgatgatggagtggaggtgg

SEQ ID NO: 35749 - DNA, 28 bp, synthetic construct
  source 1..28: mol_type = other DNA
gatgatgatgatggagtggaggtggagg

SEQ ID NO: 35750 - DNA, 28 bp, synthetic construct
  source 1..28: mol_type = other DNA
atgatgatgatggagtggaggtggaggg

SEQ ID NO: 35751 - DNA, 28 bp, synthetic construct
  source 1..28: mol_type = other DNA
tcgtgaggaggaggggaggagagggagg

SEQ ID NO: 35752 - DNA, 28 bp, synthetic construct
  source 1..28: mol_type = other DNA
aggtcgtgaggaggaggggaggagaggg

SEQ ID NO: 35753 - DNA, 28 bp, synthetic construct
  source 1..28: mol_type = other DNA
aaggtcgtgaggaggaggggaggagagg

SEQ ID NO: 35754 - DNA, 28 bp, synthetic construct
  source 1..28: mol_type = other DNA
agagaaaggtcgtgaggaggaggggagg

SEQ ID NO: 35755 - DNA, 28 bp, synthetic construct
  source 1..28: mol_type = other DNA
gagagagaaaggtcgtgaggaggagggg

SEQ ID NO: 35756 - DNA, 28 bp, synthetic construct
  source 1..28: mol_type = other DNA
ggagagagaaaggtcgtgaggaggaggg

SEQ ID NO: 35757 - DNA, 28 bp, synthetic construct
  source 1..28: mol_type = other DNA
gggagagagaaaggtcgtgaggaggagg

SEQ ID NO: 35758 - DNA, 28 bp, synthetic construct
  source 1..28: mol_type = other DNA
tgagggagagagaaaggtcgtgaggagg

SEQ ID NO: 35759 - DNA, 28 bp, synthetic construct
  source 1..28: mol_type = other DNA
acttgagggagagagaaaggtcgtgagg

SEQ ID NO: 35760 - DNA, 28 bp, synthetic construct
  source 1..28: mol_type = other DNA
agatggcaacttgagggagagagaaagg

SEQ ID NO: 35761 - DNA, 28 bp, synthetic construct
  source 1..28: mol_type = other DNA
tctccctcaagttgccatctgcacgagg

SEQ ID NO: 35762 - DNA, 28 bp, synthetic construct
  source 1..28: mol_type = other DNA
tgacctcgtgcagatggcaacttgaggg

SEQ ID NO: 35763 - DNA, 28 bp, synthetic construct
  source 1..28: mol_type = other DNA
ctgacctcgtgcagatggcaacttgagg

SEQ ID NO: 35764 - DNA, 28 bp, synthetic construct
  source 1..28: mol_type = other DNA
gttgccatctgcacgaggtcagagctgg

SEQ ID NO: 35765 - DNA, 28 bp, synthetic construct
  source 1..28: mol_type = other DNA
gccatctgcacgaggtcagagctggagg

SEQ ID NO: 35766 - DNA, 28 bp, synthetic construct
  source 1..28: mol_type = other DNA
tcctccagctctgacctcgtgcagatgg

SEQ ID NO: 35767 - DNA, 28 bp, synthetic construct
  source 1..28: mol_type = other DNA
gagctggaggatttcctgagtgaagcgg

SEQ ID NO: 35768 - DNA, 28 bp, synthetic construct
  source 1..28: mol_type = other DNA
ttcctgagtgaagcggtctgcatgaagg

SEQ ID NO: 35769 - DNA, 28 bp, synthetic construct
  source 1..28: mol_type = other DNA
ttccttcatgcagaccgcttcactcagg

SEQ ID NO: 35770 - DNA, 28 bp, synthetic construct
  source 1..28: mol_type = other DNA
ggaatttgaccatcccaacgtcatgagg

SEQ ID NO: 35771 - DNA, 28 bp, synthetic construct
  source 1..28: mol_type = other DNA
accatcccaacgtcatgaggctcatcgg

SEQ ID NO: 35772 - DNA, 28 bp, synthetic construct
  source 1..28: mol_type = other DNA
accgatgagcctcatgacgttgggatgg

SEQ ID NO: 35773 - DNA, 28 bp, synthetic construct
  source 1..28: mol_type = other DNA
tctcaccgatgagcctcatgacgttggg

SEQ ID NO: 35774 - DNA, 28 bp, synthetic construct
  source 1..28: mol_type = other DNA
ctctcaccgatgagcctcatgacgttgg

SEQ ID NO: 35775 - DNA, 28 bp, synthetic construct
  source 1..28: mol_type = other DNA
acgtcatgaggctcatcggtgagagagg

SEQ ID NO: 35776 - DNA, 28 bp, synthetic construct
  source 1..28: mol_type = other DNA
cgtcatgaggctcatcggtgagagaggg

SEQ ID NO: 35777 - DNA, 28 bp, synthetic construct
  source 1..28: mol_type = other DNA
gtcatgaggctcatcggtgagagagggg

SEQ ID NO: 35778 - DNA, 28 bp, synthetic construct
  source 1..28: mol_type = other DNA
catcggtgagagaggggcagattcaagg

SEQ ID NO: 35779 - DNA, 28 bp, synthetic construct
  source 1..28: mol_type = other DNA
atcggtgagagaggggcagattcaaggg

SEQ ID NO: 35780 - DNA, 28 bp, synthetic construct
  source 1..28: mol_type = other DNA
tcggtgagagaggggcagattcaagggg

SEQ ID NO: 35781 - DNA, 28 bp, synthetic construct
  source 1..28: mol_type = other DNA
agattcaaggggtctacaagccccatgg

SEQ ID NO: 35782 - DNA, 28 bp, synthetic construct
  source 1..28: mol_type = other DNA
gattcaaggggtctacaagccccatggg

SEQ ID NO: 35783 - DNA, 28 bp, synthetic construct
  source 1..28: mol_type = other DNA
attcaaggggtctacaagccccatgggg

SEQ ID NO: 35784 - DNA, 28 bp, synthetic construct
  source 1..28: mol_type = other DNA
ttcaaggggtctacaagccccatggggg

SEQ ID NO: 35785 - DNA, 28 bp, synthetic construct
  source 1..28: mol_type = other DNA
acaagccccatgggggccatagcagagg

SEQ ID NO: 35786 - DNA, 28 bp, synthetic construct
  source 1..28: mol_type = other DNA
caagccccatgggggccatagcagaggg

SEQ ID NO: 35787 - DNA, 28 bp, synthetic construct
  source 1..28: mol_type = other DNA
tcttccctctgctatggcccccatgggg

SEQ ID NO: 35788 - DNA, 28 bp, synthetic construct
  source 1..28: mol_type = other DNA
ctcttccctctgctatggcccccatggg

SEQ ID NO: 35789 - DNA, 28 bp, synthetic construct
  source 1..28: mol_type = other DNA
gctcttccctctgctatggcccccatgg

SEQ ID NO: 35790 - DNA, 28 bp, synthetic construct
  source 1..28: mol_type = other DNA
agaagcagggctcttccctctgctatgg

SEQ ID NO: 35791 - DNA, 28 bp, synthetic construct
  source 1..28: mol_type = other DNA
atagcagagggaagagccctgcttctgg

SEQ ID NO: 35792 - DNA, 28 bp, synthetic construct
  source 1..28: mol_type = other DNA
gagggaagagccctgcttctggccctgg

SEQ ID NO: 35793 - DNA, 28 bp, synthetic construct
  source 1..28: mol_type = other DNA
agggaagagccctgcttctggccctggg

SEQ ID NO: 35794 - DNA, 28 bp, synthetic construct
  source 1..28: mol_type = other DNA
tttgatcttcccagggccagaagcaggg

SEQ ID NO: 35795 - DNA, 28 bp, synthetic construct
  source 1..28: mol_type = other DNA
gtttgatcttcccagggccagaagcagg

SEQ ID NO: 35796 - DNA, 28 bp, synthetic construct
  source 1..28: mol_type = other DNA
ctggccctgggaagatcaaacttccagg

SEQ ID NO: 35797 - DNA, 28 bp, synthetic construct
  source 1..28: mol_type = other DNA
gaagcctggaagtttgatcttcccaggg

SEQ ID NO: 35798 - DNA, 28 bp, synthetic construct
  source 1..28: mol_type = other DNA
ggaagcctggaagtttgatcttcccagg

SEQ ID NO: 35799 - DNA, 28 bp, synthetic construct
  source 1..28: mol_type = other DNA
ctgaaggagcggggagcaggaagcctgg

SEQ ID NO: 35800 - DNA, 28 bp, synthetic construct
  source 1..28: mol_type = other DNA
caggcttcctgctccccgctccttcagg

SEQ ID NO: 35801 - DNA, 28 bp, synthetic construct
  source 1..28: mol_type = other DNA
aggcttcctgctccccgctccttcaggg

SEQ ID NO: 35802 - DNA, 28 bp, synthetic construct
  source 1..28: mol_type = other DNA
ccaatctggccaccatattgtttggggg

SEQ ID NO: 35803 - DNA, 28 bp, synthetic construct
  source 1..28: mol_type = other DNA
tccaatctggccaccatattgtttgggg

SEQ ID NO: 35804 - DNA, 28 bp, synthetic construct
  source 1..28: mol_type = other DNA
atccaatctggccaccatattgtttggg

SEQ ID NO: 35805 - DNA, 28 bp, synthetic construct
  source 1..28: mol_type = other DNA
catccaatctggccaccatattgtttgg

SEQ ID NO: 35806 - DNA, 28 bp, synthetic construct
  source 1..28: mol_type = other DNA
caaacaatatggtggccagattggatgg

SEQ ID NO: 35807 - DNA, 28 bp, synthetic construct
  source 1..28: mol_type = other DNA
aaacaatatggtggccagattggatggg

SEQ ID NO: 35808 - DNA, 28 bp, synthetic construct
  source 1..28: mol_type = other DNA
tggccagattggatgggtagtgagaagg

SEQ ID NO: 35809 - DNA, 28 bp, synthetic construct
  source 1..28: mol_type = other DNA
tctccttctcactacccatccaatctgg

SEQ ID NO: 35810 - DNA, 28 bp, synthetic construct
  source 1..28: mol_type = other DNA
agattggatgggtagtgagaaggagagg

SEQ ID NO: 35811 - DNA, 28 bp, synthetic construct
  source 1..28: mol_type = other DNA
tggatgggtagtgagaaggagaggctgg

SEQ ID NO: 35812 - DNA, 28 bp, synthetic construct
  source 1..28: mol_type = other DNA
atgggtagtgagaaggagaggctggagg

SEQ ID NO: 35813 - DNA, 28 bp, synthetic construct
  source 1..28: mol_type = other DNA
gtagtgagaaggagaggctggaggctgg

SEQ ID NO: 35814 - DNA, 28 bp, synthetic construct
  source 1..28: mol_type = other DNA
tgagaaggagaggctggaggctggctgg

SEQ ID NO: 35815 - DNA, 28 bp, synthetic construct
  source 1..28: mol_type = other DNA
gaaggagaggctggaggctggctggtgg

SEQ ID NO: 35816 - DNA, 28 bp, synthetic construct
  source 1..28: mol_type = other DNA
aaggagaggctggaggctggctggtggg

SEQ ID NO: 35817 - DNA, 28 bp, synthetic construct
  source 1..28: mol_type = other DNA
aggagaggctggaggctggctggtgggg

SEQ ID NO: 35818 - DNA, 28 bp, synthetic construct
  source 1..28: mol_type = other DNA
ggagaggctggaggctggctggtggggg

SEQ ID NO: 35819 - DNA, 28 bp, synthetic construct
  source 1..28: mol_type = other DNA
gagaggctggaggctggctggtgggggg

SEQ ID NO: 35820 - DNA, 28 bp, synthetic construct
  source 1..28: mol_type = other DNA
gctggaggctggctggtggggggcttgg

SEQ ID NO: 35821 - DNA, 28 bp, synthetic construct
  source 1..28: mol_type = other DNA
ggcttggcttccccttctgcccagcagg

SEQ ID NO: 35822 - DNA, 28 bp, synthetic construct
  source 1..28: mol_type = other DNA
tccccttctgcccagcaggagtgacagg

SEQ ID NO: 35823 - DNA, 28 bp, synthetic construct
  source 1..28: mol_type = other DNA
ccccttctgcccagcaggagtgacaggg

SEQ ID NO: 35824 - DNA, 28 bp, synthetic construct
  source 1..28: mol_type = other DNA
gccctgtcactcctgctgggcagaaggg

SEQ ID NO: 35825 - DNA, 28 bp, synthetic construct
  source 1..28: mol_type = other DNA
agccctgtcactcctgctgggcagaagg

SEQ ID NO: 35826 - DNA, 28 bp, synthetic construct
  source 1..28: mol_type = other DNA
gcccagcaggagtgacagggctacctgg

SEQ ID NO: 35827 - DNA, 28 bp, synthetic construct
  source 1..28: mol_type = other DNA
cccaggtagccctgtcactcctgctggg

SEQ ID NO: 35828 - DNA, 28 bp, synthetic construct
  source 1..28: mol_type = other DNA
ccagcaggagtgacagggctacctgggg

SEQ ID NO: 35829 - DNA, 28 bp, synthetic construct
  source 1..28: mol_type = other DNA
cagcaggagtgacagggctacctggggg

SEQ ID NO: 35830 - DNA, 28 bp, synthetic construct
  source 1..28: mol_type = other DNA
agcaggagtgacagggctacctgggggg

SEQ ID NO: 35831 - DNA, 28 bp, synthetic construct
  source 1..28: mol_type = other DNA
agtgacagggctacctggggggctcagg

SEQ ID NO: 35832 - DNA, 28 bp, synthetic construct
  source 1..28: mol_type = other DNA
ctggaaacagacacctgagccccccagg

SEQ ID NO: 35833 - DNA, 28 bp, synthetic construct
  source 1..28: mol_type = other DNA
ctggggggctcaggtgtctgtttccagg

SEQ ID NO: 35834 - DNA, 28 bp, synthetic construct
  source 1..28: mol_type = other DNA
tggggggctcaggtgtctgtttccaggg

SEQ ID NO: 35835 - DNA, 28 bp, synthetic construct
  source 1..28: mol_type = other DNA
tgggaagctctctcgttcagaaccctgg

SEQ ID NO: 35836 - DNA, 28 bp, synthetic construct
  source 1..28: mol_type = other DNA
gaacgagagagcttcccagcacctgtgg

SEQ ID NO: 35837 - DNA, 28 bp, synthetic construct
  source 1..28: mol_type = other DNA
gaaaggtaagatgaccacaggtgctggg

SEQ ID NO: 35838 - DNA, 28 bp, synthetic construct
  source 1..28: mol_type = other DNA
tgaaaggtaagatgaccacaggtgctgg

SEQ ID NO: 35839 - DNA, 28 bp, synthetic construct
  source 1..28: mol_type = other DNA
gtttcatgaaaggtaagatgaccacagg

SEQ ID NO: 35840 - DNA, 28 bp, synthetic construct
  source 1..28: mol_type = other DNA
tggtcatcttacctttcatgaaacatgg

SEQ ID NO: 35841 - DNA, 28 bp, synthetic construct
  source 1..28: mol_type = other DNA
tgtgtaggtctccatgtttcatgaaagg

SEQ ID NO: 35842 - DNA, 28 bp, synthetic construct
  source 1..28: mol_type = other DNA
ccgggaatagaggaggaagctgtgtagg

SEQ ID NO: 35843 - DNA, 28 bp, synthetic construct
  source 1..28: mol_type = other DNA
acagcttcctcctctattcccggctcgg

SEQ ID NO: 35844 - DNA, 28 bp, synthetic construct
  source 1..28: mol_type = other DNA
cagcttcctcctctattcccggctcggg

SEQ ID NO: 35845 - DNA, 28 bp, synthetic construct
  source 1..28: mol_type = other DNA
agcttcctcctctattcccggctcgggg

SEQ ID NO: 35846 - DNA, 28 bp, synthetic construct
  source 1..28: mol_type = other DNA
ctggtccccgagccgggaatagaggagg

SEQ ID NO: 35847 - DNA, 28 bp, synthetic construct
  source 1..28: mol_type = other DNA
tggctggtccccgagccgggaatagagg

SEQ ID NO: 35848 - DNA, 28 bp, synthetic construct
  source 1..28: mol_type = other DNA
tattcccggctcggggaccagccagtgg

SEQ ID NO: 35849 - DNA, 28 bp, synthetic construct
  source 1..28: mol_type = other DNA
cttaccactggctggtccccgagccggg

SEQ ID NO: 35850 - DNA, 28 bp, synthetic construct
  source 1..28: mol_type = other DNA
ccttaccactggctggtccccgagccgg

SEQ ID NO: 35851 - DNA, 28 bp, synthetic construct
  source 1..28: mol_type = other DNA
cggctcggggaccagccagtggtaaggg

SEQ ID NO: 35852 - DNA, 28 bp, synthetic construct
  source 1..28: mol_type = other DNA
ggctcggggaccagccagtggtaagggg

SEQ ID NO: 35853 - DNA, 28 bp, synthetic construct
  source 1..28: mol_type = other DNA
tgattaaacgccccttaccactggctgg

SEQ ID NO: 35854 - DNA, 28 bp, synthetic construct
  source 1..28: mol_type = other DNA
tgaatgattaaacgccccttaccactgg

SEQ ID NO: 35855 - DNA, 28 bp, synthetic construct
  source 1..28: mol_type = other DNA
tacaaatattaactgagcatctatcagg

SEQ ID NO: 35856 - DNA, 28 bp, synthetic construct
  source 1..28: mol_type = other DNA
caggtacccagtgctgctcagaccctgg

SEQ ID NO: 35857 - DNA, 28 bp, synthetic construct
  source 1..28: mol_type = other DNA
aggtacccagtgctgctcagaccctggg

SEQ ID NO: 35858 - DNA, 28 bp, synthetic construct
  source 1..28: mol_type = other DNA
gtcttcccagggtctgagcagcactggg

SEQ ID NO: 35859 - DNA, 28 bp, synthetic construct
  source 1..28: mol_type = other DNA
ggtcttcccagggtctgagcagcactgg

SEQ ID NO: 35860 - DNA, 28 bp, synthetic construct
  source 1..28: mol_type = other DNA
tgctgctcagaccctgggaagaccacgg

SEQ ID NO: 35861 - DNA, 28 bp, synthetic construct
  source 1..28: mol_type = other DNA
agaccctgggaagaccacggtgaccagg

SEQ ID NO: 35862 - DNA, 28 bp, synthetic construct
  source 1..28: mol_type = other DNA
gctcctggtcaccgtggtcttcccaggg

SEQ ID NO: 35863 - DNA, 28 bp, synthetic construct
  source 1..28: mol_type = other DNA
agctcctggtcaccgtggtcttcccagg

SEQ ID NO: 35864 - DNA, 28 bp, synthetic construct
  source 1..28: mol_type = other DNA
caggagagcaagctcctggtcaccgtgg

SEQ ID NO: 35865 - DNA, 28 bp, synthetic construct
  source 1..28: mol_type = other DNA
cacggtgaccaggagcttgctctcctgg

SEQ ID NO: 35866 - DNA, 28 bp, synthetic construct
  source 1..28: mol_type = other DNA
gaaatgctccaggagagcaagctcctgg

SEQ ID NO: 35867 - DNA, 28 bp, synthetic construct
  source 1..28: mol_type = other DNA
ttgtcagggccatgggaaaccactgcgg

SEQ ID NO: 35868 - DNA, 28 bp, synthetic construct
  source 1..28: mol_type = other DNA
tgtcagggccatgggaaaccactgcggg

SEQ ID NO: 35869 - DNA, 28 bp, synthetic construct
  source 1..28: mol_type = other DNA
tagctctgcccgcagtggtttcccatgg

SEQ ID NO: 35870 - DNA, 28 bp, synthetic construct
  source 1..28: mol_type = other DNA
atgggaaaccactgcgggcagagctagg

SEQ ID NO: 35871 - DNA, 28 bp, synthetic construct
  source 1..28: mol_type = other DNA
tgtgcaagcctagctctgcccgcagtgg

SEQ ID NO: 35872 - DNA, 28 bp, synthetic construct
  source 1..28: mol_type = other DNA
tgcgggcagagctaggcttgcacagagg

SEQ ID NO: 35873 - DNA, 28 bp, synthetic construct
  source 1..28: mol_type = other DNA
gcgggcagagctaggcttgcacagaggg

SEQ ID NO: 35874 - DNA, 28 bp, synthetic construct
  source 1..28: mol_type = other DNA
gcagagctaggcttgcacagagggatgg

SEQ ID NO: 35875 - DNA, 28 bp, synthetic construct
  source 1..28: mol_type = other DNA
gagctaggcttgcacagagggatggagg

SEQ ID NO: 35876 - DNA, 28 bp, synthetic construct
  source 1..28: mol_type = other DNA
agctaggcttgcacagagggatggaggg

SEQ ID NO: 35877 - DNA, 28 bp, synthetic construct
  source 1..28: mol_type = other DNA
taggcttgcacagagggatggagggagg

SEQ ID NO: 35878 - DNA, 28 bp, synthetic construct
  source 1..28: mol_type = other DNA
gcttgcacagagggatggagggaggagg

SEQ ID NO: 35879 - DNA, 28 bp, synthetic construct
  source 1..28: mol_type = other DNA
cttgcacagagggatggagggaggaggg

SEQ ID NO: 35880 - DNA, 28 bp, synthetic construct
  source 1..28: mol_type = other DNA
gatggagggaggagggatcgcatcaagg

SEQ ID NO: 35881 - DNA, 28 bp, synthetic construct
  source 1..28: mol_type = other DNA
tgttgacctctcctcccacctgccttgg

SEQ ID NO: 35882 - DNA, 28 bp, synthetic construct
  source 1..28: mol_type = other DNA
ggggagccaaggcaggtgggaggagagg

SEQ ID NO: 35883 - DNA, 28 bp, synthetic construct
  source 1..28: mol_type = other DNA
gtactggggagccaaggcaggtgggagg

SEQ ID NO: 35884 - DNA, 28 bp, synthetic construct
  source 1..28: mol_type = other DNA
caggtactggggagccaaggcaggtggg

SEQ ID NO: 35885 - DNA, 28 bp, synthetic construct
  source 1..28: mol_type = other DNA
gcaggtactggggagccaaggcaggtgg

SEQ ID NO: 35886 - DNA, 28 bp, synthetic construct
  source 1..28: mol_type = other DNA
tgggcaggtactggggagccaaggcagg

SEQ ID NO: 35887 - DNA, 28 bp, synthetic construct
  source 1..28: mol_type = other DNA
tgagtgggcaggtactggggagccaagg

SEQ ID NO: 35888 - DNA, 28 bp, synthetic construct
  source 1..28: mol_type = other DNA
ctagcatctgagtgggcaggtactgggg

SEQ ID NO: 35889 - DNA, 28 bp, synthetic construct
  source 1..28: mol_type = other DNA
actagcatctgagtgggcaggtactggg

SEQ ID NO: 35890 - DNA, 28 bp, synthetic construct
  source 1..28: mol_type = other DNA
cactagcatctgagtgggcaggtactgg

SEQ ID NO: 35891 - DNA, 28 bp, synthetic construct
  source 1..28: mol_type = other DNA
gaacttcactagcatctgagtgggcagg

SEQ ID NO: 35892 - DNA, 28 bp, synthetic construct
  source 1..28: mol_type = other DNA
cccactcagatgctagtgaagttcatgg

SEQ ID NO: 35893 - DNA, 28 bp, synthetic construct
  source 1..28: mol_type = other DNA
gccatgaacttcactagcatctgagtgg

SEQ ID NO: 35894 - DNA, 28 bp, synthetic construct
  source 1..28: mol_type = other DNA
tgaagttcatggcagacatcgccagtgg

SEQ ID NO: 35895 - DNA, 28 bp, synthetic construct
  source 1..28: mol_type = other DNA
ttcatggcagacatcgccagtggcatgg

SEQ ID NO: 35896 - DNA, 28 bp, synthetic construct
  source 1..28: mol_type = other DNA
ttggtactcagatactccatgccactgg

SEQ ID NO: 35897 - DNA, 28 bp, synthetic construct
  source 1..28: mol_type = other DNA
tctgagtaccaagagattcatacaccgg

SEQ ID NO: 35898 - DNA, 28 bp, synthetic construct
  source 1..28: mol_type = other DNA
ctgagtaccaagagattcatacaccggg

SEQ ID NO: 35899 - DNA, 28 bp, synthetic construct
  source 1..28: mol_type = other DNA
accaagagattcatacaccgggacctgg

SEQ ID NO: 35900 - DNA, 28 bp, synthetic construct
  source 1..28: mol_type = other DNA
gccaggtcccggtgtatgaatctcttgg

SEQ ID NO: 35901 - DNA, 28 bp, synthetic construct
  source 1..28: mol_type = other DNA
aagagattcatacaccgggacctggcgg

SEQ ID NO: 35902 - DNA, 28 bp, synthetic construct
  source 1..28: mol_type = other DNA
attcatacaccgggacctggcggccagg

SEQ ID NO: 35903 - DNA, 28 bp, synthetic construct
  source 1..28: mol_type = other DNA
catgcagttcctggccgccaggtcccgg

SEQ ID NO: 35904 - DNA, 28 bp, synthetic construct
  source 1..28: mol_type = other DNA
cactcacatgcagttcctggccgccagg

SEQ ID NO: 35905 - DNA, 28 bp, synthetic construct
  source 1..28: mol_type = other DNA
ctgaaaggcactcacatgcagttcctgg

SEQ ID NO: 35906 - DNA, 28 bp, synthetic construct
  source 1..28: mol_type = other DNA
caggaactgcatgtgagtgcctttcagg

SEQ ID NO: 35907 - DNA, 28 bp, synthetic construct
  source 1..28: mol_type = other DNA
aggaactgcatgtgagtgcctttcaggg

SEQ ID NO: 35908 - DNA, 28 bp, synthetic construct
  source 1..28: mol_type = other DNA
cagttggggggggggggtccctgaaagg

SEQ ID NO: 35909 - DNA, 28 bp, synthetic construct
  source 1..28: mol_type = other DNA
gagtgcaggagcagttgggggggggggg

SEQ ID NO: 35910 - DNA, 28 bp, synthetic construct
  source 1..28: mol_type = other DNA
ggagtgcaggagcagttggggggggggg

SEQ ID NO: 35911 - DNA, 28 bp, synthetic construct
  source 1..28: mol_type = other DNA
gggagtgcaggagcagttgggggggggg

SEQ ID NO: 35912 - DNA, 28 bp, synthetic construct
  source 1..28: mol_type = other DNA
agggagtgcaggagcagttggggggggg

SEQ ID NO: 35913 - DNA, 28 bp, synthetic construct
  source 1..28: mol_type = other DNA
cagggagtgcaggagcagttgggggggg

SEQ ID NO: 35914 - DNA, 28 bp, synthetic construct
  source 1..28: mol_type = other DNA
tcagggagtgcaggagcagttggggggg

SEQ ID NO: 35915 - DNA, 28 bp, synthetic construct
  source 1..28: mol_type = other DNA
ctcagggagtgcaggagcagttgggggg

SEQ ID NO: 35916 - DNA, 28 bp, synthetic construct
  source 1..28: mol_type = other DNA
cctcagggagtgcaggagcagttggggg

SEQ ID NO: 35917 - DNA, 28 bp, synthetic construct
  source 1..28: mol_type = other DNA
ccccaactgctcctgcactccctgaggg

SEQ ID NO: 35918 - DNA, 28 bp, synthetic construct
  source 1..28: mol_type = other DNA
tccctcagggagtgcaggagcagttggg

SEQ ID NO: 35919 - DNA, 28 bp, synthetic construct
  source 1..28: mol_type = other DNA
ctccctcagggagtgcaggagcagttgg

SEQ ID NO: 35920 - DNA, 28 bp, synthetic construct
  source 1..28: mol_type = other DNA
gggagggaactccctcagggagtgcagg

SEQ ID NO: 35921 - DNA, 28 bp, synthetic construct
  source 1..28: mol_type = other DNA
aagaaggagggagggaactccctcaggg

SEQ ID NO: 35922 - DNA, 28 bp, synthetic construct
  source 1..28: mol_type = other DNA
taagaaggagggagggaactccctcagg

SEQ ID NO: 35923 - DNA, 28 bp, synthetic construct
  source 1..28: mol_type = other DNA
tgagggagttccctccctccttcttagg

SEQ ID NO: 35924 - DNA, 28 bp, synthetic construct
  source 1..28: mol_type = other DNA
ggagttccctccctccttcttaggatgg

SEQ ID NO: 35925 - DNA, 28 bp, synthetic construct
  source 1..28: mol_type = other DNA
ctgcttccatcctaagaaggagggaggg

SEQ ID NO: 35926 - DNA, 28 bp, synthetic construct
  source 1..28: mol_type = other DNA
cctccctccttcttaggatggaagcagg

SEQ ID NO: 35927 - DNA, 28 bp, synthetic construct
  source 1..28: mol_type = other DNA
ctccctccttcttaggatggaagcaggg

SEQ ID NO: 35928 - DNA, 28 bp, synthetic construct
  source 1..28: mol_type = other DNA
agccctgcttccatcctaagaaggaggg

SEQ ID NO: 35929 - DNA, 28 bp, synthetic construct
  source 1..28: mol_type = other DNA
tagccctgcttccatcctaagaaggagg

SEQ ID NO: 35930 - DNA, 28 bp, synthetic construct
  source 1..28: mol_type = other DNA
gtctagccctgcttccatcctaagaagg

SEQ ID NO: 35931 - DNA, 28 bp, synthetic construct
  source 1..28: mol_type = other DNA
tggaagcagggctagacacccgctgagg

SEQ ID NO: 35932 - DNA, 28 bp, synthetic construct
  source 1..28: mol_type = other DNA
ggaagcagggctagacacccgctgaggg

SEQ ID NO: 35933 - DNA, 28 bp, synthetic construct
  source 1..28: mol_type = other DNA
gcagggctagacacccgctgagggcagg

SEQ ID NO: 35934 - DNA, 28 bp, synthetic construct
  source 1..28: mol_type = other DNA
acccgctgagggcaggtcagaactcagg

SEQ ID NO: 35935 - DNA, 28 bp, synthetic construct
  source 1..28: mol_type = other DNA
tcctgagttctgacctgccctcagcggg

SEQ ID NO: 35936 - DNA, 28 bp, synthetic construct
  source 1..28: mol_type = other DNA
gtcctgagttctgacctgccctcagcgg

SEQ ID NO: 35937 - DNA, 28 bp, synthetic construct
  source 1..28: mol_type = other DNA
atccccacccgcagccaggacagtgagg

SEQ ID NO: 35938 - DNA, 28 bp, synthetic construct
  source 1..28: mol_type = other DNA
tccccacccgcagccaggacagtgaggg

SEQ ID NO: 35939 - DNA, 28 bp, synthetic construct
  source 1..28: mol_type = other DNA
cccctcactgtcctggctgcgggtgggg

SEQ ID NO: 35940 - DNA, 28 bp, synthetic construct
  source 1..28: mol_type = other DNA
tcccctcactgtcctggctgcgggtggg

SEQ ID NO: 35941 - DNA, 28 bp, synthetic construct
  source 1..28: mol_type = other DNA
ctcccctcactgtcctggctgcgggtgg

SEQ ID NO: 35942 - DNA, 28 bp, synthetic construct
  source 1..28: mol_type = other DNA
cacccgcagccaggacagtgaggggagg

SEQ ID NO: 35943 - DNA, 28 bp, synthetic construct
  source 1..28: mol_type = other DNA
ctcctcccctcactgtcctggctgcggg

SEQ ID NO: 35944 - DNA, 28 bp, synthetic construct
  source 1..28: mol_type = other DNA
cctcctcccctcactgtcctggctgcgg

SEQ ID NO: 35945 - DNA, 28 bp, synthetic construct
  source 1..28: mol_type = other DNA
tctgcacctcctcccctcactgtcctgg

SEQ ID NO: 35946 - DNA, 28 bp, synthetic construct
  source 1..28: mol_type = other DNA
ggaggtgcagatgtgtctgagagccagg

SEQ ID NO: 35947 - DNA, 28 bp, synthetic construct
  source 1..28: mol_type = other DNA
gaggtgcagatgtgtctgagagccaggg

SEQ ID NO: 35948 - DNA, 28 bp, synthetic construct
  source 1..28: mol_type = other DNA
tgcagatgtgtctgagagccagggcagg

SEQ ID NO: 35949 - DNA, 28 bp, synthetic construct
  source 1..28: mol_type = other DNA
tgtctgagagccagggcaggcttcctgg

SEQ ID NO: 35950 - DNA, 28 bp, synthetic construct
  source 1..28: mol_type = other DNA
ctgagagccagggcaggcttcctggtgg

SEQ ID NO: 35951 - DNA, 28 bp, synthetic construct
  source 1..28: mol_type = other DNA
agagccagggcaggcttcctggtggagg

SEQ ID NO: 35952 - DNA, 28 bp, synthetic construct
  source 1..28: mol_type = other DNA
gtcacctccaccaggaagcctgccctgg

SEQ ID NO: 35953 - DNA, 28 bp, synthetic construct
  source 1..28: mol_type = other DNA
ggtcagggcatcagtcacctccaccagg

SEQ ID NO: 35954 - DNA, 28 bp, synthetic construct
  source 1..28: mol_type = other DNA
tggattggggaaaggaacagggtcaggg

SEQ ID NO: 35955 - DNA, 28 bp, synthetic construct
  source 1..28: mol_type = other DNA
ttggattggggaaaggaacagggtcagg

SEQ ID NO: 35956 - DNA, 28 bp, synthetic construct
  source 1..28: mol_type = other DNA
ccctgttcctttccccaatccaaacagg

SEQ ID NO: 35957 - DNA, 28 bp, synthetic construct
  source 1..28: mol_type = other DNA
gcctgtttggattggggaaaggaacagg

SEQ ID NO: 35958 - DNA, 28 bp, synthetic construct
  source 1..28: mol_type = other DNA
cattcagcctgtttggattggggaaagg

SEQ ID NO: 35959 - DNA, 28 bp, synthetic construct
  source 1..28: mol_type = other DNA
gttctcattcagcctgtttggattgggg

SEQ ID NO: 35960 - DNA, 28 bp, synthetic construct
  source 1..28: mol_type = other DNA
tgttctcattcagcctgtttggattggg

SEQ ID NO: 35961 - DNA, 28 bp, synthetic construct
  source 1..28: mol_type = other DNA
atgttctcattcagcctgtttggattgg

SEQ ID NO: 35962 - DNA, 28 bp, synthetic construct
  source 1..28: mol_type = other DNA
cggacatgttctcattcagcctgtttgg

SEQ ID NO: 35963 - DNA, 28 bp, synthetic construct
  source 1..28: mol_type = other DNA
ctgaatgagaacatgtccgtgtgtgtgg

SEQ ID NO: 35964 - DNA, 28 bp, synthetic construct
  source 1..28: mol_type = other DNA
aatgagaacatgtccgtgtgtgtggcgg

SEQ ID NO: 35965 - DNA, 28 bp, synthetic construct
  source 1..28: mol_type = other DNA
acatgtccgtgtgtgtggcggacttcgg

SEQ ID NO: 35966 - DNA, 28 bp, synthetic construct
  source 1..28: mol_type = other DNA
catgtccgtgtgtgtggcggacttcggg

SEQ ID NO: 35967 - DNA, 28 bp, synthetic construct
  source 1..28: mol_type = other DNA
gagagcccgaagtccgccacacacacgg

SEQ ID NO: 35968 - DNA, 28 bp, synthetic construct
  source 1..28: mol_type = other DNA
tcgggctctccaagaagatctacaatgg

SEQ ID NO: 35969 - DNA, 28 bp, synthetic construct
  source 1..28: mol_type = other DNA
cgggctctccaagaagatctacaatggg

SEQ ID NO: 35970 - DNA, 28 bp, synthetic construct
  source 1..28: mol_type = other DNA
gggctctccaagaagatctacaatgggg

SEQ ID NO: 35971 - DNA, 28 bp, synthetic construct
  source 1..28: mol_type = other DNA
tagtagtccccattgtagatcttcttgg

SEQ ID NO: 35972 - DNA, 28 bp, synthetic construct
  source 1..28: mol_type = other DNA
atctacaatggggactactaccgccagg

SEQ ID NO: 35973 - DNA, 28 bp, synthetic construct
  source 1..28: mol_type = other DNA
tctacaatggggactactaccgccaggg

SEQ ID NO: 35974 - DNA, 28 bp, synthetic construct
  source 1..28: mol_type = other DNA
tggcatcttggcgatacgtccctggcgg

SEQ ID NO: 35975 - DNA, 28 bp, synthetic construct
  source 1..28: mol_type = other DNA
gactggcatcttggcgatacgtccctgg

SEQ ID NO: 35976 - DNA, 28 bp, synthetic construct
  source 1..28: mol_type = other DNA
acgtatcgccaagatgccagtcaagtgg

SEQ ID NO: 35977 - DNA, 28 bp, synthetic construct
  source 1..28: mol_type = other DNA
atggcaatccacttgactggcatcttgg

SEQ ID NO: 35978 - DNA, 28 bp, synthetic construct
  source 1..28: mol_type = other DNA
gactctcaatggcaatccacttgactgg

SEQ ID NO: 35979 - DNA, 28 bp, synthetic construct
  source 1..28: mol_type = other DNA
tagacacggtcagctagactctcaatgg

SEQ ID NO: 35980 - DNA, 28 bp, synthetic construct
  source 1..28: mol_type = other DNA
cacatcgctcttgctggtgtagacacgg

SEQ ID NO: 35981 - DNA, 28 bp, synthetic construct
  source 1..28: mol_type = other DNA
cgtgtctacaccagcaagagcgatgtgg

SEQ ID NO: 35982 - DNA, 28 bp, synthetic construct
  source 1..28: mol_type = other DNA
tctacaccagcaagagcgatgtggtagg

SEQ ID NO: 35983 - DNA, 28 bp, synthetic construct
  source 1..28: mol_type = other DNA
agtgcacctaccacatcgctcttgctgg

SEQ ID NO: 35984 - DNA, 28 bp, synthetic construct
  source 1..28: mol_type = other DNA
gtggtaggtgcactcccgccaagagtgg

SEQ ID NO: 35985 - DNA, 28 bp, synthetic construct
  source 1..28: mol_type = other DNA
tggtaggtgcactcccgccaagagtggg

SEQ ID NO: 35986 - DNA, 28 bp, synthetic construct
  source 1..28: mol_type = other DNA
ggtaggtgcactcccgccaagagtgggg

SEQ ID NO: 35987 - DNA, 28 bp, synthetic construct
  source 1..28: mol_type = other DNA
cactcccgccaagagtggggaaccatgg

SEQ ID NO: 35988 - DNA, 28 bp, synthetic construct
  source 1..28: mol_type = other DNA
actcccgccaagagtggggaaccatggg

SEQ ID NO: 35989 - DNA, 28 bp, synthetic construct
  source 1..28: mol_type = other DNA
cccgccaagagtggggaaccatgggagg

SEQ ID NO: 35990 - DNA, 28 bp, synthetic construct
  source 1..28: mol_type = other DNA
ccgccaagagtggggaaccatgggaggg

SEQ ID NO: 35991 - DNA, 28 bp, synthetic construct
  source 1..28: mol_type = other DNA
atgccctcccatggttccccactcttgg

SEQ ID NO: 35992 - DNA, 28 bp, synthetic construct
  source 1..28: mol_type = other DNA
aagagtggggaaccatgggagggcatgg

SEQ ID NO: 35993 - DNA, 28 bp, synthetic construct
  source 1..28: mol_type = other DNA
gtgatggtcaggccatgccctcccatgg

SEQ ID NO: 35994 - DNA, 28 bp, synthetic construct
  source 1..28: mol_type = other DNA
tggcctgaccatcacacactatgcctgg

SEQ ID NO: 35995 - DNA, 28 bp, synthetic construct
  source 1..28: mol_type = other DNA
ggcctgaccatcacacactatgcctggg

SEQ ID NO: 35996 - DNA, 28 bp, synthetic construct
  source 1..28: mol_type = other DNA
cacccaggcatagtgtgtgatggtcagg

SEQ ID NO: 35997 - DNA, 28 bp, synthetic construct
  source 1..28: mol_type = other DNA
ctgaccatcacacactatgcctgggtgg

SEQ ID NO: 35998 - DNA, 28 bp, synthetic construct
  source 1..28: mol_type = other DNA
acagccacccaggcatagtgtgtgatgg

SEQ ID NO: 35999 - DNA, 28 bp, synthetic construct
  source 1..28: mol_type = other DNA
atcacacactatgcctgggtggctgtgg

SEQ ID NO: 36000 - DNA, 28 bp, synthetic construct
  source 1..28: mol_type = other DNA
ctatgcctgggtggctgtggatgcaagg

SEQ ID NO: 36001 - DNA, 28 bp, synthetic construct
  source 1..28: mol_type = other DNA
tatgcctgggtggctgtggatgcaaggg

SEQ ID NO: 36002 - DNA, 28 bp, synthetic construct
  source 1..28: mol_type = other DNA
gtgacccttgcatccacagccacccagg

SEQ ID NO: 36003 - DNA, 28 bp, synthetic construct
  source 1..28: mol_type = other DNA
gggtggctgtggatgcaagggtcacagg

SEQ ID NO: 36004 - DNA, 28 bp, synthetic construct
  source 1..28: mol_type = other DNA
ggtggctgtggatgcaagggtcacaggg

SEQ ID NO: 36005 - DNA, 28 bp, synthetic construct
  source 1..28: mol_type = other DNA
tggatgcaagggtcacagggacatgtgg

SEQ ID NO: 36006 - DNA, 28 bp, synthetic construct
  source 1..28: mol_type = other DNA
ggatgcaagggtcacagggacatgtggg

SEQ ID NO: 36007 - DNA, 28 bp, synthetic construct
  source 1..28: mol_type = other DNA
cagggacatgtgggcttccctttgcagg

SEQ ID NO: 36008 - DNA, 28 bp, synthetic construct
  source 1..28: mol_type = other DNA
agggacatgtgggcttccctttgcaggg

SEQ ID NO: 36009 - DNA, 28 bp, synthetic construct
  source 1..28: mol_type = other DNA
gggacatgtgggcttccctttgcagggg

SEQ ID NO: 36010 - DNA, 28 bp, synthetic construct
  source 1..28: mol_type = other DNA
gtacacatgttcacaaccatcctctggg

SEQ ID NO: 36011 - DNA, 28 bp, synthetic construct
  source 1..28: mol_type = other DNA
tgtacacatgttcacaaccatcctctgg

SEQ ID NO: 36012 - DNA, 28 bp, synthetic construct
  source 1..28: mol_type = other DNA
ggttgtgaacatgtgtacataagtgtgg

SEQ ID NO: 36013 - DNA, 28 bp, synthetic construct
  source 1..28: mol_type = other DNA
gttgtgaacatgtgtacataagtgtggg

SEQ ID NO: 36014 - DNA, 28 bp, synthetic construct
  source 1..28: mol_type = other DNA
ataagtgtgggtgtacccatgaacctgg

SEQ ID NO: 36015 - DNA, 28 bp, synthetic construct
  source 1..28: mol_type = other DNA
taagtgtgggtgtacccatgaacctggg

SEQ ID NO: 36016 - DNA, 28 bp, synthetic construct
  source 1..28: mol_type = other DNA
tgggtgtacccatgaacctgggtattgg

SEQ ID NO: 36017 - DNA, 28 bp, synthetic construct
  source 1..28: mol_type = other DNA
gtacccatgaacctgggtattggtgcgg

SEQ ID NO: 36018 - DNA, 28 bp, synthetic construct
  source 1..28: mol_type = other DNA
tacccatgaacctgggtattggtgcggg

SEQ ID NO: 36019 - DNA, 28 bp, synthetic construct
  source 1..28: mol_type = other DNA
cacccgcaccaatacccaggttcatggg

SEQ ID NO: 36020 - DNA, 28 bp, synthetic construct
  source 1..28: mol_type = other DNA
tcacccgcaccaatacccaggttcatgg

SEQ ID NO: 36021 - DNA, 28 bp, synthetic construct
  source 1..28: mol_type = other DNA
cacagaatcacccgcaccaatacccagg

SEQ ID NO: 36022 - DNA, 28 bp, synthetic construct
  source 1..28: mol_type = other DNA
ggtattggtgcgggtgattctgtgcagg

SEQ ID NO: 36023 - DNA, 28 bp, synthetic construct
  source 1..28: mol_type = other DNA
gtctaattccctctgcccctcacagtgg

SEQ ID NO: 36024 - DNA, 28 bp, synthetic construct
  source 1..28: mol_type = other DNA
ccgaaggaccactgtgaggggcagaggg

SEQ ID NO: 36025 - DNA, 28 bp, synthetic construct
  source 1..28: mol_type = other DNA
cccgaaggaccactgtgaggggcagagg

SEQ ID NO: 36026 - DNA, 28 bp, synthetic construct
  source 1..28: mol_type = other DNA
ctctgcccctcacagtggtccttcgggg

SEQ ID NO: 36027 - DNA, 28 bp, synthetic construct
  source 1..28: mol_type = other DNA
tgtcaccccgaaggaccactgtgagggg

SEQ ID NO: 36028 - DNA, 28 bp, synthetic construct
  source 1..28: mol_type = other DNA
ttgtcaccccgaaggaccactgtgaggg

SEQ ID NO: 36029 - DNA, 28 bp, synthetic construct
  source 1..28: mol_type = other DNA
attgtcaccccgaaggaccactgtgagg

SEQ ID NO: 36030 - DNA, 28 bp, synthetic construct
  source 1..28: mol_type = other DNA
acagtggtccttcggggtgacaatgtgg

SEQ ID NO: 36031 - DNA, 28 bp, synthetic construct
  source 1..28: mol_type = other DNA
cagtggtccttcggggtgacaatgtggg

SEQ ID NO: 36032 - DNA, 28 bp, synthetic construct
  source 1..28: mol_type = other DNA
gcaatctcccacattgtcaccccgaagg

SEQ ID NO: 36033 - DNA, 28 bp, synthetic construct
  source 1..28: mol_type = other DNA
tgacaatgtgggagattgccacaagagg

SEQ ID NO: 36034 - DNA, 28 bp, synthetic construct
  source 1..28: mol_type = other DNA
gccacaagaggccaaaccccatatccgg

SEQ ID NO: 36035 - DNA, 28 bp, synthetic construct
  source 1..28: mol_type = other DNA
ccacaagaggccaaaccccatatccggg

SEQ ID NO: 36036 - DNA, 28 bp, synthetic construct
  source 1..28: mol_type = other DNA
agaggccaaaccccatatccgggcgtgg

SEQ ID NO: 36037 - DNA, 28 bp, synthetic construct
  source 1..28: mol_type = other DNA
gttctccacgcccggatatggggtttgg

SEQ ID NO: 36038 - DNA, 28 bp, synthetic construct
  source 1..28: mol_type = other DNA
tcgctgttctccacgcccggatatgggg

SEQ ID NO: 36039 - DNA, 28 bp, synthetic construct
  source 1..28: mol_type = other DNA
ctcgctgttctccacgcccggatatggg

SEQ ID NO: 36040 - DNA, 28 bp, synthetic construct
  source 1..28: mol_type = other DNA
tctcgctgttctccacgcccggatatgg

SEQ ID NO: 36041 - DNA, 28 bp, synthetic construct
  source 1..28: mol_type = other DNA
cataaatctcgctgttctccacgcccgg

SEQ ID NO: 36042 - DNA, 28 bp, synthetic construct
  source 1..28: mol_type = other DNA
agcgagatttatgactatctgcgccagg

SEQ ID NO: 36043 - DNA, 28 bp, synthetic construct
  source 1..28: mol_type = other DNA
gcgagatttatgactatctgcgccaggg

SEQ ID NO: 36044 - DNA, 28 bp, synthetic construct
  source 1..28: mol_type = other DNA
cgcaggctgcttcaggcgatttccctgg

SEQ ID NO: 36045 - DNA, 28 bp, synthetic construct
  source 1..28: mol_type = other DNA
cagggaaatcgcctgaagcagcctgcgg

SEQ ID NO: 36046 - DNA, 28 bp, synthetic construct
  source 1..28: mol_type = other DNA
cgcctgaagcagcctgcggactgtctgg

SEQ ID NO: 36047 - DNA, 28 bp, synthetic construct
  source 1..28: mol_type = other DNA
atccagacagtccgcaggctgcttcagg

SEQ ID NO: 36048 - DNA, 28 bp, synthetic construct
  source 1..28: mol_type = other DNA
tgaagcagcctgcggactgtctggatgg

SEQ ID NO: 36049 - DNA, 28 bp, synthetic construct
  source 1..28: mol_type = other DNA
ctcacagtccatccagacagtccgcagg

SEQ ID NO: 36050 - DNA, 28 bp, synthetic construct
  source 1..28: mol_type = other DNA
ctgcggactgtctggatggactgtgagg

SEQ ID NO: 36051 - DNA, 28 bp, synthetic construct
  source 1..28: mol_type = other DNA
gtctggatggactgtgaggacccttagg

SEQ ID NO: 36052 - DNA, 28 bp, synthetic construct
  source 1..28: mol_type = other DNA
gaattctgggttgggggagacctaaggg

SEQ ID NO: 36053 - DNA, 28 bp, synthetic construct
  source 1..28: mol_type = other DNA
tgaattctgggttgggggagacctaagg

SEQ ID NO: 36054 - DNA, 28 bp, synthetic construct
  source 1..28: mol_type = other DNA
gggtttggaatgaattctgggttggggg

SEQ ID NO: 36055 - DNA, 28 bp, synthetic construct
  source 1..28: mol_type = other DNA
ggggtttggaatgaattctgggttgggg

SEQ ID NO: 36056 - DNA, 28 bp, synthetic construct
  source 1..28: mol_type = other DNA
aggggtttggaatgaattctgggttggg

SEQ ID NO: 36057 - DNA, 28 bp, synthetic construct
  source 1..28: mol_type = other DNA
caggggtttggaatgaattctgggttgg

SEQ ID NO: 36058 - DNA, 28 bp, synthetic construct
  source 1..28: mol_type = other DNA
tagtcaggggtttggaatgaattctggg

SEQ ID NO: 36059 - DNA, 28 bp, synthetic construct
  source 1..28: mol_type = other DNA
gtagtcaggggtttggaatgaattctgg

SEQ ID NO: 36060 - DNA, 28 bp, synthetic construct
  source 1..28: mol_type = other DNA
ttccaaacccctgactacccccagatgg

SEQ ID NO: 36061 - DNA, 28 bp, synthetic construct
  source 1..28: mol_type = other DNA
ggccatctgggggtagtcaggggtttgg

SEQ ID NO: 36062 - DNA, 28 bp, synthetic construct
  source 1..28: mol_type = other DNA
gtgagggccatctgggggtagtcagggg

SEQ ID NO: 36063 - DNA, 28 bp, synthetic construct
  source 1..28: mol_type = other DNA
tgtgagggccatctgggggtagtcaggg

SEQ ID NO: 36064 - DNA, 28 bp, synthetic construct
  source 1..28: mol_type = other DNA
ctgtgagggccatctgggggtagtcagg

SEQ ID NO: 36065 - DNA, 28 bp, synthetic construct
  source 1..28: mol_type = other DNA
ctgactacccccagatggccctcacagg

SEQ ID NO: 36066 - DNA, 28 bp, synthetic construct
  source 1..28: mol_type = other DNA
acccccagatggccctcacaggtccagg

SEQ ID NO: 36067 - DNA, 28 bp, synthetic construct
  source 1..28: mol_type = other DNA
tcctggacctgtgagggccatctggggg

SEQ ID NO: 36068 - DNA, 28 bp, synthetic construct
  source 1..28: mol_type = other DNA
gtcctggacctgtgagggccatctgggg

SEQ ID NO: 36069 - DNA, 28 bp, synthetic construct
  source 1..28: mol_type = other DNA
agtcctggacctgtgagggccatctggg

SEQ ID NO: 36070 - DNA, 28 bp, synthetic construct
  source 1..28: mol_type = other DNA
gagtcctggacctgtgagggccatctgg

SEQ ID NO: 36071 - DNA, 28 bp, synthetic construct
  source 1..28: mol_type = other DNA
gttatagagagtcctggacctgtgaggg

SEQ ID NO: 36072 - DNA, 28 bp, synthetic construct
  source 1..28: mol_type = other DNA
ggttatagagagtcctggacctgtgagg

SEQ ID NO: 36073 - DNA, 28 bp, synthetic construct
  source 1..28: mol_type = other DNA
attctgtctgggttatagagagtcctgg

SEQ ID NO: 36074 - DNA, 28 bp, synthetic construct
  source 1..28: mol_type = other DNA
ctcagcattctcagggattctgtctggg

SEQ ID NO: 36075 - DNA, 28 bp, synthetic construct
  source 1..28: mol_type = other DNA
actcagcattctcagggattctgtctgg

SEQ ID NO: 36076 - DNA, 28 bp, synthetic construct
  source 1..28: mol_type = other DNA
actgggggcattttagagggttataggg

SEQ ID NO: 36077 - DNA, 28 bp, synthetic construct
  source 1..28: mol_type = other DNA
gactgggggcattttagagggttatagg

SEQ ID NO: 36078 - DNA, 28 bp, synthetic construct
  source 1..28: mol_type = other DNA
ctcaggggactgggggcattttagaggg

SEQ ID NO: 36079 - DNA, 28 bp, synthetic construct
  source 1..28: mol_type = other DNA
actcaggggactgggggcattttagagg

SEQ ID NO: 36080 - DNA, 28 bp, synthetic construct
  source 1..28: mol_type = other DNA
cattttaggacactcaggggactggggg

SEQ ID NO: 36081 - DNA, 28 bp, synthetic construct
  source 1..28: mol_type = other DNA
acattttaggacactcaggggactgggg

SEQ ID NO: 36082 - DNA, 28 bp, synthetic construct
  source 1..28: mol_type = other DNA
gacattttaggacactcaggggactggg

SEQ ID NO: 36083 - DNA, 28 bp, synthetic construct
  source 1..28: mol_type = other DNA
ggacattttaggacactcaggggactgg

SEQ ID NO: 36084 - DNA, 28 bp, synthetic construct
  source 1..28: mol_type = other DNA
cccctgagtgtcctaaaatgtccccagg

SEQ ID NO: 36085 - DNA, 28 bp, synthetic construct
  source 1..28: mol_type = other DNA
gcctggggacattttaggacactcaggg

SEQ ID NO: 36086 - DNA, 28 bp, synthetic construct
  source 1..28: mol_type = other DNA
agcctggggacattttaggacactcagg

SEQ ID NO: 36087 - DNA, 28 bp, synthetic construct
  source 1..28: mol_type = other DNA
cattctggaagcctggggacattttagg

SEQ ID NO: 36088 - DNA, 28 bp, synthetic construct
  source 1..28: mol_type = other DNA
agaaggggtgcattctggaagcctgggg

SEQ ID NO: 36089 - DNA, 28 bp, synthetic construct
  source 1..28: mol_type = other DNA
cagaaggggtgcattctggaagcctggg

SEQ ID NO: 36090 - DNA, 28 bp, synthetic construct
  source 1..28: mol_type = other DNA
tcagaaggggtgcattctggaagcctgg

SEQ ID NO: 36091 - DNA, 28 bp, synthetic construct
  source 1..28: mol_type = other DNA
gcagggactcagaaggggtgcattctgg

SEQ ID NO: 36092 - DNA, 28 bp, synthetic construct
  source 1..28: mol_type = other DNA
gggagattgagcagggactcagaagggg

SEQ ID NO: 36093 - DNA, 28 bp, synthetic construct
  source 1..28: mol_type = other DNA
tgggagattgagcagggactcagaaggg

SEQ ID NO: 36094 - DNA, 28 bp, synthetic construct
  source 1..28: mol_type = other DNA
gtgggagattgagcagggactcagaagg

SEQ ID NO: 36095 - DNA, 28 bp, synthetic construct
  source 1..28: mol_type = other DNA
aaaatgaggggtgggagattgagcaggg

SEQ ID NO: 36096 - DNA, 28 bp, synthetic construct
  source 1..28: mol_type = other DNA
caaaatgaggggtgggagattgagcagg

SEQ ID NO: 36097 - DNA, 28 bp, synthetic construct
  source 1..28: mol_type = other DNA
ctcccacccctcattttgctgccctagg

SEQ ID NO: 36098 - DNA, 28 bp, synthetic construct
  source 1..28: mol_type = other DNA
tacctagggcagcaaaatgaggggtggg

SEQ ID NO: 36099 - DNA, 28 bp, synthetic construct
  source 1..28: mol_type = other DNA
atacctagggcagcaaaatgaggggtgg

SEQ ID NO: 36100 - DNA, 28 bp, synthetic construct
  source 1..28: mol_type = other DNA
ggcatacctagggcagcaaaatgagggg

SEQ ID NO: 36101 - DNA, 28 bp, synthetic construct
  source 1..28: mol_type = other DNA
aggcatacctagggcagcaaaatgaggg

SEQ ID NO: 36102 - DNA, 28 bp, synthetic construct
  source 1..28: mol_type = other DNA
aaggcatacctagggcagcaaaatgagg

SEQ ID NO: 36103 - DNA, 28 bp, synthetic construct
  source 1..28: mol_type = other DNA
ctgccctaggtatgccttgatgtcgcgg

SEQ ID NO: 36104 - DNA, 28 bp, synthetic construct
  source 1..28: mol_type = other DNA
gcaccgcgacatcaaggcatacctaggg

SEQ ID NO: 36105 - DNA, 28 bp, synthetic construct
  source 1..28: mol_type = other DNA
agcaccgcgacatcaaggcatacctagg

SEQ ID NO: 36106 - DNA, 28 bp, synthetic construct
  source 1..28: mol_type = other DNA
taggtatgccttgatgtcgcggtgctgg

SEQ ID NO: 36107 - DNA, 28 bp, synthetic construct
  source 1..28: mol_type = other DNA
aggtatgccttgatgtcgcggtgctggg

SEQ ID NO: 36108 - DNA, 28 bp, synthetic construct
  source 1..28: mol_type = other DNA
tttagctcccagcaccgcgacatcaagg

SEQ ID NO: 36109 - DNA, 28 bp, synthetic construct
  source 1..28: mol_type = other DNA
tcgcggtgctgggagctaaatccccagg

SEQ ID NO: 36110 - DNA, 28 bp, synthetic construct
  source 1..28: mol_type = other DNA
gtgctgggagctaaatccccaggaccgg

SEQ ID NO: 36111 - DNA, 28 bp, synthetic construct
  source 1..28: mol_type = other DNA
gctctgtaaaacttggccggtcctgggg

SEQ ID NO: 36112 - DNA, 28 bp, synthetic construct
  source 1..28: mol_type = other DNA
agctctgtaaaacttggccggtcctggg

SEQ ID NO: 36113 - DNA, 28 bp, synthetic construct
  source 1..28: mol_type = other DNA
cagctctgtaaaacttggccggtcctgg

SEQ ID NO: 36114 - DNA, 28 bp, synthetic construct
  source 1..28: mol_type = other DNA
ggaccggccaagttttacagagctgcgg

SEQ ID NO: 36115 - DNA, 28 bp, synthetic construct
  source 1..28: mol_type = other DNA
gaccggccaagttttacagagctgcggg

SEQ ID NO: 36116 - DNA, 28 bp, synthetic construct
  source 1..28: mol_type = other DNA
ttcccgcagctctgtaaaacttggccgg

SEQ ID NO: 36117 - DNA, 28 bp, synthetic construct
  source 1..28: mol_type = other DNA
aatcttcccgcagctctgtaaaacttgg

SEQ ID NO: 36118 - DNA, 28 bp, synthetic construct
  source 1..28: mol_type = other DNA
agttttacagagctgcgggaagatttgg

SEQ ID NO: 36119 - DNA, 28 bp, synthetic construct
  source 1..28: mol_type = other DNA
cgggaagatttggagaacacactgaagg

SEQ ID NO: 36120 - DNA, 28 bp, synthetic construct
  source 1..28: mol_type = other DNA
acactgaaggccttgcctcctgcccagg

SEQ ID NO: 36121 - DNA, 28 bp, synthetic construct
  source 1..28: mol_type = other DNA
tcgtcaggctcctgggcaggaggcaagg

SEQ ID NO: 36122 - DNA, 28 bp, synthetic construct
  source 1..28: mol_type = other DNA
ggatttcgtcaggctcctgggcaggagg

SEQ ID NO: 36123 - DNA, 28 bp, synthetic construct
  source 1..28: mol_type = other DNA
agaggatttcgtcaggctcctgggcagg

SEQ ID NO: 36124 - DNA, 28 bp, synthetic construct
  source 1..28: mol_type = other DNA
acatagaggatttcgtcaggctcctggg

SEQ ID NO: 36125 - DNA, 28 bp, synthetic construct
  source 1..28: mol_type = other DNA
gacatagaggatttcgtcaggctcctgg

SEQ ID NO: 36126 - DNA, 28 bp, synthetic construct
  source 1..28: mol_type = other DNA
ccatgttgacatagaggatttcgtcagg

SEQ ID NO: 36127 - DNA, 28 bp, synthetic construct
  source 1..28: mol_type = other DNA
gaaatcctctatgtcaacatggatgagg

SEQ ID NO: 36128 - DNA, 28 bp, synthetic construct
  source 1..28: mol_type = other DNA
aaatcctctatgtcaacatggatgaggg

SEQ ID NO: 36129 - DNA, 28 bp, synthetic construct
  source 1..28: mol_type = other DNA
tcctctatgtcaacatggatgagggtgg

SEQ ID NO: 36130 - DNA, 28 bp, synthetic construct
  source 1..28: mol_type = other DNA
tccaccctcatccatgttgacatagagg

SEQ ID NO: 36131 - DNA, 28 bp, synthetic construct
  source 1..28: mol_type = other DNA
tctatgtcaacatggatgagggtggagg

SEQ ID NO: 36132 - DNA, 28 bp, synthetic construct
  source 1..28: mol_type = other DNA
agggtggaggttatcctgaaccccctgg

SEQ ID NO: 36133 - DNA, 28 bp, synthetic construct
  source 1..28: mol_type = other DNA
gttatcctgaaccccctggagctgcagg

SEQ ID NO: 36134 - DNA, 28 bp, synthetic construct
  source 1..28: mol_type = other DNA
atcctgaaccccctggagctgcaggagg

SEQ ID NO: 36135 - DNA, 28 bp, synthetic construct
  source 1..28: mol_type = other DNA
ctcctcctgcagctccagggggttcagg

SEQ ID NO: 36136 - DNA, 28 bp, synthetic construct
  source 1..28: mol_type = other DNA
ggtcagctcctcctgcagctccaggggg

SEQ ID NO: 36137 - DNA, 28 bp, synthetic construct
  source 1..28: mol_type = other DNA
gggtcagctcctcctgcagctccagggg

SEQ ID NO: 36138 - DNA, 28 bp, synthetic construct
  source 1..28: mol_type = other DNA
ggggtcagctcctcctgcagctccaggg

SEQ ID NO: 36139 - DNA, 28 bp, synthetic construct
  source 1..28: mol_type = other DNA
gggggtcagctcctcctgcagctccagg

SEQ ID NO: 36140 - DNA, 28 bp, synthetic construct
  source 1..28: mol_type = other DNA
gaccccccaacccagccagaccctaagg

SEQ ID NO: 36141 - DNA, 28 bp, synthetic construct
  source 1..28: mol_type = other DNA
atccttagggtctggctgggttgggggg

SEQ ID NO: 36142 - DNA, 28 bp, synthetic construct
  source 1..28: mol_type = other DNA
aatccttagggtctggctgggttggggg

SEQ ID NO: 36143 - DNA, 28 bp, synthetic construct
  source 1..28: mol_type = other DNA
gaatccttagggtctggctgggttgggg

SEQ ID NO: 36144 - DNA, 28 bp, synthetic construct
  source 1..28: mol_type = other DNA
ggaatccttagggtctggctgggttggg

SEQ ID NO: 36145 - DNA, 28 bp, synthetic construct
  source 1..28: mol_type = other DNA
aggaatccttagggtctggctgggttgg

SEQ ID NO: 36146 - DNA, 28 bp, synthetic construct
  source 1..28: mol_type = other DNA
ctacaggaatccttagggtctggctggg

SEQ ID NO: 36147 - DNA, 28 bp, synthetic construct
  source 1..28: mol_type = other DNA
gctacaggaatccttagggtctggctgg

SEQ ID NO: 36148 - DNA, 28 bp, synthetic construct
  source 1..28: mol_type = other DNA
ggcagctacaggaatccttagggtctgg

SEQ ID NO: 36149 - DNA, 28 bp, synthetic construct
  source 1..28: mol_type = other DNA
agtgaggcagctacaggaatccttaggg

SEQ ID NO: 36150 - DNA, 28 bp, synthetic construct
  source 1..28: mol_type = other DNA
cagtgaggcagctacaggaatccttagg

SEQ ID NO: 36151 - DNA, 28 bp, synthetic construct
  source 1..28: mol_type = other DNA
aaggattcctgtagctgcctcactgcgg

SEQ ID NO: 36152 - DNA, 28 bp, synthetic construct
  source 1..28: mol_type = other DNA
tcctgtagctgcctcactgcggctgagg

SEQ ID NO: 36153 - DNA, 28 bp, synthetic construct
  source 1..28: mol_type = other DNA
acctcagccgcagtgaggcagctacagg

SEQ ID NO: 36154 - DNA, 28 bp, synthetic construct
  source 1..28: mol_type = other DNA
agcaggatggacctcagccgcagtgagg

SEQ ID NO: 36155 - DNA, 28 bp, synthetic construct
  source 1..28: mol_type = other DNA
tcactgcggctgaggtccatcctgctgg

SEQ ID NO: 36156 - DNA, 28 bp, synthetic construct
  source 1..28: mol_type = other DNA
gcagaggacatagcgtccagcaggatgg

SEQ ID NO: 36157 - DNA, 28 bp, synthetic construct
  source 1..28: mol_type = other DNA
aagggcagaggacatagcgtccagcagg

SEQ ID NO: 36158 - DNA, 28 bp, synthetic construct
  source 1..28: mol_type = other DNA
ggggctaggggttgtggaagggcagagg

SEQ ID NO: 36159 - DNA, 28 bp, synthetic construct
  source 1..28: mol_type = other DNA
ctgagcggggctaggggttgtggaaggg

SEQ ID NO: 36160 - DNA, 28 bp, synthetic construct
  source 1..28: mol_type = other DNA
gctgagcggggctaggggttgtggaagg

SEQ ID NO: 36161 - DNA, 28 bp, synthetic construct
  source 1..28: mol_type = other DNA
gcaggctgagcggggctaggggttgtgg

SEQ ID NO: 36162 - DNA, 28 bp, synthetic construct
  source 1..28: mol_type = other DNA
ctatcagcaggctgagcggggctagggg

SEQ ID NO: 36163 - DNA, 28 bp, synthetic construct
  source 1..28: mol_type = other DNA
cctatcagcaggctgagcggggctaggg

SEQ ID NO: 36164 - DNA, 28 bp, synthetic construct
  source 1..28: mol_type = other DNA
ccctatcagcaggctgagcggggctagg

SEQ ID NO: 36165 - DNA, 28 bp, synthetic construct
  source 1..28: mol_type = other DNA
ctagccccgctcagcctgctgatagggg

SEQ ID NO: 36166 - DNA, 28 bp, synthetic construct
  source 1..28: mol_type = other DNA
ggagcccctatcagcaggctgagcgggg

SEQ ID NO: 36167 - DNA, 28 bp, synthetic construct
  source 1..28: mol_type = other DNA
gggagcccctatcagcaggctgagcggg

SEQ ID NO: 36168 - DNA, 28 bp, synthetic construct
  source 1..28: mol_type = other DNA
ggggagcccctatcagcaggctgagcgg

SEQ ID NO: 36169 - DNA, 28 bp, synthetic construct
  source 1..28: mol_type = other DNA
gggctgctggggagcccctatcagcagg

SEQ ID NO: 36170 - DNA, 28 bp, synthetic construct
  source 1..28: mol_type = other DNA
ctgataggggctccccagcagccccagg

SEQ ID NO: 36171 - DNA, 28 bp, synthetic construct
  source 1..28: mol_type = other DNA
tgataggggctccccagcagccccaggg

SEQ ID NO: 36172 - DNA, 28 bp, synthetic construct
  source 1..28: mol_type = other DNA
aggggctccccagcagccccagggcagg

SEQ ID NO: 36173 - DNA, 28 bp, synthetic construct
  source 1..28: mol_type = other DNA
ggctccccagcagccccagggcaggagg

SEQ ID NO: 36174 - DNA, 28 bp, synthetic construct
  source 1..28: mol_type = other DNA
ccatcctcctgccctggggctgctgggg

SEQ ID NO: 36175 - DNA, 28 bp, synthetic construct
  source 1..28: mol_type = other DNA
accatcctcctgccctggggctgctggg

SEQ ID NO: 36176 - DNA, 28 bp, synthetic construct
  source 1..28: mol_type = other DNA
caccatcctcctgccctggggctgctgg

SEQ ID NO: 36177 - DNA, 28 bp, synthetic construct
  source 1..28: mol_type = other DNA
tctcaggcaccatcctcctgccctgggg

SEQ ID NO: 36178 - DNA, 28 bp, synthetic construct
  source 1..28: mol_type = other DNA
gtctcaggcaccatcctcctgccctggg

SEQ ID NO: 36179 - DNA, 28 bp, synthetic construct
  source 1..28: mol_type = other DNA
tgtctcaggcaccatcctcctgccctgg

SEQ ID NO: 36180 - DNA, 28 bp, synthetic construct
  source 1..28: mol_type = other DNA
atggtgcctgagacaaccctccacctgg

SEQ ID NO: 36181 - DNA, 28 bp, synthetic construct
  source 1..28: mol_type = other DNA
ggagtaccaggtggagggttgtctcagg

SEQ ID NO: 36182 - DNA, 28 bp, synthetic construct
  source 1..28: mol_type = other DNA
aaccctccacctggtactccctctcagg

SEQ ID NO: 36183 - DNA, 28 bp, synthetic construct
  source 1..28: mol_type = other DNA
atcctgagagggagtaccaggtggaggg

SEQ ID NO: 36184 - DNA, 28 bp, synthetic construct
  source 1..28: mol_type = other DNA
gatcctgagagggagtaccaggtggagg

SEQ ID NO: 36185 - DNA, 28 bp, synthetic construct
  source 1..28: mol_type = other DNA
ttggatcctgagagggagtaccaggtgg

SEQ ID NO: 36186 - DNA, 28 bp, synthetic construct
  source 1..28: mol_type = other DNA
agcttggatcctgagagggagtaccagg

SEQ ID NO: 36187 - DNA, 28 bp, synthetic construct
  source 1..28: mol_type = other DNA
gcagtgcttagcttggatcctgagaggg

SEQ ID NO: 36188 - DNA, 28 bp, synthetic construct
  source 1..28: mol_type = other DNA
ggcagtgcttagcttggatcctgagagg

SEQ ID NO: 36189 - DNA, 28 bp, synthetic construct
  source 1..28: mol_type = other DNA
caggatccaagctaagcactgccactgg

SEQ ID NO: 36190 - DNA, 28 bp, synthetic construct
  source 1..28: mol_type = other DNA
aggatccaagctaagcactgccactggg

SEQ ID NO: 36191 - DNA, 28 bp, synthetic construct
  source 1..28: mol_type = other DNA
ggatccaagctaagcactgccactgggg

SEQ ID NO: 36192 - DNA, 28 bp, synthetic construct
  source 1..28: mol_type = other DNA
ttttccccagtggcagtgcttagcttgg

SEQ ID NO: 36193 - DNA, 28 bp, synthetic construct
  source 1..28: mol_type = other DNA
agtgggaaggtggagttttccccagtgg

SEQ ID NO: 36194 - DNA, 28 bp, synthetic construct
  source 1..28: mol_type = other DNA
ggcgtggggtgggaaagtgggaaggtgg

SEQ ID NO: 36195 - DNA, 28 bp, synthetic construct
  source 1..28: mol_type = other DNA
taaggcgtggggtgggaaagtgggaagg

SEQ ID NO: 36196 - DNA, 28 bp, synthetic construct
  source 1..28: mol_type = other DNA
gggataaggcgtggggtgggaaagtggg

SEQ ID NO: 36197 - DNA, 28 bp, synthetic construct
  source 1..28: mol_type = other DNA
ggggataaggcgtggggtgggaaagtgg

SEQ ID NO: 36198 - DNA, 28 bp, synthetic construct
  source 1..28: mol_type = other DNA
tgcaagtggggataaggcgtggggtggg

SEQ ID NO: 36199 - DNA, 28 bp, synthetic construct
  source 1..28: mol_type = other DNA
ctgcaagtggggataaggcgtggggtgg

SEQ ID NO: 36200 - DNA, 28 bp, synthetic construct
  source 1..28: mol_type = other DNA
gggctgcaagtggggataaggcgtgggg

SEQ ID NO: 36201 - DNA, 28 bp, synthetic construct
  source 1..28: mol_type = other DNA
agggctgcaagtggggataaggcgtggg

SEQ ID NO: 36202 - DNA, 28 bp, synthetic construct
  source 1..28: mol_type = other DNA
cagggctgcaagtggggataaggcgtgg

SEQ ID NO: 36203 - DNA, 28 bp, synthetic construct
  source 1..28: mol_type = other DNA
gaagacagggctgcaagtggggataagg

SEQ ID NO: 36204 - DNA, 28 bp, synthetic construct
  source 1..28: mol_type = other DNA
aggtaggaagacagggctgcaagtgggg

SEQ ID NO: 36205 - DNA, 28 bp, synthetic construct
  source 1..28: mol_type = other DNA
taggtaggaagacagggctgcaagtggg

SEQ ID NO: 36206 - DNA, 28 bp, synthetic construct
  source 1..28: mol_type = other DNA
ataggtaggaagacagggctgcaagtgg

SEQ ID NO: 36207 - DNA, 28 bp, synthetic construct
  source 1..28: mol_type = other DNA
tggaggtgggataggtaggaagacaggg

SEQ ID NO: 36208 - DNA, 28 bp, synthetic construct
  source 1..28: mol_type = other DNA
atggaggtgggataggtaggaagacagg

SEQ ID NO: 36209 - DNA, 28 bp, synthetic construct
  source 1..28: mol_type = other DNA
tgtctgggatggaggtgggataggtagg

SEQ ID NO: 36210 - DNA, 28 bp, synthetic construct
  source 1..28: mol_type = other DNA
tacctatcccacctccatcccagacagg

SEQ ID NO: 36211 - DNA, 28 bp, synthetic construct
  source 1..28: mol_type = other DNA
gacctgtctgggatggaggtgggatagg

SEQ ID NO: 36212 - DNA, 28 bp, synthetic construct
  source 1..28: mol_type = other DNA
ggagggacctgtctgggatggaggtggg

SEQ ID NO: 36213 - DNA, 28 bp, synthetic construct
  source 1..28: mol_type = other DNA
gggagggacctgtctgggatggaggtgg

SEQ ID NO: 36214 - DNA, 28 bp, synthetic construct
  source 1..28: mol_type = other DNA
aaggggagggacctgtctgggatggagg

SEQ ID NO: 36215 - DNA, 28 bp, synthetic construct
  source 1..28: mol_type = other DNA
gagaaggggagggacctgtctgggatgg

SEQ ID NO: 36216 - DNA, 28 bp, synthetic construct
  source 1..28: mol_type = other DNA
cacagagaaggggagggacctgtctggg

SEQ ID NO: 36217 - DNA, 28 bp, synthetic construct
  source 1..28: mol_type = other DNA
gcacagagaaggggagggacctgtctgg

SEQ ID NO: 36218 - DNA, 28 bp, synthetic construct
  source 1..28: mol_type = other DNA
tgatgctactgcacagagaaggggaggg

SEQ ID NO: 36219 - DNA, 28 bp, synthetic construct
  source 1..28: mol_type = other DNA
gtgatgctactgcacagagaaggggagg

SEQ ID NO: 36220 - DNA, 28 bp, synthetic construct
  source 1..28: mol_type = other DNA
aaggtgatgctactgcacagagaagggg

SEQ ID NO: 36221 - DNA, 28 bp, synthetic construct
  source 1..28: mol_type = other DNA
caaggtgatgctactgcacagagaaggg

SEQ ID NO: 36222 - DNA, 28 bp, synthetic construct
  source 1..28: mol_type = other DNA
tcaaggtgatgctactgcacagagaagg

SEQ ID NO: 36223 - DNA, 28 bp, synthetic construct
  source 1..28: mol_type = other DNA
acagatggtgatgctactgctttcaagg

SEQ ID NO: 36224 - DNA, 28 bp, synthetic construct
  source 1..28: mol_type = other DNA
aagcagtagcatcaccatctgtaaaagg

SEQ ID NO: 36225 - DNA, 28 bp, synthetic construct
  source 1..28: mol_type = other DNA
agtagcatcaccatctgtaaaaggaagg

SEQ ID NO: 36226 - DNA, 28 bp, synthetic construct
  source 1..28: mol_type = other DNA
gtagcatcaccatctgtaaaaggaaggg

SEQ ID NO: 36227 - DNA, 28 bp, synthetic construct
  source 1..28: mol_type = other DNA
tagcatcaccatctgtaaaaggaagggg

SEQ ID NO: 36228 - DNA, 28 bp, synthetic construct
  source 1..28: mol_type = other DNA
atcaccatctgtaaaaggaaggggttgg

SEQ ID NO: 36229 - DNA, 28 bp, synthetic construct
  source 1..28: mol_type = other DNA
caatccaaccccttccttttacagatgg

SEQ ID NO: 36230 - DNA, 28 bp, synthetic construct
  source 1..28: mol_type = other DNA
ggattgcaatatctgaagccctcccagg

SEQ ID NO: 36231 - DNA, 28 bp, synthetic construct
  source 1..28: mol_type = other DNA
agtcttggaatgttaacacctgggaggg

SEQ ID NO: 36232 - DNA, 28 bp, synthetic construct
  source 1..28: mol_type = other DNA
gagtcttggaatgttaacacctgggagg

SEQ ID NO: 36233 - DNA, 28 bp, synthetic construct
  source 1..28: mol_type = other DNA
ctagagtcttggaatgttaacacctggg

SEQ ID NO: 36234 - DNA, 28 bp, synthetic construct
  source 1..28: mol_type = other DNA
tctagagtcttggaatgttaacacctgg

SEQ ID NO: 36235 - DNA, 28 bp, synthetic construct
  source 1..28: mol_type = other DNA
taacattccaagactctagagtccaagg

SEQ ID NO: 36236 - DNA, 28 bp, synthetic construct
  source 1..28: mol_type = other DNA
ctttaaaccttggactctagagtcttgg

SEQ ID NO: 36237 - DNA, 28 bp, synthetic construct
  source 1..28: mol_type = other DNA
ctttgaatctagactctttaaaccttgg

SEQ ID NO: 36238 - DNA, 28 bp, synthetic construct
  source 1..28: mol_type = other DNA
caaggtttaaagagtctagattcaaagg

SEQ ID NO: 36239 - DNA, 28 bp, synthetic construct
  source 1..28: mol_type = other DNA
taaagagtctagattcaaaggttctagg

SEQ ID NO: 36240 - DNA, 28 bp, synthetic construct
  source 1..28: mol_type = other DNA
aggtttcaaagatgctgtgagtctttgg

SEQ ID NO: 36241 - DNA, 28 bp, synthetic construct
  source 1..28: mol_type = other DNA
aagatgctgtgagtctttggttctaagg

SEQ ID NO: 36242 - DNA, 28 bp, synthetic construct
  source 1..28: mol_type = other DNA
atagaattagagactttggaatttcagg

SEQ ID NO: 36243 - DNA, 28 bp, synthetic construct
  source 1..28: mol_type = other DNA
agcactttaatagaattagagactttgg

SEQ ID NO: 36244 - DNA, 28 bp, synthetic construct
  source 1..28: mol_type = other DNA
agtctctaattctattaaagtgctaagg

SEQ ID NO: 36245 - DNA, 28 bp, synthetic construct
  source 1..28: mol_type = other DNA
attctattaaagtgctaaggttctaagg

SEQ ID NO: 36246 - DNA, 28 bp, synthetic construct
  source 1..28: mol_type = other DNA
aaaaaaaaaaaaaaaaaaaaaaagtagg

SEQ ID NO: 36247 - DNA, 28 bp, synthetic construct
  source 1..28: mol_type = other DNA
gcgatagagtctcactgtgtcacccagg

SEQ ID NO: 36248 - DNA, 28 bp, synthetic construct
  source 1..28: mol_type = other DNA
tagagtctcactgtgtcacccaggctgg

SEQ ID NO: 36249 - DNA, 28 bp, synthetic construct
  source 1..28: mol_type = other DNA
ctgtgtcacccaggctggagtgcagtgg

SEQ ID NO: 36250 - DNA, 28 bp, synthetic construct
  source 1..28: mol_type = other DNA
agattgcaccactgcactccagcctggg

SEQ ID NO: 36251 - DNA, 28 bp, synthetic construct
  source 1..28: mol_type = other DNA
gagattgcaccactgcactccagcctgg

SEQ ID NO: 36252 - DNA, 28 bp, synthetic construct
  source 1..28: mol_type = other DNA
aactcggtaggtgaaggttgcagtgagg

SEQ ID NO: 36253 - DNA, 28 bp, synthetic construct
  source 1..28: mol_type = other DNA
aaaatcacttgaactcggtaggtgaagg

SEQ ID NO: 36254 - DNA, 28 bp, synthetic construct
  source 1..28: mol_type = other DNA
ggcaggaaaatcacttgaactcggtagg

SEQ ID NO: 36255 - DNA, 28 bp, synthetic construct
  source 1..28: mol_type = other DNA
ccgagttcaagtgattttcctgccttgg

SEQ ID NO: 36256 - DNA, 28 bp, synthetic construct
  source 1..28: mol_type = other DNA
ttcctgccttggcctcccaagtagctgg

SEQ ID NO: 36257 - DNA, 28 bp, synthetic construct
  source 1..28: mol_type = other DNA
tcctgccttggcctcccaagtagctggg

SEQ ID NO: 36258 - DNA, 28 bp, synthetic construct
  source 1..28: mol_type = other DNA
tcccagctacttgggaggccaaggcagg

SEQ ID NO: 36259 - DNA, 28 bp, synthetic construct
  source 1..28: mol_type = other DNA
gtaatcccagctacttgggaggccaagg

SEQ ID NO: 36260 - DNA, 28 bp, synthetic construct
  source 1..28: mol_type = other DNA
tggcctcccaagtagctgggattacagg

SEQ ID NO: 36261 - DNA, 28 bp, synthetic construct
  source 1..28: mol_type = other DNA
acacctgtaatcccagctacttgggagg

SEQ ID NO: 36262 - DNA, 28 bp, synthetic construct
  source 1..28: mol_type = other DNA
cacacacctgtaatcccagctacttggg

SEQ ID NO: 36263 - DNA, 28 bp, synthetic construct
  source 1..28: mol_type = other DNA
gcacacacctgtaatcccagctacttgg

SEQ ID NO: 36264 - DNA, 28 bp, synthetic construct
  source 1..28: mol_type = other DNA
gattacaggtgtgtgccaccacacccgg

SEQ ID NO: 36265 - DNA, 28 bp, synthetic construct
  source 1..28: mol_type = other DNA
aaatataaaaattagccgggtgtggtgg

SEQ ID NO: 36266 - DNA, 28 bp, synthetic construct
  source 1..28: mol_type = other DNA
taaaaatataaaaattagccgggtgtgg

SEQ ID NO: 36267 - DNA, 28 bp, synthetic construct
  source 1..28: mol_type = other DNA
tctactaaaaatataaaaattagccggg

SEQ ID NO: 36268 - DNA, 28 bp, synthetic construct
  source 1..28: mol_type = other DNA
ctctactaaaaatataaaaattagccgg

SEQ ID NO: 36269 - DNA, 28 bp, synthetic construct
  source 1..28: mol_type = other DNA
taatttttatatttttagtagagacagg

SEQ ID NO: 36270 - DNA, 28 bp, synthetic construct
  source 1..28: mol_type = other DNA
aatttttatatttttagtagagacaggg

SEQ ID NO: 36271 - DNA, 28 bp, synthetic construct
  source 1..28: mol_type = other DNA
tagtagagacagggtttcaccatgttgg

SEQ ID NO: 36272 - DNA, 28 bp, synthetic construct
  source 1..28: mol_type = other DNA
gagacagggtttcaccatgttggccagg

SEQ ID NO: 36273 - DNA, 28 bp, synthetic construct
  source 1..28: mol_type = other DNA
cagggtttcaccatgttggccaggctgg

SEQ ID NO: 36274 - DNA, 28 bp, synthetic construct
  source 1..28: mol_type = other DNA
gagttttagaccagcctggccaacatgg

SEQ ID NO: 36275 - DNA, 28 bp, synthetic construct
  source 1..28: mol_type = other DNA
tgaggtcaggagttttagaccagcctgg

SEQ ID NO: 36276 - DNA, 28 bp, synthetic construct
  source 1..28: mol_type = other DNA
tgaggtgggcagatcacttgaggtcagg

SEQ ID NO: 36277 - DNA, 28 bp, synthetic construct
  source 1..28: mol_type = other DNA
gaggctgaggtgggcagatcacttgagg

SEQ ID NO: 36278 - DNA, 28 bp, synthetic construct
  source 1..28: mol_type = other DNA
tctcagcactttgggaggctgaggtggg

SEQ ID NO: 36279 - DNA, 28 bp, synthetic construct
  source 1..28: mol_type = other DNA
atctcagcactttgggaggctgaggtgg

SEQ ID NO: 36280 - DNA, 28 bp, synthetic construct
  source 1..28: mol_type = other DNA
gtaatctcagcactttgggaggctgagg

SEQ ID NO: 36281 - DNA, 28 bp, synthetic construct
  source 1..28: mol_type = other DNA
cagcctcccaaagtgctgagattacagg

SEQ ID NO: 36282 - DNA, 28 bp, synthetic construct
  source 1..28: mol_type = other DNA
atgcctgtaatctcagcactttgggagg

SEQ ID NO: 36283 - DNA, 28 bp, synthetic construct
  source 1..28: mol_type = other DNA
ctcatgcctgtaatctcagcactttggg

SEQ ID NO: 36284 - DNA, 28 bp, synthetic construct
  source 1..28: mol_type = other DNA
gctcatgcctgtaatctcagcactttgg

SEQ ID NO: 36285 - DNA, 28 bp, synthetic construct
  source 1..28: mol_type = other DNA
cagtaggtcttaaggttgagtgcagtgg

SEQ ID NO: 36286 - DNA, 28 bp, synthetic construct
  source 1..28: mol_type = other DNA
cagagctttagaacagtaggtcttaagg

SEQ ID NO: 36287 - DNA, 28 bp, synthetic construct
  source 1..28: mol_type = other DNA
cataatgtcagagctttagaacagtagg

SEQ ID NO: 36288 - DNA, 28 bp, synthetic construct
  source 1..28: mol_type = other DNA
actgttctaaagctctgacattatgtgg

SEQ ID NO: 36289 - DNA, 28 bp, synthetic construct
  source 1..28: mol_type = other DNA
tgacattatgtggttttagattttctgg

SEQ ID NO: 36290 - DNA, 28 bp, synthetic construct
  source 1..28: mol_type = other DNA
ttctaacatttttgataaagcctcaagg

SEQ ID NO: 36291 - DNA, 28 bp, synthetic construct
  source 1..28: mol_type = other DNA
atttttgataaagcctcaaggttttagg

SEQ ID NO: 36292 - DNA, 28 bp, synthetic construct
  source 1..28: mol_type = other DNA
tagaactttagaacctaaaaccttgagg

SEQ ID NO: 36293 - DNA, 28 bp, synthetic construct
  source 1..28: mol_type = other DNA
tctaaagttctaagattctgattttagg

SEQ ID NO: 36294 - DNA, 28 bp, synthetic construct
  source 1..28: mol_type = other DNA
tctaagattctgattttaggagctaagg

SEQ ID NO: 36295 - DNA, 28 bp, synthetic construct
  source 1..28: mol_type = other DNA
ttagaatctataatcttacattttaagg

SEQ ID NO: 36296 - DNA, 28 bp, synthetic construct
  source 1..28: mol_type = other DNA
tctaaagattctatagttctagacatgg

SEQ ID NO: 36297 - DNA, 28 bp, synthetic construct
  source 1..28: mol_type = other DNA
aaagattctatagttctagacatggagg

SEQ ID NO: 36298 - DNA, 28 bp, synthetic construct
  source 1..28: mol_type = other DNA
tatagttctagacatggaggttctaagg

SEQ ID NO: 36299 - DNA, 28 bp, synthetic construct
  source 1..28: mol_type = other DNA
tctagacatggaggttctaaggcctagg

SEQ ID NO: 36300 - DNA, 28 bp, synthetic construct
  source 1..28: mol_type = other DNA
ttagaacatcacattttagaatcctagg

SEQ ID NO: 36301 - DNA, 28 bp, synthetic construct
  source 1..28: mol_type = other DNA
taggattctaaaatgtgatgttctaagg

SEQ ID NO: 36302 - DNA, 28 bp, synthetic construct
  source 1..28: mol_type = other DNA
taaggctctgagagtctagattctctgg

SEQ ID NO: 36303 - DNA, 28 bp, synthetic construct
  source 1..28: mol_type = other DNA
tgagagtctagattctctggctgtaagg

SEQ ID NO: 36304 - DNA, 28 bp, synthetic construct
  source 1..28: mol_type = other DNA
tctggctgtaaggctctagatcataagg

SEQ ID NO: 36305 - DNA, 28 bp, synthetic construct
  source 1..28: mol_type = other DNA
taatgatgatcaattatagtttctgagg

SEQ ID NO: 36306 - DNA, 28 bp, synthetic construct
  source 1..28: mol_type = other DNA
ctcttgtataagatcctagatcctaagg

SEQ ID NO: 36307 - DNA, 28 bp, synthetic construct
  source 1..28: mol_type = other DNA
tcttgtataagatcctagatcctaaggg

SEQ ID NO: 36308 - DNA, 28 bp, synthetic construct
  source 1..28: mol_type = other DNA
ctagagctttcgacccttaggatctagg

SEQ ID NO: 36309 - DNA, 28 bp, synthetic construct
  source 1..28: mol_type = other DNA
gcagattctagagctttcgacccttagg

SEQ ID NO: 36310 - DNA, 28 bp, synthetic construct
  source 1..28: mol_type = other DNA
ttcaaaagttccaagagtctaaagatgg

SEQ ID NO: 36311 - DNA, 28 bp, synthetic construct
  source 1..28: mol_type = other DNA
cttagaaactccatctttagactcttgg

SEQ ID NO: 36312 - DNA, 28 bp, synthetic construct
  source 1..28: mol_type = other DNA
caagagtctaaagatggagtttctaagg

SEQ ID NO: 36313 - DNA, 28 bp, synthetic construct
  source 1..28: mol_type = other DNA
gtctaaagatggagtttctaaggtccgg

SEQ ID NO: 36314 - DNA, 28 bp, synthetic construct
  source 1..28: mol_type = other DNA
cttagaatatcacatcttagaacaccgg

SEQ ID NO: 36315 - DNA, 28 bp, synthetic construct
  source 1..28: mol_type = other DNA
aatcttatttaatcatctagaatcttgg

SEQ ID NO: 36316 - DNA, 28 bp, synthetic construct
  source 1..28: mol_type = other DNA
tctagatgattaaataagattctaacgg

SEQ ID NO: 36317 - DNA, 28 bp, synthetic construct
  source 1..28: mol_type = other DNA
gattctaacggtctgttctgtttcaagg

SEQ ID NO: 36318 - DNA, 28 bp, synthetic construct
  source 1..28: mol_type = other DNA
tgtttcaaggcactctagattccattgg

SEQ ID NO: 36319 - DNA, 28 bp, synthetic construct
  source 1..28: mol_type = other DNA
tctagattccattggtccaagattccgg

SEQ ID NO: 36320 - DNA, 28 bp, synthetic construct
  source 1..28: mol_type = other DNA
cttaggatccggaatcttggaccaatgg

SEQ ID NO: 36321 - DNA, 28 bp, synthetic construct
  source 1..28: mol_type = other DNA
cttagatgcttaggatccggaatcttgg

SEQ ID NO: 36322 - DNA, 28 bp, synthetic construct
  source 1..28: mol_type = other DNA
tcttataacttagatgcttaggatccgg

SEQ ID NO: 36323 - DNA, 28 bp, synthetic construct
  source 1..28: mol_type = other DNA
tgagagtcttataacttagatgcttagg

SEQ ID NO: 36324 - DNA, 28 bp, synthetic construct
  source 1..28: mol_type = other DNA
ccaacattagaaattattagaactttgg

SEQ ID NO: 36325 - DNA, 28 bp, synthetic construct
  source 1..28: mol_type = other DNA
ataatttctaatgttggacacctttagg

SEQ ID NO: 36326 - DNA, 28 bp, synthetic construct
  source 1..28: mol_type = other DNA
aggcagaatgcagcaaagaacctaaagg

SEQ ID NO: 36327 - DNA, 28 bp, synthetic construct
  source 1..28: mol_type = other DNA
gttctttgctgcattctgcctctctagg

SEQ ID NO: 36328 - DNA, 28 bp, synthetic construct
  source 1..28: mol_type = other DNA
gctgcattctgcctctctaggaccatgg

SEQ ID NO: 36329 - DNA, 28 bp, synthetic construct
  source 1..28: mol_type = other DNA
tggactcttaaccatggtcctagagagg

SEQ ID NO: 36330 - DNA, 28 bp, synthetic construct
  source 1..28: mol_type = other DNA
atgtggattcttggactcttaaccatgg

SEQ ID NO: 36331 - DNA, 28 bp, synthetic construct
  source 1..28: mol_type = other DNA
ataagattttagaaatgtggattcttgg

SEQ ID NO: 36332 - DNA, 28 bp, synthetic construct
  source 1..28: mol_type = other DNA
ctagaactataagattttagaaatgtgg

SEQ ID NO: 36333 - DNA, 28 bp, synthetic construct
  source 1..28: mol_type = other DNA
cacatttctaaaatcttatagttctagg

SEQ ID NO: 36334 - DNA, 28 bp, synthetic construct
  source 1..28: mol_type = other DNA
atgttctaagtttctaagattctaaagg

SEQ ID NO: 36335 - DNA, 28 bp, synthetic construct
  source 1..28: mol_type = other DNA
agtttctaagattctaaaggtccacagg

SEQ ID NO: 36336 - DNA, 28 bp, synthetic construct
  source 1..28: mol_type = other DNA
taaaggtccacaggtctagactattagg

SEQ ID NO: 36337 - DNA, 28 bp, synthetic construct
  source 1..28: mol_type = other DNA
aattgcacctaatagtctagacctgtgg

SEQ ID NO: 36338 - DNA, 28 bp, synthetic construct
  source 1..28: mol_type = other DNA
gtctagactattaggtgcaatttcaagg

SEQ ID NO: 36339 - DNA, 28 bp, synthetic construct
  source 1..28: mol_type = other DNA
tctaaccctatactgtagtattctttgg

SEQ ID NO: 36340 - DNA, 28 bp, synthetic construct
  source 1..28: mol_type = other DNA
ctaaccctatactgtagtattctttggg

SEQ ID NO: 36341 - DNA, 28 bp, synthetic construct
  source 1..28: mol_type = other DNA
taaccctatactgtagtattctttgggg

SEQ ID NO: 36342 - DNA, 28 bp, synthetic construct
  source 1..28: mol_type = other DNA
gcaccccaaagaatactacagtataggg

SEQ ID NO: 36343 - DNA, 28 bp, synthetic construct
  source 1..28: mol_type = other DNA
ggcaccccaaagaatactacagtatagg

SEQ ID NO: 36344 - DNA, 28 bp, synthetic construct
  source 1..28: mol_type = other DNA
aagcaatgatagctaagaaggagagggg

SEQ ID NO: 36345 - DNA, 28 bp, synthetic construct
  source 1..28: mol_type = other DNA
gaagcaatgatagctaagaaggagaggg

SEQ ID NO: 36346 - DNA, 28 bp, synthetic construct
  source 1..28: mol_type = other DNA
ggaagcaatgatagctaagaaggagagg

SEQ ID NO: 36347 - DNA, 28 bp, synthetic construct
  source 1..28: mol_type = other DNA
gaggaggaagcaatgatagctaagaagg

SEQ ID NO: 36348 - DNA, 28 bp, synthetic construct
  source 1..28: mol_type = other DNA
atcattgcttcctcctccccaactgtgg

SEQ ID NO: 36349 - DNA, 28 bp, synthetic construct
  source 1..28: mol_type = other DNA
tcattgcttcctcctccccaactgtggg

SEQ ID NO: 36350 - DNA, 28 bp, synthetic construct
  source 1..28: mol_type = other DNA
cattgcttcctcctccccaactgtgggg

SEQ ID NO: 36351 - DNA, 28 bp, synthetic construct
  source 1..28: mol_type = other DNA
attgcttcctcctccccaactgtggggg

SEQ ID NO: 36352 - DNA, 28 bp, synthetic construct
  source 1..28: mol_type = other DNA
gggcacacccccacagttggggaggagg

SEQ ID NO: 36353 - DNA, 28 bp, synthetic construct
  source 1..28: mol_type = other DNA
agggggcacacccccacagttggggagg

SEQ ID NO: 36354 - DNA, 28 bp, synthetic construct
  source 1..28: mol_type = other DNA
tgaagggggcacacccccacagttgggg

SEQ ID NO: 36355 - DNA, 28 bp, synthetic construct
  source 1..28: mol_type = other DNA
ttgaagggggcacacccccacagttggg

SEQ ID NO: 36356 - DNA, 28 bp, synthetic construct
  source 1..28: mol_type = other DNA
cttgaagggggcacacccccacagttgg

SEQ ID NO: 36357 - DNA, 28 bp, synthetic construct
  source 1..28: mol_type = other DNA
ctaatgcattgcacaggcttgaaggggg

SEQ ID NO: 36358 - DNA, 28 bp, synthetic construct
  source 1..28: mol_type = other DNA
ccccttcaagcctgtgcaatgcattagg

SEQ ID NO: 36359 - DNA, 28 bp, synthetic construct
  source 1..28: mol_type = other DNA
cccttcaagcctgtgcaatgcattaggg

SEQ ID NO: 36360 - DNA, 28 bp, synthetic construct
  source 1..28: mol_type = other DNA
tccctaatgcattgcacaggcttgaagg

SEQ ID NO: 36361 - DNA, 28 bp, synthetic construct
  source 1..28: mol_type = other DNA
aggaggcatccctaatgcattgcacagg

SEQ ID NO: 36362 - DNA, 28 bp, synthetic construct
  source 1..28: mol_type = other DNA
gcattagggatgcctcctttcccgcagg

SEQ ID NO: 36363 - DNA, 28 bp, synthetic construct
  source 1..28: mol_type = other DNA
cattagggatgcctcctttcccgcaggg

SEQ ID NO: 36364 - DNA, 28 bp, synthetic construct
  source 1..28: mol_type = other DNA
attagggatgcctcctttcccgcagggg

SEQ ID NO: 36365 - DNA, 28 bp, synthetic construct
  source 1..28: mol_type = other DNA
gggatgcctcctttcccgcaggggatgg

SEQ ID NO: 36366 - DNA, 28 bp, synthetic construct
  source 1..28: mol_type = other DNA
gatcgtccatcccctgcgggaaaggagg

SEQ ID NO: 36367 - DNA, 28 bp, synthetic construct
  source 1..28: mol_type = other DNA
ggagatcgtccatcccctgcgggaaagg

SEQ ID NO: 36368 - DNA, 28 bp, synthetic construct
  source 1..28: mol_type = other DNA
aggtgggagatcgtccatcccctgcggg

SEQ ID NO: 36369 - DNA, 28 bp, synthetic construct
  source 1..28: mol_type = other DNA
aaggtgggagatcgtccatcccctgcgg

SEQ ID NO: 36370 - DNA, 28 bp, synthetic construct
  source 1..28: mol_type = other DNA
aggggatggacgatctcccacctttcgg

SEQ ID NO: 36371 - DNA, 28 bp, synthetic construct
  source 1..28: mol_type = other DNA
ggggatggacgatctcccacctttcggg

SEQ ID NO: 36372 - DNA, 28 bp, synthetic construct
  source 1..28: mol_type = other DNA
acgggggcaacatggcccgaaaggtggg

SEQ ID NO: 36373 - DNA, 28 bp, synthetic construct
  source 1..28: mol_type = other DNA
cacgggggcaacatggcccgaaaggtgg

SEQ ID NO: 36374 - DNA, 28 bp, synthetic construct
  source 1..28: mol_type = other DNA
gctcacgggggcaacatggcccgaaagg

SEQ ID NO: 36375 - DNA, 28 bp, synthetic construct
  source 1..28: mol_type = other DNA
gagggattggctcacgggggcaacatgg

SEQ ID NO: 36376 - DNA, 28 bp, synthetic construct
  source 1..28: mol_type = other DNA
cagaaggtgagggattggctcacggggg

SEQ ID NO: 36377 - DNA, 28 bp, synthetic construct
  source 1..28: mol_type = other DNA
tcagaaggtgagggattggctcacgggg

SEQ ID NO: 36378 - DNA, 28 bp, synthetic construct
  source 1..28: mol_type = other DNA
ctcagaaggtgagggattggctcacggg

SEQ ID NO: 36379 - DNA, 28 bp, synthetic construct
  source 1..28: mol_type = other DNA
actcagaaggtgagggattggctcacgg

SEQ ID NO: 36380 - DNA, 28 bp, synthetic construct
  source 1..28: mol_type = other DNA
actctgtactcagaaggtgagggattgg

SEQ ID NO: 36381 - DNA, 28 bp, synthetic construct
  source 1..28: mol_type = other DNA
tccctcaccttctgagtacagagtgtgg

SEQ ID NO: 36382 - DNA, 28 bp, synthetic construct
  source 1..28: mol_type = other DNA
tccacactctgtactcagaaggtgaggg

SEQ ID NO: 36383 - DNA, 28 bp, synthetic construct
  source 1..28: mol_type = other DNA
gtccacactctgtactcagaaggtgagg

SEQ ID NO: 36384 - DNA, 28 bp, synthetic construct
  source 1..28: mol_type = other DNA
ccagagtccacactctgtactcagaagg

SEQ ID NO: 36385 - DNA, 28 bp, synthetic construct
  source 1..28: mol_type = other DNA
agagtgtggactctggtgcctccagagg

SEQ ID NO: 36386 - DNA, 28 bp, synthetic construct
  source 1..28: mol_type = other DNA
gagtgtggactctggtgcctccagaggg

SEQ ID NO: 36387 - DNA, 28 bp, synthetic construct
  source 1..28: mol_type = other DNA
agtgtggactctggtgcctccagagggg

SEQ ID NO: 36388 - DNA, 28 bp, synthetic construct
  source 1..28: mol_type = other DNA
gactctggtgcctccagaggggctcagg

SEQ ID NO: 36389 - DNA, 28 bp, synthetic construct
  source 1..28: mol_type = other DNA
ttttatgtgacctgagcccctctggagg

SEQ ID NO: 36390 - DNA, 28 bp, synthetic construct
  source 1..28: mol_type = other DNA
aagttttatgtgacctgagcccctctgg

SEQ ID NO: 36391 - DNA, 28 bp, synthetic construct
  source 1..28: mol_type = other DNA
tctagtcctcatgttgtttatactcagg

SEQ ID NO: 36392 - DNA, 28 bp, synthetic construct
  source 1..28: mol_type = other DNA
taaatacctgagtataaacaacatgagg

SEQ ID NO: 36393 - DNA, 28 bp, synthetic construct
  source 1..28: mol_type = other DNA
atgttgtttatactcaggtatttattgg

SEQ ID NO: 36394 - DNA, 28 bp, synthetic construct
  source 1..28: mol_type = other DNA
tgttgtttatactcaggtatttattggg

SEQ ID NO: 36395 - DNA, 28 bp, synthetic construct
  source 1..28: mol_type = other DNA
acacgcgtcagtagtccctgataaatgg

SEQ ID NO: 36396 - DNA, 28 bp, synthetic construct
  source 1..28: mol_type = other DNA
actcaagcgatctttccatttatcaggg

SEQ ID NO: 36397 - DNA, 28 bp, synthetic construct
  source 1..28: mol_type = other DNA
gactcaagcgatctttccatttatcagg

SEQ ID NO: 36398 - DNA, 28 bp, synthetic construct
  source 1..28: mol_type = other DNA
ataaatggaaagatcgcttgagtccagg

SEQ ID NO: 36399 - DNA, 28 bp, synthetic construct
  source 1..28: mol_type = other DNA
ctattctaggctggactggaactcctgg

SEQ ID NO: 36400 - DNA, 28 bp, synthetic construct
  source 1..28: mol_type = other DNA
caggagttccagtccagcctagaatagg

SEQ ID NO: 36401 - DNA, 28 bp, synthetic construct
  source 1..28: mol_type = other DNA
atgttttacctattctaggctggactgg

SEQ ID NO: 36402 - DNA, 28 bp, synthetic construct
  source 1..28: mol_type = other DNA
agagcatgttttacctattctaggctgg

SEQ ID NO: 36403 - DNA, 28 bp, synthetic construct
  source 1..28: mol_type = other DNA
tcagagagcatgttttacctattctagg

SEQ ID NO: 36404 - DNA, 28 bp, synthetic construct
  source 1..28: mol_type = other DNA
tgctctctgaattagtctttgaaactgg

SEQ ID NO: 36405 - DNA, 28 bp, synthetic construct
  source 1..28: mol_type = other DNA
gaagtttttttaagaattccatgagtgg

SEQ ID NO: 36406 - DNA, 28 bp, synthetic construct
  source 1..28: mol_type = other DNA
tttaagaattccatgagtggtttgctgg

SEQ ID NO: 36407 - DNA, 28 bp, synthetic construct
  source 1..28: mol_type = other DNA
taaacgtacaccagcaaaccactcatgg

SEQ ID NO: 36408 - DNA, 28 bp, synthetic construct
  source 1..28: mol_type = other DNA
tgcgagttaggggcttaatttggggtgg

SEQ ID NO: 36409 - DNA, 28 bp, synthetic construct
  source 1..28: mol_type = other DNA
gcttgcgagttaggggcttaatttgggg

SEQ ID NO: 36410 - DNA, 28 bp, synthetic construct
  source 1..28: mol_type = other DNA
tgcttgcgagttaggggcttaatttggg

SEQ ID NO: 36411 - DNA, 28 bp, synthetic construct
  source 1..28: mol_type = other DNA
gtgcttgcgagttaggggcttaatttgg

SEQ ID NO: 36412 - DNA, 28 bp, synthetic construct
  source 1..28: mol_type = other DNA
aagcccctaactcgcaagcacaaaatgg

SEQ ID NO: 36413 - DNA, 28 bp, synthetic construct
  source 1..28: mol_type = other DNA
agtccattttgtgcttgcgagttagggg

SEQ ID NO: 36414 - DNA, 28 bp, synthetic construct
  source 1..28: mol_type = other DNA
gagtccattttgtgcttgcgagttaggg

SEQ ID NO: 36415 - DNA, 28 bp, synthetic construct
  source 1..28: mol_type = other DNA
cgagtccattttgtgcttgcgagttagg

SEQ ID NO: 36416 - DNA, 28 bp, synthetic construct
  source 1..28: mol_type = other DNA
ctcgattatttactgagttatcagttgg

SEQ ID NO: 36417 - DNA, 28 bp, synthetic construct
  source 1..28: mol_type = other DNA
cagttggccttgtccttagttgtacagg

SEQ ID NO: 36418 - DNA, 28 bp, synthetic construct
  source 1..28: mol_type = other DNA
agttggccttgtccttagttgtacaggg

SEQ ID NO: 36419 - DNA, 28 bp, synthetic construct
  source 1..28: mol_type = other DNA
attagtccctgtacaactaaggacaagg

SEQ ID NO: 36420 - DNA, 28 bp, synthetic construct
  source 1..28: mol_type = other DNA
tgagtcattagtccctgtacaactaagg

SEQ ID NO: 36421 - DNA, 28 bp, synthetic construct
  source 1..28: mol_type = other DNA
ggactaatgactcacctataaataatgg

SEQ ID NO: 36422 - DNA, 28 bp, synthetic construct
  source 1..28: mol_type = other DNA
gactaatgactcacctataaataatggg

SEQ ID NO: 36423 - DNA, 28 bp, synthetic construct
  source 1..28: mol_type = other DNA
cttcttagaagagcccattatttatagg

SEQ ID NO: 36424 - DNA, 28 bp, synthetic construct
  source 1..28: mol_type = other DNA
agttgacacctctttgtcctatagctgg

SEQ ID NO: 36425 - DNA, 28 bp, synthetic construct
  source 1..28: mol_type = other DNA
gttgacacctctttgtcctatagctggg

SEQ ID NO: 36426 - DNA, 28 bp, synthetic construct
  source 1..28: mol_type = other DNA
gacacctctttgtcctatagctgggagg

SEQ ID NO: 36427 - DNA, 28 bp, synthetic construct
  source 1..28: mol_type = other DNA
cgttcctcccagctataggacaaagagg

SEQ ID NO: 36428 - DNA, 28 bp, synthetic construct
  source 1..28: mol_type = other DNA
tttgcaatgcgttcctcccagctatagg

SEQ ID NO: 36429 - DNA, 28 bp, synthetic construct
  source 1..28: mol_type = other DNA
aacgccaacccaatgattccctaaatgg

SEQ ID NO: 36430 - DNA, 28 bp, synthetic construct
  source 1..28: mol_type = other DNA
acgccaacccaatgattccctaaatggg

SEQ ID NO: 36431 - DNA, 28 bp, synthetic construct
  source 1..28: mol_type = other DNA
cgccaacccaatgattccctaaatgggg

SEQ ID NO: 36432 - DNA, 28 bp, synthetic construct
  source 1..28: mol_type = other DNA
gaccccatttagggaatcattgggttgg

SEQ ID NO: 36433 - DNA, 28 bp, synthetic construct
  source 1..28: mol_type = other DNA
cgaagaccccatttagggaatcattggg

SEQ ID NO: 36434 - DNA, 28 bp, synthetic construct
  source 1..28: mol_type = other DNA
gcgaagaccccatttagggaatcattgg

SEQ ID NO: 36435 - DNA, 28 bp, synthetic construct
  source 1..28: mol_type = other DNA
gcagctgatgcgaagaccccatttaggg

SEQ ID NO: 36436 - DNA, 28 bp, synthetic construct
  source 1..28: mol_type = other DNA
cgcagctgatgcgaagaccccatttagg

SEQ ID NO: 36437 - DNA, 28 bp, synthetic construct
  source 1..28: mol_type = other DNA
tcagctgcgttaaaatcaccccagcagg

SEQ ID NO: 36438 - DNA, 28 bp, synthetic construct
  source 1..28: mol_type = other DNA
ctgcgttaaaatcaccccagcaggcagg

SEQ ID NO: 36439 - DNA, 28 bp, synthetic construct
  source 1..28: mol_type = other DNA
aaatcaccccagcaggcaggttatccgg

SEQ ID NO: 36440 - DNA, 28 bp, synthetic construct
  source 1..28: mol_type = other DNA
tggcggccggataacctgcctgctgggg

SEQ ID NO: 36441 - DNA, 28 bp, synthetic construct
  source 1..28: mol_type = other DNA
gtggcggccggataacctgcctgctggg

SEQ ID NO: 36442 - DNA, 28 bp, synthetic construct
  source 1..28: mol_type = other DNA
agtggcggccggataacctgcctgctgg

SEQ ID NO: 36443 - DNA, 28 bp, synthetic construct
  source 1..28: mol_type = other DNA
aggcaggttatccggccgccactccagg

SEQ ID NO: 36444 - DNA, 28 bp, synthetic construct
  source 1..28: mol_type = other DNA
ggcaggttatccggccgccactccaggg

SEQ ID NO: 36445 - DNA, 28 bp, synthetic construct
  source 1..28: mol_type = other DNA
gatttaatgaccctggagtggcggccgg

SEQ ID NO: 36446 - DNA, 28 bp, synthetic construct
  source 1..28: mol_type = other DNA
gtctgatttaatgaccctggagtggcgg

SEQ ID NO: 36447 - DNA, 28 bp, synthetic construct
  source 1..28: mol_type = other DNA
agagtctgatttaatgaccctggagtgg

SEQ ID NO: 36448 - DNA, 28 bp, synthetic construct
  source 1..28: mol_type = other DNA
actggagagtctgatttaatgaccctgg

SEQ ID NO: 36449 - DNA, 28 bp, synthetic construct
  source 1..28: mol_type = other DNA
agggtcattaaatcagactctccagtgg

SEQ ID NO: 36450 - DNA, 28 bp, synthetic construct
  source 1..28: mol_type = other DNA
gggtcattaaatcagactctccagtggg

SEQ ID NO: 36451 - DNA, 28 bp, synthetic construct
  source 1..28: mol_type = other DNA
taaatcagactctccagtgggacctcgg

SEQ ID NO: 36452 - DNA, 28 bp, synthetic construct
  source 1..28: mol_type = other DNA
taagctacgaattccgaggtcccactgg

SEQ ID NO: 36453 - DNA, 28 bp, synthetic construct
  source 1..28: mol_type = other DNA
ggagcttgctaagctacgaattccgagg

SEQ ID NO: 36454 - DNA, 28 bp, synthetic construct
  source 1..28: mol_type = other DNA
gcttagcaagctccccaagtgatgctgg

SEQ ID NO: 36455 - DNA, 28 bp, synthetic construct
  source 1..28: mol_type = other DNA
cttagcaagctccccaagtgatgctggg

SEQ ID NO: 36456 - DNA, 28 bp, synthetic construct
  source 1..28: mol_type = other DNA
gttagtttactcccagcatcacttgggg

SEQ ID NO: 36457 - DNA, 28 bp, synthetic construct
  source 1..28: mol_type = other DNA
cgttagtttactcccagcatcacttggg

SEQ ID NO: 36458 - DNA, 28 bp, synthetic construct
  source 1..28: mol_type = other DNA
acgttagtttactcccagcatcacttgg

SEQ ID NO: 36459 - DNA, 28 bp, synthetic construct
  source 1..28: mol_type = other DNA
acgtttgagagtcacaaacatgttttgg

SEQ ID NO: 36460 - DNA, 28 bp, synthetic construct
  source 1..28: mol_type = other DNA
aacatgttttggcaatataaccagatgg

SEQ ID NO: 36461 - DNA, 28 bp, synthetic construct
  source 1..28: mol_type = other DNA
acatgttttggcaatataaccagatggg

SEQ ID NO: 36462 - DNA, 28 bp, synthetic construct
  source 1..28: mol_type = other DNA
ttttggcaatataaccagatgggactgg

SEQ ID NO: 36463 - DNA, 28 bp, synthetic construct
  source 1..28: mol_type = other DNA
attttttaatttctccagtcccatctgg

SEQ ID NO: 36464 - DNA, 28 bp, synthetic construct
  source 1..28: mol_type = other DNA
cacgcagcttagtcttgcttttttaggg

SEQ ID NO: 36465 - DNA, 28 bp, synthetic construct
  source 1..28: mol_type = other DNA
cctaaaaaagcaagactaagctgcgtgg

SEQ ID NO: 36466 - DNA, 28 bp, synthetic construct
  source 1..28: mol_type = other DNA
ctaaaaaagcaagactaagctgcgtggg

SEQ ID NO: 36467 - DNA, 28 bp, synthetic construct
  source 1..28: mol_type = other DNA
aaaaagcaagactaagctgcgtgggagg

SEQ ID NO: 36468 - DNA, 28 bp, synthetic construct
  source 1..28: mol_type = other DNA
actaagctgcgtgggaggccaaacgagg

SEQ ID NO: 36469 - DNA, 28 bp, synthetic construct
  source 1..28: mol_type = other DNA
ctaagctgcgtgggaggccaaacgaggg

SEQ ID NO: 36470 - DNA, 28 bp, synthetic construct
  source 1..28: mol_type = other DNA
taagctgcgtgggaggccaaacgagggg

SEQ ID NO: 36471 - DNA, 28 bp, synthetic construct
  source 1..28: mol_type = other DNA
aagctgcgtgggaggccaaacgaggggg

SEQ ID NO: 36472 - DNA, 28 bp, synthetic construct
  source 1..28: mol_type = other DNA
agctgcgtgggaggccaaacgagggggg

SEQ ID NO: 36473 - DNA, 28 bp, synthetic construct
  source 1..28: mol_type = other DNA
gggaggccaaacgaggggggtcctttgg

SEQ ID NO: 36474 - DNA, 28 bp, synthetic construct
  source 1..28: mol_type = other DNA
ggaggccaaacgaggggggtcctttggg

SEQ ID NO: 36475 - DNA, 28 bp, synthetic construct
  source 1..28: mol_type = other DNA
aacagcccaaaggacccccctcgtttgg

SEQ ID NO: 36476 - DNA, 28 bp, synthetic construct
  source 1..28: mol_type = other DNA
ttttgtcatggtagaaacagcccaaagg

SEQ ID NO: 36477 - DNA, 28 bp, synthetic construct
  source 1..28: mol_type = other DNA
tgtggggtaatggcgatttttgtcatgg

SEQ ID NO: 36478 - DNA, 28 bp, synthetic construct
  source 1..28: mol_type = other DNA
tggcggtgtgagaggtgtggggtaatgg

SEQ ID NO: 36479 - DNA, 28 bp, synthetic construct
  source 1..28: mol_type = other DNA
gaacgttggcggtgtgagaggtgtgggg

SEQ ID NO: 36480 - DNA, 28 bp, synthetic construct
  source 1..28: mol_type = other DNA
ggaacgttggcggtgtgagaggtgtggg

SEQ ID NO: 36481 - DNA, 28 bp, synthetic construct
  source 1..28: mol_type = other DNA
cggaacgttggcggtgtgagaggtgtgg

SEQ ID NO: 36482 - DNA, 28 bp, synthetic construct
  source 1..28: mol_type = other DNA
gttggcggaacgttggcggtgtgagagg

SEQ ID NO: 36483 - DNA, 28 bp, synthetic construct
  source 1..28: mol_type = other DNA
tggcggaacgttggcggaacgttggcgg

SEQ ID NO: 36484 - DNA, 28 bp, synthetic construct
  source 1..28: mol_type = other DNA
cgttggcggaacgttggcggaacgttgg

SEQ ID NO: 36485 - DNA, 28 bp, synthetic construct
  source 1..28: mol_type = other DNA
tggtgggacgttggcggaacgttggcgg

SEQ ID NO: 36486 - DNA, 28 bp, synthetic construct
  source 1..28: mol_type = other DNA
gggtggtgggacgttggcggaacgttgg

SEQ ID NO: 36487 - DNA, 28 bp, synthetic construct
  source 1..28: mol_type = other DNA
tatcatgagggtggtgggacgttggcgg

SEQ ID NO: 36488 - DNA, 28 bp, synthetic construct
  source 1..28: mol_type = other DNA
ggatatcatgagggtggtgggacgttgg

SEQ ID NO: 36489 - DNA, 28 bp, synthetic construct
  source 1..28: mol_type = other DNA
cgcggacggatatcatgagggtggtggg

SEQ ID NO: 36490 - DNA, 28 bp, synthetic construct
  source 1..28: mol_type = other DNA
ccgcggacggatatcatgagggtggtgg

SEQ ID NO: 36491 - DNA, 28 bp, synthetic construct
  source 1..28: mol_type = other DNA
gtaccgcggacggatatcatgagggtgg

SEQ ID NO: 36492 - DNA, 28 bp, synthetic construct
  source 1..28: mol_type = other DNA
gcagtaccgcggacggatatcatgaggg

SEQ ID NO: 36493 - DNA, 28 bp, synthetic construct
  source 1..28: mol_type = other DNA
agcagtaccgcggacggatatcatgagg

SEQ ID NO: 36494 - DNA, 28 bp, synthetic construct
  source 1..28: mol_type = other DNA
tccgtccgcggtactgctccagcgaagg

SEQ ID NO: 36495 - DNA, 28 bp, synthetic construct
  source 1..28: mol_type = other DNA
accttcgctggagcagtaccgcggacgg

SEQ ID NO: 36496 - DNA, 28 bp, synthetic construct
  source 1..28: mol_type = other DNA
gggtaccttcgctggagcagtaccgcgg

SEQ ID NO: 36497 - DNA, 28 bp, synthetic construct
  source 1..28: mol_type = other DNA
ctgctccagcgaaggtacccttgcctgg

SEQ ID NO: 36498 - DNA, 28 bp, synthetic construct
  source 1..28: mol_type = other DNA
tgctccagcgaaggtacccttgcctggg

SEQ ID NO: 36499 - DNA, 28 bp, synthetic construct
  source 1..28: mol_type = other DNA
atggcccaggcaagggtaccttcgctgg

SEQ ID NO: 36500 - DNA, 28 bp, synthetic construct
  source 1..28: mol_type = other DNA
cgaaggtacccttgcctgggccatgagg

SEQ ID NO: 36501 - DNA, 28 bp, synthetic construct
  source 1..28: mol_type = other DNA
cggttgcgcctcatggcccaggcaaggg

SEQ ID NO: 36502 - DNA, 28 bp, synthetic construct
  source 1..28: mol_type = other DNA
acggttgcgcctcatggcccaggcaagg

SEQ ID NO: 36503 - DNA, 28 bp, synthetic construct
  source 1..28: mol_type = other DNA
gagggacggttgcgcctcatggcccagg

SEQ ID NO: 36504 - DNA, 28 bp, synthetic construct
  source 1..28: mol_type = other DNA
agctgtgagggacggttgcgcctcatgg

SEQ ID NO: 36505 - DNA, 28 bp, synthetic construct
  source 1..28: mol_type = other DNA
atgaggcgcaaccgtccctcacagctgg

SEQ ID NO: 36506 - DNA, 28 bp, synthetic construct
  source 1..28: mol_type = other DNA
tgaggcgcaaccgtccctcacagctggg

SEQ ID NO: 36507 - DNA, 28 bp, synthetic construct
  source 1..28: mol_type = other DNA
gaggcgcaaccgtccctcacagctgggg

SEQ ID NO: 36508 - DNA, 28 bp, synthetic construct
  source 1..28: mol_type = other DNA
gcgcaaccgtccctcacagctggggtgg

SEQ ID NO: 36509 - DNA, 28 bp, synthetic construct
  source 1..28: mol_type = other DNA
gagaagccaccccagctgtgagggacgg

SEQ ID NO: 36510 - DNA, 28 bp, synthetic construct
  source 1..28: mol_type = other DNA
cctggagaagccaccccagctgtgaggg

SEQ ID NO: 36511 - DNA, 28 bp, synthetic construct
  source 1..28: mol_type = other DNA
acctggagaagccaccccagctgtgagg

SEQ ID NO: 36512 - DNA, 28 bp, synthetic construct
  source 1..28: mol_type = other DNA
gggtggcttctccaggttcgcaccgagg

SEQ ID NO: 36513 - DNA, 28 bp, synthetic construct
  source 1..28: mol_type = other DNA
ggtggcttctccaggttcgcaccgaggg

SEQ ID NO: 36514 - DNA, 28 bp, synthetic construct
  source 1..28: mol_type = other DNA
gtggcttctccaggttcgcaccgagggg

SEQ ID NO: 36515 - DNA, 28 bp, synthetic construct
  source 1..28: mol_type = other DNA
ctccaggttcgcaccgaggggaagttgg

SEQ ID NO: 36516 - DNA, 28 bp, synthetic construct
  source 1..28: mol_type = other DNA
tccaggttcgcaccgaggggaagttggg

SEQ ID NO: 36517 - DNA, 28 bp, synthetic construct
  source 1..28: mol_type = other DNA
ccccaacttcccctcggtgcgaacctgg

SEQ ID NO: 36518 - DNA, 28 bp, synthetic construct
  source 1..28: mol_type = other DNA
tcgcaccgaggggaagttggggtaccgg

SEQ ID NO: 36519 - DNA, 28 bp, synthetic construct
  source 1..28: mol_type = other DNA
ggaaaccggtaccccaacttcccctcgg

SEQ ID NO: 36520 - DNA, 28 bp, synthetic construct
  source 1..28: mol_type = other DNA
catcttgggtgctggcggcggaaaccgg

SEQ ID NO: 36521 - DNA, 28 bp, synthetic construct
  source 1..28: mol_type = other DNA
cggtttccgccgccagcacccaagatgg

SEQ ID NO: 36522 - DNA, 28 bp, synthetic construct
  source 1..28: mol_type = other DNA
tttccgccgccagcacccaagatggcgg

SEQ ID NO: 36523 - DNA, 28 bp, synthetic construct
  source 1..28: mol_type = other DNA
gtgccgccatcttgggtgctggcggcgg

SEQ ID NO: 36524 - DNA, 28 bp, synthetic construct
  source 1..28: mol_type = other DNA
ctcgtgccgccatcttgggtgctggcgg

SEQ ID NO: 36525 - DNA, 28 bp, synthetic construct
  source 1..28: mol_type = other DNA
acgctcgtgccgccatcttgggtgctgg

SEQ ID NO: 36526 - DNA, 28 bp, synthetic construct
  source 1..28: mol_type = other DNA
gttgcgacgctcgtgccgccatcttggg

SEQ ID NO: 36527 - DNA, 28 bp, synthetic construct
  source 1..28: mol_type = other DNA
ggttgcgacgctcgtgccgccatcttgg

SEQ ID NO: 36528 - DNA, 28 bp, synthetic construct
  source 1..28: mol_type = other DNA
cgggacacgaagcatgtggttcttgtgg

SEQ ID NO: 36529 - DNA, 28 bp, synthetic construct
  source 1..28: mol_type = other DNA
atgctgaggcgggacacgaagcatgtgg

SEQ ID NO: 36530 - DNA, 28 bp, synthetic construct
  source 1..28: mol_type = other DNA
gcttcgtgtcccgcctcagcattctcgg

SEQ ID NO: 36531 - DNA, 28 bp, synthetic construct
  source 1..28: mol_type = other DNA
cttcgtgtcccgcctcagcattctcggg

SEQ ID NO: 36532 - DNA, 28 bp, synthetic construct
  source 1..28: mol_type = other DNA
tagtgagacccgagaatgctgaggcggg

SEQ ID NO: 36533 - DNA, 28 bp, synthetic construct
  source 1..28: mol_type = other DNA
ctagtgagacccgagaatgctgaggcgg

SEQ ID NO: 36534 - DNA, 28 bp, synthetic construct
  source 1..28: mol_type = other DNA
agtctagtgagacccgagaatgctgagg

SEQ ID NO: 36535 - DNA, 28 bp, synthetic construct
  source 1..28: mol_type = other DNA
ctcactagacttttgcaagtcactgtgg

SEQ ID NO: 36536 - DNA, 28 bp, synthetic construct
  source 1..28: mol_type = other DNA
tcactagacttttgcaagtcactgtggg

SEQ ID NO: 36537 - DNA, 28 bp, synthetic construct
  source 1..28: mol_type = other DNA
ttgcaagtcactgtgggaaccctcaagg

SEQ ID NO: 36538 - DNA, 28 bp, synthetic construct
  source 1..28: mol_type = other DNA
agtcactgtgggaaccctcaaggcgagg

SEQ ID NO: 36539 - DNA, 28 bp, synthetic construct
  source 1..28: mol_type = other DNA
gtcactgtgggaaccctcaaggcgaggg

SEQ ID NO: 36540 - DNA, 28 bp, synthetic construct
  source 1..28: mol_type = other DNA
agagtgcggaacaccctcgccttgaggg

SEQ ID NO: 36541 - DNA, 28 bp, synthetic construct
  source 1..28: mol_type = other DNA
cagagtgcggaacaccctcgccttgagg

SEQ ID NO: 36542 - DNA, 28 bp, synthetic construct
  source 1..28: mol_type = other DNA
ctcaaggcgagggtgttccgcactctgg

SEQ ID NO: 36543 - DNA, 28 bp, synthetic construct
  source 1..28: mol_type = other DNA
aaggcgagggtgttccgcactctggcgg

SEQ ID NO: 36544 - DNA, 28 bp, synthetic construct
  source 1..28: mol_type = other DNA
aggaaggtgtatcgccgccagagtgcgg

SEQ ID NO: 36545 - DNA, 28 bp, synthetic construct
  source 1..28: mol_type = other DNA
gatacaccttcctattccctgacctagg

SEQ ID NO: 36546 - DNA, 28 bp, synthetic construct
  source 1..28: mol_type = other DNA
tgaaggcctaggtcagggaataggaagg

SEQ ID NO: 36547 - DNA, 28 bp, synthetic construct
  source 1..28: mol_type = other DNA
ggaatgaaggcctaggtcagggaatagg

SEQ ID NO: 36548 - DNA, 28 bp, synthetic construct
  source 1..28: mol_type = other DNA
ggcgggggaatgaaggcctaggtcaggg

SEQ ID NO: 36549 - DNA, 28 bp, synthetic construct
  source 1..28: mol_type = other DNA
tggcgggggaatgaaggcctaggtcagg

SEQ ID NO: 36550 - DNA, 28 bp, synthetic construct
  source 1..28: mol_type = other DNA
ttctgtggcgggggaatgaaggcctagg

SEQ ID NO: 36551 - DNA, 28 bp, synthetic construct
  source 1..28: mol_type = other DNA
agcgctttctgtggcgggggaatgaagg

SEQ ID NO: 36552 - DNA, 28 bp, synthetic construct
  source 1..28: mol_type = other DNA
ttcattcccccgccacagaaagcgctgg

SEQ ID NO: 36553 - DNA, 28 bp, synthetic construct
  source 1..28: mol_type = other DNA
gcgcttccagcgctttctgtggcggggg

SEQ ID NO: 36554 - DNA, 28 bp, synthetic construct
  source 1..28: mol_type = other DNA
ggcgcttccagcgctttctgtggcgggg

SEQ ID NO: 36555 - DNA, 28 bp, synthetic construct
  source 1..28: mol_type = other DNA
gggcgcttccagcgctttctgtggcggg

SEQ ID NO: 36556 - DNA, 28 bp, synthetic construct
  source 1..28: mol_type = other DNA
tgggcgcttccagcgctttctgtggcgg

SEQ ID NO: 36557 - DNA, 28 bp, synthetic construct
  source 1..28: mol_type = other DNA
ggttgggcgcttccagcgctttctgtgg

SEQ ID NO: 36558 - DNA, 28 bp, synthetic construct
  source 1..28: mol_type = other DNA
cagaaagcgctggaagcgcccaacctgg

SEQ ID NO: 36559 - DNA, 28 bp, synthetic construct
  source 1..28: mol_type = other DNA
gggcgttgggtgaagtatccaggttggg

SEQ ID NO: 36560 - DNA, 28 bp, synthetic construct
  source 1..28: mol_type = other DNA
tgggcgttgggtgaagtatccaggttgg

SEQ ID NO: 36561 - DNA, 28 bp, synthetic construct
  source 1..28: mol_type = other DNA
ggcttgggcgttgggtgaagtatccagg

SEQ ID NO: 36562 - DNA, 28 bp, synthetic construct
  source 1..28: mol_type = other DNA
ggcgatgttagtgggcttgggcgttggg

SEQ ID NO: 36563 - DNA, 28 bp, synthetic construct
  source 1..28: mol_type = other DNA
gggcgatgttagtgggcttgggcgttgg

SEQ ID NO: 36564 - DNA, 28 bp, synthetic construct
  source 1..28: mol_type = other DNA
cgcggcgggcgatgttagtgggcttggg

SEQ ID NO: 36565 - DNA, 28 bp, synthetic construct
  source 1..28: mol_type = other DNA
tcgcggcgggcgatgttagtgggcttgg

SEQ ID NO: 36566 - DNA, 28 bp, synthetic construct
  source 1..28: mol_type = other DNA
agcccactaacatcgcccgccgcgaagg

SEQ ID NO: 36567 - DNA, 28 bp, synthetic construct
  source 1..28: mol_type = other DNA
cgccttcgcggcgggcgatgttagtggg

SEQ ID NO: 36568 - DNA, 28 bp, synthetic construct
  source 1..28: mol_type = other DNA
gcgccttcgcggcgggcgatgttagtgg

SEQ ID NO: 36569 - DNA, 28 bp, synthetic construct
  source 1..28: mol_type = other DNA
actaacatcgcccgccgcgaaggcgcgg

SEQ ID NO: 36570 - DNA, 28 bp, synthetic construct
  source 1..28: mol_type = other DNA
atcgcccgccgcgaaggcgcggccgagg

SEQ ID NO: 36571 - DNA, 28 bp, synthetic construct
  source 1..28: mol_type = other DNA
tcgcccgccgcgaaggcgcggccgaggg

SEQ ID NO: 36572 - DNA, 28 bp, synthetic construct
  source 1..28: mol_type = other DNA
cgcccgccgcgaaggcgcggccgagggg

SEQ ID NO: 36573 - DNA, 28 bp, synthetic construct
  source 1..28: mol_type = other DNA
ggcccctcggccgcgccttcgcggcggg

SEQ ID NO: 36574 - DNA, 28 bp, synthetic construct
  source 1..28: mol_type = other DNA
gggcccctcggccgcgccttcgcggcgg

SEQ ID NO: 36575 - DNA, 28 bp, synthetic construct
  source 1..28: mol_type = other DNA
tctgggcccctcggccgcgccttcgcgg

SEQ ID NO: 36576 - DNA, 28 bp, synthetic construct
  source 1..28: mol_type = other DNA
ctagtgtctggcattctgggcccctcgg

SEQ ID NO: 36577 - DNA, 28 bp, synthetic construct
  source 1..28: mol_type = other DNA
cgaggggcccagaatgccagacactagg

SEQ ID NO: 36578 - DNA, 28 bp, synthetic construct
  source 1..28: mol_type = other DNA
gaggggcccagaatgccagacactaggg

SEQ ID NO: 36579 - DNA, 28 bp, synthetic construct
  source 1..28: mol_type = other DNA
cgaaggccctagtgtctggcattctggg

SEQ ID NO: 36580 - DNA, 28 bp, synthetic construct
  source 1..28: mol_type = other DNA
gcgaaggccctagtgtctggcattctgg

SEQ ID NO: 36581 - DNA, 28 bp, synthetic construct
  source 1..28: mol_type = other DNA
tgaggagggcgaaggccctagtgtctgg

SEQ ID NO: 36582 - DNA, 28 bp, synthetic construct
  source 1..28: mol_type = other DNA
acactagggccttcgccctcctcattgg

SEQ ID NO: 36583 - DNA, 28 bp, synthetic construct
  source 1..28: mol_type = other DNA
ctagggccttcgccctcctcattggtgg

SEQ ID NO: 36584 - DNA, 28 bp, synthetic construct
  source 1..28: mol_type = other DNA
tagggccttcgccctcctcattggtggg

SEQ ID NO: 36585 - DNA, 28 bp, synthetic construct
  source 1..28: mol_type = other DNA
atggacccaccaatgaggagggcgaagg

SEQ ID NO: 36586 - DNA, 28 bp, synthetic construct
  source 1..28: mol_type = other DNA
cgcggtatggacccaccaatgaggaggg

SEQ ID NO: 36587 - DNA, 28 bp, synthetic construct
  source 1..28: mol_type = other DNA
cctcctcattggtgggtccataccgcgg

SEQ ID NO: 36588 - DNA, 28 bp, synthetic construct
  source 1..28: mol_type = other DNA
ctcctcattggtgggtccataccgcggg

SEQ ID NO: 36589 - DNA, 28 bp, synthetic construct
  source 1..28: mol_type = other DNA
tcctcattggtgggtccataccgcgggg

SEQ ID NO: 36590 - DNA, 28 bp, synthetic construct
  source 1..28: mol_type = other DNA
gccccgcggtatggacccaccaatgagg

SEQ ID NO: 36591 - DNA, 28 bp, synthetic construct
  source 1..28: mol_type = other DNA
tcattggtgggtccataccgcggggcgg

SEQ ID NO: 36592 - DNA, 28 bp, synthetic construct
  source 1..28: mol_type = other DNA
cattggtgggtccataccgcggggcggg

SEQ ID NO: 36593 - DNA, 28 bp, synthetic construct
  source 1..28: mol_type = other DNA
tgggtccataccgcggggcgggcctagg

SEQ ID NO: 36594 - DNA, 28 bp, synthetic construct
  source 1..28: mol_type = other DNA
gagtacctaggcccgccccgcggtatgg

SEQ ID NO: 36595 - DNA, 28 bp, synthetic construct
  source 1..28: mol_type = other DNA
ccaatgagtacctaggcccgccccgcgg

SEQ ID NO: 36596 - DNA, 28 bp, synthetic construct
  source 1..28: mol_type = other DNA
cgcggggcgggcctaggtactcattggg

SEQ ID NO: 36597 - DNA, 28 bp, synthetic construct
  source 1..28: mol_type = other DNA
gggcgggcctaggtactcattgggccgg

SEQ ID NO: 36598 - DNA, 28 bp, synthetic construct
  source 1..28: mol_type = other DNA
ggcgggcctaggtactcattgggccggg

SEQ ID NO: 36599 - DNA, 28 bp, synthetic construct
  source 1..28: mol_type = other DNA
ataattcccggcccaatgagtacctagg

SEQ ID NO: 36600 - DNA, 28 bp, synthetic construct
  source 1..28: mol_type = other DNA
attgggccgggaattatgtcagtcttgg

SEQ ID NO: 36601 - DNA, 28 bp, synthetic construct
  source 1..28: mol_type = other DNA
ttgggccgggaattatgtcagtcttggg

SEQ ID NO: 36602 - DNA, 28 bp, synthetic construct
  source 1..28: mol_type = other DNA
gatttcccaagactgacataattcccgg

SEQ ID NO: 36603 - DNA, 28 bp, synthetic construct
  source 1..28: mol_type = other DNA
ggaattatgtcagtcttgggaaatcagg

SEQ ID NO: 36604 - DNA, 28 bp, synthetic construct
  source 1..28: mol_type = other DNA
tatgtcagtcttgggaaatcaggtccgg

SEQ ID NO: 36605 - DNA, 28 bp, synthetic construct
  source 1..28: mol_type = other DNA
atgtcagtcttgggaaatcaggtccggg

SEQ ID NO: 36606 - DNA, 28 bp, synthetic construct
  source 1..28: mol_type = other DNA
tgtcagtcttgggaaatcaggtccgggg

SEQ ID NO: 36607 - DNA, 28 bp, synthetic construct
  source 1..28: mol_type = other DNA
tcttgggaaatcaggtccggggatgagg

SEQ ID NO: 36608 - DNA, 28 bp, synthetic construct
  source 1..28: mol_type = other DNA
tgggaaatcaggtccggggatgaggagg

SEQ ID NO: 36609 - DNA, 28 bp, synthetic construct
  source 1..28: mol_type = other DNA
atggctgagtgtacctcctcatccccgg

SEQ ID NO: 36610 - DNA, 28 bp, synthetic construct
  source 1..28: mol_type = other DNA
gggatgaggaggtacactcagccattgg

SEQ ID NO: 36611 - DNA, 28 bp, synthetic construct
  source 1..28: mol_type = other DNA
ggatgaggaggtacactcagccattggg

SEQ ID NO: 36612 - DNA, 28 bp, synthetic construct
  source 1..28: mol_type = other DNA
ctgattggcagcagagagggcccaatgg

SEQ ID NO: 36613 - DNA, 28 bp, synthetic construct
  source 1..28: mol_type = other DNA
ttgggccctctctgctgccaatcagagg

SEQ ID NO: 36614 - DNA, 28 bp, synthetic construct
  source 1..28: mol_type = other DNA
tgggccctctctgctgccaatcagaggg

SEQ ID NO: 36615 - DNA, 28 bp, synthetic construct
  source 1..28: mol_type = other DNA
atgtccctctgattggcagcagagaggg

SEQ ID NO: 36616 - DNA, 28 bp, synthetic construct
  source 1..28: mol_type = other DNA
gatgtccctctgattggcagcagagagg

SEQ ID NO: 36617 - DNA, 28 bp, synthetic construct
  source 1..28: mol_type = other DNA
tgccaatcagagggacatccgtcgacgg

SEQ ID NO: 36618 - DNA, 28 bp, synthetic construct
  source 1..28: mol_type = other DNA
ggccgtcgacggatgtccctctgattgg

SEQ ID NO: 36619 - DNA, 28 bp, synthetic construct
  source 1..28: mol_type = other DNA
tcagagggacatccgtcgacggccccgg

SEQ ID NO: 36620 - DNA, 28 bp, synthetic construct
  source 1..28: mol_type = other DNA
ggacatccgtcgacggccccggcctcgg

SEQ ID NO: 36621 - DNA, 28 bp, synthetic construct
  source 1..28: mol_type = other DNA
aacgagccgaggccggggccgtcgacgg

SEQ ID NO: 36622 - DNA, 28 bp, synthetic construct
  source 1..28: mol_type = other DNA
acggccccggcctcggctcgttgattgg

SEQ ID NO: 36623 - DNA, 28 bp, synthetic construct
  source 1..28: mol_type = other DNA
ttctccaatcaacgagccgaggccgggg

SEQ ID NO: 36624 - DNA, 28 bp, synthetic construct
  source 1..28: mol_type = other DNA
tttctccaatcaacgagccgaggccggg

SEQ ID NO: 36625 - DNA, 28 bp, synthetic construct
  source 1..28: mol_type = other DNA
gtttctccaatcaacgagccgaggccgg

SEQ ID NO: 36626 - DNA, 28 bp, synthetic construct
  source 1..28: mol_type = other DNA
aacagtttctccaatcaacgagccgagg

SEQ ID NO: 36627 - DNA, 28 bp, synthetic construct
  source 1..28: mol_type = other DNA
ctcgttgattggagaaactgttcctagg

SEQ ID NO: 36628 - DNA, 28 bp, synthetic construct
  source 1..28: mol_type = other DNA
tcgttgattggagaaactgttcctaggg

SEQ ID NO: 36629 - DNA, 28 bp, synthetic construct
  source 1..28: mol_type = other DNA
ggagaaactgttcctagggtgtttgcgg

SEQ ID NO: 36630 - DNA, 28 bp, synthetic construct
  source 1..28: mol_type = other DNA
gaaactgttcctagggtgtttgcggcgg

SEQ ID NO: 36631 - DNA, 28 bp, synthetic construct
  source 1..28: mol_type = other DNA
aaactgttcctagggtgtttgcggcggg

SEQ ID NO: 36632 - DNA, 28 bp, synthetic construct
  source 1..28: mol_type = other DNA
ctgttcctagggtgtttgcggcgggcgg

SEQ ID NO: 36633 - DNA, 28 bp, synthetic construct
  source 1..28: mol_type = other DNA
tgttcctagggtgtttgcggcgggcggg

SEQ ID NO: 36634 - DNA, 28 bp, synthetic construct
  source 1..28: mol_type = other DNA
gaaacccgcccgccgcaaacaccctagg

SEQ ID NO: 36635 - DNA, 28 bp, synthetic construct
  source 1..28: mol_type = other DNA
tttgcggcgggcgggtttccgagtgcgg

SEQ ID NO: 36636 - DNA, 28 bp, synthetic construct
  source 1..28: mol_type = other DNA
cgggcgggtttccgagtgcggtagcagg

SEQ ID NO: 36637 - DNA, 28 bp, synthetic construct
  source 1..28: mol_type = other DNA
gcgggtttccgagtgcggtagcaggagg

SEQ ID NO: 36638 - DNA, 28 bp, synthetic construct
  source 1..28: mol_type = other DNA
cgggtttccgagtgcggtagcaggaggg

SEQ ID NO: 36639 - DNA, 28 bp, synthetic construct
  source 1..28: mol_type = other DNA
gggtttccgagtgcggtagcaggagggg

SEQ ID NO: 36640 - DNA, 28 bp, synthetic construct
  source 1..28: mol_type = other DNA
ggtttccgagtgcggtagcaggaggggg

SEQ ID NO: 36641 - DNA, 28 bp, synthetic construct
  source 1..28: mol_type = other DNA
ttccgagtgcggtagcaggagggggcgg

SEQ ID NO: 36642 - DNA, 28 bp, synthetic construct
  source 1..28: mol_type = other DNA
tccgagtgcggtagcaggagggggcggg

SEQ ID NO: 36643 - DNA, 28 bp, synthetic construct
  source 1..28: mol_type = other DNA
ccccgccccctcctgctaccgcactcgg

SEQ ID NO: 36644 - DNA, 28 bp, synthetic construct
  source 1..28: mol_type = other DNA
agtgcggtagcaggagggggcggggagg

SEQ ID NO: 36645 - DNA, 28 bp, synthetic construct
  source 1..28: mol_type = other DNA
tagcaggagggggcggggaggtaagcgg

SEQ ID NO: 36646 - DNA, 28 bp, synthetic construct
  source 1..28: mol_type = other DNA
caggagggggcggggaggtaagcggagg

SEQ ID NO: 36647 - DNA, 28 bp, synthetic construct
  source 1..28: mol_type = other DNA
gaggtaagcggaggctccgagctctagg

SEQ ID NO: 36648 - DNA, 28 bp, synthetic construct
  source 1..28: mol_type = other DNA
taagcggaggctccgagctctaggccgg

SEQ ID NO: 36649 - DNA, 28 bp, synthetic construct
  source 1..28: mol_type = other DNA
cggaggctccgagctctaggccggccgg

SEQ ID NO: 36650 - DNA, 28 bp, synthetic construct
  source 1..28: mol_type = other DNA
aggctccgagctctaggccggccggcgg

SEQ ID NO: 36651 - DNA, 28 bp, synthetic construct
  source 1..28: mol_type = other DNA
ctccgagctctaggccggccggcggtgg

SEQ ID NO: 36652 - DNA, 28 bp, synthetic construct
  source 1..28: mol_type = other DNA
cgccaccgccggccggcctagagctcgg

SEQ ID NO: 36653 - DNA, 28 bp, synthetic construct
  source 1..28: mol_type = other DNA
cgagctctaggccggccggcggtggcgg

SEQ ID NO: 36654 - DNA, 28 bp, synthetic construct
  source 1..28: mol_type = other DNA
gctctaggccggccggcggtggcggcgg

SEQ ID NO: 36655 - DNA, 28 bp, synthetic construct
  source 1..28: mol_type = other DNA
aggccggccggcggtggcggcggcgagg

SEQ ID NO: 36656 - DNA, 28 bp, synthetic construct
  source 1..28: mol_type = other DNA
cggcctcgccgccgccaccgccggccgg

SEQ ID NO: 36657 - DNA, 28 bp, synthetic construct
  source 1..28: mol_type = other DNA
cggccggcggtggcggcggcgaggccgg

SEQ ID NO: 36658 - DNA, 28 bp, synthetic construct
  source 1..28: mol_type = other DNA
ggccggcggtggcggcggcgaggccggg

SEQ ID NO: 36659 - DNA, 28 bp, synthetic construct
  source 1..28: mol_type = other DNA
gtcccggcctcgccgccgccaccgccgg

SEQ ID NO: 36660 - DNA, 28 bp, synthetic construct
  source 1..28: mol_type = other DNA
cggtggcggcggcgaggccgggactcgg

SEQ ID NO: 36661 - DNA, 28 bp, synthetic construct
  source 1..28: mol_type = other DNA
ggtggcggcggcgaggccgggactcggg

SEQ ID NO: 36662 - DNA, 28 bp, synthetic construct
  source 1..28: mol_type = other DNA
ggcggcgaggccgggactcgggcttagg

SEQ ID NO: 36663 - DNA, 28 bp, synthetic construct
  source 1..28: mol_type = other DNA
gcggcgaggccgggactcgggcttaggg

SEQ ID NO: 36664 - DNA, 28 bp, synthetic construct
  source 1..28: mol_type = other DNA
cacagcaggccctaagcccgagtcccgg

SEQ ID NO: 36665 - DNA, 28 bp, synthetic construct
  source 1..28: mol_type = other DNA
cgggactcgggcttagggcctgctgtgg

SEQ ID NO: 36666 - DNA, 28 bp, synthetic construct
  source 1..28: mol_type = other DNA
gactcgggcttagggcctgctgtggagg

SEQ ID NO: 36667 - DNA, 28 bp, synthetic construct
  source 1..28: mol_type = other DNA
ggcttagggcctgctgtggaggcagcgg

SEQ ID NO: 36668 - DNA, 28 bp, synthetic construct
  source 1..28: mol_type = other DNA
ttagggcctgctgtggaggcagcggcgg

SEQ ID NO: 36669 - DNA, 28 bp, synthetic construct
  source 1..28: mol_type = other DNA
cggcgtccgccgctgcctccacagcagg

SEQ ID NO: 36670 - DNA, 28 bp, synthetic construct
  source 1..28: mol_type = other DNA
cagcggcggacgccgagctaagcagtgg

SEQ ID NO: 36671 - DNA, 28 bp, synthetic construct
  source 1..28: mol_type = other DNA
agcggcggacgccgagctaagcagtggg

SEQ ID NO: 36672 - DNA, 28 bp, synthetic construct
  source 1..28: mol_type = other DNA
ggacgccgagctaagcagtgggtatcgg

SEQ ID NO: 36673 - DNA, 28 bp, synthetic construct
  source 1..28: mol_type = other DNA
gacgccgagctaagcagtgggtatcggg

SEQ ID NO: 36674 - DNA, 28 bp, synthetic construct
  source 1..28: mol_type = other DNA
tgtgcccgatacccactgcttagctcgg

SEQ ID NO: 36675 - DNA, 28 bp, synthetic construct
  source 1..28: mol_type = other DNA
gtatcgggcacattcctttcccagaagg

SEQ ID NO: 36676 - DNA, 28 bp, synthetic construct
  source 1..28: mol_type = other DNA
tatcgggcacattcctttcccagaaggg

SEQ ID NO: 36677 - DNA, 28 bp, synthetic construct
  source 1..28: mol_type = other DNA
cgggcacattcctttcccagaagggagg

SEQ ID NO: 36678 - DNA, 28 bp, synthetic construct
  source 1..28: mol_type = other DNA
gggcacattcctttcccagaagggaggg

SEQ ID NO: 36679 - DNA, 28 bp, synthetic construct
  source 1..28: mol_type = other DNA
gcgctgcaaccctcccttctgggaaagg

SEQ ID NO: 36680 - DNA, 28 bp, synthetic construct
  source 1..28: mol_type = other DNA
cccagaagggagggttgcagcgccgcgg

SEQ ID NO: 36681 - DNA, 28 bp, synthetic construct
  source 1..28: mol_type = other DNA
ccagaagggagggttgcagcgccgcggg

SEQ ID NO: 36682 - DNA, 28 bp, synthetic construct
  source 1..28: mol_type = other DNA
cagaagggagggttgcagcgccgcgggg

SEQ ID NO: 36683 - DNA, 28 bp, synthetic construct
  source 1..28: mol_type = other DNA
ggagggttgcagcgccgcggggccgagg

SEQ ID NO: 36684 - DNA, 28 bp, synthetic construct
  source 1..28: mol_type = other DNA
tgcagcgccgcggggccgaggcttatgg

SEQ ID NO: 36685 - DNA, 28 bp, synthetic construct
  source 1..28: mol_type = other DNA
gcagcgccgcggggccgaggcttatggg

SEQ ID NO: 36686 - DNA, 28 bp, synthetic construct
  source 1..28: mol_type = other DNA
cagcgccgcggggccgaggcttatgggg

SEQ ID NO: 36687 - DNA, 28 bp, synthetic construct
  source 1..28: mol_type = other DNA
cgtcgccccataagcctcggccccgcgg

SEQ ID NO: 36688 - DNA, 28 bp, synthetic construct
  source 1..28: mol_type = other DNA
cgcggggccgaggcttatggggcgacgg

SEQ ID NO: 36689 - DNA, 28 bp, synthetic construct
  source 1..28: mol_type = other DNA
gcggggccgaggcttatggggcgacggg

SEQ ID NO: 36690 - DNA, 28 bp, synthetic construct
  source 1..28: mol_type = other DNA
ggccgaggcttatggggcgacgggatgg

SEQ ID NO: 36691 - DNA, 28 bp, synthetic construct
  source 1..28: mol_type = other DNA
caccatcccgtcgccccataagcctcgg

SEQ ID NO: 36692 - DNA, 28 bp, synthetic construct
  source 1..28: mol_type = other DNA
cttatggggcgacgggatggtgctgagg

SEQ ID NO: 36693 - DNA, 28 bp, synthetic construct
  source 1..28: mol_type = other DNA
gggcgacgggatggtgctgaggtgcagg

SEQ ID NO: 36694 - DNA, 28 bp, synthetic construct
  source 1..28: mol_type = other DNA
cgacgggatggtgctgaggtgcaggagg

SEQ ID NO: 36695 - DNA, 28 bp, synthetic construct
  source 1..28: mol_type = other DNA
cgggatggtgctgaggtgcaggaggcgg

SEQ ID NO: 36696 - DNA, 28 bp, synthetic construct
  source 1..28: mol_type = other DNA
gggatggtgctgaggtgcaggaggcggg

SEQ ID NO: 36697 - DNA, 28 bp, synthetic construct
  source 1..28: mol_type = other DNA
ggatggtgctgaggtgcaggaggcgggg

SEQ ID NO: 36698 - DNA, 28 bp, synthetic construct
  source 1..28: mol_type = other DNA
gatggtgctgaggtgcaggaggcggggg

SEQ ID NO: 36699 - DNA, 28 bp, synthetic construct
  source 1..28: mol_type = other DNA
tgaggtgcaggaggcgggggccgagcgg

SEQ ID NO: 36700 - DNA, 28 bp, synthetic construct
  source 1..28: mol_type = other DNA
gaggtgcaggaggcgggggccgagcggg

SEQ ID NO: 36701 - DNA, 28 bp, synthetic construct
  source 1..28: mol_type = other DNA
aggtgcaggaggcgggggccgagcgggg

SEQ ID NO: 36702 - DNA, 28 bp, synthetic construct
  source 1..28: mol_type = other DNA
gccgagcggggttcccgccagagcccgg

SEQ ID NO: 36703 - DNA, 28 bp, synthetic construct
  source 1..28: mol_type = other DNA
gccgggctctggcgggaaccccgctcgg

SEQ ID NO: 36704 - DNA, 28 bp, synthetic construct
  source 1..28: mol_type = other DNA
cggggttcccgccagagcccggccctgg

SEQ ID NO: 36705 - DNA, 28 bp, synthetic construct
  source 1..28: mol_type = other DNA
ggggttcccgccagagcccggccctggg

SEQ ID NO: 36706 - DNA, 28 bp, synthetic construct
  source 1..28: mol_type = other DNA
gtcaggcccagggccgggctctggcggg

SEQ ID NO: 36707 - DNA, 28 bp, synthetic construct
  source 1..28: mol_type = other DNA
tgtcaggcccagggccgggctctggcgg

SEQ ID NO: 36708 - DNA, 28 bp, synthetic construct
  source 1..28: mol_type = other DNA
gccagagcccggccctgggcctgacagg

SEQ ID NO: 36709 - DNA, 28 bp, synthetic construct
  source 1..28: mol_type = other DNA
ccagagcccggccctgggcctgacaggg

SEQ ID NO: 36710 - DNA, 28 bp, synthetic construct
  source 1..28: mol_type = other DNA
gagcccggccctgggcctgacagggagg

SEQ ID NO: 36711 - DNA, 28 bp, synthetic construct
  source 1..28: mol_type = other DNA
agcccggccctgggcctgacagggaggg

SEQ ID NO: 36712 - DNA, 28 bp, synthetic construct
  source 1..28: mol_type = other DNA
gcccggccctgggcctgacagggagggg

SEQ ID NO: 36713 - DNA, 28 bp, synthetic construct
  source 1..28: mol_type = other DNA
gcccctccctgtcaggcccagggccggg

SEQ ID NO: 36714 - DNA, 28 bp, synthetic construct
  source 1..28: mol_type = other DNA
ggcccctccctgtcaggcccagggccgg

SEQ ID NO: 36715 - DNA, 28 bp, synthetic construct
  source 1..28: mol_type = other DNA
gcggggcccctccctgtcaggcccaggg

SEQ ID NO: 36716 - DNA, 28 bp, synthetic construct
  source 1..28: mol_type = other DNA
cgcggggcccctccctgtcaggcccagg

SEQ ID NO: 36717 - DNA, 28 bp, synthetic construct
  source 1..28: mol_type = other DNA
gggcctgacagggaggggccccgcgcgg

SEQ ID NO: 36718 - DNA, 28 bp, synthetic construct
  source 1..28: mol_type = other DNA
ggcctgacagggaggggccccgcgcggg

SEQ ID NO: 36719 - DNA, 28 bp, synthetic construct
  source 1..28: mol_type = other DNA
gcctgacagggaggggccccgcgcgggg

SEQ ID NO: 36720 - DNA, 28 bp, synthetic construct
  source 1..28: mol_type = other DNA
gccccgcgcggggcccctccctgtcagg

SEQ ID NO: 36721 - DNA, 28 bp, synthetic construct
  source 1..28: mol_type = other DNA
gggaggggccccgcgcggggccgagagg

SEQ ID NO: 36722 - DNA, 28 bp, synthetic construct
  source 1..28: mol_type = other DNA
ccccgcgcggggccgagaggaaagctgg

SEQ ID NO: 36723 - DNA, 28 bp, synthetic construct
  source 1..28: mol_type = other DNA
gccagctttcctctcggccccgcgcggg

SEQ ID NO: 36724 - DNA, 28 bp, synthetic construct
  source 1..28: mol_type = other DNA
agccagctttcctctcggccccgcgcgg

SEQ ID NO: 36725 - DNA, 28 bp, synthetic construct
  source 1..28: mol_type = other DNA
gcggggccgagaggaaagctggctccgg

SEQ ID NO: 36726 - DNA, 28 bp, synthetic construct
  source 1..28: mol_type = other DNA
cggggccgagaggaaagctggctccggg

SEQ ID NO: 36727 - DNA, 28 bp, synthetic construct
  source 1..28: mol_type = other DNA
ggggccgagaggaaagctggctccgggg

SEQ ID NO: 36728 - DNA, 28 bp, synthetic construct
  source 1..28: mol_type = other DNA
gccgagaggaaagctggctccggggtgg

SEQ ID NO: 36729 - DNA, 28 bp, synthetic construct
  source 1..28: mol_type = other DNA
ccgagaggaaagctggctccggggtggg

SEQ ID NO: 36730 - DNA, 28 bp, synthetic construct
  source 1..28: mol_type = other DNA
gaggaaagctggctccggggtgggatgg

SEQ ID NO: 36731 - DNA, 28 bp, synthetic construct
  source 1..28: mol_type = other DNA
aagctggctccggggtgggatggactgg

SEQ ID NO: 36732 - DNA, 28 bp, synthetic construct
  source 1..28: mol_type = other DNA
agctggctccggggtgggatggactggg

SEQ ID NO: 36733 - DNA, 28 bp, synthetic construct
  source 1..28: mol_type = other DNA
ggctccggggtgggatggactgggcagg

SEQ ID NO: 36734 - DNA, 28 bp, synthetic construct
  source 1..28: mol_type = other DNA
gctccggggtgggatggactgggcaggg

SEQ ID NO: 36735 - DNA, 28 bp, synthetic construct
  source 1..28: mol_type = other DNA
caaccctgcccagtccatcccaccccgg

SEQ ID NO: 36736 - DNA, 28 bp, synthetic construct
  source 1..28: mol_type = other DNA
gggtgggatggactgggcagggttgagg

SEQ ID NO: 36737 - DNA, 28 bp, synthetic construct
  source 1..28: mol_type = other DNA
ggtgggatggactgggcagggttgaggg

SEQ ID NO: 36738 - DNA, 28 bp, synthetic construct
  source 1..28: mol_type = other DNA
actgggcagggttgagggcacgagaagg

SEQ ID NO: 36739 - DNA, 28 bp, synthetic construct
  source 1..28: mol_type = other DNA
gcagggttgagggcacgagaaggcgtgg

SEQ ID NO: 36740 - DNA, 28 bp, synthetic construct
  source 1..28: mol_type = other DNA
tgagggcacgagaaggcgtggtgtgagg

SEQ ID NO: 36741 - DNA, 28 bp, synthetic construct
  source 1..28: mol_type = other DNA
gcacgagaaggcgtggtgtgaggcctgg

SEQ ID NO: 36742 - DNA, 28 bp, synthetic construct
  source 1..28: mol_type = other DNA
gaaggcgtggtgtgaggcctggacttgg

SEQ ID NO: 36743 - DNA, 28 bp, synthetic construct
  source 1..28: mol_type = other DNA
aaggcgtggtgtgaggcctggacttggg

SEQ ID NO: 36744 - DNA, 28 bp, synthetic construct
  source 1..28: mol_type = other DNA
gtggtgtgaggcctggacttgggagtgg

SEQ ID NO: 36745 - DNA, 28 bp, synthetic construct
  source 1..28: mol_type = other DNA
tggtgtgaggcctggacttgggagtggg

SEQ ID NO: 36746 - DNA, 28 bp, synthetic construct
  source 1..28: mol_type = other DNA
ggtgtgaggcctggacttgggagtgggg

SEQ ID NO: 36747 - DNA, 28 bp, synthetic construct
  source 1..28: mol_type = other DNA
gtgaggcctggacttgggagtggggtgg

SEQ ID NO: 36748 - DNA, 28 bp, synthetic construct
  source 1..28: mol_type = other DNA
tgaggcctggacttgggagtggggtggg

SEQ ID NO: 36749 - DNA, 28 bp, synthetic construct
  source 1..28: mol_type = other DNA
gaggcctggacttgggagtggggtgggg

SEQ ID NO: 36750 - DNA, 28 bp, synthetic construct
  source 1..28: mol_type = other DNA
atggccccaccccactcccaagtccagg

SEQ ID NO: 36751 - DNA, 28 bp, synthetic construct
  source 1..28: mol_type = other DNA
ggacttgggagtggggtggggccatcgg

SEQ ID NO: 36752 - DNA, 28 bp, synthetic construct
  source 1..28: mol_type = other DNA
gacttgggagtggggtggggccatcggg

SEQ ID NO: 36753 - DNA, 28 bp, synthetic construct
  source 1..28: mol_type = other DNA
tgggagtggggtggggccatcgggacgg

SEQ ID NO: 36754 - DNA, 28 bp, synthetic construct
  source 1..28: mol_type = other DNA
gagtggggtggggccatcgggacggagg

SEQ ID NO: 36755 - DNA, 28 bp, synthetic construct
  source 1..28: mol_type = other DNA
agtggggtggggccatcgggacggaggg

SEQ ID NO: 36756 - DNA, 28 bp, synthetic construct
  source 1..28: mol_type = other DNA
ggggtggggccatcgggacggagggcgg

SEQ ID NO: 36757 - DNA, 28 bp, synthetic construct
  source 1..28: mol_type = other DNA
gggtggggccatcgggacggagggcggg

SEQ ID NO: 36758 - DNA, 28 bp, synthetic construct
  source 1..28: mol_type = other DNA
ggtggggccatcgggacggagggcgggg

SEQ ID NO: 36759 - DNA, 28 bp, synthetic construct
  source 1..28: mol_type = other DNA
ggggccatcgggacggagggcggggtgg

SEQ ID NO: 36760 - DNA, 28 bp, synthetic construct
  source 1..28: mol_type = other DNA
gggccatcgggacggagggcggggtggg

SEQ ID NO: 36761 - DNA, 28 bp, synthetic construct
  source 1..28: mol_type = other DNA
ggccatcgggacggagggcggggtgggg

SEQ ID NO: 36762 - DNA, 28 bp, synthetic construct
  source 1..28: mol_type = other DNA
aaccccaccccgccctccgtcccgatgg

SEQ ID NO: 36763 - DNA, 28 bp, synthetic construct
  source 1..28: mol_type = other DNA
ggagggcggggtggggtttgctgtaagg

SEQ ID NO: 36764 - DNA, 28 bp, synthetic construct
  source 1..28: mol_type = other DNA
gagggcggggtggggtttgctgtaaggg

SEQ ID NO: 36765 - DNA, 28 bp, synthetic construct
  source 1..28: mol_type = other DNA
ggcggggtggggtttgctgtaagggtgg

SEQ ID NO: 36766 - DNA, 28 bp, synthetic construct
  source 1..28: mol_type = other DNA
gcggggtggggtttgctgtaagggtggg

SEQ ID NO: 36767 - DNA, 28 bp, synthetic construct
  source 1..28: mol_type = other DNA
tggggtttgctgtaagggtgggtcaagg

SEQ ID NO: 36768 - DNA, 28 bp, synthetic construct
  source 1..28: mol_type = other DNA
tttgctgtaagggtgggtcaaggccagg

SEQ ID NO: 36769 - DNA, 28 bp, synthetic construct
  source 1..28: mol_type = other DNA
ttgctgtaagggtgggtcaaggccaggg

SEQ ID NO: 36770 - DNA, 28 bp, synthetic construct
  source 1..28: mol_type = other DNA
ggccagggaagtagcacttgttcgctgg

SEQ ID NO: 36771 - DNA, 28 bp, synthetic construct
  source 1..28: mol_type = other DNA
ggccagcgaacaagtgctacttccctgg

SEQ ID NO: 36772 - DNA, 28 bp, synthetic construct
  source 1..28: mol_type = other DNA
gtagcacttgttcgctggccgcccctgg

SEQ ID NO: 36773 - DNA, 28 bp, synthetic construct
  source 1..28: mol_type = other DNA
gcacttgttcgctggccgcccctggagg

SEQ ID NO: 36774 - DNA, 28 bp, synthetic construct
  source 1..28: mol_type = other DNA
ggccgcccctggaggctagaagctccgg

SEQ ID NO: 36775 - DNA, 28 bp, synthetic construct
  source 1..28: mol_type = other DNA
cgccggagcttctagcctccaggggcgg

SEQ ID NO: 36776 - DNA, 28 bp, synthetic construct
  source 1..28: mol_type = other DNA
cggcgccggagcttctagcctccagggg

SEQ ID NO: 36777 - DNA, 28 bp, synthetic construct
  source 1..28: mol_type = other DNA
tcggcgccggagcttctagcctccaggg

SEQ ID NO: 36778 - DNA, 28 bp, synthetic construct
  source 1..28: mol_type = other DNA
ctcggcgccggagcttctagcctccagg

SEQ ID NO: 36779 - DNA, 28 bp, synthetic construct
  source 1..28: mol_type = other DNA
aggctagaagctccggcgccgagagtgg

SEQ ID NO: 36780 - DNA, 28 bp, synthetic construct
  source 1..28: mol_type = other DNA
ggctagaagctccggcgccgagagtggg

SEQ ID NO: 36781 - DNA, 28 bp, synthetic construct
  source 1..28: mol_type = other DNA
gaagctccggcgccgagagtgggcatgg

SEQ ID NO: 36782 - DNA, 28 bp, synthetic construct
  source 1..28: mol_type = other DNA
aagtcgccatgcccactctcggcgccgg

SEQ ID NO: 36783 - DNA, 28 bp, synthetic construct
  source 1..28: mol_type = other DNA
ggcgccgagagtgggcatggcgacttgg

SEQ ID NO: 36784 - DNA, 28 bp, synthetic construct
  source 1..28: mol_type = other DNA
gagaccaagtcgccatgcccactctcgg

SEQ ID NO: 36785 - DNA, 28 bp, synthetic construct
  source 1..28: mol_type = other DNA
gtgggcatggcgacttggtctcagccgg

SEQ ID NO: 36786 - DNA, 28 bp, synthetic construct
  source 1..28: mol_type = other DNA
atggcgacttggtctcagccggactcgg

SEQ ID NO: 36787 - DNA, 28 bp, synthetic construct
  source 1..28: mol_type = other DNA
tggcgacttggtctcagccggactcggg

SEQ ID NO: 36788 - DNA, 28 bp, synthetic construct
  source 1..28: mol_type = other DNA
ttggtctcagccggactcgggtatccgg

SEQ ID NO: 36789 - DNA, 28 bp, synthetic construct
  source 1..28: mol_type = other DNA
tggtctcagccggactcgggtatccggg

SEQ ID NO: 36790 - DNA, 28 bp, synthetic construct
  source 1..28: mol_type = other DNA
ctcagccggactcgggtatccgggcagg

SEQ ID NO: 36791 - DNA, 28 bp, synthetic construct
  source 1..28: mol_type = other DNA
tcagccggactcgggtatccgggcaggg

SEQ ID NO: 36792 - DNA, 28 bp, synthetic construct
  source 1..28: mol_type = other DNA
gccggactcgggtatccgggcagggtgg

SEQ ID NO: 36793 - DNA, 28 bp, synthetic construct
  source 1..28: mol_type = other DNA
cccaccctgcccggatacccgagtccgg

SEQ ID NO: 36794 - DNA, 28 bp, synthetic construct
  source 1..28: mol_type = other DNA
atccgggcagggtgggaccagcctcagg

SEQ ID NO: 36795 - DNA, 28 bp, synthetic construct
  source 1..28: mol_type = other DNA
agcctgaggctggtcccaccctgcccgg

SEQ ID NO: 36796 - DNA, 28 bp, synthetic construct
  source 1..28: mol_type = other DNA
gcagggtgggaccagcctcaggctatgg

SEQ ID NO: 36797 - DNA, 28 bp, synthetic construct
  source 1..28: mol_type = other DNA
cagggtgggaccagcctcaggctatggg

SEQ ID NO: 36798 - DNA, 28 bp, synthetic construct
  source 1..28: mol_type = other DNA
aggtgcagggcccatagcctgaggctgg

SEQ ID NO: 36799 - DNA, 28 bp, synthetic construct
  source 1..28: mol_type = other DNA
aagtaggtgcagggcccatagcctgagg

SEQ ID NO: 36800 - DNA, 28 bp, synthetic construct
  source 1..28: mol_type = other DNA
gggccctgcacctacttgatttttaagg

SEQ ID NO: 36801 - DNA, 28 bp, synthetic construct
  source 1..28: mol_type = other DNA
ggccctgcacctacttgatttttaaggg

SEQ ID NO: 36802 - DNA, 28 bp, synthetic construct
  source 1..28: mol_type = other DNA
gtcccttaaaaatcaagtaggtgcaggg

SEQ ID NO: 36803 - DNA, 28 bp, synthetic construct
  source 1..28: mol_type = other DNA
agtcccttaaaaatcaagtaggtgcagg

SEQ ID NO: 36804 - DNA, 28 bp, synthetic construct
  source 1..28: mol_type = other DNA
ggacaaagtcccttaaaaatcaagtagg

SEQ ID NO: 36805 - DNA, 28 bp, synthetic construct
  source 1..28: mol_type = other DNA
tacttgatttttaagggactttgtccgg

SEQ ID NO: 36806 - DNA, 28 bp, synthetic construct
  source 1..28: mol_type = other DNA
ctttgtccggttcctcgaacttaattgg

SEQ ID NO: 36807 - DNA, 28 bp, synthetic construct
  source 1..28: mol_type = other DNA
caggagccaattaagttcgaggaaccgg

SEQ ID NO: 36808 - DNA, 28 bp, synthetic construct
  source 1..28: mol_type = other DNA
cggttcctcgaacttaattggctcctgg

SEQ ID NO: 36809 - DNA, 28 bp, synthetic construct
  source 1..28: mol_type = other DNA
ggttcctcgaacttaattggctcctggg

SEQ ID NO: 36810 - DNA, 28 bp, synthetic construct
  source 1..28: mol_type = other DNA
tcctcgaacttaattggctcctgggagg

SEQ ID NO: 36811 - DNA, 28 bp, synthetic construct
  source 1..28: mol_type = other DNA
acctcccaggagccaattaagttcgagg

SEQ ID NO: 36812 - DNA, 28 bp, synthetic construct
  source 1..28: mol_type = other DNA
acgcaatttattactaaaacctcccagg

SEQ ID NO: 36813 - DNA, 28 bp, synthetic construct
  source 1..28: mol_type = other DNA
agtagaaggtagaaaacacattcaaagg

SEQ ID NO: 36814 - DNA, 28 bp, synthetic construct
  source 1..28: mol_type = other DNA
atgtgttttctaccttctactgtgaagg

SEQ ID NO: 36815 - DNA, 28 bp, synthetic construct
  source 1..28: mol_type = other DNA
agggtaggaaaaccttcacagtagaagg

SEQ ID NO: 36816 - DNA, 28 bp, synthetic construct
  source 1..28: mol_type = other DNA
atacttttcacatcatgatcagggtagg

SEQ ID NO: 36817 - DNA, 28 bp, synthetic construct
  source 1..28: mol_type = other DNA
taccctgatcatgatgtgaaaagtatgg

SEQ ID NO: 36818 - DNA, 28 bp, synthetic construct
  source 1..28: mol_type = other DNA
ttccatacttttcacatcatgatcaggg

SEQ ID NO: 36819 - DNA, 28 bp, synthetic construct
  source 1..28: mol_type = other DNA
attccatacttttcacatcatgatcagg

SEQ ID NO: 36820 - DNA, 28 bp, synthetic construct
  source 1..28: mol_type = other DNA
ctgaaatgggaatcacaaaagcaacagg

SEQ ID NO: 36821 - DNA, 28 bp, synthetic construct
  source 1..28: mol_type = other DNA
ctgttgcttttgtgattcccatttcagg

SEQ ID NO: 36822 - DNA, 28 bp, synthetic construct
  source 1..28: mol_type = other DNA
ttgtgattcccatttcaggtttctctgg

SEQ ID NO: 36823 - DNA, 28 bp, synthetic construct
  source 1..28: mol_type = other DNA
gggggtttccagagaaacctgaaatggg

SEQ ID NO: 36824 - DNA, 28 bp, synthetic construct
  source 1..28: mol_type = other DNA
ggggggtttccagagaaacctgaaatgg

SEQ ID NO: 36825 - DNA, 28 bp, synthetic construct
  source 1..28: mol_type = other DNA
tttcaggtttctctggaaacccccctgg

SEQ ID NO: 36826 - DNA, 28 bp, synthetic construct
  source 1..28: mol_type = other DNA
tctctggaaacccccctggtaagtgtgg

SEQ ID NO: 36827 - DNA, 28 bp, synthetic construct
  source 1..28: mol_type = other DNA
ctggaaacccccctggtaagtgtggagg

SEQ ID NO: 36828 - DNA, 28 bp, synthetic construct
  source 1..28: mol_type = other DNA
gaaacccccctggtaagtgtggaggagg

SEQ ID NO: 36829 - DNA, 28 bp, synthetic construct
  source 1..28: mol_type = other DNA
acccccctggtaagtgtggaggaggcgg

SEQ ID NO: 36830 - DNA, 28 bp, synthetic construct
  source 1..28: mol_type = other DNA
cccccctggtaagtgtggaggaggcggg

SEQ ID NO: 36831 - DNA, 28 bp, synthetic construct
  source 1..28: mol_type = other DNA
tcccgcctcctccacacttaccaggggg

SEQ ID NO: 36832 - DNA, 28 bp, synthetic construct
  source 1..28: mol_type = other DNA
gtcccgcctcctccacacttaccagggg

SEQ ID NO: 36833 - DNA, 28 bp, synthetic construct
  source 1..28: mol_type = other DNA
tgtcccgcctcctccacacttaccaggg

SEQ ID NO: 36834 - DNA, 28 bp, synthetic construct
  source 1..28: mol_type = other DNA
gtgtcccgcctcctccacacttaccagg

SEQ ID NO: 36835 - DNA, 28 bp, synthetic construct
  source 1..28: mol_type = other DNA
gcgggacactctgacccaagacgaaagg

SEQ ID NO: 36836 - DNA, 28 bp, synthetic construct
  source 1..28: mol_type = other DNA
gctggagctacaggcctttcgtcttggg

SEQ ID NO: 36837 - DNA, 28 bp, synthetic construct
  source 1..28: mol_type = other DNA
ggctggagctacaggcctttcgtcttgg

SEQ ID NO: 36838 - DNA, 28 bp, synthetic construct
  source 1..28: mol_type = other DNA
gtttattttctttggctggagctacagg

SEQ ID NO: 36839 - DNA, 28 bp, synthetic construct
  source 1..28: mol_type = other DNA
gctccagccaaagaaaataaaccttagg

SEQ ID NO: 36840 - DNA, 28 bp, synthetic construct
  source 1..28: mol_type = other DNA
ccagccaaagaaaataaaccttaggagg

SEQ ID NO: 36841 - DNA, 28 bp, synthetic construct
  source 1..28: mol_type = other DNA
cagccaaagaaaataaaccttaggaggg

SEQ ID NO: 36842 - DNA, 28 bp, synthetic construct
  source 1..28: mol_type = other DNA
tctccctcctaaggtttattttctttgg

SEQ ID NO: 36843 - DNA, 28 bp, synthetic construct
  source 1..28: mol_type = other DNA
aagaaaataaaccttaggagggagaagg

SEQ ID NO: 36844 - DNA, 28 bp, synthetic construct
  source 1..28: mol_type = other DNA
attttttttttccttctccctcctaagg

SEQ ID NO: 36845 - DNA, 28 bp, synthetic construct
  source 1..28: mol_type = other DNA
gcaggctgttctcaggaacagctgatgg

SEQ ID NO: 36846 - DNA, 28 bp, synthetic construct
  source 1..28: mol_type = other DNA
agctgttcctgagaacagcctgcattgg

SEQ ID NO: 36847 - DNA, 28 bp, synthetic construct
  source 1..28: mol_type = other DNA
gtagattccaatgcaggctgttctcagg

SEQ ID NO: 36848 - DNA, 28 bp, synthetic construct
  source 1..28: mol_type = other DNA
acagcctgcattggaatctacagagagg

SEQ ID NO: 36849 - DNA, 28 bp, synthetic construct
  source 1..28: mol_type = other DNA
ttgtcctctctgtagattccaatgcagg

SEQ ID NO: 36850 - DNA, 28 bp, synthetic construct
  source 1..28: mol_type = other DNA
acagagaggacaactaatgtgagtgagg

SEQ ID NO: 36851 - DNA, 28 bp, synthetic construct
  source 1..28: mol_type = other DNA
atgtgagtgaggaagtgactgtatgtgg

SEQ ID NO: 36852 - DNA, 28 bp, synthetic construct
  source 1..28: mol_type = other DNA
tgaggaagtgactgtatgtggactgtgg

SEQ ID NO: 36853 - DNA, 28 bp, synthetic construct
  source 1..28: mol_type = other DNA
tggactgtggagaaagtaagtcacgtgg

SEQ ID NO: 36854 - DNA, 28 bp, synthetic construct
  source 1..28: mol_type = other DNA
ggactgtggagaaagtaagtcacgtggg

SEQ ID NO: 36855 - DNA, 28 bp, synthetic construct
  source 1..28: mol_type = other DNA
agaaagtaagtcacgtgggcccttgagg

SEQ ID NO: 36856 - DNA, 28 bp, synthetic construct
  source 1..28: mol_type = other DNA
taagtcacgtgggcccttgaggacctgg

SEQ ID NO: 36857 - DNA, 28 bp, synthetic construct
  source 1..28: mol_type = other DNA
cacgtgggcccttgaggacctggactgg

SEQ ID NO: 36858 - DNA, 28 bp, synthetic construct
  source 1..28: mol_type = other DNA
acgtgggcccttgaggacctggactggg

SEQ ID NO: 36859 - DNA, 28 bp, synthetic construct
  source 1..28: mol_type = other DNA
ggcccttgaggacctggactgggttagg

SEQ ID NO: 36860 - DNA, 28 bp, synthetic construct
  source 1..28: mol_type = other DNA
ttcctaacccagtccaggtcctcaaggg

SEQ ID NO: 36861 - DNA, 28 bp, synthetic construct
  source 1..28: mol_type = other DNA
gttcctaacccagtccaggtcctcaagg

SEQ ID NO: 36862 - DNA, 28 bp, synthetic construct
  source 1..28: mol_type = other DNA
agtacaactgttcctaacccagtccagg

SEQ ID NO: 36863 - DNA, 28 bp, synthetic construct
  source 1..28: mol_type = other DNA
gggttaggaacagttgtactttcagagg

SEQ ID NO: 36864 - DNA, 28 bp, synthetic construct
  source 1..28: mol_type = other DNA
aggaacagttgtactttcagaggtgagg

SEQ ID NO: 36865 - DNA, 28 bp, synthetic construct
  source 1..28: mol_type = other DNA
tactttcagaggtgaggtgtcgagaagg

SEQ ID NO: 36866 - DNA, 28 bp, synthetic construct
  source 1..28: mol_type = other DNA
actttcagaggtgaggtgtcgagaaggg

SEQ ID NO: 36867 - DNA, 28 bp, synthetic construct
  source 1..28: mol_type = other DNA
aggtgtcgagaagggaaagtgaatgtgg

SEQ ID NO: 36868 - DNA, 28 bp, synthetic construct
  source 1..28: mol_type = other DNA
tcgagaagggaaagtgaatgtggtctgg

SEQ ID NO: 36869 - DNA, 28 bp, synthetic construct
  source 1..28: mol_type = other DNA
gtgaatgtggtctggagtgtgtccttgg

SEQ ID NO: 36870 - DNA, 28 bp, synthetic construct
  source 1..28: mol_type = other DNA
gtggtctggagtgtgtccttggccttgg

SEQ ID NO: 36871 - DNA, 28 bp, synthetic construct
  source 1..28: mol_type = other DNA
agtgtgtccttggccttggctccacagg

SEQ ID NO: 36872 - DNA, 28 bp, synthetic construct
  source 1..28: mol_type = other DNA
gtgtgtccttggccttggctccacaggg

SEQ ID NO: 36873 - DNA, 28 bp, synthetic construct
  source 1..28: mol_type = other DNA
agcacaccctgtggagccaaggccaagg

SEQ ID NO: 36874 - DNA, 28 bp, synthetic construct
  source 1..28: mol_type = other DNA
gaggaaagcacaccctgtggagccaagg

SEQ ID NO: 36875 - DNA, 28 bp, synthetic construct
  source 1..28: mol_type = other DNA
tggctccacagggtgtgctttcctctgg

SEQ ID NO: 36876 - DNA, 28 bp, synthetic construct
  source 1..28: mol_type = other DNA
ggctccacagggtgtgctttcctctggg

SEQ ID NO: 36877 - DNA, 28 bp, synthetic construct
  source 1..28: mol_type = other DNA
gctccacagggtgtgctttcctctgggg

SEQ ID NO: 36878 - DNA, 28 bp, synthetic construct
  source 1..28: mol_type = other DNA
cggccccagaggaaagcacaccctgtgg

SEQ ID NO: 36879 - DNA, 28 bp, synthetic construct
  source 1..28: mol_type = other DNA
gggtgtgctttcctctggggccgtcagg

SEQ ID NO: 36880 - DNA, 28 bp, synthetic construct
  source 1..28: mol_type = other DNA
ggtgtgctttcctctggggccgtcaggg

SEQ ID NO: 36881 - DNA, 28 bp, synthetic construct
  source 1..28: mol_type = other DNA
gggatgagctccctgacggccccagagg

SEQ ID NO: 36882 - DNA, 28 bp, synthetic construct
  source 1..28: mol_type = other DNA
agaacacaagggatgagctccctgacgg

SEQ ID NO: 36883 - DNA, 28 bp, synthetic construct
  source 1..28: mol_type = other DNA
gggagctcatcccttgtgttctgccagg

SEQ ID NO: 36884 - DNA, 28 bp, synthetic construct
  source 1..28: mol_type = other DNA
ggagctcatcccttgtgttctgccaggg

SEQ ID NO: 36885 - DNA, 28 bp, synthetic construct
  source 1..28: mol_type = other DNA
gctcatcccttgtgttctgccagggtgg

SEQ ID NO: 36886 - DNA, 28 bp, synthetic construct
  source 1..28: mol_type = other DNA
ctcatcccttgtgttctgccagggtggg

SEQ ID NO: 36887 - DNA, 28 bp, synthetic construct
  source 1..28: mol_type = other DNA
tcatcccttgtgttctgccagggtgggg

SEQ ID NO: 36888 - DNA, 28 bp, synthetic construct
  source 1..28: mol_type = other DNA
cgtaccccaccctggcagaacacaaggg

SEQ ID NO: 36889 - DNA, 28 bp, synthetic construct
  source 1..28: mol_type = other DNA
ccgtaccccaccctggcagaacacaagg

SEQ ID NO: 36890 - DNA, 28 bp, synthetic construct
  source 1..28: mol_type = other DNA
cttgtgttctgccagggtggggtacggg

SEQ ID NO: 36891 - DNA, 28 bp, synthetic construct
  source 1..28: mol_type = other DNA
ttgtgttctgccagggtggggtacgggg

SEQ ID NO: 36892 - DNA, 28 bp, synthetic construct
  source 1..28: mol_type = other DNA
cagtgtcaaaccccgtaccccaccctgg

SEQ ID NO: 36893 - DNA, 28 bp, synthetic construct
  source 1..28: mol_type = other DNA
gggtggggtacggggtttgacactgagg

SEQ ID NO: 36894 - DNA, 28 bp, synthetic construct
  source 1..28: mol_type = other DNA
tggggtacggggtttgacactgaggagg

SEQ ID NO: 36895 - DNA, 28 bp, synthetic construct
  source 1..28: mol_type = other DNA
ggggtacggggtttgacactgaggaggg

SEQ ID NO: 36896 - DNA, 28 bp, synthetic construct
  source 1..28: mol_type = other DNA
tttgacactgaggagggtaacctgctgg

SEQ ID NO: 36897 - DNA, 28 bp, synthetic construct
  source 1..28: mol_type = other DNA
acactgaggagggtaacctgctggctgg

SEQ ID NO: 36898 - DNA, 28 bp, synthetic construct
  source 1..28: mol_type = other DNA
gaggagggtaacctgctggctggagcgg

SEQ ID NO: 36899 - DNA, 28 bp, synthetic construct
  source 1..28: mol_type = other DNA
cctgctggctggagcggcagagcagtgg

SEQ ID NO: 36900 - DNA, 28 bp, synthetic construct
  source 1..28: mol_type = other DNA
agagcagtggccttgatttgtcttttgg

SEQ ID NO: 36901 - DNA, 28 bp, synthetic construct
  source 1..28: mol_type = other DNA
ttaaaatcttccaaaagacaaatcaagg

SEQ ID NO: 36902 - DNA, 28 bp, synthetic construct
  source 1..28: mol_type = other DNA
taaaaaccaaaaagcataaacattctgg

SEQ ID NO: 36903 - DNA, 28 bp, synthetic construct
  source 1..28: mol_type = other DNA
gaaggaccagaatgtttatgctttttgg

SEQ ID NO: 36904 - DNA, 28 bp, synthetic construct
  source 1..28: mol_type = other DNA
atttcttcagagaaagcattgctgaagg

SEQ ID NO: 36905 - DNA, 28 bp, synthetic construct
  source 1..28: mol_type = other DNA
atgctttctctgaagaaatacttaacgg

SEQ ID NO: 36906 - DNA, 28 bp, synthetic construct
  source 1..28: mol_type = other DNA
tttctctgaagaaatacttaacggaagg

SEQ ID NO: 36907 - DNA, 28 bp, synthetic construct
  source 1..28: mol_type = other DNA
aatcaaactcagcagaatggtgaactgg

SEQ ID NO: 36908 - DNA, 28 bp, synthetic construct
  source 1..28: mol_type = other DNA
agttcaccattctgctgagtttgattgg

SEQ ID NO: 36909 - DNA, 28 bp, synthetic construct
  source 1..28: mol_type = other DNA
gttcaccattctgctgagtttgattggg

SEQ ID NO: 36910 - DNA, 28 bp, synthetic construct
  source 1..28: mol_type = other DNA
ttcaccattctgctgagtttgattgggg

SEQ ID NO: 36911 - DNA, 28 bp, synthetic construct
  source 1..28: mol_type = other DNA
cgtaccccaatcaaactcagcagaatgg

SEQ ID NO: 36912 - DNA, 28 bp, synthetic construct
  source 1..28: mol_type = other DNA
cattctgctgagtttgattggggtacgg

SEQ ID NO: 36913 - DNA, 28 bp, synthetic construct
  source 1..28: mol_type = other DNA
attctgctgagtttgattggggtacggg

SEQ ID NO: 36914 - DNA, 28 bp, synthetic construct
  source 1..28: mol_type = other DNA
ctgctgagtttgattggggtacgggtgg

SEQ ID NO: 36915 - DNA, 28 bp, synthetic construct
  source 1..28: mol_type = other DNA
agtttgattggggtacgggtggacgtgg

SEQ ID NO: 36916 - DNA, 28 bp, synthetic construct
  source 1..28: mol_type = other DNA
ccggagtgggggaagctgtgaggtcagg

SEQ ID NO: 36917 - DNA, 28 bp, synthetic construct
  source 1..28: mol_type = other DNA
ctgacctcacagcttcccccactccggg

SEQ ID NO: 36918 - DNA, 28 bp, synthetic construct
  source 1..28: mol_type = other DNA
atctcccggagtgggggaagctgtgagg

SEQ ID NO: 36919 - DNA, 28 bp, synthetic construct
  source 1..28: mol_type = other DNA
cttcccccactccgggagatcatcctgg

SEQ ID NO: 36920 - DNA, 28 bp, synthetic construct
  source 1..28: mol_type = other DNA
ttcccccactccgggagatcatcctggg

SEQ ID NO: 36921 - DNA, 28 bp, synthetic construct
  source 1..28: mol_type = other DNA
tcccccactccgggagatcatcctgggg

SEQ ID NO: 36922 - DNA, 28 bp, synthetic construct
  source 1..28: mol_type = other DNA
gccccaggatgatctcccggagtggggg

SEQ ID NO: 36923 - DNA, 28 bp, synthetic construct
  source 1..28: mol_type = other DNA
ggccccaggatgatctcccggagtgggg

SEQ ID NO: 36924 - DNA, 28 bp, synthetic construct
  source 1..28: mol_type = other DNA
gggccccaggatgatctcccggagtggg

SEQ ID NO: 36925 - DNA, 28 bp, synthetic construct
  source 1..28: mol_type = other DNA
tgggccccaggatgatctcccggagtgg

SEQ ID NO: 36926 - DNA, 28 bp, synthetic construct
  source 1..28: mol_type = other DNA
agaactgggccccaggatgatctcccgg

SEQ ID NO: 36927 - DNA, 28 bp, synthetic construct
  source 1..28: mol_type = other DNA
ctgagtataggcagaactgggccccagg

SEQ ID NO: 36928 - DNA, 28 bp, synthetic construct
  source 1..28: mol_type = other DNA
actgggtctgagtataggcagaactggg

SEQ ID NO: 36929 - DNA, 28 bp, synthetic construct
  source 1..28: mol_type = other DNA
aactgggtctgagtataggcagaactgg

SEQ ID NO: 36930 - DNA, 28 bp, synthetic construct
  source 1..28: mol_type = other DNA
aggttgtggaactgggtctgagtatagg

SEQ ID NO: 36931 - DNA, 28 bp, synthetic construct
  source 1..28: mol_type = other DNA
tactcagacccagttccacaacctgagg

SEQ ID NO: 36932 - DNA, 28 bp, synthetic construct
  source 1..28: mol_type = other DNA
aaggtattcctcaggttgtggaactggg

SEQ ID NO: 36933 - DNA, 28 bp, synthetic construct
  source 1..28: mol_type = other DNA
caaggtattcctcaggttgtggaactgg

SEQ ID NO: 36934 - DNA, 28 bp, synthetic construct
  source 1..28: mol_type = other DNA
cagttccacaacctgaggaataccttgg

SEQ ID NO: 36935 - DNA, 28 bp, synthetic construct
  source 1..28: mol_type = other DNA
tccacaacctgaggaataccttggatgg

SEQ ID NO: 36936 - DNA, 28 bp, synthetic construct
  source 1..28: mol_type = other DNA
gccatccaaggtattcctcaggttgtgg

SEQ ID NO: 36937 - DNA, 28 bp, synthetic construct
  source 1..28: mol_type = other DNA
acctgaggaataccttggatggctatgg

SEQ ID NO: 36938 - DNA, 28 bp, synthetic construct
  source 1..28: mol_type = other DNA
accatagccatccaaggtattcctcagg

SEQ ID NO: 36939 - DNA, 28 bp, synthetic construct
  source 1..28: mol_type = other DNA
ttggggtggataccatagccatccaagg

SEQ ID NO: 36940 - DNA, 28 bp, synthetic construct
  source 1..28: mol_type = other DNA
ggtatccaccccaagagcatagacctgg

SEQ ID NO: 36941 - DNA, 28 bp, synthetic construct
  source 1..28: mol_type = other DNA
attgtccaggtctatgctcttggggtgg

SEQ ID NO: 36942 - DNA, 28 bp, synthetic construct
  source 1..28: mol_type = other DNA
gtaattgtccaggtctatgctcttgggg

SEQ ID NO: 36943 - DNA, 28 bp, synthetic construct
  source 1..28: mol_type = other DNA
agtaattgtccaggtctatgctcttggg

SEQ ID NO: 36944 - DNA, 28 bp, synthetic construct
  source 1..28: mol_type = other DNA
aagtaattgtccaggtctatgctcttgg

SEQ ID NO: 36945 - DNA, 28 bp, synthetic construct
  source 1..28: mol_type = other DNA
agacctggacaattacttcactgcccgg

SEQ ID NO: 36946 - DNA, 28 bp, synthetic construct
  source 1..28: mol_type = other DNA
cctggacaattacttcactgcccggcgg

SEQ ID NO: 36947 - DNA, 28 bp, synthetic construct
  source 1..28: mol_type = other DNA
ttcactgcccggcggctcctcagtcagg

SEQ ID NO: 36948 - DNA, 28 bp, synthetic construct
  source 1..28: mol_type = other DNA
tgcccggcggctcctcagtcaggtgagg

SEQ ID NO: 36949 - DNA, 28 bp, synthetic construct
  source 1..28: mol_type = other DNA
gcccggcggctcctcagtcaggtgaggg

SEQ ID NO: 36950 - DNA, 28 bp, synthetic construct
  source 1..28: mol_type = other DNA
gccctcacctgactgaggagccgccggg

SEQ ID NO: 36951 - DNA, 28 bp, synthetic construct
  source 1..28: mol_type = other DNA
ggccctcacctgactgaggagccgccgg

SEQ ID NO: 36952 - DNA, 28 bp, synthetic construct
  source 1..28: mol_type = other DNA
cggctcctcagtcaggtgagggccctgg

SEQ ID NO: 36953 - DNA, 28 bp, synthetic construct
  source 1..28: mol_type = other DNA
cctgtccagggccctcacctgactgagg

SEQ ID NO: 36954 - DNA, 28 bp, synthetic construct
  source 1..28: mol_type = other DNA
caggtgagggccctggacaggttccagg

SEQ ID NO: 36955 - DNA, 28 bp, synthetic construct
  source 1..28: mol_type = other DNA
gtggttggcacctggaacctgtccaggg

SEQ ID NO: 36956 - DNA, 28 bp, synthetic construct
  source 1..28: mol_type = other DNA
agtggttggcacctggaacctgtccagg

SEQ ID NO: 36957 - DNA, 28 bp, synthetic construct
  source 1..28: mol_type = other DNA
gacaggttccaggtgccaaccactgagg

SEQ ID NO: 36958 - DNA, 28 bp, synthetic construct
  source 1..28: mol_type = other DNA
ggcatttacctcagtggttggcacctgg

SEQ ID NO: 36959 - DNA, 28 bp, synthetic construct
  source 1..28: mol_type = other DNA
ggtgccaaccactgaggtaaatgcctgg

SEQ ID NO: 36960 - DNA, 28 bp, synthetic construct
  source 1..28: mol_type = other DNA
ccaaccactgaggtaaatgcctggctgg

SEQ ID NO: 36961 - DNA, 28 bp, synthetic construct
  source 1..28: mol_type = other DNA
tgaaccagccaggcatttacctcagtgg

SEQ ID NO: 36962 - DNA, 28 bp, synthetic construct
  source 1..28: mol_type = other DNA
gcctggctggttcaccgagacccagagg

SEQ ID NO: 36963 - DNA, 28 bp, synthetic construct
  source 1..28: mol_type = other DNA
cctggctggttcaccgagacccagaggg

SEQ ID NO: 36964 - DNA, 28 bp, synthetic construct
  source 1..28: mol_type = other DNA
ctggctggttcaccgagacccagagggg

SEQ ID NO: 36965 - DNA, 28 bp, synthetic construct
  source 1..28: mol_type = other DNA
accgagacccagaggggtctgtctctgg

SEQ ID NO: 36966 - DNA, 28 bp, synthetic construct
  source 1..28: mol_type = other DNA
gccagagacagacccctctgggtctcgg

SEQ ID NO: 36967 - DNA, 28 bp, synthetic construct
  source 1..28: mol_type = other DNA
ctgactgccagagacagacccctctggg

SEQ ID NO: 36968 - DNA, 28 bp, synthetic construct
  source 1..28: mol_type = other DNA
gctgactgccagagacagacccctctgg

SEQ ID NO: 36969 - DNA, 28 bp, synthetic construct
  source 1..28: mol_type = other DNA
ctgtctctggcagtcagcccaactcagg

SEQ ID NO: 36970 - DNA, 28 bp, synthetic construct
  source 1..28: mol_type = other DNA
aactctcgagggcgaggcctgagttggg

SEQ ID NO: 36971 - DNA, 28 bp, synthetic construct
  source 1..28: mol_type = other DNA
gaactctcgagggcgaggcctgagttgg

SEQ ID NO: 36972 - DNA, 28 bp, synthetic construct
  source 1..28: mol_type = other DNA
caggcctcgccctcgagagttccagtgg

SEQ ID NO: 36973 - DNA, 28 bp, synthetic construct
  source 1..28: mol_type = other DNA
gaggccactggaactctcgagggcgagg

SEQ ID NO: 36974 - DNA, 28 bp, synthetic construct
  source 1..28: mol_type = other DNA
tcttggaggccactggaactctcgaggg

SEQ ID NO: 36975 - DNA, 28 bp, synthetic construct
  source 1..28: mol_type = other DNA
atcttggaggccactggaactctcgagg

SEQ ID NO: 36976 - DNA, 28 bp, synthetic construct
  source 1..28: mol_type = other DNA
gttccagtggcctccaagatgtgacagg

SEQ ID NO: 36977 - DNA, 28 bp, synthetic construct
  source 1..28: mol_type = other DNA
gggcctgtcacatcttggaggccactgg

SEQ ID NO: 36978 - DNA, 28 bp, synthetic construct
  source 1..28: mol_type = other DNA
gttgtctgggcctgtcacatcttggagg

SEQ ID NO: 36979 - DNA, 28 bp, synthetic construct
  source 1..28: mol_type = other DNA
tccaagatgtgacaggcccagacaacgg

SEQ ID NO: 36980 - DNA, 28 bp, synthetic construct
  source 1..28: mol_type = other DNA
cccgttgtctgggcctgtcacatcttgg

SEQ ID NO: 36981 - DNA, 28 bp, synthetic construct
  source 1..28: mol_type = other DNA
caagatgtgacaggcccagacaacgggg

SEQ ID NO: 36982 - DNA, 28 bp, synthetic construct
  source 1..28: mol_type = other DNA
ttcgctttctcgcaccccgttgtctggg

SEQ ID NO: 36983 - DNA, 28 bp, synthetic construct
  source 1..28: mol_type = other DNA
tttcgctttctcgcaccccgttgtctgg

SEQ ID NO: 36984 - DNA, 28 bp, synthetic construct
  source 1..28: mol_type = other DNA
gacaacggggtgcgagaaagcgaaacgg

SEQ ID NO: 36985 - DNA, 28 bp, synthetic construct
  source 1..28: mol_type = other DNA
ggggtgcgagaaagcgaaacggagcagg

SEQ ID NO: 36986 - DNA, 28 bp, synthetic construct
  source 1..28: mol_type = other DNA
gggtgcgagaaagcgaaacggagcaggg

SEQ ID NO: 36987 - DNA, 28 bp, synthetic construct
  source 1..28: mol_type = other DNA
gagaaagcgaaacggagcagggattcgg

SEQ ID NO: 36988 - DNA, 28 bp, synthetic construct
  source 1..28: mol_type = other DNA
acggagcagggattcggtgaagatttgg

SEQ ID NO: 36989 - DNA, 28 bp, synthetic construct
  source 1..28: mol_type = other DNA
gagcagggattcggtgaagatttggagg

SEQ ID NO: 36990 - DNA, 28 bp, synthetic construct
  source 1..28: mol_type = other DNA
ggattcggtgaagatttggaggatttgg

SEQ ID NO: 36991 - DNA, 28 bp, synthetic construct
  source 1..28: mol_type = other DNA
gattcggtgaagatttggaggatttggg

SEQ ID NO: 36992 - DNA, 28 bp, synthetic construct
  source 1..28: mol_type = other DNA
attcggtgaagatttggaggatttgggg

SEQ ID NO: 36993 - DNA, 28 bp, synthetic construct
  source 1..28: mol_type = other DNA
ttcggtgaagatttggaggatttggggg

SEQ ID NO: 36994 - DNA, 28 bp, synthetic construct
  source 1..28: mol_type = other DNA
tgggggctgtagcccccccagtcagtgg

SEQ ID NO: 36995 - DNA, 28 bp, synthetic construct
  source 1..28: mol_type = other DNA
ttggttaagtctccactgactggggggg

SEQ ID NO: 36996 - DNA, 28 bp, synthetic construct
  source 1..28: mol_type = other DNA
tttggttaagtctccactgactgggggg

SEQ ID NO: 36997 - DNA, 28 bp, synthetic construct
  source 1..28: mol_type = other DNA
ctttggttaagtctccactgactggggg

SEQ ID NO: 36998 - DNA, 28 bp, synthetic construct
  source 1..28: mol_type = other DNA
tctttggttaagtctccactgactgggg

SEQ ID NO: 36999 - DNA, 28 bp, synthetic construct
  source 1..28: mol_type = other DNA
ctctttggttaagtctccactgactggg

SEQ ID NO: 37000 - DNA, 28 bp, synthetic construct
  source 1..28: mol_type = other DNA
cctctttggttaagtctccactgactgg

SEQ ID NO: 37001 - DNA, 28 bp, synthetic construct
  source 1..28: mol_type = other DNA
gtggagacttaaccaaagaggttagtgg

SEQ ID NO: 37002 - DNA, 28 bp, synthetic construct
  source 1..28: mol_type = other DNA
ttaaccaaagaggttagtggacctgtgg

SEQ ID NO: 37003 - DNA, 28 bp, synthetic construct
  source 1..28: mol_type = other DNA
accaaagaggttagtggacctgtggtgg

SEQ ID NO: 37004 - DNA, 28 bp, synthetic construct
  source 1..28: mol_type = other DNA
cccaccacaggtccactaacctctttgg

SEQ ID NO: 37005 - DNA, 28 bp, synthetic construct
  source 1..28: mol_type = other DNA
ggttagtggacctgtggtgggtgtgtgg

SEQ ID NO: 37006 - DNA, 28 bp, synthetic construct
  source 1..28: mol_type = other DNA
gttagtggacctgtggtgggtgtgtggg

SEQ ID NO: 37007 - DNA, 28 bp, synthetic construct
  source 1..28: mol_type = other DNA
ttagtggacctgtggtgggtgtgtgggg

SEQ ID NO: 37008 - DNA, 28 bp, synthetic construct
  source 1..28: mol_type = other DNA
ggacctgtggtgggtgtgtggggcctgg

SEQ ID NO: 37009 - DNA, 28 bp, synthetic construct
  source 1..28: mol_type = other DNA
gacctgtggtgggtgtgtggggcctggg

SEQ ID NO: 37010 - DNA, 28 bp, synthetic construct
  source 1..28: mol_type = other DNA
acctgtggtgggtgtgtggggcctgggg

SEQ ID NO: 37011 - DNA, 28 bp, synthetic construct
  source 1..28: mol_type = other DNA
gccccaggccccacacacccaccacagg

SEQ ID NO: 37012 - DNA, 28 bp, synthetic construct
  source 1..28: mol_type = other DNA
tggtgggtgtgtggggcctggggcttgg

SEQ ID NO: 37013 - DNA, 28 bp, synthetic construct
  source 1..28: mol_type = other DNA
ggtgggtgtgtggggcctggggcttggg

SEQ ID NO: 37014 - DNA, 28 bp, synthetic construct
  source 1..28: mol_type = other DNA
gtgggtgtgtggggcctggggcttgggg

SEQ ID NO: 37015 - DNA, 28 bp, synthetic construct
  source 1..28: mol_type = other DNA
tgggtgtgtggggcctggggcttggggg

SEQ ID NO: 37016 - DNA, 28 bp, synthetic construct
  source 1..28: mol_type = other DNA
gtgtgtggggcctggggcttgggggtgg

SEQ ID NO: 37017 - DNA, 28 bp, synthetic construct
  source 1..28: mol_type = other DNA
tgtgtggggcctggggcttgggggtggg

SEQ ID NO: 37018 - DNA, 28 bp, synthetic construct
  source 1..28: mol_type = other DNA
tggggcctggggcttgggggtgggctgg

SEQ ID NO: 37019 - DNA, 28 bp, synthetic construct
  source 1..28: mol_type = other DNA
tgggaccagcccacccccaagccccagg

SEQ ID NO: 37020 - DNA, 28 bp, synthetic construct
  source 1..28: mol_type = other DNA
gggcttgggggtgggctggtcccaaagg

SEQ ID NO: 37021 - DNA, 28 bp, synthetic construct
  source 1..28: mol_type = other DNA
ggggtgggctggtcccaaaggattgtgg

SEQ ID NO: 37022 - DNA, 28 bp, synthetic construct
  source 1..28: mol_type = other DNA
ctcagtgttctgaccacaatcctttggg

SEQ ID NO: 37023 - DNA, 28 bp, synthetic construct
  source 1..28: mol_type = other DNA
gctcagtgttctgaccacaatcctttgg

SEQ ID NO: 37024 - DNA, 28 bp, synthetic construct
  source 1..28: mol_type = other DNA
cactgagccctgtaaagagccagacagg

SEQ ID NO: 37025 - DNA, 28 bp, synthetic construct
  source 1..28: mol_type = other DNA
gctgaaacctgtctggctctttacaggg

SEQ ID NO: 37026 - DNA, 28 bp, synthetic construct
  source 1..28: mol_type = other DNA
tgctgaaacctgtctggctctttacagg

SEQ ID NO: 37027 - DNA, 28 bp, synthetic construct
  source 1..28: mol_type = other DNA
tgtaaagagccagacaggtttcagcagg

SEQ ID NO: 37028 - DNA, 28 bp, synthetic construct
  source 1..28: mol_type = other DNA
gtaaagagccagacaggtttcagcaggg

SEQ ID NO: 37029 - DNA, 28 bp, synthetic construct
  source 1..28: mol_type = other DNA
gccagacaggtttcagcagggcctcagg

SEQ ID NO: 37030 - DNA, 28 bp, synthetic construct
  source 1..28: mol_type = other DNA
gcctgaggccctgctgaaacctgtctgg

SEQ ID NO: 37031 - DNA, 28 bp, synthetic construct
  source 1..28: mol_type = other DNA
tgaagagctgggaggggccccacccagg

SEQ ID NO: 37032 - DNA, 28 bp, synthetic construct
  source 1..28: mol_type = other DNA
gggaggggccccacccaggactaactgg

SEQ ID NO: 37033 - DNA, 28 bp, synthetic construct
  source 1..28: mol_type = other DNA
ggaggggccccacccaggactaactggg

SEQ ID NO: 37034 - DNA, 28 bp, synthetic construct
  source 1..28: mol_type = other DNA
gaggggccccacccaggactaactgggg

SEQ ID NO: 37035 - DNA, 28 bp, synthetic construct
  source 1..28: mol_type = other DNA
gtgtcaccccagttagtcctgggtgggg

SEQ ID NO: 37036 - DNA, 28 bp, synthetic construct
  source 1..28: mol_type = other DNA
agtgtcaccccagttagtcctgggtggg

SEQ ID NO: 37037 - DNA, 28 bp, synthetic construct
  source 1..28: mol_type = other DNA
tagtgtcaccccagttagtcctgggtgg

SEQ ID NO: 37038 - DNA, 28 bp, synthetic construct
  source 1..28: mol_type = other DNA
acccaggactaactggggtgacactagg

SEQ ID NO: 37039 - DNA, 28 bp, synthetic construct
  source 1..28: mol_type = other DNA
tcctagtgtcaccccagttagtcctggg

SEQ ID NO: 37040 - DNA, 28 bp, synthetic construct
  source 1..28: mol_type = other DNA
ctcctagtgtcaccccagttagtcctgg

SEQ ID NO: 37041 - DNA, 28 bp, synthetic construct
  source 1..28: mol_type = other DNA
caggactaactggggtgacactaggagg

SEQ ID NO: 37042 - DNA, 28 bp, synthetic construct
  source 1..28: mol_type = other DNA
aggactaactggggtgacactaggaggg

SEQ ID NO: 37043 - DNA, 28 bp, synthetic construct
  source 1..28: mol_type = other DNA
ggggtgacactaggagggaactctgagg

SEQ ID NO: 37044 - DNA, 28 bp, synthetic construct
  source 1..28: mol_type = other DNA
gggtgacactaggagggaactctgaggg

SEQ ID NO: 37045 - DNA, 28 bp, synthetic construct
  source 1..28: mol_type = other DNA
ggtgacactaggagggaactctgagggg

SEQ ID NO: 37046 - DNA, 28 bp, synthetic construct
  source 1..28: mol_type = other DNA
acactaggagggaactctgaggggcagg

SEQ ID NO: 37047 - DNA, 28 bp, synthetic construct
  source 1..28: mol_type = other DNA
ggagggaactctgaggggcaggacaagg

SEQ ID NO: 37048 - DNA, 28 bp, synthetic construct
  source 1..28: mol_type = other DNA
ggaactctgaggggcaggacaaggaagg

SEQ ID NO: 37049 - DNA, 28 bp, synthetic construct
  source 1..28: mol_type = other DNA
gaactctgaggggcaggacaaggaaggg

SEQ ID NO: 37050 - DNA, 28 bp, synthetic construct
  source 1..28: mol_type = other DNA
gaggggcaggacaaggaagggaccttgg

SEQ ID NO: 37051 - DNA, 28 bp, synthetic construct
  source 1..28: mol_type = other DNA
aggggcaggacaaggaagggaccttggg

SEQ ID NO: 37052 - DNA, 28 bp, synthetic construct
  source 1..28: mol_type = other DNA
acatgactttagctctaagatcccaagg

SEQ ID NO: 37053 - DNA, 28 bp, synthetic construct
  source 1..28: mol_type = other DNA
gctaaagtcatgtgatctgtctttcagg

SEQ ID NO: 37054 - DNA, 28 bp, synthetic construct
  source 1..28: mol_type = other DNA
ggacatagatctgattgacatcctttgg

SEQ ID NO: 37055 - DNA, 28 bp, synthetic construct
  source 1..28: mol_type = other DNA
gatctgattgacatcctttggcgacagg

SEQ ID NO: 37056 - DNA, 28 bp, synthetic construct
  source 1..28: mol_type = other DNA
atcctttggcgacaggatattgatctgg

SEQ ID NO: 37057 - DNA, 28 bp, synthetic construct
  source 1..28: mol_type = other DNA
tcctttggcgacaggatattgatctggg

SEQ ID NO: 37058 - DNA, 28 bp, synthetic construct
  source 1..28: mol_type = other DNA
ccccagatcaatatcctgtcgccaaagg

SEQ ID NO: 37059 - DNA, 28 bp, synthetic construct
  source 1..28: mol_type = other DNA
ctttggcgacaggatattgatctggggg

SEQ ID NO: 37060 - DNA, 28 bp, synthetic construct
  source 1..28: mol_type = other DNA
ggcgacaggatattgatctgggggctgg

SEQ ID NO: 37061 - DNA, 28 bp, synthetic construct
  source 1..28: mol_type = other DNA
gcgacaggatattgatctgggggctggg

SEQ ID NO: 37062 - DNA, 28 bp, synthetic construct
  source 1..28: mol_type = other DNA
gatattgatctgggggctgggcgtgagg

SEQ ID NO: 37063 - DNA, 28 bp, synthetic construct
  source 1..28: mol_type = other DNA
gtttttgactatagtcaccgccagaagg

SEQ ID NO: 37064 - DNA, 28 bp, synthetic construct
  source 1..28: mol_type = other DNA
gactatagtcaccgccagaaggagcagg

SEQ ID NO: 37065 - DNA, 28 bp, synthetic construct
  source 1..28: mol_type = other DNA
agtcaccgccagaaggagcaggatgtgg

SEQ ID NO: 37066 - DNA, 28 bp, synthetic construct
  source 1..28: mol_type = other DNA
cttctccacatcctgctccttctggcgg

SEQ ID NO: 37067 - DNA, 28 bp, synthetic construct
  source 1..28: mol_type = other DNA
cgccagaaggagcaggatgtggagaagg

SEQ ID NO: 37068 - DNA, 28 bp, synthetic construct
  source 1..28: mol_type = other DNA
ctccttctccacatcctgctccttctgg

SEQ ID NO: 37069 - DNA, 28 bp, synthetic construct
  source 1..28: mol_type = other DNA
aggatgtggagaaggagctgcgagatgg

SEQ ID NO: 37070 - DNA, 28 bp, synthetic construct
  source 1..28: mol_type = other DNA
atgtggagaaggagctgcgagatggagg

SEQ ID NO: 37071 - DNA, 28 bp, synthetic construct
  source 1..28: mol_type = other DNA
aaggagctgcgagatggaggcgagcagg

SEQ ID NO: 37072 - DNA, 28 bp, synthetic construct
  source 1..28: mol_type = other DNA
gcgagatggaggcgagcaggacacctgg

SEQ ID NO: 37073 - DNA, 28 bp, synthetic construct
  source 1..28: mol_type = other DNA
cgagatggaggcgagcaggacacctggg

SEQ ID NO: 37074 - DNA, 28 bp, synthetic construct
  source 1..28: mol_type = other DNA
atggaggcgagcaggacacctgggcagg

SEQ ID NO: 37075 - DNA, 28 bp, synthetic construct
  source 1..28: mol_type = other DNA
ggcgagcaggacacctgggcaggcgagg

SEQ ID NO: 37076 - DNA, 28 bp, synthetic construct
  source 1..28: mol_type = other DNA
gcgagcaggacacctgggcaggcgaggg

SEQ ID NO: 37077 - DNA, 28 bp, synthetic construct
  source 1..28: mol_type = other DNA
caggacacctgggcaggcgagggcgcgg

SEQ ID NO: 37078 - DNA, 28 bp, synthetic construct
  source 1..28: mol_type = other DNA
agagcttccgcgccctcgcctgcccagg

SEQ ID NO: 37079 - DNA, 28 bp, synthetic construct
  source 1..28: mol_type = other DNA
tgggcaggcgagggcgcggaagctctgg

SEQ ID NO: 37080 - DNA, 28 bp, synthetic construct
  source 1..28: mol_type = other DNA
aggcgagggcgcggaagctctggcacgg

SEQ ID NO: 37081 - DNA, 28 bp, synthetic construct
  source 1..28: mol_type = other DNA
gaagctctggcacggaacctgctagtgg

SEQ ID NO: 37082 - DNA, 28 bp, synthetic construct
  source 1..28: mol_type = other DNA
ctctggcacggaacctgctagtggatgg

SEQ ID NO: 37083 - DNA, 28 bp, synthetic construct
  source 1..28: mol_type = other DNA
ggaacctgctagtggatggagagactgg

SEQ ID NO: 37084 - DNA, 28 bp, synthetic construct
  source 1..28: mol_type = other DNA
gaacctgctagtggatggagagactggg

SEQ ID NO: 37085 - DNA, 28 bp, synthetic construct
  source 1..28: mol_type = other DNA
aacctgctagtggatggagagactgggg

SEQ ID NO: 37086 - DNA, 28 bp, synthetic construct
  source 1..28: mol_type = other DNA
ctccccagtctctccatccactagcagg

SEQ ID NO: 37087 - DNA, 28 bp, synthetic construct
  source 1..28: mol_type = other DNA
gagactggggagagcttccctgcacagg

SEQ ID NO: 37088 - DNA, 28 bp, synthetic construct
  source 1..28: mol_type = other DNA
gagcaggggcgatggtacctgtgcaggg

SEQ ID NO: 37089 - DNA, 28 bp, synthetic construct
  source 1..28: mol_type = other DNA
tgagcaggggcgatggtacctgtgcagg

SEQ ID NO: 37090 - DNA, 28 bp, synthetic construct
  source 1..28: mol_type = other DNA
cacaggtaccatcgcccctgctcactgg

SEQ ID NO: 37091 - DNA, 28 bp, synthetic construct
  source 1..28: mol_type = other DNA
acaggtaccatcgcccctgctcactggg

SEQ ID NO: 37092 - DNA, 28 bp, synthetic construct
  source 1..28: mol_type = other DNA
aagagagcccagtgagcaggggcgatgg

SEQ ID NO: 37093 - DNA, 28 bp, synthetic construct
  source 1..28: mol_type = other DNA
gacaagaagagagcccagtgagcagggg

SEQ ID NO: 37094 - DNA, 28 bp, synthetic construct
  source 1..28: mol_type = other DNA
ggacaagaagagagcccagtgagcaggg

SEQ ID NO: 37095 - DNA, 28 bp, synthetic construct
  source 1..28: mol_type = other DNA
gggacaagaagagagcccagtgagcagg

SEQ ID NO: 37096 - DNA, 28 bp, synthetic construct
  source 1..28: mol_type = other DNA
tgtccctactaccctgacacaaaccagg

SEQ ID NO: 37097 - DNA, 28 bp, synthetic construct
  source 1..28: mol_type = other DNA
cagcctggtttgtgtcagggtagtaggg

SEQ ID NO: 37098 - DNA, 28 bp, synthetic construct
  source 1..28: mol_type = other DNA
ccagcctggtttgtgtcagggtagtagg

SEQ ID NO: 37099 - DNA, 28 bp, synthetic construct
  source 1..28: mol_type = other DNA
aagaactccagcctggtttgtgtcaggg

SEQ ID NO: 37100 - DNA, 28 bp, synthetic construct
  source 1..28: mol_type = other DNA
gaagaactccagcctggtttgtgtcagg

SEQ ID NO: 37101 - DNA, 28 bp, synthetic construct
  source 1..28: mol_type = other DNA
ggaagtttctggaagaactccagcctgg

SEQ ID NO: 37102 - DNA, 28 bp, synthetic construct
  source 1..28: mol_type = other DNA
tccagaaacttcctttagagaagacagg

SEQ ID NO: 37103 - DNA, 28 bp, synthetic construct
  source 1..28: mol_type = other DNA
acctgtcttctctaaaggaagtttctgg

SEQ ID NO: 37104 - DNA, 28 bp, synthetic construct
  source 1..28: mol_type = other DNA
agaaacttcctttagagaagacaggtgg

SEQ ID NO: 37105 - DNA, 28 bp, synthetic construct
  source 1..28: mol_type = other DNA
tcctttagagaagacaggtggtgtgtgg

SEQ ID NO: 37106 - DNA, 28 bp, synthetic construct
  source 1..28: mol_type = other DNA
cccacacaccacctgtcttctctaaagg

SEQ ID NO: 37107 - DNA, 28 bp, synthetic construct
  source 1..28: mol_type = other DNA
ctttagagaagacaggtggtgtgtgggg

SEQ ID NO: 37108 - DNA, 28 bp, synthetic construct
  source 1..28: mol_type = other DNA
tagagaagacaggtggtgtgtggggtgg

SEQ ID NO: 37109 - DNA, 28 bp, synthetic construct
  source 1..28: mol_type = other DNA
tcggggccagccattagcctgggaatgg

SEQ ID NO: 37110 - DNA, 28 bp, synthetic construct
  source 1..28: mol_type = other DNA
cggggccagccattagcctgggaatggg

SEQ ID NO: 37111 - DNA, 28 bp, synthetic construct
  source 1..28: mol_type = other DNA
ggccagccattagcctgggaatgggagg

SEQ ID NO: 37112 - DNA, 28 bp, synthetic construct
  source 1..28: mol_type = other DNA
gccagccattagcctgggaatgggaggg

SEQ ID NO: 37113 - DNA, 28 bp, synthetic construct
  source 1..28: mol_type = other DNA
tccctcccattcccaggctaatggctgg

SEQ ID NO: 37114 - DNA, 28 bp, synthetic construct
  source 1..28: mol_type = other DNA
agtctccctcccattcccaggctaatgg

SEQ ID NO: 37115 - DNA, 28 bp, synthetic construct
  source 1..28: mol_type = other DNA
agcctgggaatgggagggagactgcagg

SEQ ID NO: 37116 - DNA, 28 bp, synthetic construct
  source 1..28: mol_type = other DNA
gcctgggaatgggagggagactgcaggg

SEQ ID NO: 37117 - DNA, 28 bp, synthetic construct
  source 1..28: mol_type = other DNA
gccctgcagtctccctcccattcccagg

SEQ ID NO: 37118 - DNA, 28 bp, synthetic construct
  source 1..28: mol_type = other DNA
ggagactgcagggcttcagccattctgg

SEQ ID NO: 37119 - DNA, 28 bp, synthetic construct
  source 1..28: mol_type = other DNA
gagactgcagggcttcagccattctggg

SEQ ID NO: 37120 - DNA, 28 bp, synthetic construct
  source 1..28: mol_type = other DNA
tggggctgaagcttctttcccagaatgg

SEQ ID NO: 37121 - DNA, 28 bp, synthetic construct
  source 1..28: mol_type = other DNA
attctgggaaagaagcttcagccccagg

SEQ ID NO: 37122 - DNA, 28 bp, synthetic construct
  source 1..28: mol_type = other DNA
aagaagcttcagccccaggcagccaagg

SEQ ID NO: 37123 - DNA, 28 bp, synthetic construct
  source 1..28: mol_type = other DNA
cttcagccccaggcagccaaggcccagg

SEQ ID NO: 37124 - DNA, 28 bp, synthetic construct
  source 1..28: mol_type = other DNA
gattgacctgggccttggctgcctgggg

SEQ ID NO: 37125 - DNA, 28 bp, synthetic construct
  source 1..28: mol_type = other DNA
tgattgacctgggccttggctgcctggg

SEQ ID NO: 37126 - DNA, 28 bp, synthetic construct
  source 1..28: mol_type = other DNA
ctgattgacctgggccttggctgcctgg

SEQ ID NO: 37127 - DNA, 28 bp, synthetic construct
  source 1..28: mol_type = other DNA
ctgtaagtctgattgacctgggccttgg

SEQ ID NO: 37128 - DNA, 28 bp, synthetic construct
  source 1..28: mol_type = other DNA
caggaactgtaagtctgattgacctggg

SEQ ID NO: 37129 - DNA, 28 bp, synthetic construct
  source 1..28: mol_type = other DNA
acaggaactgtaagtctgattgacctgg

SEQ ID NO: 37130 - DNA, 28 bp, synthetic construct
  source 1..28: mol_type = other DNA
tcagacttacagttcctgttgccacagg

SEQ ID NO: 37131 - DNA, 28 bp, synthetic construct
  source 1..28: mol_type = other DNA
agttcctgttgccacaggtgcctagtgg

SEQ ID NO: 37132 - DNA, 28 bp, synthetic construct
  source 1..28: mol_type = other DNA
gttcctgttgccacaggtgcctagtggg

SEQ ID NO: 37133 - DNA, 28 bp, synthetic construct
  source 1..28: mol_type = other DNA
ttcctgttgccacaggtgcctagtgggg

SEQ ID NO: 37134 - DNA, 28 bp, synthetic construct
  source 1..28: mol_type = other DNA
ctccccactaggcacctgtggcaacagg

SEQ ID NO: 37135 - DNA, 28 bp, synthetic construct
  source 1..28: mol_type = other DNA
ctgttgccacaggtgcctagtggggagg

SEQ ID NO: 37136 - DNA, 28 bp, synthetic construct
  source 1..28: mol_type = other DNA
tctggtcctccccactaggcacctgtgg

SEQ ID NO: 37137 - DNA, 28 bp, synthetic construct
  source 1..28: mol_type = other DNA
caggtgcctagtggggaggaccagacgg

SEQ ID NO: 37138 - DNA, 28 bp, synthetic construct
  source 1..28: mol_type = other DNA
acagggccgtctggtcctccccactagg

SEQ ID NO: 37139 - DNA, 28 bp, synthetic construct
  source 1..28: mol_type = other DNA
ggggaggaccagacggccctgtccctgg

SEQ ID NO: 37140 - DNA, 28 bp, synthetic construct
  source 1..28: mol_type = other DNA
gcactcttccagggacagggccgtctgg

SEQ ID NO: 37141 - DNA, 28 bp, synthetic construct
  source 1..28: mol_type = other DNA
ggccctgtccctggaagagtgccttagg

SEQ ID NO: 37142 - DNA, 28 bp, synthetic construct
  source 1..28: mol_type = other DNA
agcctaaggcactcttccagggacaggg

SEQ ID NO: 37143 - DNA, 28 bp, synthetic construct
  source 1..28: mol_type = other DNA
cagcctaaggcactcttccagggacagg

SEQ ID NO: 37144 - DNA, 28 bp, synthetic construct
  source 1..28: mol_type = other DNA
tccctggaagagtgccttaggctgctgg

SEQ ID NO: 37145 - DNA, 28 bp, synthetic construct
  source 1..28: mol_type = other DNA
tccagcagcctaaggcactcttccaggg

SEQ ID NO: 37146 - DNA, 28 bp, synthetic construct
  source 1..28: mol_type = other DNA
ttccagcagcctaaggcactcttccagg

SEQ ID NO: 37147 - DNA, 28 bp, synthetic construct
  source 1..28: mol_type = other DNA
ggggcaggtggcttccagcagcctaagg

SEQ ID NO: 37148 - DNA, 28 bp, synthetic construct
  source 1..28: mol_type = other DNA
ggctgctggaagccacctgcccctttgg

SEQ ID NO: 37149 - DNA, 28 bp, synthetic construct
  source 1..28: mol_type = other DNA
gctgctggaagccacctgcccctttggg

SEQ ID NO: 37150 - DNA, 28 bp, synthetic construct
  source 1..28: mol_type = other DNA
ctgctggaagccacctgcccctttgggg

SEQ ID NO: 37151 - DNA, 28 bp, synthetic construct
  source 1..28: mol_type = other DNA
tcagcattctccccaaaggggcaggtgg

SEQ ID NO: 37152 - DNA, 28 bp, synthetic construct
  source 1..28: mol_type = other DNA
acctgcccctttggggagaatgctgagg

SEQ ID NO: 37153 - DNA, 28 bp, synthetic construct
  source 1..28: mol_type = other DNA
acctcagcattctccccaaaggggcagg

SEQ ID NO: 37154 - DNA, 28 bp, synthetic construct
  source 1..28: mol_type = other DNA
gctcacctcagcattctccccaaagggg

SEQ ID NO: 37155 - DNA, 28 bp, synthetic construct
  source 1..28: mol_type = other DNA
tgctcacctcagcattctccccaaaggg

SEQ ID NO: 37156 - DNA, 28 bp, synthetic construct
  source 1..28: mol_type = other DNA
ctgctcacctcagcattctccccaaagg

SEQ ID NO: 37157 - DNA, 28 bp, synthetic construct
  source 1..28: mol_type = other DNA
ctttggggagaatgctgaggtgagcagg

SEQ ID NO: 37158 - DNA, 28 bp, synthetic construct
  source 1..28: mol_type = other DNA
tccagtgagagtccaccaagtgagcagg

SEQ ID NO: 37159 - DNA, 28 bp, synthetic construct
  source 1..28: mol_type = other DNA
ccctgctcacttggtggactctcactgg

SEQ ID NO: 37160 - DNA, 28 bp, synthetic construct
  source 1..28: mol_type = other DNA
ggtacaggctgccctgctcacttggtgg

SEQ ID NO: 37161 - DNA, 28 bp, synthetic construct
  source 1..28: mol_type = other DNA
ccaggtacaggctgccctgctcacttgg

SEQ ID NO: 37162 - DNA, 28 bp, synthetic construct
  source 1..28: mol_type = other DNA
agcctgtacctggtgtgtccctccatgg

SEQ ID NO: 37163 - DNA, 28 bp, synthetic construct
  source 1..28: mol_type = other DNA
agccatggagggacacaccaggtacagg

SEQ ID NO: 37164 - DNA, 28 bp, synthetic construct
  source 1..28: mol_type = other DNA
tacctggtgtgtccctccatggctgagg

SEQ ID NO: 37165 - DNA, 28 bp, synthetic construct
  source 1..28: mol_type = other DNA
acctggtgtgtccctccatggctgaggg

SEQ ID NO: 37166 - DNA, 28 bp, synthetic construct
  source 1..28: mol_type = other DNA
cccctcagccatggagggacacaccagg

SEQ ID NO: 37167 - DNA, 28 bp, synthetic construct
  source 1..28: mol_type = other DNA
caacagctggcccctcagccatggaggg

SEQ ID NO: 37168 - DNA, 28 bp, synthetic construct
  source 1..28: mol_type = other DNA
cctccatggctgaggggccagctgttgg

SEQ ID NO: 37169 - DNA, 28 bp, synthetic construct
  source 1..28: mol_type = other DNA
gaaccaacagctggcccctcagccatgg

SEQ ID NO: 37170 - DNA, 28 bp, synthetic construct
  source 1..28: mol_type = other DNA
tggctgaggggccagctgttggttctgg

SEQ ID NO: 37171 - DNA, 28 bp, synthetic construct
  source 1..28: mol_type = other DNA
ccagctgttggttctggccttattctgg

SEQ ID NO: 37172 - DNA, 28 bp, synthetic construct
  source 1..28: mol_type = other DNA
ttggttctggccttattctggctgctgg

SEQ ID NO: 37173 - DNA, 28 bp, synthetic construct
  source 1..28: mol_type = other DNA
tggttctggccttattctggctgctggg

SEQ ID NO: 37174 - DNA, 28 bp, synthetic construct
  source 1..28: mol_type = other DNA
ggttctggccttattctggctgctgggg

SEQ ID NO: 37175 - DNA, 28 bp, synthetic construct
  source 1..28: mol_type = other DNA
gttctggccttattctggctgctggggg

SEQ ID NO: 37176 - DNA, 28 bp, synthetic construct
  source 1..28: mol_type = other DNA
gcatttacccccagcagccagaataagg

SEQ ID NO: 37177 - DNA, 28 bp, synthetic construct
  source 1..28: mol_type = other DNA
ttctggctgctgggggtaaatgcagagg

SEQ ID NO: 37178 - DNA, 28 bp, synthetic construct
  source 1..28: mol_type = other DNA
ggctgctgggggtaaatgcagaggaagg

SEQ ID NO: 37179 - DNA, 28 bp, synthetic construct
  source 1..28: mol_type = other DNA
atgcagaggaaggaagaacagaaacagg

SEQ ID NO: 37180 - DNA, 28 bp, synthetic construct
  source 1..28: mol_type = other DNA
aggaaggaagaacagaaacaggtccagg

SEQ ID NO: 37181 - DNA, 28 bp, synthetic construct
  source 1..28: mol_type = other DNA
aaggaagaacagaaacaggtccaggtgg

SEQ ID NO: 37182 - DNA, 28 bp, synthetic construct
  source 1..28: mol_type = other DNA
agaaacaggtccaggtggtaatctctgg

SEQ ID NO: 37183 - DNA, 28 bp, synthetic construct
  source 1..28: mol_type = other DNA
gaaacaggtccaggtggtaatctctggg

SEQ ID NO: 37184 - DNA, 28 bp, synthetic construct
  source 1..28: mol_type = other DNA
acaggtccaggtggtaatctctgggagg

SEQ ID NO: 37185 - DNA, 28 bp, synthetic construct
  source 1..28: mol_type = other DNA
tgctttcctcccagagattaccacctgg

SEQ ID NO: 37186 - DNA, 28 bp, synthetic construct
  source 1..28: mol_type = other DNA
tggtaatctctgggaggaaagcacaagg

SEQ ID NO: 37187 - DNA, 28 bp, synthetic construct
  source 1..28: mol_type = other DNA
aacacagaggctttaacaagggggaagg

SEQ ID NO: 37188 - DNA, 28 bp, synthetic construct
  source 1..28: mol_type = other DNA
gcaaaacacagaggctttaacaaggggg

SEQ ID NO: 37189 - DNA, 28 bp, synthetic construct
  source 1..28: mol_type = other DNA
ggcaaaacacagaggctttaacaagggg

SEQ ID NO: 37190 - DNA, 28 bp, synthetic construct
  source 1..28: mol_type = other DNA
gggcaaaacacagaggctttaacaaggg

SEQ ID NO: 37191 - DNA, 28 bp, synthetic construct
  source 1..28: mol_type = other DNA
agggcaaaacacagaggctttaacaagg

SEQ ID NO: 37192 - DNA, 28 bp, synthetic construct
  source 1..28: mol_type = other DNA
tgctggaaactagggcaaaacacagagg

SEQ ID NO: 37193 - DNA, 28 bp, synthetic construct
  source 1..28: mol_type = other DNA
tgctggaaatgtctgctggaaactaggg

SEQ ID NO: 37194 - DNA, 28 bp, synthetic construct
  source 1..28: mol_type = other DNA
atgctggaaatgtctgctggaaactagg

SEQ ID NO: 37195 - DNA, 28 bp, synthetic construct
  source 1..28: mol_type = other DNA
cttctgttatgctggaaatgtctgctgg

SEQ ID NO: 37196 - DNA, 28 bp, synthetic construct
  source 1..28: mol_type = other DNA
tcactaggcactgcttctgttatgctgg

SEQ ID NO: 37197 - DNA, 28 bp, synthetic construct
  source 1..28: mol_type = other DNA
gaagagcagggggctcactctcactagg

SEQ ID NO: 37198 - DNA, 28 bp, synthetic construct
  source 1..28: mol_type = other DNA
acaagaggttgttttgaagagcaggggg

SEQ ID NO: 37199 - DNA, 28 bp, synthetic construct
  source 1..28: mol_type = other DNA
gacaagaggttgttttgaagagcagggg

SEQ ID NO: 37200 - DNA, 28 bp, synthetic construct
  source 1..28: mol_type = other DNA
agacaagaggttgttttgaagagcaggg

SEQ ID NO: 37201 - DNA, 28 bp, synthetic construct
  source 1..28: mol_type = other DNA
gagacaagaggttgttttgaagagcagg

SEQ ID NO: 37202 - DNA, 28 bp, synthetic construct
  source 1..28: mol_type = other DNA
acaacctcttgtctcctcttctgaccgg

SEQ ID NO: 37203 - DNA, 28 bp, synthetic construct
  source 1..28: mol_type = other DNA
caacctcttgtctcctcttctgaccggg

SEQ ID NO: 37204 - DNA, 28 bp, synthetic construct
  source 1..28: mol_type = other DNA
tgtcccggtcagaagaggagacaagagg

SEQ ID NO: 37205 - DNA, 28 bp, synthetic construct
  source 1..28: mol_type = other DNA
atggtgactctgtcccggtcagaagagg

SEQ ID NO: 37206 - DNA, 28 bp, synthetic construct
  source 1..28: mol_type = other DNA
accgggacagagtcaccatttgatttgg

SEQ ID NO: 37207 - DNA, 28 bp, synthetic construct
  source 1..28: mol_type = other DNA
tccaaatcaaatggtgactctgtcccgg

SEQ ID NO: 37208 - DNA, 28 bp, synthetic construct
  source 1..28: mol_type = other DNA
gtcaccatttgatttggaacagcagtgg

SEQ ID NO: 37209 - DNA, 28 bp, synthetic construct
  source 1..28: mol_type = other DNA
cttgccactgctgttccaaatcaaatgg

SEQ ID NO: 37210 - DNA, 28 bp, synthetic construct
  source 1..28: mol_type = other DNA
cagtggcaagatctcatgtccatcatgg

SEQ ID NO: 37211 - DNA, 28 bp, synthetic construct
  source 1..28: mol_type = other DNA
gatctcatgtccatcatggaaatgcagg

SEQ ID NO: 37212 - DNA, 28 bp, synthetic construct
  source 1..28: mol_type = other DNA
tcatgtccatcatggaaatgcaggtagg

SEQ ID NO: 37213 - DNA, 28 bp, synthetic construct
  source 1..28: mol_type = other DNA
gacaatcctacctgcatttccatgatgg

SEQ ID NO: 37214 - DNA, 28 bp, synthetic construct
  source 1..28: mol_type = other DNA
atcatggaaatgcaggtaggattgtcgg

SEQ ID NO: 37215 - DNA, 28 bp, synthetic construct
  source 1..28: mol_type = other DNA
gaaatgcaggtaggattgtcggaaccgg

SEQ ID NO: 37216 - DNA, 28 bp, synthetic construct
  source 1..28: mol_type = other DNA
aaatgcaggtaggattgtcggaaccggg

SEQ ID NO: 37217 - DNA, 28 bp, synthetic construct
  source 1..28: mol_type = other DNA
ttgtcggaaccgggcacaaacctattgg

SEQ ID NO: 37218 - DNA, 28 bp, synthetic construct
  source 1..28: mol_type = other DNA
gtgcaaaatccaataggtttgtgcccgg

SEQ ID NO: 37219 - DNA, 28 bp, synthetic construct
  source 1..28: mol_type = other DNA
taagacaatctgtgcaaaatccaatagg

SEQ ID NO: 37220 - DNA, 28 bp, synthetic construct
  source 1..28: mol_type = other DNA
gcactcagttgcttttccatctccaagg

SEQ ID NO: 37221 - DNA, 28 bp, synthetic construct
  source 1..28: mol_type = other DNA
gtattacactttctctccttggagatgg

SEQ ID NO: 37222 - DNA, 28 bp, synthetic construct
  source 1..28: mol_type = other DNA
gggaaagtattacactttctctccttgg

SEQ ID NO: 37223 - DNA, 28 bp, synthetic construct
  source 1..28: mol_type = other DNA
atactttccctgaatcatagagaagtgg

SEQ ID NO: 37224 - DNA, 28 bp, synthetic construct
  source 1..28: mol_type = other DNA
tactttccctgaatcatagagaagtggg

SEQ ID NO: 37225 - DNA, 28 bp, synthetic construct
  source 1..28: mol_type = other DNA
actttccctgaatcatagagaagtgggg

SEQ ID NO: 37226 - DNA, 28 bp, synthetic construct
  source 1..28: mol_type = other DNA
cagaggcacagctgcatgggtgtaaagg

SEQ ID NO: 37227 - DNA, 28 bp, synthetic construct
  source 1..28: mol_type = other DNA
tacacccatgcagctgtgcctctgttgg

SEQ ID NO: 37228 - DNA, 28 bp, synthetic construct
  source 1..28: mol_type = other DNA
acacccatgcagctgtgcctctgttggg

SEQ ID NO: 37229 - DNA, 28 bp, synthetic construct
  source 1..28: mol_type = other DNA
gcacccaacagaggcacagctgcatggg

SEQ ID NO: 37230 - DNA, 28 bp, synthetic construct
  source 1..28: mol_type = other DNA
ggcacccaacagaggcacagctgcatgg

SEQ ID NO: 37231 - DNA, 28 bp, synthetic construct
  source 1..28: mol_type = other DNA
ctcacacactgcaggcacccaacagagg

SEQ ID NO: 37232 - DNA, 28 bp, synthetic construct
  source 1..28: mol_type = other DNA
tgggtgcctgcagtgtgtgagccccagg

SEQ ID NO: 37233 - DNA, 28 bp, synthetic construct
  source 1..28: mol_type = other DNA
gggtgcctgcagtgtgtgagccccaggg

SEQ ID NO: 37234 - DNA, 28 bp, synthetic construct
  source 1..28: mol_type = other DNA
ggtgcctgcagtgtgtgagccccagggg

SEQ ID NO: 37235 - DNA, 28 bp, synthetic construct
  source 1..28: mol_type = other DNA
gcctgcagtgtgtgagccccaggggagg

SEQ ID NO: 37236 - DNA, 28 bp, synthetic construct
  source 1..28: mol_type = other DNA
ccctcccctggggctcacacactgcagg

SEQ ID NO: 37237 - DNA, 28 bp, synthetic construct
  source 1..28: mol_type = other DNA
cactaggaactgactccctcccctgggg

SEQ ID NO: 37238 - DNA, 28 bp, synthetic construct
  source 1..28: mol_type = other DNA
tcactaggaactgactccctcccctggg

SEQ ID NO: 37239 - DNA, 28 bp, synthetic construct
  source 1..28: mol_type = other DNA
ttcactaggaactgactccctcccctgg

SEQ ID NO: 37240 - DNA, 28 bp, synthetic construct
  source 1..28: mol_type = other DNA
gagggagtcagttcctagtgaacagtgg

SEQ ID NO: 37241 - DNA, 28 bp, synthetic construct
  source 1..28: mol_type = other DNA
ggggagaagagcaccactgttcactagg

SEQ ID NO: 37242 - DNA, 28 bp, synthetic construct
  source 1..28: mol_type = other DNA
aacagtggtgctcttctcccctcccagg

SEQ ID NO: 37243 - DNA, 28 bp, synthetic construct
  source 1..28: mol_type = other DNA
ggtgctcttctcccctcccaggccatgg

SEQ ID NO: 37244 - DNA, 28 bp, synthetic construct
  source 1..28: mol_type = other DNA
tgtgttcacttccatggcctgggagggg

SEQ ID NO: 37245 - DNA, 28 bp, synthetic construct
  source 1..28: mol_type = other DNA
atgtgttcacttccatggcctgggaggg

SEQ ID NO: 37246 - DNA, 28 bp, synthetic construct
  source 1..28: mol_type = other DNA
gatgtgttcacttccatggcctgggagg

SEQ ID NO: 37247 - DNA, 28 bp, synthetic construct
  source 1..28: mol_type = other DNA
gctgatgtgttcacttccatggcctggg

SEQ ID NO: 37248 - DNA, 28 bp, synthetic construct
  source 1..28: mol_type = other DNA
tgctgatgtgttcacttccatggcctgg

SEQ ID NO: 37249 - DNA, 28 bp, synthetic construct
  source 1..28: mol_type = other DNA
tcacttgctgatgtgttcacttccatgg

SEQ ID NO: 37250 - DNA, 28 bp, synthetic construct
  source 1..28: mol_type = other DNA
gtgaaatcctgtacagtgcccctcctgg

SEQ ID NO: 37251 - DNA, 28 bp, synthetic construct
  source 1..28: mol_type = other DNA
tgggtctccaggaggggcactgtacagg

SEQ ID NO: 37252 - DNA, 28 bp, synthetic construct
  source 1..28: mol_type = other DNA
ttggtgctcagtgggtctccaggagggg

SEQ ID NO: 37253 - DNA, 28 bp, synthetic construct
  source 1..28: mol_type = other DNA
gttggtgctcagtgggtctccaggaggg

SEQ ID NO: 37254 - DNA, 28 bp, synthetic construct
  source 1..28: mol_type = other DNA
agttggtgctcagtgggtctccaggagg

SEQ ID NO: 37255 - DNA, 28 bp, synthetic construct
  source 1..28: mol_type = other DNA
tgtagttggtgctcagtgggtctccagg

SEQ ID NO: 37256 - DNA, 28 bp, synthetic construct
  source 1..28: mol_type = other DNA
ggcaaggctgtagttggtgctcagtggg

SEQ ID NO: 37257 - DNA, 28 bp, synthetic construct
  source 1..28: mol_type = other DNA
gggcaaggctgtagttggtgctcagtgg

SEQ ID NO: 37258 - DNA, 28 bp, synthetic construct
  source 1..28: mol_type = other DNA
ggagtgttgggggcaaggctgtagttgg

SEQ ID NO: 37259 - DNA, 28 bp, synthetic construct
  source 1..28: mol_type = other DNA
ctgattgatgggagtgttgggggcaagg

SEQ ID NO: 37260 - DNA, 28 bp, synthetic construct
  source 1..28: mol_type = other DNA
acattctgattgatgggagtgttggggg

SEQ ID NO: 37261 - DNA, 28 bp, synthetic construct
  source 1..28: mol_type = other DNA
gacattctgattgatgggagtgttgggg

SEQ ID NO: 37262 - DNA, 28 bp, synthetic construct
  source 1..28: mol_type = other DNA
tgacattctgattgatgggagtgttggg

SEQ ID NO: 37263 - DNA, 28 bp, synthetic construct
  source 1..28: mol_type = other DNA
ctgacattctgattgatgggagtgttgg

SEQ ID NO: 37264 - DNA, 28 bp, synthetic construct
  source 1..28: mol_type = other DNA
gatgcaggctgacattctgattgatggg

SEQ ID NO: 37265 - DNA, 28 bp, synthetic construct
  source 1..28: mol_type = other DNA
tgatgcaggctgacattctgattgatgg

SEQ ID NO: 37266 - DNA, 28 bp, synthetic construct
  source 1..28: mol_type = other DNA
atcaatcagaatgtcagcctgcatcagg

SEQ ID NO: 37267 - DNA, 28 bp, synthetic construct
  source 1..28: mol_type = other DNA
aatgtcagcctgcatcaggcgtccctgg

SEQ ID NO: 37268 - DNA, 28 bp, synthetic construct
  source 1..28: mol_type = other DNA
atgtcagcctgcatcaggcgtccctggg

SEQ ID NO: 37269 - DNA, 28 bp, synthetic construct
  source 1..28: mol_type = other DNA
tgtcagcctgcatcaggcgtccctgggg

SEQ ID NO: 37270 - DNA, 28 bp, synthetic construct
  source 1..28: mol_type = other DNA
gtcagcctgcatcaggcgtccctggggg

SEQ ID NO: 37271 - DNA, 28 bp, synthetic construct
  source 1..28: mol_type = other DNA
tcagcctgcatcaggcgtccctgggggg

SEQ ID NO: 37272 - DNA, 28 bp, synthetic construct
  source 1..28: mol_type = other DNA
gcagccccccagggacgcctgatgcagg

SEQ ID NO: 37273 - DNA, 28 bp, synthetic construct
  source 1..28: mol_type = other DNA
caggcgtccctggggggctgcagccagg

SEQ ID NO: 37274 - DNA, 28 bp, synthetic construct
  source 1..28: mol_type = other DNA
aagaagtcctggctgcagccccccaggg

SEQ ID NO: 37275 - DNA, 28 bp, synthetic construct
  source 1..28: mol_type = other DNA
taagaagtcctggctgcagccccccagg

SEQ ID NO: 37276 - DNA, 28 bp, synthetic construct
  source 1..28: mol_type = other DNA
ctcggggctgaagagtaagaagtcctgg

SEQ ID NO: 37277 - DNA, 28 bp, synthetic construct
  source 1..28: mol_type = other DNA
caggacttcttactcttcagccccgagg

SEQ ID NO: 37278 - DNA, 28 bp, synthetic construct
  source 1..28: mol_type = other DNA
gacttcttactcttcagccccgaggtgg

SEQ ID NO: 37279 - DNA, 28 bp, synthetic construct
  source 1..28: mol_type = other DNA
agccccgaggtggaaagcctgcctgtgg

SEQ ID NO: 37280 - DNA, 28 bp, synthetic construct
  source 1..28: mol_type = other DNA
ggccacaggcaggctttccacctcgggg

SEQ ID NO: 37281 - DNA, 28 bp, synthetic construct
  source 1..28: mol_type = other DNA
tggccacaggcaggctttccacctcggg

SEQ ID NO: 37282 - DNA, 28 bp, synthetic construct
  source 1..28: mol_type = other DNA
ctggccacaggcaggctttccacctcgg

SEQ ID NO: 37283 - DNA, 28 bp, synthetic construct
  source 1..28: mol_type = other DNA
cagcgtggagctactggccacaggcagg

SEQ ID NO: 37284 - DNA, 28 bp, synthetic construct
  source 1..28: mol_type = other DNA
ggagcagcgtggagctactggccacagg

SEQ ID NO: 37285 - DNA, 28 bp, synthetic construct
  source 1..28: mol_type = other DNA
gccagtagctccacgctgctcccgttgg

SEQ ID NO: 37286 - DNA, 28 bp, synthetic construct
  source 1..28: mol_type = other DNA
gccaacgggagcagcgtggagctactgg

SEQ ID NO: 37287 - DNA, 28 bp, synthetic construct
  source 1..28: mol_type = other DNA
ttgctgggggccaacgggagcagcgtgg

SEQ ID NO: 37288 - DNA, 28 bp, synthetic construct
  source 1..28: mol_type = other DNA
gctggtagaattgctgggggccaacggg

SEQ ID NO: 37289 - DNA, 28 bp, synthetic construct
  source 1..28: mol_type = other DNA
ggctggtagaattgctgggggccaacgg

SEQ ID NO: 37290 - DNA, 28 bp, synthetic construct
  source 1..28: mol_type = other DNA
gagttgaggctggtagaattgctggggg

SEQ ID NO: 37291 - DNA, 28 bp, synthetic construct
  source 1..28: mol_type = other DNA
ggagttgaggctggtagaattgctgggg

SEQ ID NO: 37292 - DNA, 28 bp, synthetic construct
  source 1..28: mol_type = other DNA
tggagttgaggctggtagaattgctggg

SEQ ID NO: 37293 - DNA, 28 bp, synthetic construct
  source 1..28: mol_type = other DNA
gtggagttgaggctggtagaattgctgg

SEQ ID NO: 37294 - DNA, 28 bp, synthetic construct
  source 1..28: mol_type = other DNA
attctaccagcctcaactccaccttcgg

SEQ ID NO: 37295 - DNA, 28 bp, synthetic construct
  source 1..28: mol_type = other DNA
gtggagccgaaggtggagttgaggctgg

SEQ ID NO: 37296 - DNA, 28 bp, synthetic construct
  source 1..28: mol_type = other DNA
gttggtggagccgaaggtggagttgagg

SEQ ID NO: 37297 - DNA, 28 bp, synthetic construct
  source 1..28: mol_type = other DNA
ccaccttcggctccaccaacctgacagg

SEQ ID NO: 37298 - DNA, 28 bp, synthetic construct
  source 1..28: mol_type = other DNA
caccttcggctccaccaacctgacaggg

SEQ ID NO: 37299 - DNA, 28 bp, synthetic construct
  source 1..28: mol_type = other DNA
agccctgtcaggttggtggagccgaagg

SEQ ID NO: 37300 - DNA, 28 bp, synthetic construct
  source 1..28: mol_type = other DNA
ggaaagaagagccctgtcaggttggtgg

SEQ ID NO: 37301 - DNA, 28 bp, synthetic construct
  source 1..28: mol_type = other DNA
ggtggaaagaagagccctgtcaggttgg

SEQ ID NO: 37302 - DNA, 28 bp, synthetic construct
  source 1..28: mol_type = other DNA
ctggggtggaaagaagagccctgtcagg

SEQ ID NO: 37303 - DNA, 28 bp, synthetic construct
  source 1..28: mol_type = other DNA
ggctcttctttccaccccagctcaatgg

SEQ ID NO: 37304 - DNA, 28 bp, synthetic construct
  source 1..28: mol_type = other DNA
cattggctgtgccattgagctggggtgg

SEQ ID NO: 37305 - DNA, 28 bp, synthetic construct
  source 1..28: mol_type = other DNA
tgtcattggctgtgccattgagctgggg

SEQ ID NO: 37306 - DNA, 28 bp, synthetic construct
  source 1..28: mol_type = other DNA
gtgtcattggctgtgccattgagctggg

SEQ ID NO: 37307 - DNA, 28 bp, synthetic construct
  source 1..28: mol_type = other DNA
tgtgtcattggctgtgccattgagctgg

SEQ ID NO: 37308 - DNA, 28 bp, synthetic construct
  source 1..28: mol_type = other DNA
tcaatggcacagccaatgacacagcagg

SEQ ID NO: 37309 - DNA, 28 bp, synthetic construct
  source 1..28: mol_type = other DNA
ggcagctctgggcctgctgtgtcattgg

SEQ ID NO: 37310 - DNA, 28 bp, synthetic construct
  source 1..28: mol_type = other DNA
gcaggcccagagctgcctgaccctttgg

SEQ ID NO: 37311 - DNA, 28 bp, synthetic construct
  source 1..28: mol_type = other DNA
caggcccagagctgcctgaccctttggg

SEQ ID NO: 37312 - DNA, 28 bp, synthetic construct
  source 1..28: mol_type = other DNA
aggcccagagctgcctgaccctttgggg

SEQ ID NO: 37313 - DNA, 28 bp, synthetic construct
  source 1..28: mol_type = other DNA
ggcccagagctgcctgaccctttggggg

SEQ ID NO: 37314 - DNA, 28 bp, synthetic construct
  source 1..28: mol_type = other DNA
gcccagagctgcctgaccctttgggggg

SEQ ID NO: 37315 - DNA, 28 bp, synthetic construct
  source 1..28: mol_type = other DNA
accccccaaagggtcaggcagctctggg

SEQ ID NO: 37316 - DNA, 28 bp, synthetic construct
  source 1..28: mol_type = other DNA
gaccccccaaagggtcaggcagctctgg

SEQ ID NO: 37317 - DNA, 28 bp, synthetic construct
  source 1..28: mol_type = other DNA
catctaacagaccccccaaagggtcagg

SEQ ID NO: 37318 - DNA, 28 bp, synthetic construct
  source 1..28: mol_type = other DNA
agcttcatctaacagaccccccaaaggg

SEQ ID NO: 37319 - DNA, 28 bp, synthetic construct
  source 1..28: mol_type = other DNA
tagcttcatctaacagaccccccaaagg

SEQ ID NO: 37320 - DNA, 28 bp, synthetic construct
  source 1..28: mol_type = other DNA
gggggtctgttagatgaagctatgttgg

SEQ ID NO: 37321 - DNA, 28 bp, synthetic construct
  source 1..28: mol_type = other DNA
gctatgttggatgagatcagccttatgg

SEQ ID NO: 37322 - DNA, 28 bp, synthetic construct
  source 1..28: mol_type = other DNA
ttggatgagatcagccttatggacctgg

SEQ ID NO: 37323 - DNA, 28 bp, synthetic construct
  source 1..28: mol_type = other DNA
gccttatggacctggccattgaagaagg

SEQ ID NO: 37324 - DNA, 28 bp, synthetic construct
  source 1..28: mol_type = other DNA
gccttcttcaatggccaggtccataagg

SEQ ID NO: 37325 - DNA, 28 bp, synthetic construct
  source 1..28: mol_type = other DNA
agggttaaagccttcttcaatggccagg

SEQ ID NO: 37326 - DNA, 28 bp, synthetic construct
  source 1..28: mol_type = other DNA
tgcacagggttaaagccttcttcaatgg

SEQ ID NO: 37327 - DNA, 28 bp, synthetic construct
  source 1..28: mol_type = other DNA
attgaagaaggctttaaccctgtgcagg

SEQ ID NO: 37328 - DNA, 28 bp, synthetic construct
  source 1..28: mol_type = other DNA
tttaaccctgtgcaggcctcccagctgg

SEQ ID NO: 37329 - DNA, 28 bp, synthetic construct
  source 1..28: mol_type = other DNA
aaccctgtgcaggcctcccagctggagg

SEQ ID NO: 37330 - DNA, 28 bp, synthetic construct
  source 1..28: mol_type = other DNA
ctcctccagctgggaggcctgcacaggg

SEQ ID NO: 37331 - DNA, 28 bp, synthetic construct
  source 1..28: mol_type = other DNA
cctgtgcaggcctcccagctggaggagg

SEQ ID NO: 37332 - DNA, 28 bp, synthetic construct
  source 1..28: mol_type = other DNA
gagtcaaattcctcctccagctgggagg

SEQ ID NO: 37333 - DNA, 28 bp, synthetic construct
  source 1..28: mol_type = other DNA
tcagagtcaaattcctcctccagctggg

SEQ ID NO: 37334 - DNA, 28 bp, synthetic construct
  source 1..28: mol_type = other DNA
gtcagagtcaaattcctcctccagctgg

SEQ ID NO: 37335 - DNA, 28 bp, synthetic construct
  source 1..28: mol_type = other DNA
tggaggaggaatttgactctgactcagg

SEQ ID NO: 37336 - DNA, 28 bp, synthetic construct
  source 1..28: mol_type = other DNA
agggctatggctcgagtctaaggaaagg

SEQ ID NO: 37337 - DNA, 28 bp, synthetic construct
  source 1..28: mol_type = other DNA
gaagaagggctatggctcgagtctaagg

SEQ ID NO: 37338 - DNA, 28 bp, synthetic construct
  source 1..28: mol_type = other DNA
agagctgcttagggaagaagggctatgg

SEQ ID NO: 37339 - DNA, 28 bp, synthetic construct
  source 1..28: mol_type = other DNA
gcccttcttccctaagcagctctgaagg

SEQ ID NO: 37340 - DNA, 28 bp, synthetic construct
  source 1..28: mol_type = other DNA
gccttcagagctgcttagggaagaaggg

SEQ ID NO: 37341 - DNA, 28 bp, synthetic construct
  source 1..28: mol_type = other DNA
tgccttcagagctgcttagggaagaagg

SEQ ID NO: 37342 - DNA, 28 bp, synthetic construct
  source 1..28: mol_type = other DNA
gaagaactgccttcagagctgcttaggg

SEQ ID NO: 37343 - DNA, 28 bp, synthetic construct
  source 1..28: mol_type = other DNA
ggaagaactgccttcagagctgcttagg

SEQ ID NO: 37344 - DNA, 28 bp, synthetic construct
  source 1..28: mol_type = other DNA
gaagaggaagaggaggaggaagaagagg

SEQ ID NO: 37345 - DNA, 28 bp, synthetic construct
  source 1..28: mol_type = other DNA
gcagaggaagaagaggaagaggaggagg

SEQ ID NO: 37346 - DNA, 28 bp, synthetic construct
  source 1..28: mol_type = other DNA
gaagcagaggaagaagaggaagaggagg

SEQ ID NO: 37347 - DNA, 28 bp, synthetic construct
  source 1..28: mol_type = other DNA
gaagaagcagaggaagaagaggaagagg

SEQ ID NO: 37348 - DNA, 28 bp, synthetic construct
  source 1..28: mol_type = other DNA
gcagaggaagaagcagaggaagaagagg

SEQ ID NO: 37349 - DNA, 28 bp, synthetic construct
  source 1..28: mol_type = other DNA
gaggaagaggcagaggaagaagcagagg

SEQ ID NO: 37350 - DNA, 28 bp, synthetic construct
  source 1..28: mol_type = other DNA
tcctctgcctcttcctccttttctgagg

SEQ ID NO: 37351 - DNA, 28 bp, synthetic construct
  source 1..28: mol_type = other DNA
tcctcagaaaaggaggaagaggcagagg

SEQ ID NO: 37352 - DNA, 28 bp, synthetic construct
  source 1..28: mol_type = other DNA
ctgcctcttcctccttttctgaggaagg

SEQ ID NO: 37353 - DNA, 28 bp, synthetic construct
  source 1..28: mol_type = other DNA
gcaccttcctcagaaaaggaggaagagg

SEQ ID NO: 37354 - DNA, 28 bp, synthetic construct
  source 1..28: mol_type = other DNA
tcttcctccttttctgaggaaggtgcgg

SEQ ID NO: 37355 - DNA, 28 bp, synthetic construct
  source 1..28: mol_type = other DNA
ccaaccgcaccttcctcagaaaaggagg

SEQ ID NO: 37356 - DNA, 28 bp, synthetic construct
  source 1..28: mol_type = other DNA
tagccaaccgcaccttcctcagaaaagg

SEQ ID NO: 37357 - DNA, 28 bp, synthetic construct
  source 1..28: mol_type = other DNA
ggctacagctctgactctgagaccctgg

SEQ ID NO: 37358 - DNA, 28 bp, synthetic construct
  source 1..28: mol_type = other DNA
agctctgactctgagaccctggatctgg

SEQ ID NO: 37359 - DNA, 28 bp, synthetic construct
  source 1..28: mol_type = other DNA
gactctgagaccctggatctggaagagg

SEQ ID NO: 37360 - DNA, 28 bp, synthetic construct
  source 1..28: mol_type = other DNA
gagaccctggatctggaagaggccgagg

SEQ ID NO: 37361 - DNA, 28 bp, synthetic construct
  source 1..28: mol_type = other DNA
agaccctggatctggaagaggccgaggg

SEQ ID NO: 37362 - DNA, 28 bp, synthetic construct
  source 1..28: mol_type = other DNA
gcaccctcggcctcttccagatccaggg

SEQ ID NO: 37363 - DNA, 28 bp, synthetic construct
  source 1..28: mol_type = other DNA
agcaccctcggcctcttccagatccagg

SEQ ID NO: 37364 - DNA, 28 bp, synthetic construct
  source 1..28: mol_type = other DNA
gatctggaagaggccgagggtgctgtgg

SEQ ID NO: 37365 - DNA, 28 bp, synthetic construct
  source 1..28: mol_type = other DNA
atctggaagaggccgagggtgctgtggg

SEQ ID NO: 37366 - DNA, 28 bp, synthetic construct
  source 1..28: mol_type = other DNA
tcaggctggtagcccacagcaccctcgg

SEQ ID NO: 37367 - DNA, 28 bp, synthetic construct
  source 1..28: mol_type = other DNA
gcggcagaacttggaatactcaggctgg

SEQ ID NO: 37368 - DNA, 28 bp, synthetic construct
  source 1..28: mol_type = other DNA
tcatgcggcagaacttggaatactcagg

SEQ ID NO: 37369 - DNA, 28 bp, synthetic construct
  source 1..28: mol_type = other DNA
tccaagttctgccgcatgagctaccagg

SEQ ID NO: 37370 - DNA, 28 bp, synthetic construct
  source 1..28: mol_type = other DNA
tcctggtagctcatgcggcagaacttgg

SEQ ID NO: 37371 - DNA, 28 bp, synthetic construct
  source 1..28: mol_type = other DNA
ctgagctggatcctggtagctcatgcgg

SEQ ID NO: 37372 - DNA, 28 bp, synthetic construct
  source 1..28: mol_type = other DNA
caggcatgagagctgagctggatcctgg

SEQ ID NO: 37373 - DNA, 28 bp, synthetic construct
  source 1..28: mol_type = other DNA
ggtagggcaggcatgagagctgagctgg

SEQ ID NO: 37374 - DNA, 28 bp, synthetic construct
  source 1..28: mol_type = other DNA
gctcagctctcatgcctgccctacctgg

SEQ ID NO: 37375 - DNA, 28 bp, synthetic construct
  source 1..28: mol_type = other DNA
tcatgcctgccctacctggagcacgtgg

SEQ ID NO: 37376 - DNA, 28 bp, synthetic construct
  source 1..28: mol_type = other DNA
catgcctgccctacctggagcacgtggg

SEQ ID NO: 37377 - DNA, 28 bp, synthetic construct
  source 1..28: mol_type = other DNA
gtggcccacgtgctccaggtagggcagg

SEQ ID NO: 37378 - DNA, 28 bp, synthetic construct
  source 1..28: mol_type = other DNA
ggttgtggcccacgtgctccaggtaggg

SEQ ID NO: 37379 - DNA, 28 bp, synthetic construct
  source 1..28: mol_type = other DNA
tggttgtggcccacgtgctccaggtagg

SEQ ID NO: 37380 - DNA, 28 bp, synthetic construct
  source 1..28: mol_type = other DNA
tgtgtggttgtggcccacgtgctccagg

SEQ ID NO: 37381 - DNA, 28 bp, synthetic construct
  source 1..28: mol_type = other DNA
gtgggccacaaccacacatacaacatgg

SEQ ID NO: 37382 - DNA, 28 bp, synthetic construct
  source 1..28: mol_type = other DNA
gggtgccatgttgtatgtgtggttgtgg

SEQ ID NO: 37383 - DNA, 28 bp, synthetic construct
  source 1..28: mol_type = other DNA
ggcactgggtgccatgttgtatgtgtgg

SEQ ID NO: 37384 - DNA, 28 bp, synthetic construct
  source 1..28: mol_type = other DNA
acatacaacatggcacccagtgccctgg

SEQ ID NO: 37385 - DNA, 28 bp, synthetic construct
  source 1..28: mol_type = other DNA
gcaggtcggctgagtccagggcactggg

SEQ ID NO: 37386 - DNA, 28 bp, synthetic construct
  source 1..28: mol_type = other DNA
ggcaggtcggctgagtccagggcactgg

SEQ ID NO: 37387 - DNA, 28 bp, synthetic construct
  source 1..28: mol_type = other DNA
ggtggtggcaggtcggctgagtccaggg

SEQ ID NO: 37388 - DNA, 28 bp, synthetic construct
  source 1..28: mol_type = other DNA
gggtggtggcaggtcggctgagtccagg

SEQ ID NO: 37389 - DNA, 28 bp, synthetic construct
  source 1..28: mol_type = other DNA
ttgagggcactgggtggtggcaggtcgg

SEQ ID NO: 37390 - DNA, 28 bp, synthetic construct
  source 1..28: mol_type = other DNA
tttcttgagggcactgggtggtggcagg

SEQ ID NO: 37391 - DNA, 28 bp, synthetic construct
  source 1..28: mol_type = other DNA
tgccaccacccagtgccctcaagaaagg

SEQ ID NO: 37392 - DNA, 28 bp, synthetic construct
  source 1..28: mol_type = other DNA
tgcctttcttgagggcactgggtggtgg

SEQ ID NO: 37393 - DNA, 28 bp, synthetic construct
  source 1..28: mol_type = other DNA
tgctgcctttcttgagggcactgggtgg

SEQ ID NO: 37394 - DNA, 28 bp, synthetic construct
  source 1..28: mol_type = other DNA
cccagtgccctcaagaaaggcagcaagg

SEQ ID NO: 37395 - DNA, 28 bp, synthetic construct
  source 1..28: mol_type = other DNA
tccttgctgcctttcttgagggcactgg

SEQ ID NO: 37396 - DNA, 28 bp, synthetic construct
  source 1..28: mol_type = other DNA
tgcttctccttgctgcctttcttgaggg

SEQ ID NO: 37397 - DNA, 28 bp, synthetic construct
  source 1..28: mol_type = other DNA
ctgcttctccttgctgcctttcttgagg

SEQ ID NO: 37398 - DNA, 28 bp, synthetic construct
  source 1..28: mol_type = other DNA
ctcaagaaaggcagcaaggagaagcagg

SEQ ID NO: 37399 - DNA, 28 bp, synthetic construct
  source 1..28: mol_type = other DNA
agcaaggagaagcaggctgacttcctgg

SEQ ID NO: 37400 - DNA, 28 bp, synthetic construct
  source 1..28: mol_type = other DNA
tgacttcctggacaagcagatgagccgg

SEQ ID NO: 37401 - DNA, 28 bp, synthetic construct
  source 1..28: mol_type = other DNA
gacttcctggacaagcagatgagccggg

SEQ ID NO: 37402 - DNA, 28 bp, synthetic construct
  source 1..28: mol_type = other DNA
ctcatcccggctcatctgcttgtccagg

SEQ ID NO: 37403 - DNA, 28 bp, synthetic construct
  source 1..28: mol_type = other DNA
catggctcgggctcggtgctcatcccgg

SEQ ID NO: 37404 - DNA, 28 bp, synthetic construct
  source 1..28: mol_type = other DNA
gaaagggatcttcatggctcgggctcgg

SEQ ID NO: 37405 - DNA, 28 bp, synthetic construct
  source 1..28: mol_type = other DNA
ttggtgaaagggatcttcatggctcggg

SEQ ID NO: 37406 - DNA, 28 bp, synthetic construct
  source 1..28: mol_type = other DNA
attggtgaaagggatcttcatggctcgg

SEQ ID NO: 37407 - DNA, 28 bp, synthetic construct
  source 1..28: mol_type = other DNA
ttgtcattggtgaaagggatcttcatgg

SEQ ID NO: 37408 - DNA, 28 bp, synthetic construct
  source 1..28: mol_type = other DNA
gttgatgattttgtcattggtgaaaggg

SEQ ID NO: 37409 - DNA, 28 bp, synthetic construct
  source 1..28: mol_type = other DNA
ggttgatgattttgtcattggtgaaagg

SEQ ID NO: 37410 - DNA, 28 bp, synthetic construct
  source 1..28: mol_type = other DNA
acaggcaggttgatgattttgtcattgg

SEQ ID NO: 37411 - DNA, 28 bp, synthetic construct
  source 1..28: mol_type = other DNA
aatgacaaaatcatcaacctgcctgtgg

SEQ ID NO: 37412 - DNA, 28 bp, synthetic construct
  source 1..28: mol_type = other DNA
gacaaaatcatcaacctgcctgtggagg

SEQ ID NO: 37413 - DNA, 28 bp, synthetic construct
  source 1..28: mol_type = other DNA
cagttcattgaactcctccacaggcagg

SEQ ID NO: 37414 - DNA, 28 bp, synthetic construct
  source 1..28: mol_type = other DNA
acagcagttcattgaactcctccacagg

SEQ ID NO: 37415 - DNA, 28 bp, synthetic construct
  source 1..28: mol_type = other DNA
agctgggcttcactcaactggtatttgg

SEQ ID NO: 37416 - DNA, 28 bp, synthetic construct
  source 1..28: mol_type = other DNA
gaggctcagctgggcttcactcaactgg

SEQ ID NO: 37417 - DNA, 28 bp, synthetic construct
  source 1..28: mol_type = other DNA
cggatgtctcggatgaggctcagctggg

SEQ ID NO: 37418 - DNA, 28 bp, synthetic construct
  source 1..28: mol_type = other DNA
ccagctgagcctcatccgagacatccgg

SEQ ID NO: 37419 - DNA, 28 bp, synthetic construct
  source 1..28: mol_type = other DNA
gagcctcatccgagacatccggcgccgg

SEQ ID NO: 37420 - DNA, 28 bp, synthetic construct
  source 1..28: mol_type = other DNA
agcctcatccgagacatccggcgccggg

SEQ ID NO: 37421 - DNA, 28 bp, synthetic construct
  source 1..28: mol_type = other DNA
gcctcatccgagacatccggcgccgggg

SEQ ID NO: 37422 - DNA, 28 bp, synthetic construct
  source 1..28: mol_type = other DNA
gccccggcgccggatgtctcggatgagg

SEQ ID NO: 37423 - DNA, 28 bp, synthetic construct
  source 1..28: mol_type = other DNA
gttcttgccccggcgccggatgtctcgg

SEQ ID NO: 37424 - DNA, 28 bp, synthetic construct
  source 1..28: mol_type = other DNA
atccggcgccggggcaagaacaagatgg

SEQ ID NO: 37425 - DNA, 28 bp, synthetic construct
  source 1..28: mol_type = other DNA
cgccatcttgttcttgccccggcgccgg

SEQ ID NO: 37426 - DNA, 28 bp, synthetic construct
  source 1..28: mol_type = other DNA
cggcgccggggcaagaacaagatggcgg

SEQ ID NO: 37427 - DNA, 28 bp, synthetic construct
  source 1..28: mol_type = other DNA
ctgcgccgccatcttgttcttgccccgg

SEQ ID NO: 37428 - DNA, 28 bp, synthetic construct
  source 1..28: mol_type = other DNA
gcgcagaactgccgcaagcgcaagctgg

SEQ ID NO: 37429 - DNA, 28 bp, synthetic construct
  source 1..28: mol_type = other DNA
caggatggtgtccagcttgcgcttgcgg

SEQ ID NO: 37430 - DNA, 28 bp, synthetic construct
  source 1..28: mol_type = other DNA
cgcaagctggacaccatcctgaatctgg

SEQ ID NO: 37431 - DNA, 28 bp, synthetic construct
  source 1..28: mol_type = other DNA
accatcctgaatctggagcgtgatgtgg

SEQ ID NO: 37432 - DNA, 28 bp, synthetic construct
  source 1..28: mol_type = other DNA
tccacatcacgctccagattcaggatgg

SEQ ID NO: 37433 - DNA, 28 bp, synthetic construct
  source 1..28: mol_type = other DNA
atcctgaatctggagcgtgatgtggagg

SEQ ID NO: 37434 - DNA, 28 bp, synthetic construct
  source 1..28: mol_type = other DNA
gtcctccacatcacgctccagattcagg

SEQ ID NO: 37435 - DNA, 28 bp, synthetic construct
  source 1..28: mol_type = other DNA
ggaggacctgcagcgtgacaaagcccgg

SEQ ID NO: 37436 - DNA, 28 bp, synthetic construct
  source 1..28: mol_type = other DNA
cagcagccgggctttgtcacgctgcagg

SEQ ID NO: 37437 - DNA, 28 bp, synthetic construct
  source 1..28: mol_type = other DNA
gcagcgtgacaaagcccggctgctgcgg

SEQ ID NO: 37438 - DNA, 28 bp, synthetic construct
  source 1..28: mol_type = other DNA
cagcgtgacaaagcccggctgctgcggg

SEQ ID NO: 37439 - DNA, 28 bp, synthetic construct
  source 1..28: mol_type = other DNA
aaagcccggctgctgcgggagaaagtgg

SEQ ID NO: 37440 - DNA, 28 bp, synthetic construct
  source 1..28: mol_type = other DNA
aactccactttctcccgcagcagccggg

SEQ ID NO: 37441 - DNA, 28 bp, synthetic construct
  source 1..28: mol_type = other DNA
gaactccactttctcccgcagcagccgg

SEQ ID NO: 37442 - DNA, 28 bp, synthetic construct
  source 1..28: mol_type = other DNA
ctgcttcatctgtcgcagggagcgcagg

SEQ ID NO: 37443 - DNA, 28 bp, synthetic construct
  source 1..28: mol_type = other DNA
cgctccctgcgacagatgaagcagaagg

SEQ ID NO: 37444 - DNA, 28 bp, synthetic construct
  source 1..28: mol_type = other DNA
tggaccttctgcttcatctgtcgcaggg

SEQ ID NO: 37445 - DNA, 28 bp, synthetic construct
  source 1..28: mol_type = other DNA
ctggaccttctgcttcatctgtcgcagg

SEQ ID NO: 37446 - DNA, 28 bp, synthetic construct
  source 1..28: mol_type = other DNA
aagcagaaggtccagagcctgtaccagg

SEQ ID NO: 37447 - DNA, 28 bp, synthetic construct
  source 1..28: mol_type = other DNA
cagaaggtccagagcctgtaccaggagg

SEQ ID NO: 37448 - DNA, 28 bp, synthetic construct
  source 1..28: mol_type = other DNA
tccagagcctgtaccaggaggtgtttgg

SEQ ID NO: 37449 - DNA, 28 bp, synthetic construct
  source 1..28: mol_type = other DNA
ccagagcctgtaccaggaggtgtttggg

SEQ ID NO: 37450 - DNA, 28 bp, synthetic construct
  source 1..28: mol_type = other DNA
gagcctgtaccaggaggtgtttgggcgg

SEQ ID NO: 37451 - DNA, 28 bp, synthetic construct
  source 1..28: mol_type = other DNA
cagccgcccaaacacctcctggtacagg

SEQ ID NO: 37452 - DNA, 28 bp, synthetic construct
  source 1..28: mol_type = other DNA
atctcgcagccgcccaaacacctcctgg

SEQ ID NO: 37453 - DNA, 28 bp, synthetic construct
  source 1..28: mol_type = other DNA
tgtttgggcggctgcgagatgagaacgg

SEQ ID NO: 37454 - DNA, 28 bp, synthetic construct
  source 1..28: mol_type = other DNA
ggagcgcatactgactgggcgagtaggg

SEQ ID NO: 37455 - DNA, 28 bp, synthetic construct
  source 1..28: mol_type = other DNA
tggagcgcatactgactgggcgagtagg

SEQ ID NO: 37456 - DNA, 28 bp, synthetic construct
  source 1..28: mol_type = other DNA
cggcgtactggagcgcatactgactggg

SEQ ID NO: 37457 - DNA, 28 bp, synthetic construct
  source 1..28: mol_type = other DNA
ccagtcagtatgcgctccagtacgccgg

SEQ ID NO: 37458 - DNA, 28 bp, synthetic construct
  source 1..28: mol_type = other DNA
cagtcagtatgcgctccagtacgccggg

SEQ ID NO: 37459 - DNA, 28 bp, synthetic construct
  source 1..28: mol_type = other DNA
agtcagtatgcgctccagtacgccgggg

SEQ ID NO: 37460 - DNA, 28 bp, synthetic construct
  source 1..28: mol_type = other DNA
agtatgcgctccagtacgccggggacgg

SEQ ID NO: 37461 - DNA, 28 bp, synthetic construct
  source 1..28: mol_type = other DNA
gaggacactgccgtccccggcgtactgg

SEQ ID NO: 37462 - DNA, 28 bp, synthetic construct
  source 1..28: mol_type = other DNA
gggatgaggaggacactgccgtccccgg

SEQ ID NO: 37463 - DNA, 28 bp, synthetic construct
  source 1..28: mol_type = other DNA
agtgtcctcctcatcccccgcacgatgg

SEQ ID NO: 37464 - DNA, 28 bp, synthetic construct
  source 1..28: mol_type = other DNA
gtcggccatcgtgcgggggatgaggagg

SEQ ID NO: 37465 - DNA, 28 bp, synthetic construct
  source 1..28: mol_type = other DNA
ctggtcggccatcgtgcgggggatgagg

SEQ ID NO: 37466 - DNA, 28 bp, synthetic construct
  source 1..28: mol_type = other DNA
atcccccgcacgatggccgaccagcagg

SEQ ID NO: 37467 - DNA, 28 bp, synthetic construct
  source 1..28: mol_type = other DNA
ggcctgctggtcggccatcgtgcggggg

SEQ ID NO: 37468 - DNA, 28 bp, synthetic construct
  source 1..28: mol_type = other DNA
gggcctgctggtcggccatcgtgcgggg

SEQ ID NO: 37469 - DNA, 28 bp, synthetic construct
  source 1..28: mol_type = other DNA
cgggcctgctggtcggccatcgtgcggg

SEQ ID NO: 37470 - DNA, 28 bp, synthetic construct
  source 1..28: mol_type = other DNA
ccgcacgatggccgaccagcaggcccgg

SEQ ID NO: 37471 - DNA, 28 bp, synthetic construct
  source 1..28: mol_type = other DNA
cacgatggccgaccagcaggcccggcgg

SEQ ID NO: 37472 - DNA, 28 bp, synthetic construct
  source 1..28: mol_type = other DNA
atggccgaccagcaggcccggcggcagg

SEQ ID NO: 37473 - DNA, 28 bp, synthetic construct
  source 1..28: mol_type = other DNA
ctctcctgccgccgggcctgctggtcgg

SEQ ID NO: 37474 - DNA, 28 bp, synthetic construct
  source 1..28: mol_type = other DNA
cgaccagcaggcccggcggcaggagagg

SEQ ID NO: 37475 - DNA, 28 bp, synthetic construct
  source 1..28: mol_type = other DNA
cttcctctcctgccgccgggcctgctgg

SEQ ID NO: 37476 - DNA, 28 bp, synthetic construct
  source 1..28: mol_type = other DNA
gcccggcggcaggagaggaagccaaagg

SEQ ID NO: 37477 - DNA, 28 bp, synthetic construct
  source 1..28: mol_type = other DNA
tcctttggcttcctctcctgccgccggg

SEQ ID NO: 37478 - DNA, 28 bp, synthetic construct
  source 1..28: mol_type = other DNA
gtcctttggcttcctctcctgccgccgg

SEQ ID NO: 37479 - DNA, 28 bp, synthetic construct
  source 1..28: mol_type = other DNA
gcggcaggagaggaagccaaaggaccgg

SEQ ID NO: 37480 - DNA, 28 bp, synthetic construct
  source 1..28: mol_type = other DNA
gccaaaggaccggagaaagtgagcctgg

SEQ ID NO: 37481 - DNA, 28 bp, synthetic construct
  source 1..28: mol_type = other DNA
cccaggctcactttctccggtcctttgg

SEQ ID NO: 37482 - DNA, 28 bp, synthetic construct
  source 1..28: mol_type = other DNA
caaaggaccggagaaagtgagcctgggg

SEQ ID NO: 37483 - DNA, 28 bp, synthetic construct
  source 1..28: mol_type = other DNA
ccggagaaagtgagcctggggaagaagg

SEQ ID NO: 37484 - DNA, 28 bp, synthetic construct
  source 1..28: mol_type = other DNA
cggagaaagtgagcctggggaagaaggg

SEQ ID NO: 37485 - DNA, 28 bp, synthetic construct
  source 1..28: mol_type = other DNA
ggagaaagtgagcctggggaagaagggg

SEQ ID NO: 37486 - DNA, 28 bp, synthetic construct
  source 1..28: mol_type = other DNA
gagaaagtgagcctggggaagaaggggg

SEQ ID NO: 37487 - DNA, 28 bp, synthetic construct
  source 1..28: mol_type = other DNA
tgggcttcaaacccccttcttccccagg

SEQ ID NO: 37488 - DNA, 28 bp, synthetic construct
  source 1..28: mol_type = other DNA
gtttgaagcccaccaagaccgaaactgg

SEQ ID NO: 37489 - DNA, 28 bp, synthetic construct
  source 1..28: mol_type = other DNA
agcccaccaagaccgaaactggagaagg

SEQ ID NO: 37490 - DNA, 28 bp, synthetic construct
  source 1..28: mol_type = other DNA
gcccaccaagaccgaaactggagaaggg

SEQ ID NO: 37491 - DNA, 28 bp, synthetic construct
  source 1..28: mol_type = other DNA
gcccttctccagtttcggtcttggtggg

SEQ ID NO: 37492 - DNA, 28 bp, synthetic construct
  source 1..28: mol_type = other DNA
agcccttctccagtttcggtcttggtgg

SEQ ID NO: 37493 - DNA, 28 bp, synthetic construct
  source 1..28: mol_type = other DNA
accaagaccgaaactggagaagggctgg

SEQ ID NO: 37494 - DNA, 28 bp, synthetic construct
  source 1..28: mol_type = other DNA
tccagcccttctccagtttcggtcttgg

SEQ ID NO: 37495 - DNA, 28 bp, synthetic construct
  source 1..28: mol_type = other DNA
accgaaactggagaagggctggacctgg

SEQ ID NO: 37496 - DNA, 28 bp, synthetic construct
  source 1..28: mol_type = other DNA
tccaggtccagcccttctccagtttcgg

SEQ ID NO: 37497 - DNA, 28 bp, synthetic construct
  source 1..28: mol_type = other DNA
actggagaagggctggacctggacctgg

SEQ ID NO: 37498 - DNA, 28 bp, synthetic construct
  source 1..28: mol_type = other DNA
gaagggctggacctggacctggacctgg

SEQ ID NO: 37499 - DNA, 28 bp, synthetic construct
  source 1..28: mol_type = other DNA
cctggacctggacctggacctacagcgg

SEQ ID NO: 37500 - DNA, 28 bp, synthetic construct
  source 1..28: mol_type = other DNA
ctggacctggacctggacctacagcggg

SEQ ID NO: 37501 - DNA, 28 bp, synthetic construct
  source 1..28: mol_type = other DNA
tggacctggacctggacctacagcgggg

SEQ ID NO: 37502 - DNA, 28 bp, synthetic construct
  source 1..28: mol_type = other DNA
aagtccccgctgtaggtccaggtccagg

SEQ ID NO: 37503 - DNA, 28 bp, synthetic construct
  source 1..28: mol_type = other DNA
gcatttaagtccccgctgtaggtccagg

SEQ ID NO: 37504 - DNA, 28 bp, synthetic construct
  source 1..28: mol_type = other DNA
aagaaggcatttaagtccccgctgtagg

SEQ ID NO: 37505 - DNA, 28 bp, synthetic construct
  source 1..28: mol_type = other DNA
atctgagaagatatattggataagaagg

SEQ ID NO: 37506 - DNA, 28 bp, synthetic construct
  source 1..28: mol_type = other DNA
ttcttatccaatatatcttctcagatgg

SEQ ID NO: 37507 - DNA, 28 bp, synthetic construct
  source 1..28: mol_type = other DNA
tcttatccaatatatcttctcagatggg

SEQ ID NO: 37508 - DNA, 28 bp, synthetic construct
  source 1..28: mol_type = other DNA
agtcatcccatctgagaagatatattgg

SEQ ID NO: 37509 - DNA, 28 bp, synthetic construct
  source 1..28: mol_type = other DNA
tatatcttctcagatgggatgactgcgg

SEQ ID NO: 37510 - DNA, 28 bp, synthetic construct
  source 1..28: mol_type = other DNA
atatcttctcagatgggatgactgcggg

SEQ ID NO: 37511 - DNA, 28 bp, synthetic construct
  source 1..28: mol_type = other DNA
atgggatgactgcgggtcagtgtacagg

SEQ ID NO: 37512 - DNA, 28 bp, synthetic construct
  source 1..28: mol_type = other DNA
tgactgcgggtcagtgtacaggaagagg

SEQ ID NO: 37513 - DNA, 28 bp, synthetic construct
  source 1..28: mol_type = other DNA
tgcgggtcagtgtacaggaagaggcagg

SEQ ID NO: 37514 - DNA, 28 bp, synthetic construct
  source 1..28: mol_type = other DNA
tcagtgtacaggaagaggcaggcactgg

SEQ ID NO: 37515 - DNA, 28 bp, synthetic construct
  source 1..28: mol_type = other DNA
tgtacaggaagaggcaggcactggctgg

SEQ ID NO: 37516 - DNA, 28 bp, synthetic construct
  source 1..28: mol_type = other DNA
aggcactggctggctcagctccactcgg

SEQ ID NO: 37517 - DNA, 28 bp, synthetic construct
  source 1..28: mol_type = other DNA
ggcactggctggctcagctccactcggg

SEQ ID NO: 37518 - DNA, 28 bp, synthetic construct
  source 1..28: mol_type = other DNA
actggctggctcagctccactcgggtgg

SEQ ID NO: 37519 - DNA, 28 bp, synthetic construct
  source 1..28: mol_type = other DNA
ctggctcagctccactcgggtggagtgg

SEQ ID NO: 37520 - DNA, 28 bp, synthetic construct
  source 1..28: mol_type = other DNA
cagctccactcgggtggagtggaagtgg

SEQ ID NO: 37521 - DNA, 28 bp, synthetic construct
  source 1..28: mol_type = other DNA
tctggccacttccactccacccgagtgg

SEQ ID NO: 37522 - DNA, 28 bp, synthetic construct
  source 1..28: mol_type = other DNA
agtggaagtggccagaccatttagacgg

SEQ ID NO: 37523 - DNA, 28 bp, synthetic construct
  source 1..28: mol_type = other DNA
aagtggccagaccatttagacggacagg

SEQ ID NO: 37524 - DNA, 28 bp, synthetic construct
  source 1..28: mol_type = other DNA
agtggccagaccatttagacggacaggg

SEQ ID NO: 37525 - DNA, 28 bp, synthetic construct
  source 1..28: mol_type = other DNA
gaggaccctgtccgtctaaatggtctgg

SEQ ID NO: 37526 - DNA, 28 bp, synthetic construct
  source 1..28: mol_type = other DNA
agggtgaggaccctgtccgtctaaatgg

SEQ ID NO: 37527 - DNA, 28 bp, synthetic construct
  source 1..28: mol_type = other DNA
gtcctcaccctacccctttcctgtgagg

SEQ ID NO: 37528 - DNA, 28 bp, synthetic construct
  source 1..28: mol_type = other DNA
tgcctcacaggaaaggggtagggtgagg

SEQ ID NO: 37529 - DNA, 28 bp, synthetic construct
  source 1..28: mol_type = other DNA
tcaccctacccctttcctgtgaggcagg

SEQ ID NO: 37530 - DNA, 28 bp, synthetic construct
  source 1..28: mol_type = other DNA
caccctacccctttcctgtgaggcaggg

SEQ ID NO: 37531 - DNA, 28 bp, synthetic construct
  source 1..28: mol_type = other DNA
accctacccctttcctgtgaggcagggg

SEQ ID NO: 37532 - DNA, 28 bp, synthetic construct
  source 1..28: mol_type = other DNA
acccctgcctcacaggaaaggggtaggg

SEQ ID NO: 37533 - DNA, 28 bp, synthetic construct
  source 1..28: mol_type = other DNA
cacccctgcctcacaggaaaggggtagg

SEQ ID NO: 37534 - DNA, 28 bp, synthetic construct
  source 1..28: mol_type = other DNA
ctacccctttcctgtgaggcaggggtgg

SEQ ID NO: 37535 - DNA, 28 bp, synthetic construct
  source 1..28: mol_type = other DNA
ccaccacccctgcctcacaggaaagggg

SEQ ID NO: 37536 - DNA, 28 bp, synthetic construct
  source 1..28: mol_type = other DNA
accaccacccctgcctcacaggaaaggg

SEQ ID NO: 37537 - DNA, 28 bp, synthetic construct
  source 1..28: mol_type = other DNA
caccaccacccctgcctcacaggaaagg

SEQ ID NO: 37538 - DNA, 28 bp, synthetic construct
  source 1..28: mol_type = other DNA
ctttcctgtgaggcaggggtggtggtgg

SEQ ID NO: 37539 - DNA, 28 bp, synthetic construct
  source 1..28: mol_type = other DNA
aactccaccaccacccctgcctcacagg

SEQ ID NO: 37540 - DNA, 28 bp, synthetic construct
  source 1..28: mol_type = other DNA
gaggcaggggtggtggtggagttgctgg

SEQ ID NO: 37541 - DNA, 28 bp, synthetic construct
  source 1..28: mol_type = other DNA
gcaggggtggtggtggagttgctggagg

SEQ ID NO: 37542 - DNA, 28 bp, synthetic construct
  source 1..28: mol_type = other DNA
gtggtggtggagttgctggaggtagagg

SEQ ID NO: 37543 - DNA, 28 bp, synthetic construct
  source 1..28: mol_type = other DNA
agttgctggaggtagaggagctatgtgg

SEQ ID NO: 37544 - DNA, 28 bp, synthetic construct
  source 1..28: mol_type = other DNA
gaggtagaggagctatgtggagcaaagg

SEQ ID NO: 37545 - DNA, 28 bp, synthetic construct
  source 1..28: mol_type = other DNA
agctatgtggagcaaaggccgacagagg

SEQ ID NO: 37546 - DNA, 28 bp, synthetic construct
  source 1..28: mol_type = other DNA
gctatgtggagcaaaggccgacagaggg

SEQ ID NO: 37547 - DNA, 28 bp, synthetic construct
  source 1..28: mol_type = other DNA
ctatgtggagcaaaggccgacagagggg

SEQ ID NO: 37548 - DNA, 28 bp, synthetic construct
  source 1..28: mol_type = other DNA
gtggagcaaaggccgacagaggggaagg

SEQ ID NO: 37549 - DNA, 28 bp, synthetic construct
  source 1..28: mol_type = other DNA
gcaaaggccgacagaggggaaggaatgg

SEQ ID NO: 37550 - DNA, 28 bp, synthetic construct
  source 1..28: mol_type = other DNA
cacaggtccattccttcccctctgtcgg

SEQ ID NO: 37551 - DNA, 28 bp, synthetic construct
  source 1..28: mol_type = other DNA
agaggggaaggaatggacctgtgagagg

SEQ ID NO: 37552 - DNA, 28 bp, synthetic construct
  source 1..28: mol_type = other DNA
gggaaggaatggacctgtgagaggaagg

SEQ ID NO: 37553 - DNA, 28 bp, synthetic construct
  source 1..28: mol_type = other DNA
ggaaggaatggacctgtgagaggaaggg

SEQ ID NO: 37554 - DNA, 28 bp, synthetic construct
  source 1..28: mol_type = other DNA
ggaatggacctgtgagaggaagggaagg

SEQ ID NO: 37555 - DNA, 28 bp, synthetic construct
  source 1..28: mol_type = other DNA
atggacctgtgagaggaagggaaggtgg

SEQ ID NO: 37556 - DNA, 28 bp, synthetic construct
  source 1..28: mol_type = other DNA
ttctgccaccttcccttcctctcacagg

SEQ ID NO: 37557 - DNA, 28 bp, synthetic construct
  source 1..28: mol_type = other DNA
ggaaggtggcagaaagtctcatttcagg

SEQ ID NO: 37558 - DNA, 28 bp, synthetic construct
  source 1..28: mol_type = other DNA
ggtggcagaaagtctcatttcaggaagg

SEQ ID NO: 37559 - DNA, 28 bp, synthetic construct
  source 1..28: mol_type = other DNA
ggcagaaagtctcatttcaggaaggagg

SEQ ID NO: 37560 - DNA, 28 bp, synthetic construct
  source 1..28: mol_type = other DNA
gcagaaagtctcatttcaggaaggaggg

SEQ ID NO: 37561 - DNA, 28 bp, synthetic construct
  source 1..28: mol_type = other DNA
tctcatttcaggaaggagggatagaagg

SEQ ID NO: 37562 - DNA, 28 bp, synthetic construct
  source 1..28: mol_type = other DNA
atttcaggaaggagggatagaaggaagg

SEQ ID NO: 37563 - DNA, 28 bp, synthetic construct
  source 1..28: mol_type = other DNA
caggaaggagggatagaaggaaggaagg

SEQ ID NO: 37564 - DNA, 28 bp, synthetic construct
  source 1..28: mol_type = other DNA
aaggagggatagaaggaaggaaggaagg

SEQ ID NO: 37565 - DNA, 28 bp, synthetic construct
  source 1..28: mol_type = other DNA
tttgatttttttttcggggggggggggg

SEQ ID NO: 37566 - DNA, 28 bp, synthetic construct
  source 1..28: mol_type = other DNA
ctttgatttttttttcgggggggggggg

SEQ ID NO: 37567 - DNA, 28 bp, synthetic construct
  source 1..28: mol_type = other DNA
gctttgatttttttttcggggggggggg

SEQ ID NO: 37568 - DNA, 28 bp, synthetic construct
  source 1..28: mol_type = other DNA
cgctttgatttttttttcgggggggggg

SEQ ID NO: 37569 - DNA, 28 bp, synthetic construct
  source 1..28: mol_type = other DNA
ccgctttgatttttttttcggggggggg

SEQ ID NO: 37570 - DNA, 28 bp, synthetic construct
  source 1..28: mol_type = other DNA
ccccccccgaaaaaaaaatcaaagcggg

SEQ ID NO: 37571 - DNA, 28 bp, synthetic construct
  source 1..28: mol_type = other DNA
tcccgctttgatttttttttcggggggg

SEQ ID NO: 37572 - DNA, 28 bp, synthetic construct
  source 1..28: mol_type = other DNA
ttcccgctttgatttttttttcgggggg

SEQ ID NO: 37573 - DNA, 28 bp, synthetic construct
  source 1..28: mol_type = other DNA
cttcccgctttgatttttttttcggggg

SEQ ID NO: 37574 - DNA, 28 bp, synthetic construct
  source 1..28: mol_type = other DNA
tcttcccgctttgatttttttttcgggg

SEQ ID NO: 37575 - DNA, 28 bp, synthetic construct
  source 1..28: mol_type = other DNA
ttcttcccgctttgatttttttttcggg

SEQ ID NO: 37576 - DNA, 28 bp, synthetic construct
  source 1..28: mol_type = other DNA
tttcttcccgctttgatttttttttcgg

SEQ ID NO: 37577 - DNA, 28 bp, synthetic construct
  source 1..28: mol_type = other DNA
aaaatcaaagcgggaagaaaatcagagg

SEQ ID NO: 37578 - DNA, 28 bp, synthetic construct
  source 1..28: mol_type = other DNA
aaatcaaagcgggaagaaaatcagaggg

SEQ ID NO: 37579 - DNA, 28 bp, synthetic construct
  source 1..28: mol_type = other DNA
caaagcgggaagaaaatcagagggaagg

SEQ ID NO: 37580 - DNA, 28 bp, synthetic construct
  source 1..28: mol_type = other DNA
gggaagaaaatcagagggaaggttaagg

SEQ ID NO: 37581 - DNA, 28 bp, synthetic construct
  source 1..28: mol_type = other DNA
agaaaatcagagggaaggttaaggttgg

SEQ ID NO: 37582 - DNA, 28 bp, synthetic construct
  source 1..28: mol_type = other DNA
tcagagggaaggttaaggttggctctgg

SEQ ID NO: 37583 - DNA, 28 bp, synthetic construct
  source 1..28: mol_type = other DNA
gggaaggttaaggttggctctggccagg

SEQ ID NO: 37584 - DNA, 28 bp, synthetic construct
  source 1..28: mol_type = other DNA
taaggttggctctggccaggattccagg

SEQ ID NO: 37585 - DNA, 28 bp, synthetic construct
  source 1..28: mol_type = other DNA
ggctctggccaggattccaggcagcagg

SEQ ID NO: 37586 - DNA, 28 bp, synthetic construct
  source 1..28: mol_type = other DNA
ctggccaggattccaggcagcaggttgg

SEQ ID NO: 37587 - DNA, 28 bp, synthetic construct
  source 1..28: mol_type = other DNA
cactccaacctgctgcctggaatcctgg

SEQ ID NO: 37588 - DNA, 28 bp, synthetic construct
  source 1..28: mol_type = other DNA
attccaggcagcaggttggagtgactgg

SEQ ID NO: 37589 - DNA, 28 bp, synthetic construct
  source 1..28: mol_type = other DNA
ccaccagtcactccaacctgctgcctgg

SEQ ID NO: 37590 - DNA, 28 bp, synthetic construct
  source 1..28: mol_type = other DNA
caggcagcaggttggagtgactggtggg

SEQ ID NO: 37591 - DNA, 28 bp, synthetic construct
  source 1..28: mol_type = other DNA
ggagtgactggtgggcctagatcactgg

SEQ ID NO: 37592 - DNA, 28 bp, synthetic construct
  source 1..28: mol_type = other DNA
ttggggtttatcacaccagtgatctagg

SEQ ID NO: 37593 - DNA, 28 bp, synthetic construct
  source 1..28: mol_type = other DNA
gtgtgataaaccccaattttcaccccgg

SEQ ID NO: 37594 - DNA, 28 bp, synthetic construct
  source 1..28: mol_type = other DNA
tgtgataaaccccaattttcaccccggg

SEQ ID NO: 37595 - DNA, 28 bp, synthetic construct
  source 1..28: mol_type = other DNA
gtgataaaccccaattttcaccccgggg

SEQ ID NO: 37596 - DNA, 28 bp, synthetic construct
  source 1..28: mol_type = other DNA
tgataaaccccaattttcaccccggggg

SEQ ID NO: 37597 - DNA, 28 bp, synthetic construct
  source 1..28: mol_type = other DNA
gataaaccccaattttcaccccgggggg

SEQ ID NO: 37598 - DNA, 28 bp, synthetic construct
  source 1..28: mol_type = other DNA
ataaaccccaattttcaccccggggggg

SEQ ID NO: 37599 - DNA, 28 bp, synthetic construct
  source 1..28: mol_type = other DNA
taaaccccaattttcaccccgggggggg

SEQ ID NO: 37600 - DNA, 28 bp, synthetic construct
  source 1..28: mol_type = other DNA
accccaattttcaccccggggggggtgg

SEQ ID NO: 37601 - DNA, 28 bp, synthetic construct
  source 1..28: mol_type = other DNA
cccaccccccccggggtgaaaattgggg

SEQ ID NO: 37602 - DNA, 28 bp, synthetic construct
  source 1..28: mol_type = other DNA
ccccaccccccccggggtgaaaattggg

SEQ ID NO: 37603 - DNA, 28 bp, synthetic construct
  source 1..28: mol_type = other DNA
accccaccccccccggggtgaaaattgg

SEQ ID NO: 37604 - DNA, 28 bp, synthetic construct
  source 1..28: mol_type = other DNA
gtgtctgtgtaccccaccccccccgggg

SEQ ID NO: 37605 - DNA, 28 bp, synthetic construct
  source 1..28: mol_type = other DNA
tgtgtctgtgtaccccaccccccccggg

SEQ ID NO: 37606 - DNA, 28 bp, synthetic construct
  source 1..28: mol_type = other DNA
ctgtgtctgtgtaccccaccccccccgg

SEQ ID NO: 37607 - DNA, 28 bp, synthetic construct
  source 1..28: mol_type = other DNA
cggggggggtggggtacacagacacagg

SEQ ID NO: 37608 - DNA, 28 bp, synthetic construct
  source 1..28: mol_type = other DNA
ggggggggtggggtacacagacacaggg

SEQ ID NO: 37609 - DNA, 28 bp, synthetic construct
  source 1..28: mol_type = other DNA
gggggtggggtacacagacacagggtgg

SEQ ID NO: 37610 - DNA, 28 bp, synthetic construct
  source 1..28: mol_type = other DNA
ggggtggggtacacagacacagggtggg

SEQ ID NO: 37611 - DNA, 28 bp, synthetic construct
  source 1..28: mol_type = other DNA
gggtggggtacacagacacagggtgggg

SEQ ID NO: 37612 - DNA, 28 bp, synthetic construct
  source 1..28: mol_type = other DNA
ggtggggtacacagacacagggtggggg

SEQ ID NO: 37613 - DNA, 28 bp, synthetic construct
  source 1..28: mol_type = other DNA
ggggtacacagacacagggtgggggtgg

SEQ ID NO: 37614 - DNA, 28 bp, synthetic construct
  source 1..28: mol_type = other DNA
gggtacacagacacagggtgggggtggg

SEQ ID NO: 37615 - DNA, 28 bp, synthetic construct
  source 1..28: mol_type = other DNA
ggtacacagacacagggtgggggtgggg

SEQ ID NO: 37616 - DNA, 28 bp, synthetic construct
  source 1..28: mol_type = other DNA
acacagacacagggtgggggtggggagg

SEQ ID NO: 37617 - DNA, 28 bp, synthetic construct
  source 1..28: mol_type = other DNA
cacagacacagggtgggggtggggaggg

SEQ ID NO: 37618 - DNA, 28 bp, synthetic construct
  source 1..28: mol_type = other DNA
gacacagggtgggggtggggagggacgg

SEQ ID NO: 37619 - DNA, 28 bp, synthetic construct
  source 1..28: mol_type = other DNA
gctccttgcattttgacatccctgaagg

SEQ ID NO: 37620 - DNA, 28 bp, synthetic construct
  source 1..28: mol_type = other DNA
ctccttgcattttgacatccctgaaggg

SEQ ID NO: 37621 - DNA, 28 bp, synthetic construct
  source 1..28: mol_type = other DNA
tccttgcattttgacatccctgaagggg

SEQ ID NO: 37622 - DNA, 28 bp, synthetic construct
  source 1..28: mol_type = other DNA
tccccttcagggatgtcaaaatgcaagg

SEQ ID NO: 37623 - DNA, 28 bp, synthetic construct
  source 1..28: mol_type = other DNA
tttgacatccctgaaggggagctcttgg

SEQ ID NO: 37624 - DNA, 28 bp, synthetic construct
  source 1..28: mol_type = other DNA
aatgatatccaagagctccccttcaggg

SEQ ID NO: 37625 - DNA, 28 bp, synthetic construct
  source 1..28: mol_type = other DNA
caatgatatccaagagctccccttcagg

SEQ ID NO: 37626 - DNA, 28 bp, synthetic construct
  source 1..28: mol_type = other DNA
ctgaaggggagctcttggatatcattgg

SEQ ID NO: 37627 - DNA, 28 bp, synthetic construct
  source 1..28: mol_type = other DNA
tatcattggccatgtttcaatcgaatgg

SEQ ID NO: 37628 - DNA, 28 bp, synthetic construct
  source 1..28: mol_type = other DNA
ccatgtttcaatcgaatggagccactgg

SEQ ID NO: 37629 - DNA, 28 bp, synthetic construct
  source 1..28: mol_type = other DNA
catgtttcaatcgaatggagccactggg

SEQ ID NO: 37630 - DNA, 28 bp, synthetic construct
  source 1..28: mol_type = other DNA
gaatggagccactgggccccaacactgg

SEQ ID NO: 37631 - DNA, 28 bp, synthetic construct
  source 1..28: mol_type = other DNA
tctcaaagccagtgttggggcccagtgg

SEQ ID NO: 37632 - DNA, 28 bp, synthetic construct
  source 1..28: mol_type = other DNA
actctaaatctcaaagccagtgttgggg

SEQ ID NO: 37633 - DNA, 28 bp, synthetic construct
  source 1..28: mol_type = other DNA
gactctaaatctcaaagccagtgttggg

SEQ ID NO: 37634 - DNA, 28 bp, synthetic construct
  source 1..28: mol_type = other DNA
tgactctaaatctcaaagccagtgttgg

SEQ ID NO: 37635 - DNA, 28 bp, synthetic construct
  source 1..28: mol_type = other DNA
cactggctttgagatttagagtcaaagg

SEQ ID NO: 37636 - DNA, 28 bp, synthetic construct
  source 1..28: mol_type = other DNA
actggctttgagatttagagtcaaaggg

SEQ ID NO: 37637 - DNA, 28 bp, synthetic construct
  source 1..28: mol_type = other DNA
tttagagtcaaagggtagagtgaacagg

SEQ ID NO: 37638 - DNA, 28 bp, synthetic construct
  source 1..28: mol_type = other DNA
agtcaaagggtagagtgaacaggaaagg

SEQ ID NO: 37639 - DNA, 28 bp, synthetic construct
  source 1..28: mol_type = other DNA
gtcaaagggtagagtgaacaggaaaggg

SEQ ID NO: 37640 - DNA, 28 bp, synthetic construct
  source 1..28: mol_type = other DNA
gtagagtgaacaggaaagggtcacgtgg

SEQ ID NO: 37641 - DNA, 28 bp, synthetic construct
  source 1..28: mol_type = other DNA
cgtgatgttggggctgttgcaacatggg

SEQ ID NO: 37642 - DNA, 28 bp, synthetic construct
  source 1..28: mol_type = other DNA
gcgtgatgttggggctgttgcaacatgg

SEQ ID NO: 37643 - DNA, 28 bp, synthetic construct
  source 1..28: mol_type = other DNA
gcagtgaatgacatgcgtgatgttgggg

SEQ ID NO: 37644 - DNA, 28 bp, synthetic construct
  source 1..28: mol_type = other DNA
ggcagtgaatgacatgcgtgatgttggg

SEQ ID NO: 37645 - DNA, 28 bp, synthetic construct
  source 1..28: mol_type = other DNA
aggcagtgaatgacatgcgtgatgttgg

SEQ ID NO: 37646 - DNA, 28 bp, synthetic construct
  source 1..28: mol_type = other DNA
gagcacggagggagatggagtggcaagg

SEQ ID NO: 37647 - DNA, 28 bp, synthetic construct
  source 1..28: mol_type = other DNA
ggctggagcacggagggagatggagtgg

SEQ ID NO: 37648 - DNA, 28 bp, synthetic construct
  source 1..28: mol_type = other DNA
ggggtggctggagcacggagggagatgg

SEQ ID NO: 37649 - DNA, 28 bp, synthetic construct
  source 1..28: mol_type = other DNA
agctcaggggtggctggagcacggaggg

SEQ ID NO: 37650 - DNA, 28 bp, synthetic construct
  source 1..28: mol_type = other DNA
cagctcaggggtggctggagcacggagg

SEQ ID NO: 37651 - DNA, 28 bp, synthetic construct
  source 1..28: mol_type = other DNA
ccgtgctccagccacccctgagctgagg

SEQ ID NO: 37652 - DNA, 28 bp, synthetic construct
  source 1..28: mol_type = other DNA
atgggagcctcagctcaggggtggctgg

SEQ ID NO: 37653 - DNA, 28 bp, synthetic construct
  source 1..28: mol_type = other DNA
gacaatgggagcctcagctcaggggtgg

SEQ ID NO: 37654 - DNA, 28 bp, synthetic construct
  source 1..28: mol_type = other DNA
ggagacaatgggagcctcagctcagggg

SEQ ID NO: 37655 - DNA, 28 bp, synthetic construct
  source 1..28: mol_type = other DNA
tggagacaatgggagcctcagctcaggg

SEQ ID NO: 37656 - DNA, 28 bp, synthetic construct
  source 1..28: mol_type = other DNA
atggagacaatgggagcctcagctcagg

SEQ ID NO: 37657 - DNA, 28 bp, synthetic construct
  source 1..28: mol_type = other DNA
acatgcaggctctgatggagacaatggg

SEQ ID NO: 37658 - DNA, 28 bp, synthetic construct
  source 1..28: mol_type = other DNA
cacatgcaggctctgatggagacaatgg

SEQ ID NO: 37659 - DNA, 28 bp, synthetic construct
  source 1..28: mol_type = other DNA
gacggcatacacatgcaggctctgatgg

SEQ ID NO: 37660 - DNA, 28 bp, synthetic construct
  source 1..28: mol_type = other DNA
cctgcatgtgtatgccgtcctcccctgg

SEQ ID NO: 37661 - DNA, 28 bp, synthetic construct
  source 1..28: mol_type = other DNA
atgtgtatgccgtcctcccctggtccgg

SEQ ID NO: 37662 - DNA, 28 bp, synthetic construct
  source 1..28: mol_type = other DNA
acacaaacaccggaccaggggaggacgg

SEQ ID NO: 37663 - DNA, 28 bp, synthetic construct
  source 1..28: mol_type = other DNA
gggaacacaaacaccggaccaggggagg

SEQ ID NO: 37664 - DNA, 28 bp, synthetic construct
  source 1..28: mol_type = other DNA
gtggggaacacaaacaccggaccagggg

SEQ ID NO: 37665 - DNA, 28 bp, synthetic construct
  source 1..28: mol_type = other DNA
ggtggggaacacaaacaccggaccaggg

SEQ ID NO: 37666 - DNA, 28 bp, synthetic construct
  source 1..28: mol_type = other DNA
gggtggggaacacaaacaccggaccagg

SEQ ID NO: 37667 - DNA, 28 bp, synthetic construct
  source 1..28: mol_type = other DNA
tgtgaggggtggggaacacaaacaccgg

SEQ ID NO: 37668 - DNA, 28 bp, synthetic construct
  source 1..28: mol_type = other DNA
gagctcaggcagtctgtgaggggtgggg

SEQ ID NO: 37669 - DNA, 28 bp, synthetic construct
  source 1..28: mol_type = other DNA
agagctcaggcagtctgtgaggggtggg

SEQ ID NO: 37670 - DNA, 28 bp, synthetic construct
  source 1..28: mol_type = other DNA
aagagctcaggcagtctgtgaggggtgg

SEQ ID NO: 37671 - DNA, 28 bp, synthetic construct
  source 1..28: mol_type = other DNA
cagaagagctcaggcagtctgtgagggg

SEQ ID NO: 37672 - DNA, 28 bp, synthetic construct
  source 1..28: mol_type = other DNA
acagaagagctcaggcagtctgtgaggg

SEQ ID NO: 37673 - DNA, 28 bp, synthetic construct
  source 1..28: mol_type = other DNA
tacagaagagctcaggcagtctgtgagg

SEQ ID NO: 37674 - DNA, 28 bp, synthetic construct
  source 1..28: mol_type = other DNA
agactgcctgagctcttctgtaagctgg

SEQ ID NO: 37675 - DNA, 28 bp, synthetic construct
  source 1..28: mol_type = other DNA
gactgcctgagctcttctgtaagctggg

SEQ ID NO: 37676 - DNA, 28 bp, synthetic construct
  source 1..28: mol_type = other DNA
actgcctgagctcttctgtaagctgggg

SEQ ID NO: 37677 - DNA, 28 bp, synthetic construct
  source 1..28: mol_type = other DNA
cctaccccagcttacagaagagctcagg

SEQ ID NO: 37678 - DNA, 28 bp, synthetic construct
  source 1..28: mol_type = other DNA
ctgagctcttctgtaagctggggtaggg

SEQ ID NO: 37679 - DNA, 28 bp, synthetic construct
  source 1..28: mol_type = other DNA
tcttctgtaagctggggtagggtgatgg

SEQ ID NO: 37680 - DNA, 28 bp, synthetic construct
  source 1..28: mol_type = other DNA
ctggggtagggtgatggcagtgctccgg

SEQ ID NO: 37681 - DNA, 28 bp, synthetic construct
  source 1..28: mol_type = other DNA
tggggtagggtgatggcagtgctccggg

SEQ ID NO: 37682 - DNA, 28 bp, synthetic construct
  source 1..28: mol_type = other DNA
agggtgatggcagtgctccgggaactgg

SEQ ID NO: 37683 - DNA, 28 bp, synthetic construct
  source 1..28: mol_type = other DNA
gggtgatggcagtgctccgggaactggg

SEQ ID NO: 37684 - DNA, 28 bp, synthetic construct
  source 1..28: mol_type = other DNA
agaggaaggctgcaggcccagttcccgg

SEQ ID NO: 37685 - DNA, 28 bp, synthetic construct
  source 1..28: mol_type = other DNA
aactgggcctgcagccttcctcttctgg

SEQ ID NO: 37686 - DNA, 28 bp, synthetic construct
  source 1..28: mol_type = other DNA
actgggcctgcagccttcctcttctggg

SEQ ID NO: 37687 - DNA, 28 bp, synthetic construct
  source 1..28: mol_type = other DNA
agcagtcccagaagaggaaggctgcagg

SEQ ID NO: 37688 - DNA, 28 bp, synthetic construct
  source 1..28: mol_type = other DNA
gccttcctcttctgggactgctgtgagg

SEQ ID NO: 37689 - DNA, 28 bp, synthetic construct
  source 1..28: mol_type = other DNA
gcctcacagcagtcccagaagaggaagg

SEQ ID NO: 37690 - DNA, 28 bp, synthetic construct
  source 1..28: mol_type = other DNA
ctctgcctcacagcagtcccagaagagg

SEQ ID NO: 37691 - DNA, 28 bp, synthetic construct
  source 1..28: mol_type = other DNA
ctcttctgggactgctgtgaggcagagg

SEQ ID NO: 37692 - DNA, 28 bp, synthetic construct
  source 1..28: mol_type = other DNA
ggactgctgtgaggcagaggaatgatgg

SEQ ID NO: 37693 - DNA, 28 bp, synthetic construct
  source 1..28: mol_type = other DNA
tggagaatctagtgtagcagcctccagg

SEQ ID NO: 37694 - DNA, 28 bp, synthetic construct
  source 1..28: mol_type = other DNA
gaatctagtgtagcagcctccaggcagg

SEQ ID NO: 37695 - DNA, 28 bp, synthetic construct
  source 1..28: mol_type = other DNA
cagtgttgtgctgaatcctgcctggagg

SEQ ID NO: 37696 - DNA, 28 bp, synthetic construct
  source 1..28: mol_type = other DNA
ctccaggcaggattcagcacaacactgg

SEQ ID NO: 37697 - DNA, 28 bp, synthetic construct
  source 1..28: mol_type = other DNA
tccaggcaggattcagcacaacactggg

SEQ ID NO: 37698 - DNA, 28 bp, synthetic construct
  source 1..28: mol_type = other DNA
ccaggcaggattcagcacaacactgggg

SEQ ID NO: 37699 - DNA, 28 bp, synthetic construct
  source 1..28: mol_type = other DNA
caacactggggagtcacccttccctcgg

SEQ ID NO: 37700 - DNA, 28 bp, synthetic construct
  source 1..28: mol_type = other DNA
aacactggggagtcacccttccctcggg

SEQ ID NO: 37701 - DNA, 28 bp, synthetic construct
  source 1..28: mol_type = other DNA
gttggtaggcagaggcccgagggaaggg

SEQ ID NO: 37702 - DNA, 28 bp, synthetic construct
  source 1..28: mol_type = other DNA
tgttggtaggcagaggcccgagggaagg

SEQ ID NO: 37703 - DNA, 28 bp, synthetic construct
  source 1..28: mol_type = other DNA
cagttgttggtaggcagaggcccgaggg

SEQ ID NO: 37704 - DNA, 28 bp, synthetic construct
  source 1..28: mol_type = other DNA
ccagttgttggtaggcagaggcccgagg

SEQ ID NO: 37705 - DNA, 28 bp, synthetic construct
  source 1..28: mol_type = other DNA
ctcgggcctctgcctaccaacaactggg

SEQ ID NO: 37706 - DNA, 28 bp, synthetic construct
  source 1..28: mol_type = other DNA
gataagcccagttgttggtaggcagagg

SEQ ID NO: 37707 - DNA, 28 bp, synthetic construct
  source 1..28: mol_type = other DNA
gcctaccaacaactgggcttatcactgg

SEQ ID NO: 37708 - DNA, 28 bp, synthetic construct
  source 1..28: mol_type = other DNA
cctaccaacaactgggcttatcactggg

SEQ ID NO: 37709 - DNA, 28 bp, synthetic construct
  source 1..28: mol_type = other DNA
ttttcccagtgataagcccagttgttgg

SEQ ID NO: 37710 - DNA, 28 bp, synthetic construct
  source 1..28: mol_type = other DNA
gaggactagttcttttgttgttgctggg

SEQ ID NO: 37711 - DNA, 28 bp, synthetic construct
  source 1..28: mol_type = other DNA
agaggactagttcttttgttgttgctgg

SEQ ID NO: 37712 - DNA, 28 bp, synthetic construct
  source 1..28: mol_type = other DNA
aaatcaaagcgcaagaaattctaagagg

SEQ ID NO: 37713 - DNA, 28 bp, synthetic construct
  source 1..28: mol_type = other DNA
gaatttcttgcgctttgatttttttagg

SEQ ID NO: 37714 - DNA, 28 bp, synthetic construct
  source 1..28: mol_type = other DNA
aatttcttgcgctttgatttttttaggg

SEQ ID NO: 37715 - DNA, 28 bp, synthetic construct
  source 1..28: mol_type = other DNA
agggcttgtgccctgtttcacttatagg

SEQ ID NO: 37716 - DNA, 28 bp, synthetic construct
  source 1..28: mol_type = other DNA
gggcttgtgccctgtttcacttataggg

SEQ ID NO: 37717 - DNA, 28 bp, synthetic construct
  source 1..28: mol_type = other DNA
cattctagaccctataagtgaaacaggg

SEQ ID NO: 37718 - DNA, 28 bp, synthetic construct
  source 1..28: mol_type = other DNA
gcattctagaccctataagtgaaacagg

SEQ ID NO: 37719 - DNA, 28 bp, synthetic construct
  source 1..28: mol_type = other DNA
tctagaatgcttgtgttgagtaaaaagg

SEQ ID NO: 37720 - DNA, 28 bp, synthetic construct
  source 1..28: mol_type = other DNA
agaacatttagcagctttgaatattggg

SEQ ID NO: 37721 - DNA, 28 bp, synthetic construct
  source 1..28: mol_type = other DNA
gagaacatttagcagctttgaatattgg

SEQ ID NO: 37722 - DNA, 28 bp, synthetic construct
  source 1..28: mol_type = other DNA
ttcacacagttacacggagtctttatgg

SEQ ID NO: 37723 - DNA, 28 bp, synthetic construct
  source 1..28: mol_type = other DNA
gactccgtgtaactgtgtgaacacttgg

SEQ ID NO: 37724 - DNA, 28 bp, synthetic construct
  source 1..28: mol_type = other DNA
actccgtgtaactgtgtgaacacttggg

SEQ ID NO: 37725 - DNA, 28 bp, synthetic construct
  source 1..28: mol_type = other DNA
aatcccaagtgttcacacagttacacgg

SEQ ID NO: 37726 - DNA, 28 bp, synthetic construct
  source 1..28: mol_type = other DNA
cttgggatttttctcctctgtcccgagg

SEQ ID NO: 37727 - DNA, 28 bp, synthetic construct
  source 1..28: mol_type = other DNA
aaagcagacgacgacctcgggacagagg

SEQ ID NO: 37728 - DNA, 28 bp, synthetic construct
  source 1..28: mol_type = other DNA
aaaaaagaaagcagacgacgacctcggg

SEQ ID NO: 37729 - DNA, 28 bp, synthetic construct
  source 1..28: mol_type = other DNA
caaaaaagaaagcagacgacgacctcgg

SEQ ID NO: 37730 - DNA, 28 bp, synthetic construct
  source 1..28: mol_type = other DNA
cgaggtcgtcgtctgctttcttttttgg

SEQ ID NO: 37731 - DNA, 28 bp, synthetic construct
  source 1..28: mol_type = other DNA
gaggtcgtcgtctgctttcttttttggg

SEQ ID NO: 37732 - DNA, 28 bp, synthetic construct
  source 1..28: mol_type = other DNA
tagaagattgagaagtgcatatgacagg

SEQ ID NO: 37733 - DNA, 28 bp, synthetic construct
  source 1..28: mol_type = other DNA
tggctgagagcttgtgtgtttggggagg

SEQ ID NO: 37734 - DNA, 28 bp, synthetic construct
  source 1..28: mol_type = other DNA
ctgtggctgagagcttgtgtgtttgggg

SEQ ID NO: 37735 - DNA, 28 bp, synthetic construct
  source 1..28: mol_type = other DNA
cctgtggctgagagcttgtgtgtttggg

SEQ ID NO: 37736 - DNA, 28 bp, synthetic construct
  source 1..28: mol_type = other DNA
gcctgtggctgagagcttgtgtgtttgg

SEQ ID NO: 37737 - DNA, 28 bp, synthetic construct
  source 1..28: mol_type = other DNA
gctggggctgtggagaagctgcctgtgg

SEQ ID NO: 37738 - DNA, 28 bp, synthetic construct
  source 1..28: mol_type = other DNA
cttctccacagccccagcttcgcacagg

SEQ ID NO: 37739 - DNA, 28 bp, synthetic construct
  source 1..28: mol_type = other DNA
aggagcctgtgcgaagctggggctgtgg

SEQ ID NO: 37740 - DNA, 28 bp, synthetic construct
  source 1..28: mol_type = other DNA
acagccccagcttcgcacaggctcctgg

SEQ ID NO: 37741 - DNA, 28 bp, synthetic construct
  source 1..28: mol_type = other DNA
gccccagcttcgcacaggctcctggagg

SEQ ID NO: 37742 - DNA, 28 bp, synthetic construct
  source 1..28: mol_type = other DNA
ccctccaggagcctgtgcgaagctgggg

SEQ ID NO: 37743 - DNA, 28 bp, synthetic construct
  source 1..28: mol_type = other DNA
gccctccaggagcctgtgcgaagctggg

SEQ ID NO: 37744 - DNA, 28 bp, synthetic construct
  source 1..28: mol_type = other DNA
agccctccaggagcctgtgcgaagctgg

SEQ ID NO: 37745 - DNA, 28 bp, synthetic construct
  source 1..28: mol_type = other DNA
tcgcacaggctcctggagggctgcctgg

SEQ ID NO: 37746 - DNA, 28 bp, synthetic construct
  source 1..28: mol_type = other DNA
cgcacaggctcctggagggctgcctggg

SEQ ID NO: 37747 - DNA, 28 bp, synthetic construct
  source 1..28: mol_type = other DNA
gcacaggctcctggagggctgcctgggg

SEQ ID NO: 37748 - DNA, 28 bp, synthetic construct
  source 1..28: mol_type = other DNA
cacaggctcctggagggctgcctggggg

SEQ ID NO: 37749 - DNA, 28 bp, synthetic construct
  source 1..28: mol_type = other DNA
aggctcctggagggctgcctgggggagg

SEQ ID NO: 37750 - DNA, 28 bp, synthetic construct
  source 1..28: mol_type = other DNA
gtctgcctcccccaggcagccctccagg

SEQ ID NO: 37751 - DNA, 28 bp, synthetic construct
  source 1..28: mol_type = other DNA
gagggctgcctgggggaggcagacatgg

SEQ ID NO: 37752 - DNA, 28 bp, synthetic construct
  source 1..28: mol_type = other DNA
agggctgcctgggggaggcagacatggg

SEQ ID NO: 37753 - DNA, 28 bp, synthetic construct
  source 1..28: mol_type = other DNA
tggcactcccatgtctgcctcccccagg

SEQ ID NO: 37754 - DNA, 28 bp, synthetic construct
  source 1..28: mol_type = other DNA
gggggaggcagacatgggagtgccaagg

SEQ ID NO: 37755 - DNA, 28 bp, synthetic construct
  source 1..28: mol_type = other DNA
ggaggcagacatgggagtgccaaggtgg

SEQ ID NO: 37756 - DNA, 28 bp, synthetic construct
  source 1..28: mol_type = other DNA
acatgggagtgccaaggtggccagatgg

SEQ ID NO: 37757 - DNA, 28 bp, synthetic construct
  source 1..28: mol_type = other DNA
agtgccaaggtggccagatggttccagg

SEQ ID NO: 37758 - DNA, 28 bp, synthetic construct
  source 1..28: mol_type = other DNA
tagtcctggaaccatctggccaccttgg

SEQ ID NO: 37759 - DNA, 28 bp, synthetic construct
  source 1..28: mol_type = other DNA
aagacattgtagtcctggaaccatctgg

SEQ ID NO: 37760 - DNA, 28 bp, synthetic construct
  source 1..28: mol_type = other DNA
gttaaaaataaagacattgtagtcctgg

SEQ ID NO: 37761 - DNA, 28 bp, synthetic construct
  source 1..28: mol_type = other DNA
tgccactgctgccctcacccctgcccgg

SEQ ID NO: 37762 - DNA, 28 bp, synthetic construct
  source 1..28: mol_type = other DNA
agccgggcaggggtgagggcagcagtgg

SEQ ID NO: 37763 - DNA, 28 bp, synthetic construct
  source 1..28: mol_type = other DNA
tgctgccctcacccctgcccggctctgg

SEQ ID NO: 37764 - DNA, 28 bp, synthetic construct
  source 1..28: mol_type = other DNA
gtactccagagccgggcaggggtgaggg

SEQ ID NO: 37765 - DNA, 28 bp, synthetic construct
  source 1..28: mol_type = other DNA
ggtactccagagccgggcaggggtgagg

SEQ ID NO: 37766 - DNA, 28 bp, synthetic construct
  source 1..28: mol_type = other DNA
cagacggtactccagagccgggcagggg

SEQ ID NO: 37767 - DNA, 28 bp, synthetic construct
  source 1..28: mol_type = other DNA
gcagacggtactccagagccgggcaggg

SEQ ID NO: 37768 - DNA, 28 bp, synthetic construct
  source 1..28: mol_type = other DNA
ggcagacggtactccagagccgggcagg

SEQ ID NO: 37769 - DNA, 28 bp, synthetic construct
  source 1..28: mol_type = other DNA
ctggggcagacggtactccagagccggg

SEQ ID NO: 37770 - DNA, 28 bp, synthetic construct
  source 1..28: mol_type = other DNA
tctggggcagacggtactccagagccgg

SEQ ID NO: 37771 - DNA, 28 bp, synthetic construct
  source 1..28: mol_type = other DNA
tggagtaccgtctgccccagacaagtgg

SEQ ID NO: 37772 - DNA, 28 bp, synthetic construct
  source 1..28: mol_type = other DNA
ggagtaccgtctgccccagacaagtggg

SEQ ID NO: 37773 - DNA, 28 bp, synthetic construct
  source 1..28: mol_type = other DNA
ttcactcccacttgtctggggcagacgg

SEQ ID NO: 37774 - DNA, 28 bp, synthetic construct
  source 1..28: mol_type = other DNA
ctgccccagacaagtgggagtgaaatgg

SEQ ID NO: 37775 - DNA, 28 bp, synthetic construct
  source 1..28: mol_type = other DNA
tgccccagacaagtgggagtgaaatggg

SEQ ID NO: 37776 - DNA, 28 bp, synthetic construct
  source 1..28: mol_type = other DNA
gccccagacaagtgggagtgaaatgggg

SEQ ID NO: 37777 - DNA, 28 bp, synthetic construct
  source 1..28: mol_type = other DNA
cccccatttcactcccacttgtctgggg

SEQ ID NO: 37778 - DNA, 28 bp, synthetic construct
  source 1..28: mol_type = other DNA
acccccatttcactcccacttgtctggg

SEQ ID NO: 37779 - DNA, 28 bp, synthetic construct
  source 1..28: mol_type = other DNA
cacccccatttcactcccacttgtctgg

SEQ ID NO: 37780 - DNA, 28 bp, synthetic construct
  source 1..28: mol_type = other DNA
cagacaagtgggagtgaaatgggggtgg

SEQ ID NO: 37781 - DNA, 28 bp, synthetic construct
  source 1..28: mol_type = other DNA
agacaagtgggagtgaaatgggggtggg

SEQ ID NO: 37782 - DNA, 28 bp, synthetic construct
  source 1..28: mol_type = other DNA
gacaagtgggagtgaaatgggggtgggg

SEQ ID NO: 37783 - DNA, 28 bp, synthetic construct
  source 1..28: mol_type = other DNA
acaagtgggagtgaaatgggggtggggg

SEQ ID NO: 37784 - DNA, 28 bp, synthetic construct
  source 1..28: mol_type = other DNA
caagtgggagtgaaatgggggtgggggg

SEQ ID NO: 37785 - DNA, 28 bp, synthetic construct
  source 1..28: mol_type = other DNA
tggggggaagcactgattcccagttagg

SEQ ID NO: 37786 - DNA, 28 bp, synthetic construct
  source 1..28: mol_type = other DNA
ggggggaagcactgattcccagttaggg

SEQ ID NO: 37787 - DNA, 28 bp, synthetic construct
  source 1..28: mol_type = other DNA
gggggaagcactgattcccagttagggg

SEQ ID NO: 37788 - DNA, 28 bp, synthetic construct
  source 1..28: mol_type = other DNA
ggggaagcactgattcccagttaggggg

SEQ ID NO: 37789 - DNA, 28 bp, synthetic construct
  source 1..28: mol_type = other DNA
ctgctcagttaggcaccccctaactggg

SEQ ID NO: 37790 - DNA, 28 bp, synthetic construct
  source 1..28: mol_type = other DNA
actgctcagttaggcaccccctaactgg

SEQ ID NO: 37791 - DNA, 28 bp, synthetic construct
  source 1..28: mol_type = other DNA
gttagggggtgcctaactgagcagtagg

SEQ ID NO: 37792 - DNA, 28 bp, synthetic construct
  source 1..28: mol_type = other DNA
ttagggggtgcctaactgagcagtaggg

SEQ ID NO: 37793 - DNA, 28 bp, synthetic construct
  source 1..28: mol_type = other DNA
tgcctaactgagcagtagggatagaagg

SEQ ID NO: 37794 - DNA, 28 bp, synthetic construct
  source 1..28: mol_type = other DNA
caccttctatccctactgctcagttagg

SEQ ID NO: 37795 - DNA, 28 bp, synthetic construct
  source 1..28: mol_type = other DNA
gcagtagggatagaaggtgtgaacctgg

SEQ ID NO: 37796 - DNA, 28 bp, synthetic construct
  source 1..28: mol_type = other DNA
cagtagggatagaaggtgtgaacctggg

SEQ ID NO: 37797 - DNA, 28 bp, synthetic construct
  source 1..28: mol_type = other DNA
gaaaataatttataaaagcactcccagg

SEQ ID NO: 37798 - DNA, 28 bp, synthetic construct
  source 1..28: mol_type = other DNA
agataaattaaaaataaaatctacaagg

SEQ ID NO: 37799 - DNA, 28 bp, synthetic construct
  source 1..28: mol_type = other DNA
ttttaatttatctctgtgacctgccagg

SEQ ID NO: 37800 - DNA, 28 bp, synthetic construct
  source 1..28: mol_type = other DNA
tttaatttatctctgtgacctgccaggg

SEQ ID NO: 37801 - DNA, 28 bp, synthetic construct
  source 1..28: mol_type = other DNA
tttatctctgtgacctgccagggagagg

SEQ ID NO: 37802 - DNA, 28 bp, synthetic construct
  source 1..28: mol_type = other DNA
ttatctctgtgacctgccagggagaggg

SEQ ID NO: 37803 - DNA, 28 bp, synthetic construct
  source 1..28: mol_type = other DNA
tatctctgtgacctgccagggagagggg

SEQ ID NO: 37804 - DNA, 28 bp, synthetic construct
  source 1..28: mol_type = other DNA
tctctctctctcccctctccctggcagg

SEQ ID NO: 37805 - DNA, 28 bp, synthetic construct
  source 1..28: mol_type = other DNA
catctctctctctctcccctctccctgg

SEQ ID NO: 37806 - DNA, 28 bp, synthetic construct
  source 1..28: mol_type = other DNA
gagcacatgacaaaataaaataaaatgg

SEQ ID NO: 37807 - DNA, 28 bp, synthetic construct
  source 1..28: mol_type = other DNA
ttattctcaatttaaattcaaagtgggg

SEQ ID NO: 37808 - DNA, 28 bp, synthetic construct
  source 1..28: mol_type = other DNA
tttattctcaatttaaattcaaagtggg

SEQ ID NO: 37809 - DNA, 28 bp, synthetic construct
  source 1..28: mol_type = other DNA
ctttattctcaatttaaattcaaagtgg

SEQ ID NO: 37810 - DNA, 28 bp, synthetic construct
  source 1..28: mol_type = other DNA
cactttgaatttaaattgagaataaagg

SEQ ID NO: 37811 - DNA, 28 bp, synthetic construct
  source 1..28: mol_type = other DNA
gaatttaaattgagaataaaggaaatgg

SEQ ID NO: 37812 - DNA, 28 bp, synthetic construct
  source 1..28: mol_type = other DNA
agaataaaggaaatggactcattgtagg

SEQ ID NO: 37813 - DNA, 28 bp, synthetic construct
  source 1..28: mol_type = other DNA
tttctatttttgcaaaataaagtgatgg

SEQ ID NO: 37814 - DNA, 28 bp, synthetic construct
  source 1..28: mol_type = other DNA
gaaaactcagcaatatgcgatacagcgg

SEQ ID NO: 37815 - DNA, 28 bp, synthetic construct
  source 1..28: mol_type = other DNA
aaaactcagcaatatgcgatacagcggg

SEQ ID NO: 37816 - DNA, 28 bp, synthetic construct
  source 1..28: mol_type = other DNA
aaactcagcaatatgcgatacagcgggg

SEQ ID NO: 37817 - DNA, 28 bp, synthetic construct
  source 1..28: mol_type = other DNA
agcaatatgcgatacagcggggtagagg

SEQ ID NO: 37818 - DNA, 28 bp, synthetic construct
  source 1..28: mol_type = other DNA
gcaatatgcgatacagcggggtagaggg

SEQ ID NO: 37819 - DNA, 28 bp, synthetic construct
  source 1..28: mol_type = other DNA
caatatgcgatacagcggggtagagggg

SEQ ID NO: 37820 - DNA, 28 bp, synthetic construct
  source 1..28: mol_type = other DNA
cggggtagaggggagatgtaaacagagg

SEQ ID NO: 37821 - DNA, 28 bp, synthetic construct
  source 1..28: mol_type = other DNA
ggggtagaggggagatgtaaacagaggg

SEQ ID NO: 37822 - DNA, 28 bp, synthetic construct
  source 1..28: mol_type = other DNA
gggtagaggggagatgtaaacagagggg

SEQ ID NO: 37823 - DNA, 28 bp, synthetic construct
  source 1..28: mol_type = other DNA
tagaggggagatgtaaacagaggggagg

SEQ ID NO: 37824 - DNA, 28 bp, synthetic construct
  source 1..28: mol_type = other DNA
agaggggagatgtaaacagaggggaggg

SEQ ID NO: 37825 - DNA, 28 bp, synthetic construct
  source 1..28: mol_type = other DNA
gaggggagatgtaaacagaggggagggg

SEQ ID NO: 37826 - DNA, 28 bp, synthetic construct
  source 1..28: mol_type = other DNA
gcaccctgaccccccaagagaacacagg

SEQ ID NO: 37827 - DNA, 28 bp, synthetic construct
  source 1..28: mol_type = other DNA
caccctgaccccccaagagaacacaggg

SEQ ID NO: 37828 - DNA, 28 bp, synthetic construct
  source 1..28: mol_type = other DNA
ctccctgtgttctcttggggggtcaggg

SEQ ID NO: 37829 - DNA, 28 bp, synthetic construct
  source 1..28: mol_type = other DNA
gctccctgtgttctcttggggggtcagg

SEQ ID NO: 37830 - DNA, 28 bp, synthetic construct
  source 1..28: mol_type = other DNA
cattggctccctgtgttctcttgggggg

SEQ ID NO: 37831 - DNA, 28 bp, synthetic construct
  source 1..28: mol_type = other DNA
ccattggctccctgtgttctcttggggg

SEQ ID NO: 37832 - DNA, 28 bp, synthetic construct
  source 1..28: mol_type = other DNA
cccattggctccctgtgttctcttgggg

SEQ ID NO: 37833 - DNA, 28 bp, synthetic construct
  source 1..28: mol_type = other DNA
tcccattggctccctgtgttctcttggg

SEQ ID NO: 37834 - DNA, 28 bp, synthetic construct
  source 1..28: mol_type = other DNA
ttcccattggctccctgtgttctcttgg

SEQ ID NO: 37835 - DNA, 28 bp, synthetic construct
  source 1..28: mol_type = other DNA
acagggagccaatgggaatcttatttgg

SEQ ID NO: 37836 - DNA, 28 bp, synthetic construct
  source 1..28: mol_type = other DNA
tttagctgccaaataagattcccattgg

SEQ ID NO: 37837 - DNA, 28 bp, synthetic construct
  source 1..28: mol_type = other DNA
tcttatttggcagctaaatacaaactgg

SEQ ID NO: 37838 - DNA, 28 bp, synthetic construct
  source 1..28: mol_type = other DNA
cttatttggcagctaaatacaaactggg

SEQ ID NO: 37839 - DNA, 28 bp, synthetic construct
  source 1..28: mol_type = other DNA
ttatttggcagctaaatacaaactgggg

SEQ ID NO: 37840 - DNA, 28 bp, synthetic construct
  source 1..28: mol_type = other DNA
tggcagctaaatacaaactggggattgg

SEQ ID NO: 37841 - DNA, 28 bp, synthetic construct
  source 1..28: mol_type = other DNA
cagctaaatacaaactggggattggagg

SEQ ID NO: 37842 - DNA, 28 bp, synthetic construct
  source 1..28: mol_type = other DNA
tacaaactggggattggaggaagaaagg

SEQ ID NO: 37843 - DNA, 28 bp, synthetic construct
  source 1..28: mol_type = other DNA
aaactggggattggaggaagaaaggagg

SEQ ID NO: 37844 - DNA, 28 bp, synthetic construct
  source 1..28: mol_type = other DNA
aactggggattggaggaagaaaggaggg

SEQ ID NO: 37845 - DNA, 28 bp, synthetic construct
  source 1..28: mol_type = other DNA
actggggattggaggaagaaaggagggg

SEQ ID NO: 37846 - DNA, 28 bp, synthetic construct
  source 1..28: mol_type = other DNA
attggaggaagaaaggaggggtcacagg

SEQ ID NO: 37847 - DNA, 28 bp, synthetic construct
  source 1..28: mol_type = other DNA
ttggaggaagaaaggaggggtcacaggg

SEQ ID NO: 37848 - DNA, 28 bp, synthetic construct
  source 1..28: mol_type = other DNA
tggaggaagaaaggaggggtcacagggg

SEQ ID NO: 37849 - DNA, 28 bp, synthetic construct
  source 1..28: mol_type = other DNA
aagaaaggaggggtcacaggggccctgg

SEQ ID NO: 37850 - DNA, 28 bp, synthetic construct
  source 1..28: mol_type = other DNA
agaaaggaggggtcacaggggccctggg

SEQ ID NO: 37851 - DNA, 28 bp, synthetic construct
  source 1..28: mol_type = other DNA
caggggtcttgggtgggggagcccaggg

SEQ ID NO: 37852 - DNA, 28 bp, synthetic construct
  source 1..28: mol_type = other DNA
cctgggctcccccacccaagacccctgg

SEQ ID NO: 37853 - DNA, 28 bp, synthetic construct
  source 1..28: mol_type = other DNA
gggctcccccacccaagacccctggagg

SEQ ID NO: 37854 - DNA, 28 bp, synthetic construct
  source 1..28: mol_type = other DNA
tcccccacccaagacccctggaggaagg

SEQ ID NO: 37855 - DNA, 28 bp, synthetic construct
  source 1..28: mol_type = other DNA
cccttcctccaggggtcttgggtggggg

SEQ ID NO: 37856 - DNA, 28 bp, synthetic construct
  source 1..28: mol_type = other DNA
ccccacccaagacccctggaggaagggg

SEQ ID NO: 37857 - DNA, 28 bp, synthetic construct
  source 1..28: mol_type = other DNA
accccttcctccaggggtcttgggtggg

SEQ ID NO: 37858 - DNA, 28 bp, synthetic construct
  source 1..28: mol_type = other DNA
gaccccttcctccaggggtcttgggtgg

SEQ ID NO: 37859 - DNA, 28 bp, synthetic construct
  source 1..28: mol_type = other DNA
attgaccccttcctccaggggtcttggg

SEQ ID NO: 37860 - DNA, 28 bp, synthetic construct
  source 1..28: mol_type = other DNA
aattgaccccttcctccaggggtcttgg

SEQ ID NO: 37861 - DNA, 28 bp, synthetic construct
  source 1..28: mol_type = other DNA
ccgtggaattgaccccttcctccagggg

SEQ ID NO: 37862 - DNA, 28 bp, synthetic construct
  source 1..28: mol_type = other DNA
accgtggaattgaccccttcctccaggg

SEQ ID NO: 37863 - DNA, 28 bp, synthetic construct
  source 1..28: mol_type = other DNA
caccgtggaattgaccccttcctccagg

SEQ ID NO: 37864 - DNA, 28 bp, synthetic construct
  source 1..28: mol_type = other DNA
tatttattagcttttgtttacaccgtgg

SEQ ID NO: 37865 - DNA, 28 bp, synthetic construct
  source 1..28: mol_type = other DNA
taaacaaaagctaataaataaatagagg

SEQ ID NO: 37866 - DNA, 28 bp, synthetic construct
  source 1..28: mol_type = other DNA
ctaataaataaatagaggcttcctctgg

SEQ ID NO: 37867 - DNA, 28 bp, synthetic construct
  source 1..28: mol_type = other DNA
taataaataaatagaggcttcctctggg

SEQ ID NO: 37868 - DNA, 28 bp, synthetic construct
  source 1..28: mol_type = other DNA
aataaatagaggcttcctctgggtcagg

SEQ ID NO: 37869 - DNA, 28 bp, synthetic construct
  source 1..28: mol_type = other DNA
ataaatagaggcttcctctgggtcaggg

SEQ ID NO: 37870 - DNA, 28 bp, synthetic construct
  source 1..28: mol_type = other DNA
aatagaggcttcctctgggtcagggcgg

SEQ ID NO: 37871 - DNA, 28 bp, synthetic construct
  source 1..28: mol_type = other DNA
atagaggcttcctctgggtcagggcggg

SEQ ID NO: 37872 - DNA, 28 bp, synthetic construct
  source 1..28: mol_type = other DNA
cttagctgatcccgccctgacccagagg

SEQ ID NO: 37873 - DNA, 28 bp, synthetic construct
  source 1..28: mol_type = other DNA
tcagctaagcagcatcccccctccctgg

SEQ ID NO: 37874 - DNA, 28 bp, synthetic construct
  source 1..28: mol_type = other DNA
cagctaagcagcatcccccctccctggg

SEQ ID NO: 37875 - DNA, 28 bp, synthetic construct
  source 1..28: mol_type = other DNA
cccccctccctgggccaagctgctctgg

SEQ ID NO: 37876 - DNA, 28 bp, synthetic construct
  source 1..28: mol_type = other DNA
ccccctccctgggccaagctgctctggg

SEQ ID NO: 37877 - DNA, 28 bp, synthetic construct
  source 1..28: mol_type = other DNA
cccctccctgggccaagctgctctgggg

SEQ ID NO: 37878 - DNA, 28 bp, synthetic construct
  source 1..28: mol_type = other DNA
tccccagagcagcttggcccagggaggg

SEQ ID NO: 37879 - DNA, 28 bp, synthetic construct
  source 1..28: mol_type = other DNA
ctccccagagcagcttggcccagggagg

SEQ ID NO: 37880 - DNA, 28 bp, synthetic construct
  source 1..28: mol_type = other DNA
ttactccccagagcagcttggcccaggg

SEQ ID NO: 37881 - DNA, 28 bp, synthetic construct
  source 1..28: mol_type = other DNA
tttactccccagagcagcttggcccagg

SEQ ID NO: 37882 - DNA, 28 bp, synthetic construct
  source 1..28: mol_type = other DNA
tgggccaagctgctctggggagtaaagg

SEQ ID NO: 37883 - DNA, 28 bp, synthetic construct
  source 1..28: mol_type = other DNA
gggccaagctgctctggggagtaaaggg

SEQ ID NO: 37884 - DNA, 28 bp, synthetic construct
  source 1..28: mol_type = other DNA
ccaccctttactccccagagcagcttgg

SEQ ID NO: 37885 - DNA, 28 bp, synthetic construct
  source 1..28: mol_type = other DNA
gctgctctggggagtaaagggtggaagg

SEQ ID NO: 37886 - DNA, 28 bp, synthetic construct
  source 1..28: mol_type = other DNA
tggggagtaaagggtggaaggcactagg

SEQ ID NO: 37887 - DNA, 28 bp, synthetic construct
  source 1..28: mol_type = other DNA
ggggagtaaagggtggaaggcactaggg

SEQ ID NO: 37888 - DNA, 28 bp, synthetic construct
  source 1..28: mol_type = other DNA
aaagggtggaaggcactagggagagagg

SEQ ID NO: 37889 - DNA, 28 bp, synthetic construct
  source 1..28: mol_type = other DNA
aagggtggaaggcactagggagagaggg

SEQ ID NO: 37890 - DNA, 28 bp, synthetic construct
  source 1..28: mol_type = other DNA
aggcactagggagagagggatcccctgg

SEQ ID NO: 37891 - DNA, 28 bp, synthetic construct
  source 1..28: mol_type = other DNA
ggatcccctggcccctctgtagtgtagg

SEQ ID NO: 37892 - DNA, 28 bp, synthetic construct
  source 1..28: mol_type = other DNA
tcccctggcccctctgtagtgtaggagg

SEQ ID NO: 37893 - DNA, 28 bp, synthetic construct
  source 1..28: mol_type = other DNA
cccctggcccctctgtagtgtaggaggg

SEQ ID NO: 37894 - DNA, 28 bp, synthetic construct
  source 1..28: mol_type = other DNA
accctcctacactacagaggggccaggg

SEQ ID NO: 37895 - DNA, 28 bp, synthetic construct
  source 1..28: mol_type = other DNA
gaccctcctacactacagaggggccagg

SEQ ID NO: 37896 - DNA, 28 bp, synthetic construct
  source 1..28: mol_type = other DNA
gcagggaccctcctacactacagagggg

SEQ ID NO: 37897 - DNA, 28 bp, synthetic construct
  source 1..28: mol_type = other DNA
ggcagggaccctcctacactacagaggg

SEQ ID NO: 37898 - DNA, 28 bp, synthetic construct
  source 1..28: mol_type = other DNA
gggcagggaccctcctacactacagagg

SEQ ID NO: 37899 - DNA, 28 bp, synthetic construct
  source 1..28: mol_type = other DNA
tagtgtaggagggtccctgccccaatgg

SEQ ID NO: 37900 - DNA, 28 bp, synthetic construct
  source 1..28: mol_type = other DNA
agggtccctgccccaatggctgagatgg

SEQ ID NO: 37901 - DNA, 28 bp, synthetic construct
  source 1..28: mol_type = other DNA
gtccctgccccaatggctgagatggagg

SEQ ID NO: 37902 - DNA, 28 bp, synthetic construct
  source 1..28: mol_type = other DNA
tccctgccccaatggctgagatggaggg

SEQ ID NO: 37903 - DNA, 28 bp, synthetic construct
  source 1..28: mol_type = other DNA
gccctccatctcagccattggggcaggg

SEQ ID NO: 37904 - DNA, 28 bp, synthetic construct
  source 1..28: mol_type = other DNA
tgccctccatctcagccattggggcagg

SEQ ID NO: 37905 - DNA, 28 bp, synthetic construct
  source 1..28: mol_type = other DNA
tgccccaatggctgagatggagggcagg

SEQ ID NO: 37906 - DNA, 28 bp, synthetic construct
  source 1..28: mol_type = other DNA
ctcctgccctccatctcagccattgggg

SEQ ID NO: 37907 - DNA, 28 bp, synthetic construct
  source 1..28: mol_type = other DNA
cctcctgccctccatctcagccattggg

SEQ ID NO: 37908 - DNA, 28 bp, synthetic construct
  source 1..28: mol_type = other DNA
tcctcctgccctccatctcagccattgg

SEQ ID NO: 37909 - DNA, 28 bp, synthetic construct
  source 1..28: mol_type = other DNA
tgagatggagggcaggaggagcccaagg

SEQ ID NO: 37910 - DNA, 28 bp, synthetic construct
  source 1..28: mol_type = other DNA
gcaggaggagcccaaggcacatgacagg

SEQ ID NO: 37911 - DNA, 28 bp, synthetic construct
  source 1..28: mol_type = other DNA
caggaggagcccaaggcacatgacaggg

SEQ ID NO: 37912 - DNA, 28 bp, synthetic construct
  source 1..28: mol_type = other DNA
aggagcccaaggcacatgacagggctgg

SEQ ID NO: 37913 - DNA, 28 bp, synthetic construct
  source 1..28: mol_type = other DNA
ggagcccaaggcacatgacagggctggg

SEQ ID NO: 37914 - DNA, 28 bp, synthetic construct
  source 1..28: mol_type = other DNA
gagcccaaggcacatgacagggctgggg

SEQ ID NO: 37915 - DNA, 28 bp, synthetic construct
  source 1..28: mol_type = other DNA
agcccaaggcacatgacagggctggggg

SEQ ID NO: 37916 - DNA, 28 bp, synthetic construct
  source 1..28: mol_type = other DNA
ctcccccagccctgtcatgtgccttggg

SEQ ID NO: 37917 - DNA, 28 bp, synthetic construct
  source 1..28: mol_type = other DNA
ccaaggcacatgacagggctgggggagg

SEQ ID NO: 37918 - DNA, 28 bp, synthetic construct
  source 1..28: mol_type = other DNA
caaggcacatgacagggctgggggaggg

SEQ ID NO: 37919 - DNA, 28 bp, synthetic construct
  source 1..28: mol_type = other DNA
acagggctgggggagggacttataacgg

SEQ ID NO: 37920 - DNA, 28 bp, synthetic construct
  source 1..28: mol_type = other DNA
gggctgggggagggacttataacggagg

SEQ ID NO: 37921 - DNA, 28 bp, synthetic construct
  source 1..28: mol_type = other DNA
ggctgggggagggacttataacggaggg

SEQ ID NO: 37922 - DNA, 28 bp, synthetic construct
  source 1..28: mol_type = other DNA
gggagggacttataacggagggcacagg

SEQ ID NO: 37923 - DNA, 28 bp, synthetic construct
  source 1..28: mol_type = other DNA
ggagggacttataacggagggcacaggg

SEQ ID NO: 37924 - DNA, 28 bp, synthetic construct
  source 1..28: mol_type = other DNA
gggtgaactctgcacccgagccaagagg

SEQ ID NO: 37925 - DNA, 28 bp, synthetic construct
  source 1..28: mol_type = other DNA
tgcacccgagccaagaggtgcagaatgg

SEQ ID NO: 37926 - DNA, 28 bp, synthetic construct
  source 1..28: mol_type = other DNA
aggtccattctgcacctcttggctcggg

SEQ ID NO: 37927 - DNA, 28 bp, synthetic construct
  source 1..28: mol_type = other DNA
caggtccattctgcacctcttggctcgg

SEQ ID NO: 37928 - DNA, 28 bp, synthetic construct
  source 1..28: mol_type = other DNA
agatgcaggtccattctgcacctcttgg

SEQ ID NO: 37929 - DNA, 28 bp, synthetic construct
  source 1..28: mol_type = other DNA
gagggtgaaagggacagatagatgcagg

SEQ ID NO: 37930 - DNA, 28 bp, synthetic construct
  source 1..28: mol_type = other DNA
tctggggcaggaacagagggtgaaaggg

SEQ ID NO: 37931 - DNA, 28 bp, synthetic construct
  source 1..28: mol_type = other DNA
ttctggggcaggaacagagggtgaaagg

SEQ ID NO: 37932 - DNA, 28 bp, synthetic construct
  source 1..28: mol_type = other DNA
ccctctgttcctgccccagaaatgcagg

SEQ ID NO: 37933 - DNA, 28 bp, synthetic construct
  source 1..28: mol_type = other DNA
cctctgttcctgccccagaaatgcaggg

SEQ ID NO: 37934 - DNA, 28 bp, synthetic construct
  source 1..28: mol_type = other DNA
aggctgggccctgcatttctggggcagg

SEQ ID NO: 37935 - DNA, 28 bp, synthetic construct
  source 1..28: mol_type = other DNA
gggcaggctgggccctgcatttctgggg

SEQ ID NO: 37936 - DNA, 28 bp, synthetic construct
  source 1..28: mol_type = other DNA
ggggcaggctgggccctgcatttctggg

SEQ ID NO: 37937 - DNA, 28 bp, synthetic construct
  source 1..28: mol_type = other DNA
gggggcaggctgggccctgcatttctgg

SEQ ID NO: 37938 - DNA, 28 bp, synthetic construct
  source 1..28: mol_type = other DNA
ggcccagcctgcccccaccttgacctgg

SEQ ID NO: 37939 - DNA, 28 bp, synthetic construct
  source 1..28: mol_type = other DNA
tgccaggtcaaggtgggggcaggctggg

SEQ ID NO: 37940 - DNA, 28 bp, synthetic construct
  source 1..28: mol_type = other DNA
gtgccaggtcaaggtgggggcaggctgg

SEQ ID NO: 37941 - DNA, 28 bp, synthetic construct
  source 1..28: mol_type = other DNA
ccttgtgccaggtcaaggtgggggcagg

SEQ ID NO: 37942 - DNA, 28 bp, synthetic construct
  source 1..28: mol_type = other DNA
ccgtccttgtgccaggtcaaggtggggg

SEQ ID NO: 37943 - DNA, 28 bp, synthetic construct
  source 1..28: mol_type = other DNA
cccgtccttgtgccaggtcaaggtgggg

SEQ ID NO: 37944 - DNA, 28 bp, synthetic construct
  source 1..28: mol_type = other DNA
cccaccttgacctggcacaaggacgggg

SEQ ID NO: 37945 - DNA, 28 bp, synthetic construct
  source 1..28: mol_type = other DNA
gccccgtccttgtgccaggtcaaggtgg

SEQ ID NO: 37946 - DNA, 28 bp, synthetic construct
  source 1..28: mol_type = other DNA
tgtgccccgtccttgtgccaggtcaagg

SEQ ID NO: 37947 - DNA, 28 bp, synthetic construct
  source 1..28: mol_type = other DNA
gacctggcacaaggacggggcacagagg

SEQ ID NO: 37948 - DNA, 28 bp, synthetic construct
  source 1..28: mol_type = other DNA
agcctctgtgccccgtccttgtgccagg

SEQ ID NO: 37949 - DNA, 28 bp, synthetic construct
  source 1..28: mol_type = other DNA
gcacagaggctagcacacaccctgcagg

SEQ ID NO: 37950 - DNA, 28 bp, synthetic construct
  source 1..28: mol_type = other DNA
cctaatgctgtgtgatgcacctgcaggg

SEQ ID NO: 37951 - DNA, 28 bp, synthetic construct
  source 1..28: mol_type = other DNA
gcctaatgctgtgtgatgcacctgcagg

SEQ ID NO: 37952 - DNA, 28 bp, synthetic construct
  source 1..28: mol_type = other DNA
gtgcatcacacagcattaggcaccaagg

SEQ ID NO: 37953 - DNA, 28 bp, synthetic construct
  source 1..28: mol_type = other DNA
tgcatcacacagcattaggcaccaaggg

SEQ ID NO: 37954 - DNA, 28 bp, synthetic construct
  source 1..28: mol_type = other DNA
tcacacagcattaggcaccaagggtagg

SEQ ID NO: 37955 - DNA, 28 bp, synthetic construct
  source 1..28: mol_type = other DNA
ttaggcaccaagggtaggagcaagaagg

SEQ ID NO: 37956 - DNA, 28 bp, synthetic construct
  source 1..28: mol_type = other DNA
ggcaccaagggtaggagcaagaaggtgg

SEQ ID NO: 37957 - DNA, 28 bp, synthetic construct
  source 1..28: mol_type = other DNA
gcaccaagggtaggagcaagaaggtggg

SEQ ID NO: 37958 - DNA, 28 bp, synthetic construct
  source 1..28: mol_type = other DNA
gagcccaccttcttgctcctacccttgg

SEQ ID NO: 37959 - DNA, 28 bp, synthetic construct
  source 1..28: mol_type = other DNA
cagcccttctcctttgtcccctttttgg

SEQ ID NO: 37960 - DNA, 28 bp, synthetic construct
  source 1..28: mol_type = other DNA
agaccaaaaaggggacaaaggagaaggg

SEQ ID NO: 37961 - DNA, 28 bp, synthetic construct
  source 1..28: mol_type = other DNA
gagaccaaaaaggggacaaaggagaagg

SEQ ID NO: 37962 - DNA, 28 bp, synthetic construct
  source 1..28: mol_type = other DNA
acactagagaccaaaaaggggacaaagg

SEQ ID NO: 37963 - DNA, 28 bp, synthetic construct
  source 1..28: mol_type = other DNA
aacaggaacactagagaccaaaaagggg

SEQ ID NO: 37964 - DNA, 28 bp, synthetic construct
  source 1..28: mol_type = other DNA
aaacaggaacactagagaccaaaaaggg

SEQ ID NO: 37965 - DNA, 28 bp, synthetic construct
  source 1..28: mol_type = other DNA
caaacaggaacactagagaccaaaaagg

SEQ ID NO: 37966 - DNA, 28 bp, synthetic construct
  source 1..28: mol_type = other DNA
ggtgcttggctctctgagagcaaacagg

SEQ ID NO: 37967 - DNA, 28 bp, synthetic construct
  source 1..28: mol_type = other DNA
gtttgctctcagagagccaagcacctgg

SEQ ID NO: 37968 - DNA, 28 bp, synthetic construct
  source 1..28: mol_type = other DNA
tctcagagagccaagcacctggcagagg

SEQ ID NO: 37969 - DNA, 28 bp, synthetic construct
  source 1..28: mol_type = other DNA
agagagccaagcacctggcagaggaagg

SEQ ID NO: 37970 - DNA, 28 bp, synthetic construct
  source 1..28: mol_type = other DNA
gagagccaagcacctggcagaggaaggg

SEQ ID NO: 37971 - DNA, 28 bp, synthetic construct
  source 1..28: mol_type = other DNA
agagccaagcacctggcagaggaagggg

SEQ ID NO: 37972 - DNA, 28 bp, synthetic construct
  source 1..28: mol_type = other DNA
acagccccttcctctgccaggtgcttgg

SEQ ID NO: 37973 - DNA, 28 bp, synthetic construct
  source 1..28: mol_type = other DNA
aagcacctggcagaggaaggggctgtgg

SEQ ID NO: 37974 - DNA, 28 bp, synthetic construct
  source 1..28: mol_type = other DNA
ccattccacagccccttcctctgccagg

SEQ ID NO: 37975 - DNA, 28 bp, synthetic construct
  source 1..28: mol_type = other DNA
gcagaggaaggggctgtggaatggcagg

SEQ ID NO: 37976 - DNA, 28 bp, synthetic construct
  source 1..28: mol_type = other DNA
cagaggaaggggctgtggaatggcaggg

SEQ ID NO: 37977 - DNA, 28 bp, synthetic construct
  source 1..28: mol_type = other DNA
gaatggcagggtcttcctcttgccctgg

SEQ ID NO: 37978 - DNA, 28 bp, synthetic construct
  source 1..28: mol_type = other DNA
aatggcagggtcttcctcttgccctggg

SEQ ID NO: 37979 - DNA, 28 bp, synthetic construct
  source 1..28: mol_type = other DNA
gtcttcctcttgccctgggaagtctagg

SEQ ID NO: 37980 - DNA, 28 bp, synthetic construct
  source 1..28: mol_type = other DNA
tgggtcctagacttcccagggcaagagg

SEQ ID NO: 37981 - DNA, 28 bp, synthetic construct
  source 1..28: mol_type = other DNA
cttgccctgggaagtctaggacccatgg

SEQ ID NO: 37982 - DNA, 28 bp, synthetic construct
  source 1..28: mol_type = other DNA
ttgccctgggaagtctaggacccatggg

SEQ ID NO: 37983 - DNA, 28 bp, synthetic construct
  source 1..28: mol_type = other DNA
tgccctgggaagtctaggacccatgggg

SEQ ID NO: 37984 - DNA, 28 bp, synthetic construct
  source 1..28: mol_type = other DNA
tgccccatgggtcctagacttcccaggg

SEQ ID NO: 37985 - DNA, 28 bp, synthetic construct
  source 1..28: mol_type = other DNA
ctgccccatgggtcctagacttcccagg

SEQ ID NO: 37986 - DNA, 28 bp, synthetic construct
  source 1..28: mol_type = other DNA
ctctaaaatctcagcactgccccatggg

SEQ ID NO: 37987 - DNA, 28 bp, synthetic construct
  source 1..28: mol_type = other DNA
actctaaaatctcagcactgccccatgg

SEQ ID NO: 37988 - DNA, 28 bp, synthetic construct
  source 1..28: mol_type = other DNA
tgctgagattttagagtccaaacccagg

SEQ ID NO: 37989 - DNA, 28 bp, synthetic construct
  source 1..28: mol_type = other DNA
gagggcaaagggatgagcctgggtttgg

SEQ ID NO: 37990 - DNA, 28 bp, synthetic construct
  source 1..28: mol_type = other DNA
ggagagagggcaaagggatgagcctggg

SEQ ID NO: 37991 - DNA, 28 bp, synthetic construct
  source 1..28: mol_type = other DNA
aggagagagggcaaagggatgagcctgg

SEQ ID NO: 37992 - DNA, 28 bp, synthetic construct
  source 1..28: mol_type = other DNA
aggctcatccctttgccctctctcctgg

SEQ ID NO: 37993 - DNA, 28 bp, synthetic construct
  source 1..28: mol_type = other DNA
ctcatccctttgccctctctcctggtgg

SEQ ID NO: 37994 - DNA, 28 bp, synthetic construct
  source 1..28: mol_type = other DNA
tcatccctttgccctctctcctggtggg

SEQ ID NO: 37995 - DNA, 28 bp, synthetic construct
  source 1..28: mol_type = other DNA
tgctcccaccaggagagagggcaaaggg

SEQ ID NO: 37996 - DNA, 28 bp, synthetic construct
  source 1..28: mol_type = other DNA
ctgctcccaccaggagagagggcaaagg

SEQ ID NO: 37997 - DNA, 28 bp, synthetic construct
  source 1..28: mol_type = other DNA
ctttgccctctctcctggtgggagcagg

SEQ ID NO: 37998 - DNA, 28 bp, synthetic construct
  source 1..28: mol_type = other DNA
tttgccctctctcctggtgggagcaggg

SEQ ID NO: 37999 - DNA, 28 bp, synthetic construct
  source 1..28: mol_type = other DNA
cctgccctgctcccaccaggagagaggg

SEQ ID NO: 38000 - DNA, 28 bp, synthetic construct
  source 1..28: mol_type = other DNA
gcctgccctgctcccaccaggagagagg

SEQ ID NO: 38001 - DNA, 28 bp, synthetic construct
  source 1..28: mol_type = other DNA
tcctggtgggagcagggcaggcccccgg

SEQ ID NO: 38002 - DNA, 28 bp, synthetic construct
  source 1..28: mol_type = other DNA
cctggtgggagcagggcaggcccccggg

SEQ ID NO: 38003 - DNA, 28 bp, synthetic construct
  source 1..28: mol_type = other DNA
tgggagcagggcaggcccccgggactgg

SEQ ID NO: 38004 - DNA, 28 bp, synthetic construct
  source 1..28: mol_type = other DNA
gcagggcaggcccccgggactggcgagg

SEQ ID NO: 38005 - DNA, 28 bp, synthetic construct
  source 1..28: mol_type = other DNA
cagggcaggcccccgggactggcgaggg

SEQ ID NO: 38006 - DNA, 28 bp, synthetic construct
  source 1..28: mol_type = other DNA
aggcccccgggactggcgagggagccgg

SEQ ID NO: 38007 - DNA, 28 bp, synthetic construct
  source 1..28: mol_type = other DNA
taaccggctccctcgccagtcccggggg

SEQ ID NO: 38008 - DNA, 28 bp, synthetic construct
  source 1..28: mol_type = other DNA
ctaaccggctccctcgccagtcccgggg

SEQ ID NO: 38009 - DNA, 28 bp, synthetic construct
  source 1..28: mol_type = other DNA
tctaaccggctccctcgccagtcccggg

SEQ ID NO: 38010 - DNA, 28 bp, synthetic construct
  source 1..28: mol_type = other DNA
atctaaccggctccctcgccagtcccgg

SEQ ID NO: 38011 - DNA, 28 bp, synthetic construct
  source 1..28: mol_type = other DNA
gactggcgagggagccggttagatcagg

SEQ ID NO: 38012 - DNA, 28 bp, synthetic construct
  source 1..28: mol_type = other DNA
ggcgagggagccggttagatcaggaagg

SEQ ID NO: 38013 - DNA, 28 bp, synthetic construct
  source 1..28: mol_type = other DNA
gcgagggagccggttagatcaggaaggg

SEQ ID NO: 38014 - DNA, 28 bp, synthetic construct
  source 1..28: mol_type = other DNA
cgagggagccggttagatcaggaagggg

SEQ ID NO: 38015 - DNA, 28 bp, synthetic construct
  source 1..28: mol_type = other DNA
gtgttcatccccttcctgatctaaccgg

SEQ ID NO: 38016 - DNA, 28 bp, synthetic construct
  source 1..28: mol_type = other DNA
tagatcaggaaggggatgaacacagagg

SEQ ID NO: 38017 - DNA, 28 bp, synthetic construct
  source 1..28: mol_type = other DNA
aacacagaggcacccctagaaactttgg

SEQ ID NO: 38018 - DNA, 28 bp, synthetic construct
  source 1..28: mol_type = other DNA
acccctagaaactttggcaaaaacaagg

SEQ ID NO: 38019 - DNA, 28 bp, synthetic construct
  source 1..28: mol_type = other DNA
tccttgtttttgccaaagtttctagggg

SEQ ID NO: 38020 - DNA, 28 bp, synthetic construct
  source 1..28: mol_type = other DNA
ctccttgtttttgccaaagtttctaggg

SEQ ID NO: 38021 - DNA, 28 bp, synthetic construct
  source 1..28: mol_type = other DNA
gctccttgtttttgccaaagtttctagg

SEQ ID NO: 38022 - DNA, 28 bp, synthetic construct
  source 1..28: mol_type = other DNA
actttggcaaaaacaaggagctcattgg

SEQ ID NO: 38023 - DNA, 28 bp, synthetic construct
  source 1..28: mol_type = other DNA
tggcaaaaacaaggagctcattggaagg

SEQ ID NO: 38024 - DNA, 28 bp, synthetic construct
  source 1..28: mol_type = other DNA
ggcaaaaacaaggagctcattggaaggg

SEQ ID NO: 38025 - DNA, 28 bp, synthetic construct
  source 1..28: mol_type = other DNA
gcaaaaacaaggagctcattggaagggg

SEQ ID NO: 38026 - DNA, 28 bp, synthetic construct
  source 1..28: mol_type = other DNA
aaaacaaggagctcattggaaggggtgg

SEQ ID NO: 38027 - DNA, 28 bp, synthetic construct
  source 1..28: mol_type = other DNA
aaacaaggagctcattggaaggggtggg

SEQ ID NO: 38028 - DNA, 28 bp, synthetic construct
  source 1..28: mol_type = other DNA
aacaaggagctcattggaaggggtgggg

SEQ ID NO: 38029 - DNA, 28 bp, synthetic construct
  source 1..28: mol_type = other DNA
ggagctcattggaaggggtggggagagg

SEQ ID NO: 38030 - DNA, 28 bp, synthetic construct
  source 1..28: mol_type = other DNA
gagctcattggaaggggtggggagaggg

SEQ ID NO: 38031 - DNA, 28 bp, synthetic construct
  source 1..28: mol_type = other DNA
ggaaggggtggggagagggcagagcagg

SEQ ID NO: 38032 - DNA, 28 bp, synthetic construct
  source 1..28: mol_type = other DNA
gcagagcaggtcctcccccagtcactgg

SEQ ID NO: 38033 - DNA, 28 bp, synthetic construct
  source 1..28: mol_type = other DNA
gagcaggtcctcccccagtcactggcgg

SEQ ID NO: 38034 - DNA, 28 bp, synthetic construct
  source 1..28: mol_type = other DNA
ggtcctcccccagtcactggcggtctgg

SEQ ID NO: 38035 - DNA, 28 bp, synthetic construct
  source 1..28: mol_type = other DNA
gtcctcccccagtcactggcggtctggg

SEQ ID NO: 38036 - DNA, 28 bp, synthetic construct
  source 1..28: mol_type = other DNA
ctcccagaccgccagtgactgggggagg

SEQ ID NO: 38037 - DNA, 28 bp, synthetic construct
  source 1..28: mol_type = other DNA
catctcccagaccgccagtgactggggg

SEQ ID NO: 38038 - DNA, 28 bp, synthetic construct
  source 1..28: mol_type = other DNA
ccccagtcactggcggtctgggagatgg

SEQ ID NO: 38039 - DNA, 28 bp, synthetic construct
  source 1..28: mol_type = other DNA
accatctcccagaccgccagtgactggg

SEQ ID NO: 38040 - DNA, 28 bp, synthetic construct
  source 1..28: mol_type = other DNA
gaccatctcccagaccgccagtgactgg

SEQ ID NO: 38041 - DNA, 28 bp, synthetic construct
  source 1..28: mol_type = other DNA
ctgcctgaagccccaacccccacagcgg

SEQ ID NO: 38042 - DNA, 28 bp, synthetic construct
  source 1..28: mol_type = other DNA
tgcctgaagccccaacccccacagcggg

SEQ ID NO: 38043 - DNA, 28 bp, synthetic construct
  source 1..28: mol_type = other DNA
gcctgaagccccaacccccacagcgggg

SEQ ID NO: 38044 - DNA, 28 bp, synthetic construct
  source 1..28: mol_type = other DNA
tccccgctgtgggggttggggcttcagg

SEQ ID NO: 38045 - DNA, 28 bp, synthetic construct
  source 1..28: mol_type = other DNA
tgaagccccaacccccacagcggggagg

SEQ ID NO: 38046 - DNA, 28 bp, synthetic construct
  source 1..28: mol_type = other DNA
cctgacctccccgctgtgggggttgggg

SEQ ID NO: 38047 - DNA, 28 bp, synthetic construct
  source 1..28: mol_type = other DNA
cccaacccccacagcggggaggtcaggg

SEQ ID NO: 38048 - DNA, 28 bp, synthetic construct
  source 1..28: mol_type = other DNA
cccctgacctccccgctgtgggggttgg

SEQ ID NO: 38049 - DNA, 28 bp, synthetic construct
  source 1..28: mol_type = other DNA
agggcccctgacctccccgctgtggggg

SEQ ID NO: 38050 - DNA, 28 bp, synthetic construct
  source 1..28: mol_type = other DNA
cagggcccctgacctccccgctgtgggg

SEQ ID NO: 38051 - DNA, 28 bp, synthetic construct
  source 1..28: mol_type = other DNA
ccagggcccctgacctccccgctgtggg

SEQ ID NO: 38052 - DNA, 28 bp, synthetic construct
  source 1..28: mol_type = other DNA
accagggcccctgacctccccgctgtgg

SEQ ID NO: 38053 - DNA, 28 bp, synthetic construct
  source 1..28: mol_type = other DNA
agcggggaggtcaggggccctggtcagg

SEQ ID NO: 38054 - DNA, 28 bp, synthetic construct
  source 1..28: mol_type = other DNA
gggaggtcaggggccctggtcaggctgg

SEQ ID NO: 38055 - DNA, 28 bp, synthetic construct
  source 1..28: mol_type = other DNA
ggaggtcaggggccctggtcaggctggg

SEQ ID NO: 38056 - DNA, 28 bp, synthetic construct
  source 1..28: mol_type = other DNA
gaggtcaggggccctggtcaggctgggg

SEQ ID NO: 38057 - DNA, 28 bp, synthetic construct
  source 1..28: mol_type = other DNA
gggccctggtcaggctggggacttcagg

SEQ ID NO: 38058 - DNA, 28 bp, synthetic construct
  source 1..28: mol_type = other DNA
gggcctgaagtccccagcctgaccaggg

SEQ ID NO: 38059 - DNA, 28 bp, synthetic construct
  source 1..28: mol_type = other DNA
ggggcctgaagtccccagcctgaccagg

SEQ ID NO: 38060 - DNA, 28 bp, synthetic construct
  source 1..28: mol_type = other DNA
tggggacttcaggccccctttgccctgg

SEQ ID NO: 38061 - DNA, 28 bp, synthetic construct
  source 1..28: mol_type = other DNA
tcaggccccctttgccctggcccccagg

SEQ ID NO: 38062 - DNA, 28 bp, synthetic construct
  source 1..28: mol_type = other DNA
aggttcctgggggccagggcaaaggggg

SEQ ID NO: 38063 - DNA, 28 bp, synthetic construct
  source 1..28: mol_type = other DNA
gaggttcctgggggccagggcaaagggg

SEQ ID NO: 38064 - DNA, 28 bp, synthetic construct
  source 1..28: mol_type = other DNA
tgaggttcctgggggccagggcaaaggg

SEQ ID NO: 38065 - DNA, 28 bp, synthetic construct
  source 1..28: mol_type = other DNA
atgaggttcctgggggccagggcaaagg

SEQ ID NO: 38066 - DNA, 28 bp, synthetic construct
  source 1..28: mol_type = other DNA
gcgaggatgaggttcctgggggccaggg

SEQ ID NO: 38067 - DNA, 28 bp, synthetic construct
  source 1..28: mol_type = other DNA
agcgaggatgaggttcctgggggccagg

SEQ ID NO: 38068 - DNA, 28 bp, synthetic construct
  source 1..28: mol_type = other DNA
cctctagcgaggatgaggttcctggggg

SEQ ID NO: 38069 - DNA, 28 bp, synthetic construct
  source 1..28: mol_type = other DNA
gcctctagcgaggatgaggttcctgggg

SEQ ID NO: 38070 - DNA, 28 bp, synthetic construct
  source 1..28: mol_type = other DNA
tgcctctagcgaggatgaggttcctggg

SEQ ID NO: 38071 - DNA, 28 bp, synthetic construct
  source 1..28: mol_type = other DNA
atgcctctagcgaggatgaggttcctgg

SEQ ID NO: 38072 - DNA, 28 bp, synthetic construct
  source 1..28: mol_type = other DNA
ggaacctcatcctcgctagaggcattgg

SEQ ID NO: 38073 - DNA, 28 bp, synthetic construct
  source 1..28: mol_type = other DNA
gaacctcatcctcgctagaggcattggg

SEQ ID NO: 38074 - DNA, 28 bp, synthetic construct
  source 1..28: mol_type = other DNA
aacctcatcctcgctagaggcattgggg

SEQ ID NO: 38075 - DNA, 28 bp, synthetic construct
  source 1..28: mol_type = other DNA
caccccaatgcctctagcgaggatgagg

SEQ ID NO: 38076 - DNA, 28 bp, synthetic construct
  source 1..28: mol_type = other DNA
ctcatcctcgctagaggcattggggtgg

SEQ ID NO: 38077 - DNA, 28 bp, synthetic construct
  source 1..28: mol_type = other DNA
tcatcctcgctagaggcattggggtggg

SEQ ID NO: 38078 - DNA, 28 bp, synthetic construct
  source 1..28: mol_type = other DNA
catcctcgctagaggcattggggtgggg

SEQ ID NO: 38079 - DNA, 28 bp, synthetic construct
  source 1..28: mol_type = other DNA
ggtccccaccccaatgcctctagcgagg

SEQ ID NO: 38080 - DNA, 28 bp, synthetic construct
  source 1..28: mol_type = other DNA
cgctagaggcattggggtggggaccagg

SEQ ID NO: 38081 - DNA, 28 bp, synthetic construct
  source 1..28: mol_type = other DNA
gcattggggtggggaccaggctgcgagg

SEQ ID NO: 38082 - DNA, 28 bp, synthetic construct
  source 1..28: mol_type = other DNA
tgtttgaggatgactcctcgcagcctgg

SEQ ID NO: 38083 - DNA, 28 bp, synthetic construct
  source 1..28: mol_type = other DNA
gcgaggagtcatcctcaaacatttcagg

SEQ ID NO: 38084 - DNA, 28 bp, synthetic construct
  source 1..28: mol_type = other DNA
cgaggagtcatcctcaaacatttcaggg

SEQ ID NO: 38085 - DNA, 28 bp, synthetic construct
  source 1..28: mol_type = other DNA
atgctggagaaccctgaaatgtttgagg

SEQ ID NO: 38086 - DNA, 28 bp, synthetic construct
  source 1..28: mol_type = other DNA
catttcagggttctccagcatctctcgg

SEQ ID NO: 38087 - DNA, 28 bp, synthetic construct
  source 1..28: mol_type = other DNA
gggttctccagcatctctcggattaagg

SEQ ID NO: 38088 - DNA, 28 bp, synthetic construct
  source 1..28: mol_type = other DNA
ggttctccagcatctctcggattaaggg

SEQ ID NO: 38089 - DNA, 28 bp, synthetic construct
  source 1..28: mol_type = other DNA
tctccagcatctctcggattaagggagg

SEQ ID NO: 38090 - DNA, 28 bp, synthetic construct
  source 1..28: mol_type = other DNA
atgcctcccttaatccgagagatgctgg

SEQ ID NO: 38091 - DNA, 28 bp, synthetic construct
  source 1..28: mol_type = other DNA
gcatctctcggattaagggaggcatcgg

SEQ ID NO: 38092 - DNA, 28 bp, synthetic construct
  source 1..28: mol_type = other DNA
catctctcggattaagggaggcatcggg

SEQ ID NO: 38093 - DNA, 28 bp, synthetic construct
  source 1..28: mol_type = other DNA
ctcggattaagggaggcatcgggcctgg

SEQ ID NO: 38094 - DNA, 28 bp, synthetic construct
  source 1..28: mol_type = other DNA
cctggaatctccatcttcagagtaatgg

SEQ ID NO: 38095 - DNA, 28 bp, synthetic construct
  source 1..28: mol_type = other DNA
gctgaaagggccattactctgaagatgg

SEQ ID NO: 38096 - DNA, 28 bp, synthetic construct
  source 1..28: mol_type = other DNA
gtaatggccctttcagctcctacaatgg

SEQ ID NO: 38097 - DNA, 28 bp, synthetic construct
  source 1..28: mol_type = other DNA
tctctctccattgtaggagctgaaaggg

SEQ ID NO: 38098 - DNA, 28 bp, synthetic construct
  source 1..28: mol_type = other DNA
ttctctctccattgtaggagctgaaagg

SEQ ID NO: 38099 - DNA, 28 bp, synthetic construct
  source 1..28: mol_type = other DNA
tcctacaatggagagagaaagagagagg

SEQ ID NO: 38100 - DNA, 28 bp, synthetic construct
  source 1..28: mol_type = other DNA
gcctctctctttctctctccattgtagg

SEQ ID NO: 38101 - DNA, 28 bp, synthetic construct
  source 1..28: mol_type = other DNA
aatggagagagaaagagagaggctcagg

SEQ ID NO: 38102 - DNA, 28 bp, synthetic construct
  source 1..28: mol_type = other DNA
ggagagagaaagagagaggctcaggagg

SEQ ID NO: 38103 - DNA, 28 bp, synthetic construct
  source 1..28: mol_type = other DNA
gaaagagagaggctcaggaggacagagg

SEQ ID NO: 38104 - DNA, 28 bp, synthetic construct
  source 1..28: mol_type = other DNA
agaggctcaggaggacagaggcacatgg

SEQ ID NO: 38105 - DNA, 28 bp, synthetic construct
  source 1..28: mol_type = other DNA
ggaggacagaggcacatggcccttaagg

SEQ ID NO: 38106 - DNA, 28 bp, synthetic construct
  source 1..28: mol_type = other DNA
agaaaggttagggagatggccttaaggg

SEQ ID NO: 38107 - DNA, 28 bp, synthetic construct
  source 1..28: mol_type = other DNA
gagaaaggttagggagatggccttaagg

SEQ ID NO: 38108 - DNA, 28 bp, synthetic construct
  source 1..28: mol_type = other DNA
gggcagttgagaaaggttagggagatgg

SEQ ID NO: 38109 - DNA, 28 bp, synthetic construct
  source 1..28: mol_type = other DNA
agtcaggggcagttgagaaaggttaggg

SEQ ID NO: 38110 - DNA, 28 bp, synthetic construct
  source 1..28: mol_type = other DNA
gagtcaggggcagttgagaaaggttagg

SEQ ID NO: 38111 - DNA, 28 bp, synthetic construct
  source 1..28: mol_type = other DNA
taggggagtcaggggcagttgagaaagg

SEQ ID NO: 38112 - DNA, 28 bp, synthetic construct
  source 1..28: mol_type = other DNA
tttctcaactgcccctgactcccctagg

SEQ ID NO: 38113 - DNA, 28 bp, synthetic construct
  source 1..28: mol_type = other DNA
ttctcaactgcccctgactcccctaggg

SEQ ID NO: 38114 - DNA, 28 bp, synthetic construct
  source 1..28: mol_type = other DNA
tctcaactgcccctgactcccctagggg

SEQ ID NO: 38115 - DNA, 28 bp, synthetic construct
  source 1..28: mol_type = other DNA
ctcaactgcccctgactcccctaggggg

SEQ ID NO: 38116 - DNA, 28 bp, synthetic construct
  source 1..28: mol_type = other DNA
gctgggcgccccctaggggagtcagggg

SEQ ID NO: 38117 - DNA, 28 bp, synthetic construct
  source 1..28: mol_type = other DNA
tgctgggcgccccctaggggagtcaggg

SEQ ID NO: 38118 - DNA, 28 bp, synthetic construct
  source 1..28: mol_type = other DNA
gtgctgggcgccccctaggggagtcagg

SEQ ID NO: 38119 - DNA, 28 bp, synthetic construct
  source 1..28: mol_type = other DNA
gactcccctagggggcgcccagcacagg

SEQ ID NO: 38120 - DNA, 28 bp, synthetic construct
  source 1..28: mol_type = other DNA
tgggcctgtgctgggcgccccctagggg

SEQ ID NO: 38121 - DNA, 28 bp, synthetic construct
  source 1..28: mol_type = other DNA
gtgggcctgtgctgggcgccccctaggg

SEQ ID NO: 38122 - DNA, 28 bp, synthetic construct
  source 1..28: mol_type = other DNA
ggtgggcctgtgctgggcgccccctagg

SEQ ID NO: 38123 - DNA, 28 bp, synthetic construct
  source 1..28: mol_type = other DNA
tagttgagaaccaggcaatctacactgg

SEQ ID NO: 38124 - DNA, 28 bp, synthetic construct
  source 1..28: mol_type = other DNA
gacaagaacagagtagttgagaaccagg

SEQ ID NO: 38125 - DNA, 28 bp, synthetic construct
  source 1..28: mol_type = other DNA
tctctgtgtgtcctcctgtccgacctgg

SEQ ID NO: 38126 - DNA, 28 bp, synthetic construct
  source 1..28: mol_type = other DNA
ctctgtgtgtcctcctgtccgacctggg

SEQ ID NO: 38127 - DNA, 28 bp, synthetic construct
  source 1..28: mol_type = other DNA
ctgttggtctcccaggtcggacaggagg

SEQ ID NO: 38128 - DNA, 28 bp, synthetic construct
  source 1..28: mol_type = other DNA
gggctgttggtctcccaggtcggacagg

SEQ ID NO: 38129 - DNA, 28 bp, synthetic construct
  source 1..28: mol_type = other DNA
gtccgacctgggagaccaacagccctgg

SEQ ID NO: 38130 - DNA, 28 bp, synthetic construct
  source 1..28: mol_type = other DNA
tccgacctgggagaccaacagccctggg

SEQ ID NO: 38131 - DNA, 28 bp, synthetic construct
  source 1..28: mol_type = other DNA
tcccagggctgttggtctcccaggtcgg

SEQ ID NO: 38132 - DNA, 28 bp, synthetic construct
  source 1..28: mol_type = other DNA
gtcttcccagggctgttggtctcccagg

SEQ ID NO: 38133 - DNA, 28 bp, synthetic construct
  source 1..28: mol_type = other DNA
gaccaacagccctgggaagacagagagg

SEQ ID NO: 38134 - DNA, 28 bp, synthetic construct
  source 1..28: mol_type = other DNA
accaacagccctgggaagacagagaggg

SEQ ID NO: 38135 - DNA, 28 bp, synthetic construct
  source 1..28: mol_type = other DNA
ccaacagccctgggaagacagagagggg

SEQ ID NO: 38136 - DNA, 28 bp, synthetic construct
  source 1..28: mol_type = other DNA
tgggtgtcccctctctgtcttcccaggg

SEQ ID NO: 38137 - DNA, 28 bp, synthetic construct
  source 1..28: mol_type = other DNA
gtgggtgtcccctctctgtcttcccagg

SEQ ID NO: 38138 - DNA, 28 bp, synthetic construct
  source 1..28: mol_type = other DNA
tcagcactaagggtgagtcatgagtggg

SEQ ID NO: 38139 - DNA, 28 bp, synthetic construct
  source 1..28: mol_type = other DNA
atcagcactaagggtgagtcatgagtgg

SEQ ID NO: 38140 - DNA, 28 bp, synthetic construct
  source 1..28: mol_type = other DNA
tgactcacccttagtgctgatgccccgg

SEQ ID NO: 38141 - DNA, 28 bp, synthetic construct
  source 1..28: mol_type = other DNA
ctcacccttagtgctgatgccccggagg

SEQ ID NO: 38142 - DNA, 28 bp, synthetic construct
  source 1..28: mol_type = other DNA
cccttagtgctgatgccccggaggtcgg

SEQ ID NO: 38143 - DNA, 28 bp, synthetic construct
  source 1..28: mol_type = other DNA
accgacctccggggcatcagcactaagg

SEQ ID NO: 38144 - DNA, 28 bp, synthetic construct
  source 1..28: mol_type = other DNA
tgctaatgaaaatcaccgacctccgggg

SEQ ID NO: 38145 - DNA, 28 bp, synthetic construct
  source 1..28: mol_type = other DNA
atgctaatgaaaatcaccgacctccggg

SEQ ID NO: 38146 - DNA, 28 bp, synthetic construct
  source 1..28: mol_type = other DNA
gatgctaatgaaaatcaccgacctccgg

SEQ ID NO: 38147 - DNA, 28 bp, synthetic construct
  source 1..28: mol_type = other DNA
ggtcggtgattttcattagcatccttgg

SEQ ID NO: 38148 - DNA, 28 bp, synthetic construct
  source 1..28: mol_type = other DNA
gtcggtgattttcattagcatccttggg

SEQ ID NO: 38149 - DNA, 28 bp, synthetic construct
  source 1..28: mol_type = other DNA
ttcattagcatccttgggaacatgtagg

SEQ ID NO: 38150 - DNA, 28 bp, synthetic construct
  source 1..28: mol_type = other DNA
tcattagcatccttgggaacatgtaggg

SEQ ID NO: 38151 - DNA, 28 bp, synthetic construct
  source 1..28: mol_type = other DNA
tagcatccttgggaacatgtagggctgg

SEQ ID NO: 38152 - DNA, 28 bp, synthetic construct
  source 1..28: mol_type = other DNA
atccttgggaacatgtagggctggctgg

SEQ ID NO: 38153 - DNA, 28 bp, synthetic construct
  source 1..28: mol_type = other DNA
tccttgggaacatgtagggctggctggg

SEQ ID NO: 38154 - DNA, 28 bp, synthetic construct
  source 1..28: mol_type = other DNA
gcccagccagccctacatgttcccaagg

SEQ ID NO: 38155 - DNA, 28 bp, synthetic construct
  source 1..28: mol_type = other DNA
gaacatgtagggctggctgggccgccgg

SEQ ID NO: 38156 - DNA, 28 bp, synthetic construct
  source 1..28: mol_type = other DNA
gtagggctggctgggccgccggcgccgg

SEQ ID NO: 38157 - DNA, 28 bp, synthetic construct
  source 1..28: mol_type = other DNA
tagggctggctgggccgccggcgccggg

SEQ ID NO: 38158 - DNA, 28 bp, synthetic construct
  source 1..28: mol_type = other DNA
cctgaggctgtacgcccggcgccggcgg

SEQ ID NO: 38159 - DNA, 28 bp, synthetic construct
  source 1..28: mol_type = other DNA
cgccggcgccgggcgtacagcctcaggg

SEQ ID NO: 38160 - DNA, 28 bp, synthetic construct
  source 1..28: mol_type = other DNA
agccctgaggctgtacgcccggcgccgg

SEQ ID NO: 38161 - DNA, 28 bp, synthetic construct
  source 1..28: mol_type = other DNA
gctggaagccctgaggctgtacgcccgg

SEQ ID NO: 38162 - DNA, 28 bp, synthetic construct
  source 1..28: mol_type = other DNA
cgtacagcctcagggcttccagcagtgg

SEQ ID NO: 38163 - DNA, 28 bp, synthetic construct
  source 1..28: mol_type = other DNA
gcaggagccactgctggaagccctgagg

SEQ ID NO: 38164 - DNA, 28 bp, synthetic construct
  source 1..28: mol_type = other DNA
gtggacaagctgcaggagccactgctgg

SEQ ID NO: 38165 - DNA, 28 bp, synthetic construct
  source 1..28: mol_type = other DNA
ggctcctgcagcttgtccactttttcgg

SEQ ID NO: 38166 - DNA, 28 bp, synthetic construct
  source 1..28: mol_type = other DNA
gctcctgcagcttgtccactttttcggg

SEQ ID NO: 38167 - DNA, 28 bp, synthetic construct
  source 1..28: mol_type = other DNA
gagcccgaaaaagtggacaagctgcagg

SEQ ID NO: 38168 - DNA, 28 bp, synthetic construct
  source 1..28: mol_type = other DNA
cttgtccactttttcgggctcctccagg

SEQ ID NO: 38169 - DNA, 28 bp, synthetic construct
  source 1..28: mol_type = other DNA
atggacctggaggagcccgaaaaagtgg

SEQ ID NO: 38170 - DNA, 28 bp, synthetic construct
  source 1..28: mol_type = other DNA
tttttcgggctcctccaggtccatgcgg

SEQ ID NO: 38171 - DNA, 28 bp, synthetic construct
  source 1..28: mol_type = other DNA
ggctcctccaggtccatgcggtctatgg

SEQ ID NO: 38172 - DNA, 28 bp, synthetic construct
  source 1..28: mol_type = other DNA
gctcctccaggtccatgcggtctatggg

SEQ ID NO: 38173 - DNA, 28 bp, synthetic construct
  source 1..28: mol_type = other DNA
ctcctccaggtccatgcggtctatgggg

SEQ ID NO: 38174 - DNA, 28 bp, synthetic construct
  source 1..28: mol_type = other DNA
gtccccatagaccgcatggacctggagg

SEQ ID NO: 38175 - DNA, 28 bp, synthetic construct
  source 1..28: mol_type = other DNA
cttgtccccatagaccgcatggacctgg

SEQ ID NO: 38176 - DNA, 28 bp, synthetic construct
  source 1..28: mol_type = other DNA
agtatacttgtccccatagaccgcatgg

SEQ ID NO: 38177 - DNA, 28 bp, synthetic construct
  source 1..28: mol_type = other DNA
atgcggtctatggggacaagtatactgg

SEQ ID NO: 38178 - DNA, 28 bp, synthetic construct
  source 1..28: mol_type = other DNA
atggggacaagtatactggagtgagagg

SEQ ID NO: 38179 - DNA, 28 bp, synthetic construct
  source 1..28: mol_type = other DNA
tggggacaagtatactggagtgagaggg

SEQ ID NO: 38180 - DNA, 28 bp, synthetic construct
  source 1..28: mol_type = other DNA
ggggacaagtatactggagtgagagggg

SEQ ID NO: 38181 - DNA, 28 bp, synthetic construct
  source 1..28: mol_type = other DNA
acaagtatactggagtgagaggggaagg

SEQ ID NO: 38182 - DNA, 28 bp, synthetic construct
  source 1..28: mol_type = other DNA
ctggagtgagaggggaaggaagagatgg

SEQ ID NO: 38183 - DNA, 28 bp, synthetic construct
  source 1..28: mol_type = other DNA
tggagtgagaggggaaggaagagatggg

SEQ ID NO: 38184 - DNA, 28 bp, synthetic construct
  source 1..28: mol_type = other DNA
ggagtgagaggggaaggaagagatgggg

SEQ ID NO: 38185 - DNA, 28 bp, synthetic construct
  source 1..28: mol_type = other DNA
gagatggggaagacacagtgacagatgg

SEQ ID NO: 38186 - DNA, 28 bp, synthetic construct
  source 1..28: mol_type = other DNA
cagtgacagatggctgatcaccaaccgg

SEQ ID NO: 38187 - DNA, 28 bp, synthetic construct
  source 1..28: mol_type = other DNA
gatggctgatcaccaaccggcgttttgg

SEQ ID NO: 38188 - DNA, 28 bp, synthetic construct
  source 1..28: mol_type = other DNA
atggctgatcaccaaccggcgttttggg

SEQ ID NO: 38189 - DNA, 28 bp, synthetic construct
  source 1..28: mol_type = other DNA
tgtacaggcttcccaaaacgccggttgg

SEQ ID NO: 38190 - DNA, 28 bp, synthetic construct
  source 1..28: mol_type = other DNA
aaccggcgttttgggaagcctgtacagg

SEQ ID NO: 38191 - DNA, 28 bp, synthetic construct
  source 1..28: mol_type = other DNA
accggcgttttgggaagcctgtacaggg

SEQ ID NO: 38192 - DNA, 28 bp, synthetic construct
  source 1..28: mol_type = other DNA
accctgtacaggcttcccaaaacgccgg

SEQ ID NO: 38193 - DNA, 28 bp, synthetic construct
  source 1..28: mol_type = other DNA
gcctgtacagggtttcagaactctctgg

SEQ ID NO: 38194 - DNA, 28 bp, synthetic construct
  source 1..28: mol_type = other DNA
tccagagagttctgaaaccctgtacagg

SEQ ID NO: 38195 - DNA, 28 bp, synthetic construct
  source 1..28: mol_type = other DNA
gtacagggtttcagaactctctggatgg

SEQ ID NO: 38196 - DNA, 28 bp, synthetic construct
  source 1..28: mol_type = other DNA
tacagggtttcagaactctctggatggg

SEQ ID NO: 38197 - DNA, 28 bp, synthetic construct
  source 1..28: mol_type = other DNA
acagggtttcagaactctctggatgggg

SEQ ID NO: 38198 - DNA, 28 bp, synthetic construct
  source 1..28: mol_type = other DNA
ctcttctgctggtaattcttgcacctgg

SEQ ID NO: 38199 - DNA, 28 bp, synthetic construct
  source 1..28: mol_type = other DNA
aagaattaccagcagaagagaccactgg

SEQ ID NO: 38200 - DNA, 28 bp, synthetic construct
  source 1..28: mol_type = other DNA
agaattaccagcagaagagaccactggg

SEQ ID NO: 38201 - DNA, 28 bp, synthetic construct
  source 1..28: mol_type = other DNA
tggaggacccagtggtctcttctgctgg

SEQ ID NO: 38202 - DNA, 28 bp, synthetic construct
  source 1..28: mol_type = other DNA
ctgggagggggcgtggaggacccagtgg

SEQ ID NO: 38203 - DNA, 28 bp, synthetic construct
  source 1..28: mol_type = other DNA
ggaatctgtctgggagggggcgtggagg

SEQ ID NO: 38204 - DNA, 28 bp, synthetic construct
  source 1..28: mol_type = other DNA
tgcggaatctgtctgggagggggcgtgg

SEQ ID NO: 38205 - DNA, 28 bp, synthetic construct
  source 1..28: mol_type = other DNA
cgccccctcccagacagattccgcatgg

SEQ ID NO: 38206 - DNA, 28 bp, synthetic construct
  source 1..28: mol_type = other DNA
ctccatgcggaatctgtctgggaggggg

SEQ ID NO: 38207 - DNA, 28 bp, synthetic construct
  source 1..28: mol_type = other DNA
actccatgcggaatctgtctgggagggg

SEQ ID NO: 38208 - DNA, 28 bp, synthetic construct
  source 1..28: mol_type = other DNA
cactccatgcggaatctgtctgggaggg

SEQ ID NO: 38209 - DNA, 28 bp, synthetic construct
  source 1..28: mol_type = other DNA
cctcccagacagattccgcatggagtgg

SEQ ID NO: 38210 - DNA, 28 bp, synthetic construct
  source 1..28: mol_type = other DNA
ccaccactccatgcggaatctgtctggg

SEQ ID NO: 38211 - DNA, 28 bp, synthetic construct
  source 1..28: mol_type = other DNA
ccagacagattccgcatggagtggtggg

SEQ ID NO: 38212 - DNA, 28 bp, synthetic construct
  source 1..28: mol_type = other DNA
cagattccgcatggagtggtgggaaagg

SEQ ID NO: 38213 - DNA, 28 bp, synthetic construct
  source 1..28: mol_type = other DNA
cagtctcctttcccaccactccatgcgg

SEQ ID NO: 38214 - DNA, 28 bp, synthetic construct
  source 1..28: mol_type = other DNA
ggagactgagcactgagcagacgccagg

SEQ ID NO: 38215 - DNA, 28 bp, synthetic construct
  source 1..28: mol_type = other DNA
gagactgagcactgagcagacgccaggg

SEQ ID NO: 38216 - DNA, 28 bp, synthetic construct
  source 1..28: mol_type = other DNA
agactgagcactgagcagacgccagggg

SEQ ID NO: 38217 - DNA, 28 bp, synthetic construct
  source 1..28: mol_type = other DNA
gactgagcactgagcagacgccaggggg

SEQ ID NO: 38218 - DNA, 28 bp, synthetic construct
  source 1..28: mol_type = other DNA
tctgcggaggtgcgggggcgccccctgg

SEQ ID NO: 38219 - DNA, 28 bp, synthetic construct
  source 1..28: mol_type = other DNA
gggcgcccccgcacctccgcagatgagg

SEQ ID NO: 38220 - DNA, 28 bp, synthetic construct
  source 1..28: mol_type = other DNA
atctgcctcatctgcggaggtgcggggg

SEQ ID NO: 38221 - DNA, 28 bp, synthetic construct
  source 1..28: mol_type = other DNA
catctgcctcatctgcggaggtgcgggg

SEQ ID NO: 38222 - DNA, 28 bp, synthetic construct
  source 1..28: mol_type = other DNA
ccatctgcctcatctgcggaggtgcggg

SEQ ID NO: 38223 - DNA, 28 bp, synthetic construct
  source 1..28: mol_type = other DNA
gccatctgcctcatctgcggaggtgcgg

SEQ ID NO: 38224 - DNA, 28 bp, synthetic construct
  source 1..28: mol_type = other DNA
tcagcgccatctgcctcatctgcggagg

SEQ ID NO: 38225 - DNA, 28 bp, synthetic construct
  source 1..28: mol_type = other DNA
tgctcagcgccatctgcctcatctgcgg

SEQ ID NO: 38226 - DNA, 28 bp, synthetic construct
  source 1..28: mol_type = other DNA
cagatggcgctgagcagccctgtctcgg

SEQ ID NO: 38227 - DNA, 28 bp, synthetic construct
  source 1..28: mol_type = other DNA
cctggagatggatgacaccgagacaggg

SEQ ID NO: 38228 - DNA, 28 bp, synthetic construct
  source 1..28: mol_type = other DNA
ccctggagatggatgacaccgagacagg

SEQ ID NO: 38229 - DNA, 28 bp, synthetic construct
  source 1..28: mol_type = other DNA
ctgtctcggtgtcatccatctccagggg

SEQ ID NO: 38230 - DNA, 28 bp, synthetic construct
  source 1..28: mol_type = other DNA
ctcggtgtcatccatctccaggggcagg

SEQ ID NO: 38231 - DNA, 28 bp, synthetic construct
  source 1..28: mol_type = other DNA
gctgggcagctcctgcccctggagatgg

SEQ ID NO: 38232 - DNA, 28 bp, synthetic construct
  source 1..28: mol_type = other DNA
tccaggggcaggagctgcccagcaaagg

SEQ ID NO: 38233 - DNA, 28 bp, synthetic construct
  source 1..28: mol_type = other DNA
gcctttgctgggcagctcctgcccctgg

SEQ ID NO: 38234 - DNA, 28 bp, synthetic construct
  source 1..28: mol_type = other DNA
gagctgcccagcaaaggcaaagacaagg

SEQ ID NO: 38235 - DNA, 28 bp, synthetic construct
  source 1..28: mol_type = other DNA
cacagaccttgtctttgcctttgctggg

SEQ ID NO: 38236 - DNA, 28 bp, synthetic construct
  source 1..28: mol_type = other DNA
tcacagaccttgtctttgcctttgctgg

SEQ ID NO: 38237 - DNA, 28 bp, synthetic construct
  source 1..28: mol_type = other DNA
agcaaaggcaaagacaaggtctgtgagg

SEQ ID NO: 38238 - DNA, 28 bp, synthetic construct
  source 1..28: mol_type = other DNA
gcaaaggcaaagacaaggtctgtgaggg

SEQ ID NO: 38239 - DNA, 28 bp, synthetic construct
  source 1..28: mol_type = other DNA
caaaggcaaagacaaggtctgtgagggg

SEQ ID NO: 38240 - DNA, 28 bp, synthetic construct
  source 1..28: mol_type = other DNA
acaaggtctgtgaggggcccgaagccgg

SEQ ID NO: 38241 - DNA, 28 bp, synthetic construct
  source 1..28: mol_type = other DNA
gggcccgaagccggcattgtgcatctgg

SEQ ID NO: 38242 - DNA, 28 bp, synthetic construct
  source 1..28: mol_type = other DNA
ggcccgaagccggcattgtgcatctggg

SEQ ID NO: 38243 - DNA, 28 bp, synthetic construct
  source 1..28: mol_type = other DNA
gacccagatgcacaatgccggcttcggg

SEQ ID NO: 38244 - DNA, 28 bp, synthetic construct
  source 1..28: mol_type = other DNA
ggacccagatgcacaatgccggcttcgg

SEQ ID NO: 38245 - DNA, 28 bp, synthetic construct
  source 1..28: mol_type = other DNA
gaagccggcattgtgcatctgggtccgg

SEQ ID NO: 38246 - DNA, 28 bp, synthetic construct
  source 1..28: mol_type = other DNA
tgaaccggacccagatgcacaatgccgg

SEQ ID NO: 38247 - DNA, 28 bp, synthetic construct
  source 1..28: mol_type = other DNA
ggcattgtgcatctgggtccggttcagg

SEQ ID NO: 38248 - DNA, 28 bp, synthetic construct
  source 1..28: mol_type = other DNA
gcattgtgcatctgggtccggttcaggg

SEQ ID NO: 38249 - DNA, 28 bp, synthetic construct
  source 1..28: mol_type = other DNA
tgggtccggttcagggtcagcccgtcgg

SEQ ID NO: 38250 - DNA, 28 bp, synthetic construct
  source 1..28: mol_type = other DNA
cttctccgacgggctgaccctgaaccgg

SEQ ID NO: 38251 - DNA, 28 bp, synthetic construct
  source 1..28: mol_type = other DNA
cggttcagggtcagcccgtcggagaagg

SEQ ID NO: 38252 - DNA, 28 bp, synthetic construct
  source 1..28: mol_type = other DNA
agggtcagcccgtcggagaaggtcatgg

SEQ ID NO: 38253 - DNA, 28 bp, synthetic construct
  source 1..28: mol_type = other DNA
gcaggacaccatgaccttctccgacggg

SEQ ID NO: 38254 - DNA, 28 bp, synthetic construct
  source 1..28: mol_type = other DNA
agcaggacaccatgaccttctccgacgg

SEQ ID NO: 38255 - DNA, 28 bp, synthetic construct
  source 1..28: mol_type = other DNA
cggagaaggtcatggtgtcctgctctgg

SEQ ID NO: 38256 - DNA, 28 bp, synthetic construct
  source 1..28: mol_type = other DNA
ggagaaggtcatggtgtcctgctctggg

SEQ ID NO: 38257 - DNA, 28 bp, synthetic construct
  source 1..28: mol_type = other DNA
gagaaggtcatggtgtcctgctctgggg

SEQ ID NO: 38258 - DNA, 28 bp, synthetic construct
  source 1..28: mol_type = other DNA
atctgcacaaggtacaccccagagcagg

SEQ ID NO: 38259 - DNA, 28 bp, synthetic construct
  source 1..28: mol_type = other DNA
gtaccttgtgcagatacgcagcatctgg

SEQ ID NO: 38260 - DNA, 28 bp, synthetic construct
  source 1..28: mol_type = other DNA
cctccagatgctgcgtatctgcacaagg

SEQ ID NO: 38261 - DNA, 28 bp, synthetic construct
  source 1..28: mol_type = other DNA
tgtgcagatacgcagcatctggaggtgg

SEQ ID NO: 38262 - DNA, 28 bp, synthetic construct
  source 1..28: mol_type = other DNA
gtgcagatacgcagcatctggaggtggg

SEQ ID NO: 38263 - DNA, 28 bp, synthetic construct
  source 1..28: mol_type = other DNA
tgcagatacgcagcatctggaggtgggg

SEQ ID NO: 38264 - DNA, 28 bp, synthetic construct
  source 1..28: mol_type = other DNA
gcagatacgcagcatctggaggtggggg

SEQ ID NO: 38265 - DNA, 28 bp, synthetic construct
  source 1..28: mol_type = other DNA
cagatacgcagcatctggaggtgggggg

SEQ ID NO: 38266 - DNA, 28 bp, synthetic construct
  source 1..28: mol_type = other DNA
atacgcagcatctggaggtggggggtgg

SEQ ID NO: 38267 - DNA, 28 bp, synthetic construct
  source 1..28: mol_type = other DNA
cgcagcatctggaggtggggggtggagg

SEQ ID NO: 38268 - DNA, 28 bp, synthetic construct
  source 1..28: mol_type = other DNA
agcatctggaggtggggggtggaggagg

SEQ ID NO: 38269 - DNA, 28 bp, synthetic construct
  source 1..28: mol_type = other DNA
gcatctggaggtggggggtggaggaggg

SEQ ID NO: 38270 - DNA, 28 bp, synthetic construct
  source 1..28: mol_type = other DNA
ggtggaggagggttagtgctgtttctgg

SEQ ID NO: 38271 - DNA, 28 bp, synthetic construct
  source 1..28: mol_type = other DNA
gtggaggagggttagtgctgtttctggg

SEQ ID NO: 38272 - DNA, 28 bp, synthetic construct
  source 1..28: mol_type = other DNA
tggaggagggttagtgctgtttctgggg

SEQ ID NO: 38273 - DNA, 28 bp, synthetic construct
  source 1..28: mol_type = other DNA
ggaggagggttagtgctgtttctggggg

SEQ ID NO: 38274 - DNA, 28 bp, synthetic construct
  source 1..28: mol_type = other DNA
gagggttagtgctgtttctgggggatgg

SEQ ID NO: 38275 - DNA, 28 bp, synthetic construct
  source 1..28: mol_type = other DNA
agggttagtgctgtttctgggggatggg

SEQ ID NO: 38276 - DNA, 28 bp, synthetic construct
  source 1..28: mol_type = other DNA
gggttagtgctgtttctgggggatgggg

SEQ ID NO: 38277 - DNA, 28 bp, synthetic construct
  source 1..28: mol_type = other DNA
gctgtttctgggggatggggaaaagagg

SEQ ID NO: 38278 - DNA, 28 bp, synthetic construct
  source 1..28: mol_type = other DNA
ctgtttctgggggatggggaaaagaggg

SEQ ID NO: 38279 - DNA, 28 bp, synthetic construct
  source 1..28: mol_type = other DNA
ggggatggggaaaagagggaatgagtgg

SEQ ID NO: 38280 - DNA, 28 bp, synthetic construct
  source 1..28: mol_type = other DNA
gaaaagagggaatgagtggaaagtgagg

SEQ ID NO: 38281 - DNA, 28 bp, synthetic construct
  source 1..28: mol_type = other DNA
aagagggaatgagtggaaagtgaggagg

SEQ ID NO: 38282 - DNA, 28 bp, synthetic construct
  source 1..28: mol_type = other DNA
ggaatgagtggaaagtgaggaggttagg

SEQ ID NO: 38283 - DNA, 28 bp, synthetic construct
  source 1..28: mol_type = other DNA
gtccccagtgagtgcaacctgaagcagg

SEQ ID NO: 38284 - DNA, 28 bp, synthetic construct
  source 1..28: mol_type = other DNA
tgcctgcttcaggttgcactcactgggg

SEQ ID NO: 38285 - DNA, 28 bp, synthetic construct
  source 1..28: mol_type = other DNA
atgcctgcttcaggttgcactcactggg

SEQ ID NO: 38286 - DNA, 28 bp, synthetic construct
  source 1..28: mol_type = other DNA
catgcctgcttcaggttgcactcactgg

SEQ ID NO: 38287 - DNA, 28 bp, synthetic construct
  source 1..28: mol_type = other DNA
cagtgagtgcaacctgaagcaggcatgg

SEQ ID NO: 38288 - DNA, 28 bp, synthetic construct
  source 1..28: mol_type = other DNA
gtgcaacctgaagcaggcatggagaagg

SEQ ID NO: 38289 - DNA, 28 bp, synthetic construct
  source 1..28: mol_type = other DNA
agctgaggagtcccacatgtgtggcagg

SEQ ID NO: 38290 - DNA, 28 bp, synthetic construct
  source 1..28: mol_type = other DNA
gctgaggagtcccacatgtgtggcaggg

SEQ ID NO: 38291 - DNA, 28 bp, synthetic construct
  source 1..28: mol_type = other DNA
ctgaggagtcccacatgtgtggcagggg

SEQ ID NO: 38292 - DNA, 28 bp, synthetic construct
  source 1..28: mol_type = other DNA
tgaggagtcccacatgtgtggcaggggg

SEQ ID NO: 38293 - DNA, 28 bp, synthetic construct
  source 1..28: mol_type = other DNA
gtcccacatgtgtggcagggggtgcagg

SEQ ID NO: 38294 - DNA, 28 bp, synthetic construct
  source 1..28: mol_type = other DNA
tcccacatgtgtggcagggggtgcaggg

SEQ ID NO: 38295 - DNA, 28 bp, synthetic construct
  source 1..28: mol_type = other DNA
accctgcaccccctgccacacatgtggg

SEQ ID NO: 38296 - DNA, 28 bp, synthetic construct
  source 1..28: mol_type = other DNA
taccctgcaccccctgccacacatgtgg

SEQ ID NO: 38297 - DNA, 28 bp, synthetic construct
  source 1..28: mol_type = other DNA
catgtgtggcagggggtgcagggtaagg

SEQ ID NO: 38298 - DNA, 28 bp, synthetic construct
  source 1..28: mol_type = other DNA
ggtgcagggtaaggaaatctttgcatgg

SEQ ID NO: 38299 - DNA, 28 bp, synthetic construct
  source 1..28: mol_type = other DNA
ggtaaggaaatctttgcatggatcaagg

SEQ ID NO: 38300 - DNA, 28 bp, synthetic construct
  source 1..28: mol_type = other DNA
ctttgcatggatcaaggaattgttgagg

SEQ ID NO: 38301 - DNA, 28 bp, synthetic construct
  source 1..28: mol_type = other DNA
tttgcatggatcaaggaattgttgaggg

SEQ ID NO: 38302 - DNA, 28 bp, synthetic construct
  source 1..28: mol_type = other DNA
aaggaattgttgagggtcccatatgtgg

SEQ ID NO: 38303 - DNA, 28 bp, synthetic construct
  source 1..28: mol_type = other DNA
aggaattgttgagggtcccatatgtggg

SEQ ID NO: 38304 - DNA, 28 bp, synthetic construct
  source 1..28: mol_type = other DNA
attgttgagggtcccatatgtgggtcgg

SEQ ID NO: 38305 - DNA, 28 bp, synthetic construct
  source 1..28: mol_type = other DNA
ttgttgagggtcccatatgtgggtcggg

SEQ ID NO: 38306 - DNA, 28 bp, synthetic construct
  source 1..28: mol_type = other DNA
agggtcccatatgtgggtcgggctgtgg

SEQ ID NO: 38307 - DNA, 28 bp, synthetic construct
  source 1..28: mol_type = other DNA
tcccatatgtgggtcgggctgtggcagg

SEQ ID NO: 38308 - DNA, 28 bp, synthetic construct
  source 1..28: mol_type = other DNA
tcctgccacagcccgacccacatatggg

SEQ ID NO: 38309 - DNA, 28 bp, synthetic construct
  source 1..28: mol_type = other DNA
gtcctgccacagcccgacccacatatgg

SEQ ID NO: 38310 - DNA, 28 bp, synthetic construct
  source 1..28: mol_type = other DNA
tgggtcgggctgtggcaggacccacagg

SEQ ID NO: 38311 - DNA, 28 bp, synthetic construct
  source 1..28: mol_type = other DNA
gggtcgggctgtggcaggacccacaggg

SEQ ID NO: 38312 - DNA, 28 bp, synthetic construct
  source 1..28: mol_type = other DNA
caggacccacagggcctaacttaccagg

SEQ ID NO: 38313 - DNA, 28 bp, synthetic construct
  source 1..28: mol_type = other DNA
gatatcctggtaagttaggccctgtggg

SEQ ID NO: 38314 - DNA, 28 bp, synthetic construct
  source 1..28: mol_type = other DNA
agatatcctggtaagttaggccctgtgg

SEQ ID NO: 38315 - DNA, 28 bp, synthetic construct
  source 1..28: mol_type = other DNA
cagggcctaacttaccaggatatctagg

SEQ ID NO: 38316 - DNA, 28 bp, synthetic construct
  source 1..28: mol_type = other DNA
gcctaacttaccaggatatctaggcagg

SEQ ID NO: 38317 - DNA, 28 bp, synthetic construct
  source 1..28: mol_type = other DNA
gcctgcctagatatcctggtaagttagg

SEQ ID NO: 38318 - DNA, 28 bp, synthetic construct
  source 1..28: mol_type = other DNA
ctcaaagctgcctgcctagatatcctgg

SEQ ID NO: 38319 - DNA, 28 bp, synthetic construct
  source 1..28: mol_type = other DNA
gcaggcagctttgagcagagtgatctgg

SEQ ID NO: 38320 - DNA, 28 bp, synthetic construct
  source 1..28: mol_type = other DNA
cagcaatgctgagccctgtaaagccagg

SEQ ID NO: 38321 - DNA, 28 bp, synthetic construct
  source 1..28: mol_type = other DNA
agccctgtaaagccaggcaaccgcttgg

SEQ ID NO: 38322 - DNA, 28 bp, synthetic construct
  source 1..28: mol_type = other DNA
tgccaagcggttgcctggctttacaggg

SEQ ID NO: 38323 - DNA, 28 bp, synthetic construct
  source 1..28: mol_type = other DNA
ttgccaagcggttgcctggctttacagg

SEQ ID NO: 38324 - DNA, 28 bp, synthetic construct
  source 1..28: mol_type = other DNA
tcgtggagtttgccaagcggttgcctgg

SEQ ID NO: 38325 - DNA, 28 bp, synthetic construct
  source 1..28: mol_type = other DNA
catcaagatcgtggagtttgccaagcgg

SEQ ID NO: 38326 - DNA, 28 bp, synthetic construct
  source 1..28: mol_type = other DNA
aactccacgatcttgatgatgcacttgg

SEQ ID NO: 38327 - DNA, 28 bp, synthetic construct
  source 1..28: mol_type = other DNA
gctaccaagtgcatcatcaagatcgtgg

SEQ ID NO: 38328 - DNA, 28 bp, synthetic construct
  source 1..28: mol_type = other DNA
gggctgtgggacaagttcagtgagctgg

SEQ ID NO: 38329 - DNA, 28 bp, synthetic construct
  source 1..28: mol_type = other DNA
cgcgtgcagctggatctggggctgtggg

SEQ ID NO: 38330 - DNA, 28 bp, synthetic construct
  source 1..28: mol_type = other DNA
ccgcgtgcagctggatctggggctgtgg

SEQ ID NO: 38331 - DNA, 28 bp, synthetic construct
  source 1..28: mol_type = other DNA
cagccccagatccagctgcacgcggtgg

SEQ ID NO: 38332 - DNA, 28 bp, synthetic construct
  source 1..28: mol_type = other DNA
agaccaccgcgtgcagctggatctgggg

SEQ ID NO: 38333 - DNA, 28 bp, synthetic construct
  source 1..28: mol_type = other DNA
cagaccaccgcgtgcagctggatctggg

SEQ ID NO: 38334 - DNA, 28 bp, synthetic construct
  source 1..28: mol_type = other DNA
gcagaccaccgcgtgcagctggatctgg

SEQ ID NO: 38335 - DNA, 28 bp, synthetic construct
  source 1..28: mol_type = other DNA
tccagctgcacgcggtggtctgcactgg

SEQ ID NO: 38336 - DNA, 28 bp, synthetic construct
  source 1..28: mol_type = other DNA
tccagtgcagaccaccgcgtgcagctgg

SEQ ID NO: 38337 - DNA, 28 bp, synthetic construct
  source 1..28: mol_type = other DNA
ggtggtctgcactggagttctgcagagg

SEQ ID NO: 38338 - DNA, 28 bp, synthetic construct
  source 1..28: mol_type = other DNA
gtggtctgcactggagttctgcagaggg

SEQ ID NO: 38339 - DNA, 28 bp, synthetic construct
  source 1..28: mol_type = other DNA
tggtctgcactggagttctgcagagggg

SEQ ID NO: 38340 - DNA, 28 bp, synthetic construct
  source 1..28: mol_type = other DNA
tctgcactggagttctgcagaggggagg

SEQ ID NO: 38341 - DNA, 28 bp, synthetic construct
  source 1..28: mol_type = other DNA
ctgcactggagttctgcagaggggaggg

SEQ ID NO: 38342 - DNA, 28 bp, synthetic construct
  source 1..28: mol_type = other DNA
tgcactggagttctgcagaggggagggg

SEQ ID NO: 38343 - DNA, 28 bp, synthetic construct
  source 1..28: mol_type = other DNA
gagttctgcagaggggaggggtagaagg

SEQ ID NO: 38344 - DNA, 28 bp, synthetic construct
  source 1..28: mol_type = other DNA
tctgcagaggggaggggtagaaggttgg

SEQ ID NO: 38345 - DNA, 28 bp, synthetic construct
  source 1..28: mol_type = other DNA
cagaggggaggggtagaaggttggaagg

SEQ ID NO: 38346 - DNA, 28 bp, synthetic construct
  source 1..28: mol_type = other DNA
gggtagaaggttggaaggcaagctaagg

SEQ ID NO: 38347 - DNA, 28 bp, synthetic construct
  source 1..28: mol_type = other DNA
tggaaggcaagctaaggcccacctctgg

SEQ ID NO: 38348 - DNA, 28 bp, synthetic construct
  source 1..28: mol_type = other DNA
ggaaggcaagctaaggcccacctctggg

SEQ ID NO: 38349 - DNA, 28 bp, synthetic construct
  source 1..28: mol_type = other DNA
gaaggcaagctaaggcccacctctgggg

SEQ ID NO: 38350 - DNA, 28 bp, synthetic construct
  source 1..28: mol_type = other DNA
aaggcaagctaaggcccacctctggggg

SEQ ID NO: 38351 - DNA, 28 bp, synthetic construct
  source 1..28: mol_type = other DNA
tagagagaagacagcccccagaggtggg

SEQ ID NO: 38352 - DNA, 28 bp, synthetic construct
  source 1..28: mol_type = other DNA
gtagagagaagacagcccccagaggtgg

SEQ ID NO: 38353 - DNA, 28 bp, synthetic construct
  source 1..28: mol_type = other DNA
ttggtagagagaagacagcccccagagg

SEQ ID NO: 38354 - DNA, 28 bp, synthetic construct
  source 1..28: mol_type = other DNA
atgcagaggagagagcttgggatattgg

SEQ ID NO: 38355 - DNA, 28 bp, synthetic construct
  source 1..28: mol_type = other DNA
catcagaatgcagaggagagagcttggg

SEQ ID NO: 38356 - DNA, 28 bp, synthetic construct
  source 1..28: mol_type = other DNA
gcatcagaatgcagaggagagagcttgg

SEQ ID NO: 38357 - DNA, 28 bp, synthetic construct
  source 1..28: mol_type = other DNA
ggacaaggagggcatcagaatgcagagg

SEQ ID NO: 38358 - DNA, 28 bp, synthetic construct
  source 1..28: mol_type = other DNA
catcgactggtgctgaggacaaggaggg

SEQ ID NO: 38359 - DNA, 28 bp, synthetic construct
  source 1..28: mol_type = other DNA
tcatcgactggtgctgaggacaaggagg

SEQ ID NO: 38360 - DNA, 28 bp, synthetic construct
  source 1..28: mol_type = other DNA
ctatcatcgactggtgctgaggacaagg

SEQ ID NO: 38361 - DNA, 28 bp, synthetic construct
  source 1..28: mol_type = other DNA
tggaggctatcatcgactggtgctgagg

SEQ ID NO: 38362 - DNA, 28 bp, synthetic construct
  source 1..28: mol_type = other DNA
ggttgtgttggaggctatcatcgactgg

SEQ ID NO: 38363 - DNA, 28 bp, synthetic construct
  source 1..28: mol_type = other DNA
ggggaatggggctgggttgtgttggagg

SEQ ID NO: 38364 - DNA, 28 bp, synthetic construct
  source 1..28: mol_type = other DNA
tttggggaatggggctgggttgtgttgg

SEQ ID NO: 38365 - DNA, 28 bp, synthetic construct
  source 1..28: mol_type = other DNA
actcttcactttggggaatggggctggg

SEQ ID NO: 38366 - DNA, 28 bp, synthetic construct
  source 1..28: mol_type = other DNA
cactcttcactttggggaatggggctgg

SEQ ID NO: 38367 - DNA, 28 bp, synthetic construct
  source 1..28: mol_type = other DNA
agggcactcttcactttggggaatgggg

SEQ ID NO: 38368 - DNA, 28 bp, synthetic construct
  source 1..28: mol_type = other DNA
cagggcactcttcactttggggaatggg

SEQ ID NO: 38369 - DNA, 28 bp, synthetic construct
  source 1..28: mol_type = other DNA
gcagggcactcttcactttggggaatgg

SEQ ID NO: 38370 - DNA, 28 bp, synthetic construct
  source 1..28: mol_type = other DNA
tgagggcagggcactcttcactttgggg

SEQ ID NO: 38371 - DNA, 28 bp, synthetic construct
  source 1..28: mol_type = other DNA
gtgagggcagggcactcttcactttggg

SEQ ID NO: 38372 - DNA, 28 bp, synthetic construct
  source 1..28: mol_type = other DNA
agtgagggcagggcactcttcactttgg

SEQ ID NO: 38373 - DNA, 28 bp, synthetic construct
  source 1..28: mol_type = other DNA
aaagtgaagagtgccctgccctcactgg

SEQ ID NO: 38374 - DNA, 28 bp, synthetic construct
  source 1..28: mol_type = other DNA
aagtgaagagtgccctgccctcactggg

SEQ ID NO: 38375 - DNA, 28 bp, synthetic construct
  source 1..28: mol_type = other DNA
gaatgggcagagcccagtgagggcaggg

SEQ ID NO: 38376 - DNA, 28 bp, synthetic construct
  source 1..28: mol_type = other DNA
ggaatgggcagagcccagtgagggcagg

SEQ ID NO: 38377 - DNA, 28 bp, synthetic construct
  source 1..28: mol_type = other DNA
gtgaggaatgggcagagcccagtgaggg

SEQ ID NO: 38378 - DNA, 28 bp, synthetic construct
  source 1..28: mol_type = other DNA
ggtgaggaatgggcagagcccagtgagg

SEQ ID NO: 38379 - DNA, 28 bp, synthetic construct
  source 1..28: mol_type = other DNA
actgggctctgcccattcctcaccgtgg

SEQ ID NO: 38380 - DNA, 28 bp, synthetic construct
  source 1..28: mol_type = other DNA
gggcaagtataccacggtgaggaatggg

SEQ ID NO: 38381 - DNA, 28 bp, synthetic construct
  source 1..28: mol_type = other DNA
tgggcaagtataccacggtgaggaatgg

SEQ ID NO: 38382 - DNA, 28 bp, synthetic construct
  source 1..28: mol_type = other DNA
cctcaccgtggtatacttgcccagctgg

SEQ ID NO: 38383 - DNA, 28 bp, synthetic construct
  source 1..28: mol_type = other DNA
ctctgccagctgggcaagtataccacgg

SEQ ID NO: 38384 - DNA, 28 bp, synthetic construct
  source 1..28: mol_type = other DNA
gtatacttgcccagctggcagagcgagg

SEQ ID NO: 38385 - DNA, 28 bp, synthetic construct
  source 1..28: mol_type = other DNA
tatacttgcccagctggcagagcgaggg

SEQ ID NO: 38386 - DNA, 28 bp, synthetic construct
  source 1..28: mol_type = other DNA
atacttgcccagctggcagagcgagggg

SEQ ID NO: 38387 - DNA, 28 bp, synthetic construct
  source 1..28: mol_type = other DNA
agactttcccctcgctctgccagctggg

SEQ ID NO: 38388 - DNA, 28 bp, synthetic construct
  source 1..28: mol_type = other DNA
gagactttcccctcgctctgccagctgg

SEQ ID NO: 38389 - DNA, 28 bp, synthetic construct
  source 1..28: mol_type = other DNA
gcagagcgaggggaaagtctcctgatgg

SEQ ID NO: 38390 - DNA, 28 bp, synthetic construct
  source 1..28: mol_type = other DNA
cagagcgaggggaaagtctcctgatggg

SEQ ID NO: 38391 - DNA, 28 bp, synthetic construct
  source 1..28: mol_type = other DNA
gtctcctgatgggctttgctgaccttgg

SEQ ID NO: 38392 - DNA, 28 bp, synthetic construct
  source 1..28: mol_type = other DNA
atcaccaaggtcagcaaagcccatcagg

SEQ ID NO: 38393 - DNA, 28 bp, synthetic construct
  source 1..28: mol_type = other DNA
ccttggtgatgagctcttctaactgagg

SEQ ID NO: 38394 - DNA, 28 bp, synthetic construct
  source 1..28: mol_type = other DNA
cttggtgatgagctcttctaactgaggg

SEQ ID NO: 38395 - DNA, 28 bp, synthetic construct
  source 1..28: mol_type = other DNA
actgagggctcagctcatagctgtcagg

SEQ ID NO: 38396 - DNA, 28 bp, synthetic construct
  source 1..28: mol_type = other DNA
gaagaagaaagaggtgaaggaagaaggg

SEQ ID NO: 38397 - DNA, 28 bp, synthetic construct
  source 1..28: mol_type = other DNA
agaagaagaaagaggtgaaggaagaagg

SEQ ID NO: 38398 - DNA, 28 bp, synthetic construct
  source 1..28: mol_type = other DNA
cggaacaagaagaagaaagaggtgaagg

SEQ ID NO: 38399 - DNA, 28 bp, synthetic construct
  source 1..28: mol_type = other DNA
cttcacctctttcttcttcttgttccgg

SEQ ID NO: 38400 - DNA, 28 bp, synthetic construct
  source 1..28: mol_type = other DNA
aatgaccggaacaagaagaagaaagagg

SEQ ID NO: 38401 - DNA, 28 bp, synthetic construct
  source 1..28: mol_type = other DNA
tgttccggtcatttcgcacagcttgtgg

SEQ ID NO: 38402 - DNA, 28 bp, synthetic construct
  source 1..28: mol_type = other DNA
gttccggtcatttcgcacagcttgtggg

SEQ ID NO: 38403 - DNA, 28 bp, synthetic construct
  source 1..28: mol_type = other DNA
ccggtcatttcgcacagcttgtgggtgg

SEQ ID NO: 38404 - DNA, 28 bp, synthetic construct
  source 1..28: mol_type = other DNA
gtcatttcgcacagcttgtgggtggagg

SEQ ID NO: 38405 - DNA, 28 bp, synthetic construct
  source 1..28: mol_type = other DNA
cgcacagcttgtgggtggaggcgcaagg

SEQ ID NO: 38406 - DNA, 28 bp, synthetic construct
  source 1..28: mol_type = other DNA
agcttgtgggtggaggcgcaaggagagg

SEQ ID NO: 38407 - DNA, 28 bp, synthetic construct
  source 1..28: mol_type = other DNA
gcttgtgggtggaggcgcaaggagaggg

SEQ ID NO: 38408 - DNA, 28 bp, synthetic construct
  source 1..28: mol_type = other DNA
tgggtggaggcgcaaggagagggtcagg

SEQ ID NO: 38409 - DNA, 28 bp, synthetic construct
  source 1..28: mol_type = other DNA
ggtcaggaccctcagagcctccctttgg

SEQ ID NO: 38410 - DNA, 28 bp, synthetic construct
  source 1..28: mol_type = other DNA
gtcaggaccctcagagcctccctttggg

SEQ ID NO: 38411 - DNA, 28 bp, synthetic construct
  source 1..28: mol_type = other DNA
gaggacacccaaagggaggctctgaggg

SEQ ID NO: 38412 - DNA, 28 bp, synthetic construct
  source 1..28: mol_type = other DNA
agaggacacccaaagggaggctctgagg

SEQ ID NO: 38413 - DNA, 28 bp, synthetic construct
  source 1..28: mol_type = other DNA
agggtgagagaggacacccaaagggagg

SEQ ID NO: 38414 - DNA, 28 bp, synthetic construct
  source 1..28: mol_type = other DNA
attagggtgagagaggacacccaaaggg

SEQ ID NO: 38415 - DNA, 28 bp, synthetic construct
  source 1..28: mol_type = other DNA
aattagggtgagagaggacacccaaagg

SEQ ID NO: 38416 - DNA, 28 bp, synthetic construct
  source 1..28: mol_type = other DNA
tgagcatattaaattagggtgagagagg

SEQ ID NO: 38417 - DNA, 28 bp, synthetic construct
  source 1..28: mol_type = other DNA
gataaggactgagcatattaaattaggg

SEQ ID NO: 38418 - DNA, 28 bp, synthetic construct
  source 1..28: mol_type = other DNA
tgataaggactgagcatattaaattagg

SEQ ID NO: 38419 - DNA, 28 bp, synthetic construct
  source 1..28: mol_type = other DNA
gtccttatcatgaatatctattctctgg

SEQ ID NO: 38420 - DNA, 28 bp, synthetic construct
  source 1..28: mol_type = other DNA
tgccagagaatagatattcatgataagg

SEQ ID NO: 38421 - DNA, 28 bp, synthetic construct
  source 1..28: mol_type = other DNA
caccccagggcaggccaagtctcagagg

SEQ ID NO: 38422 - DNA, 28 bp, synthetic construct
  source 1..28: mol_type = other DNA
gacctctgagacttggcctgccctgggg

SEQ ID NO: 38423 - DNA, 28 bp, synthetic construct
  source 1..28: mol_type = other DNA
tgacctctgagacttggcctgccctggg

SEQ ID NO: 38424 - DNA, 28 bp, synthetic construct
  source 1..28: mol_type = other DNA
ctgacctctgagacttggcctgccctgg

SEQ ID NO: 38425 - DNA, 28 bp, synthetic construct
  source 1..28: mol_type = other DNA
cagggcaggccaagtctcagaggtcagg

SEQ ID NO: 38426 - DNA, 28 bp, synthetic construct
  source 1..28: mol_type = other DNA
agggcaggccaagtctcagaggtcaggg

SEQ ID NO: 38427 - DNA, 28 bp, synthetic construct
  source 1..28: mol_type = other DNA
ggccaagtctcagaggtcagggaagtgg

SEQ ID NO: 38428 - DNA, 28 bp, synthetic construct
  source 1..28: mol_type = other DNA
gccaagtctcagaggtcagggaagtggg

SEQ ID NO: 38429 - DNA, 28 bp, synthetic construct
  source 1..28: mol_type = other DNA
tcccacttccctgacctctgagacttgg

SEQ ID NO: 38430 - DNA, 28 bp, synthetic construct
  source 1..28: mol_type = other DNA
gtctcagaggtcagggaagtgggagtgg

SEQ ID NO: 38431 - DNA, 28 bp, synthetic construct
  source 1..28: mol_type = other DNA
aggtcagggaagtgggagtggccagagg

SEQ ID NO: 38432 - DNA, 28 bp, synthetic construct
  source 1..28: mol_type = other DNA
ggaagtgggagtggccagaggaaagagg

SEQ ID NO: 38433 - DNA, 28 bp, synthetic construct
  source 1..28: mol_type = other DNA
gaagtgggagtggccagaggaaagaggg

SEQ ID NO: 38434 - DNA, 28 bp, synthetic construct
  source 1..28: mol_type = other DNA
cctatggctgtggccctctttcctctgg

SEQ ID NO: 38435 - DNA, 28 bp, synthetic construct
  source 1..28: mol_type = other DNA
cagaggaaagagggccacagccataggg

SEQ ID NO: 38436 - DNA, 28 bp, synthetic construct
  source 1..28: mol_type = other DNA
ggaaagagggccacagccatagggtagg

SEQ ID NO: 38437 - DNA, 28 bp, synthetic construct
  source 1..28: mol_type = other DNA
gcacttcggtcctaccctatggctgtgg

SEQ ID NO: 38438 - DNA, 28 bp, synthetic construct
  source 1..28: mol_type = other DNA
gcaggagcacttcggtcctaccctatgg

SEQ ID NO: 38439 - DNA, 28 bp, synthetic construct
  source 1..28: mol_type = other DNA
gaccgaagtgctcctgcccaagccaagg

SEQ ID NO: 38440 - DNA, 28 bp, synthetic construct
  source 1..28: mol_type = other DNA
atccttggcttgggcaggagcacttcgg

SEQ ID NO: 38441 - DNA, 28 bp, synthetic construct
  source 1..28: mol_type = other DNA
gaagtgctcctgcccaagccaaggatgg

SEQ ID NO: 38442 - DNA, 28 bp, synthetic construct
  source 1..28: mol_type = other DNA
gtaggctgccatccttggcttgggcagg

SEQ ID NO: 38443 - DNA, 28 bp, synthetic construct
  source 1..28: mol_type = other DNA
gaaggtaggctgccatccttggcttggg

SEQ ID NO: 38444 - DNA, 28 bp, synthetic construct
  source 1..28: mol_type = other DNA
ggaaggtaggctgccatccttggcttgg

SEQ ID NO: 38445 - DNA, 28 bp, synthetic construct
  source 1..28: mol_type = other DNA
gccaaggatggcagcctaccttccttgg

SEQ ID NO: 38446 - DNA, 28 bp, synthetic construct
  source 1..28: mol_type = other DNA
tccaaggaaggtaggctgccatccttgg

SEQ ID NO: 38447 - DNA, 28 bp, synthetic construct
  source 1..28: mol_type = other DNA
cgaagtgggcatgtccaaggaaggtagg

SEQ ID NO: 38448 - DNA, 28 bp, synthetic construct
  source 1..28: mol_type = other DNA
gcttcgaagtgggcatgtccaaggaagg

SEQ ID NO: 38449 - DNA, 28 bp, synthetic construct
  source 1..28: mol_type = other DNA
aagtgcttcgaagtgggcatgtccaagg

SEQ ID NO: 38450 - DNA, 28 bp, synthetic construct
  source 1..28: mol_type = other DNA
gcccacttcgaagcacttctgtagccgg

SEQ ID NO: 38451 - DNA, 28 bp, synthetic construct
  source 1..28: mol_type = other DNA
gccggctacagaagtgcttcgaagtggg

SEQ ID NO: 38452 - DNA, 28 bp, synthetic construct
  source 1..28: mol_type = other DNA
tgccggctacagaagtgcttcgaagtgg

SEQ ID NO: 38453 - DNA, 28 bp, synthetic construct
  source 1..28: mol_type = other DNA
gaagcacttctgtagccggcagtactgg

SEQ ID NO: 38454 - DNA, 28 bp, synthetic construct
  source 1..28: mol_type = other DNA
agccggcagtactggcagcgattcctgg

SEQ ID NO: 38455 - DNA, 28 bp, synthetic construct
  source 1..28: mol_type = other DNA
gaccaggaatcgctgccagtactgccgg

SEQ ID NO: 38456 - DNA, 28 bp, synthetic construct
  source 1..28: mol_type = other DNA
aaactgtatcatcaacaaggtgaccagg

SEQ ID NO: 38457 - DNA, 28 bp, synthetic construct
  source 1..28: mol_type = other DNA
cgcgacaaaaactgtatcatcaacaagg

SEQ ID NO: 38458 - DNA, 28 bp, synthetic construct
  source 1..28: mol_type = other DNA
cttgttgatgatacagtttttgtcgcgg

SEQ ID NO: 38459 - DNA, 28 bp, synthetic construct
  source 1..28: mol_type = other DNA
gtgacacgtgtacaccatgttcttctgg

SEQ ID NO: 38460 - DNA, 28 bp, synthetic construct
  source 1..28: mol_type = other DNA
gtacaccatgttcttctggatgcttcgg

SEQ ID NO: 38461 - DNA, 28 bp, synthetic construct
  source 1..28: mol_type = other DNA
tttcgccgaagcatccagaagaacatgg

SEQ ID NO: 38462 - DNA, 28 bp, synthetic construct
  source 1..28: mol_type = other DNA
ctggatgcttcggcgaaagaagccctgg

SEQ ID NO: 38463 - DNA, 28 bp, synthetic construct
  source 1..28: mol_type = other DNA
ttcggcgaaagaagccctggagttgagg

SEQ ID NO: 38464 - DNA, 28 bp, synthetic construct
  source 1..28: mol_type = other DNA
tcggcgaaagaagccctggagttgaggg

SEQ ID NO: 38465 - DNA, 28 bp, synthetic construct
  source 1..28: mol_type = other DNA
agccctggagttgagggaaagagagagg

SEQ ID NO: 38466 - DNA, 28 bp, synthetic construct
  source 1..28: mol_type = other DNA
gccctggagttgagggaaagagagaggg

SEQ ID NO: 38467 - DNA, 28 bp, synthetic construct
  source 1..28: mol_type = other DNA
gccctctctctttccctcaactccaggg

SEQ ID NO: 38468 - DNA, 28 bp, synthetic construct
  source 1..28: mol_type = other DNA
ggccctctctctttccctcaactccagg

SEQ ID NO: 38469 - DNA, 28 bp, synthetic construct
  source 1..28: mol_type = other DNA
agagagggcctctgaagcacaatgctgg

SEQ ID NO: 38470 - DNA, 28 bp, synthetic construct
  source 1..28: mol_type = other DNA
gagagggcctctgaagcacaatgctggg

SEQ ID NO: 38471 - DNA, 28 bp, synthetic construct
  source 1..28: mol_type = other DNA
tggtactcccagcattgtgcttcagagg

SEQ ID NO: 38472 - DNA, 28 bp, synthetic construct
  source 1..28: mol_type = other DNA
aatgctgggagtaccagcctctcactgg

SEQ ID NO: 38473 - DNA, 28 bp, synthetic construct
  source 1..28: mol_type = other DNA
agtaccagcctctcactggccttgcagg

SEQ ID NO: 38474 - DNA, 28 bp, synthetic construct
  source 1..28: mol_type = other DNA
gcaacctgcaaggccagtgagaggctgg

SEQ ID NO: 38475 - DNA, 28 bp, synthetic construct
  source 1..28: mol_type = other DNA
tggggcaacctgcaaggccagtgagagg

SEQ ID NO: 38476 - DNA, 28 bp, synthetic construct
  source 1..28: mol_type = other DNA
taggtcaggcttggggcaacctgcaagg

SEQ ID NO: 38477 - DNA, 28 bp, synthetic construct
  source 1..28: mol_type = other DNA
tggttaatagattaggtcaggcttgggg

SEQ ID NO: 38478 - DNA, 28 bp, synthetic construct
  source 1..28: mol_type = other DNA
gtggttaatagattaggtcaggcttggg

SEQ ID NO: 38479 - DNA, 28 bp, synthetic construct
  source 1..28: mol_type = other DNA
ggtggttaatagattaggtcaggcttgg

SEQ ID NO: 38480 - DNA, 28 bp, synthetic construct
  source 1..28: mol_type = other DNA
acataggtggttaatagattaggtcagg

SEQ ID NO: 38481 - DNA, 28 bp, synthetic construct
  source 1..28: mol_type = other DNA
tttgcacataggtggttaatagattagg

SEQ ID NO: 38482 - DNA, 28 bp, synthetic construct
  source 1..28: mol_type = other DNA
tgagcagcactgctttgcacataggtgg

SEQ ID NO: 38483 - DNA, 28 bp, synthetic construct
  source 1..28: mol_type = other DNA
gtctgagcagcactgctttgcacatagg

SEQ ID NO: 38484 - DNA, 28 bp, synthetic construct
  source 1..28: mol_type = other DNA
tgctcagacacagcatctgtgtgcctgg

SEQ ID NO: 38485 - DNA, 28 bp, synthetic construct
  source 1..28: mol_type = other DNA
tgtgtgcctggtctctcatcttactagg

SEQ ID NO: 38486 - DNA, 28 bp, synthetic construct
  source 1..28: mol_type = other DNA
gtgtgcctggtctctcatcttactaggg

SEQ ID NO: 38487 - DNA, 28 bp, synthetic construct
  source 1..28: mol_type = other DNA
agttaccctagtaagatgagagaccagg

SEQ ID NO: 38488 - DNA, 28 bp, synthetic construct
  source 1..28: mol_type = other DNA
tggtctctcatcttactagggtaactgg

SEQ ID NO: 38489 - DNA, 28 bp, synthetic construct
  source 1..28: mol_type = other DNA
gtacgtggtgggagtgggcagacggggg

SEQ ID NO: 38490 - DNA, 28 bp, synthetic construct
  source 1..28: mol_type = other DNA
tgtacgtggtgggagtgggcagacgggg

SEQ ID NO: 38491 - DNA, 28 bp, synthetic construct
  source 1..28: mol_type = other DNA
gtgtacgtggtgggagtgggcagacggg

SEQ ID NO: 38492 - DNA, 28 bp, synthetic construct
  source 1..28: mol_type = other DNA
tgtgtacgtggtgggagtgggcagacgg

SEQ ID NO: 38493 - DNA, 28 bp, synthetic construct
  source 1..28: mol_type = other DNA
tgcaaggtgtgtacgtggtgggagtggg

SEQ ID NO: 38494 - DNA, 28 bp, synthetic construct
  source 1..28: mol_type = other DNA
ctgcaaggtgtgtacgtggtgggagtgg

SEQ ID NO: 38495 - DNA, 28 bp, synthetic construct
  source 1..28: mol_type = other DNA
gaaggctgcaaggtgtgtacgtggtggg

SEQ ID NO: 38496 - DNA, 28 bp, synthetic construct
  source 1..28: mol_type = other DNA
tgaaggctgcaaggtgtgtacgtggtgg

SEQ ID NO: 38497 - DNA, 28 bp, synthetic construct
  source 1..28: mol_type = other DNA
ttgtgaaggctgcaaggtgtgtacgtgg

SEQ ID NO: 38498 - DNA, 28 bp, synthetic construct
  source 1..28: mol_type = other DNA
ggggtcagctcttgtgaaggctgcaagg

SEQ ID NO: 38499 - DNA, 28 bp, synthetic construct
  source 1..28: mol_type = other DNA
gccttcacaagagctgaccccatagtgg

SEQ ID NO: 38500 - DNA, 28 bp, synthetic construct
  source 1..28: mol_type = other DNA
accactatggggtcagctcttgtgaagg

SEQ ID NO: 38501 - DNA, 28 bp, synthetic construct
  source 1..28: mol_type = other DNA
gagctgaccccatagtggtagccagagg

SEQ ID NO: 38502 - DNA, 28 bp, synthetic construct
  source 1..28: mol_type = other DNA
gacaagtcctctggctaccactatgggg

SEQ ID NO: 38503 - DNA, 28 bp, synthetic construct
  source 1..28: mol_type = other DNA
tgacaagtcctctggctaccactatggg

SEQ ID NO: 38504 - DNA, 28 bp, synthetic construct
  source 1..28: mol_type = other DNA
atgacaagtcctctggctaccactatgg

SEQ ID NO: 38505 - DNA, 28 bp, synthetic construct
  source 1..28: mol_type = other DNA
gcttcgtgtgcaatgacaagtcctctgg

SEQ ID NO: 38506 - DNA, 28 bp, synthetic construct
  source 1..28: mol_type = other DNA
aggacttgtcattgcacacgaagcatgg

SEQ ID NO: 38507 - DNA, 28 bp, synthetic construct
  source 1..28: mol_type = other DNA
acacgaagcatggcttgtagacccgagg

SEQ ID NO: 38508 - DNA, 28 bp, synthetic construct
  source 1..28: mol_type = other DNA
cgaagcatggcttgtagacccgaggagg

SEQ ID NO: 38509 - DNA, 28 bp, synthetic construct
  source 1..28: mol_type = other DNA
agcatggcttgtagacccgaggaggcgg

SEQ ID NO: 38510 - DNA, 28 bp, synthetic construct
  source 1..28: mol_type = other DNA
atggcttgtagacccgaggaggcggagg

SEQ ID NO: 38511 - DNA, 28 bp, synthetic construct
  source 1..28: mol_type = other DNA
tggcttgtagacccgaggaggcggaggg

SEQ ID NO: 38512 - DNA, 28 bp, synthetic construct
  source 1..28: mol_type = other DNA
ggcttgtagacccgaggaggcggagggg

SEQ ID NO: 38513 - DNA, 28 bp, synthetic construct
  source 1..28: mol_type = other DNA
gcttgtagacccgaggaggcggaggggg

SEQ ID NO: 38514 - DNA, 28 bp, synthetic construct
  source 1..28: mol_type = other DNA
tagacccgaggaggcggagggggcgagg

SEQ ID NO: 38515 - DNA, 28 bp, synthetic construct
  source 1..28: mol_type = other DNA
agacccgaggaggcggagggggcgaggg

SEQ ID NO: 38516 - DNA, 28 bp, synthetic construct
  source 1..28: mol_type = other DNA
tcgccctcgccccctccgcctcctcggg

SEQ ID NO: 38517 - DNA, 28 bp, synthetic construct
  source 1..28: mol_type = other DNA
ctcgccctcgccccctccgcctcctcgg

SEQ ID NO: 38518 - DNA, 28 bp, synthetic construct
  source 1..28: mol_type = other DNA
ggaggcggagggggcgagggcgagctgg

SEQ ID NO: 38519 - DNA, 28 bp, synthetic construct
  source 1..28: mol_type = other DNA
gaggcggagggggcgagggcgagctggg

SEQ ID NO: 38520 - DNA, 28 bp, synthetic construct
  source 1..28: mol_type = other DNA
gagctgggcaccatctcctctgagctgg

SEQ ID NO: 38521 - DNA, 28 bp, synthetic construct
  source 1..28: mol_type = other DNA
acacagagcaccagctcagaggagatgg

SEQ ID NO: 38522 - DNA, 28 bp, synthetic construct
  source 1..28: mol_type = other DNA
gtggagacacagagcaccagctcagagg

SEQ ID NO: 38523 - DNA, 28 bp, synthetic construct
  source 1..28: mol_type = other DNA
agctggtgctctgtgtctccaccgctgg

SEQ ID NO: 38524 - DNA, 28 bp, synthetic construct
  source 1..28: mol_type = other DNA
gctggtgctctgtgtctccaccgctggg

SEQ ID NO: 38525 - DNA, 28 bp, synthetic construct
  source 1..28: mol_type = other DNA
ggtgctctgtgtctccaccgctgggagg

SEQ ID NO: 38526 - DNA, 28 bp, synthetic construct
  source 1..28: mol_type = other DNA
gtgctctgtgtctccaccgctgggaggg

SEQ ID NO: 38527 - DNA, 28 bp, synthetic construct
  source 1..28: mol_type = other DNA
cacatcactgcttccctcccagcggtgg

SEQ ID NO: 38528 - DNA, 28 bp, synthetic construct
  source 1..28: mol_type = other DNA
cctcacatcactgcttccctcccagcgg

SEQ ID NO: 38529 - DNA, 28 bp, synthetic construct
  source 1..28: mol_type = other DNA
cgctgggagggaagcagtgatgtgaggg

SEQ ID NO: 38530 - DNA, 28 bp, synthetic construct
  source 1..28: mol_type = other DNA
ggagggaagcagtgatgtgagggtcagg

SEQ ID NO: 38531 - DNA, 28 bp, synthetic construct
  source 1..28: mol_type = other DNA
gagggaagcagtgatgtgagggtcaggg

SEQ ID NO: 38532 - DNA, 28 bp, synthetic construct
  source 1..28: mol_type = other DNA
agggaagcagtgatgtgagggtcagggg

SEQ ID NO: 38533 - DNA, 28 bp, synthetic construct
  source 1..28: mol_type = other DNA
gcagtgatgtgagggtcaggggagaagg

SEQ ID NO: 38534 - DNA, 28 bp, synthetic construct
  source 1..28: mol_type = other DNA
ggggagaaggaccccacagacctccagg

SEQ ID NO: 38535 - DNA, 28 bp, synthetic construct
  source 1..28: mol_type = other DNA
tgatgaggaagcctggaggtctgtgggg

SEQ ID NO: 38536 - DNA, 28 bp, synthetic construct
  source 1..28: mol_type = other DNA
gtgatgaggaagcctggaggtctgtggg

SEQ ID NO: 38537 - DNA, 28 bp, synthetic construct
  source 1..28: mol_type = other DNA
tgtgatgaggaagcctggaggtctgtgg

SEQ ID NO: 38538 - DNA, 28 bp, synthetic construct
  source 1..28: mol_type = other DNA
gggtgtgtgtgatgaggaagcctggagg

SEQ ID NO: 38539 - DNA, 28 bp, synthetic construct
  source 1..28: mol_type = other DNA
atggggtgtgtgtgatgaggaagcctgg

SEQ ID NO: 38540 - DNA, 28 bp, synthetic construct
  source 1..28: mol_type = other DNA
aaatgcacatggggtgtgtgtgatgagg

SEQ ID NO: 38541 - DNA, 28 bp, synthetic construct
  source 1..28: mol_type = other DNA
acacaccccatgtgcatttgttccttgg

SEQ ID NO: 38542 - DNA, 28 bp, synthetic construct
  source 1..28: mol_type = other DNA
gtgggccaaggaacaaatgcacatgggg

SEQ ID NO: 38543 - DNA, 28 bp, synthetic construct
  source 1..28: mol_type = other DNA
agtgggccaaggaacaaatgcacatggg

SEQ ID NO: 38544 - DNA, 28 bp, synthetic construct
  source 1..28: mol_type = other DNA
cagtgggccaaggaacaaatgcacatgg

SEQ ID NO: 38545 - DNA, 28 bp, synthetic construct
  source 1..28: mol_type = other DNA
catgtgcatttgttccttggcccactgg

SEQ ID NO: 38546 - DNA, 28 bp, synthetic construct
  source 1..28: mol_type = other DNA
agtgatggctgtcaccagtgggccaagg

SEQ ID NO: 38547 - DNA, 28 bp, synthetic construct
  source 1..28: mol_type = other DNA
tgtggtagtgatggctgtcaccagtggg

SEQ ID NO: 38548 - DNA, 28 bp, synthetic construct
  source 1..28: mol_type = other DNA
ctgtggtagtgatggctgtcaccagtgg

SEQ ID NO: 38549 - DNA, 28 bp, synthetic construct
  source 1..28: mol_type = other DNA
ttctggccctttctatgtaaggtactgg

SEQ ID NO: 38550 - DNA, 28 bp, synthetic construct
  source 1..28: mol_type = other DNA
aggagcttctggccctttctatgtaagg

SEQ ID NO: 38551 - DNA, 28 bp, synthetic construct
  source 1..28: mol_type = other DNA
gaactgaggtgcaaggaggagcttctgg

SEQ ID NO: 38552 - DNA, 28 bp, synthetic construct
  source 1..28: mol_type = other DNA
taaagagtggaactgaggtgcaaggagg

SEQ ID NO: 38553 - DNA, 28 bp, synthetic construct
  source 1..28: mol_type = other DNA
gtgtaaagagtggaactgaggtgcaagg

SEQ ID NO: 38554 - DNA, 28 bp, synthetic construct
  source 1..28: mol_type = other DNA
gcacctcagttccactctttacacacgg

SEQ ID NO: 38555 - DNA, 28 bp, synthetic construct
  source 1..28: mol_type = other DNA
tttccgtgtgtaaagagtggaactgagg

SEQ ID NO: 38556 - DNA, 28 bp, synthetic construct
  source 1..28: mol_type = other DNA
atttactctttccgtgtgtaaagagtgg

SEQ ID NO: 38557 - DNA, 28 bp, synthetic construct
  source 1..28: mol_type = other DNA
tggggtgtagggtgcaggagagggtggg

SEQ ID NO: 38558 - DNA, 28 bp, synthetic construct
  source 1..28: mol_type = other DNA
ctggggtgtagggtgcaggagagggtgg

SEQ ID NO: 38559 - DNA, 28 bp, synthetic construct
  source 1..28: mol_type = other DNA
gggctggggtgtagggtgcaggagaggg

SEQ ID NO: 38560 - DNA, 28 bp, synthetic construct
  source 1..28: mol_type = other DNA
ggggctggggtgtagggtgcaggagagg

SEQ ID NO: 38561 - DNA, 28 bp, synthetic construct
  source 1..28: mol_type = other DNA
tctcctgcaccctacaccccagccccgg

SEQ ID NO: 38562 - DNA, 28 bp, synthetic construct
  source 1..28: mol_type = other DNA
agtccggggctggggtgtagggtgcagg

SEQ ID NO: 38563 - DNA, 28 bp, synthetic construct
  source 1..28: mol_type = other DNA
caccctacaccccagccccggactccgg

SEQ ID NO: 38564 - DNA, 28 bp, synthetic construct
  source 1..28: mol_type = other DNA
taccggagtccggggctggggtgtaggg

SEQ ID NO: 38565 - DNA, 28 bp, synthetic construct
  source 1..28: mol_type = other DNA
gtaccggagtccggggctggggtgtagg

SEQ ID NO: 38566 - DNA, 28 bp, synthetic construct
  source 1..28: mol_type = other DNA
atgtaggtaccggagtccggggctgggg

SEQ ID NO: 38567 - DNA, 28 bp, synthetic construct
  source 1..28: mol_type = other DNA
aatgtaggtaccggagtccggggctggg

SEQ ID NO: 38568 - DNA, 28 bp, synthetic construct
  source 1..28: mol_type = other DNA
caatgtaggtaccggagtccggggctgg

SEQ ID NO: 38569 - DNA, 28 bp, synthetic construct
  source 1..28: mol_type = other DNA
cctgcaatgtaggtaccggagtccgggg

SEQ ID NO: 38570 - DNA, 28 bp, synthetic construct
  source 1..28: mol_type = other DNA
gcctgcaatgtaggtaccggagtccggg

SEQ ID NO: 38571 - DNA, 28 bp, synthetic construct
  source 1..28: mol_type = other DNA
agcctgcaatgtaggtaccggagtccgg

SEQ ID NO: 38572 - DNA, 28 bp, synthetic construct
  source 1..28: mol_type = other DNA
ggactccggtacctacattgcaggctgg

SEQ ID NO: 38573 - DNA, 28 bp, synthetic construct
  source 1..28: mol_type = other DNA
ctccggtacctacattgcaggctggcgg

SEQ ID NO: 38574 - DNA, 28 bp, synthetic construct
  source 1..28: mol_type = other DNA
tccggtacctacattgcaggctggcggg

SEQ ID NO: 38575 - DNA, 28 bp, synthetic construct
  source 1..28: mol_type = other DNA
acccgccagcctgcaatgtaggtaccgg

SEQ ID NO: 38576 - DNA, 28 bp, synthetic construct
  source 1..28: mol_type = other DNA
acctacattgcaggctggcgggttgcgg

SEQ ID NO: 38577 - DNA, 28 bp, synthetic construct
  source 1..28: mol_type = other DNA
gccgcaacccgccagcctgcaatgtagg

SEQ ID NO: 38578 - DNA, 28 bp, synthetic construct
  source 1..28: mol_type = other DNA
cattgcaggctggcgggttgcggccagg

SEQ ID NO: 38579 - DNA, 28 bp, synthetic construct
  source 1..28: mol_type = other DNA
tgcggccaggcaaaagattcaagtccgg

SEQ ID NO: 38580 - DNA, 28 bp, synthetic construct
  source 1..28: mol_type = other DNA
tttcgccggacttgaatcttttgcctgg

SEQ ID NO: 38581 - DNA, 28 bp, synthetic construct
  source 1..28: mol_type = other DNA
gcaaaagattcaagtccggcgaaacagg

SEQ ID NO: 38582 - DNA, 28 bp, synthetic construct
  source 1..28: mol_type = other DNA
tcaagtccggcgaaacaggagccgccgg

SEQ ID NO: 38583 - DNA, 28 bp, synthetic construct
  source 1..28: mol_type = other DNA
agtccggcgaaacaggagccgccggtgg

SEQ ID NO: 38584 - DNA, 28 bp, synthetic construct
  source 1..28: mol_type = other DNA
gagccaccggcggctcctgtttcgccgg

SEQ ID NO: 38585 - DNA, 28 bp, synthetic construct
  source 1..28: mol_type = other DNA
ccggcttgctgcgcagagccaccggcgg

SEQ ID NO: 38586 - DNA, 28 bp, synthetic construct
  source 1..28: mol_type = other DNA
gggccggcttgctgcgcagagccaccgg

SEQ ID NO: 38587 - DNA, 28 bp, synthetic construct
  source 1..28: mol_type = other DNA
gtggctctgcgcagcaagccggccccgg

SEQ ID NO: 38588 - DNA, 28 bp, synthetic construct
  source 1..28: mol_type = other DNA
tggctctgcgcagcaagccggccccggg

SEQ ID NO: 38589 - DNA, 28 bp, synthetic construct
  source 1..28: mol_type = other DNA
ctgcgcagcaagccggccccgggcccgg

SEQ ID NO: 38590 - DNA, 28 bp, synthetic construct
  source 1..28: mol_type = other DNA
tgtacggggcggccgggcccggggccgg

SEQ ID NO: 38591 - DNA, 28 bp, synthetic construct
  source 1..28: mol_type = other DNA
cggctgtacggggcggccgggcccgggg

SEQ ID NO: 38592 - DNA, 28 bp, synthetic construct
  source 1..28: mol_type = other DNA
acggctgtacggggcggccgggcccggg

SEQ ID NO: 38593 - DNA, 28 bp, synthetic construct
  source 1..28: mol_type = other DNA
gacggctgtacggggcggccgggcccgg

SEQ ID NO: 38594 - DNA, 28 bp, synthetic construct
  source 1..28: mol_type = other DNA
gcccggccgccccgtacagccgtcgcgg

SEQ ID NO: 38595 - DNA, 28 bp, synthetic construct
  source 1..28: mol_type = other DNA
tccgcgacggctgtacggggcggccggg

SEQ ID NO: 38596 - DNA, 28 bp, synthetic construct
  source 1..28: mol_type = other DNA
gtccgcgacggctgtacggggcggccgg

SEQ ID NO: 38597 - DNA, 28 bp, synthetic construct
  source 1..28: mol_type = other DNA
ccgccccgtacagccgtcgcggacccgg

SEQ ID NO: 38598 - DNA, 28 bp, synthetic construct
  source 1..28: mol_type = other DNA
cgccccgtacagccgtcgcggacccggg

SEQ ID NO: 38599 - DNA, 28 bp, synthetic construct
  source 1..28: mol_type = other DNA
gccccgtacagccgtcgcggacccgggg

SEQ ID NO: 38600 - DNA, 28 bp, synthetic construct
  source 1..28: mol_type = other DNA
gccccgggtccgcgacggctgtacgggg

SEQ ID NO: 38601 - DNA, 28 bp, synthetic construct
  source 1..28: mol_type = other DNA
tgccccgggtccgcgacggctgtacggg

SEQ ID NO: 38602 - DNA, 28 bp, synthetic construct
  source 1..28: mol_type = other DNA
ttgccccgggtccgcgacggctgtacgg

SEQ ID NO: 38603 - DNA, 28 bp, synthetic construct
  source 1..28: mol_type = other DNA
ggaaacgtttgccccgggtccgcgacgg

SEQ ID NO: 38604 - DNA, 28 bp, synthetic construct
  source 1..28: mol_type = other DNA
acgactgtatggaaacgtttgccccggg

SEQ ID NO: 38605 - DNA, 28 bp, synthetic construct
  source 1..28: mol_type = other DNA
tacgactgtatggaaacgtttgccccgg

SEQ ID NO: 38606 - DNA, 28 bp, synthetic construct
  source 1..28: mol_type = other DNA
ttccatacagtcgtacatcgcgacccgg

SEQ ID NO: 38607 - DNA, 28 bp, synthetic construct
  source 1..28: mol_type = other DNA
agccgggtcgcgatgtacgactgtatgg

SEQ ID NO: 38608 - DNA, 28 bp, synthetic construct
  source 1..28: mol_type = other DNA
agtcgtacatcgcgacccggcttgaagg

SEQ ID NO: 38609 - DNA, 28 bp, synthetic construct
  source 1..28: mol_type = other DNA
gtcgtacatcgcgacccggcttgaaggg

SEQ ID NO: 38610 - DNA, 28 bp, synthetic construct
  source 1..28: mol_type = other DNA
atcgcgacccggcttgaagggaaactgg

SEQ ID NO: 38611 - DNA, 28 bp, synthetic construct
  source 1..28: mol_type = other DNA
tcgcgacccggcttgaagggaaactggg

SEQ ID NO: 38612 - DNA, 28 bp, synthetic construct
  source 1..28: mol_type = other DNA
ccagcacccagtttcccttcaagccggg

SEQ ID NO: 38613 - DNA, 28 bp, synthetic construct
  source 1..28: mol_type = other DNA
tccagcacccagtttcccttcaagccgg

SEQ ID NO: 38614 - DNA, 28 bp, synthetic construct
  source 1..28: mol_type = other DNA
gggaaactgggtgctggaaacaccaagg

SEQ ID NO: 38615 - DNA, 28 bp, synthetic construct
  source 1..28: mol_type = other DNA
ggagggggaatcggctgcgggtccttgg

SEQ ID NO: 38616 - DNA, 28 bp, synthetic construct
  source 1..28: mol_type = other DNA
cgggggaggagggggaatcggctgcggg

SEQ ID NO: 38617 - DNA, 28 bp, synthetic construct
  source 1..28: mol_type = other DNA
ccgcagccgattccccctcctcccccgg

SEQ ID NO: 38618 - DNA, 28 bp, synthetic construct
  source 1..28: mol_type = other DNA
cagccgattccccctcctcccccggcgg

SEQ ID NO: 38619 - DNA, 28 bp, synthetic construct
  source 1..28: mol_type = other DNA
gcgccgccgggggaggagggggaatcgg

SEQ ID NO: 38620 - DNA, 28 bp, synthetic construct
  source 1..28: mol_type = other DNA
agcggggcgccgccgggggaggaggggg

SEQ ID NO: 38621 - DNA, 28 bp, synthetic construct
  source 1..28: mol_type = other DNA
gagcggggcgccgccgggggaggagggg

SEQ ID NO: 38622 - DNA, 28 bp, synthetic construct
  source 1..28: mol_type = other DNA
ggagcggggcgccgccgggggaggaggg

SEQ ID NO: 38623 - DNA, 28 bp, synthetic construct
  source 1..28: mol_type = other DNA
tggagcggggcgccgccgggggaggagg

SEQ ID NO: 38624 - DNA, 28 bp, synthetic construct
  source 1..28: mol_type = other DNA
tgctggagcggggcgccgccgggggagg

SEQ ID NO: 38625 - DNA, 28 bp, synthetic construct
  source 1..28: mol_type = other DNA
tcccccggcggcgccccgctccagcagg

SEQ ID NO: 38626 - DNA, 28 bp, synthetic construct
  source 1..28: mol_type = other DNA
ccctgctggagcggggcgccgccggggg

SEQ ID NO: 38627 - DNA, 28 bp, synthetic construct
  source 1..28: mol_type = other DNA
cccctgctggagcggggcgccgccgggg

SEQ ID NO: 38628 - DNA, 28 bp, synthetic construct
  source 1..28: mol_type = other DNA
cccggcggcgccccgctccagcaggggg

SEQ ID NO: 38629 - DNA, 28 bp, synthetic construct
  source 1..28: mol_type = other DNA
cccccctgctggagcggggcgccgccgg

SEQ ID NO: 38630 - DNA, 28 bp, synthetic construct
  source 1..28: mol_type = other DNA
cggcggcgccccgctccagcaggggggg

SEQ ID NO: 38631 - DNA, 28 bp, synthetic construct
  source 1..28: mol_type = other DNA
cggcgccccgctccagcagggggggagg

SEQ ID NO: 38632 - DNA, 28 bp, synthetic construct
  source 1..28: mol_type = other DNA
ggcgccccgctccagcagggggggaggg

SEQ ID NO: 38633 - DNA, 28 bp, synthetic construct
  source 1..28: mol_type = other DNA
gcgccccgctccagcagggggggagggg

SEQ ID NO: 38634 - DNA, 28 bp, synthetic construct
  source 1..28: mol_type = other DNA
cgccccgctccagcagggggggaggggg

SEQ ID NO: 38635 - DNA, 28 bp, synthetic construct
  source 1..28: mol_type = other DNA
ctccccctccccccctgctggagcgggg

SEQ ID NO: 38636 - DNA, 28 bp, synthetic construct
  source 1..28: mol_type = other DNA
cctccccctccccccctgctggagcggg

SEQ ID NO: 38637 - DNA, 28 bp, synthetic construct
  source 1..28: mol_type = other DNA
ccctccccctccccccctgctggagcgg

SEQ ID NO: 38638 - DNA, 28 bp, synthetic construct
  source 1..28: mol_type = other DNA
gctagccctccccctccccccctgctgg

SEQ ID NO: 38639 - DNA, 28 bp, synthetic construct
  source 1..28: mol_type = other DNA
agggggggagggggagggctagcatagg

SEQ ID NO: 38640 - DNA, 28 bp, synthetic construct
  source 1..28: mol_type = other DNA
gggggggagggggagggctagcataggg

SEQ ID NO: 38641 - DNA, 28 bp, synthetic construct
  source 1..28: mol_type = other DNA
gagggggagggctagcatagggcgctgg

SEQ ID NO: 38642 - DNA, 28 bp, synthetic construct
  source 1..28: mol_type = other DNA
agggggagggctagcatagggcgctggg

SEQ ID NO: 38643 - DNA, 28 bp, synthetic construct
  source 1..28: mol_type = other DNA
ctagcatagggcgctgggctgcatgcgg

SEQ ID NO: 38644 - DNA, 28 bp, synthetic construct
  source 1..28: mol_type = other DNA
tagcatagggcgctgggctgcatgcggg

SEQ ID NO: 38645 - DNA, 28 bp, synthetic construct
  source 1..28: mol_type = other DNA
tagggcgctgggctgcatgcgggtaagg

SEQ ID NO: 38646 - DNA, 28 bp, synthetic construct
  source 1..28: mol_type = other DNA
agggcgctgggctgcatgcgggtaaggg

SEQ ID NO: 38647 - DNA, 28 bp, synthetic construct
  source 1..28: mol_type = other DNA
gggcgctgggctgcatgcgggtaagggg

SEQ ID NO: 38648 - DNA, 28 bp, synthetic construct
  source 1..28: mol_type = other DNA
cgctgggctgcatgcgggtaaggggtgg

SEQ ID NO: 38649 - DNA, 28 bp, synthetic construct
  source 1..28: mol_type = other DNA
gctgggctgcatgcgggtaaggggtggg

SEQ ID NO: 38650 - DNA, 28 bp, synthetic construct
  source 1..28: mol_type = other DNA
gggctgcatgcgggtaaggggtgggcgg

SEQ ID NO: 38651 - DNA, 28 bp, synthetic construct
  source 1..28: mol_type = other DNA
ggctgcatgcgggtaaggggtgggcggg

SEQ ID NO: 38652 - DNA, 28 bp, synthetic construct
  source 1..28: mol_type = other DNA
gctgcatgcgggtaaggggtgggcgggg

SEQ ID NO: 38653 - DNA, 28 bp, synthetic construct
  source 1..28: mol_type = other DNA
tgcgggtaaggggtgggcggggaagagg

SEQ ID NO: 38654 - DNA, 28 bp, synthetic construct
  source 1..28: mol_type = other DNA
gcgggtaaggggtgggcggggaagaggg

SEQ ID NO: 38655 - DNA, 28 bp, synthetic construct
  source 1..28: mol_type = other DNA
cgggtaaggggtgggcggggaagagggg

SEQ ID NO: 38656 - DNA, 28 bp, synthetic construct
  source 1..28: mol_type = other DNA
gggtaaggggtgggcggggaagaggggg

SEQ ID NO: 38657 - DNA, 28 bp, synthetic construct
  source 1..28: mol_type = other DNA
ggtaaggggtgggcggggaagagggggg

SEQ ID NO: 38658 - DNA, 28 bp, synthetic construct
  source 1..28: mol_type = other DNA
gcggggaagaggggggatccccagcagg

SEQ ID NO: 38659 - DNA, 28 bp, synthetic construct
  source 1..28: mol_type = other DNA
cggggaagaggggggatccccagcaggg

SEQ ID NO: 38660 - DNA, 28 bp, synthetic construct
  source 1..28: mol_type = other DNA
ggggaagaggggggatccccagcagggg

SEQ ID NO: 38661 - DNA, 28 bp, synthetic construct
  source 1..28: mol_type = other DNA
agaggggggatccccagcaggggaaagg

SEQ ID NO: 38662 - DNA, 28 bp, synthetic construct
  source 1..28: mol_type = other DNA
gaggggggatccccagcaggggaaaggg

SEQ ID NO: 38663 - DNA, 28 bp, synthetic construct
  source 1..28: mol_type = other DNA
gggatccccagcaggggaaagggactgg

SEQ ID NO: 38664 - DNA, 28 bp, synthetic construct
  source 1..28: mol_type = other DNA
ggatccccagcaggggaaagggactggg

SEQ ID NO: 38665 - DNA, 28 bp, synthetic construct
  source 1..28: mol_type = other DNA
tccccagcaggggaaagggactgggcgg

SEQ ID NO: 38666 - DNA, 28 bp, synthetic construct
  source 1..28: mol_type = other DNA
ccccagcaggggaaagggactgggcggg

SEQ ID NO: 38667 - DNA, 28 bp, synthetic construct
  source 1..28: mol_type = other DNA
cccagcaggggaaagggactgggcgggg

SEQ ID NO: 38668 - DNA, 28 bp, synthetic construct
  source 1..28: mol_type = other DNA
gccccgcccagtccctttcccctgctgg

SEQ ID NO: 38669 - DNA, 28 bp, synthetic construct
  source 1..28: mol_type = other DNA
aaagggactgggcggggcgcgaagctgg

SEQ ID NO: 38670 - DNA, 28 bp, synthetic construct
  source 1..28: mol_type = other DNA
aagggactgggcggggcgcgaagctggg

SEQ ID NO: 38671 - DNA, 28 bp, synthetic construct
  source 1..28: mol_type = other DNA
agggactgggcggggcgcgaagctgggg

SEQ ID NO: 38672 - DNA, 28 bp, synthetic construct
  source 1..28: mol_type = other DNA
gataagagctggacggaggctaaagcgg

SEQ ID NO: 38673 - DNA, 28 bp, synthetic construct
  source 1..28: mol_type = other DNA
ctttagcctccgtccagctcttatctgg

SEQ ID NO: 38674 - DNA, 28 bp, synthetic construct
  source 1..28: mol_type = other DNA
tttagcctccgtccagctcttatctggg

SEQ ID NO: 38675 - DNA, 28 bp, synthetic construct
  source 1..28: mol_type = other DNA
aagcacccagataagagctggacggagg

SEQ ID NO: 38676 - DNA, 28 bp, synthetic construct
  source 1..28: mol_type = other DNA
ccgtccagctcttatctgggtgcttcgg

SEQ ID NO: 38677 - DNA, 28 bp, synthetic construct
  source 1..28: mol_type = other DNA
gctgccgaagcacccagataagagctgg

SEQ ID NO: 38678 - DNA, 28 bp, synthetic construct
  source 1..28: mol_type = other DNA
atctgggtgcttcggcagctagcactgg

SEQ ID NO: 38679 - DNA, 28 bp, synthetic construct
  source 1..28: mol_type = other DNA
tctgggtgcttcggcagctagcactggg

SEQ ID NO: 38680 - DNA, 28 bp, synthetic construct
  source 1..28: mol_type = other DNA
ctgggtgcttcggcagctagcactgggg

SEQ ID NO: 38681 - DNA, 28 bp, synthetic construct
  source 1..28: mol_type = other DNA
ggagaccttttttaaaagcgaagcctgg

SEQ ID NO: 38682 - DNA, 28 bp, synthetic construct
  source 1..28: mol_type = other DNA
gaccttttttaaaagcgaagcctggagg

SEQ ID NO: 38683 - DNA, 28 bp, synthetic construct
  source 1..28: mol_type = other DNA
accttttttaaaagcgaagcctggaggg

SEQ ID NO: 38684 - DNA, 28 bp, synthetic construct
  source 1..28: mol_type = other DNA
cccctccaggcttcgcttttaaaaaagg

SEQ ID NO: 38685 - DNA, 28 bp, synthetic construct
  source 1..28: mol_type = other DNA
tttttaaaagcgaagcctggaggggtgg

SEQ ID NO: 38686 - DNA, 28 bp, synthetic construct
  source 1..28: mol_type = other DNA
ttttaaaagcgaagcctggaggggtggg

SEQ ID NO: 38687 - DNA, 28 bp, synthetic construct
  source 1..28: mol_type = other DNA
tttaaaagcgaagcctggaggggtgggg

SEQ ID NO: 38688 - DNA, 28 bp, synthetic construct
  source 1..28: mol_type = other DNA
ttaaaagcgaagcctggaggggtggggg

SEQ ID NO: 38689 - DNA, 28 bp, synthetic construct
  source 1..28: mol_type = other DNA
taaaagcgaagcctggaggggtgggggg

SEQ ID NO: 38690 - DNA, 28 bp, synthetic construct
  source 1..28: mol_type = other DNA
aagcgaagcctggaggggtggggggtgg

SEQ ID NO: 38691 - DNA, 28 bp, synthetic construct
  source 1..28: mol_type = other DNA
agcgaagcctggaggggtggggggtggg

SEQ ID NO: 38692 - DNA, 28 bp, synthetic construct
  source 1..28: mol_type = other DNA
gcgaagcctggaggggtggggggtgggg

SEQ ID NO: 38693 - DNA, 28 bp, synthetic construct
  source 1..28: mol_type = other DNA
gcctggaggggtggggggtggggcttgg

SEQ ID NO: 38694 - DNA, 28 bp, synthetic construct
  source 1..28: mol_type = other DNA
tccaagccccaccccccacccctccagg

SEQ ID NO: 38695 - DNA, 28 bp, synthetic construct
  source 1..28: mol_type = other DNA
gtggggggtggggcttggagagcgaagg

SEQ ID NO: 38696 - DNA, 28 bp, synthetic construct
  source 1..28: mol_type = other DNA
tggggggtggggcttggagagcgaaggg

SEQ ID NO: 38697 - DNA, 28 bp, synthetic construct
  source 1..28: mol_type = other DNA
ggggggtggggcttggagagcgaagggg

SEQ ID NO: 38698 - DNA, 28 bp, synthetic construct
  source 1..28: mol_type = other DNA
gggggtggggcttggagagcgaaggggg

SEQ ID NO: 38699 - DNA, 28 bp, synthetic construct
  source 1..28: mol_type = other DNA
gtggggcttggagagcgaagggggccgg

SEQ ID NO: 38700 - DNA, 28 bp, synthetic construct
  source 1..28: mol_type = other DNA
tggggcttggagagcgaagggggccggg

SEQ ID NO: 38701 - DNA, 28 bp, synthetic construct
  source 1..28: mol_type = other DNA
tctcagctttgctcatctcggtgcccgg

SEQ ID NO: 38702 - DNA, 28 bp, synthetic construct
  source 1..28: mol_type = other DNA
gcaccgagatgagcaaagctgagagtgg

SEQ ID NO: 38703 - DNA, 28 bp, synthetic construct
  source 1..28: mol_type = other DNA
gctccactctcagctttgctcatctcgg

SEQ ID NO: 38704 - DNA, 28 bp, synthetic construct
  source 1..28: mol_type = other DNA
catacacatacgtacactcgctccgcgg

SEQ ID NO: 38705 - DNA, 28 bp, synthetic construct
  source 1..28: mol_type = other DNA
tgtgtctaagcaagcgcgcgcgccgcgg

SEQ ID NO: 38706 - DNA, 28 bp, synthetic construct
  source 1..28: mol_type = other DNA
catccgtgcatgcatttatcttatcagg

SEQ ID NO: 38707 - DNA, 28 bp, synthetic construct
  source 1..28: mol_type = other DNA
gtgcctgataagataaatgcatgcacgg

SEQ ID NO: 38708 - DNA, 28 bp, synthetic construct
  source 1..28: mol_type = other DNA
tcactcttgcatatttgcaaattcttgg

SEQ ID NO: 38709 - DNA, 28 bp, synthetic construct
  source 1..28: mol_type = other DNA
catgtgagcacgcatataaaatcatagg

SEQ ID NO: 38710 - DNA, 28 bp, synthetic construct
  source 1..28: mol_type = other DNA
cacgtttgtgcaaacacaccttgctcgg

SEQ ID NO: 38711 - DNA, 28 bp, synthetic construct
  source 1..28: mol_type = other DNA
acgtttgtgcaaacacaccttgctcggg

SEQ ID NO: 38712 - DNA, 28 bp, synthetic construct
  source 1..28: mol_type = other DNA
acaccttgctcgggagaatgcttgcagg

SEQ ID NO: 38713 - DNA, 28 bp, synthetic construct
  source 1..28: mol_type = other DNA
atgcctgcaagcattctcccgagcaagg

SEQ ID NO: 38714 - DNA, 28 bp, synthetic construct
  source 1..28: mol_type = other DNA
tgcaggcatactctccacagctcatagg

SEQ ID NO: 38715 - DNA, 28 bp, synthetic construct
  source 1..28: mol_type = other DNA
aaatgcatgcaaagcctatgagctgtgg

SEQ ID NO: 38716 - DNA, 28 bp, synthetic construct
  source 1..28: mol_type = other DNA
ataggctttgcatgcatttgcactgagg

SEQ ID NO: 38717 - DNA, 28 bp, synthetic construct
  source 1..28: mol_type = other DNA
tgcatttgcactgaggcgcgtgcccagg

SEQ ID NO: 38718 - DNA, 28 bp, synthetic construct
  source 1..28: mol_type = other DNA
tttgcactgaggcgcgtgcccaggtcgg

SEQ ID NO: 38719 - DNA, 28 bp, synthetic construct
  source 1..28: mol_type = other DNA
ttgcactgaggcgcgtgcccaggtcggg

SEQ ID NO: 38720 - DNA, 28 bp, synthetic construct
  source 1..28: mol_type = other DNA
tgcactgaggcgcgtgcccaggtcgggg

SEQ ID NO: 38721 - DNA, 28 bp, synthetic construct
  source 1..28: mol_type = other DNA
ctgaggcgcgtgcccaggtcggggttgg

SEQ ID NO: 38722 - DNA, 28 bp, synthetic construct
  source 1..28: mol_type = other DNA
gcgtgcccaggtcggggttggaagaagg

SEQ ID NO: 38723 - DNA, 28 bp, synthetic construct
  source 1..28: mol_type = other DNA
cctctccttcttccaaccccgacctggg

SEQ ID NO: 38724 - DNA, 28 bp, synthetic construct
  source 1..28: mol_type = other DNA
tcctctccttcttccaaccccgacctgg

SEQ ID NO: 38725 - DNA, 28 bp, synthetic construct
  source 1..28: mol_type = other DNA
aggtcggggttggaagaaggagaggagg

SEQ ID NO: 38726 - DNA, 28 bp, synthetic construct
  source 1..28: mol_type = other DNA
aactctgaaaggaaatgcttatgcttgg

SEQ ID NO: 38727 - DNA, 28 bp, synthetic construct
  source 1..28: mol_type = other DNA
gtttggggagagggaaaactctgaaagg

SEQ ID NO: 38728 - DNA, 28 bp, synthetic construct
  source 1..28: mol_type = other DNA
gtgaaaaagggagagtttggggagaggg

SEQ ID NO: 38729 - DNA, 28 bp, synthetic construct
  source 1..28: mol_type = other DNA
tgtgaaaaagggagagtttggggagagg

SEQ ID NO: 38730 - DNA, 28 bp, synthetic construct
  source 1..28: mol_type = other DNA
actagtgtgaaaaagggagagtttgggg

SEQ ID NO: 38731 - DNA, 28 bp, synthetic construct
  source 1..28: mol_type = other DNA
gactagtgtgaaaaagggagagtttggg

SEQ ID NO: 38732 - DNA, 28 bp, synthetic construct
  source 1..28: mol_type = other DNA
tgactagtgtgaaaaagggagagtttgg

SEQ ID NO: 38733 - DNA, 28 bp, synthetic construct
  source 1..28: mol_type = other DNA
ctccctttttcacactagtcaatacagg

SEQ ID NO: 38734 - DNA, 28 bp, synthetic construct
  source 1..28: mol_type = other DNA
tccctttttcacactagtcaatacaggg

SEQ ID NO: 38735 - DNA, 28 bp, synthetic construct
  source 1..28: mol_type = other DNA
ccctttttcacactagtcaatacagggg

SEQ ID NO: 38736 - DNA, 28 bp, synthetic construct
  source 1..28: mol_type = other DNA
acccctgtattgactagtgtgaaaaagg

SEQ ID NO: 38737 - DNA, 28 bp, synthetic construct
  source 1..28: mol_type = other DNA
cacactagtcaatacaggggtgttaagg

SEQ ID NO: 38738 - DNA, 28 bp, synthetic construct
  source 1..28: mol_type = other DNA
tcaatacaggggtgttaaggatgactgg

SEQ ID NO: 38739 - DNA, 28 bp, synthetic construct
  source 1..28: mol_type = other DNA
caatacaggggtgttaaggatgactggg

SEQ ID NO: 38740 - DNA, 28 bp, synthetic construct
  source 1..28: mol_type = other DNA
aatacaggggtgttaaggatgactgggg

SEQ ID NO: 38741 - DNA, 28 bp, synthetic construct
  source 1..28: mol_type = other DNA
aggggtgttaaggatgactggggagagg

SEQ ID NO: 38742 - DNA, 28 bp, synthetic construct
  source 1..28: mol_type = other DNA
ggggtgttaaggatgactggggagaggg

SEQ ID NO: 38743 - DNA, 28 bp, synthetic construct
  source 1..28: mol_type = other DNA
gggtgttaaggatgactggggagagggg

SEQ ID NO: 38744 - DNA, 28 bp, synthetic construct
  source 1..28: mol_type = other DNA
aaggatgactggggagaggggaacgtgg

SEQ ID NO: 38745 - DNA, 28 bp, synthetic construct
  source 1..28: mol_type = other DNA
gatgactggggagaggggaacgtggagg

SEQ ID NO: 38746 - DNA, 28 bp, synthetic construct
  source 1..28: mol_type = other DNA
gtccccgcgcgcagctgctctcctgagg

SEQ ID NO: 38747 - DNA, 28 bp, synthetic construct
  source 1..28: mol_type = other DNA
agcctcaggagagcagctgcgcgcgggg

SEQ ID NO: 38748 - DNA, 28 bp, synthetic construct
  source 1..28: mol_type = other DNA
gagcctcaggagagcagctgcgcgcggg

SEQ ID NO: 38749 - DNA, 28 bp, synthetic construct
  source 1..28: mol_type = other DNA
cgagcctcaggagagcagctgcgcgcgg

SEQ ID NO: 38750 - DNA, 28 bp, synthetic construct
  source 1..28: mol_type = other DNA
cgcgcgcagctgctctcctgaggctcgg

SEQ ID NO: 38751 - DNA, 28 bp, synthetic construct
  source 1..28: mol_type = other DNA
gcgcgcagctgctctcctgaggctcggg

SEQ ID NO: 38752 - DNA, 28 bp, synthetic construct
  source 1..28: mol_type = other DNA
ggaggtagtgcaggtcccgagcctcagg

SEQ ID NO: 38753 - DNA, 28 bp, synthetic construct
  source 1..28: mol_type = other DNA
ggaatgagaggggtggaggtagtgcagg

SEQ ID NO: 38754 - DNA, 28 bp, synthetic construct
  source 1..28: mol_type = other DNA
cactacctccacccctctcattcccagg

SEQ ID NO: 38755 - DNA, 28 bp, synthetic construct
  source 1..28: mol_type = other DNA
cctccacccctctcattcccaggcctgg

SEQ ID NO: 38756 - DNA, 28 bp, synthetic construct
  source 1..28: mol_type = other DNA
gagccaggcctgggaatgagaggggtgg

SEQ ID NO: 38757 - DNA, 28 bp, synthetic construct
  source 1..28: mol_type = other DNA
gcggagccaggcctgggaatgagagggg

SEQ ID NO: 38758 - DNA, 28 bp, synthetic construct
  source 1..28: mol_type = other DNA
ggcggagccaggcctgggaatgagaggg

SEQ ID NO: 38759 - DNA, 28 bp, synthetic construct
  source 1..28: mol_type = other DNA
gggcggagccaggcctgggaatgagagg

SEQ ID NO: 38760 - DNA, 28 bp, synthetic construct
  source 1..28: mol_type = other DNA
ggagggcgagggcggagccaggcctggg

SEQ ID NO: 38761 - DNA, 28 bp, synthetic construct
  source 1..28: mol_type = other DNA
cggagggcgagggcggagccaggcctgg

SEQ ID NO: 38762 - DNA, 28 bp, synthetic construct
  source 1..28: mol_type = other DNA
gcgcgcggagggcgagggcggagccagg

SEQ ID NO: 38763 - DNA, 28 bp, synthetic construct
  source 1..28: mol_type = other DNA
gaagcgggcgcgcggagggcgagggcgg

SEQ ID NO: 38764 - DNA, 28 bp, synthetic construct
  source 1..28: mol_type = other DNA
ccctcgccctccgcgcgcccgcttcagg

SEQ ID NO: 38765 - DNA, 28 bp, synthetic construct
  source 1..28: mol_type = other DNA
cctcgccctccgcgcgcccgcttcaggg

SEQ ID NO: 38766 - DNA, 28 bp, synthetic construct
  source 1..28: mol_type = other DNA
ttcggccctgaagcgggcgcgcggaggg

SEQ ID NO: 38767 - DNA, 28 bp, synthetic construct
  source 1..28: mol_type = other DNA
tttcggccctgaagcgggcgcgcggagg

SEQ ID NO: 38768 - DNA, 28 bp, synthetic construct
  source 1..28: mol_type = other DNA
acttttcggccctgaagcgggcgcgcgg

SEQ ID NO: 38769 - DNA, 28 bp, synthetic construct
  source 1..28: mol_type = other DNA
ggaatgcacttttcggccctgaagcggg

SEQ ID NO: 38770 - DNA, 28 bp, synthetic construct
  source 1..28: mol_type = other DNA
aggaatgcacttttcggccctgaagcgg

SEQ ID NO: 38771 - DNA, 28 bp, synthetic construct
  source 1..28: mol_type = other DNA
ttcagggccgaaaagtgcattcctgcgg

SEQ ID NO: 38772 - DNA, 28 bp, synthetic construct
  source 1..28: mol_type = other DNA
ggccgaaaagtgcattcctgcggctcgg

SEQ ID NO: 38773 - DNA, 28 bp, synthetic construct
  source 1..28: mol_type = other DNA
cgccgagccgcaggaatgcacttttcgg

SEQ ID NO: 38774 - DNA, 28 bp, synthetic construct
  source 1..28: mol_type = other DNA
gaggaggcagcgcgcgccgagccgcagg

SEQ ID NO: 38775 - DNA, 28 bp, synthetic construct
  source 1..28: mol_type = other DNA
ggtggggagacgggaaggaaggaggagg

SEQ ID NO: 38776 - DNA, 28 bp, synthetic construct
  source 1..28: mol_type = other DNA
gcgggtggggagacgggaaggaaggagg

SEQ ID NO: 38777 - DNA, 28 bp, synthetic construct
  source 1..28: mol_type = other DNA
tccttccttcccgtctccccacccgcgg

SEQ ID NO: 38778 - DNA, 28 bp, synthetic construct
  source 1..28: mol_type = other DNA
accgcgggtggggagacgggaaggaagg

SEQ ID NO: 38779 - DNA, 28 bp, synthetic construct
  source 1..28: mol_type = other DNA
taggaccgcgggtggggagacgggaagg

SEQ ID NO: 38780 - DNA, 28 bp, synthetic construct
  source 1..28: mol_type = other DNA
ttcccgtctccccacccgcggtcctagg

SEQ ID NO: 38781 - DNA, 28 bp, synthetic construct
  source 1..28: mol_type = other DNA
tcccgtctccccacccgcggtcctaggg

SEQ ID NO: 38782 - DNA, 28 bp, synthetic construct
  source 1..28: mol_type = other DNA
gccctaggaccgcgggtggggagacggg

SEQ ID NO: 38783 - DNA, 28 bp, synthetic construct
  source 1..28: mol_type = other DNA
ggccctaggaccgcgggtggggagacgg

SEQ ID NO: 38784 - DNA, 28 bp, synthetic construct
  source 1..28: mol_type = other DNA
gtctccccacccgcggtcctagggccgg

SEQ ID NO: 38785 - DNA, 28 bp, synthetic construct
  source 1..28: mol_type = other DNA
cgctccggccctaggaccgcgggtgggg

SEQ ID NO: 38786 - DNA, 28 bp, synthetic construct
  source 1..28: mol_type = other DNA
gcgctccggccctaggaccgcgggtggg

SEQ ID NO: 38787 - DNA, 28 bp, synthetic construct
  source 1..28: mol_type = other DNA
cgcgctccggccctaggaccgcgggtgg

SEQ ID NO: 38788 - DNA, 28 bp, synthetic construct
  source 1..28: mol_type = other DNA
gagcgcgctccggccctaggaccgcggg

SEQ ID NO: 38789 - DNA, 28 bp, synthetic construct
  source 1..28: mol_type = other DNA
ggagcgcgctccggccctaggaccgcgg

SEQ ID NO: 38790 - DNA, 28 bp, synthetic construct
  source 1..28: mol_type = other DNA
cacggcgggagcgcgctccggccctagg

SEQ ID NO: 38791 - DNA, 28 bp, synthetic construct
  source 1..28: mol_type = other DNA
gagagttcacggcgggagcgcgctccgg

SEQ ID NO: 38792 - DNA, 28 bp, synthetic construct
  source 1..28: mol_type = other DNA
gagcgcgctcccgccgtgaactctctgg

SEQ ID NO: 38793 - DNA, 28 bp, synthetic construct
  source 1..28: mol_type = other DNA
agcgcgctcccgccgtgaactctctggg

SEQ ID NO: 38794 - DNA, 28 bp, synthetic construct
  source 1..28: mol_type = other DNA
ggggggttcccagagagttcacggcggg

SEQ ID NO: 38795 - DNA, 28 bp, synthetic construct
  source 1..28: mol_type = other DNA
aggggggttcccagagagttcacggcgg

SEQ ID NO: 38796 - DNA, 28 bp, synthetic construct
  source 1..28: mol_type = other DNA
ccgtgaactctctgggaacccccctcgg

SEQ ID NO: 38797 - DNA, 28 bp, synthetic construct
  source 1..28: mol_type = other DNA
cgtgaactctctgggaacccccctcggg

SEQ ID NO: 38798 - DNA, 28 bp, synthetic construct
  source 1..28: mol_type = other DNA
gtgaactctctgggaacccccctcgggg

SEQ ID NO: 38799 - DNA, 28 bp, synthetic construct
  source 1..28: mol_type = other DNA
aactctctgggaacccccctcggggcgg

SEQ ID NO: 38800 - DNA, 28 bp, synthetic construct
  source 1..28: mol_type = other DNA
actctctgggaacccccctcggggcggg

SEQ ID NO: 38801 - DNA, 28 bp, synthetic construct
  source 1..28: mol_type = other DNA
ctctgggaacccccctcggggcgggtgg

SEQ ID NO: 38802 - DNA, 28 bp, synthetic construct
  source 1..28: mol_type = other DNA
cgcgctcggccacccgccccgagggggg

SEQ ID NO: 38803 - DNA, 28 bp, synthetic construct
  source 1..28: mol_type = other DNA
gcgcgctcggccacccgccccgaggggg

SEQ ID NO: 38804 - DNA, 28 bp, synthetic construct
  source 1..28: mol_type = other DNA
agcgcgctcggccacccgccccgagggg

SEQ ID NO: 38805 - DNA, 28 bp, synthetic construct
  source 1..28: mol_type = other DNA
gagcgcgctcggccacccgccccgaggg

SEQ ID NO: 38806 - DNA, 28 bp, synthetic construct
  source 1..28: mol_type = other DNA
tgagcgcgctcggccacccgccccgagg

SEQ ID NO: 38807 - DNA, 28 bp, synthetic construct
  source 1..28: mol_type = other DNA
cgggtcaggaggaggtgagcgcgctcgg

SEQ ID NO: 38808 - DNA, 28 bp, synthetic construct
  source 1..28: mol_type = other DNA
cgagcgcgctcacctcctcctgacccgg

SEQ ID NO: 38809 - DNA, 28 bp, synthetic construct
  source 1..28: mol_type = other DNA
ggtggggcggggccgggtcaggaggagg

SEQ ID NO: 38810 - DNA, 28 bp, synthetic construct
  source 1..28: mol_type = other DNA
cggggtggggcggggccgggtcaggagg

SEQ ID NO: 38811 - DNA, 28 bp, synthetic construct
  source 1..28: mol_type = other DNA
gggcggggtggggcggggccgggtcagg

SEQ ID NO: 38812 - DNA, 28 bp, synthetic construct
  source 1..28: mol_type = other DNA
gacccggccccgccccaccccgcccagg

SEQ ID NO: 38813 - DNA, 28 bp, synthetic construct
  source 1..28: mol_type = other DNA
ggcctgggcggggtggggcggggccggg

SEQ ID NO: 38814 - DNA, 28 bp, synthetic construct
  source 1..28: mol_type = other DNA
cggcctgggcggggtggggcggggccgg

SEQ ID NO: 38815 - DNA, 28 bp, synthetic construct
  source 1..28: mol_type = other DNA
aagacggcctgggcggggtggggcgggg

SEQ ID NO: 38816 - DNA, 28 bp, synthetic construct
  source 1..28: mol_type = other DNA
gaagacggcctgggcggggtggggcggg

SEQ ID NO: 38817 - DNA, 28 bp, synthetic construct
  source 1..28: mol_type = other DNA
tgaagacggcctgggcggggtggggcgg

SEQ ID NO: 38818 - DNA, 28 bp, synthetic construct
  source 1..28: mol_type = other DNA
cgctgaagacggcctgggcggggtgggg

SEQ ID NO: 38819 - DNA, 28 bp, synthetic construct
  source 1..28: mol_type = other DNA
gcgctgaagacggcctgggcggggtggg

SEQ ID NO: 38820 - DNA, 28 bp, synthetic construct
  source 1..28: mol_type = other DNA
agcgctgaagacggcctgggcggggtgg

SEQ ID NO: 38821 - DNA, 28 bp, synthetic construct
  source 1..28: mol_type = other DNA
ggcagcgctgaagacggcctgggcgggg

SEQ ID NO: 38822 - DNA, 28 bp, synthetic construct
  source 1..28: mol_type = other DNA
cggcagcgctgaagacggcctgggcggg

SEQ ID NO: 38823 - DNA, 28 bp, synthetic construct
  source 1..28: mol_type = other DNA
gcggcagcgctgaagacggcctgggcgg

SEQ ID NO: 38824 - DNA, 28 bp, synthetic construct
  source 1..28: mol_type = other DNA
gcccaggccgtcttcagcgctgccgcgg

SEQ ID NO: 38825 - DNA, 28 bp, synthetic construct
  source 1..28: mol_type = other DNA
tccgcggcagcgctgaagacggcctggg

SEQ ID NO: 38826 - DNA, 28 bp, synthetic construct
  source 1..28: mol_type = other DNA
ctccgcggcagcgctgaagacggcctgg

SEQ ID NO: 38827 - DNA, 28 bp, synthetic construct
  source 1..28: mol_type = other DNA
ggggactccgcggcagcgctgaagacgg

SEQ ID NO: 38828 - DNA, 28 bp, synthetic construct
  source 1..28: mol_type = other DNA
cgctggagggggcggggggactccgcgg

SEQ ID NO: 38829 - DNA, 28 bp, synthetic construct
  source 1..28: mol_type = other DNA
ctctggctgcgctggagggggcgggggg

SEQ ID NO: 38830 - DNA, 28 bp, synthetic construct
  source 1..28: mol_type = other DNA
actctggctgcgctggagggggcggggg

SEQ ID NO: 38831 - DNA, 28 bp, synthetic construct
  source 1..28: mol_type = other DNA
gactctggctgcgctggagggggcgggg

SEQ ID NO: 38832 - DNA, 28 bp, synthetic construct
  source 1..28: mol_type = other DNA
agactctggctgcgctggagggggcggg

SEQ ID NO: 38833 - DNA, 28 bp, synthetic construct
  source 1..28: mol_type = other DNA
tagactctggctgcgctggagggggcgg

SEQ ID NO: 38834 - DNA, 28 bp, synthetic construct
  source 1..28: mol_type = other DNA
gggtagactctggctgcgctggaggggg

SEQ ID NO: 38835 - DNA, 28 bp, synthetic construct
  source 1..28: mol_type = other DNA
ggggtagactctggctgcgctggagggg

SEQ ID NO: 38836 - DNA, 28 bp, synthetic construct
  source 1..28: mol_type = other DNA
aggggtagactctggctgcgctggaggg

SEQ ID NO: 38837 - DNA, 28 bp, synthetic construct
  source 1..28: mol_type = other DNA
gaggggtagactctggctgcgctggagg

SEQ ID NO: 38838 - DNA, 28 bp, synthetic construct
  source 1..28: mol_type = other DNA
taggaggggtagactctggctgcgctgg

SEQ ID NO: 38839 - DNA, 28 bp, synthetic construct
  source 1..28: mol_type = other DNA
tgctcgggctaggaggggtagactctgg

SEQ ID NO: 38840 - DNA, 28 bp, synthetic construct
  source 1..28: mol_type = other DNA
gagggcggactgctcgggctaggagggg

SEQ ID NO: 38841 - DNA, 28 bp, synthetic construct
  source 1..28: mol_type = other DNA
ggagggcggactgctcgggctaggaggg

SEQ ID NO: 38842 - DNA, 28 bp, synthetic construct
  source 1..28: mol_type = other DNA
cggagggcggactgctcgggctaggagg

SEQ ID NO: 38843 - DNA, 28 bp, synthetic construct
  source 1..28: mol_type = other DNA
cggcggagggcggactgctcgggctagg

SEQ ID NO: 38844 - DNA, 28 bp, synthetic construct
  source 1..28: mol_type = other DNA
agcccgagcagtccgccctccgccgcgg

SEQ ID NO: 38845 - DNA, 28 bp, synthetic construct
  source 1..28: mol_type = other DNA
ggccgcggcggagggcggactgctcggg

SEQ ID NO: 38846 - DNA, 28 bp, synthetic construct
  source 1..28: mol_type = other DNA
gggccgcggcggagggcggactgctcgg

SEQ ID NO: 38847 - DNA, 28 bp, synthetic construct
  source 1..28: mol_type = other DNA
gagcagtccgccctccgccgcggcccgg

SEQ ID NO: 38848 - DNA, 28 bp, synthetic construct
  source 1..28: mol_type = other DNA
agcagtccgccctccgccgcggcccggg

SEQ ID NO: 38849 - DNA, 28 bp, synthetic construct
  source 1..28: mol_type = other DNA
aggcggcccgggccgcggcggagggcgg

SEQ ID NO: 38850 - DNA, 28 bp, synthetic construct
  source 1..28: mol_type = other DNA
gggaggcggcccgggccgcggcggaggg

SEQ ID NO: 38851 - DNA, 28 bp, synthetic construct
  source 1..28: mol_type = other DNA
agggaggcggcccgggccgcggcggagg

SEQ ID NO: 38852 - DNA, 28 bp, synthetic construct
  source 1..28: mol_type = other DNA
cggagggaggcggcccgggccgcggcgg

SEQ ID NO: 38853 - DNA, 28 bp, synthetic construct
  source 1..28: mol_type = other DNA
actcggagggaggcggcccgggccgcgg

SEQ ID NO: 38854 - DNA, 28 bp, synthetic construct
  source 1..28: mol_type = other DNA
tcggggactcggagggaggcggcccggg

SEQ ID NO: 38855 - DNA, 28 bp, synthetic construct
  source 1..28: mol_type = other DNA
ttcggggactcggagggaggcggcccgg

SEQ ID NO: 38856 - DNA, 28 bp, synthetic construct
  source 1..28: mol_type = other DNA
aaggcttcggggactcggagggaggcgg

SEQ ID NO: 38857 - DNA, 28 bp, synthetic construct
  source 1..28: mol_type = other DNA
gataaggcttcggggactcggagggagg

SEQ ID NO: 38858 - DNA, 28 bp, synthetic construct
  source 1..28: mol_type = other DNA
cgggataaggcttcggggactcggaggg

SEQ ID NO: 38859 - DNA, 28 bp, synthetic construct
  source 1..28: mol_type = other DNA
gcgggataaggcttcggggactcggagg

SEQ ID NO: 38860 - DNA, 28 bp, synthetic construct
  source 1..28: mol_type = other DNA
gttgcgggataaggcttcggggactcgg

SEQ ID NO: 38861 - DNA, 28 bp, synthetic construct
  source 1..28: mol_type = other DNA
gcgtcagttgcgggataaggcttcgggg

SEQ ID NO: 38862 - DNA, 28 bp, synthetic construct
  source 1..28: mol_type = other DNA
ggcgtcagttgcgggataaggcttcggg

SEQ ID NO: 38863 - DNA, 28 bp, synthetic construct
  source 1..28: mol_type = other DNA
gggcgtcagttgcgggataaggcttcgg

SEQ ID NO: 38864 - DNA, 28 bp, synthetic construct
  source 1..28: mol_type = other DNA
cttagggggcgtcagttgcgggataagg

SEQ ID NO: 38865 - DNA, 28 bp, synthetic construct
  source 1..28: mol_type = other DNA
gaggcgcttagggggcgtcagttgcggg

SEQ ID NO: 38866 - DNA, 28 bp, synthetic construct
  source 1..28: mol_type = other DNA
cgaggcgcttagggggcgtcagttgcgg

SEQ ID NO: 38867 - DNA, 28 bp, synthetic construct
  source 1..28: mol_type = other DNA
gagagagacggtcgaggcgcttaggggg

SEQ ID NO: 38868 - DNA, 28 bp, synthetic construct
  source 1..28: mol_type = other DNA
cgagagagacggtcgaggcgcttagggg

SEQ ID NO: 38869 - DNA, 28 bp, synthetic construct
  source 1..28: mol_type = other DNA
tcgagagagacggtcgaggcgcttaggg

SEQ ID NO: 38870 - DNA, 28 bp, synthetic construct
  source 1..28: mol_type = other DNA
atcgagagagacggtcgaggcgcttagg

SEQ ID NO: 38871 - DNA, 28 bp, synthetic construct
  source 1..28: mol_type = other DNA
gaaggagcatcgagagagacggtcgagg

SEQ ID NO: 38872 - DNA, 28 bp, synthetic construct
  source 1..28: mol_type = other DNA
ttcgaagaaggagcatcgagagagacgg

SEQ ID NO: 38873 - DNA, 28 bp, synthetic construct
  source 1..28: mol_type = other DNA
ctaaaagtgaagttatgttcgaagaagg

SEQ ID NO: 38874 - DNA, 28 bp, synthetic construct
  source 1..28: mol_type = other DNA
gttggcacggcaggcacagcttatgggg

SEQ ID NO: 38875 - DNA, 28 bp, synthetic construct
  source 1..28: mol_type = other DNA
agttggcacggcaggcacagcttatggg

SEQ ID NO: 38876 - DNA, 28 bp, synthetic construct
  source 1..28: mol_type = other DNA
cagttggcacggcaggcacagcttatgg

SEQ ID NO: 38877 - DNA, 28 bp, synthetic construct
  source 1..28: mol_type = other DNA
ttcatcgaggcgcagttggcacggcagg

SEQ ID NO: 38878 - DNA, 28 bp, synthetic construct
  source 1..28: mol_type = other DNA
cagattcatcgaggcgcagttggcacgg

SEQ ID NO: 38879 - DNA, 28 bp, synthetic construct
  source 1..28: mol_type = other DNA
aggggcagattcatcgaggcgcagttgg

SEQ ID NO: 38880 - DNA, 28 bp, synthetic construct
  source 1..28: mol_type = other DNA
tgcgcctcgatgaatctgcccctgatgg

SEQ ID NO: 38881 - DNA, 28 bp, synthetic construct
  source 1..28: mol_type = other DNA
ttggccatcaggggcagattcatcgagg

SEQ ID NO: 38882 - DNA, 28 bp, synthetic construct
  source 1..28: mol_type = other DNA
ctggaggaggggagttggccatcagggg

SEQ ID NO: 38883 - DNA, 28 bp, synthetic construct
  source 1..28: mol_type = other DNA
actggaggaggggagttggccatcaggg

SEQ ID NO: 38884 - DNA, 28 bp, synthetic construct
  source 1..28: mol_type = other DNA
aactggaggaggggagttggccatcagg

SEQ ID NO: 38885 - DNA, 28 bp, synthetic construct
  source 1..28: mol_type = other DNA
cagtgagaaactggaggaggggagttgg

SEQ ID NO: 38886 - DNA, 28 bp, synthetic construct
  source 1..28: mol_type = other DNA
ccttggcagtgagaaactggaggagggg

SEQ ID NO: 38887 - DNA, 28 bp, synthetic construct
  source 1..28: mol_type = other DNA
cccttggcagtgagaaactggaggaggg

SEQ ID NO: 38888 - DNA, 28 bp, synthetic construct
  source 1..28: mol_type = other DNA
gcccttggcagtgagaaactggaggagg

SEQ ID NO: 38889 - DNA, 28 bp, synthetic construct
  source 1..28: mol_type = other DNA
ggagcccttggcagtgagaaactggagg

SEQ ID NO: 38890 - DNA, 28 bp, synthetic construct
  source 1..28: mol_type = other DNA
gagggagcccttggcagtgagaaactgg

SEQ ID NO: 38891 - DNA, 28 bp, synthetic construct
  source 1..28: mol_type = other DNA
agtttctcactgccaagggctccctcgg

SEQ ID NO: 38892 - DNA, 28 bp, synthetic construct
  source 1..28: mol_type = other DNA
cactgccaagggctccctcggcaatagg

SEQ ID NO: 38893 - DNA, 28 bp, synthetic construct
  source 1..28: mol_type = other DNA
actgccaagggctccctcggcaataggg

SEQ ID NO: 38894 - DNA, 28 bp, synthetic construct
  source 1..28: mol_type = other DNA
ctgccaagggctccctcggcaatagggg

SEQ ID NO: 38895 - DNA, 28 bp, synthetic construct
  source 1..28: mol_type = other DNA
gcgcccctattgccgagggagcccttgg

SEQ ID NO: 38896 - DNA, 28 bp, synthetic construct
  source 1..28: mol_type = other DNA
gctccctcggcaataggggcgcttctgg

SEQ ID NO: 38897 - DNA, 28 bp, synthetic construct
  source 1..28: mol_type = other DNA
tgaccagaagcgcccctattgccgaggg

SEQ ID NO: 38898 - DNA, 28 bp, synthetic construct
  source 1..28: mol_type = other DNA
gtgaccagaagcgcccctattgccgagg

SEQ ID NO: 38899 - DNA, 28 bp, synthetic construct
  source 1..28: mol_type = other DNA
gcgcttctggtcactgactgttctcagg

SEQ ID NO: 38900 - DNA, 28 bp, synthetic construct
  source 1..28: mol_type = other DNA
cgcttctggtcactgactgttctcaggg

SEQ ID NO: 38901 - DNA, 28 bp, synthetic construct
  source 1..28: mol_type = other DNA
agggtctttaaataccctctagcctagg

SEQ ID NO: 38902 - DNA, 28 bp, synthetic construct
  source 1..28: mol_type = other DNA
ggagggcagttatgcctaggctagaggg

SEQ ID NO: 38903 - DNA, 28 bp, synthetic construct
  source 1..28: mol_type = other DNA
gggagggcagttatgcctaggctagagg

SEQ ID NO: 38904 - DNA, 28 bp, synthetic construct
  source 1..28: mol_type = other DNA
agcctaggcataactgccctcccttcgg

SEQ ID NO: 38905 - DNA, 28 bp, synthetic construct
  source 1..28: mol_type = other DNA
aaccgaagggagggcagttatgcctagg

SEQ ID NO: 38906 - DNA, 28 bp, synthetic construct
  source 1..28: mol_type = other DNA
agctgaggggcactaaccgaagggaggg

SEQ ID NO: 38907 - DNA, 28 bp, synthetic construct
  source 1..28: mol_type = other DNA
gagctgaggggcactaaccgaagggagg

SEQ ID NO: 38908 - DNA, 28 bp, synthetic construct
  source 1..28: mol_type = other DNA
ggagagctgaggggcactaaccgaaggg

SEQ ID NO: 38909 - DNA, 28 bp, synthetic construct
  source 1..28: mol_type = other DNA
tggagagctgaggggcactaaccgaagg

SEQ ID NO: 38910 - DNA, 28 bp, synthetic construct
  source 1..28: mol_type = other DNA
tcggttagtgcccctcagctctccaagg

SEQ ID NO: 38911 - DNA, 28 bp, synthetic construct
  source 1..28: mol_type = other DNA
agtgttgcggccttggagagctgagggg

SEQ ID NO: 38912 - DNA, 28 bp, synthetic construct
  source 1..28: mol_type = other DNA
cagtgttgcggccttggagagctgaggg

SEQ ID NO: 38913 - DNA, 28 bp, synthetic construct
  source 1..28: mol_type = other DNA
acagtgttgcggccttggagagctgagg

SEQ ID NO: 38914 - DNA, 28 bp, synthetic construct
  source 1..28: mol_type = other DNA
tctccaaggccgcaacactgttccctgg

SEQ ID NO: 38915 - DNA, 28 bp, synthetic construct
  source 1..28: mol_type = other DNA
ctccaaggccgcaacactgttccctggg

SEQ ID NO: 38916 - DNA, 28 bp, synthetic construct
  source 1..28: mol_type = other DNA
aacccagggaacagtgttgcggccttgg

SEQ ID NO: 38917 - DNA, 28 bp, synthetic construct
  source 1..28: mol_type = other DNA
aggggcaacccagggaacagtgttgcgg

SEQ ID NO: 38918 - DNA, 28 bp, synthetic construct
  source 1..28: mol_type = other DNA
acactgttccctgggttgccccttccgg

SEQ ID NO: 38919 - DNA, 28 bp, synthetic construct
  source 1..28: mol_type = other DNA
gctcagtgccggaaggggcaacccaggg

SEQ ID NO: 38920 - DNA, 28 bp, synthetic construct
  source 1..28: mol_type = other DNA
cgctcagtgccggaaggggcaacccagg

SEQ ID NO: 38921 - DNA, 28 bp, synthetic construct
  source 1..28: mol_type = other DNA
gggcgagggcgctcagtgccggaagggg

SEQ ID NO: 38922 - DNA, 28 bp, synthetic construct
  source 1..28: mol_type = other DNA
cgggcgagggcgctcagtgccggaaggg

SEQ ID NO: 38923 - DNA, 28 bp, synthetic construct
  source 1..28: mol_type = other DNA
ccgggcgagggcgctcagtgccggaagg

SEQ ID NO: 38924 - DNA, 28 bp, synthetic construct
  source 1..28: mol_type = other DNA
tccggcactgagcgccctcgcccggcgg

SEQ ID NO: 38925 - DNA, 28 bp, synthetic construct
  source 1..28: mol_type = other DNA
tccgccgggcgagggcgctcagtgccgg

SEQ ID NO: 38926 - DNA, 28 bp, synthetic construct
  source 1..28: mol_type = other DNA
actgagcgccctcgcccggcggagaagg

SEQ ID NO: 38927 - DNA, 28 bp, synthetic construct
  source 1..28: mol_type = other DNA
ctgagcgccctcgcccggcggagaaggg

SEQ ID NO: 38928 - DNA, 28 bp, synthetic construct
  source 1..28: mol_type = other DNA
tgagcgccctcgcccggcggagaagggg

SEQ ID NO: 38929 - DNA, 28 bp, synthetic construct
  source 1..28: mol_type = other DNA
gagcgccctcgcccggcggagaaggggg

SEQ ID NO: 38930 - DNA, 28 bp, synthetic construct
  source 1..28: mol_type = other DNA
ccctcgcccggcggagaagggggtgagg

SEQ ID NO: 38931 - DNA, 28 bp, synthetic construct
  source 1..28: mol_type = other DNA
acctcacccccttctccgccgggcgagg

SEQ ID NO: 38932 - DNA, 28 bp, synthetic construct
  source 1..28: mol_type = other DNA
tcgcccggcggagaagggggtgaggtgg

SEQ ID NO: 38933 - DNA, 28 bp, synthetic construct
  source 1..28: mol_type = other DNA
cgcccggcggagaagggggtgaggtggg

SEQ ID NO: 38934 - DNA, 28 bp, synthetic construct
  source 1..28: mol_type = other DNA
cgcccacctcacccccttctccgccggg

SEQ ID NO: 38935 - DNA, 28 bp, synthetic construct
  source 1..28: mol_type = other DNA
ccggcggagaagggggtgaggtgggcgg

SEQ ID NO: 38936 - DNA, 28 bp, synthetic construct
  source 1..28: mol_type = other DNA
cggcggagaagggggtgaggtgggcggg

SEQ ID NO: 38937 - DNA, 28 bp, synthetic construct
  source 1..28: mol_type = other DNA
ggcggagaagggggtgaggtgggcgggg

SEQ ID NO: 38938 - DNA, 28 bp, synthetic construct
  source 1..28: mol_type = other DNA
gcggagaagggggtgaggtgggcggggg

SEQ ID NO: 38939 - DNA, 28 bp, synthetic construct
  source 1..28: mol_type = other DNA
cggagaagggggtgaggtgggcgggggg

SEQ ID NO: 38940 - DNA, 28 bp, synthetic construct
  source 1..28: mol_type = other DNA
gaagggggtgaggtgggcggggggctgg

SEQ ID NO: 38941 - DNA, 28 bp, synthetic construct
  source 1..28: mol_type = other DNA
ggctggccacgtcagaagtttgccctgg

SEQ ID NO: 38942 - DNA, 28 bp, synthetic construct
  source 1..28: mol_type = other DNA
gccacgtcagaagtttgccctggcccgg

SEQ ID NO: 38943 - DNA, 28 bp, synthetic construct
  source 1..28: mol_type = other DNA
gccgggccagggcaaacttctgacgtgg

SEQ ID NO: 38944 - DNA, 28 bp, synthetic construct
  source 1..28: mol_type = other DNA
cgtcagaagtttgccctggcccggcagg

SEQ ID NO: 38945 - DNA, 28 bp, synthetic construct
  source 1..28: mol_type = other DNA
gtcagaagtttgccctggcccggcaggg

SEQ ID NO: 38946 - DNA, 28 bp, synthetic construct
  source 1..28: mol_type = other DNA
tttgccctggcccggcagggccgaatgg

SEQ ID NO: 38947 - DNA, 28 bp, synthetic construct
  source 1..28: mol_type = other DNA
ttgccctggcccggcagggccgaatggg

SEQ ID NO: 38948 - DNA, 28 bp, synthetic construct
  source 1..28: mol_type = other DNA
tgccctggcccggcagggccgaatgggg

SEQ ID NO: 38949 - DNA, 28 bp, synthetic construct
  source 1..28: mol_type = other DNA
gccctggcccggcagggccgaatggggg

SEQ ID NO: 38950 - DNA, 28 bp, synthetic construct
  source 1..28: mol_type = other DNA
ccccccattcggccctgccgggccaggg

SEQ ID NO: 38951 - DNA, 28 bp, synthetic construct
  source 1..28: mol_type = other DNA
tccccccattcggccctgccgggccagg

SEQ ID NO: 38952 - DNA, 28 bp, synthetic construct
  source 1..28: mol_type = other DNA
cagggtccccccattcggccctgccggg

SEQ ID NO: 38953 - DNA, 28 bp, synthetic construct
  source 1..28: mol_type = other DNA
ccagggtccccccattcggccctgccgg

SEQ ID NO: 38954 - DNA, 28 bp, synthetic construct
  source 1..28: mol_type = other DNA
gggccgaatggggggaccctggccccgg

SEQ ID NO: 38955 - DNA, 28 bp, synthetic construct
  source 1..28: mol_type = other DNA
tgtccggggccagggtccccccattcgg

SEQ ID NO: 38956 - DNA, 28 bp, synthetic construct
  source 1..28: mol_type = other DNA
ccgctgctggcgctgtccggggccaggg

SEQ ID NO: 38957 - DNA, 28 bp, synthetic construct
  source 1..28: mol_type = other DNA
gccgctgctggcgctgtccggggccagg

SEQ ID NO: 38958 - DNA, 28 bp, synthetic construct
  source 1..28: mol_type = other DNA
gagtcgccgctgctggcgctgtccgggg

SEQ ID NO: 38959 - DNA, 28 bp, synthetic construct
  source 1..28: mol_type = other DNA
ggagtcgccgctgctggcgctgtccggg

SEQ ID NO: 38960 - DNA, 28 bp, synthetic construct
  source 1..28: mol_type = other DNA
gggagtcgccgctgctggcgctgtccgg

SEQ ID NO: 38961 - DNA, 28 bp, synthetic construct
  source 1..28: mol_type = other DNA
ggacagcgccagcagcggcgactcccgg

SEQ ID NO: 38962 - DNA, 28 bp, synthetic construct
  source 1..28: mol_type = other DNA
ggggatttccgggagtcgccgctgctgg

SEQ ID NO: 38963 - DNA, 28 bp, synthetic construct
  source 1..28: mol_type = other DNA
gggcgcgggggagggggggatttccggg

SEQ ID NO: 38964 - DNA, 28 bp, synthetic construct
  source 1..28: mol_type = other DNA
ggggcgcgggggagggggggatttccgg

SEQ ID NO: 38965 - DNA, 28 bp, synthetic construct
  source 1..28: mol_type = other DNA
ctgagggcggggcgcgggggaggggggg

SEQ ID NO: 38966 - DNA, 28 bp, synthetic construct
  source 1..28: mol_type = other DNA
gctgagggcggggcgcgggggagggggg

SEQ ID NO: 38967 - DNA, 28 bp, synthetic construct
  source 1..28: mol_type = other DNA
ggctgagggcggggcgcgggggaggggg

SEQ ID NO: 38968 - DNA, 28 bp, synthetic construct
  source 1..28: mol_type = other DNA
cggctgagggcggggcgcgggggagggg

SEQ ID NO: 38969 - DNA, 28 bp, synthetic construct
  source 1..28: mol_type = other DNA
gcggctgagggcggggcgcgggggaggg

SEQ ID NO: 38970 - DNA, 28 bp, synthetic construct
  source 1..28: mol_type = other DNA
ggcggctgagggcggggcgcgggggagg

SEQ ID NO: 38971 - DNA, 28 bp, synthetic construct
  source 1..28: mol_type = other DNA
tcccccgcgccccgccctcagccgccgg

SEQ ID NO: 38972 - DNA, 28 bp, synthetic construct
  source 1..28: mol_type = other DNA
cccccgcgccccgccctcagccgccggg

SEQ ID NO: 38973 - DNA, 28 bp, synthetic construct
  source 1..28: mol_type = other DNA
gcccggcggctgagggcggggcgcgggg

SEQ ID NO: 38974 - DNA, 28 bp, synthetic construct
  source 1..28: mol_type = other DNA
ggcccggcggctgagggcggggcgcggg

SEQ ID NO: 38975 - DNA, 28 bp, synthetic construct
  source 1..28: mol_type = other DNA
cggcccggcggctgagggcggggcgcgg

SEQ ID NO: 38976 - DNA, 28 bp, synthetic construct
  source 1..28: mol_type = other DNA
ccccgccctcagccgccgggccgcccgg

SEQ ID NO: 38977 - DNA, 28 bp, synthetic construct
  source 1..28: mol_type = other DNA
gccgggcggcccggcggctgagggcggg

SEQ ID NO: 38978 - DNA, 28 bp, synthetic construct
  source 1..28: mol_type = other DNA
ggccgggcggcccggcggctgagggcgg

SEQ ID NO: 38979 - DNA, 28 bp, synthetic construct
  source 1..28: mol_type = other DNA
gcaggccgggcggcccggcggctgaggg

SEQ ID NO: 38980 - DNA, 28 bp, synthetic construct
  source 1..28: mol_type = other DNA
ggcaggccgggcggcccggcggctgagg

SEQ ID NO: 38981 - DNA, 28 bp, synthetic construct
  source 1..28: mol_type = other DNA
tgggcaggcaggccgggcggcccggcgg

SEQ ID NO: 38982 - DNA, 28 bp, synthetic construct
  source 1..28: mol_type = other DNA
ggctgggcaggcaggccgggcggcccgg

SEQ ID NO: 38983 - DNA, 28 bp, synthetic construct
  source 1..28: mol_type = other DNA
gggccgcccggcctgcctgcccagccgg

SEQ ID NO: 38984 - DNA, 28 bp, synthetic construct
  source 1..28: mol_type = other DNA
gagccggctgggcaggcaggccgggcgg

SEQ ID NO: 38985 - DNA, 28 bp, synthetic construct
  source 1..28: mol_type = other DNA
acagagccggctgggcaggcaggccggg

SEQ ID NO: 38986 - DNA, 28 bp, synthetic construct
  source 1..28: mol_type = other DNA
gacagagccggctgggcaggcaggccgg

SEQ ID NO: 38987 - DNA, 28 bp, synthetic construct
  source 1..28: mol_type = other DNA
cgctgacagagccggctgggcaggcagg

SEQ ID NO: 38988 - DNA, 28 bp, synthetic construct
  source 1..28: mol_type = other DNA
gcggcgctgacagagccggctgggcagg

SEQ ID NO: 38989 - DNA, 28 bp, synthetic construct
  source 1..28: mol_type = other DNA
gtgagcggcgctgacagagccggctggg

SEQ ID NO: 38990 - DNA, 28 bp, synthetic construct
  source 1..28: mol_type = other DNA
tgtgagcggcgctgacagagccggctgg

SEQ ID NO: 38991 - DNA, 28 bp, synthetic construct
  source 1..28: mol_type = other DNA
gccggctctgtcagcgccgctcacacgg

SEQ ID NO: 38992 - DNA, 28 bp, synthetic construct
  source 1..28: mol_type = other DNA
ccggctctgtcagcgccgctcacacggg

SEQ ID NO: 38993 - DNA, 28 bp, synthetic construct
  source 1..28: mol_type = other DNA
agcgccgctcacacgggcagcgccgcgg

SEQ ID NO: 38994 - DNA, 28 bp, synthetic construct
  source 1..28: mol_type = other DNA
cgctccgcggcgctgcccgtgtgagcgg

SEQ ID NO: 38995 - DNA, 28 bp, synthetic construct
  source 1..28: mol_type = other DNA
cgctcacacgggcagcgccgcggagcgg

SEQ ID NO: 38996 - DNA, 28 bp, synthetic construct
  source 1..28: mol_type = other DNA
gctcacacgggcagcgccgcggagcggg

SEQ ID NO: 38997 - DNA, 28 bp, synthetic construct
  source 1..28: mol_type = other DNA
cacgggcagcgccgcggagcgggagcgg

SEQ ID NO: 38998 - DNA, 28 bp, synthetic construct
  source 1..28: mol_type = other DNA
agcgccgcggagcgggagcggcgcccgg

SEQ ID NO: 38999 - DNA, 28 bp, synthetic construct
  source 1..28: mol_type = other DNA
cgggccgggcgccgctcccgctccgcgg

SEQ ID NO: 39000 - DNA, 28 bp, synthetic construct
  source 1..28: mol_type = other DNA
cgcggagcgggagcggcgcccggcccgg

SEQ ID NO: 39001 - DNA, 28 bp, synthetic construct
  source 1..28: mol_type = other DNA
cgcccggcccggcccttcccccgccagg

SEQ ID NO: 39002 - DNA, 28 bp, synthetic construct
  source 1..28: mol_type = other DNA
cgcctggcgggggaagggccgggccggg

SEQ ID NO: 39003 - DNA, 28 bp, synthetic construct
  source 1..28: mol_type = other DNA
ccgcctggcgggggaagggccgggccgg

SEQ ID NO: 39004 - DNA, 28 bp, synthetic construct
  source 1..28: mol_type = other DNA
acagccgcctggcgggggaagggccggg

SEQ ID NO: 39005 - DNA, 28 bp, synthetic construct
  source 1..28: mol_type = other DNA
cacagccgcctggcgggggaagggccgg

SEQ ID NO: 39006 - DNA, 28 bp, synthetic construct
  source 1..28: mol_type = other DNA
cggcccttcccccgccaggcggctgtgg

SEQ ID NO: 39007 - DNA, 28 bp, synthetic construct
  source 1..28: mol_type = other DNA
cagccacagccgcctggcgggggaaggg

SEQ ID NO: 39008 - DNA, 28 bp, synthetic construct
  source 1..28: mol_type = other DNA
ccagccacagccgcctggcgggggaagg

SEQ ID NO: 39009 - DNA, 28 bp, synthetic construct
  source 1..28: mol_type = other DNA
cttcccccgccaggcggctgtggctggg

SEQ ID NO: 39010 - DNA, 28 bp, synthetic construct
  source 1..28: mol_type = other DNA
tggcccagccacagccgcctggcggggg

SEQ ID NO: 39011 - DNA, 28 bp, synthetic construct
  source 1..28: mol_type = other DNA
ctggcccagccacagccgcctggcgggg

SEQ ID NO: 39012 - DNA, 28 bp, synthetic construct
  source 1..28: mol_type = other DNA
cctggcccagccacagccgcctggcggg

SEQ ID NO: 39013 - DNA, 28 bp, synthetic construct
  source 1..28: mol_type = other DNA
ccctggcccagccacagccgcctggcgg

SEQ ID NO: 39014 - DNA, 28 bp, synthetic construct
  source 1..28: mol_type = other DNA
ccgccctggcccagccacagccgcctgg

SEQ ID NO: 39015 - DNA, 28 bp, synthetic construct
  source 1..28: mol_type = other DNA
caggcggctgtggctgggccagggcggg

SEQ ID NO: 39016 - DNA, 28 bp, synthetic construct
  source 1..28: mol_type = other DNA
aggcggctgtggctgggccagggcgggg

SEQ ID NO: 39017 - DNA, 28 bp, synthetic construct
  source 1..28: mol_type = other DNA
ggcaggggacaggggtttggcctaatgg

SEQ ID NO: 39018 - DNA, 28 bp, synthetic construct
  source 1..28: mol_type = other DNA
ggaaggcaggcaggggacaggggtttgg

SEQ ID NO: 39019 - DNA, 28 bp, synthetic construct
  source 1..28: mol_type = other DNA
agttaggaaggcaggcaggggacagggg

SEQ ID NO: 39020 - DNA, 28 bp, synthetic construct
  source 1..28: mol_type = other DNA
cagttaggaaggcaggcaggggacaggg

SEQ ID NO: 39021 - DNA, 28 bp, synthetic construct
  source 1..28: mol_type = other DNA
ccagttaggaaggcaggcaggggacagg

SEQ ID NO: 39022 - DNA, 28 bp, synthetic construct
  source 1..28: mol_type = other DNA
ctgtcccctgcctgccttcctaactggg

SEQ ID NO: 39023 - DNA, 28 bp, synthetic construct
  source 1..28: mol_type = other DNA
tgtcccctgcctgccttcctaactgggg

SEQ ID NO: 39024 - DNA, 28 bp, synthetic construct
  source 1..28: mol_type = other DNA
gcaccccagttaggaaggcaggcagggg

SEQ ID NO: 39025 - DNA, 28 bp, synthetic construct
  source 1..28: mol_type = other DNA
ggcaccccagttaggaaggcaggcaggg

SEQ ID NO: 39026 - DNA, 28 bp, synthetic construct
  source 1..28: mol_type = other DNA
tggcaccccagttaggaaggcaggcagg

SEQ ID NO: 39027 - DNA, 28 bp, synthetic construct
  source 1..28: mol_type = other DNA
gagttggcaccccagttaggaaggcagg

SEQ ID NO: 39028 - DNA, 28 bp, synthetic construct
  source 1..28: mol_type = other DNA
aaaagagttggcaccccagttaggaagg

SEQ ID NO: 39029 - DNA, 28 bp, synthetic construct
  source 1..28: mol_type = other DNA
tggtaaaagagttggcaccccagttagg

SEQ ID NO: 39030 - DNA, 28 bp, synthetic construct
  source 1..28: mol_type = other DNA
tcaggagggtggatggtaaaagagttgg

SEQ ID NO: 39031 - DNA, 28 bp, synthetic construct
  source 1..28: mol_type = other DNA
aacaagaaggcatcaggagggtggatgg

SEQ ID NO: 39032 - DNA, 28 bp, synthetic construct
  source 1..28: mol_type = other DNA
tgttaacaagaaggcatcaggagggtgg

SEQ ID NO: 39033 - DNA, 28 bp, synthetic construct
  source 1..28: mol_type = other DNA
aaatgttaacaagaaggcatcaggaggg

SEQ ID NO: 39034 - DNA, 28 bp, synthetic construct
  source 1..28: mol_type = other DNA
caaatgttaacaagaaggcatcaggagg

SEQ ID NO: 39035 - DNA, 28 bp, synthetic construct
  source 1..28: mol_type = other DNA
aggcaaatgttaacaagaaggcatcagg

SEQ ID NO: 39036 - DNA, 28 bp, synthetic construct
  source 1..28: mol_type = other DNA
ggaatgaaggcaaatgttaacaagaagg

SEQ ID NO: 39037 - DNA, 28 bp, synthetic construct
  source 1..28: mol_type = other DNA
gagtctcagggatcttggggaatgaagg

SEQ ID NO: 39038 - DNA, 28 bp, synthetic construct
  source 1..28: mol_type = other DNA
ctctgtgtgagtctcagggatcttgggg

SEQ ID NO: 39039 - DNA, 28 bp, synthetic construct
  source 1..28: mol_type = other DNA
tctctgtgtgagtctcagggatcttggg

SEQ ID NO: 39040 - DNA, 28 bp, synthetic construct
  source 1..28: mol_type = other DNA
ctctctgtgtgagtctcagggatcttgg

SEQ ID NO: 39041 - DNA, 28 bp, synthetic construct
  source 1..28: mol_type = other DNA
caagatccctgagactcacacagagagg

SEQ ID NO: 39042 - DNA, 28 bp, synthetic construct
  source 1..28: mol_type = other DNA
agatggcctctctgtgtgagtctcaggg

SEQ ID NO: 39043 - DNA, 28 bp, synthetic construct
  source 1..28: mol_type = other DNA
gagatggcctctctgtgtgagtctcagg

SEQ ID NO: 39044 - DNA, 28 bp, synthetic construct
  source 1..28: mol_type = other DNA
gactcacacagagaggccatctccttgg

SEQ ID NO: 39045 - DNA, 28 bp, synthetic construct
  source 1..28: mol_type = other DNA
actcacacagagaggccatctccttggg

SEQ ID NO: 39046 - DNA, 28 bp, synthetic construct
  source 1..28: mol_type = other DNA
ctcacacagagaggccatctccttgggg

SEQ ID NO: 39047 - DNA, 28 bp, synthetic construct
  source 1..28: mol_type = other DNA
acacagagaggccatctccttggggagg

SEQ ID NO: 39048 - DNA, 28 bp, synthetic construct
  source 1..28: mol_type = other DNA
gagaggccatctccttggggaggtcagg

SEQ ID NO: 39049 - DNA, 28 bp, synthetic construct
  source 1..28: mol_type = other DNA
ggccatctccttggggaggtcaggctgg

SEQ ID NO: 39050 - DNA, 28 bp, synthetic construct
  source 1..28: mol_type = other DNA
ggccagcctgacctccccaaggagatgg

SEQ ID NO: 39051 - DNA, 28 bp, synthetic construct
  source 1..28: mol_type = other DNA
ctccttggggaggtcaggctggcccagg

SEQ ID NO: 39052 - DNA, 28 bp, synthetic construct
  source 1..28: mol_type = other DNA
ggcctgggccagcctgacctccccaagg

SEQ ID NO: 39053 - DNA, 28 bp, synthetic construct
  source 1..28: mol_type = other DNA
ggggaggtcaggctggcccaggccccgg

SEQ ID NO: 39054 - DNA, 28 bp, synthetic construct
  source 1..28: mol_type = other DNA
caggctggcccaggccccggaagctagg

SEQ ID NO: 39055 - DNA, 28 bp, synthetic construct
  source 1..28: mol_type = other DNA
aggctggcccaggccccggaagctaggg

SEQ ID NO: 39056 - DNA, 28 bp, synthetic construct
  source 1..28: mol_type = other DNA
tgctgagccctagcttccggggcctggg

SEQ ID NO: 39057 - DNA, 28 bp, synthetic construct
  source 1..28: mol_type = other DNA
atgctgagccctagcttccggggcctgg

SEQ ID NO: 39058 - DNA, 28 bp, synthetic construct
  source 1..28: mol_type = other DNA
tcgagatgctgagccctagcttccgggg

SEQ ID NO: 39059 - DNA, 28 bp, synthetic construct
  source 1..28: mol_type = other DNA
ttcgagatgctgagccctagcttccggg

SEQ ID NO: 39060 - DNA, 28 bp, synthetic construct
  source 1..28: mol_type = other DNA
tttcgagatgctgagccctagcttccgg

SEQ ID NO: 39061 - DNA, 28 bp, synthetic construct
  source 1..28: mol_type = other DNA
ggaagctagggctcagcatctcgaaagg

SEQ ID NO: 39062 - DNA, 28 bp, synthetic construct
  source 1..28: mol_type = other DNA
agctagggctcagcatctcgaaaggcgg

SEQ ID NO: 39063 - DNA, 28 bp, synthetic construct
  source 1..28: mol_type = other DNA
aaggcggagaccccctgagtgcccctgg

SEQ ID NO: 39064 - DNA, 28 bp, synthetic construct
  source 1..28: mol_type = other DNA
aggcggagaccccctgagtgcccctggg

SEQ ID NO: 39065 - DNA, 28 bp, synthetic construct
  source 1..28: mol_type = other DNA
ggagaccccctgagtgcccctgggaagg

SEQ ID NO: 39066 - DNA, 28 bp, synthetic construct
  source 1..28: mol_type = other DNA
cttcgccttcccaggggcactcaggggg

SEQ ID NO: 39067 - DNA, 28 bp, synthetic construct
  source 1..28: mol_type = other DNA
cccctgagtgcccctgggaaggcgaagg

SEQ ID NO: 39068 - DNA, 28 bp, synthetic construct
  source 1..28: mol_type = other DNA
cccttcgccttcccaggggcactcaggg

SEQ ID NO: 39069 - DNA, 28 bp, synthetic construct
  source 1..28: mol_type = other DNA
ccccttcgccttcccaggggcactcagg

SEQ ID NO: 39070 - DNA, 28 bp, synthetic construct
  source 1..28: mol_type = other DNA
gcaggtttccccttcgccttcccagggg

SEQ ID NO: 39071 - DNA, 28 bp, synthetic construct
  source 1..28: mol_type = other DNA
ggcaggtttccccttcgccttcccaggg

SEQ ID NO: 39072 - DNA, 28 bp, synthetic construct
  source 1..28: mol_type = other DNA
gggcaggtttccccttcgccttcccagg

SEQ ID NO: 39073 - DNA, 28 bp, synthetic construct
  source 1..28: mol_type = other DNA
ggaaggcgaaggggaaacctgcccctgg

SEQ ID NO: 39074 - DNA, 28 bp, synthetic construct
  source 1..28: mol_type = other DNA
gaaggcgaaggggaaacctgcccctggg

SEQ ID NO: 39075 - DNA, 28 bp, synthetic construct
  source 1..28: mol_type = other DNA
aacctgcccctgggtagccagatccagg

SEQ ID NO: 39076 - DNA, 28 bp, synthetic construct
  source 1..28: mol_type = other DNA
ggcctggatctggctacccaggggcagg

SEQ ID NO: 39077 - DNA, 28 bp, synthetic construct
  source 1..28: mol_type = other DNA
ctggggcctggatctggctacccagggg

SEQ ID NO: 39078 - DNA, 28 bp, synthetic construct
  source 1..28: mol_type = other DNA
cctggggcctggatctggctacccaggg

SEQ ID NO: 39079 - DNA, 28 bp, synthetic construct
  source 1..28: mol_type = other DNA
cctgggtagccagatccaggccccaggg

SEQ ID NO: 39080 - DNA, 28 bp, synthetic construct
  source 1..28: mol_type = other DNA
cggctggtgccctggggcctggatctgg

SEQ ID NO: 39081 - DNA, 28 bp, synthetic construct
  source 1..28: mol_type = other DNA
tctttgcggctggtgccctggggcctgg

SEQ ID NO: 39082 - DNA, 28 bp, synthetic construct
  source 1..28: mol_type = other DNA
gcgactctttgcggctggtgccctgggg

SEQ ID NO: 39083 - DNA, 28 bp, synthetic construct
  source 1..28: mol_type = other DNA
agcgactctttgcggctggtgccctggg

SEQ ID NO: 39084 - DNA, 28 bp, synthetic construct
  source 1..28: mol_type = other DNA
gagcgactctttgcggctggtgccctgg

SEQ ID NO: 39085 - DNA, 28 bp, synthetic construct
  source 1..28: mol_type = other DNA
ccaataaggagcgactctttgcggctgg

SEQ ID NO: 39086 - DNA, 28 bp, synthetic construct
  source 1..28: mol_type = other DNA
gccgcaaagagtcgctccttattggtgg

SEQ ID NO: 39087 - DNA, 28 bp, synthetic construct
  source 1..28: mol_type = other DNA
gccaccaataaggagcgactctttgcgg

SEQ ID NO: 39088 - DNA, 28 bp, synthetic construct
  source 1..28: mol_type = other DNA
aagagtcgctccttattggtggccatgg

SEQ ID NO: 39089 - DNA, 28 bp, synthetic construct
  source 1..28: mol_type = other DNA
tccttattggtggccatggcagctgcgg

SEQ ID NO: 39090 - DNA, 28 bp, synthetic construct
  source 1..28: mol_type = other DNA
accgcagctgccatggccaccaataagg

SEQ ID NO: 39091 - DNA, 28 bp, synthetic construct
  source 1..28: mol_type = other DNA
ggggactctcacaccgcagctgccatgg

SEQ ID NO: 39092 - DNA, 28 bp, synthetic construct
  source 1..28: mol_type = other DNA
tggcagctgcggtgtgagagtcccctgg

SEQ ID NO: 39093 - DNA, 28 bp, synthetic construct
  source 1..28: mol_type = other DNA
ggcagctgcggtgtgagagtcccctggg

SEQ ID NO: 39094 - DNA, 28 bp, synthetic construct
  source 1..28: mol_type = other DNA
gcagctgcggtgtgagagtcccctgggg

SEQ ID NO: 39095 - DNA, 28 bp, synthetic construct
  source 1..28: mol_type = other DNA
tgtgagagtcccctggggtctgcagtgg

SEQ ID NO: 39096 - DNA, 28 bp, synthetic construct
  source 1..28: mol_type = other DNA
gtgagagtcccctggggtctgcagtggg

SEQ ID NO: 39097 - DNA, 28 bp, synthetic construct
  source 1..28: mol_type = other DNA
agagtcccctggggtctgcagtgggcgg

SEQ ID NO: 39098 - DNA, 28 bp, synthetic construct
  source 1..28: mol_type = other DNA
gagtcccctggggtctgcagtgggcggg

SEQ ID NO: 39099 - DNA, 28 bp, synthetic construct
  source 1..28: mol_type = other DNA
ctcgcccgcccactgcagaccccagggg

SEQ ID NO: 39100 - DNA, 28 bp, synthetic construct
  source 1..28: mol_type = other DNA
ccctggggtctgcagtgggcgggcgagg

SEQ ID NO: 39101 - DNA, 28 bp, synthetic construct
  source 1..28: mol_type = other DNA
acctcgcccgcccactgcagaccccagg

SEQ ID NO: 39102 - DNA, 28 bp, synthetic construct
  source 1..28: mol_type = other DNA
gggcagtgggcatgggcaggggctgtgg

SEQ ID NO: 39103 - DNA, 28 bp, synthetic construct
  source 1..28: mol_type = other DNA
aggctggggcagtgggcatgggcagggg

SEQ ID NO: 39104 - DNA, 28 bp, synthetic construct
  source 1..28: mol_type = other DNA
caggctggggcagtgggcatgggcaggg

SEQ ID NO: 39105 - DNA, 28 bp, synthetic construct
  source 1..28: mol_type = other DNA
cctgcccatgcccactgccccagcctgg

SEQ ID NO: 39106 - DNA, 28 bp, synthetic construct
  source 1..28: mol_type = other DNA
ctgcccatgcccactgccccagcctggg

SEQ ID NO: 39107 - DNA, 28 bp, synthetic construct
  source 1..28: mol_type = other DNA
cctcccaggctggggcagtgggcatggg

SEQ ID NO: 39108 - DNA, 28 bp, synthetic construct
  source 1..28: mol_type = other DNA
gcctcccaggctggggcagtgggcatgg

SEQ ID NO: 39109 - DNA, 28 bp, synthetic construct
  source 1..28: mol_type = other DNA
acggagcctcccaggctggggcagtggg

SEQ ID NO: 39110 - DNA, 28 bp, synthetic construct
  source 1..28: mol_type = other DNA
tacggagcctcccaggctggggcagtgg

SEQ ID NO: 39111 - DNA, 28 bp, synthetic construct
  source 1..28: mol_type = other DNA
ggcgggtacggagcctcccaggctgggg

SEQ ID NO: 39112 - DNA, 28 bp, synthetic construct
  source 1..28: mol_type = other DNA
gggcgggtacggagcctcccaggctggg

SEQ ID NO: 39113 - DNA, 28 bp, synthetic construct
  source 1..28: mol_type = other DNA
agggcgggtacggagcctcccaggctgg

SEQ ID NO: 39114 - DNA, 28 bp, synthetic construct
  source 1..28: mol_type = other DNA
aggcagggcgggtacggagcctcccagg

SEQ ID NO: 39115 - DNA, 28 bp, synthetic construct
  source 1..28: mol_type = other DNA
tgggaggctccgtacccgccctgcctgg

SEQ ID NO: 39116 - DNA, 28 bp, synthetic construct
  source 1..28: mol_type = other DNA
gtgggcaggccaggcagggcgggtacgg

SEQ ID NO: 39117 - DNA, 28 bp, synthetic construct
  source 1..28: mol_type = other DNA
tacccgccctgcctggcctgcccactgg

SEQ ID NO: 39118 - DNA, 28 bp, synthetic construct
  source 1..28: mol_type = other DNA
acccgccctgcctggcctgcccactggg

SEQ ID NO: 39119 - DNA, 28 bp, synthetic construct
  source 1..28: mol_type = other DNA
gcccagtgggcaggccaggcagggcggg

SEQ ID NO: 39120 - DNA, 28 bp, synthetic construct
  source 1..28: mol_type = other DNA
ggcccagtgggcaggccaggcagggcgg

SEQ ID NO: 39121 - DNA, 28 bp, synthetic construct
  source 1..28: mol_type = other DNA
ggaggcccagtgggcaggccaggcaggg

SEQ ID NO: 39122 - DNA, 28 bp, synthetic construct
  source 1..28: mol_type = other DNA
tggaggcccagtgggcaggccaggcagg

SEQ ID NO: 39123 - DNA, 28 bp, synthetic construct
  source 1..28: mol_type = other DNA
cttttggaggcccagtgggcaggccagg

SEQ ID NO: 39124 - DNA, 28 bp, synthetic construct
  source 1..28: mol_type = other DNA
taggacttttggaggcccagtgggcagg

SEQ ID NO: 39125 - DNA, 28 bp, synthetic construct
  source 1..28: mol_type = other DNA
tgcccactgggcctccaaaagtcctagg

SEQ ID NO: 39126 - DNA, 28 bp, synthetic construct
  source 1..28: mol_type = other DNA
gcccactgggcctccaaaagtcctaggg

SEQ ID NO: 39127 - DNA, 28 bp, synthetic construct
  source 1..28: mol_type = other DNA
tccctaggacttttggaggcccagtggg

SEQ ID NO: 39128 - DNA, 28 bp, synthetic construct
  source 1..28: mol_type = other DNA
ctccctaggacttttggaggcccagtgg

SEQ ID NO: 39129 - DNA, 28 bp, synthetic construct
  source 1..28: mol_type = other DNA
ctctctttctccctaggacttttggagg

SEQ ID NO: 39130 - DNA, 28 bp, synthetic construct
  source 1..28: mol_type = other DNA
tctctctctttctccctaggacttttgg

SEQ ID NO: 39131 - DNA, 28 bp, synthetic construct
  source 1..28: mol_type = other DNA
aagtcctagggagaaagagagagaaagg

SEQ ID NO: 39132 - DNA, 28 bp, synthetic construct
  source 1..28: mol_type = other DNA
ctctcctttctctctctttctccctagg

SEQ ID NO: 39133 - DNA, 28 bp, synthetic construct
  source 1..28: mol_type = other DNA
gagagatgagagaatgaccactctgagg

SEQ ID NO: 39134 - DNA, 28 bp, synthetic construct
  source 1..28: mol_type = other DNA
ggtcacagggcttggaacctcagagtgg

SEQ ID NO: 39135 - DNA, 28 bp, synthetic construct
  source 1..28: mol_type = other DNA
gcaactgagagagggtcacagggcttgg

SEQ ID NO: 39136 - DNA, 28 bp, synthetic construct
  source 1..28: mol_type = other DNA
agactgcaactgagagagggtcacaggg

SEQ ID NO: 39137 - DNA, 28 bp, synthetic construct
  source 1..28: mol_type = other DNA
aagactgcaactgagagagggtcacagg

SEQ ID NO: 39138 - DNA, 28 bp, synthetic construct
  source 1..28: mol_type = other DNA
gagggagaagactgcaactgagagaggg

SEQ ID NO: 39139 - DNA, 28 bp, synthetic construct
  source 1..28: mol_type = other DNA
agagggagaagactgcaactgagagagg

SEQ ID NO: 39140 - DNA, 28 bp, synthetic construct
  source 1..28: mol_type = other DNA
gcaggataaactgtagcagcacagaggg

SEQ ID NO: 39141 - DNA, 28 bp, synthetic construct
  source 1..28: mol_type = other DNA
ggcaggataaactgtagcagcacagagg

SEQ ID NO: 39142 - DNA, 28 bp, synthetic construct
  source 1..28: mol_type = other DNA
tgtgctgctacagtttatcctgccctgg

SEQ ID NO: 39143 - DNA, 28 bp, synthetic construct
  source 1..28: mol_type = other DNA
gctacagtttatcctgccctggctcagg

SEQ ID NO: 39144 - DNA, 28 bp, synthetic construct
  source 1..28: mol_type = other DNA
ctttagggctctggtcctgggcagctgg

SEQ ID NO: 39145 - DNA, 28 bp, synthetic construct
  source 1..28: mol_type = other DNA
gctgcccaggaccagagccctaaagcgg

SEQ ID NO: 39146 - DNA, 28 bp, synthetic construct
  source 1..28: mol_type = other DNA
ctgcccaggaccagagccctaaagcggg

SEQ ID NO: 39147 - DNA, 28 bp, synthetic construct
  source 1..28: mol_type = other DNA
tgtcccgctttagggctctggtcctggg

SEQ ID NO: 39148 - DNA, 28 bp, synthetic construct
  source 1..28: mol_type = other DNA
ctgtcccgctttagggctctggtcctgg

SEQ ID NO: 39149 - DNA, 28 bp, synthetic construct
  source 1..28: mol_type = other DNA
agatgactgtcccgctttagggctctgg

SEQ ID NO: 39150 - DNA, 28 bp, synthetic construct
  source 1..28: mol_type = other DNA
aaactgagatgactgtcccgctttaggg

SEQ ID NO: 39151 - DNA, 28 bp, synthetic construct
  source 1..28: mol_type = other DNA
gaaactgagatgactgtcccgctttagg

SEQ ID NO: 39152 - DNA, 28 bp, synthetic construct
  source 1..28: mol_type = other DNA
ttcttgccctgaagacctcctactcagg

SEQ ID NO: 39153 - DNA, 28 bp, synthetic construct
  source 1..28: mol_type = other DNA
ggggagcctgagtaggaggtcttcaggg

SEQ ID NO: 39154 - DNA, 28 bp, synthetic construct
  source 1..28: mol_type = other DNA
aggggagcctgagtaggaggtcttcagg

SEQ ID NO: 39155 - DNA, 28 bp, synthetic construct
  source 1..28: mol_type = other DNA
gtgggggcaggggagcctgagtaggagg

SEQ ID NO: 39156 - DNA, 28 bp, synthetic construct
  source 1..28: mol_type = other DNA
gtggtgggggcaggggagcctgagtagg

SEQ ID NO: 39157 - DNA, 28 bp, synthetic construct
  source 1..28: mol_type = other DNA
tggttgttagtggtggtgggggcagggg

SEQ ID NO: 39158 - DNA, 28 bp, synthetic construct
  source 1..28: mol_type = other DNA
ttggttgttagtggtggtgggggcaggg

SEQ ID NO: 39159 - DNA, 28 bp, synthetic construct
  source 1..28: mol_type = other DNA
cttggttgttagtggtggtgggggcagg

SEQ ID NO: 39160 - DNA, 28 bp, synthetic construct
  source 1..28: mol_type = other DNA
gatgcttggttgttagtggtggtggggg

SEQ ID NO: 39161 - DNA, 28 bp, synthetic construct
  source 1..28: mol_type = other DNA
agatgcttggttgttagtggtggtgggg

SEQ ID NO: 39162 - DNA, 28 bp, synthetic construct
  source 1..28: mol_type = other DNA
aagatgcttggttgttagtggtggtggg

SEQ ID NO: 39163 - DNA, 28 bp, synthetic construct
  source 1..28: mol_type = other DNA
gaagatgcttggttgttagtggtggtgg

SEQ ID NO: 39164 - DNA, 28 bp, synthetic construct
  source 1..28: mol_type = other DNA
taagaagatgcttggttgttagtggtgg

SEQ ID NO: 39165 - DNA, 28 bp, synthetic construct
  source 1..28: mol_type = other DNA
gggtaagaagatgcttggttgttagtgg

SEQ ID NO: 39166 - DNA, 28 bp, synthetic construct
  source 1..28: mol_type = other DNA
aacaaccaagcatcttcttacccgctgg

SEQ ID NO: 39167 - DNA, 28 bp, synthetic construct
  source 1..28: mol_type = other DNA
ggcggccagcgggtaagaagatgcttgg

SEQ ID NO: 39168 - DNA, 28 bp, synthetic construct
  source 1..28: mol_type = other DNA
ttacccgctggccgcctgcagagactgg

SEQ ID NO: 39169 - DNA, 28 bp, synthetic construct
  source 1..28: mol_type = other DNA
aagccagtctctgcaggcggccagcggg

SEQ ID NO: 39170 - DNA, 28 bp, synthetic construct
  source 1..28: mol_type = other DNA
gaagccagtctctgcaggcggccagcgg

SEQ ID NO: 39171 - DNA, 28 bp, synthetic construct
  source 1..28: mol_type = other DNA
gtatgtagaagccagtctctgcaggcgg

SEQ ID NO: 39172 - DNA, 28 bp, synthetic construct
  source 1..28: mol_type = other DNA
cctgcagagactggcttctacatactgg

SEQ ID NO: 39173 - DNA, 28 bp, synthetic construct
  source 1..28: mol_type = other DNA
ctgcagagactggcttctacatactggg

SEQ ID NO: 39174 - DNA, 28 bp, synthetic construct
  source 1..28: mol_type = other DNA
gagactggcttctacatactgggtcagg

SEQ ID NO: 39175 - DNA, 28 bp, synthetic construct
  source 1..28: mol_type = other DNA
ggcttctacatactgggtcaggttgagg

SEQ ID NO: 39176 - DNA, 28 bp, synthetic construct
  source 1..28: mol_type = other DNA
gcttctacatactgggtcaggttgaggg

SEQ ID NO: 39177 - DNA, 28 bp, synthetic construct
  source 1..28: mol_type = other DNA
acatactgggtcaggttgagggaactgg

SEQ ID NO: 39178 - DNA, 28 bp, synthetic construct
  source 1..28: mol_type = other DNA
catactgggtcaggttgagggaactggg

SEQ ID NO: 39179 - DNA, 28 bp, synthetic construct
  source 1..28: mol_type = other DNA
tgggccgtagctgctaaagacagagagg

SEQ ID NO: 39180 - DNA, 28 bp, synthetic construct
  source 1..28: mol_type = other DNA
gctgcctctctgtctttagcagctacgg

SEQ ID NO: 39181 - DNA, 28 bp, synthetic construct
  source 1..28: mol_type = other DNA
gctaaagacagagaggcagcgtcagtgg

SEQ ID NO: 39182 - DNA, 28 bp, synthetic construct
  source 1..28: mol_type = other DNA
cagagaggcagcgtcagtggaactctgg

SEQ ID NO: 39183 - DNA, 28 bp, synthetic construct
  source 1..28: mol_type = other DNA
agagaggcagcgtcagtggaactctggg

SEQ ID NO: 39184 - DNA, 28 bp, synthetic construct
  source 1..28: mol_type = other DNA
agtggaactctgggaccagcactcctgg

SEQ ID NO: 39185 - DNA, 28 bp, synthetic construct
  source 1..28: mol_type = other DNA
gtggaactctgggaccagcactcctggg

SEQ ID NO: 39186 - DNA, 28 bp, synthetic construct
  source 1..28: mol_type = other DNA
gaccagcactcctgggtccctgtcccgg

SEQ ID NO: 39187 - DNA, 28 bp, synthetic construct
  source 1..28: mol_type = other DNA
gaccgggacagggacccaggagtgctgg

SEQ ID NO: 39188 - DNA, 28 bp, synthetic construct
  source 1..28: mol_type = other DNA
agcaggaagaccgggacagggacccagg

SEQ ID NO: 39189 - DNA, 28 bp, synthetic construct
  source 1..28: mol_type = other DNA
aagaaagagcaggaagaccgggacaggg

SEQ ID NO: 39190 - DNA, 28 bp, synthetic construct
  source 1..28: mol_type = other DNA
aaagaaagagcaggaagaccgggacagg

SEQ ID NO: 39191 - DNA, 28 bp, synthetic construct
  source 1..28: mol_type = other DNA
ggaacaaagaaagagcaggaagaccggg

SEQ ID NO: 39192 - DNA, 28 bp, synthetic construct
  source 1..28: mol_type = other DNA
tggaacaaagaaagagcaggaagaccgg

SEQ ID NO: 39193 - DNA, 28 bp, synthetic construct
  source 1..28: mol_type = other DNA
cttcctgctctttctttgttccatttgg

SEQ ID NO: 39194 - DNA, 28 bp, synthetic construct
  source 1..28: mol_type = other DNA
ttcctgctctttctttgttccatttggg

SEQ ID NO: 39195 - DNA, 28 bp, synthetic construct
  source 1..28: mol_type = other DNA
agcccaaatggaacaaagaaagagcagg

SEQ ID NO: 39196 - DNA, 28 bp, synthetic construct
  source 1..28: mol_type = other DNA
ggagtattcttgagggaagcccaaatgg

SEQ ID NO: 39197 - DNA, 28 bp, synthetic construct
  source 1..28: mol_type = other DNA
tgggcttccctcaagaatactccagagg

SEQ ID NO: 39198 - DNA, 28 bp, synthetic construct
  source 1..28: mol_type = other DNA
gggggcacctctggagtattcttgaggg

SEQ ID NO: 39199 - DNA, 28 bp, synthetic construct
  source 1..28: mol_type = other DNA
ggggggcacctctggagtattcttgagg

SEQ ID NO: 39200 - DNA, 28 bp, synthetic construct
  source 1..28: mol_type = other DNA
ggcggccagcctggccagcctcgggagg

SEQ ID NO: 39201 - DNA, 28 bp, synthetic construct
  source 1..28: mol_type = other DNA
gcggccagcctggccagcctcgggaggg

SEQ ID NO: 39202 - DNA, 28 bp, synthetic construct
  source 1..28: mol_type = other DNA
aatgccctcccgaggctggccaggctgg

SEQ ID NO: 39203 - DNA, 28 bp, synthetic construct
  source 1..28: mol_type = other DNA
ggcgaatgccctcccgaggctggccagg

SEQ ID NO: 39204 - DNA, 28 bp, synthetic construct
  source 1..28: mol_type = other DNA
gcacgggcgaatgccctcccgaggctgg

SEQ ID NO: 39205 - DNA, 28 bp, synthetic construct
  source 1..28: mol_type = other DNA
agctgcacgggcgaatgccctcccgagg

SEQ ID NO: 39206 - DNA, 28 bp, synthetic construct
  source 1..28: mol_type = other DNA
gggagggggcgcggaggagctgcacggg

SEQ ID NO: 39207 - DNA, 28 bp, synthetic construct
  source 1..28: mol_type = other DNA
ggggagggggcgcggaggagctgcacgg

SEQ ID NO: 39208 - DNA, 28 bp, synthetic construct
  source 1..28: mol_type = other DNA
gaggcggctgggggagggggcgcggagg

SEQ ID NO: 39209 - DNA, 28 bp, synthetic construct
  source 1..28: mol_type = other DNA
ggcgaggcggctgggggagggggcgcgg

SEQ ID NO: 39210 - DNA, 28 bp, synthetic construct
  source 1..28: mol_type = other DNA
gcgccccctcccccagccgcctcgccgg

SEQ ID NO: 39211 - DNA, 28 bp, synthetic construct
  source 1..28: mol_type = other DNA
ccccctcccccagccgcctcgccggagg

SEQ ID NO: 39212 - DNA, 28 bp, synthetic construct
  source 1..28: mol_type = other DNA
tcctccggcgaggcggctgggggagggg

SEQ ID NO: 39213 - DNA, 28 bp, synthetic construct
  source 1..28: mol_type = other DNA
gtcctccggcgaggcggctgggggaggg

SEQ ID NO: 39214 - DNA, 28 bp, synthetic construct
  source 1..28: mol_type = other DNA
ggtcctccggcgaggcggctgggggagg

SEQ ID NO: 39215 - DNA, 28 bp, synthetic construct
  source 1..28: mol_type = other DNA
ctgggtcctccggcgaggcggctggggg

SEQ ID NO: 39216 - DNA, 28 bp, synthetic construct
  source 1..28: mol_type = other DNA
cctgggtcctccggcgaggcggctgggg

SEQ ID NO: 39217 - DNA, 28 bp, synthetic construct
  source 1..28: mol_type = other DNA
gcctgggtcctccggcgaggcggctggg

SEQ ID NO: 39218 - DNA, 28 bp, synthetic construct
  source 1..28: mol_type = other DNA
cgcctgggtcctccggcgaggcggctgg

SEQ ID NO: 39219 - DNA, 28 bp, synthetic construct
  source 1..28: mol_type = other DNA
ccgtcgcctgggtcctccggcgaggcgg

SEQ ID NO: 39220 - DNA, 28 bp, synthetic construct
  source 1..28: mol_type = other DNA
cgcctcgccggaggacccaggcgacggg

SEQ ID NO: 39221 - DNA, 28 bp, synthetic construct
  source 1..28: mol_type = other DNA
gcctcgccggaggacccaggcgacgggg

SEQ ID NO: 39222 - DNA, 28 bp, synthetic construct
  source 1..28: mol_type = other DNA
gccccgtcgcctgggtcctccggcgagg

SEQ ID NO: 39223 - DNA, 28 bp, synthetic construct
  source 1..28: mol_type = other DNA
tcgccggaggacccaggcgacggggcgg

SEQ ID NO: 39224 - DNA, 28 bp, synthetic construct
  source 1..28: mol_type = other DNA
cgccggaggacccaggcgacggggcggg

SEQ ID NO: 39225 - DNA, 28 bp, synthetic construct
  source 1..28: mol_type = other DNA
cgcccgccccgtcgcctgggtcctccgg

SEQ ID NO: 39226 - DNA, 28 bp, synthetic construct
  source 1..28: mol_type = other DNA
agcaggctcgcccgccccgtcgcctggg

SEQ ID NO: 39227 - DNA, 28 bp, synthetic construct
  source 1..28: mol_type = other DNA
aagcaggctcgcccgccccgtcgcctgg

SEQ ID NO: 39228 - DNA, 28 bp, synthetic construct
  source 1..28: mol_type = other DNA
agcctgcttccccgcctgactcacctgg

SEQ ID NO: 39229 - DNA, 28 bp, synthetic construct
  source 1..28: mol_type = other DNA
ctccaggtgagtcaggcggggaagcagg

SEQ ID NO: 39230 - DNA, 28 bp, synthetic construct
  source 1..28: mol_type = other DNA
gcttccccgcctgactcacctggagtgg

SEQ ID NO: 39231 - DNA, 28 bp, synthetic construct
  source 1..28: mol_type = other DNA
cttccccgcctgactcacctggagtggg

SEQ ID NO: 39232 - DNA, 28 bp, synthetic construct
  source 1..28: mol_type = other DNA
cctcccactccaggtgagtcaggcgggg

SEQ ID NO: 39233 - DNA, 28 bp, synthetic construct
  source 1..28: mol_type = other DNA
cccgcctgactcacctggagtgggaggg

SEQ ID NO: 39234 - DNA, 28 bp, synthetic construct
  source 1..28: mol_type = other DNA
ccgcctgactcacctggagtgggagggg

SEQ ID NO: 39235 - DNA, 28 bp, synthetic construct
  source 1..28: mol_type = other DNA
cgcctgactcacctggagtgggaggggg

SEQ ID NO: 39236 - DNA, 28 bp, synthetic construct
  source 1..28: mol_type = other DNA
ttccccctcccactccaggtgagtcagg

SEQ ID NO: 39237 - DNA, 28 bp, synthetic construct
  source 1..28: mol_type = other DNA
tgactcacctggagtgggagggggaagg

SEQ ID NO: 39238 - DNA, 28 bp, synthetic construct
  source 1..28: mol_type = other DNA
gactcacctggagtgggagggggaaggg

SEQ ID NO: 39239 - DNA, 28 bp, synthetic construct
  source 1..28: mol_type = other DNA
tcacctggagtgggagggggaagggagg

SEQ ID NO: 39240 - DNA, 28 bp, synthetic construct
  source 1..28: mol_type = other DNA
ccgcctcccttccccctcccactccagg

SEQ ID NO: 39241 - DNA, 28 bp, synthetic construct
  source 1..28: mol_type = other DNA
ggagtgggagggggaagggaggcggcgg

SEQ ID NO: 39242 - DNA, 28 bp, synthetic construct
  source 1..28: mol_type = other DNA
ggggaagggaggcggcggagccccgagg

SEQ ID NO: 39243 - DNA, 28 bp, synthetic construct
  source 1..28: mol_type = other DNA
gggaggcggcggagccccgaggtcccgg

SEQ ID NO: 39244 - DNA, 28 bp, synthetic construct
  source 1..28: mol_type = other DNA
cggcggagccccgaggtcccggcgtcgg

SEQ ID NO: 39245 - DNA, 28 bp, synthetic construct
  source 1..28: mol_type = other DNA
ggcggagccccgaggtcccggcgtcggg

SEQ ID NO: 39246 - DNA, 28 bp, synthetic construct
  source 1..28: mol_type = other DNA
gagactgcccgacgccgggacctcgggg

SEQ ID NO: 39247 - DNA, 28 bp, synthetic construct
  source 1..28: mol_type = other DNA
agagactgcccgacgccgggacctcggg

SEQ ID NO: 39248 - DNA, 28 bp, synthetic construct
  source 1..28: mol_type = other DNA
aagagactgcccgacgccgggacctcgg

SEQ ID NO: 39249 - DNA, 28 bp, synthetic construct
  source 1..28: mol_type = other DNA
gaggtcccggcgtcgggcagtctcttgg

SEQ ID NO: 39250 - DNA, 28 bp, synthetic construct
  source 1..28: mol_type = other DNA
tcccggcgtcgggcagtctcttggatgg

SEQ ID NO: 39251 - DNA, 28 bp, synthetic construct
  source 1..28: mol_type = other DNA
tccatccaagagactgcccgacgccggg

SEQ ID NO: 39252 - DNA, 28 bp, synthetic construct
  source 1..28: mol_type = other DNA
ctccatccaagagactgcccgacgccgg

SEQ ID NO: 39253 - DNA, 28 bp, synthetic construct
  source 1..28: mol_type = other DNA
ctcttggatggagcgtcgcaatgtccgg

SEQ ID NO: 39254 - DNA, 28 bp, synthetic construct
  source 1..28: mol_type = other DNA
tcttggatggagcgtcgcaatgtccggg

SEQ ID NO: 39255 - DNA, 28 bp, synthetic construct
  source 1..28: mol_type = other DNA
cttggatggagcgtcgcaatgtccgggg

SEQ ID NO: 39256 - DNA, 28 bp, synthetic construct
  source 1..28: mol_type = other DNA
tcgcaatgtccggggctcgccgtactgg

SEQ ID NO: 39257 - DNA, 28 bp, synthetic construct
  source 1..28: mol_type = other DNA
cgcaatgtccggggctcgccgtactggg

SEQ ID NO: 39258 - DNA, 28 bp, synthetic construct
  source 1..28: mol_type = other DNA
gcaatgtccggggctcgccgtactgggg

SEQ ID NO: 39259 - DNA, 28 bp, synthetic construct
  source 1..28: mol_type = other DNA
caatgtccggggctcgccgtactggggg

SEQ ID NO: 39260 - DNA, 28 bp, synthetic construct
  source 1..28: mol_type = other DNA
aatgtccggggctcgccgtactgggggg

SEQ ID NO: 39261 - DNA, 28 bp, synthetic construct
  source 1..28: mol_type = other DNA
aggagccccccagtacggcgagccccgg

SEQ ID NO: 39262 - DNA, 28 bp, synthetic construct
  source 1..28: mol_type = other DNA
ggggctcgccgtactggggggctcctgg

SEQ ID NO: 39263 - DNA, 28 bp, synthetic construct
  source 1..28: mol_type = other DNA
gggctcgccgtactggggggctcctggg

SEQ ID NO: 39264 - DNA, 28 bp, synthetic construct
  source 1..28: mol_type = other DNA
ggctcgccgtactggggggctcctgggg

SEQ ID NO: 39265 - DNA, 28 bp, synthetic construct
  source 1..28: mol_type = other DNA
gctcgccgtactggggggctcctggggg

SEQ ID NO: 39266 - DNA, 28 bp, synthetic construct
  source 1..28: mol_type = other DNA
ctcgccgtactggggggctcctgggggg

SEQ ID NO: 39267 - DNA, 28 bp, synthetic construct
  source 1..28: mol_type = other DNA
tcgccgtactggggggctcctggggggg

SEQ ID NO: 39268 - DNA, 28 bp, synthetic construct
  source 1..28: mol_type = other DNA
gtgcccccccaggagccccccagtacgg

SEQ ID NO: 39269 - DNA, 28 bp, synthetic construct
  source 1..28: mol_type = other DNA
gtactggggggctcctgggggggcacgg

SEQ ID NO: 39270 - DNA, 28 bp, synthetic construct
  source 1..28: mol_type = other DNA
ggggctcctgggggggcacggctctagg

SEQ ID NO: 39271 - DNA, 28 bp, synthetic construct
  source 1..28: mol_type = other DNA
ctcctgggggggcacggctctaggctgg

SEQ ID NO: 39272 - DNA, 28 bp, synthetic construct
  source 1..28: mol_type = other DNA
tcctgggggggcacggctctaggctggg

SEQ ID NO: 39273 - DNA, 28 bp, synthetic construct
  source 1..28: mol_type = other DNA
tcccagcctagagccgtgcccccccagg

SEQ ID NO: 39274 - DNA, 28 bp, synthetic construct
  source 1..28: mol_type = other DNA
gcacggctctaggctgggactgtcccgg

SEQ ID NO: 39275 - DNA, 28 bp, synthetic construct
  source 1..28: mol_type = other DNA
cacggctctaggctgggactgtcccggg

SEQ ID NO: 39276 - DNA, 28 bp, synthetic construct
  source 1..28: mol_type = other DNA
acggctctaggctgggactgtcccgggg

SEQ ID NO: 39277 - DNA, 28 bp, synthetic construct
  source 1..28: mol_type = other DNA
aggctgggactgtcccggggcctctcgg

SEQ ID NO: 39278 - DNA, 28 bp, synthetic construct
  source 1..28: mol_type = other DNA
gggcgggcgggctccgagaggccccggg

SEQ ID NO: 39279 - DNA, 28 bp, synthetic construct
  source 1..28: mol_type = other DNA
tgggcgggcgggctccgagaggccccgg

SEQ ID NO: 39280 - DNA, 28 bp, synthetic construct
  source 1..28: mol_type = other DNA
gtcacgtgggcgggcgggctccgagagg

SEQ ID NO: 39281 - DNA, 28 bp, synthetic construct
  source 1..28: mol_type = other DNA
ttttggggcggtcacgtgggcgggcggg

SEQ ID NO: 39282 - DNA, 28 bp, synthetic construct
  source 1..28: mol_type = other DNA
attttggggcggtcacgtgggcgggcgg

SEQ ID NO: 39283 - DNA, 28 bp, synthetic construct
  source 1..28: mol_type = other DNA
gatattttggggcggtcacgtgggcggg

SEQ ID NO: 39284 - DNA, 28 bp, synthetic construct
  source 1..28: mol_type = other DNA
ggatattttggggcggtcacgtgggcgg

SEQ ID NO: 39285 - DNA, 28 bp, synthetic construct
  source 1..28: mol_type = other DNA
gtcggatattttggggcggtcacgtggg

SEQ ID NO: 39286 - DNA, 28 bp, synthetic construct
  source 1..28: mol_type = other DNA
tgtcggatattttggggcggtcacgtgg

SEQ ID NO: 39287 - DNA, 28 bp, synthetic construct
  source 1..28: mol_type = other DNA
agaaaatgtgtcggatattttggggcgg

SEQ ID NO: 39288 - DNA, 28 bp, synthetic construct
  source 1..28: mol_type = other DNA
gggagaaaatgtgtcggatattttgggg

SEQ ID NO: 39289 - DNA, 28 bp, synthetic construct
  source 1..28: mol_type = other DNA
tgggagaaaatgtgtcggatattttggg

SEQ ID NO: 39290 - DNA, 28 bp, synthetic construct
  source 1..28: mol_type = other DNA
ttgggagaaaatgtgtcggatattttgg

SEQ ID NO: 39291 - DNA, 28 bp, synthetic construct
  source 1..28: mol_type = other DNA
gtgtgcggtttgggagaaaatgtgtcgg

SEQ ID NO: 39292 - DNA, 28 bp, synthetic construct
  source 1..28: mol_type = other DNA
ctcccaaaccgcacactgactctgcagg

SEQ ID NO: 39293 - DNA, 28 bp, synthetic construct
  source 1..28: mol_type = other DNA
cgcctgcagagtcagtgtgcggtttggg

SEQ ID NO: 39294 - DNA, 28 bp, synthetic construct
  source 1..28: mol_type = other DNA
ccgcctgcagagtcagtgtgcggtttgg

SEQ ID NO: 39295 - DNA, 28 bp, synthetic construct
  source 1..28: mol_type = other DNA
caaaccgcacactgactctgcaggcggg

SEQ ID NO: 39296 - DNA, 28 bp, synthetic construct
  source 1..28: mol_type = other DNA
aaaccgcacactgactctgcaggcgggg

SEQ ID NO: 39297 - DNA, 28 bp, synthetic construct
  source 1..28: mol_type = other DNA
tgtccccgcctgcagagtcagtgtgcgg

SEQ ID NO: 39298 - DNA, 28 bp, synthetic construct
  source 1..28: mol_type = other DNA
cacactgactctgcaggcggggacacgg

SEQ ID NO: 39299 - DNA, 28 bp, synthetic construct
  source 1..28: mol_type = other DNA
agggaggttggggggggggtggggaggg

SEQ ID NO: 39300 - DNA, 28 bp, synthetic construct
  source 1..28: mol_type = other DNA
gagggaggttggggggggggtggggagg

SEQ ID NO: 39301 - DNA, 28 bp, synthetic construct
  source 1..28: mol_type = other DNA
agggagggaggttggggggggggtgggg

SEQ ID NO: 39302 - DNA, 28 bp, synthetic construct
  source 1..28: mol_type = other DNA
cagggagggaggttggggggggggtggg

SEQ ID NO: 39303 - DNA, 28 bp, synthetic construct
  source 1..28: mol_type = other DNA
gcagggagggaggttggggggggggtgg

SEQ ID NO: 39304 - DNA, 28 bp, synthetic construct
  source 1..28: mol_type = other DNA
tgggcagggagggaggttgggggggggg

SEQ ID NO: 39305 - DNA, 28 bp, synthetic construct
  source 1..28: mol_type = other DNA
ttgggcagggagggaggttggggggggg

SEQ ID NO: 39306 - DNA, 28 bp, synthetic construct
  source 1..28: mol_type = other DNA
gttgggcagggagggaggttgggggggg

SEQ ID NO: 39307 - DNA, 28 bp, synthetic construct
  source 1..28: mol_type = other DNA
agttgggcagggagggaggttggggggg

SEQ ID NO: 39308 - DNA, 28 bp, synthetic construct
  source 1..28: mol_type = other DNA
gagttgggcagggagggaggttgggggg

SEQ ID NO: 39309 - DNA, 28 bp, synthetic construct
  source 1..28: mol_type = other DNA
ggagttgggcagggagggaggttggggg

SEQ ID NO: 39310 - DNA, 28 bp, synthetic construct
  source 1..28: mol_type = other DNA
gggagttgggcagggagggaggttgggg

SEQ ID NO: 39311 - DNA, 28 bp, synthetic construct
  source 1..28: mol_type = other DNA
agggagttgggcagggagggaggttggg

SEQ ID NO: 39312 - DNA, 28 bp, synthetic construct
  source 1..28: mol_type = other DNA
gagggagttgggcagggagggaggttgg

SEQ ID NO: 39313 - DNA, 28 bp, synthetic construct
  source 1..28: mol_type = other DNA
ggaggagggagttgggcagggagggagg

SEQ ID NO: 39314 - DNA, 28 bp, synthetic construct
  source 1..28: mol_type = other DNA
gggggaggagggagttgggcagggaggg

SEQ ID NO: 39315 - DNA, 28 bp, synthetic construct
  source 1..28: mol_type = other DNA
agggggaggagggagttgggcagggagg

SEQ ID NO: 39316 - DNA, 28 bp, synthetic construct
  source 1..28: mol_type = other DNA
gggagggggaggagggagttgggcaggg

SEQ ID NO: 39317 - DNA, 28 bp, synthetic construct
  source 1..28: mol_type = other DNA
cgggagggggaggagggagttgggcagg

SEQ ID NO: 39318 - DNA, 28 bp, synthetic construct
  source 1..28: mol_type = other DNA
agggcgggagggggaggagggagttggg

SEQ ID NO: 39319 - DNA, 28 bp, synthetic construct
  source 1..28: mol_type = other DNA
gagggcgggagggggaggagggagttgg

SEQ ID NO: 39320 - DNA, 28 bp, synthetic construct
  source 1..28: mol_type = other DNA
aggagcgagggcgggagggggaggaggg

SEQ ID NO: 39321 - DNA, 28 bp, synthetic construct
  source 1..28: mol_type = other DNA
gaggagcgagggcgggagggggaggagg

SEQ ID NO: 39322 - DNA, 28 bp, synthetic construct
  source 1..28: mol_type = other DNA
agggaggagcgagggcgggagggggagg

SEQ ID NO: 39323 - DNA, 28 bp, synthetic construct
  source 1..28: mol_type = other DNA
gggagggaggagcgagggcgggaggggg

SEQ ID NO: 39324 - DNA, 28 bp, synthetic construct
  source 1..28: mol_type = other DNA
ggggagggaggagcgagggcgggagggg

SEQ ID NO: 39325 - DNA, 28 bp, synthetic construct
  source 1..28: mol_type = other DNA
aggggagggaggagcgagggcgggaggg

SEQ ID NO: 39326 - DNA, 28 bp, synthetic construct
  source 1..28: mol_type = other DNA
caggggagggaggagcgagggcgggagg

SEQ ID NO: 39327 - DNA, 28 bp, synthetic construct
  source 1..28: mol_type = other DNA
aggcaggggagggaggagcgagggcggg

SEQ ID NO: 39328 - DNA, 28 bp, synthetic construct
  source 1..28: mol_type = other DNA
caggcaggggagggaggagcgagggcgg

SEQ ID NO: 39329 - DNA, 28 bp, synthetic construct
  source 1..28: mol_type = other DNA
gggcaggcaggggagggaggagcgaggg

SEQ ID NO: 39330 - DNA, 28 bp, synthetic construct
  source 1..28: mol_type = other DNA
ggggcaggcaggggagggaggagcgagg

SEQ ID NO: 39331 - DNA, 28 bp, synthetic construct
  source 1..28: mol_type = other DNA
ccgggcaggggcaggcaggggagggagg

SEQ ID NO: 39332 - DNA, 28 bp, synthetic construct
  source 1..28: mol_type = other DNA
gagccgggcaggggcaggcaggggaggg

SEQ ID NO: 39333 - DNA, 28 bp, synthetic construct
  source 1..28: mol_type = other DNA
ggagccgggcaggggcaggcaggggagg

SEQ ID NO: 39334 - DNA, 28 bp, synthetic construct
  source 1..28: mol_type = other DNA
gagggagccgggcaggggcaggcagggg

SEQ ID NO: 39335 - DNA, 28 bp, synthetic construct
  source 1..28: mol_type = other DNA
ggagggagccgggcaggggcaggcaggg

SEQ ID NO: 39336 - DNA, 28 bp, synthetic construct
  source 1..28: mol_type = other DNA
aggagggagccgggcaggggcaggcagg

SEQ ID NO: 39337 - DNA, 28 bp, synthetic construct
  source 1..28: mol_type = other DNA
acagaggagggagccgggcaggggcagg

SEQ ID NO: 39338 - DNA, 28 bp, synthetic construct
  source 1..28: mol_type = other DNA
gggcacagaggagggagccgggcagggg

SEQ ID NO: 39339 - DNA, 28 bp, synthetic construct
  source 1..28: mol_type = other DNA
agggcacagaggagggagccgggcaggg

SEQ ID NO: 39340 - DNA, 28 bp, synthetic construct
  source 1..28: mol_type = other DNA
cagggcacagaggagggagccgggcagg

SEQ ID NO: 39341 - DNA, 28 bp, synthetic construct
  source 1..28: mol_type = other DNA
ctgcccggctccctcctctgtgccctgg

SEQ ID NO: 39342 - DNA, 28 bp, synthetic construct
  source 1..28: mol_type = other DNA
tgcccggctccctcctctgtgccctggg

SEQ ID NO: 39343 - DNA, 28 bp, synthetic construct
  source 1..28: mol_type = other DNA
gcccggctccctcctctgtgccctgggg

SEQ ID NO: 39344 - DNA, 28 bp, synthetic construct
  source 1..28: mol_type = other DNA
gccccagggcacagaggagggagccggg

SEQ ID NO: 39345 - DNA, 28 bp, synthetic construct
  source 1..28: mol_type = other DNA
agccccagggcacagaggagggagccgg

SEQ ID NO: 39346 - DNA, 28 bp, synthetic construct
  source 1..28: mol_type = other DNA
ggctccctcctctgtgccctggggctgg

SEQ ID NO: 39347 - DNA, 28 bp, synthetic construct
  source 1..28: mol_type = other DNA
gctccctcctctgtgccctggggctggg

SEQ ID NO: 39348 - DNA, 28 bp, synthetic construct
  source 1..28: mol_type = other DNA
ctccctcctctgtgccctggggctgggg

SEQ ID NO: 39349 - DNA, 28 bp, synthetic construct
  source 1..28: mol_type = other DNA
tccctcctctgtgccctggggctggggg

SEQ ID NO: 39350 - DNA, 28 bp, synthetic construct
  source 1..28: mol_type = other DNA
ccccccagccccagggcacagaggaggg

SEQ ID NO: 39351 - DNA, 28 bp, synthetic construct
  source 1..28: mol_type = other DNA
gccccccagccccagggcacagaggagg

SEQ ID NO: 39352 - DNA, 28 bp, synthetic construct
  source 1..28: mol_type = other DNA
tcctctgtgccctggggctggggggcgg

SEQ ID NO: 39353 - DNA, 28 bp, synthetic construct
  source 1..28: mol_type = other DNA
tccgccccccagccccagggcacagagg

SEQ ID NO: 39354 - DNA, 28 bp, synthetic construct
  source 1..28: mol_type = other DNA
tctgtgccctggggctggggggcggagg

SEQ ID NO: 39355 - DNA, 28 bp, synthetic construct
  source 1..28: mol_type = other DNA
ctgtgccctggggctggggggcggaggg

SEQ ID NO: 39356 - DNA, 28 bp, synthetic construct
  source 1..28: mol_type = other DNA
gccctggggctggggggcggagggatgg

SEQ ID NO: 39357 - DNA, 28 bp, synthetic construct
  source 1..28: mol_type = other DNA
ccctggggctggggggcggagggatggg

SEQ ID NO: 39358 - DNA, 28 bp, synthetic construct
  source 1..28: mol_type = other DNA
acccatccctccgccccccagccccagg

SEQ ID NO: 39359 - DNA, 28 bp, synthetic construct
  source 1..28: mol_type = other DNA
tggggctggggggcggagggatgggtgg

SEQ ID NO: 39360 - DNA, 28 bp, synthetic construct
  source 1..28: mol_type = other DNA
ggggctggggggcggagggatgggtggg

SEQ ID NO: 39361 - DNA, 28 bp, synthetic construct
  source 1..28: mol_type = other DNA
gctggggggcggagggatgggtgggcgg

SEQ ID NO: 39362 - DNA, 28 bp, synthetic construct
  source 1..28: mol_type = other DNA
ctggggggcggagggatgggtgggcggg

SEQ ID NO: 39363 - DNA, 28 bp, synthetic construct
  source 1..28: mol_type = other DNA
gggggcggagggatgggtgggcgggagg

SEQ ID NO: 39364 - DNA, 28 bp, synthetic construct
  source 1..28: mol_type = other DNA
ggggcggagggatgggtgggcgggaggg

SEQ ID NO: 39365 - DNA, 28 bp, synthetic construct
  source 1..28: mol_type = other DNA
gggcggagggatgggtgggcgggagggg

SEQ ID NO: 39366 - DNA, 28 bp, synthetic construct
  source 1..28: mol_type = other DNA
ggcggagggatgggtgggcgggaggggg

SEQ ID NO: 39367 - DNA, 28 bp, synthetic construct
  source 1..28: mol_type = other DNA
agggatgggtgggcgggagggggactgg

SEQ ID NO: 39368 - DNA, 28 bp, synthetic construct
  source 1..28: mol_type = other DNA
gggatgggtgggcgggagggggactggg

SEQ ID NO: 39369 - DNA, 28 bp, synthetic construct
  source 1..28: mol_type = other DNA
atgggtgggcgggagggggactgggcgg

SEQ ID NO: 39370 - DNA, 28 bp, synthetic construct
  source 1..28: mol_type = other DNA
tgggtgggcgggagggggactgggcggg

SEQ ID NO: 39371 - DNA, 28 bp, synthetic construct
  source 1..28: mol_type = other DNA
gggtgggcgggagggggactgggcgggg

SEQ ID NO: 39372 - DNA, 28 bp, synthetic construct
  source 1..28: mol_type = other DNA
tgggcgggagggggactgggcggggcgg

SEQ ID NO: 39373 - DNA, 28 bp, synthetic construct
  source 1..28: mol_type = other DNA
gggagggggactgggcggggcggcccgg

SEQ ID NO: 39374 - DNA, 28 bp, synthetic construct
  source 1..28: mol_type = other DNA
ggagggggactgggcggggcggcccggg

SEQ ID NO: 39375 - DNA, 28 bp, synthetic construct
  source 1..28: mol_type = other DNA
actgggcggggcggcccgggacgcctgg

SEQ ID NO: 39376 - DNA, 28 bp, synthetic construct
  source 1..28: mol_type = other DNA
ctgggcggggcggcccgggacgcctggg

SEQ ID NO: 39377 - DNA, 28 bp, synthetic construct
  source 1..28: mol_type = other DNA
ggaagggcagagacccaggcgtcccggg

SEQ ID NO: 39378 - DNA, 28 bp, synthetic construct
  source 1..28: mol_type = other DNA
gggaagggcagagacccaggcgtcccgg

SEQ ID NO: 39379 - DNA, 28 bp, synthetic construct
  source 1..28: mol_type = other DNA
tagcaaatgggaagggcagagacccagg

SEQ ID NO: 39380 - DNA, 28 bp, synthetic construct
  source 1..28: mol_type = other DNA
tgggtctctgcccttcccatttgctagg

SEQ ID NO: 39381 - DNA, 28 bp, synthetic construct
  source 1..28: mol_type = other DNA
gtcacggaagcctagcaaatgggaaggg

SEQ ID NO: 39382 - DNA, 28 bp, synthetic construct
  source 1..28: mol_type = other DNA
agtcacggaagcctagcaaatgggaagg

SEQ ID NO: 39383 - DNA, 28 bp, synthetic construct
  source 1..28: mol_type = other DNA
atggagtcacggaagcctagcaaatggg

SEQ ID NO: 39384 - DNA, 28 bp, synthetic construct
  source 1..28: mol_type = other DNA
gatggagtcacggaagcctagcaaatgg

SEQ ID NO: 39385 - DNA, 28 bp, synthetic construct
  source 1..28: mol_type = other DNA
gctaggcttccgtgactccatcctctgg

SEQ ID NO: 39386 - DNA, 28 bp, synthetic construct
  source 1..28: mol_type = other DNA
ctaggcttccgtgactccatcctctggg

SEQ ID NO: 39387 - DNA, 28 bp, synthetic construct
  source 1..28: mol_type = other DNA
ggcttccgtgactccatcctctgggagg

SEQ ID NO: 39388 - DNA, 28 bp, synthetic construct
  source 1..28: mol_type = other DNA
tccgtgactccatcctctgggaggccgg

SEQ ID NO: 39389 - DNA, 28 bp, synthetic construct
  source 1..28: mol_type = other DNA
cccggcctcccagaggatggagtcacgg

SEQ ID NO: 39390 - DNA, 28 bp, synthetic construct
  source 1..28: mol_type = other DNA
actccatcctctgggaggccgggcacgg

SEQ ID NO: 39391 - DNA, 28 bp, synthetic construct
  source 1..28: mol_type = other DNA
cagccgtgcccggcctcccagaggatgg

SEQ ID NO: 39392 - DNA, 28 bp, synthetic construct
  source 1..28: mol_type = other DNA
catcctctgggaggccgggcacggctgg

SEQ ID NO: 39393 - DNA, 28 bp, synthetic construct
  source 1..28: mol_type = other DNA
ctgccagccgtgcccggcctcccagagg

SEQ ID NO: 39394 - DNA, 28 bp, synthetic construct
  source 1..28: mol_type = other DNA
ctgggaggccgggcacggctggcagagg

SEQ ID NO: 39395 - DNA, 28 bp, synthetic construct
  source 1..28: mol_type = other DNA
ggaggccgggcacggctggcagaggagg

SEQ ID NO: 39396 - DNA, 28 bp, synthetic construct
  source 1..28: mol_type = other DNA
actgacctcctctgccagccgtgcccgg

SEQ ID NO: 39397 - DNA, 28 bp, synthetic construct
  source 1..28: mol_type = other DNA
cggctggcagaggaggtcagtgtcctgg

SEQ ID NO: 39398 - DNA, 28 bp, synthetic construct
  source 1..28: mol_type = other DNA
gagaaaaggttggcatcacggggccagg

SEQ ID NO: 39399 - DNA, 28 bp, synthetic construct
  source 1..28: mol_type = other DNA
ccccgtgatgccaaccttttctctctgg

SEQ ID NO: 39400 - DNA, 28 bp, synthetic construct
  source 1..28: mol_type = other DNA
gccagagagaaaaggttggcatcacggg

SEQ ID NO: 39401 - DNA, 28 bp, synthetic construct
  source 1..28: mol_type = other DNA
tgccagagagaaaaggttggcatcacgg

SEQ ID NO: 39402 - DNA, 28 bp, synthetic construct
  source 1..28: mol_type = other DNA
gagaaaagtgccagagagaaaaggttgg

SEQ ID NO: 39403 - DNA, 28 bp, synthetic construct
  source 1..28: mol_type = other DNA
aaaggagaaaagtgccagagagaaaagg

SEQ ID NO: 39404 - DNA, 28 bp, synthetic construct
  source 1..28: mol_type = other DNA
tggcacttttctcctttctgccttttgg

SEQ ID NO: 39405 - DNA, 28 bp, synthetic construct
  source 1..28: mol_type = other DNA
ggcacttttctcctttctgccttttggg

SEQ ID NO: 39406 - DNA, 28 bp, synthetic construct
  source 1..28: mol_type = other DNA
gcacttttctcctttctgccttttgggg

SEQ ID NO: 39407 - DNA, 28 bp, synthetic construct
  source 1..28: mol_type = other DNA
cacttttctcctttctgccttttggggg

SEQ ID NO: 39408 - DNA, 28 bp, synthetic construct
  source 1..28: mol_type = other DNA
acttttctcctttctgccttttgggggg

SEQ ID NO: 39409 - DNA, 28 bp, synthetic construct
  source 1..28: mol_type = other DNA
caactagtccccccaaaaggcagaaagg

SEQ ID NO: 39410 - DNA, 28 bp, synthetic construct
  source 1..28: mol_type = other DNA
agacaactcaactagtccccccaaaagg

SEQ ID NO: 39411 - DNA, 28 bp, synthetic construct
  source 1..28: mol_type = other DNA
ttggggggactagttgagttgtctgtgg

SEQ ID NO: 39412 - DNA, 28 bp, synthetic construct
  source 1..28: mol_type = other DNA
gggactagttgagttgtctgtggccagg

SEQ ID NO: 39413 - DNA, 28 bp, synthetic construct
  source 1..28: mol_type = other DNA
ctgtggccaggctgtgactcttgcgagg

SEQ ID NO: 39414 - DNA, 28 bp, synthetic construct
  source 1..28: mol_type = other DNA
gactggcctcgcaagagtcacagcctgg

SEQ ID NO: 39415 - DNA, 28 bp, synthetic construct
  source 1..28: mol_type = other DNA
ctgtgactcttgcgaggccagtctctgg

SEQ ID NO: 39416 - DNA, 28 bp, synthetic construct
  source 1..28: mol_type = other DNA
cgaggccagtctctggcgcctccccagg

SEQ ID NO: 39417 - DNA, 28 bp, synthetic construct
  source 1..28: mol_type = other DNA
gaggccagtctctggcgcctccccaggg

SEQ ID NO: 39418 - DNA, 28 bp, synthetic construct
  source 1..28: mol_type = other DNA
cctaccctggggaggcgccagagactgg

SEQ ID NO: 39419 - DNA, 28 bp, synthetic construct
  source 1..28: mol_type = other DNA
tctggcgcctccccagggtaggcaatgg

SEQ ID NO: 39420 - DNA, 28 bp, synthetic construct
  source 1..28: mol_type = other DNA
ctggcgcctccccagggtaggcaatggg

SEQ ID NO: 39421 - DNA, 28 bp, synthetic construct
  source 1..28: mol_type = other DNA
tggcgcctccccagggtaggcaatgggg

SEQ ID NO: 39422 - DNA, 28 bp, synthetic construct
  source 1..28: mol_type = other DNA
cgcctccccagggtaggcaatggggcgg

SEQ ID NO: 39423 - DNA, 28 bp, synthetic construct
  source 1..28: mol_type = other DNA
taccgccccattgcctaccctggggagg

SEQ ID NO: 39424 - DNA, 28 bp, synthetic construct
  source 1..28: mol_type = other DNA
gggtaccgccccattgcctaccctgggg

SEQ ID NO: 39425 - DNA, 28 bp, synthetic construct
  source 1..28: mol_type = other DNA
tgggtaccgccccattgcctaccctggg

SEQ ID NO: 39426 - DNA, 28 bp, synthetic construct
  source 1..28: mol_type = other DNA
gtgggtaccgccccattgcctaccctgg

SEQ ID NO: 39427 - DNA, 28 bp, synthetic construct
  source 1..28: mol_type = other DNA
ggcggtacccactccctcccagtgctgg

SEQ ID NO: 39428 - DNA, 28 bp, synthetic construct
  source 1..28: mol_type = other DNA
tacccactccctcccagtgctggattgg

SEQ ID NO: 39429 - DNA, 28 bp, synthetic construct
  source 1..28: mol_type = other DNA
ggccaatccagcactgggagggagtggg

SEQ ID NO: 39430 - DNA, 28 bp, synthetic construct
  source 1..28: mol_type = other DNA
cggccaatccagcactgggagggagtgg

SEQ ID NO: 39431 - DNA, 28 bp, synthetic construct
  source 1..28: mol_type = other DNA
cactccctcccagtgctggattggccgg

SEQ ID NO: 39432 - DNA, 28 bp, synthetic construct
  source 1..28: mol_type = other DNA
actccctcccagtgctggattggccggg

SEQ ID NO: 39433 - DNA, 28 bp, synthetic construct
  source 1..28: mol_type = other DNA
ctgcccggccaatccagcactgggaggg

SEQ ID NO: 39434 - DNA, 28 bp, synthetic construct
  source 1..28: mol_type = other DNA
cctcccagtgctggattggccgggcagg

SEQ ID NO: 39435 - DNA, 28 bp, synthetic construct
  source 1..28: mol_type = other DNA
actcctgcccggccaatccagcactggg

SEQ ID NO: 39436 - DNA, 28 bp, synthetic construct
  source 1..28: mol_type = other DNA
tactcctgcccggccaatccagcactgg

SEQ ID NO: 39437 - DNA, 28 bp, synthetic construct
  source 1..28: mol_type = other DNA
attctagatctggcatactcctgcccgg

SEQ ID NO: 39438 - DNA, 28 bp, synthetic construct
  source 1..28: mol_type = other DNA
agggcaggagcatctattctagatctgg

SEQ ID NO: 39439 - DNA, 28 bp, synthetic construct
  source 1..28: mol_type = other DNA
tgaaggctgagcaaagagtaagggcagg

SEQ ID NO: 39440 - DNA, 28 bp, synthetic construct
  source 1..28: mol_type = other DNA
caggtgaaggctgagcaaagagtaaggg

SEQ ID NO: 39441 - DNA, 28 bp, synthetic construct
  source 1..28: mol_type = other DNA
gcaggtgaaggctgagcaaagagtaagg

SEQ ID NO: 39442 - DNA, 28 bp, synthetic construct
  source 1..28: mol_type = other DNA
agaggctacttggatctgcaggtgaagg

SEQ ID NO: 39443 - DNA, 28 bp, synthetic construct
  source 1..28: mol_type = other DNA
gaagggagaggctacttggatctgcagg

SEQ ID NO: 39444 - DNA, 28 bp, synthetic construct
  source 1..28: mol_type = other DNA
gggctaggggaagggagaggctacttgg

SEQ ID NO: 39445 - DNA, 28 bp, synthetic construct
  source 1..28: mol_type = other DNA
actgaggtgggctaggggaagggagagg

SEQ ID NO: 39446 - DNA, 28 bp, synthetic construct
  source 1..28: mol_type = other DNA
aaaggactgaggtgggctaggggaaggg

SEQ ID NO: 39447 - DNA, 28 bp, synthetic construct
  source 1..28: mol_type = other DNA
caaaggactgaggtgggctaggggaagg

SEQ ID NO: 39448 - DNA, 28 bp, synthetic construct
  source 1..28: mol_type = other DNA
cttcccctagcccacctcagtcctttgg

SEQ ID NO: 39449 - DNA, 28 bp, synthetic construct
  source 1..28: mol_type = other DNA
ggaccaaaggactgaggtgggctagggg

SEQ ID NO: 39450 - DNA, 28 bp, synthetic construct
  source 1..28: mol_type = other DNA
gggaccaaaggactgaggtgggctaggg

SEQ ID NO: 39451 - DNA, 28 bp, synthetic construct
  source 1..28: mol_type = other DNA
tgggaccaaaggactgaggtgggctagg

SEQ ID NO: 39452 - DNA, 28 bp, synthetic construct
  source 1..28: mol_type = other DNA
tagcccacctcagtcctttggtcccagg

SEQ ID NO: 39453 - DNA, 28 bp, synthetic construct
  source 1..28: mol_type = other DNA
gctcctgggaccaaaggactgaggtggg

SEQ ID NO: 39454 - DNA, 28 bp, synthetic construct
  source 1..28: mol_type = other DNA
tgctcctgggaccaaaggactgaggtgg

SEQ ID NO: 39455 - DNA, 28 bp, synthetic construct
  source 1..28: mol_type = other DNA
gtttgctcctgggaccaaaggactgagg

SEQ ID NO: 39456 - DNA, 28 bp, synthetic construct
  source 1..28: mol_type = other DNA
cagtcctttggtcccaggagcaaactgg

SEQ ID NO: 39457 - DNA, 28 bp, synthetic construct
  source 1..28: mol_type = other DNA
tcaaccagtttgctcctgggaccaaagg

SEQ ID NO: 39458 - DNA, 28 bp, synthetic construct
  source 1..28: mol_type = other DNA
tcccaggagcaaactggttgactagtgg

SEQ ID NO: 39459 - DNA, 28 bp, synthetic construct
  source 1..28: mol_type = other DNA
gccactagtcaaccagtttgctcctggg

SEQ ID NO: 39460 - DNA, 28 bp, synthetic construct
  source 1..28: mol_type = other DNA
agccactagtcaaccagtttgctcctgg

SEQ ID NO: 39461 - DNA, 28 bp, synthetic construct
  source 1..28: mol_type = other DNA
aaactggttgactagtggctgttgctgg

SEQ ID NO: 39462 - DNA, 28 bp, synthetic construct
  source 1..28: mol_type = other DNA
aactggttgactagtggctgttgctggg

SEQ ID NO: 39463 - DNA, 28 bp, synthetic construct
  source 1..28: mol_type = other DNA
actggttgactagtggctgttgctgggg

SEQ ID NO: 39464 - DNA, 28 bp, synthetic construct
  source 1..28: mol_type = other DNA
ctggttgactagtggctgttgctggggg

SEQ ID NO: 39465 - DNA, 28 bp, synthetic construct
  source 1..28: mol_type = other DNA
ctagtggctgttgctgggggtgctgagg

SEQ ID NO: 39466 - DNA, 28 bp, synthetic construct
  source 1..28: mol_type = other DNA
ggctgttgctgggggtgctgaggccagg

SEQ ID NO: 39467 - DNA, 28 bp, synthetic construct
  source 1..28: mol_type = other DNA
gctgttgctgggggtgctgaggccaggg

SEQ ID NO: 39468 - DNA, 28 bp, synthetic construct
  source 1..28: mol_type = other DNA
tgacagggaagatgtctgtgagccctgg

SEQ ID NO: 39469 - DNA, 28 bp, synthetic construct
  source 1..28: mol_type = other DNA
cagacatcttccctgtcatcttgcctgg

SEQ ID NO: 39470 - DNA, 28 bp, synthetic construct
  source 1..28: mol_type = other DNA
ggagcttactccaggcaagatgacaggg

SEQ ID NO: 39471 - DNA, 28 bp, synthetic construct
  source 1..28: mol_type = other DNA
tggagcttactccaggcaagatgacagg

SEQ ID NO: 39472 - DNA, 28 bp, synthetic construct
  source 1..28: mol_type = other DNA
tgtcatcttgcctggagtaagctccagg

SEQ ID NO: 39473 - DNA, 28 bp, synthetic construct
  source 1..28: mol_type = other DNA
ttgcctggagtaagctccaggagttagg

SEQ ID NO: 39474 - DNA, 28 bp, synthetic construct
  source 1..28: mol_type = other DNA
tgcctggagtaagctccaggagttaggg

SEQ ID NO: 39475 - DNA, 28 bp, synthetic construct
  source 1..28: mol_type = other DNA
cgccctaactcctggagcttactccagg

SEQ ID NO: 39476 - DNA, 28 bp, synthetic construct
  source 1..28: mol_type = other DNA
agtaagctccaggagttagggcgcctgg

SEQ ID NO: 39477 - DNA, 28 bp, synthetic construct
  source 1..28: mol_type = other DNA
gtaagctccaggagttagggcgcctggg

SEQ ID NO: 39478 - DNA, 28 bp, synthetic construct
  source 1..28: mol_type = other DNA
ccagggacccaggcgccctaactcctgg

SEQ ID NO: 39479 - DNA, 28 bp, synthetic construct
  source 1..28: mol_type = other DNA
ggggacaactggcagccagggacccagg

SEQ ID NO: 39480 - DNA, 28 bp, synthetic construct
  source 1..28: mol_type = other DNA
aaaggtgggggacaactggcagccaggg

SEQ ID NO: 39481 - DNA, 28 bp, synthetic construct
  source 1..28: mol_type = other DNA
taaaggtgggggacaactggcagccagg

SEQ ID NO: 39482 - DNA, 28 bp, synthetic construct
  source 1..28: mol_type = other DNA
tggctgccagttgtcccccacctttagg

SEQ ID NO: 39483 - DNA, 28 bp, synthetic construct
  source 1..28: mol_type = other DNA
gccagttgtcccccacctttaggcctgg

SEQ ID NO: 39484 - DNA, 28 bp, synthetic construct
  source 1..28: mol_type = other DNA
tccaggcctaaaggtgggggacaactgg

SEQ ID NO: 39485 - DNA, 28 bp, synthetic construct
  source 1..28: mol_type = other DNA
tgtcccccacctttaggcctggatttgg

SEQ ID NO: 39486 - DNA, 28 bp, synthetic construct
  source 1..28: mol_type = other DNA
cttccaaatccaggcctaaaggtggggg

SEQ ID NO: 39487 - DNA, 28 bp, synthetic construct
  source 1..28: mol_type = other DNA
ccccacctttaggcctggatttggaagg

SEQ ID NO: 39488 - DNA, 28 bp, synthetic construct
  source 1..28: mol_type = other DNA
cccacctttaggcctggatttggaaggg

SEQ ID NO: 39489 - DNA, 28 bp, synthetic construct
  source 1..28: mol_type = other DNA
ccccttccaaatccaggcctaaaggtgg

SEQ ID NO: 39490 - DNA, 28 bp, synthetic construct
  source 1..28: mol_type = other DNA
tctccccttccaaatccaggcctaaagg

SEQ ID NO: 39491 - DNA, 28 bp, synthetic construct
  source 1..28: mol_type = other DNA
tttaggcctggatttggaaggggagagg

SEQ ID NO: 39492 - DNA, 28 bp, synthetic construct
  source 1..28: mol_type = other DNA
ggcctggatttggaaggggagaggctgg

SEQ ID NO: 39493 - DNA, 28 bp, synthetic construct
  source 1..28: mol_type = other DNA
ctccagcctctccccttccaaatccagg

SEQ ID NO: 39494 - DNA, 28 bp, synthetic construct
  source 1..28: mol_type = other DNA
ggatttggaaggggagaggctggagagg

SEQ ID NO: 39495 - DNA, 28 bp, synthetic construct
  source 1..28: mol_type = other DNA
tttggaaggggagaggctggagaggagg

SEQ ID NO: 39496 - DNA, 28 bp, synthetic construct
  source 1..28: mol_type = other DNA
ttggaaggggagaggctggagaggaggg

SEQ ID NO: 39497 - DNA, 28 bp, synthetic construct
  source 1..28: mol_type = other DNA
aaggggagaggctggagaggagggcagg

SEQ ID NO: 39498 - DNA, 28 bp, synthetic construct
  source 1..28: mol_type = other DNA
gggagaggctggagaggagggcaggagg

SEQ ID NO: 39499 - DNA, 28 bp, synthetic construct
  source 1..28: mol_type = other DNA
ctggagaggagggcaggaggaactgtgg

SEQ ID NO: 39500 - DNA, 28 bp, synthetic construct
  source 1..28: mol_type = other DNA
agaggagggcaggaggaactgtggctgg

SEQ ID NO: 39501 - DNA, 28 bp, synthetic construct
  source 1..28: mol_type = other DNA
gaggagggcaggaggaactgtggctggg

SEQ ID NO: 39502 - DNA, 28 bp, synthetic construct
  source 1..28: mol_type = other DNA
gggcaggaggaactgtggctgggagtgg

SEQ ID NO: 39503 - DNA, 28 bp, synthetic construct
  source 1..28: mol_type = other DNA
ggcaggaggaactgtggctgggagtggg

SEQ ID NO: 39504 - DNA, 28 bp, synthetic construct
  source 1..28: mol_type = other DNA
aggaggaactgtggctgggagtgggagg

SEQ ID NO: 39505 - DNA, 28 bp, synthetic construct
  source 1..28: mol_type = other DNA
ctgtggctgggagtgggaggagccttgg

SEQ ID NO: 39506 - DNA, 28 bp, synthetic construct
  source 1..28: mol_type = other DNA
tgtggctgggagtgggaggagccttggg

SEQ ID NO: 39507 - DNA, 28 bp, synthetic construct
  source 1..28: mol_type = other DNA
gctgggagtgggaggagccttgggctgg

SEQ ID NO: 39508 - DNA, 28 bp, synthetic construct
  source 1..28: mol_type = other DNA
ctgggagtgggaggagccttgggctggg

SEQ ID NO: 39509 - DNA, 28 bp, synthetic construct
  source 1..28: mol_type = other DNA
ggctttctctctcacacccagcccaagg

SEQ ID NO: 39510 - DNA, 28 bp, synthetic construct
  source 1..28: mol_type = other DNA
gggctgggtgtgagagagaaagcccagg

SEQ ID NO: 39511 - DNA, 28 bp, synthetic construct
  source 1..28: mol_type = other DNA
ggtgtgagagagaaagcccaggcagagg

SEQ ID NO: 39512 - DNA, 28 bp, synthetic construct
  source 1..28: mol_type = other DNA
gtgtgagagagaaagcccaggcagaggg

SEQ ID NO: 39513 - DNA, 28 bp, synthetic construct
  source 1..28: mol_type = other DNA
tagggcagacacacaccctctgcctggg

SEQ ID NO: 39514 - DNA, 28 bp, synthetic construct
  source 1..28: mol_type = other DNA
ctagggcagacacacaccctctgcctgg

SEQ ID NO: 39515 - DNA, 28 bp, synthetic construct
  source 1..28: mol_type = other DNA
ggtgtgtgtctgccctagccagcaccgg

SEQ ID NO: 39516 - DNA, 28 bp, synthetic construct
  source 1..28: mol_type = other DNA
caggcaggcaggccggtgctggctaggg

SEQ ID NO: 39517 - DNA, 28 bp, synthetic construct
  source 1..28: mol_type = other DNA
gcaggcaggcaggccggtgctggctagg

SEQ ID NO: 39518 - DNA, 28 bp, synthetic construct
  source 1..28: mol_type = other DNA
ggcaggcaggcaggcaggccggtgctgg

SEQ ID NO: 39519 - DNA, 28 bp, synthetic construct
  source 1..28: mol_type = other DNA
gcaccggcctgcctgcctgcctgcctgg

SEQ ID NO: 39520 - DNA, 28 bp, synthetic construct
  source 1..28: mol_type = other DNA
ctaccaggcaggcaggcaggcaggccgg

SEQ ID NO: 39521 - DNA, 28 bp, synthetic construct
  source 1..28: mol_type = other DNA
acatctaccaggcaggcaggcaggcagg

SEQ ID NO: 39522 - DNA, 28 bp, synthetic construct
  source 1..28: mol_type = other DNA
tggcacatctaccaggcaggcaggcagg

SEQ ID NO: 39523 - DNA, 28 bp, synthetic construct
  source 1..28: mol_type = other DNA
ttcatggcacatctaccaggcaggcagg

SEQ ID NO: 39524 - DNA, 28 bp, synthetic construct
  source 1..28: mol_type = other DNA
agcattcatggcacatctaccaggcagg

SEQ ID NO: 39525 - DNA, 28 bp, synthetic construct
  source 1..28: mol_type = other DNA
caacagcattcatggcacatctaccagg

SEQ ID NO: 39526 - DNA, 28 bp, synthetic construct
  source 1..28: mol_type = other DNA
gatgtgccatgaatgctgttgactccgg

SEQ ID NO: 39527 - DNA, 28 bp, synthetic construct
  source 1..28: mol_type = other DNA
atgtgccatgaatgctgttgactccggg

SEQ ID NO: 39528 - DNA, 28 bp, synthetic construct
  source 1..28: mol_type = other DNA
acacacccggagtcaacagcattcatgg

SEQ ID NO: 39529 - DNA, 28 bp, synthetic construct
  source 1..28: mol_type = other DNA
acacacacgcacacacacacacacccgg

SEQ ID NO: 39530 - DNA, 28 bp, synthetic construct
  source 1..28: mol_type = other DNA
agacacagacactcactctcggcactgg

SEQ ID NO: 39531 - DNA, 28 bp, synthetic construct
  source 1..28: mol_type = other DNA
gccgagagtgagtgtctgtgtctgatgg

SEQ ID NO: 39532 - DNA, 28 bp, synthetic construct
  source 1..28: mol_type = other DNA
ccgagagtgagtgtctgtgtctgatggg

SEQ ID NO: 39533 - DNA, 28 bp, synthetic construct
  source 1..28: mol_type = other DNA
cgagagtgagtgtctgtgtctgatgggg

SEQ ID NO: 39534 - DNA, 28 bp, synthetic construct
  source 1..28: mol_type = other DNA
gagagtgagtgtctgtgtctgatggggg

SEQ ID NO: 39535 - DNA, 28 bp, synthetic construct
  source 1..28: mol_type = other DNA
tcaaccctagagtgagagaacccagtgg

SEQ ID NO: 39536 - DNA, 28 bp, synthetic construct
  source 1..28: mol_type = other DNA
gaaaccactgggttctctcactctaggg

SEQ ID NO: 39537 - DNA, 28 bp, synthetic construct
  source 1..28: mol_type = other DNA
tgaaaccactgggttctctcactctagg

SEQ ID NO: 39538 - DNA, 28 bp, synthetic construct
  source 1..28: mol_type = other DNA
cagtagaatgcagagtgaaaccactggg

SEQ ID NO: 39539 - DNA, 28 bp, synthetic construct
  source 1..28: mol_type = other DNA
tcagtagaatgcagagtgaaaccactgg

SEQ ID NO: 39540 - DNA, 28 bp, synthetic construct
  source 1..28: mol_type = other DNA
agtggtttcactctgcattctactgagg

SEQ ID NO: 39541 - DNA, 28 bp, synthetic construct
  source 1..28: mol_type = other DNA
tcactctgcattctactgaggacagagg

SEQ ID NO: 39542 - DNA, 28 bp, synthetic construct
  source 1..28: mol_type = other DNA
cactctgcattctactgaggacagaggg

SEQ ID NO: 39543 - DNA, 28 bp, synthetic construct
  source 1..28: mol_type = other DNA
ctgaggacagagggagagaaaagaatgg

SEQ ID NO: 39544 - DNA, 28 bp, synthetic construct
  source 1..28: mol_type = other DNA
tgaggacagagggagagaaaagaatggg

SEQ ID NO: 39545 - DNA, 28 bp, synthetic construct
  source 1..28: mol_type = other DNA
gggtctgcagtccaagctctgtgcacgg

SEQ ID NO: 39546 - DNA, 28 bp, synthetic construct
  source 1..28: mol_type = other DNA
gtgtttgggatccgtgcacagagcttgg

SEQ ID NO: 39547 - DNA, 28 bp, synthetic construct
  source 1..28: mol_type = other DNA
tgtgcacggatcccaaacactcccatgg

SEQ ID NO: 39548 - DNA, 28 bp, synthetic construct
  source 1..28: mol_type = other DNA
gtgcacggatcccaaacactcccatggg

SEQ ID NO: 39549 - DNA, 28 bp, synthetic construct
  source 1..28: mol_type = other DNA
tgcacggatcccaaacactcccatgggg

SEQ ID NO: 39550 - DNA, 28 bp, synthetic construct
  source 1..28: mol_type = other DNA
ggatcccaaacactcccatggggactgg

SEQ ID NO: 39551 - DNA, 28 bp, synthetic construct
  source 1..28: mol_type = other DNA
aactccagtccccatgggagtgtttggg

SEQ ID NO: 39552 - DNA, 28 bp, synthetic construct
  source 1..28: mol_type = other DNA
caactccagtccccatgggagtgtttgg

SEQ ID NO: 39553 - DNA, 28 bp, synthetic construct
  source 1..28: mol_type = other DNA
caaacactcccatggggactggagttgg

SEQ ID NO: 39554 - DNA, 28 bp, synthetic construct
  source 1..28: mol_type = other DNA
aaacactcccatggggactggagttggg

SEQ ID NO: 39555 - DNA, 28 bp, synthetic construct
  source 1..28: mol_type = other DNA
cactcccatggggactggagttgggagg

SEQ ID NO: 39556 - DNA, 28 bp, synthetic construct
  source 1..28: mol_type = other DNA
actcccatggggactggagttgggaggg

SEQ ID NO: 39557 - DNA, 28 bp, synthetic construct
  source 1..28: mol_type = other DNA
tctccctcccaactccagtccccatggg

SEQ ID NO: 39558 - DNA, 28 bp, synthetic construct
  source 1..28: mol_type = other DNA
ttctccctcccaactccagtccccatgg

SEQ ID NO: 39559 - DNA, 28 bp, synthetic construct
  source 1..28: mol_type = other DNA
gggactggagttgggagggagaaagagg

SEQ ID NO: 39560 - DNA, 28 bp, synthetic construct
  source 1..28: mol_type = other DNA
ggagttgggagggagaaagaggagaagg

SEQ ID NO: 39561 - DNA, 28 bp, synthetic construct
  source 1..28: mol_type = other DNA
gagttgggagggagaaagaggagaaggg

SEQ ID NO: 39562 - DNA, 28 bp, synthetic construct
  source 1..28: mol_type = other DNA
agttgggagggagaaagaggagaagggg

SEQ ID NO: 39563 - DNA, 28 bp, synthetic construct
  source 1..28: mol_type = other DNA
agaggagaaggggagagtctgagctagg

SEQ ID NO: 39564 - DNA, 28 bp, synthetic construct
  source 1..28: mol_type = other DNA
aggggagagtctgagctaggctgatagg

SEQ ID NO: 39565 - DNA, 28 bp, synthetic construct
  source 1..28: mol_type = other DNA
gagagtctgagctaggctgataggctgg

SEQ ID NO: 39566 - DNA, 28 bp, synthetic construct
  source 1..28: mol_type = other DNA
cgagcattgctggggaaggtactttggg

SEQ ID NO: 39567 - DNA, 28 bp, synthetic construct
  source 1..28: mol_type = other DNA
gcgagcattgctggggaaggtactttgg

SEQ ID NO: 39568 - DNA, 28 bp, synthetic construct
  source 1..28: mol_type = other DNA
aagtaccttccccagcaatgctcgcagg

SEQ ID NO: 39569 - DNA, 28 bp, synthetic construct
  source 1..28: mol_type = other DNA
agtaccttccccagcaatgctcgcaggg

SEQ ID NO: 39570 - DNA, 28 bp, synthetic construct
  source 1..28: mol_type = other DNA
gtcaccctgcgagcattgctggggaagg

SEQ ID NO: 39571 - DNA, 28 bp, synthetic construct
  source 1..28: mol_type = other DNA
ccccagcaatgctcgcagggtgaccagg

SEQ ID NO: 39572 - DNA, 28 bp, synthetic construct
  source 1..28: mol_type = other DNA
tcctggtcaccctgcgagcattgctggg

SEQ ID NO: 39573 - DNA, 28 bp, synthetic construct
  source 1..28: mol_type = other DNA
gtcctggtcaccctgcgagcattgctgg

SEQ ID NO: 39574 - DNA, 28 bp, synthetic construct
  source 1..28: mol_type = other DNA
caatgctcgcagggtgaccaggacctgg

SEQ ID NO: 39575 - DNA, 28 bp, synthetic construct
  source 1..28: mol_type = other DNA
aatgctcgcagggtgaccaggacctggg

SEQ ID NO: 39576 - DNA, 28 bp, synthetic construct
  source 1..28: mol_type = other DNA
gaccaggacctgggacacagactcctgg

SEQ ID NO: 39577 - DNA, 28 bp, synthetic construct
  source 1..28: mol_type = other DNA
accaggacctgggacacagactcctggg

SEQ ID NO: 39578 - DNA, 28 bp, synthetic construct
  source 1..28: mol_type = other DNA
acccaggagtctgtgtcccaggtcctgg

SEQ ID NO: 39579 - DNA, 28 bp, synthetic construct
  source 1..28: mol_type = other DNA
gacgtgacccaggagtctgtgtcccagg

SEQ ID NO: 39580 - DNA, 28 bp, synthetic construct
  source 1..28: mol_type = other DNA
cagtatggaaaatgtgacgtgacccagg

SEQ ID NO: 39581 - DNA, 28 bp, synthetic construct
  source 1..28: mol_type = other DNA
ctgggtcacgtcacattttccatactgg

SEQ ID NO: 39582 - DNA, 28 bp, synthetic construct
  source 1..28: mol_type = other DNA
tcacattttccatactggaattacttgg

SEQ ID NO: 39583 - DNA, 28 bp, synthetic construct
  source 1..28: mol_type = other DNA
aggacaaagccaagtaattccagtatgg

SEQ ID NO: 39584 - DNA, 28 bp, synthetic construct
  source 1..28: mol_type = other DNA
acttggctttgtccttgctcccccctgg

SEQ ID NO: 39585 - DNA, 28 bp, synthetic construct
  source 1..28: mol_type = other DNA
cttggctttgtccttgctcccccctggg

SEQ ID NO: 39586 - DNA, 28 bp, synthetic construct
  source 1..28: mol_type = other DNA
ttggctttgtccttgctcccccctgggg

SEQ ID NO: 39587 - DNA, 28 bp, synthetic construct
  source 1..28: mol_type = other DNA
tggctttgtccttgctcccccctggggg

SEQ ID NO: 39588 - DNA, 28 bp, synthetic construct
  source 1..28: mol_type = other DNA
ttgtccttgctcccccctgggggccagg

SEQ ID NO: 39589 - DNA, 28 bp, synthetic construct
  source 1..28: mol_type = other DNA
gacacctggcccccaggggggagcaagg

SEQ ID NO: 39590 - DNA, 28 bp, synthetic construct
  source 1..28: mol_type = other DNA
gagggaggacacctggcccccagggggg

SEQ ID NO: 39591 - DNA, 28 bp, synthetic construct
  source 1..28: mol_type = other DNA
ggagggaggacacctggcccccaggggg

SEQ ID NO: 39592 - DNA, 28 bp, synthetic construct
  source 1..28: mol_type = other DNA
aggagggaggacacctggcccccagggg

SEQ ID NO: 39593 - DNA, 28 bp, synthetic construct
  source 1..28: mol_type = other DNA
caggagggaggacacctggcccccaggg

SEQ ID NO: 39594 - DNA, 28 bp, synthetic construct
  source 1..28: mol_type = other DNA
ccaggagggaggacacctggcccccagg

SEQ ID NO: 39595 - DNA, 28 bp, synthetic construct
  source 1..28: mol_type = other DNA
ctgggggccaggtgtcctccctcctggg

SEQ ID NO: 39596 - DNA, 28 bp, synthetic construct
  source 1..28: mol_type = other DNA
ggccaggtgtcctccctcctgggaaagg

SEQ ID NO: 39597 - DNA, 28 bp, synthetic construct
  source 1..28: mol_type = other DNA
agcctttcccaggagggaggacacctgg

SEQ ID NO: 39598 - DNA, 28 bp, synthetic construct
  source 1..28: mol_type = other DNA
ccaaaagcagcctttcccaggagggagg

SEQ ID NO: 39599 - DNA, 28 bp, synthetic construct
  source 1..28: mol_type = other DNA
ctaccaaaagcagcctttcccaggaggg

SEQ ID NO: 39600 - DNA, 28 bp, synthetic construct
  source 1..28: mol_type = other DNA
gctaccaaaagcagcctttcccaggagg

SEQ ID NO: 39601 - DNA, 28 bp, synthetic construct
  source 1..28: mol_type = other DNA
ttggctaccaaaagcagcctttcccagg

SEQ ID NO: 39602 - DNA, 28 bp, synthetic construct
  source 1..28: mol_type = other DNA
aaggctgcttttggtagccaaagtcagg

SEQ ID NO: 39603 - DNA, 28 bp, synthetic construct
  source 1..28: mol_type = other DNA
gcttttggtagccaaagtcaggtgaagg

SEQ ID NO: 39604 - DNA, 28 bp, synthetic construct
  source 1..28: mol_type = other DNA
ggtagccaaagtcaggtgaaggagatgg

SEQ ID NO: 39605 - DNA, 28 bp, synthetic construct
  source 1..28: mol_type = other DNA
gtagccaaagtcaggtgaaggagatggg

SEQ ID NO: 39606 - DNA, 28 bp, synthetic construct
  source 1..28: mol_type = other DNA
tagccaaagtcaggtgaaggagatgggg

SEQ ID NO: 39607 - DNA, 28 bp, synthetic construct
  source 1..28: mol_type = other DNA
agccaaagtcaggtgaaggagatggggg

SEQ ID NO: 39608 - DNA, 28 bp, synthetic construct
  source 1..28: mol_type = other DNA
ttcccccatctccttcacctgactttgg

SEQ ID NO: 39609 - DNA, 28 bp, synthetic construct
  source 1..28: mol_type = other DNA
aggtgaaggagatgggggaaagaagagg

SEQ ID NO: 39610 - DNA, 28 bp, synthetic construct
  source 1..28: mol_type = other DNA
gatgggggaaagaagaggcatgctgtgg

SEQ ID NO: 39611 - DNA, 28 bp, synthetic construct
  source 1..28: mol_type = other DNA
agaagaggcatgctgtggttacctcagg

SEQ ID NO: 39612 - DNA, 28 bp, synthetic construct
  source 1..28: mol_type = other DNA
gaagaggcatgctgtggttacctcaggg

SEQ ID NO: 39613 - DNA, 28 bp, synthetic construct
  source 1..28: mol_type = other DNA
ggcatgctgtggttacctcagggaatgg

SEQ ID NO: 39614 - DNA, 28 bp, synthetic construct
  source 1..28: mol_type = other DNA
gcatgctgtggttacctcagggaatggg

SEQ ID NO: 39615 - DNA, 28 bp, synthetic construct
  source 1..28: mol_type = other DNA
tgtggttacctcagggaatgggagatgg

SEQ ID NO: 39616 - DNA, 28 bp, synthetic construct
  source 1..28: mol_type = other DNA
tacctcagggaatgggagatggcaatgg

SEQ ID NO: 39617 - DNA, 28 bp, synthetic construct
  source 1..28: mol_type = other DNA
acctcagggaatgggagatggcaatggg

SEQ ID NO: 39618 - DNA, 28 bp, synthetic construct
  source 1..28: mol_type = other DNA
ccccattgccatctcccattccctgagg

SEQ ID NO: 39619 - DNA, 28 bp, synthetic construct
  source 1..28: mol_type = other DNA
ctcagggaatgggagatggcaatggggg

SEQ ID NO: 39620 - DNA, 28 bp, synthetic construct
  source 1..28: mol_type = other DNA
gcagacaagccctctctttcactccagg

SEQ ID NO: 39621 - DNA, 28 bp, synthetic construct
  source 1..28: mol_type = other DNA
cagacaagccctctctttcactccaggg

SEQ ID NO: 39622 - DNA, 28 bp, synthetic construct
  source 1..28: mol_type = other DNA
aagccctctctttcactccagggatagg

SEQ ID NO: 39623 - DNA, 28 bp, synthetic construct
  source 1..28: mol_type = other DNA
cttcctatccctggagtgaaagagaggg

SEQ ID NO: 39624 - DNA, 28 bp, synthetic construct
  source 1..28: mol_type = other DNA
tcttcctatccctggagtgaaagagagg

SEQ ID NO: 39625 - DNA, 28 bp, synthetic construct
  source 1..28: mol_type = other DNA
tttcactccagggataggaagagctagg

SEQ ID NO: 39626 - DNA, 28 bp, synthetic construct
  source 1..28: mol_type = other DNA
atctattcctagctcttcctatccctgg

SEQ ID NO: 39627 - DNA, 28 bp, synthetic construct
  source 1..28: mol_type = other DNA
gctaggccacctggggacgggaccctgg

SEQ ID NO: 39628 - DNA, 28 bp, synthetic construct
  source 1..28: mol_type = other DNA
ggtagccttactggtgggaaccaaaagg

SEQ ID NO: 39629 - DNA, 28 bp, synthetic construct
  source 1..28: mol_type = other DNA
tgttggagatctcgtcagggccttttgg

SEQ ID NO: 39630 - DNA, 28 bp, synthetic construct
  source 1..28: mol_type = other DNA
aaaaggccctgacgagatctccaacagg

SEQ ID NO: 39631 - DNA, 28 bp, synthetic construct
  source 1..28: mol_type = other DNA
gtatagcctgttggagatctcgtcaggg

SEQ ID NO: 39632 - DNA, 28 bp, synthetic construct
  source 1..28: mol_type = other DNA
tgtatagcctgttggagatctcgtcagg

SEQ ID NO: 39633 - DNA, 28 bp, synthetic construct
  source 1..28: mol_type = other DNA
acgagatctccaacaggctatacaatgg

SEQ ID NO: 39634 - DNA, 28 bp, synthetic construct
  source 1..28: mol_type = other DNA
cgagatctccaacaggctatacaatggg

SEQ ID NO: 39635 - DNA, 28 bp, synthetic construct
  source 1..28: mol_type = other DNA
gacagaggcccattgtatagcctgttgg

SEQ ID NO: 39636 - DNA, 28 bp, synthetic construct
  source 1..28: mol_type = other DNA
agcttagcaagctagagggtgacagagg

SEQ ID NO: 39637 - DNA, 28 bp, synthetic construct
  source 1..28: mol_type = other DNA
gctgttgggagcttagcaagctagaggg

SEQ ID NO: 39638 - DNA, 28 bp, synthetic construct
  source 1..28: mol_type = other DNA
tgctgttgggagcttagcaagctagagg

SEQ ID NO: 39639 - DNA, 28 bp, synthetic construct
  source 1..28: mol_type = other DNA
tcccaacagcactagcacagtgccttgg

SEQ ID NO: 39640 - DNA, 28 bp, synthetic construct
  source 1..28: mol_type = other DNA
accaaggcactgtgctagtgctgttggg

SEQ ID NO: 39641 - DNA, 28 bp, synthetic construct
  source 1..28: mol_type = other DNA
taccaaggcactgtgctagtgctgttgg

SEQ ID NO: 39642 - DNA, 28 bp, synthetic construct
  source 1..28: mol_type = other DNA
tgggtagaggaaatcgcaggtaccaagg

SEQ ID NO: 39643 - DNA, 28 bp, synthetic construct
  source 1..28: mol_type = other DNA
gtacctgcgatttcctctacccagaagg

SEQ ID NO: 39644 - DNA, 28 bp, synthetic construct
  source 1..28: mol_type = other DNA
gaaccttctgggtagaggaaatcgcagg

SEQ ID NO: 39645 - DNA, 28 bp, synthetic construct
  source 1..28: mol_type = other DNA
aaaaaagaaggaaccttctgggtagagg

SEQ ID NO: 39646 - DNA, 28 bp, synthetic construct
  source 1..28: mol_type = other DNA
aaaaacaaaaaagaaggaaccttctggg

SEQ ID NO: 39647 - DNA, 28 bp, synthetic construct
  source 1..28: mol_type = other DNA
caaaaacaaaaaagaaggaaccttctgg

SEQ ID NO: 39648 - DNA, 28 bp, synthetic construct
  source 1..28: mol_type = other DNA
aactgtgtctcaaaaacaaaaaagaagg

SEQ ID NO: 39649 - DNA, 28 bp, synthetic construct
  source 1..28: mol_type = other DNA
agacacagtttcgctcttgttgcccagg

SEQ ID NO: 39650 - DNA, 28 bp, synthetic construct
  source 1..28: mol_type = other DNA
acagtttcgctcttgttgcccaggctgg

SEQ ID NO: 39651 - DNA, 28 bp, synthetic construct
  source 1..28: mol_type = other DNA
tcttgttgcccaggctggagtgcaatgg

SEQ ID NO: 39652 - DNA, 28 bp, synthetic construct
  source 1..28: mol_type = other DNA
agatcgcgccattgcactccagcctggg

SEQ ID NO: 39653 - DNA, 28 bp, synthetic construct
  source 1..28: mol_type = other DNA
aagatcgcgccattgcactccagcctgg

SEQ ID NO: 39654 - DNA, 28 bp, synthetic construct
  source 1..28: mol_type = other DNA
aggctggagtgcaatggcgcgatcttgg

SEQ ID NO: 39655 - DNA, 28 bp, synthetic construct
  source 1..28: mol_type = other DNA
gcttgaacgcaggaggtggagattgcgg

SEQ ID NO: 39656 - DNA, 28 bp, synthetic construct
  source 1..28: mol_type = other DNA
aggagaatcgcttgaacgcaggaggtgg

SEQ ID NO: 39657 - DNA, 28 bp, synthetic construct
  source 1..28: mol_type = other DNA
ggcaggagaatcgcttgaacgcaggagg

SEQ ID NO: 39658 - DNA, 28 bp, synthetic construct
  source 1..28: mol_type = other DNA
tgaggcaggagaatcgcttgaacgcagg

SEQ ID NO: 39659 - DNA, 28 bp, synthetic construct
  source 1..28: mol_type = other DNA
ctcctgcctcagcctcccaagtagctgg

SEQ ID NO: 39660 - DNA, 28 bp, synthetic construct
  source 1..28: mol_type = other DNA
tcctgcctcagcctcccaagtagctggg

SEQ ID NO: 39661 - DNA, 28 bp, synthetic construct
  source 1..28: mol_type = other DNA
tcccagctacttgggaggctgaggcagg

SEQ ID NO: 39662 - DNA, 28 bp, synthetic construct
  source 1..28: mol_type = other DNA
gtaatcccagctacttgggaggctgagg

SEQ ID NO: 39663 - DNA, 28 bp, synthetic construct
  source 1..28: mol_type = other DNA
cagcctcccaagtagctgggattacagg

SEQ ID NO: 39664 - DNA, 28 bp, synthetic construct
  source 1..28: mol_type = other DNA
atgcctgtaatcccagctacttgggagg

SEQ ID NO: 39665 - DNA, 28 bp, synthetic construct
  source 1..28: mol_type = other DNA
cgcatgcctgtaatcccagctacttggg

SEQ ID NO: 39666 - DNA, 28 bp, synthetic construct
  source 1..28: mol_type = other DNA
gcgcatgcctgtaatcccagctacttgg

SEQ ID NO: 39667 - DNA, 28 bp, synthetic construct
  source 1..28: mol_type = other DNA
aaaatacaaaattatctgggcatggtgg

SEQ ID NO: 39668 - DNA, 28 bp, synthetic construct
  source 1..28: mol_type = other DNA
ctaaaaatacaaaattatctgggcatgg

SEQ ID NO: 39669 - DNA, 28 bp, synthetic construct
  source 1..28: mol_type = other DNA
ctctactaaaaatacaaaattatctggg

SEQ ID NO: 39670 - DNA, 28 bp, synthetic construct
  source 1..28: mol_type = other DNA
tctctactaaaaatacaaaattatctgg

SEQ ID NO: 39671 - DNA, 28 bp, synthetic construct
  source 1..28: mol_type = other DNA
ataattttgtatttttagtagagacagg

SEQ ID NO: 39672 - DNA, 28 bp, synthetic construct
  source 1..28: mol_type = other DNA
taattttgtatttttagtagagacaggg

SEQ ID NO: 39673 - DNA, 28 bp, synthetic construct
  source 1..28: mol_type = other DNA
tagtagagacagggcttcaccatgttgg

SEQ ID NO: 39674 - DNA, 28 bp, synthetic construct
  source 1..28: mol_type = other DNA
acagggcttcaccatgttggtcagacgg

SEQ ID NO: 39675 - DNA, 28 bp, synthetic construct
  source 1..28: mol_type = other DNA
tcacttgagagccgtctgaccaacatgg

SEQ ID NO: 39676 - DNA, 28 bp, synthetic construct
  source 1..28: mol_type = other DNA
ggtgggtgcatcacttgaggtcaagtgg

SEQ ID NO: 39677 - DNA, 28 bp, synthetic construct
  source 1..28: mol_type = other DNA
gaggcagaggtgggtgcatcacttgagg

SEQ ID NO: 39678 - DNA, 28 bp, synthetic construct
  source 1..28: mol_type = other DNA
cacccacctctgcctcccaaagtgctgg

SEQ ID NO: 39679 - DNA, 28 bp, synthetic construct
  source 1..28: mol_type = other DNA
acccacctctgcctcccaaagtgctggg

SEQ ID NO: 39680 - DNA, 28 bp, synthetic construct
  source 1..28: mol_type = other DNA
tcccagcactttgggaggcagaggtggg

SEQ ID NO: 39681 - DNA, 28 bp, synthetic construct
  source 1..28: mol_type = other DNA
atcccagcactttgggaggcagaggtgg

SEQ ID NO: 39682 - DNA, 28 bp, synthetic construct
  source 1..28: mol_type = other DNA
gtaatcccagcactttgggaggcagagg

SEQ ID NO: 39683 - DNA, 28 bp, synthetic construct
  source 1..28: mol_type = other DNA
acgcttgtaatcccagcactttgggagg

SEQ ID NO: 39684 - DNA, 28 bp, synthetic construct
  source 1..28: mol_type = other DNA
ctcacgcttgtaatcccagcactttggg

SEQ ID NO: 39685 - DNA, 28 bp, synthetic construct
  source 1..28: mol_type = other DNA
gctcacgcttgtaatcccagcactttgg

SEQ ID NO: 39686 - DNA, 28 bp, synthetic construct
  source 1..28: mol_type = other DNA
gattacaagcgtgagccaccgcgcctgg

SEQ ID NO: 39687 - DNA, 28 bp, synthetic construct
  source 1..28: mol_type = other DNA
tgagccaccgcgcctggcctccagaagg

SEQ ID NO: 39688 - DNA, 28 bp, synthetic construct
  source 1..28: mol_type = other DNA
ggaaccttctggaggccaggcgcggtgg

SEQ ID NO: 39689 - DNA, 28 bp, synthetic construct
  source 1..28: mol_type = other DNA
gaaggaaccttctggaggccaggcgcgg

SEQ ID NO: 39690 - DNA, 28 bp, synthetic construct
  source 1..28: mol_type = other DNA
ctatagaaggaaccttctggaggccagg

SEQ ID NO: 39691 - DNA, 28 bp, synthetic construct
  source 1..28: mol_type = other DNA
ctggcctccagaaggttccttctatagg

SEQ ID NO: 39692 - DNA, 28 bp, synthetic construct
  source 1..28: mol_type = other DNA
gaagcctatagaaggaaccttctggagg

SEQ ID NO: 39693 - DNA, 28 bp, synthetic construct
  source 1..28: mol_type = other DNA
tgtgaagcctatagaaggaaccttctgg

SEQ ID NO: 39694 - DNA, 28 bp, synthetic construct
  source 1..28: mol_type = other DNA
gagcacgctatgtgaagcctatagaagg

SEQ ID NO: 39695 - DNA, 28 bp, synthetic construct
  source 1..28: mol_type = other DNA
acatagcgtgctccttcttgtcatttgg

SEQ ID NO: 39696 - DNA, 28 bp, synthetic construct
  source 1..28: mol_type = other DNA
ttgagctgagatccaaatgacaagaagg

SEQ ID NO: 39697 - DNA, 28 bp, synthetic construct
  source 1..28: mol_type = other DNA
atgttacctgctcagtaaagccttctgg

SEQ ID NO: 39698 - DNA, 28 bp, synthetic construct
  source 1..28: mol_type = other DNA
gacgctccagaaggctttactgagcagg

SEQ ID NO: 39699 - DNA, 28 bp, synthetic construct
  source 1..28: mol_type = other DNA
tggggattaagaaggacgctccagaagg

SEQ ID NO: 39700 - DNA, 28 bp, synthetic construct
  source 1..28: mol_type = other DNA
caggataggagactggggattaagaagg

SEQ ID NO: 39701 - DNA, 28 bp, synthetic construct
  source 1..28: mol_type = other DNA
ggaagtgaaacaggataggagactgggg

SEQ ID NO: 39702 - DNA, 28 bp, synthetic construct
  source 1..28: mol_type = other DNA
gggaagtgaaacaggataggagactggg

SEQ ID NO: 39703 - DNA, 28 bp, synthetic construct
  source 1..28: mol_type = other DNA
cgggaagtgaaacaggataggagactgg

SEQ ID NO: 39704 - DNA, 28 bp, synthetic construct
  source 1..28: mol_type = other DNA
ctcctatcctgtttcacttcccgcatgg

SEQ ID NO: 39705 - DNA, 28 bp, synthetic construct
  source 1..28: mol_type = other DNA
tgccatgcgggaagtgaaacaggatagg

SEQ ID NO: 39706 - DNA, 28 bp, synthetic construct
  source 1..28: mol_type = other DNA
acatgtgccatgcgggaagtgaaacagg

SEQ ID NO: 39707 - DNA, 28 bp, synthetic construct
  source 1..28: mol_type = other DNA
aattttagagtcacatgtgccatgcggg

SEQ ID NO: 39708 - DNA, 28 bp, synthetic construct
  source 1..28: mol_type = other DNA
taattttagagtcacatgtgccatgcgg

SEQ ID NO: 39709 - DNA, 28 bp, synthetic construct
  source 1..28: mol_type = other DNA
tacacttattttttataagtgtctgcgg

SEQ ID NO: 39710 - DNA, 28 bp, synthetic construct
  source 1..28: mol_type = other DNA
tgctctgtggaagtctgcattctagtgg

SEQ ID NO: 39711 - DNA, 28 bp, synthetic construct
  source 1..28: mol_type = other DNA
ctagaatgcagacttccacagagcaagg

SEQ ID NO: 39712 - DNA, 28 bp, synthetic construct
  source 1..28: mol_type = other DNA
tgagaaaggtaggggccttgctctgtgg

SEQ ID NO: 39713 - DNA, 28 bp, synthetic construct
  source 1..28: mol_type = other DNA
atacagtgatcattgagaaaggtagggg

SEQ ID NO: 39714 - DNA, 28 bp, synthetic construct
  source 1..28: mol_type = other DNA
gatacagtgatcattgagaaaggtaggg

SEQ ID NO: 39715 - DNA, 28 bp, synthetic construct
  source 1..28: mol_type = other DNA
ggatacagtgatcattgagaaaggtagg

SEQ ID NO: 39716 - DNA, 28 bp, synthetic construct
  source 1..28: mol_type = other DNA
gctgggatacagtgatcattgagaaagg

SEQ ID NO: 39717 - DNA, 28 bp, synthetic construct
  source 1..28: mol_type = other DNA
ctgtgtaacaggtgttgtagacgctggg

SEQ ID NO: 39718 - DNA, 28 bp, synthetic construct
  source 1..28: mol_type = other DNA
ccagcgtctacaacacctgttacacagg

SEQ ID NO: 39719 - DNA, 28 bp, synthetic construct
  source 1..28: mol_type = other DNA
gtgcattgatgacaacctgtgtaacagg

SEQ ID NO: 39720 - DNA, 28 bp, synthetic construct
  source 1..28: mol_type = other DNA
acaggttgtcatcaatgcacatgtatgg

SEQ ID NO: 39721 - DNA, 28 bp, synthetic construct
  source 1..28: mol_type = other DNA
tgcatgaaaaaaagatcgaaagagatgg

SEQ ID NO: 39722 - DNA, 28 bp, synthetic construct
  source 1..28: mol_type = other DNA
gcatgaaaaaaagatcgaaagagatggg

SEQ ID NO: 39723 - DNA, 28 bp, synthetic construct
  source 1..28: mol_type = other DNA
gaaaaaaagatcgaaagagatgggatgg

SEQ ID NO: 39724 - DNA, 28 bp, synthetic construct
  source 1..28: mol_type = other DNA
tggcacaaaaaacacaagaaactcctgg

SEQ ID NO: 39725 - DNA, 28 bp, synthetic construct
  source 1..28: mol_type = other DNA
aggagcggaaataattcaaattgccagg

SEQ ID NO: 39726 - DNA, 28 bp, synthetic construct
  source 1..28: mol_type = other DNA
agaggcggaaactgaggtgcaggagcgg

SEQ ID NO: 39727 - DNA, 28 bp, synthetic construct
  source 1..28: mol_type = other DNA
tttacagaggcggaaactgaggtgcagg

SEQ ID NO: 39728 - DNA, 28 bp, synthetic construct
  source 1..28: mol_type = other DNA
cacctcagtttccgcctctgtaaaatgg

SEQ ID NO: 39729 - DNA, 28 bp, synthetic construct
  source 1..28: mol_type = other DNA
acctcagtttccgcctctgtaaaatggg

SEQ ID NO: 39730 - DNA, 28 bp, synthetic construct
  source 1..28: mol_type = other DNA
gcccattttacagaggcggaaactgagg

SEQ ID NO: 39731 - DNA, 28 bp, synthetic construct
  source 1..28: mol_type = other DNA
gcagcgcgagcccattttacagaggcgg

SEQ ID NO: 39732 - DNA, 28 bp, synthetic construct
  source 1..28: mol_type = other DNA
aaggcagcgcgagcccattttacagagg

SEQ ID NO: 39733 - DNA, 28 bp, synthetic construct
  source 1..28: mol_type = other DNA
agagtgggcgggcggaggagggttaagg

SEQ ID NO: 39734 - DNA, 28 bp, synthetic construct
  source 1..28: mol_type = other DNA
ggtgtcagagtgggcgggcggaggaggg

SEQ ID NO: 39735 - DNA, 28 bp, synthetic construct
  source 1..28: mol_type = other DNA
tggtgtcagagtgggcgggcggaggagg

SEQ ID NO: 39736 - DNA, 28 bp, synthetic construct
  source 1..28: mol_type = other DNA
cggtggtgtcagagtgggcgggcggagg

SEQ ID NO: 39737 - DNA, 28 bp, synthetic construct
  source 1..28: mol_type = other DNA
ctccgcccgcccactctgacaccaccgg

SEQ ID NO: 39738 - DNA, 28 bp, synthetic construct
  source 1..28: mol_type = other DNA
ttccggtggtgtcagagtgggcgggcgg

SEQ ID NO: 39739 - DNA, 28 bp, synthetic construct
  source 1..28: mol_type = other DNA
cccgcccactctgacaccaccggaaagg

SEQ ID NO: 39740 - DNA, 28 bp, synthetic construct
  source 1..28: mol_type = other DNA
tcctttccggtggtgtcagagtgggcgg

SEQ ID NO: 39741 - DNA, 28 bp, synthetic construct
  source 1..28: mol_type = other DNA
gaatcctttccggtggtgtcagagtggg

SEQ ID NO: 39742 - DNA, 28 bp, synthetic construct
  source 1..28: mol_type = other DNA
tgaatcctttccggtggtgtcagagtgg

SEQ ID NO: 39743 - DNA, 28 bp, synthetic construct
  source 1..28: mol_type = other DNA
ctgacaccaccggaaaggattcattcgg

SEQ ID NO: 39744 - DNA, 28 bp, synthetic construct
  source 1..28: mol_type = other DNA
tgacaccaccggaaaggattcattcggg

SEQ ID NO: 39745 - DNA, 28 bp, synthetic construct
  source 1..28: mol_type = other DNA
atgttcccgaatgaatcctttccggtgg

SEQ ID NO: 39746 - DNA, 28 bp, synthetic construct
  source 1..28: mol_type = other DNA
cgaatgttcccgaatgaatcctttccgg

SEQ ID NO: 39747 - DNA, 28 bp, synthetic construct
  source 1..28: mol_type = other DNA
gaaaggattcattcgggaacattcgtgg

SEQ ID NO: 39748 - DNA, 28 bp, synthetic construct
  source 1..28: mol_type = other DNA
aaaggattcattcgggaacattcgtggg

SEQ ID NO: 39749 - DNA, 28 bp, synthetic construct
  source 1..28: mol_type = other DNA
aaggattcattcgggaacattcgtgggg

SEQ ID NO: 39750 - DNA, 28 bp, synthetic construct
  source 1..28: mol_type = other DNA
gattcattcgggaacattcgtggggcgg

SEQ ID NO: 39751 - DNA, 28 bp, synthetic construct
  source 1..28: mol_type = other DNA
ttcgggaacattcgtggggcggagacgg

SEQ ID NO: 39752 - DNA, 28 bp, synthetic construct
  source 1..28: mol_type = other DNA
tcgggaacattcgtggggcggagacggg

SEQ ID NO: 39753 - DNA, 28 bp, synthetic construct
  source 1..28: mol_type = other DNA
aacattcgtggggcggagacgggacagg

SEQ ID NO: 39754 - DNA, 28 bp, synthetic construct
  source 1..28: mol_type = other DNA
acattcgtggggcggagacgggacaggg

SEQ ID NO: 39755 - DNA, 28 bp, synthetic construct
  source 1..28: mol_type = other DNA
cattcgtggggcggagacgggacagggg

SEQ ID NO: 39756 - DNA, 28 bp, synthetic construct
  source 1..28: mol_type = other DNA
attcgtggggcggagacgggacaggggg

SEQ ID NO: 39757 - DNA, 28 bp, synthetic construct
  source 1..28: mol_type = other DNA
ggggcggagacgggacagggggcctcgg

SEQ ID NO: 39758 - DNA, 28 bp, synthetic construct
  source 1..28: mol_type = other DNA
ctggcggacgtgacgctacaggccgagg

SEQ ID NO: 39759 - DNA, 28 bp, synthetic construct
  source 1..28: mol_type = other DNA
ctcggcctgtagcgtcacgtccgccagg

SEQ ID NO: 39760 - DNA, 28 bp, synthetic construct
  source 1..28: mol_type = other DNA
tcggcctgtagcgtcacgtccgccaggg

SEQ ID NO: 39761 - DNA, 28 bp, synthetic construct
  source 1..28: mol_type = other DNA
gtaaccctggcggacgtgacgctacagg

SEQ ID NO: 39762 - DNA, 28 bp, synthetic construct
  source 1..28: mol_type = other DNA
gcgtcacgtccgccagggttacctgtgg

SEQ ID NO: 39763 - DNA, 28 bp, synthetic construct
  source 1..28: mol_type = other DNA
cgtcacgtccgccagggttacctgtggg

SEQ ID NO: 39764 - DNA, 28 bp, synthetic construct
  source 1..28: mol_type = other DNA
gtcacgtccgccagggttacctgtgggg

SEQ ID NO: 39765 - DNA, 28 bp, synthetic construct
  source 1..28: mol_type = other DNA
cgtccgccagggttacctgtggggctgg

SEQ ID NO: 39766 - DNA, 28 bp, synthetic construct
  source 1..28: mol_type = other DNA
gtccgccagggttacctgtggggctggg

SEQ ID NO: 39767 - DNA, 28 bp, synthetic construct
  source 1..28: mol_type = other DNA
ctcccagccccacaggtaaccctggcgg

SEQ ID NO: 39768 - DNA, 28 bp, synthetic construct
  source 1..28: mol_type = other DNA
tcgctcccagccccacaggtaaccctgg

SEQ ID NO: 39769 - DNA, 28 bp, synthetic construct
  source 1..28: mol_type = other DNA
gagtgcggttcgctcccagccccacagg

SEQ ID NO: 39770 - DNA, 28 bp, synthetic construct
  source 1..28: mol_type = other DNA
gcgaaccgcactcgcaccgcaaccccgg

SEQ ID NO: 39771 - DNA, 28 bp, synthetic construct
  source 1..28: mol_type = other DNA
tgatgccggggttgcggtgcgagtgcgg

SEQ ID NO: 39772 - DNA, 28 bp, synthetic construct
  source 1..28: mol_type = other DNA
caccgcaaccccggcatcagtgcccagg

SEQ ID NO: 39773 - DNA, 28 bp, synthetic construct
  source 1..28: mol_type = other DNA
aacctgggcactgatgccggggttgcgg

SEQ ID NO: 39774 - DNA, 28 bp, synthetic construct
  source 1..28: mol_type = other DNA
gcaaccccggcatcagtgcccaggttgg

SEQ ID NO: 39775 - DNA, 28 bp, synthetic construct
  source 1..28: mol_type = other DNA
gaggccaacctgggcactgatgccgggg

SEQ ID NO: 39776 - DNA, 28 bp, synthetic construct
  source 1..28: mol_type = other DNA
cgaggccaacctgggcactgatgccggg

SEQ ID NO: 39777 - DNA, 28 bp, synthetic construct
  source 1..28: mol_type = other DNA
gcgaggccaacctgggcactgatgccgg

SEQ ID NO: 39778 - DNA, 28 bp, synthetic construct
  source 1..28: mol_type = other DNA
ccgtaggacggcgcgaggccaacctggg

SEQ ID NO: 39779 - DNA, 28 bp, synthetic construct
  source 1..28: mol_type = other DNA
cccgtaggacggcgcgaggccaacctgg

SEQ ID NO: 39780 - DNA, 28 bp, synthetic construct
  source 1..28: mol_type = other DNA
caggttggcctcgcgccgtcctacgggg

SEQ ID NO: 39781 - DNA, 28 bp, synthetic construct
  source 1..28: mol_type = other DNA
gttggcctcgcgccgtcctacggggcgg

SEQ ID NO: 39782 - DNA, 28 bp, synthetic construct
  source 1..28: mol_type = other DNA
tctggccgccccgtaggacggcgcgagg

SEQ ID NO: 39783 - DNA, 28 bp, synthetic construct
  source 1..28: mol_type = other DNA
tcgcgccgtcctacggggcggccagagg

SEQ ID NO: 39784 - DNA, 28 bp, synthetic construct
  source 1..28: mol_type = other DNA
ggcggcctctggccgccccgtaggacgg

SEQ ID NO: 39785 - DNA, 28 bp, synthetic construct
  source 1..28: mol_type = other DNA
cttcggcggcctctggccgccccgtagg

SEQ ID NO: 39786 - DNA, 28 bp, synthetic construct
  source 1..28: mol_type = other DNA
ctacggggcggccagaggccgccgaagg

SEQ ID NO: 39787 - DNA, 28 bp, synthetic construct
  source 1..28: mol_type = other DNA
agcgcgagaggccttcggcggcctctgg

SEQ ID NO: 39788 - DNA, 28 bp, synthetic construct
  source 1..28: mol_type = other DNA
ctgctgcagcgcgagaggccttcggcgg

SEQ ID NO: 39789 - DNA, 28 bp, synthetic construct
  source 1..28: mol_type = other DNA
agactgctgcagcgcgagaggccttcgg

SEQ ID NO: 39790 - DNA, 28 bp, synthetic construct
  source 1..28: mol_type = other DNA
cctgaggagactgctgcagcgcgagagg

SEQ ID NO: 39791 - DNA, 28 bp, synthetic construct
  source 1..28: mol_type = other DNA
cagtctcctcaggagcgccgccatgtgg

SEQ ID NO: 39792 - DNA, 28 bp, synthetic construct
  source 1..28: mol_type = other DNA
agtctcctcaggagcgccgccatgtggg

SEQ ID NO: 39793 - DNA, 28 bp, synthetic construct
  source 1..28: mol_type = other DNA
tcctcaggagcgccgccatgtgggatgg

SEQ ID NO: 39794 - DNA, 28 bp, synthetic construct
  source 1..28: mol_type = other DNA
tccatcccacatggcggcgctcctgagg

SEQ ID NO: 39795 - DNA, 28 bp, synthetic construct
  source 1..28: mol_type = other DNA
acgtgtgctattccatcccacatggcgg

SEQ ID NO: 39796 - DNA, 28 bp, synthetic construct
  source 1..28: mol_type = other DNA
gccatgtgggatggaatagcacacgtgg

SEQ ID NO: 39797 - DNA, 28 bp, synthetic construct
  source 1..28: mol_type = other DNA
cccacgtgtgctattccatcccacatgg

SEQ ID NO: 39798 - DNA, 28 bp, synthetic construct
  source 1..28: mol_type = other DNA
cgtgggcttctccctgcgtcacttccgg

SEQ ID NO: 39799 - DNA, 28 bp, synthetic construct
  source 1..28: mol_type = other DNA
gtgggcttctccctgcgtcacttccggg

SEQ ID NO: 39800 - DNA, 28 bp, synthetic construct
  source 1..28: mol_type = other DNA
tgggcttctccctgcgtcacttccgggg

SEQ ID NO: 39801 - DNA, 28 bp, synthetic construct
  source 1..28: mol_type = other DNA
ggaagcagtccccggaagtgacgcaggg

SEQ ID NO: 39802 - DNA, 28 bp, synthetic construct
  source 1..28: mol_type = other DNA
tggaagcagtccccggaagtgacgcagg

SEQ ID NO: 39803 - DNA, 28 bp, synthetic construct
  source 1..28: mol_type = other DNA
cttccggggactgcttccagccaatcgg

SEQ ID NO: 39804 - DNA, 28 bp, synthetic construct
  source 1..28: mol_type = other DNA
aggccgattggctggaagcagtccccgg

SEQ ID NO: 39805 - DNA, 28 bp, synthetic construct
  source 1..28: mol_type = other DNA
ctggctgtggcggaggccgattggctgg

SEQ ID NO: 39806 - DNA, 28 bp, synthetic construct
  source 1..28: mol_type = other DNA
tgcgctggctgtggcggaggccgattgg

SEQ ID NO: 39807 - DNA, 28 bp, synthetic construct
  source 1..28: mol_type = other DNA
ggcaaggctgcgctggctgtggcggagg

SEQ ID NO: 39808 - DNA, 28 bp, synthetic construct
  source 1..28: mol_type = other DNA
aggggcaaggctgcgctggctgtggcgg

SEQ ID NO: 39809 - DNA, 28 bp, synthetic construct
  source 1..28: mol_type = other DNA
ttaaggggcaaggctgcgctggctgtgg

SEQ ID NO: 39810 - DNA, 28 bp, synthetic construct
  source 1..28: mol_type = other DNA
gtgactttaaggggcaaggctgcgctgg

SEQ ID NO: 39811 - DNA, 28 bp, synthetic construct
  source 1..28: mol_type = other DNA
gcgcagccttgccccttaaagtcacagg

SEQ ID NO: 39812 - DNA, 28 bp, synthetic construct
  source 1..28: mol_type = other DNA
agggggcctgtgactttaaggggcaagg

SEQ ID NO: 39813 - DNA, 28 bp, synthetic construct
  source 1..28: mol_type = other DNA
gcgctagggggcctgtgactttaagggg

SEQ ID NO: 39814 - DNA, 28 bp, synthetic construct
  source 1..28: mol_type = other DNA
cgcgctagggggcctgtgactttaaggg

SEQ ID NO: 39815 - DNA, 28 bp, synthetic construct
  source 1..28: mol_type = other DNA
tcgcgctagggggcctgtgactttaagg

SEQ ID NO: 39816 - DNA, 28 bp, synthetic construct
  source 1..28: mol_type = other DNA
ggggggcgtgggatttcgcgctaggggg

SEQ ID NO: 39817 - DNA, 28 bp, synthetic construct
  source 1..28: mol_type = other DNA
aggggggcgtgggatttcgcgctagggg

SEQ ID NO: 39818 - DNA, 28 bp, synthetic construct
  source 1..28: mol_type = other DNA
caggggggcgtgggatttcgcgctaggg

SEQ ID NO: 39819 - DNA, 28 bp, synthetic construct
  source 1..28: mol_type = other DNA
ccaggggggcgtgggatttcgcgctagg

SEQ ID NO: 39820 - DNA, 28 bp, synthetic construct
  source 1..28: mol_type = other DNA
gcgcgaaatcccacgcccccctggacgg

SEQ ID NO: 39821 - DNA, 28 bp, synthetic construct
  source 1..28: mol_type = other DNA
aatcccacgcccccctggacggctgcgg

SEQ ID NO: 39822 - DNA, 28 bp, synthetic construct
  source 1..28: mol_type = other DNA
cggccgcagccgtccaggggggcgtggg

SEQ ID NO: 39823 - DNA, 28 bp, synthetic construct
  source 1..28: mol_type = other DNA
gcggccgcagccgtccaggggggcgtgg

SEQ ID NO: 39824 - DNA, 28 bp, synthetic construct
  source 1..28: mol_type = other DNA
cgagtgcggccgcagccgtccagggggg

SEQ ID NO: 39825 - DNA, 28 bp, synthetic construct
  source 1..28: mol_type = other DNA
gcgagtgcggccgcagccgtccaggggg

SEQ ID NO: 39826 - DNA, 28 bp, synthetic construct
  source 1..28: mol_type = other DNA
ggcgagtgcggccgcagccgtccagggg

SEQ ID NO: 39827 - DNA, 28 bp, synthetic construct
  source 1..28: mol_type = other DNA
tggcgagtgcggccgcagccgtccaggg

SEQ ID NO: 39828 - DNA, 28 bp, synthetic construct
  source 1..28: mol_type = other DNA
gtggcgagtgcggccgcagccgtccagg

SEQ ID NO: 39829 - DNA, 28 bp, synthetic construct
  source 1..28: mol_type = other DNA
gacggctgcggccgcactcgccaccagg

SEQ ID NO: 39830 - DNA, 28 bp, synthetic construct
  source 1..28: mol_type = other DNA
acggctgcggccgcactcgccaccaggg

SEQ ID NO: 39831 - DNA, 28 bp, synthetic construct
  source 1..28: mol_type = other DNA
cggctgcggccgcactcgccaccagggg

SEQ ID NO: 39832 - DNA, 28 bp, synthetic construct
  source 1..28: mol_type = other DNA
ggctgcggccgcactcgccaccaggggg

SEQ ID NO: 39833 - DNA, 28 bp, synthetic construct
  source 1..28: mol_type = other DNA
ggccgcactcgccaccagggggcagagg

SEQ ID NO: 39834 - DNA, 28 bp, synthetic construct
  source 1..28: mol_type = other DNA
ggcctctgccccctggtggcgagtgcgg

SEQ ID NO: 39835 - DNA, 28 bp, synthetic construct
  source 1..28: mol_type = other DNA
ccaccagggggcagaggccagagaaagg

SEQ ID NO: 39836 - DNA, 28 bp, synthetic construct
  source 1..28: mol_type = other DNA
caccagggggcagaggccagagaaaggg

SEQ ID NO: 39837 - DNA, 28 bp, synthetic construct
  source 1..28: mol_type = other DNA
agccctttctctggcctctgccccctgg

SEQ ID NO: 39838 - DNA, 28 bp, synthetic construct
  source 1..28: mol_type = other DNA
agaggccagagaaagggctatttcccgg

SEQ ID NO: 39839 - DNA, 28 bp, synthetic construct
  source 1..28: mol_type = other DNA
cgggtccgggaaatagccctttctctgg

SEQ ID NO: 39840 - DNA, 28 bp, synthetic construct
  source 1..28: mol_type = other DNA
tttcccggacccgcccccttcagcttgg

SEQ ID NO: 39841 - DNA, 28 bp, synthetic construct
  source 1..28: mol_type = other DNA
ttcccggacccgcccccttcagcttggg

SEQ ID NO: 39842 - DNA, 28 bp, synthetic construct
  source 1..28: mol_type = other DNA
ttcccaagctgaagggggcgggtccggg

SEQ ID NO: 39843 - DNA, 28 bp, synthetic construct
  source 1..28: mol_type = other DNA
tttcccaagctgaagggggcgggtccgg

SEQ ID NO: 39844 - DNA, 28 bp, synthetic construct
  source 1..28: mol_type = other DNA
ttcgctttcccaagctgaagggggcggg

SEQ ID NO: 39845 - DNA, 28 bp, synthetic construct
  source 1..28: mol_type = other DNA
tttcgctttcccaagctgaagggggcgg

SEQ ID NO: 39846 - DNA, 28 bp, synthetic construct
  source 1..28: mol_type = other DNA
cgctttcgctttcccaagctgaaggggg

SEQ ID NO: 39847 - DNA, 28 bp, synthetic construct
  source 1..28: mol_type = other DNA
acgctttcgctttcccaagctgaagggg

SEQ ID NO: 39848 - DNA, 28 bp, synthetic construct
  source 1..28: mol_type = other DNA
cacgctttcgctttcccaagctgaaggg

SEQ ID NO: 39849 - DNA, 28 bp, synthetic construct
  source 1..28: mol_type = other DNA
ccttcagcttgggaaagcgaaagcgtgg

SEQ ID NO: 39850 - DNA, 28 bp, synthetic construct
  source 1..28: mol_type = other DNA
cagcttgggaaagcgaaagcgtggcagg

SEQ ID NO: 39851 - DNA, 28 bp, synthetic construct
  source 1..28: mol_type = other DNA
agcttgggaaagcgaaagcgtggcaggg

SEQ ID NO: 39852 - DNA, 28 bp, synthetic construct
  source 1..28: mol_type = other DNA
gcttgggaaagcgaaagcgtggcagggg

SEQ ID NO: 39853 - DNA, 28 bp, synthetic construct
  source 1..28: mol_type = other DNA
gggaaagcgaaagcgtggcaggggccgg

SEQ ID NO: 39854 - DNA, 28 bp, synthetic construct
  source 1..28: mol_type = other DNA
gcgaaagcgtggcaggggccggacctgg

SEQ ID NO: 39855 - DNA, 28 bp, synthetic construct
  source 1..28: mol_type = other DNA
cgaaagcgtggcaggggccggacctggg

SEQ ID NO: 39856 - DNA, 28 bp, synthetic construct
  source 1..28: mol_type = other DNA
gcgtggcaggggccggacctgggagcgg

SEQ ID NO: 39857 - DNA, 28 bp, synthetic construct
  source 1..28: mol_type = other DNA
tggcaggggccggacctgggagcggagg

SEQ ID NO: 39858 - DNA, 28 bp, synthetic construct
  source 1..28: mol_type = other DNA
caggggccggacctgggagcggaggagg

SEQ ID NO: 39859 - DNA, 28 bp, synthetic construct
  source 1..28: mol_type = other DNA
gggccggacctgggagcggaggaggcgg

SEQ ID NO: 39860 - DNA, 28 bp, synthetic construct
  source 1..28: mol_type = other DNA
ggccggacctgggagcggaggaggcggg

SEQ ID NO: 39861 - DNA, 28 bp, synthetic construct
  source 1..28: mol_type = other DNA
gacccgcctcctccgctcccaggtccgg

SEQ ID NO: 39862 - DNA, 28 bp, synthetic construct
  source 1..28: mol_type = other DNA
atggagacccgcctcctccgctcccagg

SEQ ID NO: 39863 - DNA, 28 bp, synthetic construct
  source 1..28: mol_type = other DNA
ctccatagaaacctccacctgtttccgg

SEQ ID NO: 39864 - DNA, 28 bp, synthetic construct
  source 1..28: mol_type = other DNA
ggccggaaacaggtggaggtttctatgg

SEQ ID NO: 39865 - DNA, 28 bp, synthetic construct
  source 1..28: mol_type = other DNA
atagaaacctccacctgtttccggccgg

SEQ ID NO: 39866 - DNA, 28 bp, synthetic construct
  source 1..28: mol_type = other DNA
tagaaacctccacctgtttccggccggg

SEQ ID NO: 39867 - DNA, 28 bp, synthetic construct
  source 1..28: mol_type = other DNA
tcacagcccggccggaaacaggtggagg

SEQ ID NO: 39868 - DNA, 28 bp, synthetic construct
  source 1..28: mol_type = other DNA
ctctcacagcccggccggaaacaggtgg

SEQ ID NO: 39869 - DNA, 28 bp, synthetic construct
  source 1..28: mol_type = other DNA
aatctctcacagcccggccggaaacagg

SEQ ID NO: 39870 - DNA, 28 bp, synthetic construct
  source 1..28: mol_type = other DNA
gtttccggccgggctgtgagagattagg

SEQ ID NO: 39871 - DNA, 28 bp, synthetic construct
  source 1..28: mol_type = other DNA
tttccggccgggctgtgagagattaggg

SEQ ID NO: 39872 - DNA, 28 bp, synthetic construct
  source 1..28: mol_type = other DNA
ttccggccgggctgtgagagattagggg

SEQ ID NO: 39873 - DNA, 28 bp, synthetic construct
  source 1..28: mol_type = other DNA
agcccctaatctctcacagcccggccgg

SEQ ID NO: 39874 - DNA, 28 bp, synthetic construct
  source 1..28: mol_type = other DNA
cagcagcccctaatctctcacagcccgg

SEQ ID NO: 39875 - DNA, 28 bp, synthetic construct
  source 1..28: mol_type = other DNA
ggctgtgagagattaggggctgctgcgg

SEQ ID NO: 39876 - DNA, 28 bp, synthetic construct
  source 1..28: mol_type = other DNA
gctgtgagagattaggggctgctgcggg

SEQ ID NO: 39877 - DNA, 28 bp, synthetic construct
  source 1..28: mol_type = other DNA
ctgtgagagattaggggctgctgcgggg

SEQ ID NO: 39878 - DNA, 28 bp, synthetic construct
  source 1..28: mol_type = other DNA
tgtgagagattaggggctgctgcggggg

SEQ ID NO: 39879 - DNA, 28 bp, synthetic construct
  source 1..28: mol_type = other DNA
tgggaagaggcgagctggctgagattgg

SEQ ID NO: 39880 - DNA, 28 bp, synthetic construct
  source 1..28: mol_type = other DNA
tctcagccagctcgcctcttcccagcgg

SEQ ID NO: 39881 - DNA, 28 bp, synthetic construct
  source 1..28: mol_type = other DNA
cagaggccgctgggaagaggcgagctgg

SEQ ID NO: 39882 - DNA, 28 bp, synthetic construct
  source 1..28: mol_type = other DNA
gctcgcctcttcccagcggcctctgcgg

SEQ ID NO: 39883 - DNA, 28 bp, synthetic construct
  source 1..28: mol_type = other DNA
ctcgcctcttcccagcggcctctgcggg

SEQ ID NO: 39884 - DNA, 28 bp, synthetic construct
  source 1..28: mol_type = other DNA
cgctcccgcagaggccgctgggaagagg

SEQ ID NO: 39885 - DNA, 28 bp, synthetic construct
  source 1..28: mol_type = other DNA
ctcttcccagcggcctctgcgggagcgg

SEQ ID NO: 39886 - DNA, 28 bp, synthetic construct
  source 1..28: mol_type = other DNA
ttcccagcggcctctgcgggagcggtgg

SEQ ID NO: 39887 - DNA, 28 bp, synthetic construct
  source 1..28: mol_type = other DNA
tcccagcggcctctgcgggagcggtggg

SEQ ID NO: 39888 - DNA, 28 bp, synthetic construct
  source 1..28: mol_type = other DNA
acccaccgctcccgcagaggccgctggg

SEQ ID NO: 39889 - DNA, 28 bp, synthetic construct
  source 1..28: mol_type = other DNA
cacccaccgctcccgcagaggccgctgg

SEQ ID NO: 39890 - DNA, 28 bp, synthetic construct
  source 1..28: mol_type = other DNA
tgtacaacacccaccgctcccgcagagg

SEQ ID NO: 39891 - DNA, 28 bp, synthetic construct
  source 1..28: mol_type = other DNA
cggtgggtgttgtacacaatcatcatgg

SEQ ID NO: 39892 - DNA, 28 bp, synthetic construct
  source 1..28: mol_type = other DNA
tgggtgttgtacacaatcatcatggcgg

SEQ ID NO: 39893 - DNA, 28 bp, synthetic construct
  source 1..28: mol_type = other DNA
gtgttgtacacaatcatcatggcggcgg

SEQ ID NO: 39894 - DNA, 28 bp, synthetic construct
  source 1..28: mol_type = other DNA
tgtacacaatcatcatggcggcggccgg

SEQ ID NO: 39895 - DNA, 28 bp, synthetic construct
  source 1..28: mol_type = other DNA
gtacacaatcatcatggcggcggccggg

SEQ ID NO: 39896 - DNA, 28 bp, synthetic construct
  source 1..28: mol_type = other DNA
tacacaatcatcatggcggcggccgggg

SEQ ID NO: 39897 - DNA, 28 bp, synthetic construct
  source 1..28: mol_type = other DNA
atcatcatggcggcggccggggccccgg

SEQ ID NO: 39898 - DNA, 28 bp, synthetic construct
  source 1..28: mol_type = other DNA
tcatggcggcggccggggccccggatgg

SEQ ID NO: 39899 - DNA, 28 bp, synthetic construct
  source 1..28: mol_type = other DNA
cggccggggccccggatggtgagtgcgg

SEQ ID NO: 39900 - DNA, 28 bp, synthetic construct
  source 1..28: mol_type = other DNA
ccggggccccggatggtgagtgcggcgg

SEQ ID NO: 39901 - DNA, 28 bp, synthetic construct
  source 1..28: mol_type = other DNA
cggggccccggatggtgagtgcggcggg

SEQ ID NO: 39902 - DNA, 28 bp, synthetic construct
  source 1..28: mol_type = other DNA
ggggccccggatggtgagtgcggcgggg

SEQ ID NO: 39903 - DNA, 28 bp, synthetic construct
  source 1..28: mol_type = other DNA
gggccccggatggtgagtgcggcggggg

SEQ ID NO: 39904 - DNA, 28 bp, synthetic construct
  source 1..28: mol_type = other DNA
ccccggatggtgagtgcggcgggggtgg

SEQ ID NO: 39905 - DNA, 28 bp, synthetic construct
  source 1..28: mol_type = other DNA
gccacccccgccgcactcaccatccggg

SEQ ID NO: 39906 - DNA, 28 bp, synthetic construct
  source 1..28: mol_type = other DNA
cgccacccccgccgcactcaccatccgg

SEQ ID NO: 39907 - DNA, 28 bp, synthetic construct
  source 1..28: mol_type = other DNA
cggatggtgagtgcggcgggggtggcgg

SEQ ID NO: 39908 - DNA, 28 bp, synthetic construct
  source 1..28: mol_type = other DNA
ggatggtgagtgcggcgggggtggcggg

SEQ ID NO: 39909 - DNA, 28 bp, synthetic construct
  source 1..28: mol_type = other DNA
tgagtgcggcgggggtggcgggcgccgg

SEQ ID NO: 39910 - DNA, 28 bp, synthetic construct
  source 1..28: mol_type = other DNA
gagtgcggcgggggtggcgggcgccggg

SEQ ID NO: 39911 - DNA, 28 bp, synthetic construct
  source 1..28: mol_type = other DNA
gcggcgggggtggcgggcgccgggccgg

SEQ ID NO: 39912 - DNA, 28 bp, synthetic construct
  source 1..28: mol_type = other DNA
cggcgggggtggcgggcgccgggccggg

SEQ ID NO: 39913 - DNA, 28 bp, synthetic construct
  source 1..28: mol_type = other DNA
ggcgggggtggcgggcgccgggccgggg

SEQ ID NO: 39914 - DNA, 28 bp, synthetic construct
  source 1..28: mol_type = other DNA
ggtggcgggcgccgggccggggctgagg

SEQ ID NO: 39915 - DNA, 28 bp, synthetic construct
  source 1..28: mol_type = other DNA
gggcgccgggccggggctgaggttgcgg

SEQ ID NO: 39916 - DNA, 28 bp, synthetic construct
  source 1..28: mol_type = other DNA
agcgaccgcaacctcagccccggcccgg

SEQ ID NO: 39917 - DNA, 28 bp, synthetic construct
  source 1..28: mol_type = other DNA
agaggagcgaccgcaacctcagccccgg

SEQ ID NO: 39918 - DNA, 28 bp, synthetic construct
  source 1..28: mol_type = other DNA
ggggctgaggttgcggtcgctcctctgg

SEQ ID NO: 39919 - DNA, 28 bp, synthetic construct
  source 1..28: mol_type = other DNA
gggctgaggttgcggtcgctcctctggg

SEQ ID NO: 39920 - DNA, 28 bp, synthetic construct
  source 1..28: mol_type = other DNA
ggctgaggttgcggtcgctcctctgggg

SEQ ID NO: 39921 - DNA, 28 bp, synthetic construct
  source 1..28: mol_type = other DNA
gctgaggttgcggtcgctcctctggggg

SEQ ID NO: 39922 - DNA, 28 bp, synthetic construct
  source 1..28: mol_type = other DNA
gttgcggtcgctcctctgggggatgcgg

SEQ ID NO: 39923 - DNA, 28 bp, synthetic construct
  source 1..28: mol_type = other DNA
ggtcgctcctctgggggatgcggcccgg

SEQ ID NO: 39924 - DNA, 28 bp, synthetic construct
  source 1..28: mol_type = other DNA
ctcctctgggggatgcggcccggcccgg

SEQ ID NO: 39925 - DNA, 28 bp, synthetic construct
  source 1..28: mol_type = other DNA
tcctctgggggatgcggcccggcccggg

SEQ ID NO: 39926 - DNA, 28 bp, synthetic construct
  source 1..28: mol_type = other DNA
tcccgggccgggccgcatcccccagagg

SEQ ID NO: 39927 - DNA, 28 bp, synthetic construct
  source 1..28: mol_type = other DNA
tctgggggatgcggcccggcccgggagg

SEQ ID NO: 39928 - DNA, 28 bp, synthetic construct
  source 1..28: mol_type = other DNA
ctgggggatgcggcccggcccgggaggg

SEQ ID NO: 39929 - DNA, 28 bp, synthetic construct
  source 1..28: mol_type = other DNA
cggcccggcccgggagggagaaccgcgg

SEQ ID NO: 39930 - DNA, 28 bp, synthetic construct
  source 1..28: mol_type = other DNA
gagccgcggttctccctcccgggccggg

SEQ ID NO: 39931 - DNA, 28 bp, synthetic construct
  source 1..28: mol_type = other DNA
cgagccgcggttctccctcccgggccgg

SEQ ID NO: 39932 - DNA, 28 bp, synthetic construct
  source 1..28: mol_type = other DNA
cggcccgggagggagaaccgcggctcgg

SEQ ID NO: 39933 - DNA, 28 bp, synthetic construct
  source 1..28: mol_type = other DNA
ggcccgggagggagaaccgcggctcggg

SEQ ID NO: 39934 - DNA, 28 bp, synthetic construct
  source 1..28: mol_type = other DNA
ttcccgagccgcggttctccctcccggg

SEQ ID NO: 39935 - DNA, 28 bp, synthetic construct
  source 1..28: mol_type = other DNA
gttcccgagccgcggttctccctcccgg

SEQ ID NO: 39936 - DNA, 28 bp, synthetic construct
  source 1..28: mol_type = other DNA
gggagggagaaccgcggctcgggaacgg

SEQ ID NO: 39937 - DNA, 28 bp, synthetic construct
  source 1..28: mol_type = other DNA
agggagaaccgcggctcgggaacggagg

SEQ ID NO: 39938 - DNA, 28 bp, synthetic construct
  source 1..28: mol_type = other DNA
gaaccgcggctcgggaacggaggtccgg

SEQ ID NO: 39939 - DNA, 28 bp, synthetic construct
  source 1..28: mol_type = other DNA
ccgcggctcgggaacggaggtccggcgg

SEQ ID NO: 39940 - DNA, 28 bp, synthetic construct
  source 1..28: mol_type = other DNA
tcgggaacggaggtccggcggcgcccgg

SEQ ID NO: 39941 - DNA, 28 bp, synthetic construct
  source 1..28: mol_type = other DNA
ggaacggacgctgtccgggcgccgccgg

SEQ ID NO: 39942 - DNA, 28 bp, synthetic construct
  source 1..28: mol_type = other DNA
ctgggcttgggaacggacgctgtccggg

SEQ ID NO: 39943 - DNA, 28 bp, synthetic construct
  source 1..28: mol_type = other DNA
gctgggcttgggaacggacgctgtccgg

SEQ ID NO: 39944 - DNA, 28 bp, synthetic construct
  source 1..28: mol_type = other DNA
agcgtccgttcccaagcccagcccgcgg

SEQ ID NO: 39945 - DNA, 28 bp, synthetic construct
  source 1..28: mol_type = other DNA
gctcgccgcgggctgggcttgggaacgg

SEQ ID NO: 39946 - DNA, 28 bp, synthetic construct
  source 1..28: mol_type = other DNA
tgggcgctcgccgcgggctgggcttggg

SEQ ID NO: 39947 - DNA, 28 bp, synthetic construct
  source 1..28: mol_type = other DNA
gtgggcgctcgccgcgggctgggcttgg

SEQ ID NO: 39948 - DNA, 28 bp, synthetic construct
  source 1..28: mol_type = other DNA
agggggtgggcgctcgccgcgggctggg

SEQ ID NO: 39949 - DNA, 28 bp, synthetic construct
  source 1..28: mol_type = other DNA
tagggggtgggcgctcgccgcgggctgg

SEQ ID NO: 39950 - DNA, 28 bp, synthetic construct
  source 1..28: mol_type = other DNA
gggttagggggtgggcgctcgccgcggg

SEQ ID NO: 39951 - DNA, 28 bp, synthetic construct
  source 1..28: mol_type = other DNA
ggggttagggggtgggcgctcgccgcgg

SEQ ID NO: 39952 - DNA, 28 bp, synthetic construct
  source 1..28: mol_type = other DNA
agcgcccaccccctaacccccttgcagg

SEQ ID NO: 39953 - DNA, 28 bp, synthetic construct
  source 1..28: mol_type = other DNA
catgcctgcaagggggttagggggtggg

SEQ ID NO: 39954 - DNA, 28 bp, synthetic construct
  source 1..28: mol_type = other DNA
ccatgcctgcaagggggttagggggtgg

SEQ ID NO: 39955 - DNA, 28 bp, synthetic construct
  source 1..28: mol_type = other DNA
cctccatgcctgcaagggggttaggggg

SEQ ID NO: 39956 - DNA, 28 bp, synthetic construct
  source 1..28: mol_type = other DNA
tcctccatgcctgcaagggggttagggg

SEQ ID NO: 39957 - DNA, 28 bp, synthetic construct
  source 1..28: mol_type = other DNA
ttcctccatgcctgcaagggggttaggg

SEQ ID NO: 39958 - DNA, 28 bp, synthetic construct
  source 1..28: mol_type = other DNA
gttcctccatgcctgcaagggggttagg

SEQ ID NO: 39959 - DNA, 28 bp, synthetic construct
  source 1..28: mol_type = other DNA
acccccttgcaggcatggaggaacctgg

SEQ ID NO: 39960 - DNA, 28 bp, synthetic construct
  source 1..28: mol_type = other DNA
gccaggttcctccatgcctgcaaggggg

SEQ ID NO: 39961 - DNA, 28 bp, synthetic construct
  source 1..28: mol_type = other DNA
tgccaggttcctccatgcctgcaagggg

SEQ ID NO: 39962 - DNA, 28 bp, synthetic construct
  source 1..28: mol_type = other DNA
atgccaggttcctccatgcctgcaaggg

SEQ ID NO: 39963 - DNA, 28 bp, synthetic construct
  source 1..28: mol_type = other DNA
catgccaggttcctccatgcctgcaagg

SEQ ID NO: 39964 - DNA, 28 bp, synthetic construct
  source 1..28: mol_type = other DNA
cttgcaggcatggaggaacctggcatgg

SEQ ID NO: 39965 - DNA, 28 bp, synthetic construct
  source 1..28: mol_type = other DNA
ggcatggaggaacctggcatggacacgg

SEQ ID NO: 39966 - DNA, 28 bp, synthetic construct
  source 1..28: mol_type = other DNA
atggaggaacctggcatggacacggagg

SEQ ID NO: 39967 - DNA, 28 bp, synthetic construct
  source 1..28: mol_type = other DNA
cagtctcggcctccgtgtccatgccagg

SEQ ID NO: 39968 - DNA, 28 bp, synthetic construct
  source 1..28: mol_type = other DNA
ggcatggacacggaggccgagactgtgg

SEQ ID NO: 39969 - DNA, 28 bp, synthetic construct
  source 1..28: mol_type = other DNA
acggaggccgagactgtggctactgagg

SEQ ID NO: 39970 - DNA, 28 bp, synthetic construct
  source 1..28: mol_type = other DNA
gcgggagcctcagtagccacagtctcgg

SEQ ID NO: 39971 - DNA, 28 bp, synthetic construct
  source 1..28: mol_type = other DNA
gactgtggctactgaggctcccgcgcgg

SEQ ID NO: 39972 - DNA, 28 bp, synthetic construct
  source 1..28: mol_type = other DNA
gctcccgcgcggcccgtcaactgcctgg

SEQ ID NO: 39973 - DNA, 28 bp, synthetic construct
  source 1..28: mol_type = other DNA
cccgcgcggcccgtcaactgcctggagg

SEQ ID NO: 39974 - DNA, 28 bp, synthetic construct
  source 1..28: mol_type = other DNA
gcctccaggcagttgacgggccgcgcgg

SEQ ID NO: 39975 - DNA, 28 bp, synthetic construct
  source 1..28: mol_type = other DNA
cggcttcagcctccaggcagttgacggg

SEQ ID NO: 39976 - DNA, 28 bp, synthetic construct
  source 1..28: mol_type = other DNA
gcggcttcagcctccaggcagttgacgg

SEQ ID NO: 39977 - DNA, 28 bp, synthetic construct
  source 1..28: mol_type = other DNA
gtcaactgcctggaggctgaagccgcgg

SEQ ID NO: 39978 - DNA, 28 bp, synthetic construct
  source 1..28: mol_type = other DNA
aactgcctggaggctgaagccgcggcgg

SEQ ID NO: 39979 - DNA, 28 bp, synthetic construct
  source 1..28: mol_type = other DNA
actgcctggaggctgaagccgcggcggg

SEQ ID NO: 39980 - DNA, 28 bp, synthetic construct
  source 1..28: mol_type = other DNA
ctgcctggaggctgaagccgcggcgggg

SEQ ID NO: 39981 - DNA, 28 bp, synthetic construct
  source 1..28: mol_type = other DNA
tgcctggaggctgaagccgcggcggggg

SEQ ID NO: 39982 - DNA, 28 bp, synthetic construct
  source 1..28: mol_type = other DNA
cgcccccgccgcggcttcagcctccagg

SEQ ID NO: 39983 - DNA, 28 bp, synthetic construct
  source 1..28: mol_type = other DNA
ctggaggctgaagccgcggcgggggcgg

SEQ ID NO: 39984 - DNA, 28 bp, synthetic construct
  source 1..28: mol_type = other DNA
gaggctgaagccgcggcgggggcggcgg

SEQ ID NO: 39985 - DNA, 28 bp, synthetic construct
  source 1..28: mol_type = other DNA
gaagccgcggcgggggcggcggccgagg

SEQ ID NO: 39986 - DNA, 28 bp, synthetic construct
  source 1..28: mol_type = other DNA
gagtcctcggccgccgcccccgccgcgg

SEQ ID NO: 39987 - DNA, 28 bp, synthetic construct
  source 1..28: mol_type = other DNA
cggcgggggcggcggccgaggactccgg

SEQ ID NO: 39988 - DNA, 28 bp, synthetic construct
  source 1..28: mol_type = other DNA
cggccgaggactccggcgccgcacgagg

SEQ ID NO: 39989 - DNA, 28 bp, synthetic construct
  source 1..28: mol_type = other DNA
ctgcctcgtgcggcgccggagtcctcgg

SEQ ID NO: 39990 - DNA, 28 bp, synthetic construct
  source 1..28: mol_type = other DNA
ggctgcaggctgcctcgtgcggcgccgg

SEQ ID NO: 39991 - DNA, 28 bp, synthetic construct
  source 1..28: mol_type = other DNA
ggcgccgcacgaggcagcctgcagccgg

SEQ ID NO: 39992 - DNA, 28 bp, synthetic construct
  source 1..28: mol_type = other DNA
ggggccggctgcaggctgcctcgtgcgg

SEQ ID NO: 39993 - DNA, 28 bp, synthetic construct
  source 1..28: mol_type = other DNA
gcacgaggcagcctgcagccggccccgg

SEQ ID NO: 39994 - DNA, 28 bp, synthetic construct
  source 1..28: mol_type = other DNA
agggggctgggccggggccggctgcagg

SEQ ID NO: 39995 - DNA, 28 bp, synthetic construct
  source 1..28: mol_type = other DNA
tgcagccggccccggcccagccccctgg

SEQ ID NO: 39996 - DNA, 28 bp, synthetic construct
  source 1..28: mol_type = other DNA
gcagccggccccggcccagccccctggg

SEQ ID NO: 39997 - DNA, 28 bp, synthetic construct
  source 1..28: mol_type = other DNA
cagccggccccggcccagccccctgggg

SEQ ID NO: 39998 - DNA, 28 bp, synthetic construct
  source 1..28: mol_type = other DNA
ggtccccagggggctgggccggggccgg

SEQ ID NO: 39999 - DNA, 28 bp, synthetic construct
  source 1..28: mol_type = other DNA
gcggggtccccagggggctgggccgggg

SEQ ID NO: 40000 - DNA, 28 bp, synthetic construct
  source 1..28: mol_type = other DNA
tgcggggtccccagggggctgggccggg

SEQ ID NO: 40001 - DNA, 28 bp, synthetic construct
  source 1..28: mol_type = other DNA
ctgcggggtccccagggggctgggccgg

SEQ ID NO: 40002 - DNA, 28 bp, synthetic construct
  source 1..28: mol_type = other DNA
tgggctgcggggtccccagggggctggg

SEQ ID NO: 40003 - DNA, 28 bp, synthetic construct
  source 1..28: mol_type = other DNA
ctgggctgcggggtccccagggggctgg

SEQ ID NO: 40004 - DNA, 28 bp, synthetic construct
  source 1..28: mol_type = other DNA
cagccccctggggaccccgcagcccagg

SEQ ID NO: 40005 - DNA, 28 bp, synthetic construct
  source 1..28: mol_type = other DNA
aggcctgggctgcggggtccccaggggg

SEQ ID NO: 40006 - DNA, 28 bp, synthetic construct
  source 1..28: mol_type = other DNA
gaggcctgggctgcggggtccccagggg

SEQ ID NO: 40007 - DNA, 28 bp, synthetic construct
  source 1..28: mol_type = other DNA
cgaggcctgggctgcggggtccccaggg

SEQ ID NO: 40008 - DNA, 28 bp, synthetic construct
  source 1..28: mol_type = other DNA
cctggggaccccgcagcccaggcctcgg

SEQ ID NO: 40009 - DNA, 28 bp, synthetic construct
  source 1..28: mol_type = other DNA
gttgctgaccgaggcctgggctgcgggg

SEQ ID NO: 40010 - DNA, 28 bp, synthetic construct
  source 1..28: mol_type = other DNA
cgttgctgaccgaggcctgggctgcggg

SEQ ID NO: 40011 - DNA, 28 bp, synthetic construct
  source 1..28: mol_type = other DNA
ccgttgctgaccgaggcctgggctgcgg

SEQ ID NO: 40012 - DNA, 28 bp, synthetic construct
  source 1..28: mol_type = other DNA
tcttcgccgttgctgaccgaggcctggg

SEQ ID NO: 40013 - DNA, 28 bp, synthetic construct
  source 1..28: mol_type = other DNA
gtcttcgccgttgctgaccgaggcctgg

SEQ ID NO: 40014 - DNA, 28 bp, synthetic construct
  source 1..28: mol_type = other DNA
gcctcggtcagcaacggcgaagacgcgg

SEQ ID NO: 40015 - DNA, 28 bp, synthetic construct
  source 1..28: mol_type = other DNA
cctcggtcagcaacggcgaagacgcggg

SEQ ID NO: 40016 - DNA, 28 bp, synthetic construct
  source 1..28: mol_type = other DNA
cggtcagcaacggcgaagacgcgggcgg

SEQ ID NO: 40017 - DNA, 28 bp, synthetic construct
  source 1..28: mol_type = other DNA
tcagcaacggcgaagacgcgggcggcgg

SEQ ID NO: 40018 - DNA, 28 bp, synthetic construct
  source 1..28: mol_type = other DNA
aacggcgaagacgcgggcggcggcgcgg

SEQ ID NO: 40019 - DNA, 28 bp, synthetic construct
  source 1..28: mol_type = other DNA
acggcgaagacgcgggcggcggcgcggg

SEQ ID NO: 40020 - DNA, 28 bp, synthetic construct
  source 1..28: mol_type = other DNA
cgaagacgcgggcggcggcgcgggcagg

SEQ ID NO: 40021 - DNA, 28 bp, synthetic construct
  source 1..28: mol_type = other DNA
gaagacgcgggcggcggcgcgggcaggg

SEQ ID NO: 40022 - DNA, 28 bp, synthetic construct
  source 1..28: mol_type = other DNA
gcgggcggcggcgcgggcagggagctgg

SEQ ID NO: 40023 - DNA, 28 bp, synthetic construct
  source 1..28: mol_type = other DNA
ggcggcggcgcgggcagggagctggtgg

SEQ ID NO: 40024 - DNA, 28 bp, synthetic construct
  source 1..28: mol_type = other DNA
ggagctggtggacttgaagatcatctgg

SEQ ID NO: 40025 - DNA, 28 bp, synthetic construct
  source 1..28: mol_type = other DNA
accaagcatgacgtgaagttccccctgg

SEQ ID NO: 40026 - DNA, 28 bp, synthetic construct
  source 1..28: mol_type = other DNA
tccagggggaacttcacgtcatgcttgg

SEQ ID NO: 40027 - DNA, 28 bp, synthetic construct
  source 1..28: mol_type = other DNA
acgtgaagttccccctggacagcacagg

SEQ ID NO: 40028 - DNA, 28 bp, synthetic construct
  source 1..28: mol_type = other DNA
cagctcggagcctgtgctgtccaggggg

SEQ ID NO: 40029 - DNA, 28 bp, synthetic construct
  source 1..28: mol_type = other DNA
tcagctcggagcctgtgctgtccagggg

SEQ ID NO: 40030 - DNA, 28 bp, synthetic construct
  source 1..28: mol_type = other DNA
ttcagctcggagcctgtgctgtccaggg

SEQ ID NO: 40031 - DNA, 28 bp, synthetic construct
  source 1..28: mol_type = other DNA
tttcagctcggagcctgtgctgtccagg

SEQ ID NO: 40032 - DNA, 28 bp, synthetic construct
  source 1..28: mol_type = other DNA
atcgagtggatcttctgtttcagctcgg

SEQ ID NO: 40033 - DNA, 28 bp, synthetic construct
  source 1..28: mol_type = other DNA
tgaaacagaagatccactcgattacagg

SEQ ID NO: 40034 - DNA, 28 bp, synthetic construct
  source 1..28: mol_type = other DNA
tccactcgattacaggtaattcctgtgg

SEQ ID NO: 40035 - DNA, 28 bp, synthetic construct
  source 1..28: mol_type = other DNA
gccacaggaattacctgtaatcgagtgg

SEQ ID NO: 40036 - DNA, 28 bp, synthetic construct
  source 1..28: mol_type = other DNA
ggggaagactggctgtcagcgccacagg

SEQ ID NO: 40037 - DNA, 28 bp, synthetic construct
  source 1..28: mol_type = other DNA
catcaggaggcggggtggggaagactgg

SEQ ID NO: 40038 - DNA, 28 bp, synthetic construct
  source 1..28: mol_type = other DNA
cagtcttccccaccccgcctcctgatgg

SEQ ID NO: 40039 - DNA, 28 bp, synthetic construct
  source 1..28: mol_type = other DNA
gcaagggccatcaggaggcggggtgggg

SEQ ID NO: 40040 - DNA, 28 bp, synthetic construct
  source 1..28: mol_type = other DNA
tgcaagggccatcaggaggcggggtggg

SEQ ID NO: 40041 - DNA, 28 bp, synthetic construct
  source 1..28: mol_type = other DNA
gtgcaagggccatcaggaggcggggtgg

SEQ ID NO: 40042 - DNA, 28 bp, synthetic construct
  source 1..28: mol_type = other DNA
agggtgcaagggccatcaggaggcgggg

SEQ ID NO: 40043 - DNA, 28 bp, synthetic construct
  source 1..28: mol_type = other DNA
tagggtgcaagggccatcaggaggcggg

SEQ ID NO: 40044 - DNA, 28 bp, synthetic construct
  source 1..28: mol_type = other DNA
gtagggtgcaagggccatcaggaggcgg

SEQ ID NO: 40045 - DNA, 28 bp, synthetic construct
  source 1..28: mol_type = other DNA
ctagtagggtgcaagggccatcaggagg

SEQ ID NO: 40046 - DNA, 28 bp, synthetic construct
  source 1..28: mol_type = other DNA
ctcctgatggcccttgcaccctactagg

SEQ ID NO: 40047 - DNA, 28 bp, synthetic construct
  source 1..28: mol_type = other DNA
tgcctagtagggtgcaagggccatcagg

SEQ ID NO: 40048 - DNA, 28 bp, synthetic construct
  source 1..28: mol_type = other DNA
tggcccttgcaccctactaggcacctgg

SEQ ID NO: 40049 - DNA, 28 bp, synthetic construct
  source 1..28: mol_type = other DNA
cccttgcaccctactaggcacctggtgg

SEQ ID NO: 40050 - DNA, 28 bp, synthetic construct
  source 1..28: mol_type = other DNA
gccaccaggtgcctagtagggtgcaagg

SEQ ID NO: 40051 - DNA, 28 bp, synthetic construct
  source 1..28: mol_type = other DNA
aaggaaagccaccaggtgcctagtaggg

SEQ ID NO: 40052 - DNA, 28 bp, synthetic construct
  source 1..28: mol_type = other DNA
caaggaaagccaccaggtgcctagtagg

SEQ ID NO: 40053 - DNA, 28 bp, synthetic construct
  source 1..28: mol_type = other DNA
ggcacctggtggctttccttgcatcagg

SEQ ID NO: 40054 - DNA, 28 bp, synthetic construct
  source 1..28: mol_type = other DNA
gggacctgatgcaaggaaagccaccagg

SEQ ID NO: 40055 - DNA, 28 bp, synthetic construct
  source 1..28: mol_type = other DNA
tgtaaggatggggggacctgatgcaagg

SEQ ID NO: 40056 - DNA, 28 bp, synthetic construct
  source 1..28: mol_type = other DNA
ttcagaagactgctgtaaggatgggggg

SEQ ID NO: 40057 - DNA, 28 bp, synthetic construct
  source 1..28: mol_type = other DNA
cttcagaagactgctgtaaggatggggg

SEQ ID NO: 40058 - DNA, 28 bp, synthetic construct
  source 1..28: mol_type = other DNA
ccccatccttacagcagtcttctgaagg

SEQ ID NO: 40059 - DNA, 28 bp, synthetic construct
  source 1..28: mol_type = other DNA
tccttcagaagactgctgtaaggatggg

SEQ ID NO: 40060 - DNA, 28 bp, synthetic construct
  source 1..28: mol_type = other DNA
ggtggtggaggcagtattcactttttgg

SEQ ID NO: 40061 - DNA, 28 bp, synthetic construct
  source 1..28: mol_type = other DNA
aatgtatggatactacacagctctttgg

SEQ ID NO: 40062 - DNA, 28 bp, synthetic construct
  source 1..28: mol_type = other DNA
aaggaaggaaggacagaaaaatgtatgg

SEQ ID NO: 40063 - DNA, 28 bp, synthetic construct
  source 1..28: mol_type = other DNA
agaaggtggacagtgaaaggaaggaagg

SEQ ID NO: 40064 - DNA, 28 bp, synthetic construct
  source 1..28: mol_type = other DNA
aggtagaaggtggacagtgaaaggaagg

SEQ ID NO: 40065 - DNA, 28 bp, synthetic construct
  source 1..28: mol_type = other DNA
gaaaaggtagaaggtggacagtgaaagg

SEQ ID NO: 40066 - DNA, 28 bp, synthetic construct
  source 1..28: mol_type = other DNA
actgtccaccttctaccttttcccaagg

SEQ ID NO: 40067 - DNA, 28 bp, synthetic construct
  source 1..28: mol_type = other DNA
ggagaccttgggaaaaggtagaaggtgg

SEQ ID NO: 40068 - DNA, 28 bp, synthetic construct
  source 1..28: mol_type = other DNA
gcgggagaccttgggaaaaggtagaagg

SEQ ID NO: 40069 - DNA, 28 bp, synthetic construct
  source 1..28: mol_type = other DNA
atggcaggcgggagaccttgggaaaagg

SEQ ID NO: 40070 - DNA, 28 bp, synthetic construct
  source 1..28: mol_type = other DNA
ttctgcatggcaggcgggagaccttggg

SEQ ID NO: 40071 - DNA, 28 bp, synthetic construct
  source 1..28: mol_type = other DNA
tttctgcatggcaggcgggagaccttgg

SEQ ID NO: 40072 - DNA, 28 bp, synthetic construct
  source 1..28: mol_type = other DNA
atacatgactttctgcatggcaggcggg

SEQ ID NO: 40073 - DNA, 28 bp, synthetic construct
  source 1..28: mol_type = other DNA
tatacatgactttctgcatggcaggcgg

SEQ ID NO: 40074 - DNA, 28 bp, synthetic construct
  source 1..28: mol_type = other DNA
cctgccatgcagaaagtcatgtataagg

SEQ ID NO: 40075 - DNA, 28 bp, synthetic construct
  source 1..28: mol_type = other DNA
ctgccatgcagaaagtcatgtataaggg

SEQ ID NO: 40076 - DNA, 28 bp, synthetic construct
  source 1..28: mol_type = other DNA
agtcccttatacatgactttctgcatgg

SEQ ID NO: 40077 - DNA, 28 bp, synthetic construct
  source 1..28: mol_type = other DNA
gtcatgtataagggactcgtccccgagg

SEQ ID NO: 40078 - DNA, 28 bp, synthetic construct
  source 1..28: mol_type = other DNA
tatttctctcaatgttttatcctcgggg

SEQ ID NO: 40079 - DNA, 28 bp, synthetic construct
  source 1..28: mol_type = other DNA
ttatttctctcaatgttttatcctcggg

SEQ ID NO: 40080 - DNA, 28 bp, synthetic construct
  source 1..28: mol_type = other DNA
tttatttctctcaatgttttatcctcgg

SEQ ID NO: 40081 - DNA, 28 bp, synthetic construct
  source 1..28: mol_type = other DNA
cattgagagaaataaaagtgaccagtgg

SEQ ID NO: 40082 - DNA, 28 bp, synthetic construct
  source 1..28: mol_type = other DNA
attgagagaaataaaagtgaccagtggg

SEQ ID NO: 40083 - DNA, 28 bp, synthetic construct
  source 1..28: mol_type = other DNA
ttgagagaaataaaagtgaccagtgggg

SEQ ID NO: 40084 - DNA, 28 bp, synthetic construct
  source 1..28: mol_type = other DNA
aaagtgaccagtggggccaagatcatgg

SEQ ID NO: 40085 - DNA, 28 bp, synthetic construct
  source 1..28: mol_type = other DNA
gtgaccagtggggccaagatcatggtgg

SEQ ID NO: 40086 - DNA, 28 bp, synthetic construct
  source 1..28: mol_type = other DNA
ccagtggggccaagatcatggtggttgg

SEQ ID NO: 40087 - DNA, 28 bp, synthetic construct
  source 1..28: mol_type = other DNA
atggtggagccaaccaccatgatcttgg

SEQ ID NO: 40088 - DNA, 28 bp, synthetic construct
  source 1..28: mol_type = other DNA
tttactgctaaaacatcattgatggtgg

SEQ ID NO: 40089 - DNA, 28 bp, synthetic construct
  source 1..28: mol_type = other DNA
gtgtttactgctaaaacatcattgatgg

SEQ ID NO: 40090 - DNA, 28 bp, synthetic construct
  source 1..28: mol_type = other DNA
aacacacccaaagatgctgcgcagcagg

SEQ ID NO: 40091 - DNA, 28 bp, synthetic construct
  source 1..28: mol_type = other DNA
ttgcatcctgctgcgcagcatctttggg

SEQ ID NO: 40092 - DNA, 28 bp, synthetic construct
  source 1..28: mol_type = other DNA
tttgcatcctgctgcgcagcatctttgg

SEQ ID NO: 40093 - DNA, 28 bp, synthetic construct
  source 1..28: mol_type = other DNA
aaagatgctgcgcagcaggatgcaaagg

SEQ ID NO: 40094 - DNA, 28 bp, synthetic construct
  source 1..28: mol_type = other DNA
gatgcaaaggccgaagagaacaagaagg

SEQ ID NO: 40095 - DNA, 28 bp, synthetic construct
  source 1..28: mol_type = other DNA
cagagaggctccttcttgttctcttcgg

SEQ ID NO: 40096 - DNA, 28 bp, synthetic construct
  source 1..28: mol_type = other DNA
agagaacaagaaggagcctctctgcagg

SEQ ID NO: 40097 - DNA, 28 bp, synthetic construct
  source 1..28: mol_type = other DNA
atggactcactttctgcctgcagagagg

SEQ ID NO: 40098 - DNA, 28 bp, synthetic construct
  source 1..28: mol_type = other DNA
gaaagtgagtccatcttgtgcttcttgg

SEQ ID NO: 40099 - DNA, 28 bp, synthetic construct
  source 1..28: mol_type = other DNA
tttctcaagaccaagaagcacaagatgg

SEQ ID NO: 40100 - DNA, 28 bp, synthetic construct
  source 1..28: mol_type = other DNA
gtgcttcttggtcttgagaaatttgagg

SEQ ID NO: 40101 - DNA, 28 bp, synthetic construct
  source 1..28: mol_type = other DNA
tttgaggctttgtcctcttgagccgtgg

SEQ ID NO: 40102 - DNA, 28 bp, synthetic construct
  source 1..28: mol_type = other DNA
aggctttgtcctcttgagccgtggctgg

SEQ ID NO: 40103 - DNA, 28 bp, synthetic construct
  source 1..28: mol_type = other DNA
agaatataaccagccacggctcaagagg

SEQ ID NO: 40104 - DNA, 28 bp, synthetic construct
  source 1..28: mol_type = other DNA
attctagggagaatataaccagccacgg

SEQ ID NO: 40105 - DNA, 28 bp, synthetic construct
  source 1..28: mol_type = other DNA
attctccctagaataagctcctttttgg

SEQ ID NO: 40106 - DNA, 28 bp, synthetic construct
  source 1..28: mol_type = other DNA
ccctagaataagctcctttttggacagg

SEQ ID NO: 40107 - DNA, 28 bp, synthetic construct
  source 1..28: mol_type = other DNA
cctagaataagctcctttttggacaggg

SEQ ID NO: 40108 - DNA, 28 bp, synthetic construct
  source 1..28: mol_type = other DNA
gctcctttttggacagggcccatgatgg

SEQ ID NO: 40109 - DNA, 28 bp, synthetic construct
  source 1..28: mol_type = other DNA
tttccatcatgggccctgtccaaaaagg

SEQ ID NO: 40110 - DNA, 28 bp, synthetic construct
  source 1..28: mol_type = other DNA
ggacagggcccatgatggaaatttatgg

SEQ ID NO: 40111 - DNA, 28 bp, synthetic construct
  source 1..28: mol_type = other DNA
aactgctgccataaatttccatcatggg

SEQ ID NO: 40112 - DNA, 28 bp, synthetic construct
  source 1..28: mol_type = other DNA
caactgctgccataaatttccatcatgg

SEQ ID NO: 40113 - DNA, 28 bp, synthetic construct
  source 1..28: mol_type = other DNA
catgatggaaatttatggcagcagttgg

SEQ ID NO: 40114 - DNA, 28 bp, synthetic construct
  source 1..28: mol_type = other DNA
atgatggaaatttatggcagcagttggg

SEQ ID NO: 40115 - DNA, 28 bp, synthetic construct
  source 1..28: mol_type = other DNA
atggcagcagttgggtgccgcagagtgg

SEQ ID NO: 40116 - DNA, 28 bp, synthetic construct
  source 1..28: mol_type = other DNA
gcagcagttgggtgccgcagagtggagg

SEQ ID NO: 40117 - DNA, 28 bp, synthetic construct
  source 1..28: mol_type = other DNA
tcaggtagttgtcacctccactctgcgg

SEQ ID NO: 40118 - DNA, 28 bp, synthetic construct
  source 1..28: mol_type = other DNA
cagatgagacaaagttgcaaatctcagg

SEQ ID NO: 40119 - DNA, 28 bp, synthetic construct
  source 1..28: mol_type = other DNA
ctgagatttgcaactttgtctcatctgg

SEQ ID NO: 40120 - DNA, 28 bp, synthetic construct
  source 1..28: mol_type = other DNA
agatttgcaactttgtctcatctggcgg

SEQ ID NO: 40121 - DNA, 28 bp, synthetic construct
  source 1..28: mol_type = other DNA
gatttgcaactttgtctcatctggcggg

SEQ ID NO: 40122 - DNA, 28 bp, synthetic construct
  source 1..28: mol_type = other DNA
agtgtgtctcaagtctacctactttagg

SEQ ID NO: 40123 - DNA, 28 bp, synthetic construct
  source 1..28: mol_type = other DNA
gtctacctactttaggataagaccttgg

SEQ ID NO: 40124 - DNA, 28 bp, synthetic construct
  source 1..28: mol_type = other DNA
ctttaccaaggtcttatcctaaagtagg

SEQ ID NO: 40125 - DNA, 28 bp, synthetic construct
  source 1..28: mol_type = other DNA
ctactttaggataagaccttggtaaagg

SEQ ID NO: 40126 - DNA, 28 bp, synthetic construct
  source 1..28: mol_type = other DNA
tactttaggataagaccttggtaaaggg

SEQ ID NO: 40127 - DNA, 28 bp, synthetic construct
  source 1..28: mol_type = other DNA
tttaggataagaccttggtaaagggagg

SEQ ID NO: 40128 - DNA, 28 bp, synthetic construct
  source 1..28: mol_type = other DNA
catggtctgaagcctccctttaccaagg

SEQ ID NO: 40129 - DNA, 28 bp, synthetic construct
  source 1..28: mol_type = other DNA
gggaggcttcagaccatgtgttgaaagg

SEQ ID NO: 40130 - DNA, 28 bp, synthetic construct
  source 1..28: mol_type = other DNA
accatgtgttgaaaggaatcagacgtgg

SEQ ID NO: 40131 - DNA, 28 bp, synthetic construct
  source 1..28: mol_type = other DNA
ccatgtgttgaaaggaatcagacgtggg

SEQ ID NO: 40132 - DNA, 28 bp, synthetic construct
  source 1..28: mol_type = other DNA
taaaagcttttgagccaaaacactaagg

SEQ ID NO: 40133 - DNA, 28 bp, synthetic construct
  source 1..28: mol_type = other DNA
gaggatgaagaaagccttagtgttttgg

SEQ ID NO: 40134 - DNA, 28 bp, synthetic construct
  source 1..28: mol_type = other DNA
aaggctttcttcatcctctctttcaagg

SEQ ID NO: 40135 - DNA, 28 bp, synthetic construct
  source 1..28: mol_type = other DNA
aggctttcttcatcctctctttcaaggg

SEQ ID NO: 40136 - DNA, 28 bp, synthetic construct
  source 1..28: mol_type = other DNA
tcgtgttactattcccttgaaagagagg

SEQ ID NO: 40137 - DNA, 28 bp, synthetic construct
  source 1..28: mol_type = other DNA
tctctcttctgacttatagcaacacagg

SEQ ID NO: 40138 - DNA, 28 bp, synthetic construct
  source 1..28: mol_type = other DNA
gacttatagcaacacaggaaagtgttgg

SEQ ID NO: 40139 - DNA, 28 bp, synthetic construct
  source 1..28: mol_type = other DNA
agcaacacaggaaagtgttggataaagg

SEQ ID NO: 40140 - DNA, 28 bp, synthetic construct
  source 1..28: mol_type = other DNA
ccttaacagatggcatcacatcttcagg

SEQ ID NO: 40141 - DNA, 28 bp, synthetic construct
  source 1..28: mol_type = other DNA
ctgaagatgtgatgccatctgttaaggg

SEQ ID NO: 40142 - DNA, 28 bp, synthetic construct
  source 1..28: mol_type = other DNA
tgaagatgtgatgccatctgttaagggg

SEQ ID NO: 40143 - DNA, 28 bp, synthetic construct
  source 1..28: mol_type = other DNA
gaagatgtgatgccatctgttaaggggg

SEQ ID NO: 40144 - DNA, 28 bp, synthetic construct
  source 1..28: mol_type = other DNA
gtgatgccatctgttaagggggcccagg

SEQ ID NO: 40145 - DNA, 28 bp, synthetic construct
  source 1..28: mol_type = other DNA
gccatctgttaagggggcccaggtaagg

SEQ ID NO: 40146 - DNA, 28 bp, synthetic construct
  source 1..28: mol_type = other DNA
gccttacctgggcccccttaacagatgg

SEQ ID NO: 40147 - DNA, 28 bp, synthetic construct
  source 1..28: mol_type = other DNA
atctgttaagggggcccaggtaaggcgg

SEQ ID NO: 40148 - DNA, 28 bp, synthetic construct
  source 1..28: mol_type = other DNA
gctcacaaagaaatccgccttacctggg

SEQ ID NO: 40149 - DNA, 28 bp, synthetic construct
  source 1..28: mol_type = other DNA
tgctcacaaagaaatccgccttacctgg

SEQ ID NO: 40150 - DNA, 28 bp, synthetic construct
  source 1..28: mol_type = other DNA
tttctttgtgagcattctgaaaatgagg

SEQ ID NO: 40151 - DNA, 28 bp, synthetic construct
  source 1..28: mol_type = other DNA
tgaggcagccccaccgtctgacttgagg

SEQ ID NO: 40152 - DNA, 28 bp, synthetic construct
  source 1..28: mol_type = other DNA
tggaggaacctcaagtcagacggtgggg

SEQ ID NO: 40153 - DNA, 28 bp, synthetic construct
  source 1..28: mol_type = other DNA
ttggaggaacctcaagtcagacggtggg

SEQ ID NO: 40154 - DNA, 28 bp, synthetic construct
  source 1..28: mol_type = other DNA
attggaggaacctcaagtcagacggtgg

SEQ ID NO: 40155 - DNA, 28 bp, synthetic construct
  source 1..28: mol_type = other DNA
aggattggaggaacctcaagtcagacgg

SEQ ID NO: 40156 - DNA, 28 bp, synthetic construct
  source 1..28: mol_type = other DNA
gaaaaaagagaagggacaggattggagg

SEQ ID NO: 40157 - DNA, 28 bp, synthetic construct
  source 1..28: mol_type = other DNA
agggaaaaaagagaagggacaggattgg

SEQ ID NO: 40158 - DNA, 28 bp, synthetic construct
  source 1..28: mol_type = other DNA
aaaacagggaaaaaagagaagggacagg

SEQ ID NO: 40159 - DNA, 28 bp, synthetic construct
  source 1..28: mol_type = other DNA
aaaaaaaaacagggaaaaaagagaaggg

SEQ ID NO: 40160 - DNA, 28 bp, synthetic construct
  source 1..28: mol_type = other DNA
aaaaaaaaaacagggaaaaaagagaagg

SEQ ID NO: 40161 - DNA, 28 bp, synthetic construct
  source 1..28: mol_type = other DNA
actctgtctcaaaaaaaaaaaaacaggg

SEQ ID NO: 40162 - DNA, 28 bp, synthetic construct
  source 1..28: mol_type = other DNA
gactctgtctcaaaaaaaaaaaaacagg

SEQ ID NO: 40163 - DNA, 28 bp, synthetic construct
  source 1..28: mol_type = other DNA
gaggccaaagcggtcagatcacctgagg

SEQ ID NO: 40164 - DNA, 28 bp, synthetic construct
  source 1..28: mol_type = other DNA
tgaccgctttggcctcccagtgtgctgg

SEQ ID NO: 40165 - DNA, 28 bp, synthetic construct
  source 1..28: mol_type = other DNA
gaccgctttggcctcccagtgtgctggg

SEQ ID NO: 40166 - DNA, 28 bp, synthetic construct
  source 1..28: mol_type = other DNA
atcccagcacactgggaggccaaagcgg

SEQ ID NO: 40167 - DNA, 28 bp, synthetic construct
  source 1..28: mol_type = other DNA
tggcctcccagtgtgctgggattacagg

SEQ ID NO: 40168 - DNA, 28 bp, synthetic construct
  source 1..28: mol_type = other DNA
acgcctgtaatcccagcacactgggagg

SEQ ID NO: 40169 - DNA, 28 bp, synthetic construct
  source 1..28: mol_type = other DNA
ctcacgcctgtaatcccagcacactggg

SEQ ID NO: 40170 - DNA, 28 bp, synthetic construct
  source 1..28: mol_type = other DNA
gctcacgcctgtaatcccagcacactgg

SEQ ID NO: 40171 - DNA, 28 bp, synthetic construct
  source 1..28: mol_type = other DNA
gattacaggcgtgagccaccgcgcttgg

SEQ ID NO: 40172 - DNA, 28 bp, synthetic construct
  source 1..28: mol_type = other DNA
aaaaagagaagggggccaagcgcggtgg

SEQ ID NO: 40173 - DNA, 28 bp, synthetic construct
  source 1..28: mol_type = other DNA
gaaaaaaagagaagggggccaagcgcgg

SEQ ID NO: 40174 - DNA, 28 bp, synthetic construct
  source 1..28: mol_type = other DNA
gggacagtcagaaaaaaagagaaggggg

SEQ ID NO: 40175 - DNA, 28 bp, synthetic construct
  source 1..28: mol_type = other DNA
agggacagtcagaaaaaaagagaagggg

SEQ ID NO: 40176 - DNA, 28 bp, synthetic construct
  source 1..28: mol_type = other DNA
gagggacagtcagaaaaaaagagaaggg

SEQ ID NO: 40177 - DNA, 28 bp, synthetic construct
  source 1..28: mol_type = other DNA
ggagggacagtcagaaaaaaagagaagg

SEQ ID NO: 40178 - DNA, 28 bp, synthetic construct
  source 1..28: mol_type = other DNA
gcacgagagaatggtaagagatggaggg

SEQ ID NO: 40179 - DNA, 28 bp, synthetic construct
  source 1..28: mol_type = other DNA
ggcacgagagaatggtaagagatggagg

SEQ ID NO: 40180 - DNA, 28 bp, synthetic construct
  source 1..28: mol_type = other DNA
gaaggcacgagagaatggtaagagatgg

SEQ ID NO: 40181 - DNA, 28 bp, synthetic construct
  source 1..28: mol_type = other DNA
tctcttaccattctctcgtgccttcagg

SEQ ID NO: 40182 - DNA, 28 bp, synthetic construct
  source 1..28: mol_type = other DNA
aggcgctcctgaaggcacgagagaatgg

SEQ ID NO: 40183 - DNA, 28 bp, synthetic construct
  source 1..28: mol_type = other DNA
tcgtgccttcaggagcgcctgccaacgg

SEQ ID NO: 40184 - DNA, 28 bp, synthetic construct
  source 1..28: mol_type = other DNA
cggtaccgttggcaggcgctcctgaagg

SEQ ID NO: 40185 - DNA, 28 bp, synthetic construct
  source 1..28: mol_type = other DNA
agcgcctgccaacggtaccgctgtccgg

SEQ ID NO: 40186 - DNA, 28 bp, synthetic construct
  source 1..28: mol_type = other DNA
catgccggacagcggtaccgttggcagg

SEQ ID NO: 40187 - DNA, 28 bp, synthetic construct
  source 1..28: mol_type = other DNA
tgtacatgccggacagcggtaccgttgg

SEQ ID NO: 40188 - DNA, 28 bp, synthetic construct
  source 1..28: mol_type = other DNA
cagatttattgtacatgccggacagcgg

SEQ ID NO: 40189 - DNA, 28 bp, synthetic construct
  source 1..28: mol_type = other DNA
cgctgtccggcatgtacaataaatctgg

SEQ ID NO: 40190 - DNA, 28 bp, synthetic construct
  source 1..28: mol_type = other DNA
tgtccggcatgtacaataaatctggagg

SEQ ID NO: 40191 - DNA, 28 bp, synthetic construct
  source 1..28: mol_type = other DNA
tttcctccagatttattgtacatgccgg

SEQ ID NO: 40192 - DNA, 28 bp, synthetic construct
  source 1..28: mol_type = other DNA
cacagctggtcttgttctagtttaaagg

SEQ ID NO: 40193 - DNA, 28 bp, synthetic construct
  source 1..28: mol_type = other DNA
ctttaaactagaacaagaccagctgtgg

SEQ ID NO: 40194 - DNA, 28 bp, synthetic construct
  source 1..28: mol_type = other DNA
aactagaacaagaccagctgtggattgg

SEQ ID NO: 40195 - DNA, 28 bp, synthetic construct
  source 1..28: mol_type = other DNA
aagaccagctgtggattggcactaaagg

SEQ ID NO: 40196 - DNA, 28 bp, synthetic construct
  source 1..28: mol_type = other DNA
catacctttagtgccaatccacagctgg

SEQ ID NO: 40197 - DNA, 28 bp, synthetic construct
  source 1..28: mol_type = other DNA
ggtatgttcttcctcgcctccttgctgg

SEQ ID NO: 40198 - DNA, 28 bp, synthetic construct
  source 1..28: mol_type = other DNA
caggcagtgggccagcaaggaggcgagg

SEQ ID NO: 40199 - DNA, 28 bp, synthetic construct
  source 1..28: mol_type = other DNA
agaggcaggcagtgggccagcaaggagg

SEQ ID NO: 40200 - DNA, 28 bp, synthetic construct
  source 1..28: mol_type = other DNA
tccttgctggcccactgcctgcctctgg

SEQ ID NO: 40201 - DNA, 28 bp, synthetic construct
  source 1..28: mol_type = other DNA
gccagaggcaggcagtgggccagcaagg

SEQ ID NO: 40202 - DNA, 28 bp, synthetic construct
  source 1..28: mol_type = other DNA
ctgctgggtgccagaggcaggcagtggg

SEQ ID NO: 40203 - DNA, 28 bp, synthetic construct
  source 1..28: mol_type = other DNA
gctgctgggtgccagaggcaggcagtgg

SEQ ID NO: 40204 - DNA, 28 bp, synthetic construct
  source 1..28: mol_type = other DNA
gtgagtgctgctgggtgccagaggcagg

SEQ ID NO: 40205 - DNA, 28 bp, synthetic construct
  source 1..28: mol_type = other DNA
aaatgtgagtgctgctgggtgccagagg

SEQ ID NO: 40206 - DNA, 28 bp, synthetic construct
  source 1..28: mol_type = other DNA
cgcactctaaaatgtgagtgctgctggg

SEQ ID NO: 40207 - DNA, 28 bp, synthetic construct
  source 1..28: mol_type = other DNA
tcgcactctaaaatgtgagtgctgctgg

SEQ ID NO: 40208 - DNA, 28 bp, synthetic construct
  source 1..28: mol_type = other DNA
gtggagagagaggtttcagaaggagggg

SEQ ID NO: 40209 - DNA, 28 bp, synthetic construct
  source 1..28: mol_type = other DNA
agtggagagagaggtttcagaaggaggg

SEQ ID NO: 40210 - DNA, 28 bp, synthetic construct
  source 1..28: mol_type = other DNA
cagtggagagagaggtttcagaaggagg

SEQ ID NO: 40211 - DNA, 28 bp, synthetic construct
  source 1..28: mol_type = other DNA
gcacagtggagagagaggtttcagaagg

SEQ ID NO: 40212 - DNA, 28 bp, synthetic construct
  source 1..28: mol_type = other DNA
agcaagcaaagcacagtggagagagagg

SEQ ID NO: 40213 - DNA, 28 bp, synthetic construct
  source 1..28: mol_type = other DNA
tggagggtggggggagaatcaaggaagg

SEQ ID NO: 40214 - DNA, 28 bp, synthetic construct
  source 1..28: mol_type = other DNA
catttggagggtggggggagaatcaagg

SEQ ID NO: 40215 - DNA, 28 bp, synthetic construct
  source 1..28: mol_type = other DNA
ggcagcaagtcatttggagggtgggggg

SEQ ID NO: 40216 - DNA, 28 bp, synthetic construct
  source 1..28: mol_type = other DNA
cggcagcaagtcatttggagggtggggg

SEQ ID NO: 40217 - DNA, 28 bp, synthetic construct
  source 1..28: mol_type = other DNA
gcggcagcaagtcatttggagggtgggg

SEQ ID NO: 40218 - DNA, 28 bp, synthetic construct
  source 1..28: mol_type = other DNA
agcggcagcaagtcatttggagggtggg

SEQ ID NO: 40219 - DNA, 28 bp, synthetic construct
  source 1..28: mol_type = other DNA
aagcggcagcaagtcatttggagggtgg

SEQ ID NO: 40220 - DNA, 28 bp, synthetic construct
  source 1..28: mol_type = other DNA
cagaagcggcagcaagtcatttggaggg

SEQ ID NO: 40221 - DNA, 28 bp, synthetic construct
  source 1..28: mol_type = other DNA
acagaagcggcagcaagtcatttggagg

SEQ ID NO: 40222 - DNA, 28 bp, synthetic construct
  source 1..28: mol_type = other DNA
tgaacagaagcggcagcaagtcatttgg

SEQ ID NO: 40223 - DNA, 28 bp, synthetic construct
  source 1..28: mol_type = other DNA
aaacgaagcgctctatgaacagaagcgg

SEQ ID NO: 40224 - DNA, 28 bp, synthetic construct
  source 1..28: mol_type = other DNA
aagtcagagagtaatgagtgctctgggg

SEQ ID NO: 40225 - DNA, 28 bp, synthetic construct
  source 1..28: mol_type = other DNA
caagtcagagagtaatgagtgctctggg

SEQ ID NO: 40226 - DNA, 28 bp, synthetic construct
  source 1..28: mol_type = other DNA
acaagtcagagagtaatgagtgctctgg

SEQ ID NO: 40227 - DNA, 28 bp, synthetic construct
  source 1..28: mol_type = other DNA
cttgtctgtccccctgttagattcctgg

SEQ ID NO: 40228 - DNA, 28 bp, synthetic construct
  source 1..28: mol_type = other DNA
gtctgtccccctgttagattcctggagg

SEQ ID NO: 40229 - DNA, 28 bp, synthetic construct
  source 1..28: mol_type = other DNA
tctgtccccctgttagattcctggaggg

SEQ ID NO: 40230 - DNA, 28 bp, synthetic construct
  source 1..28: mol_type = other DNA
cggttccctccaggaatctaacaggggg

SEQ ID NO: 40231 - DNA, 28 bp, synthetic construct
  source 1..28: mol_type = other DNA
tcggttccctccaggaatctaacagggg

SEQ ID NO: 40232 - DNA, 28 bp, synthetic construct
  source 1..28: mol_type = other DNA
ttcggttccctccaggaatctaacaggg

SEQ ID NO: 40233 - DNA, 28 bp, synthetic construct
  source 1..28: mol_type = other DNA
gttcggttccctccaggaatctaacagg

SEQ ID NO: 40234 - DNA, 28 bp, synthetic construct
  source 1..28: mol_type = other DNA
gatttaggcatgttcggttccctccagg

SEQ ID NO: 40235 - DNA, 28 bp, synthetic construct
  source 1..28: mol_type = other DNA
cagaaacaggtgatttaggcatgttcgg

SEQ ID NO: 40236 - DNA, 28 bp, synthetic construct
  source 1..28: mol_type = other DNA
agtgctggtcagaaacaggtgatttagg

SEQ ID NO: 40237 - DNA, 28 bp, synthetic construct
  source 1..28: mol_type = other DNA
atcacctgtttctgaccagcactgtagg

SEQ ID NO: 40238 - DNA, 28 bp, synthetic construct
  source 1..28: mol_type = other DNA
aatacctacagtgctggtcagaaacagg

SEQ ID NO: 40239 - DNA, 28 bp, synthetic construct
  source 1..28: mol_type = other DNA
ctcgaacactgaatacctacagtgctgg

SEQ ID NO: 40240 - DNA, 28 bp, synthetic construct
  source 1..28: mol_type = other DNA
cagcactgtaggtattcagtgttcgagg

SEQ ID NO: 40241 - DNA, 28 bp, synthetic construct
  source 1..28: mol_type = other DNA
cgaggtaaatgctaaagagaagtatagg

SEQ ID NO: 40242 - DNA, 28 bp, synthetic construct
  source 1..28: mol_type = other DNA
gaggtaaatgctaaagagaagtataggg

SEQ ID NO: 40243 - DNA, 28 bp, synthetic construct
  source 1..28: mol_type = other DNA
aggtaaatgctaaagagaagtatagggg

SEQ ID NO: 40244 - DNA, 28 bp, synthetic construct
  source 1..28: mol_type = other DNA
ggtaaatgctaaagagaagtataggggg

SEQ ID NO: 40245 - DNA, 28 bp, synthetic construct
  source 1..28: mol_type = other DNA
gggggtcccatcatctgacgttcactgg

SEQ ID NO: 40246 - DNA, 28 bp, synthetic construct
  source 1..28: mol_type = other DNA
ctgaaaccagtgaacgtcagatgatggg

SEQ ID NO: 40247 - DNA, 28 bp, synthetic construct
  source 1..28: mol_type = other DNA
cctgaaaccagtgaacgtcagatgatgg

SEQ ID NO: 40248 - DNA, 28 bp, synthetic construct
  source 1..28: mol_type = other DNA
catcatctgacgttcactggtttcaggg

SEQ ID NO: 40249 - DNA, 28 bp, synthetic construct
  source 1..28: mol_type = other DNA
ccatttagtgagactccacttaaaatgg

SEQ ID NO: 40250 - DNA, 28 bp, synthetic construct
  source 1..28: mol_type = other DNA
catttagtgagactccacttaaaatggg

SEQ ID NO: 40251 - DNA, 28 bp, synthetic construct
  source 1..28: mol_type = other DNA
ccacttaaaatgggaccaagttttatgg

SEQ ID NO: 40252 - DNA, 28 bp, synthetic construct
  source 1..28: mol_type = other DNA
gggaccaagttttatggagaataattgg

SEQ ID NO: 40253 - DNA, 28 bp, synthetic construct
  source 1..28: mol_type = other DNA
ggaccaagttttatggagaataattggg

SEQ ID NO: 40254 - DNA, 28 bp, synthetic construct
  source 1..28: mol_type = other DNA
gaccaagttttatggagaataattgggg

SEQ ID NO: 40255 - DNA, 28 bp, synthetic construct
  source 1..28: mol_type = other DNA
tgccccaattattctccataaaacttgg

SEQ ID NO: 40256 - DNA, 28 bp, synthetic construct
  source 1..28: mol_type = other DNA
aagttttatggagaataattggggcagg

SEQ ID NO: 40257 - DNA, 28 bp, synthetic construct
  source 1..28: mol_type = other DNA
agttttatggagaataattggggcaggg

SEQ ID NO: 40258 - DNA, 28 bp, synthetic construct
  source 1..28: mol_type = other DNA
gttttatggagaataattggggcagggg

SEQ ID NO: 40259 - DNA, 28 bp, synthetic construct
  source 1..28: mol_type = other DNA
ctgagggttccccccagtttttgcaagg

SEQ ID NO: 40260 - DNA, 28 bp, synthetic construct
  source 1..28: mol_type = other DNA
tgagggttccccccagtttttgcaaggg

SEQ ID NO: 40261 - DNA, 28 bp, synthetic construct
  source 1..28: mol_type = other DNA
ttcaaaggcccttgcaaaaactgggggg

SEQ ID NO: 40262 - DNA, 28 bp, synthetic construct
  source 1..28: mol_type = other DNA
gttcaaaggcccttgcaaaaactggggg

SEQ ID NO: 40263 - DNA, 28 bp, synthetic construct
  source 1..28: mol_type = other DNA
ggttcaaaggcccttgcaaaaactgggg

SEQ ID NO: 40264 - DNA, 28 bp, synthetic construct
  source 1..28: mol_type = other DNA
gggttcaaaggcccttgcaaaaactggg

SEQ ID NO: 40265 - DNA, 28 bp, synthetic construct
  source 1..28: mol_type = other DNA
agggttcaaaggcccttgcaaaaactgg

SEQ ID NO: 40266 - DNA, 28 bp, synthetic construct
  source 1..28: mol_type = other DNA
gagaatgatctagcagagggttcaaagg

SEQ ID NO: 40267 - DNA, 28 bp, synthetic construct
  source 1..28: mol_type = other DNA
ctacagaagagaatgatctagcagaggg

SEQ ID NO: 40268 - DNA, 28 bp, synthetic construct
  source 1..28: mol_type = other DNA
tctacagaagagaatgatctagcagagg

SEQ ID NO: 40269 - DNA, 28 bp, synthetic construct
  source 1..28: mol_type = other DNA
tactactgataaagggaagatggacagg

SEQ ID NO: 40270 - DNA, 28 bp, synthetic construct
  source 1..28: mol_type = other DNA
cagcttactactgataaagggaagatgg

SEQ ID NO: 40271 - DNA, 28 bp, synthetic construct
  source 1..28: mol_type = other DNA
ggctgggcagcttactactgataaaggg

SEQ ID NO: 40272 - DNA, 28 bp, synthetic construct
  source 1..28: mol_type = other DNA
aggctgggcagcttactactgataaagg

SEQ ID NO: 40273 - DNA, 28 bp, synthetic construct
  source 1..28: mol_type = other DNA
gctgcccagcctctgtcaactttgcagg

SEQ ID NO: 40274 - DNA, 28 bp, synthetic construct
  source 1..28: mol_type = other DNA
atcacctgcaaagttgacagaggctggg

SEQ ID NO: 40275 - DNA, 28 bp, synthetic construct
  source 1..28: mol_type = other DNA
aatcacctgcaaagttgacagaggctgg

SEQ ID NO: 40276 - DNA, 28 bp, synthetic construct
  source 1..28: mol_type = other DNA
gcaaaatcacctgcaaagttgacagagg

SEQ ID NO: 40277 - DNA, 28 bp, synthetic construct
  source 1..28: mol_type = other DNA
agtgcatagacttcctgcctcttgctgg

SEQ ID NO: 40278 - DNA, 28 bp, synthetic construct
  source 1..28: mol_type = other DNA
caaaagtagaggtccagcaagaggcagg

SEQ ID NO: 40279 - DNA, 28 bp, synthetic construct
  source 1..28: mol_type = other DNA
caagcaaaagtagaggtccagcaagagg

SEQ ID NO: 40280 - DNA, 28 bp, synthetic construct
  source 1..28: mol_type = other DNA
cttgctggacctctacttttgcttgtgg

SEQ ID NO: 40281 - DNA, 28 bp, synthetic construct
  source 1..28: mol_type = other DNA
ttgctggacctctacttttgcttgtggg

SEQ ID NO: 40282 - DNA, 28 bp, synthetic construct
  source 1..28: mol_type = other DNA
tgaggctgcccacaagcaaaagtagagg

SEQ ID NO: 40283 - DNA, 28 bp, synthetic construct
  source 1..28: mol_type = other DNA
ttttgcttgtgggcagcctcattgaagg

SEQ ID NO: 40284 - DNA, 28 bp, synthetic construct
  source 1..28: mol_type = other DNA
gcagcctcattgaaggcagttgctacgg

SEQ ID NO: 40285 - DNA, 28 bp, synthetic construct
  source 1..28: mol_type = other DNA
tcagccgtagcaactgccttcaatgagg

SEQ ID NO: 40286 - DNA, 28 bp, synthetic construct
  source 1..28: mol_type = other DNA
ttgaaggcagttgctacggctgacctgg

SEQ ID NO: 40287 - DNA, 28 bp, synthetic construct
  source 1..28: mol_type = other DNA
cctatcttcatggcagggtctttccagg

SEQ ID NO: 40288 - DNA, 28 bp, synthetic construct
  source 1..28: mol_type = other DNA
aagaccctgccatgaagataggtgcagg

SEQ ID NO: 40289 - DNA, 28 bp, synthetic construct
  source 1..28: mol_type = other DNA
tctgcctgcacctatcttcatggcaggg

SEQ ID NO: 40290 - DNA, 28 bp, synthetic construct
  source 1..28: mol_type = other DNA
ctctgcctgcacctatcttcatggcagg

SEQ ID NO: 40291 - DNA, 28 bp, synthetic construct
  source 1..28: mol_type = other DNA
acttctctgcctgcacctatcttcatgg

SEQ ID NO: 40292 - DNA, 28 bp, synthetic construct
  source 1..28: mol_type = other DNA
gaagataggtgcaggcagagaagtctgg

SEQ ID NO: 40293 - DNA, 28 bp, synthetic construct
  source 1..28: mol_type = other DNA
ataggtgcaggcagagaagtctggatgg

SEQ ID NO: 40294 - DNA, 28 bp, synthetic construct
  source 1..28: mol_type = other DNA
taggtgcaggcagagaagtctggatggg

SEQ ID NO: 40295 - DNA, 28 bp, synthetic construct
  source 1..28: mol_type = other DNA
gggaactaagtctgtaagtgctcattgg

SEQ ID NO: 40296 - DNA, 28 bp, synthetic construct
  source 1..28: mol_type = other DNA
agtctgtaagtgctcattggttccttgg

SEQ ID NO: 40297 - DNA, 28 bp, synthetic construct
  source 1..28: mol_type = other DNA
gtctgtaagtgctcattggttccttggg

SEQ ID NO: 40298 - DNA, 28 bp, synthetic construct
  source 1..28: mol_type = other DNA
tctgtaagtgctcattggttccttgggg

SEQ ID NO: 40299 - DNA, 28 bp, synthetic construct
  source 1..28: mol_type = other DNA
gttccttggggaatatttctgtgtcagg

SEQ ID NO: 40300 - DNA, 28 bp, synthetic construct
  source 1..28: mol_type = other DNA
cttcctgacacagaaatattccccaagg

SEQ ID NO: 40301 - DNA, 28 bp, synthetic construct
  source 1..28: mol_type = other DNA
atatttctgtgtcaggaagttgtatagg

SEQ ID NO: 40302 - DNA, 28 bp, synthetic construct
  source 1..28: mol_type = other DNA
tatttctgtgtcaggaagttgtataggg

SEQ ID NO: 40303 - DNA, 28 bp, synthetic construct
  source 1..28: mol_type = other DNA
tgtatagggaacacatcataactgcagg

SEQ ID NO: 40304 - DNA, 28 bp, synthetic construct
  source 1..28: mol_type = other DNA
gaacaagaacttcctgaccctgtattgg

SEQ ID NO: 40305 - DNA, 28 bp, synthetic construct
  source 1..28: mol_type = other DNA
aaaagaaaacttccaatacagggtcagg

SEQ ID NO: 40306 - DNA, 28 bp, synthetic construct
  source 1..28: mol_type = other DNA
tagcaaaaagaaaacttccaatacaggg

SEQ ID NO: 40307 - DNA, 28 bp, synthetic construct
  source 1..28: mol_type = other DNA
ctagcaaaaagaaaacttccaatacagg

SEQ ID NO: 40308 - DNA, 28 bp, synthetic construct
  source 1..28: mol_type = other DNA
tattggaagttttctttttgctagtagg

SEQ ID NO: 40309 - DNA, 28 bp, synthetic construct
  source 1..28: mol_type = other DNA
agtaggagcagccgccttcctgctttgg

SEQ ID NO: 40310 - DNA, 28 bp, synthetic construct
  source 1..28: mol_type = other DNA
cagccgccttcctgctttggcctaaagg

SEQ ID NO: 40311 - DNA, 28 bp, synthetic construct
  source 1..28: mol_type = other DNA
agccgccttcctgctttggcctaaaggg

SEQ ID NO: 40312 - DNA, 28 bp, synthetic construct
  source 1..28: mol_type = other DNA
ctccctttaggccaaagcaggaaggcgg

SEQ ID NO: 40313 - DNA, 28 bp, synthetic construct
  source 1..28: mol_type = other DNA
gctctccctttaggccaaagcaggaagg

SEQ ID NO: 40314 - DNA, 28 bp, synthetic construct
  source 1..28: mol_type = other DNA
tacagctctccctttaggccaaagcagg

SEQ ID NO: 40315 - DNA, 28 bp, synthetic construct
  source 1..28: mol_type = other DNA
gagcttcttctacagctctccctttagg

SEQ ID NO: 40316 - DNA, 28 bp, synthetic construct
  source 1..28: mol_type = other DNA
gagctgtagaagaagctcaatatgttgg

SEQ ID NO: 40317 - DNA, 28 bp, synthetic construct
  source 1..28: mol_type = other DNA
agctgtagaagaagctcaatatgttggg

SEQ ID NO: 40318 - DNA, 28 bp, synthetic construct
  source 1..28: mol_type = other DNA
gctgtagaagaagctcaatatgttgggg

SEQ ID NO: 40319 - DNA, 28 bp, synthetic construct
  source 1..28: mol_type = other DNA
gactggtgagtaaggaggctttcaaggg

SEQ ID NO: 40320 - DNA, 28 bp, synthetic construct
  source 1..28: mol_type = other DNA
agactggtgagtaaggaggctttcaagg

SEQ ID NO: 40321 - DNA, 28 bp, synthetic construct
  source 1..28: mol_type = other DNA
gcctccttactcaccagtcttgttgagg

SEQ ID NO: 40322 - DNA, 28 bp, synthetic construct
  source 1..28: mol_type = other DNA
tcctcaacaagactggtgagtaaggagg

SEQ ID NO: 40323 - DNA, 28 bp, synthetic construct
  source 1..28: mol_type = other DNA
tgctcctcaacaagactggtgagtaagg

SEQ ID NO: 40324 - DNA, 28 bp, synthetic construct
  source 1..28: mol_type = other DNA
tactcaccagtcttgttgaggagcatgg

SEQ ID NO: 40325 - DNA, 28 bp, synthetic construct
  source 1..28: mol_type = other DNA
ccatggccatgctcctcaacaagactgg

SEQ ID NO: 40326 - DNA, 28 bp, synthetic construct
  source 1..28: mol_type = other DNA
tggccatggactactcatgttttctagg

SEQ ID NO: 40327 - DNA, 28 bp, synthetic construct
  source 1..28: mol_type = other DNA
ggccatggactactcatgttttctaggg

SEQ ID NO: 40328 - DNA, 28 bp, synthetic construct
  source 1..28: mol_type = other DNA
aaccctagaaaacatgagtagtccatgg

SEQ ID NO: 40329 - DNA, 28 bp, synthetic construct
  source 1..28: mol_type = other DNA
tactcatgttttctagggttgaacaagg

SEQ ID NO: 40330 - DNA, 28 bp, synthetic construct
  source 1..28: mol_type = other DNA
attcccacccatagcactgtacctctgg

SEQ ID NO: 40331 - DNA, 28 bp, synthetic construct
  source 1..28: mol_type = other DNA
gctccagaggtacagtgctatgggtggg

SEQ ID NO: 40332 - DNA, 28 bp, synthetic construct
  source 1..28: mol_type = other DNA
ggctccagaggtacagtgctatgggtgg

SEQ ID NO: 40333 - DNA, 28 bp, synthetic construct
  source 1..28: mol_type = other DNA
ttgggctccagaggtacagtgctatggg

SEQ ID NO: 40334 - DNA, 28 bp, synthetic construct
  source 1..28: mol_type = other DNA
cttgggctccagaggtacagtgctatgg

SEQ ID NO: 40335 - DNA, 28 bp, synthetic construct
  source 1..28: mol_type = other DNA
catagcactgtacctctggagcccaagg

SEQ ID NO: 40336 - DNA, 28 bp, synthetic construct
  source 1..28: mol_type = other DNA
atagcactgtacctctggagcccaaggg

SEQ ID NO: 40337 - DNA, 28 bp, synthetic construct
  source 1..28: mol_type = other DNA
tagcactgtacctctggagcccaagggg

SEQ ID NO: 40338 - DNA, 28 bp, synthetic construct
  source 1..28: mol_type = other DNA
actgtacctctggagcccaaggggcagg

SEQ ID NO: 40339 - DNA, 28 bp, synthetic construct
  source 1..28: mol_type = other DNA
agactgcctgccccttgggctccagagg

SEQ ID NO: 40340 - DNA, 28 bp, synthetic construct
  source 1..28: mol_type = other DNA
caagtgacaagactgcctgccccttggg

SEQ ID NO: 40341 - DNA, 28 bp, synthetic construct
  source 1..28: mol_type = other DNA
gcaagtgacaagactgcctgccccttgg

SEQ ID NO: 40342 - DNA, 28 bp, synthetic construct
  source 1..28: mol_type = other DNA
cttatgacacttaggtaacaggactggg

SEQ ID NO: 40343 - DNA, 28 bp, synthetic construct
  source 1..28: mol_type = other DNA
gcttatgacacttaggtaacaggactgg

SEQ ID NO: 40344 - DNA, 28 bp, synthetic construct
  source 1..28: mol_type = other DNA
tgagtgcttatgacacttaggtaacagg

SEQ ID NO: 40345 - DNA, 28 bp, synthetic construct
  source 1..28: mol_type = other DNA
cctcttatgagtgcttatgacacttagg

SEQ ID NO: 40346 - DNA, 28 bp, synthetic construct
  source 1..28: mol_type = other DNA
gcactcataagaggacagcttgttctgg

SEQ ID NO: 40347 - DNA, 28 bp, synthetic construct
  source 1..28: mol_type = other DNA
cactcataagaggacagcttgttctggg

SEQ ID NO: 40348 - DNA, 28 bp, synthetic construct
  source 1..28: mol_type = other DNA
taagaggacagcttgttctgggagttgg

SEQ ID NO: 40349 - DNA, 28 bp, synthetic construct
  source 1..28: mol_type = other DNA
gttctgggagttggctgctagccactgg

SEQ ID NO: 40350 - DNA, 28 bp, synthetic construct
  source 1..28: mol_type = other DNA
ctagccactggcttcgtctttctgctgg

SEQ ID NO: 40351 - DNA, 28 bp, synthetic construct
  source 1..28: mol_type = other DNA
cttgccagcagaaagacgaagccagtgg

SEQ ID NO: 40352 - DNA, 28 bp, synthetic construct
  source 1..28: mol_type = other DNA
tcgtctttctgctggcaagaagaagcgg

SEQ ID NO: 40353 - DNA, 28 bp, synthetic construct
  source 1..28: mol_type = other DNA
ttctgctggcaagaagaagcggctatgg

SEQ ID NO: 40354 - DNA, 28 bp, synthetic construct
  source 1..28: mol_type = other DNA
tggaatgaccatcccagcagcgagttgg

SEQ ID NO: 40355 - DNA, 28 bp, synthetic construct
  source 1..28: mol_type = other DNA
cgaagaggccaactcgctgctgggatgg

SEQ ID NO: 40356 - DNA, 28 bp, synthetic construct
  source 1..28: mol_type = other DNA
tcccagcagcgagttggcctcttcgtgg

SEQ ID NO: 40357 - DNA, 28 bp, synthetic construct
  source 1..28: mol_type = other DNA
cccacgaagaggccaactcgctgctggg

SEQ ID NO: 40358 - DNA, 28 bp, synthetic construct
  source 1..28: mol_type = other DNA
ccagcagcgagttggcctcttcgtgggg

SEQ ID NO: 40359 - DNA, 28 bp, synthetic construct
  source 1..28: mol_type = other DNA
ttactcagcaaagcgccccacgaagagg

SEQ ID NO: 40360 - DNA, 28 bp, synthetic construct
  source 1..28: mol_type = other DNA
cgctttgctgagtaagtgacccttaagg

SEQ ID NO: 40361 - DNA, 28 bp, synthetic construct
  source 1..28: mol_type = other DNA
gctttgctgagtaagtgacccttaaggg

SEQ ID NO: 40362 - DNA, 28 bp, synthetic construct
  source 1..28: mol_type = other DNA
tttagtcaagagtagcagcccttaaggg

SEQ ID NO: 40363 - DNA, 28 bp, synthetic construct
  source 1..28: mol_type = other DNA
gtttagtcaagagtagcagcccttaagg

SEQ ID NO: 40364 - DNA, 28 bp, synthetic construct
  source 1..28: mol_type = other DNA
ttgactaaactctgctagcttgtgtagg

SEQ ID NO: 40365 - DNA, 28 bp, synthetic construct
  source 1..28: mol_type = other DNA
actaaactctgctagcttgtgtaggagg

SEQ ID NO: 40366 - DNA, 28 bp, synthetic construct
  source 1..28: mol_type = other DNA
aaactctgctagcttgtgtaggaggagg

SEQ ID NO: 40367 - DNA, 28 bp, synthetic construct
  source 1..28: mol_type = other DNA
cctggagcttgttctcattcttttgagg

SEQ ID NO: 40368 - DNA, 28 bp, synthetic construct
  source 1..28: mol_type = other DNA
aaaagaatgagaacaagctccaggcagg

SEQ ID NO: 40369 - DNA, 28 bp, synthetic construct
  source 1..28: mol_type = other DNA
tgagaacaagctccaggcaggaaaccgg

SEQ ID NO: 40370 - DNA, 28 bp, synthetic construct
  source 1..28: mol_type = other DNA
ctccaggcaggaaaccggaagccgctgg

SEQ ID NO: 40371 - DNA, 28 bp, synthetic construct
  source 1..28: mol_type = other DNA
ctccagcggcttccggtttcctgcctgg

SEQ ID NO: 40372 - DNA, 28 bp, synthetic construct
  source 1..28: mol_type = other DNA
caggcaggaaaccggaagccgctggagg

SEQ ID NO: 40373 - DNA, 28 bp, synthetic construct
  source 1..28: mol_type = other DNA
gtacatgctctcctccagcggcttccgg

SEQ ID NO: 40374 - DNA, 28 bp, synthetic construct
  source 1..28: mol_type = other DNA
gagcagggtacatgctctcctccagcgg

SEQ ID NO: 40375 - DNA, 28 bp, synthetic construct
  source 1..28: mol_type = other DNA
ggaggagagcatgtaccctgctcgtagg

SEQ ID NO: 40376 - DNA, 28 bp, synthetic construct
  source 1..28: mol_type = other DNA
accctgctcgtaggaaagttgaatctgg

SEQ ID NO: 40377 - DNA, 28 bp, synthetic construct
  source 1..28: mol_type = other DNA
gccagattcaactttcctacgagcaggg

SEQ ID NO: 40378 - DNA, 28 bp, synthetic construct
  source 1..28: mol_type = other DNA
agccagattcaactttcctacgagcagg

SEQ ID NO: 40379 - DNA, 28 bp, synthetic construct
  source 1..28: mol_type = other DNA
tcgtaggaaagttgaatctggctgaagg

SEQ ID NO: 40380 - DNA, 28 bp, synthetic construct
  source 1..28: mol_type = other DNA
tggctgaaggtctgatgtagtgatcagg

SEQ ID NO: 40381 - DNA, 28 bp, synthetic construct
  source 1..28: mol_type = other DNA
aggtctgatgtagtgatcaggagtgtgg

SEQ ID NO: 40382 - DNA, 28 bp, synthetic construct
  source 1..28: mol_type = other DNA
ggtctgatgtagtgatcaggagtgtggg

SEQ ID NO: 40383 - DNA, 28 bp, synthetic construct
  source 1..28: mol_type = other DNA
tgtgggtccagaattgcccaatttttgg

SEQ ID NO: 40384 - DNA, 28 bp, synthetic construct
  source 1..28: mol_type = other DNA
gaaaactccaaaaattgggcaattctgg

SEQ ID NO: 40385 - DNA, 28 bp, synthetic construct
  source 1..28: mol_type = other DNA
gcttctcttgaaaactccaaaaattggg

SEQ ID NO: 40386 - DNA, 28 bp, synthetic construct
  source 1..28: mol_type = other DNA
ggcttctcttgaaaactccaaaaattgg

SEQ ID NO: 40387 - DNA, 28 bp, synthetic construct
  source 1..28: mol_type = other DNA
ttcacaaaaatatacaacagatttctgg

SEQ ID NO: 40388 - DNA, 28 bp, synthetic construct
  source 1..28: mol_type = other DNA
tttttgtgaaatctccagacatttcagg

SEQ ID NO: 40389 - DNA, 28 bp, synthetic construct
  source 1..28: mol_type = other DNA
aaatctccagacatttcaggatgaaagg

SEQ ID NO: 40390 - DNA, 28 bp, synthetic construct
  source 1..28: mol_type = other DNA
aaaacacctttcatcctgaaatgtctgg

SEQ ID NO: 40391 - DNA, 28 bp, synthetic construct
  source 1..28: mol_type = other DNA
tccatcttaaagacagctgctgcccagg

SEQ ID NO: 40392 - DNA, 28 bp, synthetic construct
  source 1..28: mol_type = other DNA
acctgggcagcagctgtctttaagatgg

SEQ ID NO: 40393 - DNA, 28 bp, synthetic construct
  source 1..28: mol_type = other DNA
acagctgctgcccaggtcctgctttagg

SEQ ID NO: 40394 - DNA, 28 bp, synthetic construct
  source 1..28: mol_type = other DNA
cagctgctgcccaggtcctgctttaggg

SEQ ID NO: 40395 - DNA, 28 bp, synthetic construct
  source 1..28: mol_type = other DNA
aacagtcggccctaaagcaggacctggg

SEQ ID NO: 40396 - DNA, 28 bp, synthetic construct
  source 1..28: mol_type = other DNA
caacagtcggccctaaagcaggacctgg

SEQ ID NO: 40397 - DNA, 28 bp, synthetic construct
  source 1..28: mol_type = other DNA
gctctacaacagtcggccctaaagcagg

SEQ ID NO: 40398 - DNA, 28 bp, synthetic construct
  source 1..28: mol_type = other DNA
ggacttctagtggctctacaacagtcgg

SEQ ID NO: 40399 - DNA, 28 bp, synthetic construct
  source 1..28: mol_type = other DNA
tgtttatttaggtttggacttctagtgg

SEQ ID NO: 40400 - DNA, 28 bp, synthetic construct
  source 1..28: mol_type = other DNA
agtccaaacctaaataaacatcttcagg

SEQ ID NO: 40401 - DNA, 28 bp, synthetic construct
  source 1..28: mol_type = other DNA
ggacctgaagatgtttatttaggtttgg

SEQ ID NO: 40402 - DNA, 28 bp, synthetic construct
  source 1..28: mol_type = other DNA
agaagggacctgaagatgtttatttagg

SEQ ID NO: 40403 - DNA, 28 bp, synthetic construct
  source 1..28: mol_type = other DNA
tctgaaaaatgggggctggggagaaggg

SEQ ID NO: 40404 - DNA, 28 bp, synthetic construct
  source 1..28: mol_type = other DNA
atctgaaaaatgggggctggggagaagg

SEQ ID NO: 40405 - DNA, 28 bp, synthetic construct
  source 1..28: mol_type = other DNA
ctcagtatctgaaaaatgggggctgggg

SEQ ID NO: 40406 - DNA, 28 bp, synthetic construct
  source 1..28: mol_type = other DNA
cccagcccccatttttcagatactgagg

SEQ ID NO: 40407 - DNA, 28 bp, synthetic construct
  source 1..28: mol_type = other DNA
gcctcagtatctgaaaaatgggggctgg

SEQ ID NO: 40408 - DNA, 28 bp, synthetic construct
  source 1..28: mol_type = other DNA
gtgggcctcagtatctgaaaaatggggg

SEQ ID NO: 40409 - DNA, 28 bp, synthetic construct
  source 1..28: mol_type = other DNA
tgtgggcctcagtatctgaaaaatgggg

SEQ ID NO: 40410 - DNA, 28 bp, synthetic construct
  source 1..28: mol_type = other DNA
ctgtgggcctcagtatctgaaaaatggg

SEQ ID NO: 40411 - DNA, 28 bp, synthetic construct
  source 1..28: mol_type = other DNA
tctgtgggcctcagtatctgaaaaatgg

SEQ ID NO: 40412 - DNA, 28 bp, synthetic construct
  source 1..28: mol_type = other DNA
ttaagacattttacttcagttctgtggg

SEQ ID NO: 40413 - DNA, 28 bp, synthetic construct
  source 1..28: mol_type = other DNA
cttaagacattttacttcagttctgtgg

SEQ ID NO: 40414 - DNA, 28 bp, synthetic construct
  source 1..28: mol_type = other DNA
taagtccccagctagaccagaacgctgg

SEQ ID NO: 40415 - DNA, 28 bp, synthetic construct
  source 1..28: mol_type = other DNA
agagaccagcgttctggtctagctgggg

SEQ ID NO: 40416 - DNA, 28 bp, synthetic construct
  source 1..28: mol_type = other DNA
tagagaccagcgttctggtctagctggg

SEQ ID NO: 40417 - DNA, 28 bp, synthetic construct
  source 1..28: mol_type = other DNA
ttagagaccagcgttctggtctagctgg

SEQ ID NO: 40418 - DNA, 28 bp, synthetic construct
  source 1..28: mol_type = other DNA
actaggaatttagagaccagcgttctgg

SEQ ID NO: 40419 - DNA, 28 bp, synthetic construct
  source 1..28: mol_type = other DNA
ctggtctctaaattcctagtctgtttgg

SEQ ID NO: 40420 - DNA, 28 bp, synthetic construct
  source 1..28: mol_type = other DNA
aatagataagttggccaaacagactagg

SEQ ID NO: 40421 - DNA, 28 bp, synthetic construct
  source 1..28: mol_type = other DNA
agatagagtctaaaaatagataagttgg

SEQ ID NO: 40422 - DNA, 28 bp, synthetic construct
  source 1..28: mol_type = other DNA
tctttccagatttttctttctgcaaagg

SEQ ID NO: 40423 - DNA, 28 bp, synthetic construct
  source 1..28: mol_type = other DNA
tgcagcctttgcagaaagaaaaatctgg

SEQ ID NO: 40424 - DNA, 28 bp, synthetic construct
  source 1..28: mol_type = other DNA
caaaggctgcaagtttttttccacttgg

SEQ ID NO: 40425 - DNA, 28 bp, synthetic construct
  source 1..28: mol_type = other DNA
aggctcagcaaacagctaaaccaagtgg

SEQ ID NO: 40426 - DNA, 28 bp, synthetic construct
  source 1..28: mol_type = other DNA
ggggcgcagggggaggggggcagggagg

SEQ ID NO: 40427 - DNA, 28 bp, synthetic construct
  source 1..28: mol_type = other DNA
acgggggcgcagggggaggggggcaggg

SEQ ID NO: 40428 - DNA, 28 bp, synthetic construct
  source 1..28: mol_type = other DNA
gacgggggcgcagggggaggggggcagg

SEQ ID NO: 40429 - DNA, 28 bp, synthetic construct
  source 1..28: mol_type = other DNA
cagggacgggggcgcagggggagggggg

SEQ ID NO: 40430 - DNA, 28 bp, synthetic construct
  source 1..28: mol_type = other DNA
tcagggacgggggcgcagggggaggggg

SEQ ID NO: 40431 - DNA, 28 bp, synthetic construct
  source 1..28: mol_type = other DNA
ctcagggacgggggcgcagggggagggg

SEQ ID NO: 40432 - DNA, 28 bp, synthetic construct
  source 1..28: mol_type = other DNA
cctcagggacgggggcgcagggggaggg

SEQ ID NO: 40433 - DNA, 28 bp, synthetic construct
  source 1..28: mol_type = other DNA
acctcagggacgggggcgcagggggagg

SEQ ID NO: 40434 - DNA, 28 bp, synthetic construct
  source 1..28: mol_type = other DNA
gacacctcagggacgggggcgcaggggg

SEQ ID NO: 40435 - DNA, 28 bp, synthetic construct
  source 1..28: mol_type = other DNA
agacacctcagggacgggggcgcagggg

SEQ ID NO: 40436 - DNA, 28 bp, synthetic construct
  source 1..28: mol_type = other DNA
cagacacctcagggacgggggcgcaggg

SEQ ID NO: 40437 - DNA, 28 bp, synthetic construct
  source 1..28: mol_type = other DNA
gcagacacctcagggacgggggcgcagg

SEQ ID NO: 40438 - DNA, 28 bp, synthetic construct
  source 1..28: mol_type = other DNA
ggagcagcagacacctcagggacggggg

SEQ ID NO: 40439 - DNA, 28 bp, synthetic construct
  source 1..28: mol_type = other DNA
tggagcagcagacacctcagggacgggg

SEQ ID NO: 40440 - DNA, 28 bp, synthetic construct
  source 1..28: mol_type = other DNA
ctggagcagcagacacctcagggacggg

SEQ ID NO: 40441 - DNA, 28 bp, synthetic construct
  source 1..28: mol_type = other DNA
cctggagcagcagacacctcagggacgg

SEQ ID NO: 40442 - DNA, 28 bp, synthetic construct
  source 1..28: mol_type = other DNA
ccatcctggagcagcagacacctcaggg

SEQ ID NO: 40443 - DNA, 28 bp, synthetic construct
  source 1..28: mol_type = other DNA
gccatcctggagcagcagacacctcagg

SEQ ID NO: 40444 - DNA, 28 bp, synthetic construct
  source 1..28: mol_type = other DNA
ccaggatggccatgtccccttgtgcagg

SEQ ID NO: 40445 - DNA, 28 bp, synthetic construct
  source 1..28: mol_type = other DNA
cgaggtgcacctgcacaaggggacatgg

SEQ ID NO: 40446 - DNA, 28 bp, synthetic construct
  source 1..28: mol_type = other DNA
gggaggcgaggtgcacctgcacaagggg

SEQ ID NO: 40447 - DNA, 28 bp, synthetic construct
  source 1..28: mol_type = other DNA
ggggaggcgaggtgcacctgcacaaggg

SEQ ID NO: 40448 - DNA, 28 bp, synthetic construct
  source 1..28: mol_type = other DNA
aggggaggcgaggtgcacctgcacaagg

SEQ ID NO: 40449 - DNA, 28 bp, synthetic construct
  source 1..28: mol_type = other DNA
ggactgggtgaggtcaggggaggcgagg

SEQ ID NO: 40450 - DNA, 28 bp, synthetic construct
  source 1..28: mol_type = other DNA
aagcgggactgggtgaggtcaggggagg

SEQ ID NO: 40451 - DNA, 28 bp, synthetic construct
  source 1..28: mol_type = other DNA
gtgaagcgggactgggtgaggtcagggg

SEQ ID NO: 40452 - DNA, 28 bp, synthetic construct
  source 1..28: mol_type = other DNA
agtgaagcgggactgggtgaggtcaggg

SEQ ID NO: 40453 - DNA, 28 bp, synthetic construct
  source 1..28: mol_type = other DNA
aagtgaagcgggactgggtgaggtcagg

SEQ ID NO: 40454 - DNA, 28 bp, synthetic construct
  source 1..28: mol_type = other DNA
tgacctcacccagtcccgcttcacttgg

SEQ ID NO: 40455 - DNA, 28 bp, synthetic construct
  source 1..28: mol_type = other DNA
gagccaagtgaagcgggactgggtgagg

SEQ ID NO: 40456 - DNA, 28 bp, synthetic construct
  source 1..28: mol_type = other DNA
ggagtgagccaagtgaagcgggactggg

SEQ ID NO: 40457 - DNA, 28 bp, synthetic construct
  source 1..28: mol_type = other DNA
gggagtgagccaagtgaagcgggactgg

SEQ ID NO: 40458 - DNA, 28 bp, synthetic construct
  source 1..28: mol_type = other DNA
agtcccgcttcacttggctcactcccgg

SEQ ID NO: 40459 - DNA, 28 bp, synthetic construct
  source 1..28: mol_type = other DNA
ctgccgggagtgagccaagtgaagcggg

SEQ ID NO: 40460 - DNA, 28 bp, synthetic construct
  source 1..28: mol_type = other DNA
actgccgggagtgagccaagtgaagcgg

SEQ ID NO: 40461 - DNA, 28 bp, synthetic construct
  source 1..28: mol_type = other DNA
actcccggcagtctcatctcactccagg

SEQ ID NO: 40462 - DNA, 28 bp, synthetic construct
  source 1..28: mol_type = other DNA
atgcctggagtgagatgagactgccggg

SEQ ID NO: 40463 - DNA, 28 bp, synthetic construct
  source 1..28: mol_type = other DNA
gatgcctggagtgagatgagactgccgg

SEQ ID NO: 40464 - DNA, 28 bp, synthetic construct
  source 1..28: mol_type = other DNA
agagaagggggcagcaagggatgcctgg

SEQ ID NO: 40465 - DNA, 28 bp, synthetic construct
  source 1..28: mol_type = other DNA
ggcaggtaagagaagggggcagcaaggg

SEQ ID NO: 40466 - DNA, 28 bp, synthetic construct
  source 1..28: mol_type = other DNA
tggcaggtaagagaagggggcagcaagg

SEQ ID NO: 40467 - DNA, 28 bp, synthetic construct
  source 1..28: mol_type = other DNA
aaggaggatggcaggtaagagaaggggg

SEQ ID NO: 40468 - DNA, 28 bp, synthetic construct
  source 1..28: mol_type = other DNA
taaggaggatggcaggtaagagaagggg

SEQ ID NO: 40469 - DNA, 28 bp, synthetic construct
  source 1..28: mol_type = other DNA
ttaaggaggatggcaggtaagagaaggg

SEQ ID NO: 40470 - DNA, 28 bp, synthetic construct
  source 1..28: mol_type = other DNA
tttaaggaggatggcaggtaagagaagg

SEQ ID NO: 40471 - DNA, 28 bp, synthetic construct
  source 1..28: mol_type = other DNA
ttgaggcgagtttaaggaggatggcagg

SEQ ID NO: 40472 - DNA, 28 bp, synthetic construct
  source 1..28: mol_type = other DNA
gacattgaggcgagtttaaggaggatgg

SEQ ID NO: 40473 - DNA, 28 bp, synthetic construct
  source 1..28: mol_type = other DNA
agaagacattgaggcgagtttaaggagg

SEQ ID NO: 40474 - DNA, 28 bp, synthetic construct
  source 1..28: mol_type = other DNA
gtcagaagacattgaggcgagtttaagg

SEQ ID NO: 40475 - DNA, 28 bp, synthetic construct
  source 1..28: mol_type = other DNA
gatcacatggggtcagaagacattgagg

SEQ ID NO: 40476 - DNA, 28 bp, synthetic construct
  source 1..28: mol_type = other DNA
atgtcttctgaccccatgtgatcagtgg

SEQ ID NO: 40477 - DNA, 28 bp, synthetic construct
  source 1..28: mol_type = other DNA
cacttgagataccactgatcacatgggg

SEQ ID NO: 40478 - DNA, 28 bp, synthetic construct
  source 1..28: mol_type = other DNA
acacttgagataccactgatcacatggg

SEQ ID NO: 40479 - DNA, 28 bp, synthetic construct
  source 1..28: mol_type = other DNA
aacacttgagataccactgatcacatgg

SEQ ID NO: 40480 - DNA, 28 bp, synthetic construct
  source 1..28: mol_type = other DNA
tggtatctcaagtgttaatcacaaaagg

SEQ ID NO: 40481 - DNA, 28 bp, synthetic construct
  source 1..28: mol_type = other DNA
cataaaagtgtgtgaatatagagtgcgg

SEQ ID NO: 40482 - DNA, 28 bp, synthetic construct
  source 1..28: mol_type = other DNA
aaaagtgtgtgaatatagagtgcggagg

SEQ ID NO: 40483 - DNA, 28 bp, synthetic construct
  source 1..28: mol_type = other DNA
gtgaatatagagtgcggaggactcgagg

SEQ ID NO: 40484 - DNA, 28 bp, synthetic construct
  source 1..28: mol_type = other DNA
aatatagagtgcggaggactcgaggagg

SEQ ID NO: 40485 - DNA, 28 bp, synthetic construct
  source 1..28: mol_type = other DNA
atatagagtgcggaggactcgaggaggg

SEQ ID NO: 40486 - DNA, 28 bp, synthetic construct
  source 1..28: mol_type = other DNA
tagagtgcggaggactcgaggagggagg

SEQ ID NO: 40487 - DNA, 28 bp, synthetic construct
  source 1..28: mol_type = other DNA
gtgcggaggactcgaggagggaggccgg

SEQ ID NO: 40488 - DNA, 28 bp, synthetic construct
  source 1..28: mol_type = other DNA
tgcggaggactcgaggagggaggccggg

SEQ ID NO: 40489 - DNA, 28 bp, synthetic construct
  source 1..28: mol_type = other DNA
gcggaggactcgaggagggaggccgggg

SEQ ID NO: 40490 - DNA, 28 bp, synthetic construct
  source 1..28: mol_type = other DNA
aggactcgaggagggaggccggggaagg

SEQ ID NO: 40491 - DNA, 28 bp, synthetic construct
  source 1..28: mol_type = other DNA
ggactcgaggagggaggccggggaaggg

SEQ ID NO: 40492 - DNA, 28 bp, synthetic construct
  source 1..28: mol_type = other DNA
gaggagggaggccggggaagggagcagg

SEQ ID NO: 40493 - DNA, 28 bp, synthetic construct
  source 1..28: mol_type = other DNA
aggagggaggccggggaagggagcaggg

SEQ ID NO: 40494 - DNA, 28 bp, synthetic construct
  source 1..28: mol_type = other DNA
gaggccggggaagggagcagggtcgtgg

SEQ ID NO: 40495 - DNA, 28 bp, synthetic construct
  source 1..28: mol_type = other DNA
tataccacgaccctgctcccttccccgg

SEQ ID NO: 40496 - DNA, 28 bp, synthetic construct
  source 1..28: mol_type = other DNA
ggtatagaatctagccctaaaatccagg

SEQ ID NO: 40497 - DNA, 28 bp, synthetic construct
  source 1..28: mol_type = other DNA
agggaaggggagtgcctggattttaggg

SEQ ID NO: 40498 - DNA, 28 bp, synthetic construct
  source 1..28: mol_type = other DNA
aagggaaggggagtgcctggattttagg

SEQ ID NO: 40499 - DNA, 28 bp, synthetic construct
  source 1..28: mol_type = other DNA
gctctcacaagggaaggggagtgcctgg

SEQ ID NO: 40500 - DNA, 28 bp, synthetic construct
  source 1..28: mol_type = other DNA
actccccttcccttgtgagagccacagg

SEQ ID NO: 40501 - DNA, 28 bp, synthetic construct
  source 1..28: mol_type = other DNA
ctccccttcccttgtgagagccacaggg

SEQ ID NO: 40502 - DNA, 28 bp, synthetic construct
  source 1..28: mol_type = other DNA
tccccttcccttgtgagagccacagggg

SEQ ID NO: 40503 - DNA, 28 bp, synthetic construct
  source 1..28: mol_type = other DNA
tcccctgtggctctcacaagggaagggg

SEQ ID NO: 40504 - DNA, 28 bp, synthetic construct
  source 1..28: mol_type = other DNA
ttcccctgtggctctcacaagggaaggg

SEQ ID NO: 40505 - DNA, 28 bp, synthetic construct
  source 1..28: mol_type = other DNA
gttcccctgtggctctcacaagggaagg

SEQ ID NO: 40506 - DNA, 28 bp, synthetic construct
  source 1..28: mol_type = other DNA
acacgttcccctgtggctctcacaaggg

SEQ ID NO: 40507 - DNA, 28 bp, synthetic construct
  source 1..28: mol_type = other DNA
aacacgttcccctgtggctctcacaagg

SEQ ID NO: 40508 - DNA, 28 bp, synthetic construct
  source 1..28: mol_type = other DNA
aacaaagaggcaacacgttcccctgtgg

SEQ ID NO: 40509 - DNA, 28 bp, synthetic construct
  source 1..28: mol_type = other DNA
gggaacgtgttgcctctttgttcgtagg

SEQ ID NO: 40510 - DNA, 28 bp, synthetic construct
  source 1..28: mol_type = other DNA
agagtcaagaggcctacgaacaaagagg

SEQ ID NO: 40511 - DNA, 28 bp, synthetic construct
  source 1..28: mol_type = other DNA
gtcttgggcagtagggagagtcaagagg

SEQ ID NO: 40512 - DNA, 28 bp, synthetic construct
  source 1..28: mol_type = other DNA
gcattgactaaggtcttgggcagtaggg

SEQ ID NO: 40513 - DNA, 28 bp, synthetic construct
  source 1..28: mol_type = other DNA
agcattgactaaggtcttgggcagtagg

SEQ ID NO: 40514 - DNA, 28 bp, synthetic construct
  source 1..28: mol_type = other DNA
tactgcccaagaccttagtcaatgctgg

SEQ ID NO: 40515 - DNA, 28 bp, synthetic construct
  source 1..28: mol_type = other DNA
actgcccaagaccttagtcaatgctggg

SEQ ID NO: 40516 - DNA, 28 bp, synthetic construct
  source 1..28: mol_type = other DNA
caagcccagcattgactaaggtcttggg

SEQ ID NO: 40517 - DNA, 28 bp, synthetic construct
  source 1..28: mol_type = other DNA
gcaagcccagcattgactaaggtcttgg

SEQ ID NO: 40518 - DNA, 28 bp, synthetic construct
  source 1..28: mol_type = other DNA
ccttatgcaagcccagcattgactaagg

SEQ ID NO: 40519 - DNA, 28 bp, synthetic construct
  source 1..28: mol_type = other DNA
atgctgggcttgcataaggttacaaagg

SEQ ID NO: 40520 - DNA, 28 bp, synthetic construct
  source 1..28: mol_type = other DNA
tgcataaggttacaaaggaatttcttgg

SEQ ID NO: 40521 - DNA, 28 bp, synthetic construct
  source 1..28: mol_type = other DNA
gcataaggttacaaaggaatttcttggg

SEQ ID NO: 40522 - DNA, 28 bp, synthetic construct
  source 1..28: mol_type = other DNA
tattttatatttttttttgttgagatgg

SEQ ID NO: 40523 - DNA, 28 bp, synthetic construct
  source 1..28: mol_type = other DNA
tttgttgagatggagtttcgctctttgg

SEQ ID NO: 40524 - DNA, 28 bp, synthetic construct
  source 1..28: mol_type = other DNA
gagatggagtttcgctctttggcccagg

SEQ ID NO: 40525 - DNA, 28 bp, synthetic construct
  source 1..28: mol_type = other DNA
ctctttggcccaggctgaagtaaagtgg

SEQ ID NO: 40526 - DNA, 28 bp, synthetic construct
  source 1..28: mol_type = other DNA
agatcatgccactttacttcagcctggg

SEQ ID NO: 40527 - DNA, 28 bp, synthetic construct
  source 1..28: mol_type = other DNA
gagatcatgccactttacttcagcctgg

SEQ ID NO: 40528 - DNA, 28 bp, synthetic construct
  source 1..28: mol_type = other DNA
aggctgaagtaaagtggcatgatctcgg

SEQ ID NO: 40529 - DNA, 28 bp, synthetic construct
  source 1..28: mol_type = other DNA
tcggctcactgcaacttctgccccccgg

SEQ ID NO: 40530 - DNA, 28 bp, synthetic construct
  source 1..28: mol_type = other DNA
cggctcactgcaacttctgccccccggg

SEQ ID NO: 40531 - DNA, 28 bp, synthetic construct
  source 1..28: mol_type = other DNA
agcacgagaatcgcttgaacccgggggg

SEQ ID NO: 40532 - DNA, 28 bp, synthetic construct
  source 1..28: mol_type = other DNA
aagcacgagaatcgcttgaacccggggg

SEQ ID NO: 40533 - DNA, 28 bp, synthetic construct
  source 1..28: mol_type = other DNA
gaagcacgagaatcgcttgaacccgggg

SEQ ID NO: 40534 - DNA, 28 bp, synthetic construct
  source 1..28: mol_type = other DNA
tgaagcacgagaatcgcttgaacccggg

SEQ ID NO: 40535 - DNA, 28 bp, synthetic construct
  source 1..28: mol_type = other DNA
ctgaagcacgagaatcgcttgaacccgg

SEQ ID NO: 40536 - DNA, 28 bp, synthetic construct
  source 1..28: mol_type = other DNA
ctcgtgcttcagcctcctgagtagctgg

SEQ ID NO: 40537 - DNA, 28 bp, synthetic construct
  source 1..28: mol_type = other DNA
tcgtgcttcagcctcctgagtagctggg

SEQ ID NO: 40538 - DNA, 28 bp, synthetic construct
  source 1..28: mol_type = other DNA
cagcctcctgagtagctgggattatagg

SEQ ID NO: 40539 - DNA, 28 bp, synthetic construct
  source 1..28: mol_type = other DNA
gcacctataatcccagctactcaggagg

SEQ ID NO: 40540 - DNA, 28 bp, synthetic construct
  source 1..28: mol_type = other DNA
tgggcacctataatcccagctactcagg

SEQ ID NO: 40541 - DNA, 28 bp, synthetic construct
  source 1..28: mol_type = other DNA
gattataggtgcccaccaccacgcctgg

SEQ ID NO: 40542 - DNA, 28 bp, synthetic construct
  source 1..28: mol_type = other DNA
caaaaaattagccaggcgtggtggtggg

SEQ ID NO: 40543 - DNA, 28 bp, synthetic construct
  source 1..28: mol_type = other DNA
acaaaaaattagccaggcgtggtggtgg

SEQ ID NO: 40544 - DNA, 28 bp, synthetic construct
  source 1..28: mol_type = other DNA
aatacaaaaaattagccaggcgtggtgg

SEQ ID NO: 40545 - DNA, 28 bp, synthetic construct
  source 1..28: mol_type = other DNA
aaaaatacaaaaaattagccaggcgtgg

SEQ ID NO: 40546 - DNA, 28 bp, synthetic construct
  source 1..28: mol_type = other DNA
ctactaaaaatacaaaaaattagccagg

SEQ ID NO: 40547 - DNA, 28 bp, synthetic construct
  source 1..28: mol_type = other DNA
taattttttgtatttttagtagagacgg

SEQ ID NO: 40548 - DNA, 28 bp, synthetic construct
  source 1..28: mol_type = other DNA
aattttttgtatttttagtagagacggg

SEQ ID NO: 40549 - DNA, 28 bp, synthetic construct
  source 1..28: mol_type = other DNA
attttttgtatttttagtagagacgggg

SEQ ID NO: 40550 - DNA, 28 bp, synthetic construct
  source 1..28: mol_type = other DNA
tagtagagacggggtttcaccatgctgg

SEQ ID NO: 40551 - DNA, 28 bp, synthetic construct
  source 1..28: mol_type = other DNA
gagacggggtttcaccatgctggccagg

SEQ ID NO: 40552 - DNA, 28 bp, synthetic construct
  source 1..28: mol_type = other DNA
cggggtttcaccatgctggccaggctgg

SEQ ID NO: 40553 - DNA, 28 bp, synthetic construct
  source 1..28: mol_type = other DNA
gagttcgagaccagcctggccagcatgg

SEQ ID NO: 40554 - DNA, 28 bp, synthetic construct
  source 1..28: mol_type = other DNA
tgagatcaggagttcgagaccagcctgg

SEQ ID NO: 40555 - DNA, 28 bp, synthetic construct
  source 1..28: mol_type = other DNA
aggctggtctcgaactcctgatctcagg

SEQ ID NO: 40556 - DNA, 28 bp, synthetic construct
  source 1..28: mol_type = other DNA
caaggtgggtggatcacctgagatcagg

SEQ ID NO: 40557 - DNA, 28 bp, synthetic construct
  source 1..28: mol_type = other DNA
ctgatctcaggtgatccacccaccttgg

SEQ ID NO: 40558 - DNA, 28 bp, synthetic construct
  source 1..28: mol_type = other DNA
tgagtcaggatttggccaaggtgggtgg

SEQ ID NO: 40559 - DNA, 28 bp, synthetic construct
  source 1..28: mol_type = other DNA
ttgtgagtcaggatttggccaaggtggg

SEQ ID NO: 40560 - DNA, 28 bp, synthetic construct
  source 1..28: mol_type = other DNA
cttgtgagtcaggatttggccaaggtgg

SEQ ID NO: 40561 - DNA, 28 bp, synthetic construct
  source 1..28: mol_type = other DNA
catcttgtgagtcaggatttggccaagg

SEQ ID NO: 40562 - DNA, 28 bp, synthetic construct
  source 1..28: mol_type = other DNA
gccaaatcctgactcacaagatgttagg

SEQ ID NO: 40563 - DNA, 28 bp, synthetic construct
  source 1..28: mol_type = other DNA
tcctaacatcttgtgagtcaggatttgg

SEQ ID NO: 40564 - DNA, 28 bp, synthetic construct
  source 1..28: mol_type = other DNA
ctgtaatcctaacatcttgtgagtcagg

SEQ ID NO: 40565 - DNA, 28 bp, synthetic construct
  source 1..28: mol_type = other DNA
ctgactcacaagatgttaggattacagg

SEQ ID NO: 40566 - DNA, 28 bp, synthetic construct
  source 1..28: mol_type = other DNA
gattacaggcttgagccaccgcgcctgg

SEQ ID NO: 40567 - DNA, 28 bp, synthetic construct
  source 1..28: mol_type = other DNA
ttgagccaccgcgcctggcctttcttgg

SEQ ID NO: 40568 - DNA, 28 bp, synthetic construct
  source 1..28: mol_type = other DNA
aatatccaagaaaggccaggcgcggtgg

SEQ ID NO: 40569 - DNA, 28 bp, synthetic construct
  source 1..28: mol_type = other DNA
ataaatatccaagaaaggccaggcgcgg

SEQ ID NO: 40570 - DNA, 28 bp, synthetic construct
  source 1..28: mol_type = other DNA
ggttaataaatatccaagaaaggccagg

SEQ ID NO: 40571 - DNA, 28 bp, synthetic construct
  source 1..28: mol_type = other DNA
ctgatggttaataaatatccaagaaagg

SEQ ID NO: 40572 - DNA, 28 bp, synthetic construct
  source 1..28: mol_type = other DNA
ctgggattattttttaaaagtctgatgg

SEQ ID NO: 40573 - DNA, 28 bp, synthetic construct
  source 1..28: mol_type = other DNA
catcagacttttaaaaaataatcccagg

SEQ ID NO: 40574 - DNA, 28 bp, synthetic construct
  source 1..28: mol_type = other DNA
atcagacttttaaaaaataatcccaggg

SEQ ID NO: 40575 - DNA, 28 bp, synthetic construct
  source 1..28: mol_type = other DNA
ctgagggcagaattgtatcttccctggg

SEQ ID NO: 40576 - DNA, 28 bp, synthetic construct
  source 1..28: mol_type = other DNA
tctgagggcagaattgtatcttccctgg

SEQ ID NO: 40577 - DNA, 28 bp, synthetic construct
  source 1..28: mol_type = other DNA
gcaatggtatagtaaaggtctctgaggg

SEQ ID NO: 40578 - DNA, 28 bp, synthetic construct
  source 1..28: mol_type = other DNA
ggcaatggtatagtaaaggtctctgagg

SEQ ID NO: 40579 - DNA, 28 bp, synthetic construct
  source 1..28: mol_type = other DNA
actgggtttggcaatggtatagtaaagg

SEQ ID NO: 40580 - DNA, 28 bp, synthetic construct
  source 1..28: mol_type = other DNA
gcaagtgggaaactgggtttggcaatgg

SEQ ID NO: 40581 - DNA, 28 bp, synthetic construct
  source 1..28: mol_type = other DNA
gtaggagcaagtgggaaactgggtttgg

SEQ ID NO: 40582 - DNA, 28 bp, synthetic construct
  source 1..28: mol_type = other DNA
aaacccagtttcccacttgctcctacgg

SEQ ID NO: 40583 - DNA, 28 bp, synthetic construct
  source 1..28: mol_type = other DNA
actccgtaggagcaagtgggaaactggg

SEQ ID NO: 40584 - DNA, 28 bp, synthetic construct
  source 1..28: mol_type = other DNA
aactccgtaggagcaagtgggaaactgg

SEQ ID NO: 40585 - DNA, 28 bp, synthetic construct
  source 1..28: mol_type = other DNA
agctgggaactccgtaggagcaagtggg

SEQ ID NO: 40586 - DNA, 28 bp, synthetic construct
  source 1..28: mol_type = other DNA
gagctgggaactccgtaggagcaagtgg

SEQ ID NO: 40587 - DNA, 28 bp, synthetic construct
  source 1..28: mol_type = other DNA
ttcgtgtgggagctgggaactccgtagg

SEQ ID NO: 40588 - DNA, 28 bp, synthetic construct
  source 1..28: mol_type = other DNA
gcacatagggcttcgtgtgggagctggg

SEQ ID NO: 40589 - DNA, 28 bp, synthetic construct
  source 1..28: mol_type = other DNA
tgcacatagggcttcgtgtgggagctgg

SEQ ID NO: 40590 - DNA, 28 bp, synthetic construct
  source 1..28: mol_type = other DNA
ctcccacacgaagccctatgtgcactgg

SEQ ID NO: 40591 - DNA, 28 bp, synthetic construct
  source 1..28: mol_type = other DNA
gaccagtgcacatagggcttcgtgtggg

SEQ ID NO: 40592 - DNA, 28 bp, synthetic construct
  source 1..28: mol_type = other DNA
tgaccagtgcacatagggcttcgtgtgg

SEQ ID NO: 40593 - DNA, 28 bp, synthetic construct
  source 1..28: mol_type = other DNA
cagggtcttctgaccagtgcacataggg

SEQ ID NO: 40594 - DNA, 28 bp, synthetic construct
  source 1..28: mol_type = other DNA
acagggtcttctgaccagtgcacatagg

SEQ ID NO: 40595 - DNA, 28 bp, synthetic construct
  source 1..28: mol_type = other DNA
gaagaccctgtcgtgttgtccccagagg

SEQ ID NO: 40596 - DNA, 28 bp, synthetic construct
  source 1..28: mol_type = other DNA
aagaccctgtcgtgttgtccccagaggg

SEQ ID NO: 40597 - DNA, 28 bp, synthetic construct
  source 1..28: mol_type = other DNA
catgccctctggggacaacacgacaggg

SEQ ID NO: 40598 - DNA, 28 bp, synthetic construct
  source 1..28: mol_type = other DNA
ccatgccctctggggacaacacgacagg

SEQ ID NO: 40599 - DNA, 28 bp, synthetic construct
  source 1..28: mol_type = other DNA
caagtgactggcgccatgccctctgggg

SEQ ID NO: 40600 - DNA, 28 bp, synthetic construct
  source 1..28: mol_type = other DNA
tcaagtgactggcgccatgccctctggg

SEQ ID NO: 40601 - DNA, 28 bp, synthetic construct
  source 1..28: mol_type = other DNA
ctcaagtgactggcgccatgccctctgg

SEQ ID NO: 40602 - DNA, 28 bp, synthetic construct
  source 1..28: mol_type = other DNA
gggatctacagtaaactcaagtgactgg

SEQ ID NO: 40603 - DNA, 28 bp, synthetic construct
  source 1..28: mol_type = other DNA
gatcccgcagccaccagccctgatgagg

SEQ ID NO: 40604 - DNA, 28 bp, synthetic construct
  source 1..28: mol_type = other DNA
atcccgcagccaccagccctgatgaggg

SEQ ID NO: 40605 - DNA, 28 bp, synthetic construct
  source 1..28: mol_type = other DNA
gtccctcatcagggctggtggctgcggg

SEQ ID NO: 40606 - DNA, 28 bp, synthetic construct
  source 1..28: mol_type = other DNA
agtccctcatcagggctggtggctgcgg

SEQ ID NO: 40607 - DNA, 28 bp, synthetic construct
  source 1..28: mol_type = other DNA
ctcagcagtccctcatcagggctggtgg

SEQ ID NO: 40608 - DNA, 28 bp, synthetic construct
  source 1..28: mol_type = other DNA
tgactcagcagtccctcatcagggctgg

SEQ ID NO: 40609 - DNA, 28 bp, synthetic construct
  source 1..28: mol_type = other DNA
tctctgactcagcagtccctcatcaggg

SEQ ID NO: 40610 - DNA, 28 bp, synthetic construct
  source 1..28: mol_type = other DNA
ttctctgactcagcagtccctcatcagg

SEQ ID NO: 40611 - DNA, 28 bp, synthetic construct
  source 1..28: mol_type = other DNA
actgctgagtcagagaagttagaacagg

SEQ ID NO: 40612 - DNA, 28 bp, synthetic construct
  source 1..28: mol_type = other DNA
gctgagtcagagaagttagaacaggagg

SEQ ID NO: 40613 - DNA, 28 bp, synthetic construct
  source 1..28: mol_type = other DNA
ctgagtcagagaagttagaacaggaggg

SEQ ID NO: 40614 - DNA, 28 bp, synthetic construct
  source 1..28: mol_type = other DNA
agagggattacagtgattattcaaaggg

SEQ ID NO: 40615 - DNA, 28 bp, synthetic construct
  source 1..28: mol_type = other DNA
gagagggattacagtgattattcaaagg

SEQ ID NO: 40616 - DNA, 28 bp, synthetic construct
  source 1..28: mol_type = other DNA
cactgtaatccctctcaacttagagcgg

SEQ ID NO: 40617 - DNA, 28 bp, synthetic construct
  source 1..28: mol_type = other DNA
tttctcagtccgctctaagttgagaggg

SEQ ID NO: 40618 - DNA, 28 bp, synthetic construct
  source 1..28: mol_type = other DNA
atttctcagtccgctctaagttgagagg

SEQ ID NO: 40619 - DNA, 28 bp, synthetic construct
  source 1..28: mol_type = other DNA
ttagagcggactgagaaattgcccatgg

SEQ ID NO: 40620 - DNA, 28 bp, synthetic construct
  source 1..28: mol_type = other DNA
tagagcggactgagaaattgcccatggg

SEQ ID NO: 40621 - DNA, 28 bp, synthetic construct
  source 1..28: mol_type = other DNA
ttgcccatgggctccataaaaaatgtgg

SEQ ID NO: 40622 - DNA, 28 bp, synthetic construct
  source 1..28: mol_type = other DNA
tgaccacattttttatggagcccatggg

SEQ ID NO: 40623 - DNA, 28 bp, synthetic construct
  source 1..28: mol_type = other DNA
ctgaccacattttttatggagcccatgg

SEQ ID NO: 40624 - DNA, 28 bp, synthetic construct
  source 1..28: mol_type = other DNA
ataggttcactgaccacattttttatgg

SEQ ID NO: 40625 - DNA, 28 bp, synthetic construct
  source 1..28: mol_type = other DNA
aaaatgtggtcagtgaacctatcgaagg

SEQ ID NO: 40626 - DNA, 28 bp, synthetic construct
  source 1..28: mol_type = other DNA
tgtggtagtcttcatgtccttcgatagg

SEQ ID NO: 40627 - DNA, 28 bp, synthetic construct
  source 1..28: mol_type = other DNA
gaaggacatgaagactaccacatgatgg

SEQ ID NO: 40628 - DNA, 28 bp, synthetic construct
  source 1..28: mol_type = other DNA
actaccacatgatggtaagtagcgctgg

SEQ ID NO: 40629 - DNA, 28 bp, synthetic construct
  source 1..28: mol_type = other DNA
tcagccagcgctacttaccatcatgtgg

SEQ ID NO: 40630 - DNA, 28 bp, synthetic construct
  source 1..28: mol_type = other DNA
aggtgaagtgggagtctagtgagagggg

SEQ ID NO: 40631 - DNA, 28 bp, synthetic construct
  source 1..28: mol_type = other DNA
caggtgaagtgggagtctagtgagaggg

SEQ ID NO: 40632 - DNA, 28 bp, synthetic construct
  source 1..28: mol_type = other DNA
cctctcactagactcccacttcacctgg

SEQ ID NO: 40633 - DNA, 28 bp, synthetic construct
  source 1..28: mol_type = other DNA
tcactagactcccacttcacctggcagg

SEQ ID NO: 40634 - DNA, 28 bp, synthetic construct
  source 1..28: mol_type = other DNA
cactagactcccacttcacctggcaggg

SEQ ID NO: 40635 - DNA, 28 bp, synthetic construct
  source 1..28: mol_type = other DNA
aaaactgttccctgccaggtgaagtggg

SEQ ID NO: 40636 - DNA, 28 bp, synthetic construct
  source 1..28: mol_type = other DNA
taaaactgttccctgccaggtgaagtgg

SEQ ID NO: 40637 - DNA, 28 bp, synthetic construct
  source 1..28: mol_type = other DNA
agctcagttaaaactgttccctgccagg

SEQ ID NO: 40638 - DNA, 28 bp, synthetic construct
  source 1..28: mol_type = other DNA
aacagttttaactgagcttgtttaacgg

SEQ ID NO: 40639 - DNA, 28 bp, synthetic construct
  source 1..28: mol_type = other DNA
ggttgggatgtgagttaattaaaaaggg

SEQ ID NO: 40640 - DNA, 28 bp, synthetic construct
  source 1..28: mol_type = other DNA
gggttgggatgtgagttaattaaaaagg

SEQ ID NO: 40641 - DNA, 28 bp, synthetic construct
  source 1..28: mol_type = other DNA
ggcaggacaaacatgggtgagggttggg

SEQ ID NO: 40642 - DNA, 28 bp, synthetic construct
  source 1..28: mol_type = other DNA
aggcaggacaaacatgggtgagggttgg

SEQ ID NO: 40643 - DNA, 28 bp, synthetic construct
  source 1..28: mol_type = other DNA
aagcaggcaggacaaacatgggtgaggg

SEQ ID NO: 40644 - DNA, 28 bp, synthetic construct
  source 1..28: mol_type = other DNA
caagcaggcaggacaaacatgggtgagg

SEQ ID NO: 40645 - DNA, 28 bp, synthetic construct
  source 1..28: mol_type = other DNA
ctcacccatgtttgtcctgcctgcttgg

SEQ ID NO: 40646 - DNA, 28 bp, synthetic construct
  source 1..28: mol_type = other DNA
gagaccaagcaggcaggacaaacatggg

SEQ ID NO: 40647 - DNA, 28 bp, synthetic construct
  source 1..28: mol_type = other DNA
ggagaccaagcaggcaggacaaacatgg

SEQ ID NO: 40648 - DNA, 28 bp, synthetic construct
  source 1..28: mol_type = other DNA
tcagaggtcgggagaccaagcaggcagg

SEQ ID NO: 40649 - DNA, 28 bp, synthetic construct
  source 1..28: mol_type = other DNA
tacttcagaggtcgggagaccaagcagg

SEQ ID NO: 40650 - DNA, 28 bp, synthetic construct
  source 1..28: mol_type = other DNA
gtctcccgacctctgaagtaccgcttgg

SEQ ID NO: 40651 - DNA, 28 bp, synthetic construct
  source 1..28: mol_type = other DNA
aaaaccaagcggtacttcagaggtcggg

SEQ ID NO: 40652 - DNA, 28 bp, synthetic construct
  source 1..28: mol_type = other DNA
gaaaaccaagcggtacttcagaggtcgg

SEQ ID NO: 40653 - DNA, 28 bp, synthetic construct
  source 1..28: mol_type = other DNA
aaaggaaaaccaagcggtacttcagagg

SEQ ID NO: 40654 - DNA, 28 bp, synthetic construct
  source 1..28: mol_type = other DNA
ctggaagggaaaaaggaaaaccaagcgg

SEQ ID NO: 40655 - DNA, 28 bp, synthetic construct
  source 1..28: mol_type = other DNA
cgcttggttttcctttttcccttccagg

SEQ ID NO: 40656 - DNA, 28 bp, synthetic construct
  source 1..28: mol_type = other DNA
caactgaaacgcctggaagggaaaaagg

SEQ ID NO: 40657 - DNA, 28 bp, synthetic construct
  source 1..28: mol_type = other DNA
ctttttcccttccaggcgtttcagttgg

SEQ ID NO: 40658 - DNA, 28 bp, synthetic construct
  source 1..28: mol_type = other DNA
tttttcccttccaggcgtttcagttggg

SEQ ID NO: 40659 - DNA, 28 bp, synthetic construct
  source 1..28: mol_type = other DNA
tggggcccaactgaaacgcctggaaggg

SEQ ID NO: 40660 - DNA, 28 bp, synthetic construct
  source 1..28: mol_type = other DNA
gtggggcccaactgaaacgcctggaagg

SEQ ID NO: 40661 - DNA, 28 bp, synthetic construct
  source 1..28: mol_type = other DNA
ttccaggcgtttcagttgggccccacgg

SEQ ID NO: 40662 - DNA, 28 bp, synthetic construct
  source 1..28: mol_type = other DNA
ttccgtggggcccaactgaaacgcctgg

SEQ ID NO: 40663 - DNA, 28 bp, synthetic construct
  source 1..28: mol_type = other DNA
gggccccacggaagcctcttactactgg

SEQ ID NO: 40664 - DNA, 28 bp, synthetic construct
  source 1..28: mol_type = other DNA
ggccccacggaagcctcttactactggg

SEQ ID NO: 40665 - DNA, 28 bp, synthetic construct
  source 1..28: mol_type = other DNA
cacccagtagtaagaggcttccgtgggg

SEQ ID NO: 40666 - DNA, 28 bp, synthetic construct
  source 1..28: mol_type = other DNA
acacccagtagtaagaggcttccgtggg

SEQ ID NO: 40667 - DNA, 28 bp, synthetic construct
  source 1..28: mol_type = other DNA
tacacccagtagtaagaggcttccgtgg

SEQ ID NO: 40668 - DNA, 28 bp, synthetic construct
  source 1..28: mol_type = other DNA
ggaagcctcttactactgggtgtactgg

SEQ ID NO: 40669 - DNA, 28 bp, synthetic construct
  source 1..28: mol_type = other DNA
gaagcctcttactactgggtgtactggg

SEQ ID NO: 40670 - DNA, 28 bp, synthetic construct
  source 1..28: mol_type = other DNA
ggaacccagtacacccagtagtaagagg

SEQ ID NO: 40671 - DNA, 28 bp, synthetic construct
  source 1..28: mol_type = other DNA
gtgtactgggttccaactcaatatgtgg

SEQ ID NO: 40672 - DNA, 28 bp, synthetic construct
  source 1..28: mol_type = other DNA
ctttgattgcatccacatattgagttgg

SEQ ID NO: 40673 - DNA, 28 bp, synthetic construct
  source 1..28: mol_type = other DNA
gtggatgcaatcaaagacactgtgctgg

SEQ ID NO: 40674 - DNA, 28 bp, synthetic construct
  source 1..28: mol_type = other DNA
tggatgcaatcaaagacactgtgctggg

SEQ ID NO: 40675 - DNA, 28 bp, synthetic construct
  source 1..28: mol_type = other DNA
ggatgcaatcaaagacactgtgctgggg

SEQ ID NO: 40676 - DNA, 28 bp, synthetic construct
  source 1..28: mol_type = other DNA
aatcaaagacactgtgctggggaaatgg

SEQ ID NO: 40677 - DNA, 28 bp, synthetic construct
  source 1..28: mol_type = other DNA
gtatttttgaaagcactttcacctctgg

SEQ ID NO: 40678 - DNA, 28 bp, synthetic construct
  source 1..28: mol_type = other DNA
ttgaaagcactttcacctctggcccagg

SEQ ID NO: 40679 - DNA, 28 bp, synthetic construct
  source 1..28: mol_type = other DNA
actttgggtcagtctcctgggccagagg

SEQ ID NO: 40680 - DNA, 28 bp, synthetic construct
  source 1..28: mol_type = other DNA
ggcccaggagactgacccaaagtgaagg

SEQ ID NO: 40681 - DNA, 28 bp, synthetic construct
  source 1..28: mol_type = other DNA
gtccttcactttgggtcagtctcctggg

SEQ ID NO: 40682 - DNA, 28 bp, synthetic construct
  source 1..28: mol_type = other DNA
tgtccttcactttgggtcagtctcctgg

SEQ ID NO: 40683 - DNA, 28 bp, synthetic construct
  source 1..28: mol_type = other DNA
actgacccaaagtgaaggacattgccgg

SEQ ID NO: 40684 - DNA, 28 bp, synthetic construct
  source 1..28: mol_type = other DNA
ctgacccaaagtgaaggacattgccggg

SEQ ID NO: 40685 - DNA, 28 bp, synthetic construct
  source 1..28: mol_type = other DNA
ctctcccggcaatgtccttcactttggg

SEQ ID NO: 40686 - DNA, 28 bp, synthetic construct
  source 1..28: mol_type = other DNA
ccaaagtgaaggacattgccgggagagg

SEQ ID NO: 40687 - DNA, 28 bp, synthetic construct
  source 1..28: mol_type = other DNA
tgccgggagaggcctgcagcatccctgg

SEQ ID NO: 40688 - DNA, 28 bp, synthetic construct
  source 1..28: mol_type = other DNA
atccagggatgctgcaggcctctcccgg

SEQ ID NO: 40689 - DNA, 28 bp, synthetic construct
  source 1..28: mol_type = other DNA
gaactctgaaatccagggatgctgcagg

SEQ ID NO: 40690 - DNA, 28 bp, synthetic construct
  source 1..28: mol_type = other DNA
gcagcatccctggatttcagagttctgg

SEQ ID NO: 40691 - DNA, 28 bp, synthetic construct
  source 1..28: mol_type = other DNA
caaagttccagaactctgaaatccaggg

SEQ ID NO: 40692 - DNA, 28 bp, synthetic construct
  source 1..28: mol_type = other DNA
acaaagttccagaactctgaaatccagg

SEQ ID NO: 40693 - DNA, 28 bp, synthetic construct
  source 1..28: mol_type = other DNA
tcataaaaaatctatattcaatctgagg

SEQ ID NO: 40694 - DNA, 28 bp, synthetic construct
  source 1..28: mol_type = other DNA
aatctatattcaatctgaggtgatgtgg

SEQ ID NO: 40695 - DNA, 28 bp, synthetic construct
  source 1..28: mol_type = other DNA
gaggtgatgtggtgactgaagccagagg

SEQ ID NO: 40696 - DNA, 28 bp, synthetic construct
  source 1..28: mol_type = other DNA
gctaatggtgaaagtacatcacctctgg

SEQ ID NO: 40697 - DNA, 28 bp, synthetic construct
  source 1..28: mol_type = other DNA
taattttaagttaaaattaagctaatgg

SEQ ID NO: 40698 - DNA, 28 bp, synthetic construct
  source 1..28: mol_type = other DNA
tgaagctgactgcaagaaagggaactgg

SEQ ID NO: 40699 - DNA, 28 bp, synthetic construct
  source 1..28: mol_type = other DNA
atggtatgaagctgactgcaagaaaggg

SEQ ID NO: 40700 - DNA, 28 bp, synthetic construct
  source 1..28: mol_type = other DNA
aatggtatgaagctgactgcaagaaagg

SEQ ID NO: 40701 - DNA, 28 bp, synthetic construct
  source 1..28: mol_type = other DNA
cataccatttttaaagtcaatacgatgg

SEQ ID NO: 40702 - DNA, 28 bp, synthetic construct
  source 1..28: mol_type = other DNA
atttccatcgtattgactttaaaaatgg

SEQ ID NO: 40703 - DNA, 28 bp, synthetic construct
  source 1..28: mol_type = other DNA
aaatctgaattccgaacatgttgtgtgg

SEQ ID NO: 40704 - DNA, 28 bp, synthetic construct
  source 1..28: mol_type = other DNA
ttaagagtattccacacaacatgttcgg

SEQ ID NO: 40705 - DNA, 28 bp, synthetic construct
  source 1..28: mol_type = other DNA
agtagatctgccaattatgttgacaagg

SEQ ID NO: 40706 - DNA, 28 bp, synthetic construct
  source 1..28: mol_type = other DNA
gtagatctgccaattatgttgacaaggg

SEQ ID NO: 40707 - DNA, 28 bp, synthetic construct
  source 1..28: mol_type = other DNA
ttgatcattcccttgtcaacataattgg

SEQ ID NO: 40708 - DNA, 28 bp, synthetic construct
  source 1..28: mol_type = other DNA
caattgaaatattttcatacatctttgg

SEQ ID NO: 40709 - DNA, 28 bp, synthetic construct
  source 1..28: mol_type = other DNA
tcatacatctttggttgcaaacatttgg

SEQ ID NO: 40710 - DNA, 28 bp, synthetic construct
  source 1..28: mol_type = other DNA
acatttggactgcattgcaatgagttgg

SEQ ID NO: 40711 - DNA, 28 bp, synthetic construct
  source 1..28: mol_type = other DNA
catttggactgcattgcaatgagttggg

SEQ ID NO: 40712 - DNA, 28 bp, synthetic construct
  source 1..28: mol_type = other DNA
atttggactgcattgcaatgagttgggg

SEQ ID NO: 40713 - DNA, 28 bp, synthetic construct
  source 1..28: mol_type = other DNA
ttttgcatacaattttatacaaaaaagg

SEQ ID NO: 40714 - DNA, 28 bp, synthetic construct
  source 1..28: mol_type = other DNA
tttttgtataaaattgtatgcaaaatgg

SEQ ID NO: 40715 - DNA, 28 bp, synthetic construct
  source 1..28: mol_type = other DNA
ttttgtataaaattgtatgcaaaatggg

SEQ ID NO: 40716 - DNA, 28 bp, synthetic construct
  source 1..28: mol_type = other DNA
tttgtataaaattgtatgcaaaatgggg

SEQ ID NO: 40717 - DNA, 28 bp, synthetic construct
  source 1..28: mol_type = other DNA
ttgtataaaattgtatgcaaaatggggg

SEQ ID NO: 40718 - DNA, 28 bp, synthetic construct
  source 1..28: mol_type = other DNA
tataaaattgtatgcaaaatgggggtgg

SEQ ID NO: 40719 - DNA, 28 bp, synthetic construct
  source 1..28: mol_type = other DNA
ataaaattgtatgcaaaatgggggtggg

SEQ ID NO: 40720 - DNA, 28 bp, synthetic construct
  source 1..28: mol_type = other DNA
atctgaatcaatggacagaaatatgtgg

SEQ ID NO: 40721 - DNA, 28 bp, synthetic construct
  source 1..28: mol_type = other DNA
agggaaagaattaaatctgaatcaatgg

SEQ ID NO: 40722 - DNA, 28 bp, synthetic construct
  source 1..28: mol_type = other DNA
attgaggaagcgagagaatgaaaaaggg

SEQ ID NO: 40723 - DNA, 28 bp, synthetic construct
  source 1..28: mol_type = other DNA
aattgaggaagcgagagaatgaaaaagg

SEQ ID NO: 40724 - DNA, 28 bp, synthetic construct
  source 1..28: mol_type = other DNA
gttcttaaaacaaaaactcaaattgagg

SEQ ID NO: 40725 - DNA, 28 bp, synthetic construct
  source 1..28: mol_type = other DNA
aacccaaagatgtcagttcttcttttgg

SEQ ID NO: 40726 - DNA, 28 bp, synthetic construct
  source 1..28: mol_type = other DNA
taccaaaagaagaactgacatctttggg

SEQ ID NO: 40727 - DNA, 28 bp, synthetic construct
  source 1..28: mol_type = other DNA
gtaccaaaagaagaactgacatctttgg

SEQ ID NO: 40728 - DNA, 28 bp, synthetic construct
  source 1..28: mol_type = other DNA
ggtacctcatcaacgcttcctttcctgg

SEQ ID NO: 40729 - DNA, 28 bp, synthetic construct
  source 1..28: mol_type = other DNA
gtacctcatcaacgcttcctttcctggg

SEQ ID NO: 40730 - DNA, 28 bp, synthetic construct
  source 1..28: mol_type = other DNA
gagcccaggaaaggaagcgttgatgagg

SEQ ID NO: 40731 - DNA, 28 bp, synthetic construct
  source 1..28: mol_type = other DNA
agcacggcgggagggagcccaggaaagg

SEQ ID NO: 40732 - DNA, 28 bp, synthetic construct
  source 1..28: mol_type = other DNA
gcagcagcacggcgggagggagcccagg

SEQ ID NO: 40733 - DNA, 28 bp, synthetic construct
  source 1..28: mol_type = other DNA
cacaggcagcagcagcacggcgggaggg

SEQ ID NO: 40734 - DNA, 28 bp, synthetic construct
  source 1..28: mol_type = other DNA
tcacaggcagcagcagcacggcgggagg

SEQ ID NO: 40735 - DNA, 28 bp, synthetic construct
  source 1..28: mol_type = other DNA
cgttcacaggcagcagcagcacggcggg

SEQ ID NO: 40736 - DNA, 28 bp, synthetic construct
  source 1..28: mol_type = other DNA
gcgttcacaggcagcagcagcacggcgg

SEQ ID NO: 40737 - DNA, 28 bp, synthetic construct
  source 1..28: mol_type = other DNA
cgtgcgttcacaggcagcagcagcacgg

SEQ ID NO: 40738 - DNA, 28 bp, synthetic construct
  source 1..28: mol_type = other DNA
cgtgctgctgctgcctgtgaacgcacgg

SEQ ID NO: 40739 - DNA, 28 bp, synthetic construct
  source 1..28: mol_type = other DNA
gctgctgctgcctgtgaacgcacggtgg

SEQ ID NO: 40740 - DNA, 28 bp, synthetic construct
  source 1..28: mol_type = other DNA
ctgctgctgcctgtgaacgcacggtggg

SEQ ID NO: 40741 - DNA, 28 bp, synthetic construct
  source 1..28: mol_type = other DNA
gctgcctgtgaacgcacggtgggagagg

SEQ ID NO: 40742 - DNA, 28 bp, synthetic construct
  source 1..28: mol_type = other DNA
tcttcctctcccaccgtgcgttcacagg

SEQ ID NO: 40743 - DNA, 28 bp, synthetic construct
  source 1..28: mol_type = other DNA
tgggagaggaagagctgctcagtcttgg

SEQ ID NO: 40744 - DNA, 28 bp, synthetic construct
  source 1..28: mol_type = other DNA
gggagaggaagagctgctcagtcttggg

SEQ ID NO: 40745 - DNA, 28 bp, synthetic construct
  source 1..28: mol_type = other DNA
aggaagagctgctcagtcttgggcaagg

SEQ ID NO: 40746 - DNA, 28 bp, synthetic construct
  source 1..28: mol_type = other DNA
gggcaaggagctctcacacttgctgtgg

SEQ ID NO: 40747 - DNA, 28 bp, synthetic construct
  source 1..28: mol_type = other DNA
gcaagacatttaaacaggagtcactggg

SEQ ID NO: 40748 - DNA, 28 bp, synthetic construct
  source 1..28: mol_type = other DNA
ggcaagacatttaaacaggagtcactgg

SEQ ID NO: 40749 - DNA, 28 bp, synthetic construct
  source 1..28: mol_type = other DNA
actcctgtttaaatgtcttgccctttgg

SEQ ID NO: 40750 - DNA, 28 bp, synthetic construct
  source 1..28: mol_type = other DNA
ctcctgtttaaatgtcttgccctttggg

SEQ ID NO: 40751 - DNA, 28 bp, synthetic construct
  source 1..28: mol_type = other DNA
ggcccaaagggcaagacatttaaacagg

SEQ ID NO: 40752 - DNA, 28 bp, synthetic construct
  source 1..28: mol_type = other DNA
cttgccctttgggcccccatctccaagg

SEQ ID NO: 40753 - DNA, 28 bp, synthetic construct
  source 1..28: mol_type = other DNA
aactccttggagatgggggcccaaaggg

SEQ ID NO: 40754 - DNA, 28 bp, synthetic construct
  source 1..28: mol_type = other DNA
gaactccttggagatgggggcccaaagg

SEQ ID NO: 40755 - DNA, 28 bp, synthetic construct
  source 1..28: mol_type = other DNA
cagcaatggaactccttggagatggggg

SEQ ID NO: 40756 - DNA, 28 bp, synthetic construct
  source 1..28: mol_type = other DNA
ccccatctccaaggagttccattgctgg

SEQ ID NO: 40757 - DNA, 28 bp, synthetic construct
  source 1..28: mol_type = other DNA
accagcaatggaactccttggagatggg

SEQ ID NO: 40758 - DNA, 28 bp, synthetic construct
  source 1..28: mol_type = other DNA
aaccagcaatggaactccttggagatgg

SEQ ID NO: 40759 - DNA, 28 bp, synthetic construct
  source 1..28: mol_type = other DNA
atctccaaggagttccattgctggttgg

SEQ ID NO: 40760 - DNA, 28 bp, synthetic construct
  source 1..28: mol_type = other DNA
tcatccaaccagcaatggaactccttgg

SEQ ID NO: 40761 - DNA, 28 bp, synthetic construct
  source 1..28: mol_type = other DNA
gtgcagacaatcatccaaccagcaatgg

SEQ ID NO: 40762 - DNA, 28 bp, synthetic construct
  source 1..28: mol_type = other DNA
gattgtctgcacccctcactgagcttgg

SEQ ID NO: 40763 - DNA, 28 bp, synthetic construct
  source 1..28: mol_type = other DNA
gcacccctcactgagcttggcctagagg

SEQ ID NO: 40764 - DNA, 28 bp, synthetic construct
  source 1..28: mol_type = other DNA
gggcctctaggccaagctcagtgagggg

SEQ ID NO: 40765 - DNA, 28 bp, synthetic construct
  source 1..28: mol_type = other DNA
tgggcctctaggccaagctcagtgaggg

SEQ ID NO: 40766 - DNA, 28 bp, synthetic construct
  source 1..28: mol_type = other DNA
ctgggcctctaggccaagctcagtgagg

SEQ ID NO: 40767 - DNA, 28 bp, synthetic construct
  source 1..28: mol_type = other DNA
ctgagcttggcctagaggcccagcctgg

SEQ ID NO: 40768 - DNA, 28 bp, synthetic construct
  source 1..28: mol_type = other DNA
cttggcctagaggcccagcctggcatgg

SEQ ID NO: 40769 - DNA, 28 bp, synthetic construct
  source 1..28: mol_type = other DNA
cacaaccatgccaggctgggcctctagg

SEQ ID NO: 40770 - DNA, 28 bp, synthetic construct
  source 1..28: mol_type = other DNA
aggcccagcctggcatggttgtgcctgg

SEQ ID NO: 40771 - DNA, 28 bp, synthetic construct
  source 1..28: mol_type = other DNA
ggcccagcctggcatggttgtgcctggg

SEQ ID NO: 40772 - DNA, 28 bp, synthetic construct
  source 1..28: mol_type = other DNA
agcccaggcacaaccatgccaggctggg

SEQ ID NO: 40773 - DNA, 28 bp, synthetic construct
  source 1..28: mol_type = other DNA
cagcccaggcacaaccatgccaggctgg

SEQ ID NO: 40774 - DNA, 28 bp, synthetic construct
  source 1..28: mol_type = other DNA
ggcacagcccaggcacaaccatgccagg

SEQ ID NO: 40775 - DNA, 28 bp, synthetic construct
  source 1..28: mol_type = other DNA
ctggggctgttgagcggcacagcccagg

SEQ ID NO: 40776 - DNA, 28 bp, synthetic construct
  source 1..28: mol_type = other DNA
ctgcttgggagctggggctgttgagcgg

SEQ ID NO: 40777 - DNA, 28 bp, synthetic construct
  source 1..28: mol_type = other DNA
gaggtctttgtctgcttgggagctgggg

SEQ ID NO: 40778 - DNA, 28 bp, synthetic construct
  source 1..28: mol_type = other DNA
agaggtctttgtctgcttgggagctggg

SEQ ID NO: 40779 - DNA, 28 bp, synthetic construct
  source 1..28: mol_type = other DNA
aagaggtctttgtctgcttgggagctgg

SEQ ID NO: 40780 - DNA, 28 bp, synthetic construct
  source 1..28: mol_type = other DNA
tcccaagcagacaaagacctcttccagg

SEQ ID NO: 40781 - DNA, 28 bp, synthetic construct
  source 1..28: mol_type = other DNA
tcctggaagaggtctttgtctgcttggg

SEQ ID NO: 40782 - DNA, 28 bp, synthetic construct
  source 1..28: mol_type = other DNA
ctcctggaagaggtctttgtctgcttgg

SEQ ID NO: 40783 - DNA, 28 bp, synthetic construct
  source 1..28: mol_type = other DNA
caagcagacaaagacctcttccaggagg

SEQ ID NO: 40784 - DNA, 28 bp, synthetic construct
  source 1..28: mol_type = other DNA
acaaagacctcttccaggaggagccagg

SEQ ID NO: 40785 - DNA, 28 bp, synthetic construct
  source 1..28: mol_type = other DNA
tcttctacctggctcctcctggaagagg

SEQ ID NO: 40786 - DNA, 28 bp, synthetic construct
  source 1..28: mol_type = other DNA
taactatcttctacctggctcctcctgg

SEQ ID NO: 40787 - DNA, 28 bp, synthetic construct
  source 1..28: mol_type = other DNA
tatggctgtataactatcttctacctgg

SEQ ID NO: 40788 - DNA, 28 bp, synthetic construct
  source 1..28: mol_type = other DNA
aaggttatctggatctgcagctatatgg

SEQ ID NO: 40789 - DNA, 28 bp, synthetic construct
  source 1..28: mol_type = other DNA
gcagatccagataaccttctttctttgg

SEQ ID NO: 40790 - DNA, 28 bp, synthetic construct
  source 1..28: mol_type = other DNA
aaacttccaaagaaagaaggttatctgg

SEQ ID NO: 40791 - DNA, 28 bp, synthetic construct
  source 1..28: mol_type = other DNA
tttcttgaaaacttccaaagaaagaagg

SEQ ID NO: 40792 - DNA, 28 bp, synthetic construct
  source 1..28: mol_type = other DNA
tttcaagaaattcttaagcagtccaagg

SEQ ID NO: 40793 - DNA, 28 bp, synthetic construct
  source 1..28: mol_type = other DNA
ggagaagcataattgaaatcatccttgg

SEQ ID NO: 40794 - DNA, 28 bp, synthetic construct
  source 1..28: mol_type = other DNA
gatgatttcaattatgcttctccattgg

SEQ ID NO: 40795 - DNA, 28 bp, synthetic construct
  source 1..28: mol_type = other DNA
atgatttcaattatgcttctccattggg

SEQ ID NO: 40796 - DNA, 28 bp, synthetic construct
  source 1..28: mol_type = other DNA
tgaatgcatgagcagaaggacccaatgg

SEQ ID NO: 40797 - DNA, 28 bp, synthetic construct
  source 1..28: mol_type = other DNA
cacttgaactgaatgcatgagcagaagg

SEQ ID NO: 40798 - DNA, 28 bp, synthetic construct
  source 1..28: mol_type = other DNA
attcagttcaagtgtcctttatcccagg

SEQ ID NO: 40799 - DNA, 28 bp, synthetic construct
  source 1..28: mol_type = other DNA
ggcagcatctctgaacctgggataaagg

SEQ ID NO: 40800 - DNA, 28 bp, synthetic construct
  source 1..28: mol_type = other DNA
tcagaaaggcagcatctctgaacctggg

SEQ ID NO: 40801 - DNA, 28 bp, synthetic construct
  source 1..28: mol_type = other DNA
ttcagaaaggcagcatctctgaacctgg

SEQ ID NO: 40802 - DNA, 28 bp, synthetic construct
  source 1..28: mol_type = other DNA
ctagggtcagatgtcttcttcagaaagg

SEQ ID NO: 40803 - DNA, 28 bp, synthetic construct
  source 1..28: mol_type = other DNA
tctgaagaagacatctgaccctagcagg

SEQ ID NO: 40804 - DNA, 28 bp, synthetic construct
  source 1..28: mol_type = other DNA
aagaagacatctgaccctagcaggttgg

SEQ ID NO: 40805 - DNA, 28 bp, synthetic construct
  source 1..28: mol_type = other DNA
ttcaataacactggccaacctgctaggg

SEQ ID NO: 40806 - DNA, 28 bp, synthetic construct
  source 1..28: mol_type = other DNA
gttcaataacactggccaacctgctagg

SEQ ID NO: 40807 - DNA, 28 bp, synthetic construct
  source 1..28: mol_type = other DNA
ggccagtgttattgaacaacaaaaatgg

SEQ ID NO: 40808 - DNA, 28 bp, synthetic construct
  source 1..28: mol_type = other DNA
gccagtgttattgaacaacaaaaatggg

SEQ ID NO: 40809 - DNA, 28 bp, synthetic construct
  source 1..28: mol_type = other DNA
tcccatttttgttgttcaataacactgg

SEQ ID NO: 40810 - DNA, 28 bp, synthetic construct
  source 1..28: mol_type = other DNA
ctttcatgattagctcaccttcttctgg

SEQ ID NO: 40811 - DNA, 28 bp, synthetic construct
  source 1..28: mol_type = other DNA
gaacagaagggctaaaaccagaagaagg

SEQ ID NO: 40812 - DNA, 28 bp, synthetic construct
  source 1..28: mol_type = other DNA
aagttcacgtgtacagagaacagaaggg

SEQ ID NO: 40813 - DNA, 28 bp, synthetic construct
  source 1..28: mol_type = other DNA
gaagttcacgtgtacagagaacagaagg

SEQ ID NO: 40814 - DNA, 28 bp, synthetic construct
  source 1..28: mol_type = other DNA
cacgtgaacttctgtcatctccttctgg

SEQ ID NO: 40815 - DNA, 28 bp, synthetic construct
  source 1..28: mol_type = other DNA
gaacttctgtcatctccttctggcttgg

SEQ ID NO: 40816 - DNA, 28 bp, synthetic construct
  source 1..28: mol_type = other DNA
tccttctggcttggttgcctctgaaagg

SEQ ID NO: 40817 - DNA, 28 bp, synthetic construct
  source 1..28: mol_type = other DNA
tcctttcagaggcaaccaagccagaagg

SEQ ID NO: 40818 - DNA, 28 bp, synthetic construct
  source 1..28: mol_type = other DNA
ttctggcttggttgcctctgaaaggagg

SEQ ID NO: 40819 - DNA, 28 bp, synthetic construct
  source 1..28: mol_type = other DNA
tctggcttggttgcctctgaaaggaggg

SEQ ID NO: 40820 - DNA, 28 bp, synthetic construct
  source 1..28: mol_type = other DNA
gcctctgaaaggagggaaagtctcttgg

SEQ ID NO: 40821 - DNA, 28 bp, synthetic construct
  source 1..28: mol_type = other DNA
accaagagactttccctcctttcagagg

SEQ ID NO: 40822 - DNA, 28 bp, synthetic construct
  source 1..28: mol_type = other DNA
gccgtctttgcagttctcctctcactgg

SEQ ID NO: 40823 - DNA, 28 bp, synthetic construct
  source 1..28: mol_type = other DNA
accagtgagaggagaactgcaaagacgg

SEQ ID NO: 40824 - DNA, 28 bp, synthetic construct
  source 1..28: mol_type = other DNA
ttgcagttctcctctcactggttgcagg

SEQ ID NO: 40825 - DNA, 28 bp, synthetic construct
  source 1..28: mol_type = other DNA
actatgaaagcctgcaaccagtgagagg

SEQ ID NO: 40826 - DNA, 28 bp, synthetic construct
  source 1..28: mol_type = other DNA
tcactggttgcaggctttcatagtaagg

SEQ ID NO: 40827 - DNA, 28 bp, synthetic construct
  source 1..28: mol_type = other DNA
ggttgcaggctttcatagtaaggtttgg

SEQ ID NO: 40828 - DNA, 28 bp, synthetic construct
  source 1..28: mol_type = other DNA
gagaaatgttccaaacatcacattttgg

SEQ ID NO: 40829 - DNA, 28 bp, synthetic construct
  source 1..28: mol_type = other DNA
ttccaaacatcacattttggattctagg

SEQ ID NO: 40830 - DNA, 28 bp, synthetic construct
  source 1..28: mol_type = other DNA
agcctagaatccaaaatgtgatgtttgg

SEQ ID NO: 40831 - DNA, 28 bp, synthetic construct
  source 1..28: mol_type = other DNA
atgctaatacgtttcacagaatgagggg

SEQ ID NO: 40832 - DNA, 28 bp, synthetic construct
  source 1..28: mol_type = other DNA
catgctaatacgtttcacagaatgaggg

SEQ ID NO: 40833 - DNA, 28 bp, synthetic construct
  source 1..28: mol_type = other DNA
acatgctaatacgtttcacagaatgagg

SEQ ID NO: 40834 - DNA, 28 bp, synthetic construct
  source 1..28: mol_type = other DNA
ctggctcacaaggaatagtcatcttggg

SEQ ID NO: 40835 - DNA, 28 bp, synthetic construct
  source 1..28: mol_type = other DNA
actggctcacaaggaatagtcatcttgg

SEQ ID NO: 40836 - DNA, 28 bp, synthetic construct
  source 1..28: mol_type = other DNA
gaatatcatcattaactggctcacaagg

SEQ ID NO: 40837 - DNA, 28 bp, synthetic construct
  source 1..28: mol_type = other DNA
aagggcgtagaatatcatcattaactgg

SEQ ID NO: 40838 - DNA, 28 bp, synthetic construct
  source 1..28: mol_type = other DNA
gcccttcccttctaagctgtagttcagg

SEQ ID NO: 40839 - DNA, 28 bp, synthetic construct
  source 1..28: mol_type = other DNA
tcctgaactacagcttagaagggaaggg

SEQ ID NO: 40840 - DNA, 28 bp, synthetic construct
  source 1..28: mol_type = other DNA
ttcctgaactacagcttagaagggaagg

SEQ ID NO: 40841 - DNA, 28 bp, synthetic construct
  source 1..28: mol_type = other DNA
tggattcctgaactacagcttagaaggg

SEQ ID NO: 40842 - DNA, 28 bp, synthetic construct
  source 1..28: mol_type = other DNA
ctggattcctgaactacagcttagaagg

SEQ ID NO: 40843 - DNA, 28 bp, synthetic construct
  source 1..28: mol_type = other DNA
aaagcaagagtctgtctatgtgggctgg

SEQ ID NO: 40844 - DNA, 28 bp, synthetic construct
  source 1..28: mol_type = other DNA
atggaaagcaagagtctgtctatgtggg

SEQ ID NO: 40845 - DNA, 28 bp, synthetic construct
  source 1..28: mol_type = other DNA
catggaaagcaagagtctgtctatgtgg

SEQ ID NO: 40846 - DNA, 28 bp, synthetic construct
  source 1..28: mol_type = other DNA
cacatagacagactcttgctttccatgg

SEQ ID NO: 40847 - DNA, 28 bp, synthetic construct
  source 1..28: mol_type = other DNA
gcatcacttggcattgactacaccatgg

SEQ ID NO: 40848 - DNA, 28 bp, synthetic construct
  source 1..28: mol_type = other DNA
gtagtcaatgccaagtgatgcatctagg

SEQ ID NO: 40849 - DNA, 28 bp, synthetic construct
  source 1..28: mol_type = other DNA
tcaatgccaagtgatgcatctaggcagg

SEQ ID NO: 40850 - DNA, 28 bp, synthetic construct
  source 1..28: mol_type = other DNA
gattttcctgcctagatgcatcacttgg

SEQ ID NO: 40851 - DNA, 28 bp, synthetic construct
  source 1..28: mol_type = other DNA
caggaaaatctactctttgcttttttgg

SEQ ID NO: 40852 - DNA, 28 bp, synthetic construct
  source 1..28: mol_type = other DNA
aggaaaatctactctttgcttttttggg

SEQ ID NO: 40853 - DNA, 28 bp, synthetic construct
  source 1..28: mol_type = other DNA
ggaaaatctactctttgcttttttgggg

SEQ ID NO: 40854 - DNA, 28 bp, synthetic construct
  source 1..28: mol_type = other DNA
gaaaatctactctttgcttttttggggg

SEQ ID NO: 40855 - DNA, 28 bp, synthetic construct
  source 1..28: mol_type = other DNA
agggatgaaaaaacaggctgtttcttgg

SEQ ID NO: 40856 - DNA, 28 bp, synthetic construct
  source 1..28: mol_type = other DNA
agcctgttttttcatcccttgagaaagg

SEQ ID NO: 40857 - DNA, 28 bp, synthetic construct
  source 1..28: mol_type = other DNA
ctcctttctcaagggatgaaaaaacagg

SEQ ID NO: 40858 - DNA, 28 bp, synthetic construct
  source 1..28: mol_type = other DNA
gctgcaatgactgctcctttctcaaggg

SEQ ID NO: 40859 - DNA, 28 bp, synthetic construct
  source 1..28: mol_type = other DNA
agctgcaatgactgctcctttctcaagg

SEQ ID NO: 40860 - DNA, 28 bp, synthetic construct
  source 1..28: mol_type = other DNA
gtcattgcagcttttctgtccttgtcgg

SEQ ID NO: 40861 - DNA, 28 bp, synthetic construct
  source 1..28: mol_type = other DNA
tctgtccttgtcggcctgcagttcctgg

SEQ ID NO: 40862 - DNA, 28 bp, synthetic construct
  source 1..28: mol_type = other DNA
ctgtccttgtcggcctgcagttcctggg

SEQ ID NO: 40863 - DNA, 28 bp, synthetic construct
  source 1..28: mol_type = other DNA
tgtccttgtcggcctgcagttcctgggg

SEQ ID NO: 40864 - DNA, 28 bp, synthetic construct
  source 1..28: mol_type = other DNA
tttccccaggaactgcaggccgacaagg

SEQ ID NO: 40865 - DNA, 28 bp, synthetic construct
  source 1..28: mol_type = other DNA
atgtactcttttccccaggaactgcagg

SEQ ID NO: 40866 - DNA, 28 bp, synthetic construct
  source 1..28: mol_type = other DNA
gtagctcagatgtactcttttccccagg

SEQ ID NO: 40867 - DNA, 28 bp, synthetic construct
  source 1..28: mol_type = other DNA
gctacttgtccaagcctctgtctgcagg

SEQ ID NO: 40868 - DNA, 28 bp, synthetic construct
  source 1..28: mol_type = other DNA
gtccaagcctctgtctgcaggtgacagg

SEQ ID NO: 40869 - DNA, 28 bp, synthetic construct
  source 1..28: mol_type = other DNA
aacctgtcacctgcagacagaggcttgg

SEQ ID NO: 40870 - DNA, 28 bp, synthetic construct
  source 1..28: mol_type = other DNA
gcctctgtctgcaggtgacaggttttgg

SEQ ID NO: 40871 - DNA, 28 bp, synthetic construct
  source 1..28: mol_type = other DNA
cctctgtctgcaggtgacaggttttggg

SEQ ID NO: 40872 - DNA, 28 bp, synthetic construct
  source 1..28: mol_type = other DNA
ctctgtctgcaggtgacaggttttgggg

SEQ ID NO: 40873 - DNA, 28 bp, synthetic construct
  source 1..28: mol_type = other DNA
tctgtctgcaggtgacaggttttggggg

SEQ ID NO: 40874 - DNA, 28 bp, synthetic construct
  source 1..28: mol_type = other DNA
agatgcattaagtagaacatcatctcgg

SEQ ID NO: 40875 - DNA, 28 bp, synthetic construct
  source 1..28: mol_type = other DNA
gatgcattaagtagaacatcatctcggg

SEQ ID NO: 40876 - DNA, 28 bp, synthetic construct
  source 1..28: mol_type = other DNA
ggactggggcattggcaaacaaaagggg

SEQ ID NO: 40877 - DNA, 28 bp, synthetic construct
  source 1..28: mol_type = other DNA
aggactggggcattggcaaacaaaaggg

SEQ ID NO: 40878 - DNA, 28 bp, synthetic construct
  source 1..28: mol_type = other DNA
taggactggggcattggcaaacaaaagg

SEQ ID NO: 40879 - DNA, 28 bp, synthetic construct
  source 1..28: mol_type = other DNA
ggacaagtctctaggactggggcattgg

SEQ ID NO: 40880 - DNA, 28 bp, synthetic construct
  source 1..28: mol_type = other DNA
ctgtcaggacaagtctctaggactgggg

SEQ ID NO: 40881 - DNA, 28 bp, synthetic construct
  source 1..28: mol_type = other DNA
actgtcaggacaagtctctaggactggg

SEQ ID NO: 40882 - DNA, 28 bp, synthetic construct
  source 1..28: mol_type = other DNA
cactgtcaggacaagtctctaggactgg

SEQ ID NO: 40883 - DNA, 28 bp, synthetic construct
  source 1..28: mol_type = other DNA
tgcggcactgtcaggacaagtctctagg

SEQ ID NO: 40884 - DNA, 28 bp, synthetic construct
  source 1..28: mol_type = other DNA
tcaaaagtaggtgtgcggcactgtcagg

SEQ ID NO: 40885 - DNA, 28 bp, synthetic construct
  source 1..28: mol_type = other DNA
ctctgagagatcaaaagtaggtgtgcgg

SEQ ID NO: 40886 - DNA, 28 bp, synthetic construct
  source 1..28: mol_type = other DNA
acacctacttttgatctctcagagcagg

SEQ ID NO: 40887 - DNA, 28 bp, synthetic construct
  source 1..28: mol_type = other DNA
cctacttttgatctctcagagcaggtgg

SEQ ID NO: 40888 - DNA, 28 bp, synthetic construct
  source 1..28: mol_type = other DNA
aggtggctccatccccagactagcctgg

SEQ ID NO: 40889 - DNA, 28 bp, synthetic construct
  source 1..28: mol_type = other DNA
gagagcagccaggctagtctggggatgg

SEQ ID NO: 40890 - DNA, 28 bp, synthetic construct
  source 1..28: mol_type = other DNA
ctcggagagcagccaggctagtctgggg

SEQ ID NO: 40891 - DNA, 28 bp, synthetic construct
  source 1..28: mol_type = other DNA
cctcggagagcagccaggctagtctggg

SEQ ID NO: 40892 - DNA, 28 bp, synthetic construct
  source 1..28: mol_type = other DNA
gcctcggagagcagccaggctagtctgg

SEQ ID NO: 40893 - DNA, 28 bp, synthetic construct
  source 1..28: mol_type = other DNA
ggtggaggggcctcggagagcagccagg

SEQ ID NO: 40894 - DNA, 28 bp, synthetic construct
  source 1..28: mol_type = other DNA
ataaggggagcaggtggaggggcctcgg

SEQ ID NO: 40895 - DNA, 28 bp, synthetic construct
  source 1..28: mol_type = other DNA
ggggcaataaggggagcaggtggagggg

SEQ ID NO: 40896 - DNA, 28 bp, synthetic construct
  source 1..28: mol_type = other DNA
tggggcaataaggggagcaggtggaggg

SEQ ID NO: 40897 - DNA, 28 bp, synthetic construct
  source 1..28: mol_type = other DNA
atggggcaataaggggagcaggtggagg

SEQ ID NO: 40898 - DNA, 28 bp, synthetic construct
  source 1..28: mol_type = other DNA
agaatggggcaataaggggagcaggtgg

SEQ ID NO: 40899 - DNA, 28 bp, synthetic construct
  source 1..28: mol_type = other DNA
acaagaatggggcaataaggggagcagg

SEQ ID NO: 40900 - DNA, 28 bp, synthetic construct
  source 1..28: mol_type = other DNA
tgctccccttattgccccattcttgtgg

SEQ ID NO: 40901 - DNA, 28 bp, synthetic construct
  source 1..28: mol_type = other DNA
caagccacaagaatggggcaataagggg

SEQ ID NO: 40902 - DNA, 28 bp, synthetic construct
  source 1..28: mol_type = other DNA
gcaagccacaagaatggggcaataaggg

SEQ ID NO: 40903 - DNA, 28 bp, synthetic construct
  source 1..28: mol_type = other DNA
ggcaagccacaagaatggggcaataagg

SEQ ID NO: 40904 - DNA, 28 bp, synthetic construct
  source 1..28: mol_type = other DNA
ttattgccccattcttgtggcttgccgg

SEQ ID NO: 40905 - DNA, 28 bp, synthetic construct
  source 1..28: mol_type = other DNA
tattgccccattcttgtggcttgccggg

SEQ ID NO: 40906 - DNA, 28 bp, synthetic construct
  source 1..28: mol_type = other DNA
agtggcccggcaagccacaagaatgggg

SEQ ID NO: 40907 - DNA, 28 bp, synthetic construct
  source 1..28: mol_type = other DNA
aagtggcccggcaagccacaagaatggg

SEQ ID NO: 40908 - DNA, 28 bp, synthetic construct
  source 1..28: mol_type = other DNA
caagtggcccggcaagccacaagaatgg

SEQ ID NO: 40909 - DNA, 28 bp, synthetic construct
  source 1..28: mol_type = other DNA
cattcttgtggcttgccgggccacttgg

SEQ ID NO: 40910 - DNA, 28 bp, synthetic construct
  source 1..28: mol_type = other DNA
cggcaagaagggaggccaagtggcccgg

SEQ ID NO: 40911 - DNA, 28 bp, synthetic construct
  source 1..28: mol_type = other DNA
cgggccacttggcctcccttcttgccgg

SEQ ID NO: 40912 - DNA, 28 bp, synthetic construct
  source 1..28: mol_type = other DNA
gtcaccggcaagaagggaggccaagtgg

SEQ ID NO: 40913 - DNA, 28 bp, synthetic construct
  source 1..28: mol_type = other DNA
ggaacgctgtcaccggcaagaagggagg

SEQ ID NO: 40914 - DNA, 28 bp, synthetic construct
  source 1..28: mol_type = other DNA
gatggaacgctgtcaccggcaagaaggg

SEQ ID NO: 40915 - DNA, 28 bp, synthetic construct
  source 1..28: mol_type = other DNA
tgatggaacgctgtcaccggcaagaagg

SEQ ID NO: 40916 - DNA, 28 bp, synthetic construct
  source 1..28: mol_type = other DNA
cggggagatgatggaacgctgtcaccgg

SEQ ID NO: 40917 - DNA, 28 bp, synthetic construct
  source 1..28: mol_type = other DNA
cgttccatcatctccccgctccccaagg

SEQ ID NO: 40918 - DNA, 28 bp, synthetic construct
  source 1..28: mol_type = other DNA
gttccatcatctccccgctccccaaggg

SEQ ID NO: 40919 - DNA, 28 bp, synthetic construct
  source 1..28: mol_type = other DNA
tggcccttggggagcggggagatgatgg

SEQ ID NO: 40920 - DNA, 28 bp, synthetic construct
  source 1..28: mol_type = other DNA
agaagcagttggcccttggggagcgggg

SEQ ID NO: 40921 - DNA, 28 bp, synthetic construct
  source 1..28: mol_type = other DNA
gagaagcagttggcccttggggagcggg

SEQ ID NO: 40922 - DNA, 28 bp, synthetic construct
  source 1..28: mol_type = other DNA
tgagaagcagttggcccttggggagcgg

SEQ ID NO: 40923 - DNA, 28 bp, synthetic construct
  source 1..28: mol_type = other DNA
ctgagtgagaagcagttggcccttgggg

SEQ ID NO: 40924 - DNA, 28 bp, synthetic construct
  source 1..28: mol_type = other DNA
cccaagggccaactgcttctcactcagg

SEQ ID NO: 40925 - DNA, 28 bp, synthetic construct
  source 1..28: mol_type = other DNA
gcctgagtgagaagcagttggcccttgg

SEQ ID NO: 40926 - DNA, 28 bp, synthetic construct
  source 1..28: mol_type = other DNA
agggccaactgcttctcactcaggctgg

SEQ ID NO: 40927 - DNA, 28 bp, synthetic construct
  source 1..28: mol_type = other DNA
gacaccagcctgagtgagaagcagttgg

SEQ ID NO: 40928 - DNA, 28 bp, synthetic construct
  source 1..28: mol_type = other DNA
ttctcactcaggctggtgtcatttcagg

SEQ ID NO: 40929 - DNA, 28 bp, synthetic construct
  source 1..28: mol_type = other DNA
tcactcaggctggtgtcatttcaggagg

SEQ ID NO: 40930 - DNA, 28 bp, synthetic construct
  source 1..28: mol_type = other DNA
aaaataaaaaggctcacgcaggctttgg

SEQ ID NO: 40931 - DNA, 28 bp, synthetic construct
  source 1..28: mol_type = other DNA
ttactgaaaataaaaaggctcacgcagg

SEQ ID NO: 40932 - DNA, 28 bp, synthetic construct
  source 1..28: mol_type = other DNA
gtgagcctttttattttcagtaaaatgg

SEQ ID NO: 40933 - DNA, 28 bp, synthetic construct
  source 1..28: mol_type = other DNA
aagcaccattttactgaaaataaaaagg

SEQ ID NO: 40934 - DNA, 28 bp, synthetic construct
  source 1..28: mol_type = other DNA
tatttatatatagtatctcgaagtaagg

SEQ ID NO: 40935 - DNA, 28 bp, synthetic construct
  source 1..28: mol_type = other DNA
ataatgtaaatgacaccttttcgtacgg

SEQ ID NO: 40936 - DNA, 28 bp, synthetic construct
  source 1..28: mol_type = other DNA
aatactcaaacagctccgtacgaaaagg

SEQ ID NO: 40937 - DNA, 28 bp, synthetic construct
  source 1..28: mol_type = other DNA
tcagcttcaacaatcttgagctctgtgg

SEQ ID NO: 40938 - DNA, 28 bp, synthetic construct
  source 1..28: mol_type = other DNA
tctgtggctcctcaccctgtctgcatgg

SEQ ID NO: 40939 - DNA, 28 bp, synthetic construct
  source 1..28: mol_type = other DNA
caaggtcttccatgcagacagggtgagg

SEQ ID NO: 40940 - DNA, 28 bp, synthetic construct
  source 1..28: mol_type = other DNA
accctgtctgcatggaagaccttgctgg

SEQ ID NO: 40941 - DNA, 28 bp, synthetic construct
  source 1..28: mol_type = other DNA
tccagcaaggtcttccatgcagacaggg

SEQ ID NO: 40942 - DNA, 28 bp, synthetic construct
  source 1..28: mol_type = other DNA
gtccagcaaggtcttccatgcagacagg

SEQ ID NO: 40943 - DNA, 28 bp, synthetic construct
  source 1..28: mol_type = other DNA
catggaagaccttgctggacgctctcgg

SEQ ID NO: 40944 - DNA, 28 bp, synthetic construct
  source 1..28: mol_type = other DNA
atggaagaccttgctggacgctctcggg

SEQ ID NO: 40945 - DNA, 28 bp, synthetic construct
  source 1..28: mol_type = other DNA
tctgctctcccgagagcgtccagcaagg

SEQ ID NO: 40946 - DNA, 28 bp, synthetic construct
  source 1..28: mol_type = other DNA
gagcagacatagcaccagaagccactgg

SEQ ID NO: 40947 - DNA, 28 bp, synthetic construct
  source 1..28: mol_type = other DNA
agcagacatagcaccagaagccactggg

SEQ ID NO: 40948 - DNA, 28 bp, synthetic construct
  source 1..28: mol_type = other DNA
cgaaaacacttctcccagtggcttctgg

SEQ ID NO: 40949 - DNA, 28 bp, synthetic construct
  source 1..28: mol_type = other DNA
cacggatcgaaaacacttctcccagtgg

SEQ ID NO: 40950 - DNA, 28 bp, synthetic construct
  source 1..28: mol_type = other DNA
gggagaagtgttttcgatccgtgtctgg

SEQ ID NO: 40951 - DNA, 28 bp, synthetic construct
  source 1..28: mol_type = other DNA
ggagaagtgttttcgatccgtgtctggg

SEQ ID NO: 40952 - DNA, 28 bp, synthetic construct
  source 1..28: mol_type = other DNA
agtgaatactactgtggcccagacacgg

SEQ ID NO: 40953 - DNA, 28 bp, synthetic construct
  source 1..28: mol_type = other DNA
aaagactaaacagtgaatactactgtgg

SEQ ID NO: 40954 - DNA, 28 bp, synthetic construct
  source 1..28: mol_type = other DNA
aagaaatgtatgaagagactgcttacgg

SEQ ID NO: 40955 - DNA, 28 bp, synthetic construct
  source 1..28: mol_type = other DNA
gtctcttcatacatttcttacagtctgg

SEQ ID NO: 40956 - DNA, 28 bp, synthetic construct
  source 1..28: mol_type = other DNA
agcaaattgaaatactctttcttttagg

SEQ ID NO: 40957 - DNA, 28 bp, synthetic construct
  source 1..28: mol_type = other DNA
ctctttcttttaggtagcgtcacagtgg

SEQ ID NO: 40958 - DNA, 28 bp, synthetic construct
  source 1..28: mol_type = other DNA
cgtcacagtggttttttttttcctcagg

SEQ ID NO: 40959 - DNA, 28 bp, synthetic construct
  source 1..28: mol_type = other DNA
aggaaattgtatagaaattatcctgagg

SEQ ID NO: 40960 - DNA, 28 bp, synthetic construct
  source 1..28: mol_type = other DNA
ttctatacaatttccttactgtcagagg

SEQ ID NO: 40961 - DNA, 28 bp, synthetic construct
  source 1..28: mol_type = other DNA
tctatacaatttccttactgtcagaggg

SEQ ID NO: 40962 - DNA, 28 bp, synthetic construct
  source 1..28: mol_type = other DNA
gaaagatctggtccctctgacagtaagg

SEQ ID NO: 40963 - DNA, 28 bp, synthetic construct
  source 1..28: mol_type = other DNA
gagggaccagatctttccctcactgtgg

SEQ ID NO: 40964 - DNA, 28 bp, synthetic construct
  source 1..28: mol_type = other DNA
gaccagatctttccctcactgtggcagg

SEQ ID NO: 40965 - DNA, 28 bp, synthetic construct
  source 1..28: mol_type = other DNA
accagatctttccctcactgtggcaggg

SEQ ID NO: 40966 - DNA, 28 bp, synthetic construct
  source 1..28: mol_type = other DNA
ccagatctttccctcactgtggcagggg

SEQ ID NO: 40967 - DNA, 28 bp, synthetic construct
  source 1..28: mol_type = other DNA
tccctcactgtggcaggggccgtgcagg

SEQ ID NO: 40968 - DNA, 28 bp, synthetic construct
  source 1..28: mol_type = other DNA
acctgcacggcccctgccacagtgaggg

SEQ ID NO: 40969 - DNA, 28 bp, synthetic construct
  source 1..28: mol_type = other DNA
cacctgcacggcccctgccacagtgagg

SEQ ID NO: 40970 - DNA, 28 bp, synthetic construct
  source 1..28: mol_type = other DNA
ctcactgtggcaggggccgtgcaggtgg

SEQ ID NO: 40971 - DNA, 28 bp, synthetic construct
  source 1..28: mol_type = other DNA
tggcaggggccgtgcaggtggataaagg

SEQ ID NO: 40972 - DNA, 28 bp, synthetic construct
  source 1..28: mol_type = other DNA
ccagctcttcctttatccacctgcacgg

SEQ ID NO: 40973 - DNA, 28 bp, synthetic construct
  source 1..28: mol_type = other DNA
ggtggataaaggaagagctggtttccgg

SEQ ID NO: 40974 - DNA, 28 bp, synthetic construct
  source 1..28: mol_type = other DNA
agtcaacgctgttacagtcactctccgg

SEQ ID NO: 40975 - DNA, 28 bp, synthetic construct
  source 1..28: mol_type = other DNA
aacagcgttgactcgaagctagagatgg

SEQ ID NO: 40976 - DNA, 28 bp, synthetic construct
  source 1..28: mol_type = other DNA
agcgttgactcgaagctagagatggagg

SEQ ID NO: 40977 - DNA, 28 bp, synthetic construct
  source 1..28: mol_type = other DNA
gcgttgactcgaagctagagatggaggg

SEQ ID NO: 40978 - DNA, 28 bp, synthetic construct
  source 1..28: mol_type = other DNA
cgttgactcgaagctagagatggagggg

SEQ ID NO: 40979 - DNA, 28 bp, synthetic construct
  source 1..28: mol_type = other DNA
gttgactcgaagctagagatggaggggg

SEQ ID NO: 40980 - DNA, 28 bp, synthetic construct
  source 1..28: mol_type = other DNA
gactcgaagctagagatggagggggtgg

SEQ ID NO: 40981 - DNA, 28 bp, synthetic construct
  source 1..28: mol_type = other DNA
gagggggtggccgtctcttagacattgg

SEQ ID NO: 40982 - DNA, 28 bp, synthetic construct
  source 1..28: mol_type = other DNA
tgagaggtgtccaatgtctaagagacgg

SEQ ID NO: 40983 - DNA, 28 bp, synthetic construct
  source 1..28: mol_type = other DNA
attggacacctctcagagcctcctgagg

SEQ ID NO: 40984 - DNA, 28 bp, synthetic construct
  source 1..28: mol_type = other DNA
ttggacacctctcagagcctcctgaggg

SEQ ID NO: 40985 - DNA, 28 bp, synthetic construct
  source 1..28: mol_type = other DNA
aaagaagccctcaggaggctctgagagg

SEQ ID NO: 40986 - DNA, 28 bp, synthetic construct
  source 1..28: mol_type = other DNA
tctagaagacaaagaagccctcaggagg

SEQ ID NO: 40987 - DNA, 28 bp, synthetic construct
  source 1..28: mol_type = other DNA
gattctagaagacaaagaagccctcagg

SEQ ID NO: 40988 - DNA, 28 bp, synthetic construct
  source 1..28: mol_type = other DNA
cttctttgtcttctagaatctctaccgg

SEQ ID NO: 40989 - DNA, 28 bp, synthetic construct
  source 1..28: mol_type = other DNA
ctttgtcttctagaatctctaccggtgg

SEQ ID NO: 40990 - DNA, 28 bp, synthetic construct
  source 1..28: mol_type = other DNA
gaatctctaccggtggtcctcctgcagg

SEQ ID NO: 40991 - DNA, 28 bp, synthetic construct
  source 1..28: mol_type = other DNA
ctaccggtggtcctcctgcaggttctgg

SEQ ID NO: 40992 - DNA, 28 bp, synthetic construct
  source 1..28: mol_type = other DNA
gagccagaacctgcaggaggaccaccgg

SEQ ID NO: 40993 - DNA, 28 bp, synthetic construct
  source 1..28: mol_type = other DNA
atgtctgtgagccagaacctgcaggagg

SEQ ID NO: 40994 - DNA, 28 bp, synthetic construct
  source 1..28: mol_type = other DNA
atgatgtctgtgagccagaacctgcagg

SEQ ID NO: 40995 - DNA, 28 bp, synthetic construct
  source 1..28: mol_type = other DNA
catcatgcctttttttccctccctgagg

SEQ ID NO: 40996 - DNA, 28 bp, synthetic construct
  source 1..28: mol_type = other DNA
caaggcgcctcagggagggaaaaaaagg

SEQ ID NO: 40997 - DNA, 28 bp, synthetic construct
  source 1..28: mol_type = other DNA
ctttttttccctccctgaggcgccttgg

SEQ ID NO: 40998 - DNA, 28 bp, synthetic construct
  source 1..28: mol_type = other DNA
ctcttctgccaaggcgcctcagggaggg

SEQ ID NO: 40999 - DNA, 28 bp, synthetic construct
  source 1..28: mol_type = other DNA
gctcttctgccaaggcgcctcagggagg

SEQ ID NO: 41000 - DNA, 28 bp, synthetic construct
  source 1..28: mol_type = other DNA
cacgctcttctgccaaggcgcctcaggg

SEQ ID NO: 41001 - DNA, 28 bp, synthetic construct
  source 1..28: mol_type = other DNA
tcacgctcttctgccaaggcgcctcagg

SEQ ID NO: 41002 - DNA, 28 bp, synthetic construct
  source 1..28: mol_type = other DNA
ctcacagggtcacgctcttctgccaagg

SEQ ID NO: 41003 - DNA, 28 bp, synthetic construct
  source 1..28: mol_type = other DNA
gcagaagagcgtgaccctgtgagccagg

SEQ ID NO: 41004 - DNA, 28 bp, synthetic construct
  source 1..28: mol_type = other DNA
agagctaaggggggcctggctcacaggg

SEQ ID NO: 41005 - DNA, 28 bp, synthetic construct
  source 1..28: mol_type = other DNA
cagagctaaggggggcctggctcacagg

SEQ ID NO: 41006 - DNA, 28 bp, synthetic construct
  source 1..28: mol_type = other DNA
atctgaagcagagctaaggggggcctgg

SEQ ID NO: 41007 - DNA, 28 bp, synthetic construct
  source 1..28: mol_type = other DNA
ctgtgatctgaagcagagctaagggggg

SEQ ID NO: 41008 - DNA, 28 bp, synthetic construct
  source 1..28: mol_type = other DNA
tctgtgatctgaagcagagctaaggggg

SEQ ID NO: 41009 - DNA, 28 bp, synthetic construct
  source 1..28: mol_type = other DNA
ttctgtgatctgaagcagagctaagggg

SEQ ID NO: 41010 - DNA, 28 bp, synthetic construct
  source 1..28: mol_type = other DNA
gttctgtgatctgaagcagagctaaggg

SEQ ID NO: 41011 - DNA, 28 bp, synthetic construct
  source 1..28: mol_type = other DNA
tgttctgtgatctgaagcagagctaagg

SEQ ID NO: 41012 - DNA, 28 bp, synthetic construct
  source 1..28: mol_type = other DNA
gaacacagacagactcgcgagttgctgg

SEQ ID NO: 41013 - DNA, 28 bp, synthetic construct
  source 1..28: mol_type = other DNA
agactcgcgagttgctggacctctttgg

SEQ ID NO: 41014 - DNA, 28 bp, synthetic construct
  source 1..28: mol_type = other DNA
tggattcaaacacttaataccaaagagg

SEQ ID NO: 41015 - DNA, 28 bp, synthetic construct
  source 1..28: mol_type = other DNA
ctttggtattaagtgtttgaatccatgg

SEQ ID NO: 41016 - DNA, 28 bp, synthetic construct
  source 1..28: mol_type = other DNA
tggtattaagtgtttgaatccatggtgg

SEQ ID NO: 41017 - DNA, 28 bp, synthetic construct
  source 1..28: mol_type = other DNA
ggtattaagtgtttgaatccatggtggg

SEQ ID NO: 41018 - DNA, 28 bp, synthetic construct
  source 1..28: mol_type = other DNA
aacgctacttgcaaaaggcccaccatgg

SEQ ID NO: 41019 - DNA, 28 bp, synthetic construct
  source 1..28: mol_type = other DNA
aaaaagagctaacgctacttgcaaaagg

SEQ ID NO: 41020 - DNA, 28 bp, synthetic construct
  source 1..28: mol_type = other DNA
tctttttaaatgttgaactgagctaagg

SEQ ID NO: 41021 - DNA, 28 bp, synthetic construct
  source 1..28: mol_type = other DNA
actgagctaaggatgcactttcttgtgg

SEQ ID NO: 41022 - DNA, 28 bp, synthetic construct
  source 1..28: mol_type = other DNA
ggatgcactttcttgtggacatagaagg

SEQ ID NO: 41023 - DNA, 28 bp, synthetic construct
  source 1..28: mol_type = other DNA
gatgcactttcttgtggacatagaaggg

SEQ ID NO: 41024 - DNA, 28 bp, synthetic construct
  source 1..28: mol_type = other DNA
atgcactttcttgtggacatagaagggg

SEQ ID NO: 41025 - DNA, 28 bp, synthetic construct
  source 1..28: mol_type = other DNA
tgtggacatagaaggggcccacgtaagg

SEQ ID NO: 41026 - DNA, 28 bp, synthetic construct
  source 1..28: mol_type = other DNA
aaggggcccacgtaaggccctgagtagg

SEQ ID NO: 41027 - DNA, 28 bp, synthetic construct
  source 1..28: mol_type = other DNA
aaggagcctactcagggccttacgtggg

SEQ ID NO: 41028 - DNA, 28 bp, synthetic construct
  source 1..28: mol_type = other DNA
taaggagcctactcagggccttacgtgg

SEQ ID NO: 41029 - DNA, 28 bp, synthetic construct
  source 1..28: mol_type = other DNA
aagcagcaactaaggagcctactcaggg

SEQ ID NO: 41030 - DNA, 28 bp, synthetic construct
  source 1..28: mol_type = other DNA
aaagcagcaactaaggagcctactcagg

SEQ ID NO: 41031 - DNA, 28 bp, synthetic construct
  source 1..28: mol_type = other DNA
tccttagttgctgctttacctgatgagg

SEQ ID NO: 41032 - DNA, 28 bp, synthetic construct
  source 1..28: mol_type = other DNA
ccctcatcaggtaaagcagcaactaagg

SEQ ID NO: 41033 - DNA, 28 bp, synthetic construct
  source 1..28: mol_type = other DNA
agagttaatctctttggccctcatcagg

SEQ ID NO: 41034 - DNA, 28 bp, synthetic construct
  source 1..28: mol_type = other DNA
ggcaacgaggcagagttaatctctttgg

SEQ ID NO: 41035 - DNA, 28 bp, synthetic construct
  source 1..28: mol_type = other DNA
gcaacttttctgagacatggcaacgagg

SEQ ID NO: 41036 - DNA, 28 bp, synthetic construct
  source 1..28: mol_type = other DNA
gaaatatggcaacttttctgagacatgg

SEQ ID NO: 41037 - DNA, 28 bp, synthetic construct
  source 1..28: mol_type = other DNA
gaaaagttgccatatttcacccagaagg

SEQ ID NO: 41038 - DNA, 28 bp, synthetic construct
  source 1..28: mol_type = other DNA
aaaagttgccatatttcacccagaaggg

SEQ ID NO: 41039 - DNA, 28 bp, synthetic construct
  source 1..28: mol_type = other DNA
aaagttgccatatttcacccagaagggg

SEQ ID NO: 41040 - DNA, 28 bp, synthetic construct
  source 1..28: mol_type = other DNA
aaacaagccccttctgggtgaaatatgg

SEQ ID NO: 41041 - DNA, 28 bp, synthetic construct
  source 1..28: mol_type = other DNA
agtaagaggaaaacaagccccttctggg

SEQ ID NO: 41042 - DNA, 28 bp, synthetic construct
  source 1..28: mol_type = other DNA
gagtaagaggaaaacaagccccttctgg

SEQ ID NO: 41043 - DNA, 28 bp, synthetic construct
  source 1..28: mol_type = other DNA
ggcacatggttaaagtaagagtaagagg

SEQ ID NO: 41044 - DNA, 28 bp, synthetic construct
  source 1..28: mol_type = other DNA
cttactcttactttaaccatgtgcctgg

SEQ ID NO: 41045 - DNA, 28 bp, synthetic construct
  source 1..28: mol_type = other DNA
actcttactttaaccatgtgcctggagg

SEQ ID NO: 41046 - DNA, 28 bp, synthetic construct
  source 1..28: mol_type = other DNA
aaccatgtgcctggaggagccattctgg

SEQ ID NO: 41047 - DNA, 28 bp, synthetic construct
  source 1..28: mol_type = other DNA
accatgtgcctggaggagccattctggg

SEQ ID NO: 41048 - DNA, 28 bp, synthetic construct
  source 1..28: mol_type = other DNA
gcccagaatggctcctccaggcacatgg

SEQ ID NO: 41049 - DNA, 28 bp, synthetic construct
  source 1..28: mol_type = other DNA
tgcaagagcccagaatggctcctccagg

SEQ ID NO: 41050 - DNA, 28 bp, synthetic construct
  source 1..28: mol_type = other DNA
gctgggcaagtgcaagagcccagaatgg

SEQ ID NO: 41051 - DNA, 28 bp, synthetic construct
  source 1..28: mol_type = other DNA
tgcacttgcccagcctttctttgccagg

SEQ ID NO: 41052 - DNA, 28 bp, synthetic construct
  source 1..28: mol_type = other DNA
gcacttgcccagcctttctttgccaggg

SEQ ID NO: 41053 - DNA, 28 bp, synthetic construct
  source 1..28: mol_type = other DNA
cacttgcccagcctttctttgccagggg

SEQ ID NO: 41054 - DNA, 28 bp, synthetic construct
  source 1..28: mol_type = other DNA
tctctgcccctggcaaagaaaggctggg

SEQ ID NO: 41055 - DNA, 28 bp, synthetic construct
  source 1..28: mol_type = other DNA
ttctctgcccctggcaaagaaaggctgg

SEQ ID NO: 41056 - DNA, 28 bp, synthetic construct
  source 1..28: mol_type = other DNA
agcctttctttgccaggggcagagaagg

SEQ ID NO: 41057 - DNA, 28 bp, synthetic construct
  source 1..28: mol_type = other DNA
gcctttctttgccaggggcagagaaggg

SEQ ID NO: 41058 - DNA, 28 bp, synthetic construct
  source 1..28: mol_type = other DNA
tcccttctctgcccctggcaaagaaagg

SEQ ID NO: 41059 - DNA, 28 bp, synthetic construct
  source 1..28: mol_type = other DNA
tctttgccaggggcagagaagggaaagg

SEQ ID NO: 41060 - DNA, 28 bp, synthetic construct
  source 1..28: mol_type = other DNA
ctttgccaggggcagagaagggaaaggg

SEQ ID NO: 41061 - DNA, 28 bp, synthetic construct
  source 1..28: mol_type = other DNA
tttgccaggggcagagaagggaaagggg

SEQ ID NO: 41062 - DNA, 28 bp, synthetic construct
  source 1..28: mol_type = other DNA
ttgccaggggcagagaagggaaaggggg

SEQ ID NO: 41063 - DNA, 28 bp, synthetic construct
  source 1..28: mol_type = other DNA
ctaccccctttcccttctctgcccctgg

SEQ ID NO: 41064 - DNA, 28 bp, synthetic construct
  source 1..28: mol_type = other DNA
gaaagggggtagattgagtgtgccaagg

SEQ ID NO: 41065 - DNA, 28 bp, synthetic construct
  source 1..28: mol_type = other DNA
aaagggggtagattgagtgtgccaaggg

SEQ ID NO: 41066 - DNA, 28 bp, synthetic construct
  source 1..28: mol_type = other DNA
gattgagtgtgccaagggccgtgcaagg

SEQ ID NO: 41067 - DNA, 28 bp, synthetic construct
  source 1..28: mol_type = other DNA
attgagtgtgccaagggccgtgcaaggg

SEQ ID NO: 41068 - DNA, 28 bp, synthetic construct
  source 1..28: mol_type = other DNA
agtgtgccaagggccgtgcaagggcagg

SEQ ID NO: 41069 - DNA, 28 bp, synthetic construct
  source 1..28: mol_type = other DNA
agcaagcctgcccttgcacggcccttgg

SEQ ID NO: 41070 - DNA, 28 bp, synthetic construct
  source 1..28: mol_type = other DNA
ggtggaaagcaagcctgcccttgcacgg

SEQ ID NO: 41071 - DNA, 28 bp, synthetic construct
  source 1..28: mol_type = other DNA
aggcttgctttccacccatctgctgagg

SEQ ID NO: 41072 - DNA, 28 bp, synthetic construct
  source 1..28: mol_type = other DNA
ggcttgctttccacccatctgctgaggg

SEQ ID NO: 41073 - DNA, 28 bp, synthetic construct
  source 1..28: mol_type = other DNA
ggagagggctccctcagcagatgggtgg

SEQ ID NO: 41074 - DNA, 28 bp, synthetic construct
  source 1..28: mol_type = other DNA
agaggagagggctccctcagcagatggg

SEQ ID NO: 41075 - DNA, 28 bp, synthetic construct
  source 1..28: mol_type = other DNA
gagaggagagggctccctcagcagatgg

SEQ ID NO: 41076 - DNA, 28 bp, synthetic construct
  source 1..28: mol_type = other DNA
aacagaggcaaggagcgagaggagaggg

SEQ ID NO: 41077 - DNA, 28 bp, synthetic construct
  source 1..28: mol_type = other DNA
gaacagaggcaaggagcgagaggagagg

SEQ ID NO: 41078 - DNA, 28 bp, synthetic construct
  source 1..28: mol_type = other DNA
ggtgtgaacagaggcaaggagcgagagg

SEQ ID NO: 41079 - DNA, 28 bp, synthetic construct
  source 1..28: mol_type = other DNA
aagacaacaggtgtgaacagaggcaagg

SEQ ID NO: 41080 - DNA, 28 bp, synthetic construct
  source 1..28: mol_type = other DNA
ttgcctctgttcacacctgttgtcttgg

SEQ ID NO: 41081 - DNA, 28 bp, synthetic construct
  source 1..28: mol_type = other DNA
cttccaagacaacaggtgtgaacagagg

SEQ ID NO: 41082 - DNA, 28 bp, synthetic construct
  source 1..28: mol_type = other DNA
ctgttcacacctgttgtcttggaagagg

SEQ ID NO: 41083 - DNA, 28 bp, synthetic construct
  source 1..28: mol_type = other DNA
tcacacctgttgtcttggaagaggatgg

SEQ ID NO: 41084 - DNA, 28 bp, synthetic construct
  source 1..28: mol_type = other DNA
agggaccatcctcttccaagacaacagg

SEQ ID NO: 41085 - DNA, 28 bp, synthetic construct
  source 1..28: mol_type = other DNA
ggaagaggatggtccctttgtcttaagg

SEQ ID NO: 41086 - DNA, 28 bp, synthetic construct
  source 1..28: mol_type = other DNA
ctttatcacaaagccttaagacaaaggg

SEQ ID NO: 41087 - DNA, 28 bp, synthetic construct
  source 1..28: mol_type = other DNA
actttatcacaaagccttaagacaaagg

SEQ ID NO: 41088 - DNA, 28 bp, synthetic construct
  source 1..28: mol_type = other DNA
ctttgtgataaagtcatctccagttagg

SEQ ID NO: 41089 - DNA, 28 bp, synthetic construct
  source 1..28: mol_type = other DNA
gaaggaaacaggtgcagatcctaactgg

SEQ ID NO: 41090 - DNA, 28 bp, synthetic construct
  source 1..28: mol_type = other DNA
cacctgtttccttcgtaatagtgcctgg

SEQ ID NO: 41091 - DNA, 28 bp, synthetic construct
  source 1..28: mol_type = other DNA
cgccaggcactattacgaaggaaacagg

SEQ ID NO: 41092 - DNA, 28 bp, synthetic construct
  source 1..28: mol_type = other DNA
ctgtttccttcgtaatagtgcctggcgg

SEQ ID NO: 41093 - DNA, 28 bp, synthetic construct
  source 1..28: mol_type = other DNA
gaaaggccgccaggcactattacgaagg

SEQ ID NO: 41094 - DNA, 28 bp, synthetic construct
  source 1..28: mol_type = other DNA
tgcctggcggcctttctgaagttacagg

SEQ ID NO: 41095 - DNA, 28 bp, synthetic construct
  source 1..28: mol_type = other DNA
cacctgtaacttcagaaaggccgccagg

SEQ ID NO: 41096 - DNA, 28 bp, synthetic construct
  source 1..28: mol_type = other DNA
ctggcggcctttctgaagttacaggtgg

SEQ ID NO: 41097 - DNA, 28 bp, synthetic construct
  source 1..28: mol_type = other DNA
cggcctttctgaagttacaggtggttgg

SEQ ID NO: 41098 - DNA, 28 bp, synthetic construct
  source 1..28: mol_type = other DNA
ggcctttctgaagttacaggtggttggg

SEQ ID NO: 41099 - DNA, 28 bp, synthetic construct
  source 1..28: mol_type = other DNA
ctcccaaccacctgtaacttcagaaagg

SEQ ID NO: 41100 - DNA, 28 bp, synthetic construct
  source 1..28: mol_type = other DNA
ggagccctctcgcatgcagaacatctgg

SEQ ID NO: 41101 - DNA, 28 bp, synthetic construct
  source 1..28: mol_type = other DNA
tctaccagatgttctgcatgcgagaggg

SEQ ID NO: 41102 - DNA, 28 bp, synthetic construct
  source 1..28: mol_type = other DNA
atctaccagatgttctgcatgcgagagg

SEQ ID NO: 41103 - DNA, 28 bp, synthetic construct
  source 1..28: mol_type = other DNA
agaacatctggtagattgatctgccagg

SEQ ID NO: 41104 - DNA, 28 bp, synthetic construct
  source 1..28: mol_type = other DNA
catctggtagattgatctgccaggctgg

SEQ ID NO: 41105 - DNA, 28 bp, synthetic construct
  source 1..28: mol_type = other DNA
atctggtagattgatctgccaggctggg

SEQ ID NO: 41106 - DNA, 28 bp, synthetic construct
  source 1..28: mol_type = other DNA
tggtagattgatctgccaggctgggtgg

SEQ ID NO: 41107 - DNA, 28 bp, synthetic construct
  source 1..28: mol_type = other DNA
gagaaagcagtagaaccacccagcctgg

SEQ ID NO: 41108 - DNA, 28 bp, synthetic construct
  source 1..28: mol_type = other DNA
agcagaactctttaagaaaaaaaaaagg

SEQ ID NO: 41109 - DNA, 28 bp, synthetic construct
  source 1..28: mol_type = other DNA
tatttgtaagtaccatgtttccttgtgg

SEQ ID NO: 41110 - DNA, 28 bp, synthetic construct
  source 1..28: mol_type = other DNA
acagagcatacaccacaaggaaacatgg

SEQ ID NO: 41111 - DNA, 28 bp, synthetic construct
  source 1..28: mol_type = other DNA
tttccttgtggtgtatgctctgttctgg

SEQ ID NO: 41112 - DNA, 28 bp, synthetic construct
  source 1..28: mol_type = other DNA
aaaccagaacagagcatacaccacaagg

SEQ ID NO: 41113 - DNA, 28 bp, synthetic construct
  source 1..28: mol_type = other DNA
tctgttttcaaatcaaatgcctgtttgg

SEQ ID NO: 41114 - DNA, 28 bp, synthetic construct
  source 1..28: mol_type = other DNA
ctgttttcaaatcaaatgcctgtttggg

SEQ ID NO: 41115 - DNA, 28 bp, synthetic construct
  source 1..28: mol_type = other DNA
ttttcaaatcaaatgcctgtttgggagg

SEQ ID NO: 41116 - DNA, 28 bp, synthetic construct
  source 1..28: mol_type = other DNA
taaatacgttcatctcctcccaaacagg

SEQ ID NO: 41117 - DNA, 28 bp, synthetic construct
  source 1..28: mol_type = other DNA
atttagtctattagatttgcactgctgg

SEQ ID NO: 41118 - DNA, 28 bp, synthetic construct
  source 1..28: mol_type = other DNA
ggataaacaataagacagctattcaagg

SEQ ID NO: 41119 - DNA, 28 bp, synthetic construct
  source 1..28: mol_type = other DNA
actttaatcgattgactaatcttacagg

SEQ ID NO: 41120 - DNA, 28 bp, synthetic construct
  source 1..28: mol_type = other DNA
acagcttggactcactcaagtaaacagg

SEQ ID NO: 41121 - DNA, 28 bp, synthetic construct
  source 1..28: mol_type = other DNA
cagcttggactcactcaagtaaacaggg

SEQ ID NO: 41122 - DNA, 28 bp, synthetic construct
  source 1..28: mol_type = other DNA
agcttggactcactcaagtaaacagggg

SEQ ID NO: 41123 - DNA, 28 bp, synthetic construct
  source 1..28: mol_type = other DNA
tcactcaagtaaacaggggctttattgg

SEQ ID NO: 41124 - DNA, 28 bp, synthetic construct
  source 1..28: mol_type = other DNA
caggggctttattggcttatagacctgg

SEQ ID NO: 41125 - DNA, 28 bp, synthetic construct
  source 1..28: mol_type = other DNA
aggggctttattggcttatagacctggg

SEQ ID NO: 41126 - DNA, 28 bp, synthetic construct
  source 1..28: mol_type = other DNA
attggcttatagacctgggcagtccagg

SEQ ID NO: 41127 - DNA, 28 bp, synthetic construct
  source 1..28: mol_type = other DNA
gacctgggcagtccaggtgtagatctgg

SEQ ID NO: 41128 - DNA, 28 bp, synthetic construct
  source 1..28: mol_type = other DNA
aaccagatctacacctggactgcccagg

SEQ ID NO: 41129 - DNA, 28 bp, synthetic construct
  source 1..28: mol_type = other DNA
ccaggtgtagatctggttccagacaagg

SEQ ID NO: 41130 - DNA, 28 bp, synthetic construct
  source 1..28: mol_type = other DNA
gtggagtctctgaatcagccttgtctgg

SEQ ID NO: 41131 - DNA, 28 bp, synthetic construct
  source 1..28: mol_type = other DNA
acaaggctgattcagagactccacgtgg

SEQ ID NO: 41132 - DNA, 28 bp, synthetic construct
  source 1..28: mol_type = other DNA
ctgattcagagactccacgtggtcaagg

SEQ ID NO: 41133 - DNA, 28 bp, synthetic construct
  source 1..28: mol_type = other DNA
gacaaacaacagagccttgaccacgtgg

SEQ ID NO: 41134 - DNA, 28 bp, synthetic construct
  source 1..28: mol_type = other DNA
aaggctctgttgtttgtcaatcccttgg

SEQ ID NO: 41135 - DNA, 28 bp, synthetic construct
  source 1..28: mol_type = other DNA
tcccttggctcctccacttccagtttgg

SEQ ID NO: 41136 - DNA, 28 bp, synthetic construct
  source 1..28: mol_type = other DNA
gccaaactggaagtggaggagccaaggg

SEQ ID NO: 41137 - DNA, 28 bp, synthetic construct
  source 1..28: mol_type = other DNA
agccaaactggaagtggaggagccaagg

SEQ ID NO: 41138 - DNA, 28 bp, synthetic construct
  source 1..28: mol_type = other DNA
aggacagaagccaaactggaagtggagg

SEQ ID NO: 41139 - DNA, 28 bp, synthetic construct
  source 1..28: mol_type = other DNA
gtgaggacagaagccaaactggaagtgg

SEQ ID NO: 41140 - DNA, 28 bp, synthetic construct
  source 1..28: mol_type = other DNA
gagactgtgaggacagaagccaaactgg

SEQ ID NO: 41141 - DNA, 28 bp, synthetic construct
  source 1..28: mol_type = other DNA
tctgtcctcacagtctctctccatgtgg

SEQ ID NO: 41142 - DNA, 28 bp, synthetic construct
  source 1..28: mol_type = other DNA
gtttgccacatggagagagactgtgagg

SEQ ID NO: 41143 - DNA, 28 bp, synthetic construct
  source 1..28: mol_type = other DNA
gtctctctccatgtggcaaacaagatgg

SEQ ID NO: 41144 - DNA, 28 bp, synthetic construct
  source 1..28: mol_type = other DNA
tccatgtggcaaacaagatggctactgg

SEQ ID NO: 41145 - DNA, 28 bp, synthetic construct
  source 1..28: mol_type = other DNA
accagtagccatcttgtttgccacatgg

SEQ ID NO: 41146 - DNA, 28 bp, synthetic construct
  source 1..28: mol_type = other DNA
atgtggcaaacaagatggctactggtgg

SEQ ID NO: 41147 - DNA, 28 bp, synthetic construct
  source 1..28: mol_type = other DNA
aaacaagatggctactggtggtcccagg

SEQ ID NO: 41148 - DNA, 28 bp, synthetic construct
  source 1..28: mol_type = other DNA
gtcccaggttcacgtcctctcagcttgg

SEQ ID NO: 41149 - DNA, 28 bp, synthetic construct
  source 1..28: mol_type = other DNA
ttccaagctgagaggacgtgaacctggg

SEQ ID NO: 41150 - DNA, 28 bp, synthetic construct
  source 1..28: mol_type = other DNA
tttccaagctgagaggacgtgaacctgg

SEQ ID NO: 41151 - DNA, 28 bp, synthetic construct
  source 1..28: mol_type = other DNA
cttgctgctggatttccaagctgagagg

SEQ ID NO: 41152 - DNA, 28 bp, synthetic construct
  source 1..28: mol_type = other DNA
tgggagtgagacatcttcttgctgctgg

SEQ ID NO: 41153 - DNA, 28 bp, synthetic construct
  source 1..28: mol_type = other DNA
ctcccaaagtccataactcaatccttgg

SEQ ID NO: 41154 - DNA, 28 bp, synthetic construct
  source 1..28: mol_type = other DNA
tcccaaagtccataactcaatccttggg

SEQ ID NO: 41155 - DNA, 28 bp, synthetic construct
  source 1..28: mol_type = other DNA
tcccaaggattgagttatggactttggg

SEQ ID NO: 41156 - DNA, 28 bp, synthetic construct
  source 1..28: mol_type = other DNA
ttcccaaggattgagttatggactttgg

SEQ ID NO: 41157 - DNA, 28 bp, synthetic construct
  source 1..28: mol_type = other DNA
tacagtcttcccaaggattgagttatgg

SEQ ID NO: 41158 - DNA, 28 bp, synthetic construct
  source 1..28: mol_type = other DNA
actcaatccttgggaagactgtagttgg

SEQ ID NO: 41159 - DNA, 28 bp, synthetic construct
  source 1..28: mol_type = other DNA
agcaggaccaactacagtcttcccaagg

SEQ ID NO: 41160 - DNA, 28 bp, synthetic construct
  source 1..28: mol_type = other DNA
tgggaagactgtagttggtcctgctagg

SEQ ID NO: 41161 - DNA, 28 bp, synthetic construct
  source 1..28: mol_type = other DNA
agttggatagttacgtgttcctagcagg

SEQ ID NO: 41162 - DNA, 28 bp, synthetic construct
  source 1..28: mol_type = other DNA
gtaactatccaactatcctccagatagg

SEQ ID NO: 41163 - DNA, 28 bp, synthetic construct
  source 1..28: mol_type = other DNA
taactatccaactatcctccagataggg

SEQ ID NO: 41164 - DNA, 28 bp, synthetic construct
  source 1..28: mol_type = other DNA
tccaactatcctccagatagggagctgg

SEQ ID NO: 41165 - DNA, 28 bp, synthetic construct
  source 1..28: mol_type = other DNA
ccaactatcctccagatagggagctggg

SEQ ID NO: 41166 - DNA, 28 bp, synthetic construct
  source 1..28: mol_type = other DNA
caactatcctccagatagggagctgggg

SEQ ID NO: 41167 - DNA, 28 bp, synthetic construct
  source 1..28: mol_type = other DNA
tcctccagatagggagctggggagatgg

SEQ ID NO: 41168 - DNA, 28 bp, synthetic construct
  source 1..28: mol_type = other DNA
cctccagatagggagctggggagatggg

SEQ ID NO: 41169 - DNA, 28 bp, synthetic construct
  source 1..28: mol_type = other DNA
tctcccatctccccagctccctatctgg

SEQ ID NO: 41170 - DNA, 28 bp, synthetic construct
  source 1..28: mol_type = other DNA
gatagggagctggggagatgggagatgg

SEQ ID NO: 41171 - DNA, 28 bp, synthetic construct
  source 1..28: mol_type = other DNA
atagggagctggggagatgggagatggg

SEQ ID NO: 41172 - DNA, 28 bp, synthetic construct
  source 1..28: mol_type = other DNA
gagatgggagatgggctcctctgacagg

SEQ ID NO: 41173 - DNA, 28 bp, synthetic construct
  source 1..28: mol_type = other DNA
tgggctcctctgacaggacaccctgtgg

SEQ ID NO: 41174 - DNA, 28 bp, synthetic construct
  source 1..28: mol_type = other DNA
cgtgaaccacagggtgtcctgtcagagg

SEQ ID NO: 41175 - DNA, 28 bp, synthetic construct
  source 1..28: mol_type = other DNA
accctgtggttcacgtccactcttgtgg

SEQ ID NO: 41176 - DNA, 28 bp, synthetic construct
  source 1..28: mol_type = other DNA
gccacaagagtggacgtgaaccacaggg

SEQ ID NO: 41177 - DNA, 28 bp, synthetic construct
  source 1..28: mol_type = other DNA
ggccacaagagtggacgtgaaccacagg

SEQ ID NO: 41178 - DNA, 28 bp, synthetic construct
  source 1..28: mol_type = other DNA
gtggttcacgtccactcttgtggcctgg

SEQ ID NO: 41179 - DNA, 28 bp, synthetic construct
  source 1..28: mol_type = other DNA
tggttcacgtccactcttgtggcctggg

SEQ ID NO: 41180 - DNA, 28 bp, synthetic construct
  source 1..28: mol_type = other DNA
gtccactcttgtggcctgggtatattgg

SEQ ID NO: 41181 - DNA, 28 bp, synthetic construct
  source 1..28: mol_type = other DNA
tccactcttgtggcctgggtatattggg

SEQ ID NO: 41182 - DNA, 28 bp, synthetic construct
  source 1..28: mol_type = other DNA
tcccaatatacccaggccacaagagtgg

SEQ ID NO: 41183 - DNA, 28 bp, synthetic construct
  source 1..28: mol_type = other DNA
ttgtggcctgggtatattgggaatgcgg

SEQ ID NO: 41184 - DNA, 28 bp, synthetic construct
  source 1..28: mol_type = other DNA
tgtggcctgggtatattgggaatgcggg

SEQ ID NO: 41185 - DNA, 28 bp, synthetic construct
  source 1..28: mol_type = other DNA
gtggcctgggtatattgggaatgcgggg

SEQ ID NO: 41186 - DNA, 28 bp, synthetic construct
  source 1..28: mol_type = other DNA
tcatccccgcattcccaatatacccagg

SEQ ID NO: 41187 - DNA, 28 bp, synthetic construct
  source 1..28: mol_type = other DNA
tgaagaaagaattcacagccccacaagg

SEQ ID NO: 41188 - DNA, 28 bp, synthetic construct
  source 1..28: mol_type = other DNA
aattcacagccccacaaggttcgtgtgg

SEQ ID NO: 41189 - DNA, 28 bp, synthetic construct
  source 1..28: mol_type = other DNA
cagccccacaaggttcgtgtggaaaagg

SEQ ID NO: 41190 - DNA, 28 bp, synthetic construct
  source 1..28: mol_type = other DNA
agccccacaaggttcgtgtggaaaaggg

SEQ ID NO: 41191 - DNA, 28 bp, synthetic construct
  source 1..28: mol_type = other DNA
gccccacaaggttcgtgtggaaaagggg

SEQ ID NO: 41192 - DNA, 28 bp, synthetic construct
  source 1..28: mol_type = other DNA
tccccttttccacacgaaccttgtgggg

SEQ ID NO: 41193 - DNA, 28 bp, synthetic construct
  source 1..28: mol_type = other DNA
ctccccttttccacacgaaccttgtggg

SEQ ID NO: 41194 - DNA, 28 bp, synthetic construct
  source 1..28: mol_type = other DNA
ccacaaggttcgtgtggaaaaggggagg

SEQ ID NO: 41195 - DNA, 28 bp, synthetic construct
  source 1..28: mol_type = other DNA
gctttcttaattttatggctcttctggg

SEQ ID NO: 41196 - DNA, 28 bp, synthetic construct
  source 1..28: mol_type = other DNA
tgctttcttaattttatggctcttctgg

SEQ ID NO: 41197 - DNA, 28 bp, synthetic construct
  source 1..28: mol_type = other DNA
tgcttgcagtgctttcttaattttatgg

SEQ ID NO: 41198 - DNA, 28 bp, synthetic construct
  source 1..28: mol_type = other DNA
aacaaaaaccagtcatttaagttcttgg

SEQ ID NO: 41199 - DNA, 28 bp, synthetic construct
  source 1..28: mol_type = other DNA
tgttactgccaagaacttaaatgactgg

SEQ ID NO: 41200 - DNA, 28 bp, synthetic construct
  source 1..28: mol_type = other DNA
ttatacctagtgcttcattttgctctgg

SEQ ID NO: 41201 - DNA, 28 bp, synthetic construct
  source 1..28: mol_type = other DNA
tttttccagagcaaaatgaagcactagg

SEQ ID NO: 41202 - DNA, 28 bp, synthetic construct
  source 1..28: mol_type = other DNA
tggaaaaaaagcagatctgctctgctgg

SEQ ID NO: 41203 - DNA, 28 bp, synthetic construct
  source 1..28: mol_type = other DNA
ggaaaaaaagcagatctgctctgctggg

SEQ ID NO: 41204 - DNA, 28 bp, synthetic construct
  source 1..28: mol_type = other DNA
gaaaaaaagcagatctgctctgctgggg

SEQ ID NO: 41205 - DNA, 28 bp, synthetic construct
  source 1..28: mol_type = other DNA
atctgctctgctggggcaattctaatgg

SEQ ID NO: 41206 - DNA, 28 bp, synthetic construct
  source 1..28: mol_type = other DNA
gcctttccagtgtgctttgagaaagtgg

SEQ ID NO: 41207 - DNA, 28 bp, synthetic construct
  source 1..28: mol_type = other DNA
tccactttctcaaagcacactggaaagg

SEQ ID NO: 41208 - DNA, 28 bp, synthetic construct
  source 1..28: mol_type = other DNA
tttccagtgtgctttgagaaagtggagg

SEQ ID NO: 41209 - DNA, 28 bp, synthetic construct
  source 1..28: mol_type = other DNA
ttccagtgtgctttgagaaagtggaggg

SEQ ID NO: 41210 - DNA, 28 bp, synthetic construct
  source 1..28: mol_type = other DNA
gtccctccactttctcaaagcacactgg

SEQ ID NO: 41211 - DNA, 28 bp, synthetic construct
  source 1..28: mol_type = other DNA
gctttgagaaagtggagggactgcgtgg

SEQ ID NO: 41212 - DNA, 28 bp, synthetic construct
  source 1..28: mol_type = other DNA
aagtggagggactgcgtggtattgctgg

SEQ ID NO: 41213 - DNA, 28 bp, synthetic construct
  source 1..28: mol_type = other DNA
agtggagggactgcgtggtattgctggg

SEQ ID NO: 41214 - DNA, 28 bp, synthetic construct
  source 1..28: mol_type = other DNA
gtggtattgctgggcttcccatttcagg

SEQ ID NO: 41215 - DNA, 28 bp, synthetic construct
  source 1..28: mol_type = other DNA
gctgggcttcccatttcaggagacctgg

SEQ ID NO: 41216 - DNA, 28 bp, synthetic construct
  source 1..28: mol_type = other DNA
ctgggcttcccatttcaggagacctggg

SEQ ID NO: 41217 - DNA, 28 bp, synthetic construct
  source 1..28: mol_type = other DNA
ctgctgggcccaggtctcctgaaatggg

SEQ ID NO: 41218 - DNA, 28 bp, synthetic construct
  source 1..28: mol_type = other DNA
actgctgggcccaggtctcctgaaatgg

SEQ ID NO: 41219 - DNA, 28 bp, synthetic construct
  source 1..28: mol_type = other DNA
atcatgtcatagaactgctgggcccagg

SEQ ID NO: 41220 - DNA, 28 bp, synthetic construct
  source 1..28: mol_type = other DNA
ctcatcatcatgtcatagaactgctggg

SEQ ID NO: 41221 - DNA, 28 bp, synthetic construct
  source 1..28: mol_type = other DNA
gctcatcatcatgtcatagaactgctgg

SEQ ID NO: 41222 - DNA, 28 bp, synthetic construct
  source 1..28: mol_type = other DNA
ttctatgacatgatgatgagcactctgg

SEQ ID NO: 41223 - DNA, 28 bp, synthetic construct
  source 1..28: mol_type = other DNA
gcactctggacccaaaccagacacctgg

SEQ ID NO: 41224 - DNA, 28 bp, synthetic construct
  source 1..28: mol_type = other DNA
aggacactggccaggtgtctggtttggg

SEQ ID NO: 41225 - DNA, 28 bp, synthetic construct
  source 1..28: mol_type = other DNA
caggacactggccaggtgtctggtttgg

SEQ ID NO: 41226 - DNA, 28 bp, synthetic construct
  source 1..28: mol_type = other DNA
agaatcaggacactggccaggtgtctgg

SEQ ID NO: 41227 - DNA, 28 bp, synthetic construct
  source 1..28: mol_type = other DNA
cagtctcagaatcaggacactggccagg

SEQ ID NO: 41228 - DNA, 28 bp, synthetic construct
  source 1..28: mol_type = other DNA
ctcttcagtctcagaatcaggacactgg

SEQ ID NO: 41229 - DNA, 28 bp, synthetic construct
  source 1..28: mol_type = other DNA
cacagggctcttcagtctcagaatcagg

SEQ ID NO: 41230 - DNA, 28 bp, synthetic construct
  source 1..28: mol_type = other DNA
ctgagactgaagagccctgtgaatgtgg

SEQ ID NO: 41231 - DNA, 28 bp, synthetic construct
  source 1..28: mol_type = other DNA
tgagactgaagagccctgtgaatgtggg

SEQ ID NO: 41232 - DNA, 28 bp, synthetic construct
  source 1..28: mol_type = other DNA
caggagggcattgcccacattcacaggg

SEQ ID NO: 41233 - DNA, 28 bp, synthetic construct
  source 1..28: mol_type = other DNA
gcaggagggcattgcccacattcacagg

SEQ ID NO: 41234 - DNA, 28 bp, synthetic construct
  source 1..28: mol_type = other DNA
atgtgggcaatgccctcctgctttctgg

SEQ ID NO: 41235 - DNA, 28 bp, synthetic construct
  source 1..28: mol_type = other DNA
tgtgggcaatgccctcctgctttctggg

SEQ ID NO: 41236 - DNA, 28 bp, synthetic construct
  source 1..28: mol_type = other DNA
gtgggcaatgccctcctgctttctgggg

SEQ ID NO: 41237 - DNA, 28 bp, synthetic construct
  source 1..28: mol_type = other DNA
tgggcaatgccctcctgctttctggggg

SEQ ID NO: 41238 - DNA, 28 bp, synthetic construct
  source 1..28: mol_type = other DNA
atgccctcctgctttctgggggtcatgg

SEQ ID NO: 41239 - DNA, 28 bp, synthetic construct
  source 1..28: mol_type = other DNA
tgccctcctgctttctgggggtcatggg

SEQ ID NO: 41240 - DNA, 28 bp, synthetic construct
  source 1..28: mol_type = other DNA
cacccatgacccccagaaagcaggaggg

SEQ ID NO: 41241 - DNA, 28 bp, synthetic construct
  source 1..28: mol_type = other DNA
ccacccatgacccccagaaagcaggagg

SEQ ID NO: 41242 - DNA, 28 bp, synthetic construct
  source 1..28: mol_type = other DNA
ctcctgctttctgggggtcatgggtggg

SEQ ID NO: 41243 - DNA, 28 bp, synthetic construct
  source 1..28: mol_type = other DNA
tcctgctttctgggggtcatgggtgggg

SEQ ID NO: 41244 - DNA, 28 bp, synthetic construct
  source 1..28: mol_type = other DNA
tccccacccatgacccccagaaagcagg

SEQ ID NO: 41245 - DNA, 28 bp, synthetic construct
  source 1..28: mol_type = other DNA
aaaactcataaggcaagagctgagaagg

SEQ ID NO: 41246 - DNA, 28 bp, synthetic construct
  source 1..28: mol_type = other DNA
gaaatgatgttataaaaaactcataagg

SEQ ID NO: 41247 - DNA, 28 bp, synthetic construct
  source 1..28: mol_type = other DNA
tttttataacatcatttctcctttctgg

SEQ ID NO: 41248 - DNA, 28 bp, synthetic construct
  source 1..28: mol_type = other DNA
ttttataacatcatttctcctttctggg

SEQ ID NO: 41249 - DNA, 28 bp, synthetic construct
  source 1..28: mol_type = other DNA
tagatgagaaaactaacacccagaaagg

SEQ ID NO: 41250 - DNA, 28 bp, synthetic construct
  source 1..28: mol_type = other DNA
gggtgttagttttctcatctatgtgagg

SEQ ID NO: 41251 - DNA, 28 bp, synthetic construct
  source 1..28: mol_type = other DNA
tttttatttcaagttggacagatcttgg

SEQ ID NO: 41252 - DNA, 28 bp, synthetic construct
  source 1..28: mol_type = other DNA
ttttgttttcatttttatttcaagttgg

SEQ ID NO: 41253 - DNA, 28 bp, synthetic construct
  source 1..28: mol_type = other DNA
aaaacacctcaaattctgattcttttgg

SEQ ID NO: 41254 - DNA, 28 bp, synthetic construct
  source 1..28: mol_type = other DNA
aacggtccaaaagaatcagaatttgagg

SEQ ID NO: 41255 - DNA, 28 bp, synthetic construct
  source 1..28: mol_type = other DNA
ggagctcgttaactatgctgggaaacgg

SEQ ID NO: 41256 - DNA, 28 bp, synthetic construct
  source 1..28: mol_type = other DNA
ggtctgggagctcgttaactatgctggg

SEQ ID NO: 41257 - DNA, 28 bp, synthetic construct
  source 1..28: mol_type = other DNA
tggtctgggagctcgttaactatgctgg

SEQ ID NO: 41258 - DNA, 28 bp, synthetic construct
  source 1..28: mol_type = other DNA
agaatggaggtaaagtgtctggtctggg

SEQ ID NO: 41259 - DNA, 28 bp, synthetic construct
  source 1..28: mol_type = other DNA
gagaatggaggtaaagtgtctggtctgg

SEQ ID NO: 41260 - DNA, 28 bp, synthetic construct
  source 1..28: mol_type = other DNA
gaccagacactttacctccattctcagg

SEQ ID NO: 41261 - DNA, 28 bp, synthetic construct
  source 1..28: mol_type = other DNA
cgcctgagaatggaggtaaagtgtctgg

SEQ ID NO: 41262 - DNA, 28 bp, synthetic construct
  source 1..28: mol_type = other DNA
actttacctccattctcaggcgctgagg

SEQ ID NO: 41263 - DNA, 28 bp, synthetic construct
  source 1..28: mol_type = other DNA
ttacctccattctcaggcgctgaggagg

SEQ ID NO: 41264 - DNA, 28 bp, synthetic construct
  source 1..28: mol_type = other DNA
tacctccattctcaggcgctgaggaggg

SEQ ID NO: 41265 - DNA, 28 bp, synthetic construct
  source 1..28: mol_type = other DNA
caccctcctcagcgcctgagaatggagg

SEQ ID NO: 41266 - DNA, 28 bp, synthetic construct
  source 1..28: mol_type = other DNA
ctccattctcaggcgctgaggagggtgg

SEQ ID NO: 41267 - DNA, 28 bp, synthetic construct
  source 1..28: mol_type = other DNA
ctccaccctcctcagcgcctgagaatgg

SEQ ID NO: 41268 - DNA, 28 bp, synthetic construct
  source 1..28: mol_type = other DNA
tctcaggcgctgaggagggtggagcagg

SEQ ID NO: 41269 - DNA, 28 bp, synthetic construct
  source 1..28: mol_type = other DNA
ggtggagcaggcctgcaatgcatatagg

SEQ ID NO: 41270 - DNA, 28 bp, synthetic construct
  source 1..28: mol_type = other DNA
gtggagcaggcctgcaatgcatataggg

SEQ ID NO: 41271 - DNA, 28 bp, synthetic construct
  source 1..28: mol_type = other DNA
tggagcaggcctgcaatgcatatagggg

SEQ ID NO: 41272 - DNA, 28 bp, synthetic construct
  source 1..28: mol_type = other DNA
gcctgcaatgcatataggggaacaaagg

SEQ ID NO: 41273 - DNA, 28 bp, synthetic construct
  source 1..28: mol_type = other DNA
gcctttgttcccctatatgcattgcagg

SEQ ID NO: 41274 - DNA, 28 bp, synthetic construct
  source 1..28: mol_type = other DNA
gaacaaaggcccagagacagagacgtgg

SEQ ID NO: 41275 - DNA, 28 bp, synthetic construct
  source 1..28: mol_type = other DNA
aacaaaggcccagagacagagacgtggg

SEQ ID NO: 41276 - DNA, 28 bp, synthetic construct
  source 1..28: mol_type = other DNA
gcatggttcccacgtctctgtctctggg

SEQ ID NO: 41277 - DNA, 28 bp, synthetic construct
  source 1..28: mol_type = other DNA
tgcatggttcccacgtctctgtctctgg

SEQ ID NO: 41278 - DNA, 28 bp, synthetic construct
  source 1..28: mol_type = other DNA
gtgggaaccatgcagtgtaaaaaagcgg

SEQ ID NO: 41279 - DNA, 28 bp, synthetic construct
  source 1..28: mol_type = other DNA
tgggaaccatgcagtgtaaaaaagcggg

SEQ ID NO: 41280 - DNA, 28 bp, synthetic construct
  source 1..28: mol_type = other DNA
gaaccatgcagtgtaaaaaagcgggagg

SEQ ID NO: 41281 - DNA, 28 bp, synthetic construct
  source 1..28: mol_type = other DNA
gtacctcccgcttttttacactgcatgg

SEQ ID NO: 41282 - DNA, 28 bp, synthetic construct
  source 1..28: mol_type = other DNA
gcgggaggtaccagagacagagacgtgg

SEQ ID NO: 41283 - DNA, 28 bp, synthetic construct
  source 1..28: mol_type = other DNA
cgggaggtaccagagacagagacgtggg

SEQ ID NO: 41284 - DNA, 28 bp, synthetic construct
  source 1..28: mol_type = other DNA
gggaggtaccagagacagagacgtgggg

SEQ ID NO: 41285 - DNA, 28 bp, synthetic construct
  source 1..28: mol_type = other DNA
cgcatgggccccacgtctctgtctctgg

SEQ ID NO: 41286 - DNA, 28 bp, synthetic construct
  source 1..28: mol_type = other DNA
cagagacagagacgtggggcccatgcgg

SEQ ID NO: 41287 - DNA, 28 bp, synthetic construct
  source 1..28: mol_type = other DNA
gtggggcccatgcggtgtaaaaaaccgg

SEQ ID NO: 41288 - DNA, 28 bp, synthetic construct
  source 1..28: mol_type = other DNA
tggggcccatgcggtgtaaaaaaccggg

SEQ ID NO: 41289 - DNA, 28 bp, synthetic construct
  source 1..28: mol_type = other DNA
ggcccatgcggtgtaaaaaaccgggagg

SEQ ID NO: 41290 - DNA, 28 bp, synthetic construct
  source 1..28: mol_type = other DNA
tacctcccggttttttacaccgcatggg

SEQ ID NO: 41291 - DNA, 28 bp, synthetic construct
  source 1..28: mol_type = other DNA
gtacctcccggttttttacaccgcatgg

SEQ ID NO: 41292 - DNA, 28 bp, synthetic construct
  source 1..28: mol_type = other DNA
gtgtaaaaaaccgggaggtaccttcagg

SEQ ID NO: 41293 - DNA, 28 bp, synthetic construct
  source 1..28: mol_type = other DNA
agctgtgggtcctgaaggtacctcccgg

SEQ ID NO: 41294 - DNA, 28 bp, synthetic construct
  source 1..28: mol_type = other DNA
gggaggtaccttcaggacccacagctgg

SEQ ID NO: 41295 - DNA, 28 bp, synthetic construct
  source 1..28: mol_type = other DNA
ggaggtaccttcaggacccacagctggg

SEQ ID NO: 41296 - DNA, 28 bp, synthetic construct
  source 1..28: mol_type = other DNA
cctgaggcccagctgtgggtcctgaagg

SEQ ID NO: 41297 - DNA, 28 bp, synthetic construct
  source 1..28: mol_type = other DNA
cttcaggacccacagctgggcctcaggg

SEQ ID NO: 41298 - DNA, 28 bp, synthetic construct
  source 1..28: mol_type = other DNA
agctgtggccctgaggcccagctgtggg

SEQ ID NO: 41299 - DNA, 28 bp, synthetic construct
  source 1..28: mol_type = other DNA
cagctgtggccctgaggcccagctgtgg

SEQ ID NO: 41300 - DNA, 28 bp, synthetic construct
  source 1..28: mol_type = other DNA
cacagctgggcctcagggccacagctgg

SEQ ID NO: 41301 - DNA, 28 bp, synthetic construct
  source 1..28: mol_type = other DNA
acagctgggcctcagggccacagctggg

SEQ ID NO: 41302 - DNA, 28 bp, synthetic construct
  source 1..28: mol_type = other DNA
cagctgggcctcagggccacagctgggg

SEQ ID NO: 41303 - DNA, 28 bp, synthetic construct
  source 1..28: mol_type = other DNA
gggcctcagggccacagctggggtttgg

SEQ ID NO: 41304 - DNA, 28 bp, synthetic construct
  source 1..28: mol_type = other DNA
tcaccaaaccccagctgtggccctgagg

SEQ ID NO: 41305 - DNA, 28 bp, synthetic construct
  source 1..28: mol_type = other DNA
cgaagtgttcaccaaaccccagctgtgg

SEQ ID NO: 41306 - DNA, 28 bp, synthetic construct
  source 1..28: mol_type = other DNA
ggcgggcactgaagtatgaagtgcaagg

SEQ ID NO: 41307 - DNA, 28 bp, synthetic construct
  source 1..28: mol_type = other DNA
ttcatacttcagtgcccgccagttcagg

SEQ ID NO: 41308 - DNA, 28 bp, synthetic construct
  source 1..28: mol_type = other DNA
tcagtgcccgccagttcaggacattagg

SEQ ID NO: 41309 - DNA, 28 bp, synthetic construct
  source 1..28: mol_type = other DNA
ttcagtcctaatgtcctgaactggcggg

SEQ ID NO: 41310 - DNA, 28 bp, synthetic construct
  source 1..28: mol_type = other DNA
cttcagtcctaatgtcctgaactggcgg

SEQ ID NO: 41311 - DNA, 28 bp, synthetic construct
  source 1..28: mol_type = other DNA
cgccagttcaggacattaggactgaagg

SEQ ID NO: 41312 - DNA, 28 bp, synthetic construct
  source 1..28: mol_type = other DNA
gccagttcaggacattaggactgaaggg

SEQ ID NO: 41313 - DNA, 28 bp, synthetic construct
  source 1..28: mol_type = other DNA
gcccttcagtcctaatgtcctgaactgg

SEQ ID NO: 41314 - DNA, 28 bp, synthetic construct
  source 1..28: mol_type = other DNA
ggactgaagggcccgccaagatagatgg

SEQ ID NO: 41315 - DNA, 28 bp, synthetic construct
  source 1..28: mol_type = other DNA
tgagattaacaccatctatcttggcggg

SEQ ID NO: 41316 - DNA, 28 bp, synthetic construct
  source 1..28: mol_type = other DNA
atgagattaacaccatctatcttggcgg

SEQ ID NO: 41317 - DNA, 28 bp, synthetic construct
  source 1..28: mol_type = other DNA
cagatgagattaacaccatctatcttgg

SEQ ID NO: 41318 - DNA, 28 bp, synthetic construct
  source 1..28: mol_type = other DNA
caagatagatggtgttaatctcatctgg

SEQ ID NO: 41319 - DNA, 28 bp, synthetic construct
  source 1..28: mol_type = other DNA
ggagacattggaaatgtgaacatgtggg

SEQ ID NO: 41320 - DNA, 28 bp, synthetic construct
  source 1..28: mol_type = other DNA
gggagacattggaaatgtgaacatgtgg

SEQ ID NO: 41321 - DNA, 28 bp, synthetic construct
  source 1..28: mol_type = other DNA
gttcacatttccaatgtctcccaccagg

SEQ ID NO: 41322 - DNA, 28 bp, synthetic construct
  source 1..28: mol_type = other DNA
ttcacatttccaatgtctcccaccaggg

SEQ ID NO: 41323 - DNA, 28 bp, synthetic construct
  source 1..28: mol_type = other DNA
atttccaatgtctcccaccagggactgg

SEQ ID NO: 41324 - DNA, 28 bp, synthetic construct
  source 1..28: mol_type = other DNA
gaagccagtccctggtgggagacattgg

SEQ ID NO: 41325 - DNA, 28 bp, synthetic construct
  source 1..28: mol_type = other DNA
actttgaaggaagccagtccctggtggg

SEQ ID NO: 41326 - DNA, 28 bp, synthetic construct
  source 1..28: mol_type = other DNA
aactttgaaggaagccagtccctggtgg

SEQ ID NO: 41327 - DNA, 28 bp, synthetic construct
  source 1..28: mol_type = other DNA
gggaactttgaaggaagccagtccctgg

SEQ ID NO: 41328 - DNA, 28 bp, synthetic construct
  source 1..28: mol_type = other DNA
tggcttccttcaaagttcccaccgaagg

SEQ ID NO: 41329 - DNA, 28 bp, synthetic construct
  source 1..28: mol_type = other DNA
aggattccttcggtgggaactttgaagg

SEQ ID NO: 41330 - DNA, 28 bp, synthetic construct
  source 1..28: mol_type = other DNA
ggggcaggagcaggattccttcggtggg

SEQ ID NO: 41331 - DNA, 28 bp, synthetic construct
  source 1..28: mol_type = other DNA
tggggcaggagcaggattccttcggtgg

SEQ ID NO: 41332 - DNA, 28 bp, synthetic construct
  source 1..28: mol_type = other DNA
tcttggggcaggagcaggattccttcgg

SEQ ID NO: 41333 - DNA, 28 bp, synthetic construct
  source 1..28: mol_type = other DNA
gcaagcatcatcttggggcaggagcagg

SEQ ID NO: 41334 - DNA, 28 bp, synthetic construct
  source 1..28: mol_type = other DNA
gcagaagcaagcatcatcttggggcagg

SEQ ID NO: 41335 - DNA, 28 bp, synthetic construct
  source 1..28: mol_type = other DNA
gggggcagaagcaagcatcatcttgggg

SEQ ID NO: 41336 - DNA, 28 bp, synthetic construct
  source 1..28: mol_type = other DNA
tgggggcagaagcaagcatcatcttggg

SEQ ID NO: 41337 - DNA, 28 bp, synthetic construct
  source 1..28: mol_type = other DNA
gtgggggcagaagcaagcatcatcttgg

SEQ ID NO: 41338 - DNA, 28 bp, synthetic construct
  source 1..28: mol_type = other DNA
agtctgaagaagggatacactgtggggg

SEQ ID NO: 41339 - DNA, 28 bp, synthetic construct
  source 1..28: mol_type = other DNA
gagtctgaagaagggatacactgtgggg

SEQ ID NO: 41340 - DNA, 28 bp, synthetic construct
  source 1..28: mol_type = other DNA
agagtctgaagaagggatacactgtggg

SEQ ID NO: 41341 - DNA, 28 bp, synthetic construct
  source 1..28: mol_type = other DNA
aagagtctgaagaagggatacactgtgg

SEQ ID NO: 41342 - DNA, 28 bp, synthetic construct
  source 1..28: mol_type = other DNA
cccttcttcagactcttcctcaccctgg

SEQ ID NO: 41343 - DNA, 28 bp, synthetic construct
  source 1..28: mol_type = other DNA
ccttcttcagactcttcctcaccctggg

SEQ ID NO: 41344 - DNA, 28 bp, synthetic construct
  source 1..28: mol_type = other DNA
ctgggtagatgggaagcccagggtgagg

SEQ ID NO: 41345 - DNA, 28 bp, synthetic construct
  source 1..28: mol_type = other DNA
gagttctgggtagatgggaagcccaggg

SEQ ID NO: 41346 - DNA, 28 bp, synthetic construct
  source 1..28: mol_type = other DNA
ggagttctgggtagatgggaagcccagg

SEQ ID NO: 41347 - DNA, 28 bp, synthetic construct
  source 1..28: mol_type = other DNA
agggatcgtggagttctgggtagatggg

SEQ ID NO: 41348 - DNA, 28 bp, synthetic construct
  source 1..28: mol_type = other DNA
cagggatcgtggagttctgggtagatgg

SEQ ID NO: 41349 - DNA, 28 bp, synthetic construct
  source 1..28: mol_type = other DNA
tctacccagaactccacgatccctgagg

SEQ ID NO: 41350 - DNA, 28 bp, synthetic construct
  source 1..28: mol_type = other DNA
acccagaactccacgatccctgaggcgg

SEQ ID NO: 41351 - DNA, 28 bp, synthetic construct
  source 1..28: mol_type = other DNA
tccgcctcagggatcgtggagttctggg

SEQ ID NO: 41352 - DNA, 28 bp, synthetic construct
  source 1..28: mol_type = other DNA
gtccgcctcagggatcgtggagttctgg

SEQ ID NO: 41353 - DNA, 28 bp, synthetic construct
  source 1..28: mol_type = other DNA
agctgggagtccgcctcagggatcgtgg

SEQ ID NO: 41354 - DNA, 28 bp, synthetic construct
  source 1..28: mol_type = other DNA
ttgtacaagctgggagtccgcctcaggg

SEQ ID NO: 41355 - DNA, 28 bp, synthetic construct
  source 1..28: mol_type = other DNA
tttgtacaagctgggagtccgcctcagg

SEQ ID NO: 41356 - DNA, 28 bp, synthetic construct
  source 1..28: mol_type = other DNA
actcccagcttgtacaaatgtgtactgg

SEQ ID NO: 41357 - DNA, 28 bp, synthetic construct
  source 1..28: mol_type = other DNA
gctccagtacacatttgtacaagctggg

SEQ ID NO: 41358 - DNA, 28 bp, synthetic construct
  source 1..28: mol_type = other DNA
agctccagtacacatttgtacaagctgg

SEQ ID NO: 41359 - DNA, 28 bp, synthetic construct
  source 1..28: mol_type = other DNA
tgtgtactggagctactgtgacttcagg

SEQ ID NO: 41360 - DNA, 28 bp, synthetic construct
  source 1..28: mol_type = other DNA
gtgggtgggtctgaaatattattcgagg

SEQ ID NO: 41361 - DNA, 28 bp, synthetic construct
  source 1..28: mol_type = other DNA
tataggatacagttttacagtgggtggg

SEQ ID NO: 41362 - DNA, 28 bp, synthetic construct
  source 1..28: mol_type = other DNA
atataggatacagttttacagtgggtgg

SEQ ID NO: 41363 - DNA, 28 bp, synthetic construct
  source 1..28: mol_type = other DNA
aggatataggatacagttttacagtggg

SEQ ID NO: 41364 - DNA, 28 bp, synthetic construct
  source 1..28: mol_type = other DNA
aaggatataggatacagttttacagtgg

SEQ ID NO: 41365 - DNA, 28 bp, synthetic construct
  source 1..28: mol_type = other DNA
ttctcatattttggtctaaggatatagg

SEQ ID NO: 41366 - DNA, 28 bp, synthetic construct
  source 1..28: mol_type = other DNA
aatgagattctcatattttggtctaagg

SEQ ID NO: 41367 - DNA, 28 bp, synthetic construct
  source 1..28: mol_type = other DNA
acaagacaatgagattctcatattttgg

SEQ ID NO: 41368 - DNA, 28 bp, synthetic construct
  source 1..28: mol_type = other DNA
atgagaatctcattgtcttgtctcttgg

SEQ ID NO: 41369 - DNA, 28 bp, synthetic construct
  source 1..28: mol_type = other DNA
agaatctcattgtcttgtctcttggtgg

SEQ ID NO: 41370 - DNA, 28 bp, synthetic construct
  source 1..28: mol_type = other DNA
ggcatacgagaaaatactgtacccacgg

SEQ ID NO: 41371 - DNA, 28 bp, synthetic construct
  source 1..28: mol_type = other DNA
gcatacgagaaaatactgtacccacggg

SEQ ID NO: 41372 - DNA, 28 bp, synthetic construct
  source 1..28: mol_type = other DNA
gagaaaatactgtacccacgggtcgagg

SEQ ID NO: 41373 - DNA, 28 bp, synthetic construct
  source 1..28: mol_type = other DNA
ctacacggaactgtcctcgacccgtggg

SEQ ID NO: 41374 - DNA, 28 bp, synthetic construct
  source 1..28: mol_type = other DNA
tctacacggaactgtcctcgacccgtgg

SEQ ID NO: 41375 - DNA, 28 bp, synthetic construct
  source 1..28: mol_type = other DNA
ggtcgaggacagttccgtgtagaagtgg

SEQ ID NO: 41376 - DNA, 28 bp, synthetic construct
  source 1..28: mol_type = other DNA
cgaggacagttccgtgtagaagtggagg

SEQ ID NO: 41377 - DNA, 28 bp, synthetic construct
  source 1..28: mol_type = other DNA
ttcactgtgtgcctccacttctacacgg

SEQ ID NO: 41378 - DNA, 28 bp, synthetic construct
  source 1..28: mol_type = other DNA
gtgtagaagtggaggcacacagtgaagg

SEQ ID NO: 41379 - DNA, 28 bp, synthetic construct
  source 1..28: mol_type = other DNA
ggaggcacacagtgaaggctttgagagg

SEQ ID NO: 41380 - DNA, 28 bp, synthetic construct
  source 1..28: mol_type = other DNA
tgaaggctttgagaggcttcgttaacgg

SEQ ID NO: 41381 - DNA, 28 bp, synthetic construct
  source 1..28: mol_type = other DNA
gagaggcttcgttaacggtgctttgagg

SEQ ID NO: 41382 - DNA, 28 bp, synthetic construct
  source 1..28: mol_type = other DNA
agaggcttcgttaacggtgctttgaggg

SEQ ID NO: 41383 - DNA, 28 bp, synthetic construct
  source 1..28: mol_type = other DNA
gttaacggtgctttgagggatacatagg

SEQ ID NO: 41384 - DNA, 28 bp, synthetic construct
  source 1..28: mol_type = other DNA
gatacataggaagtatccgactctttgg

SEQ ID NO: 41385 - DNA, 28 bp, synthetic construct
  source 1..28: mol_type = other DNA
atacataggaagtatccgactctttggg

SEQ ID NO: 41386 - DNA, 28 bp, synthetic construct
  source 1..28: mol_type = other DNA
aaggcttttgtgtttcccaaagagtcgg

SEQ ID NO: 41387 - DNA, 28 bp, synthetic construct
  source 1..28: mol_type = other DNA
ttctggctcacagacatgtcgaggaagg

SEQ ID NO: 41388 - DNA, 28 bp, synthetic construct
  source 1..28: mol_type = other DNA
gtttttctggctcacagacatgtcgagg

SEQ ID NO: 41389 - DNA, 28 bp, synthetic construct
  source 1..28: mol_type = other DNA
agccagaaaaacaagcaaatgtgagagg

SEQ ID NO: 41390 - DNA, 28 bp, synthetic construct
  source 1..28: mol_type = other DNA
aacctctcacatttgcttgtttttctgg

SEQ ID NO: 41391 - DNA, 28 bp, synthetic construct
  source 1..28: mol_type = other DNA
atcttaaattctatacgtaagtgagggg

SEQ ID NO: 41392 - DNA, 28 bp, synthetic construct
  source 1..28: mol_type = other DNA
aatcttaaattctatacgtaagtgaggg

SEQ ID NO: 41393 - DNA, 28 bp, synthetic construct
  source 1..28: mol_type = other DNA
caatcttaaattctatacgtaagtgagg

SEQ ID NO: 41394 - DNA, 28 bp, synthetic construct
  source 1..28: mol_type = other DNA
tgtgtgtggtgtgtaactggagaagggg

SEQ ID NO: 41395 - DNA, 28 bp, synthetic construct
  source 1..28: mol_type = other DNA
aaaaaagactgtatgaacagaacagtgg

SEQ ID NO: 41396 - DNA, 28 bp, synthetic construct
  source 1..28: mol_type = other DNA
agatttgatctgaggtatgggggtgggg

SEQ ID NO: 41397 - DNA, 28 bp, synthetic construct
  source 1..28: mol_type = other DNA
gagatttgatctgaggtatgggggtggg

SEQ ID NO: 41398 - DNA, 28 bp, synthetic construct
  source 1..28: mol_type = other DNA
agagatttgatctgaggtatgggggtgg

SEQ ID NO: 41399 - DNA, 28 bp, synthetic construct
  source 1..28: mol_type = other DNA
gggagagatttgatctgaggtatggggg

SEQ ID NO: 41400 - DNA, 28 bp, synthetic construct
  source 1..28: mol_type = other DNA
tgggagagatttgatctgaggtatgggg

SEQ ID NO: 41401 - DNA, 28 bp, synthetic construct
  source 1..28: mol_type = other DNA
atgggagagatttgatctgaggtatggg

SEQ ID NO: 41402 - DNA, 28 bp, synthetic construct
  source 1..28: mol_type = other DNA
tatgggagagatttgatctgaggtatgg

SEQ ID NO: 41403 - DNA, 28 bp, synthetic construct
  source 1..28: mol_type = other DNA
caggctatgggagagatttgatctgagg

SEQ ID NO: 41404 - DNA, 28 bp, synthetic construct
  source 1..28: mol_type = other DNA
ctcagatcaaatctctcccatagcctgg

SEQ ID NO: 41405 - DNA, 28 bp, synthetic construct
  source 1..28: mol_type = other DNA
tcagatcaaatctctcccatagcctggg

SEQ ID NO: 41406 - DNA, 28 bp, synthetic construct
  source 1..28: mol_type = other DNA
cagatcaaatctctcccatagcctgggg

SEQ ID NO: 41407 - DNA, 28 bp, synthetic construct
  source 1..28: mol_type = other DNA
atcaaatctctcccatagcctggggtgg

SEQ ID NO: 41408 - DNA, 28 bp, synthetic construct
  source 1..28: mol_type = other DNA
acaggtaagggccaccccaggctatggg

SEQ ID NO: 41409 - DNA, 28 bp, synthetic construct
  source 1..28: mol_type = other DNA
gacaggtaagggccaccccaggctatgg

SEQ ID NO: 41410 - DNA, 28 bp, synthetic construct
  source 1..28: mol_type = other DNA
tagcctggggtggcccttacctgtctgg

SEQ ID NO: 41411 - DNA, 28 bp, synthetic construct
  source 1..28: mol_type = other DNA
tggccagacaggtaagggccaccccagg

SEQ ID NO: 41412 - DNA, 28 bp, synthetic construct
  source 1..28: mol_type = other DNA
ctcatgcttttggccagacaggtaaggg

SEQ ID NO: 41413 - DNA, 28 bp, synthetic construct
  source 1..28: mol_type = other DNA
tctcatgcttttggccagacaggtaagg

SEQ ID NO: 41414 - DNA, 28 bp, synthetic construct
  source 1..28: mol_type = other DNA
acctgtctggccaaaagcatgagagagg

SEQ ID NO: 41415 - DNA, 28 bp, synthetic construct
  source 1..28: mol_type = other DNA
gcctctctcatgcttttggccagacagg

SEQ ID NO: 41416 - DNA, 28 bp, synthetic construct
  source 1..28: mol_type = other DNA
gtctggccaaaagcatgagagaggctgg

SEQ ID NO: 41417 - DNA, 28 bp, synthetic construct
  source 1..28: mol_type = other DNA
tcttgaccagcctctctcatgcttttgg

SEQ ID NO: 41418 - DNA, 28 bp, synthetic construct
  source 1..28: mol_type = other DNA
accaagaaacacaacagcttctccatgg

SEQ ID NO: 41419 - DNA, 28 bp, synthetic construct
  source 1..28: mol_type = other DNA
accatggagaagctgttgtgtttcttgg

SEQ ID NO: 41420 - DNA, 28 bp, synthetic construct
  source 1..28: mol_type = other DNA
tatcactggcagcaggacgtgaccatgg

SEQ ID NO: 41421 - DNA, 28 bp, synthetic construct
  source 1..28: mol_type = other DNA
gtcacgtcctgctgccagtgatacaagg

SEQ ID NO: 41422 - DNA, 28 bp, synthetic construct
  source 1..28: mol_type = other DNA
tcacgtcctgctgccagtgatacaaggg

SEQ ID NO: 41423 - DNA, 28 bp, synthetic construct
  source 1..28: mol_type = other DNA
ttcaggcccttgtatcactggcagcagg

SEQ ID NO: 41424 - DNA, 28 bp, synthetic construct
  source 1..28: mol_type = other DNA
gagtgaattcaggcccttgtatcactgg

SEQ ID NO: 41425 - DNA, 28 bp, synthetic construct
  source 1..28: mol_type = other DNA
atacaagggcctgaattcactcctttgg

SEQ ID NO: 41426 - DNA, 28 bp, synthetic construct
  source 1..28: mol_type = other DNA
acatcttttccaaaggagtgaattcagg

SEQ ID NO: 41427 - DNA, 28 bp, synthetic construct
  source 1..28: mol_type = other DNA
ttcactcctttggaaaagatgtattcgg

SEQ ID NO: 41428 - DNA, 28 bp, synthetic construct
  source 1..28: mol_type = other DNA
tttcagccgaatacatcttttccaaagg

SEQ ID NO: 41429 - DNA, 28 bp, synthetic construct
  source 1..28: mol_type = other DNA
aaaagatgtattcggctgaaagttcagg

SEQ ID NO: 41430 - DNA, 28 bp, synthetic construct
  source 1..28: mol_type = other DNA
aaagatgtattcggctgaaagttcaggg

SEQ ID NO: 41431 - DNA, 28 bp, synthetic construct
  source 1..28: mol_type = other DNA
aagatgtattcggctgaaagttcagggg

SEQ ID NO: 41432 - DNA, 28 bp, synthetic construct
  source 1..28: mol_type = other DNA
gaggtagctctaaggcaagagatctagg

SEQ ID NO: 41433 - DNA, 28 bp, synthetic construct
  source 1..28: mol_type = other DNA
tgccttagagctacctcctcctgcctgg

SEQ ID NO: 41434 - DNA, 28 bp, synthetic construct
  source 1..28: mol_type = other DNA
atccaggcaggaggaggtagctctaagg

SEQ ID NO: 41435 - DNA, 28 bp, synthetic construct
  source 1..28: mol_type = other DNA
tttggatataaatccaggcaggaggagg

SEQ ID NO: 41436 - DNA, 28 bp, synthetic construct
  source 1..28: mol_type = other DNA
tgctttggatataaatccaggcaggagg

SEQ ID NO: 41437 - DNA, 28 bp, synthetic construct
  source 1..28: mol_type = other DNA
tactgctttggatataaatccaggcagg

SEQ ID NO: 41438 - DNA, 28 bp, synthetic construct
  source 1..28: mol_type = other DNA
gcctggatttatatccaaagcagtaagg

SEQ ID NO: 41439 - DNA, 28 bp, synthetic construct
  source 1..28: mol_type = other DNA
cccttactgctttggatataaatccagg

SEQ ID NO: 41440 - DNA, 28 bp, synthetic construct
  source 1..28: mol_type = other DNA
agtggcgcaaactcccttactgctttgg

SEQ ID NO: 41441 - DNA, 28 bp, synthetic construct
  source 1..28: mol_type = other DNA
caatgttggaaaattatttacatagtgg

SEQ ID NO: 41442 - DNA, 28 bp, synthetic construct
  source 1..28: mol_type = other DNA
taaataattttccaacattgcttgttgg

SEQ ID NO: 41443 - DNA, 28 bp, synthetic construct
  source 1..28: mol_type = other DNA
aaataattttccaacattgcttgttggg

SEQ ID NO: 41444 - DNA, 28 bp, synthetic construct
  source 1..28: mol_type = other DNA
aataattttccaacattgcttgttgggg

SEQ ID NO: 41445 - DNA, 28 bp, synthetic construct
  source 1..28: mol_type = other DNA
attttccaacattgcttgttggggcagg

SEQ ID NO: 41446 - DNA, 28 bp, synthetic construct
  source 1..28: mol_type = other DNA
tgacacctgccccaacaagcaatgttgg

SEQ ID NO: 41447 - DNA, 28 bp, synthetic construct
  source 1..28: mol_type = other DNA
cttgttggggcaggtgtcagagcttcgg

SEQ ID NO: 41448 - DNA, 28 bp, synthetic construct
  source 1..28: mol_type = other DNA
ttgttggggcaggtgtcagagcttcggg

SEQ ID NO: 41449 - DNA, 28 bp, synthetic construct
  source 1..28: mol_type = other DNA
gggcaggtgtcagagcttcgggaagagg

SEQ ID NO: 41450 - DNA, 28 bp, synthetic construct
  source 1..28: mol_type = other DNA
ggcaggtgtcagagcttcgggaagaggg

SEQ ID NO: 41451 - DNA, 28 bp, synthetic construct
  source 1..28: mol_type = other DNA
gcaggtgtcagagcttcgggaagagggg

SEQ ID NO: 41452 - DNA, 28 bp, synthetic construct
  source 1..28: mol_type = other DNA
aaagaattggtaattcagtagtcatagg

SEQ ID NO: 41453 - DNA, 28 bp, synthetic construct
  source 1..28: mol_type = other DNA
tactgaattaccaattctttatgacagg

SEQ ID NO: 41454 - DNA, 28 bp, synthetic construct
  source 1..28: mol_type = other DNA
cttcatttttcctgtcataaagaattgg

SEQ ID NO: 41455 - DNA, 28 bp, synthetic construct
  source 1..28: mol_type = other DNA
gacaggaaaaatgaagaaatctctcagg

SEQ ID NO: 41456 - DNA, 28 bp, synthetic construct
  source 1..28: mol_type = other DNA
acaggaaaaatgaagaaatctctcaggg

SEQ ID NO: 41457 - DNA, 28 bp, synthetic construct
  source 1..28: mol_type = other DNA
gaagaaatctctcagggctccactttgg

SEQ ID NO: 41458 - DNA, 28 bp, synthetic construct
  source 1..28: mol_type = other DNA
attttcgcaggatagatagccaaagtgg

SEQ ID NO: 41459 - DNA, 28 bp, synthetic construct
  source 1..28: mol_type = other DNA
ttggctatctatcctgcgaaaataatgg

SEQ ID NO: 41460 - DNA, 28 bp, synthetic construct
  source 1..28: mol_type = other DNA
tggctatctatcctgcgaaaataatggg

SEQ ID NO: 41461 - DNA, 28 bp, synthetic construct
  source 1..28: mol_type = other DNA
tctatcctgcgaaaataatgggaaatgg

SEQ ID NO: 41462 - DNA, 28 bp, synthetic construct
  source 1..28: mol_type = other DNA
tgttaccatttcccattattttcgcagg

SEQ ID NO: 41463 - DNA, 28 bp, synthetic construct
  source 1..28: mol_type = other DNA
gggaaatggtaacatattaaacgagtgg

SEQ ID NO: 41464 - DNA, 28 bp, synthetic construct
  source 1..28: mol_type = other DNA
gtaacatattaaacgagtggccatctgg

SEQ ID NO: 41465 - DNA, 28 bp, synthetic construct
  source 1..28: mol_type = other DNA
taacatattaaacgagtggccatctggg

SEQ ID NO: 41466 - DNA, 28 bp, synthetic construct
  source 1..28: mol_type = other DNA
aaacgagtggccatctgggtgcacgtgg

SEQ ID NO: 41467 - DNA, 28 bp, synthetic construct
  source 1..28: mol_type = other DNA
gaggcagctaccacgtgcacccagatgg

SEQ ID NO: 41468 - DNA, 28 bp, synthetic construct
  source 1..28: mol_type = other DNA
atttgggctgaagtaggtgttggagagg

SEQ ID NO: 41469 - DNA, 28 bp, synthetic construct
  source 1..28: mol_type = other DNA
ctatgatttgggctgaagtaggtgttgg

SEQ ID NO: 41470 - DNA, 28 bp, synthetic construct
  source 1..28: mol_type = other DNA
caaactctatgatttgggctgaagtagg

SEQ ID NO: 41471 - DNA, 28 bp, synthetic construct
  source 1..28: mol_type = other DNA
cagcccaaatcatagagtttgacaaagg

SEQ ID NO: 41472 - DNA, 28 bp, synthetic construct
  source 1..28: mol_type = other DNA
tttcctttgtcaaactctatgatttggg

SEQ ID NO: 41473 - DNA, 28 bp, synthetic construct
  source 1..28: mol_type = other DNA
atttcctttgtcaaactctatgatttgg

SEQ ID NO: 41474 - DNA, 28 bp, synthetic construct
  source 1..28: mol_type = other DNA
ttgacaaaggaaatctgacagcttctgg

SEQ ID NO: 41475 - DNA, 28 bp, synthetic construct
  source 1..28: mol_type = other DNA
aaggaaatctgacagcttctggagatgg

SEQ ID NO: 41476 - DNA, 28 bp, synthetic construct
  source 1..28: mol_type = other DNA
agtctgtaaataagcaaattgaaagggg

SEQ ID NO: 41477 - DNA, 28 bp, synthetic construct
  source 1..28: mol_type = other DNA
cagtctgtaaataagcaaattgaaaggg

SEQ ID NO: 41478 - DNA, 28 bp, synthetic construct
  source 1..28: mol_type = other DNA
cctttcaatttgcttatttacagactgg

SEQ ID NO: 41479 - DNA, 28 bp, synthetic construct
  source 1..28: mol_type = other DNA
ctttcaatttgcttatttacagactggg

SEQ ID NO: 41480 - DNA, 28 bp, synthetic construct
  source 1..28: mol_type = other DNA
ttgcttatttacagactgggaaatgagg

SEQ ID NO: 41481 - DNA, 28 bp, synthetic construct
  source 1..28: mol_type = other DNA
aacaaacatgctcctcccagagccatgg

SEQ ID NO: 41482 - DNA, 28 bp, synthetic construct
  source 1..28: mol_type = other DNA
aaaaaaatgtgtccatggctctgggagg

SEQ ID NO: 41483 - DNA, 28 bp, synthetic construct
  source 1..28: mol_type = other DNA
aataaaaaaatgtgtccatggctctggg

SEQ ID NO: 41484 - DNA, 28 bp, synthetic construct
  source 1..28: mol_type = other DNA
taataaaaaaatgtgtccatggctctgg

SEQ ID NO: 41485 - DNA, 28 bp, synthetic construct
  source 1..28: mol_type = other DNA
taataataataaaaaaatgtgtccatgg

SEQ ID NO: 41486 - DNA, 28 bp, synthetic construct
  source 1..28: mol_type = other DNA
ttattattattatactttaagttttagg

SEQ ID NO: 41487 - DNA, 28 bp, synthetic construct
  source 1..28: mol_type = other DNA
tattattattatactttaagttttaggg

SEQ ID NO: 41488 - DNA, 28 bp, synthetic construct
  source 1..28: mol_type = other DNA
tttagggtacatgtgcacaatgtgcagg

SEQ ID NO: 41489 - DNA, 28 bp, synthetic construct
  source 1..28: mol_type = other DNA
ttacatatgtatacatgtgccatgctgg

SEQ ID NO: 41490 - DNA, 28 bp, synthetic construct
  source 1..28: mol_type = other DNA
agttaatgggtgcagcacaccagcatgg

SEQ ID NO: 41491 - DNA, 28 bp, synthetic construct
  source 1..28: mol_type = other DNA
acccattaactcatcatttagcattagg

SEQ ID NO: 41492 - DNA, 28 bp, synthetic construct
  source 1..28: mol_type = other DNA
acctaatgctaaatgatgagttaatggg

SEQ ID NO: 41493 - DNA, 28 bp, synthetic construct
  source 1..28: mol_type = other DNA
tacctaatgctaaatgatgagttaatgg

SEQ ID NO: 41494 - DNA, 28 bp, synthetic construct
  source 1..28: mol_type = other DNA
tgttgtggggtggggggaggggggaggg

SEQ ID NO: 41495 - DNA, 28 bp, synthetic construct
  source 1..28: mol_type = other DNA
ctgttgtggggtggggggaggggggagg

SEQ ID NO: 41496 - DNA, 28 bp, synthetic construct
  source 1..28: mol_type = other DNA
ggactgttgtggggtggggggagggggg

SEQ ID NO: 41497 - DNA, 28 bp, synthetic construct
  source 1..28: mol_type = other DNA
gggactgttgtggggtggggggaggggg

SEQ ID NO: 41498 - DNA, 28 bp, synthetic construct
  source 1..28: mol_type = other DNA
ggggactgttgtggggtggggggagggg

SEQ ID NO: 41499 - DNA, 28 bp, synthetic construct
  source 1..28: mol_type = other DNA
tggggactgttgtggggtggggggaggg

SEQ ID NO: 41500 - DNA, 28 bp, synthetic construct
  source 1..28: mol_type = other DNA
ctggggactgttgtggggtggggggagg

SEQ ID NO: 41501 - DNA, 28 bp, synthetic construct
  source 1..28: mol_type = other DNA
actctggggactgttgtggggtgggggg

SEQ ID NO: 41502 - DNA, 28 bp, synthetic construct
  source 1..28: mol_type = other DNA
cactctggggactgttgtggggtggggg

SEQ ID NO: 41503 - DNA, 28 bp, synthetic construct
  source 1..28: mol_type = other DNA
acactctggggactgttgtggggtgggg

SEQ ID NO: 41504 - DNA, 28 bp, synthetic construct
  source 1..28: mol_type = other DNA
cacactctggggactgttgtggggtggg

SEQ ID NO: 41505 - DNA, 28 bp, synthetic construct
  source 1..28: mol_type = other DNA
tcacactctggggactgttgtggggtgg

SEQ ID NO: 41506 - DNA, 28 bp, synthetic construct
  source 1..28: mol_type = other DNA
acatcacactctggggactgttgtgggg

SEQ ID NO: 41507 - DNA, 28 bp, synthetic construct
  source 1..28: mol_type = other DNA
aacatcacactctggggactgttgtggg

SEQ ID NO: 41508 - DNA, 28 bp, synthetic construct
  source 1..28: mol_type = other DNA
gaacatcacactctggggactgttgtgg

SEQ ID NO: 41509 - DNA, 28 bp, synthetic construct
  source 1..28: mol_type = other DNA
acaggaaggggaacatcacactctgggg

SEQ ID NO: 41510 - DNA, 28 bp, synthetic construct
  source 1..28: mol_type = other DNA
cacaggaaggggaacatcacactctggg

SEQ ID NO: 41511 - DNA, 28 bp, synthetic construct
  source 1..28: mol_type = other DNA
acacaggaaggggaacatcacactctgg

SEQ ID NO: 41512 - DNA, 28 bp, synthetic construct
  source 1..28: mol_type = other DNA
aatgagaatacttggacacaggaagggg

SEQ ID NO: 41513 - DNA, 28 bp, synthetic construct
  source 1..28: mol_type = other DNA
caatgagaatacttggacacaggaaggg

SEQ ID NO: 41514 - DNA, 28 bp, synthetic construct
  source 1..28: mol_type = other DNA
acaatgagaatacttggacacaggaagg

SEQ ID NO: 41515 - DNA, 28 bp, synthetic construct
  source 1..28: mol_type = other DNA
ttgaacaatgagaatacttggacacagg

SEQ ID NO: 41516 - DNA, 28 bp, synthetic construct
  source 1..28: mol_type = other DNA
atgggaattgaacaatgagaatacttgg

SEQ ID NO: 41517 - DNA, 28 bp, synthetic construct
  source 1..28: mol_type = other DNA
attcccatctatgagtgagaacacgcgg

SEQ ID NO: 41518 - DNA, 28 bp, synthetic construct
  source 1..28: mol_type = other DNA
acaccgcgtgttctcactcatagatggg

SEQ ID NO: 41519 - DNA, 28 bp, synthetic construct
  source 1..28: mol_type = other DNA
aacaccgcgtgttctcactcatagatgg

SEQ ID NO: 41520 - DNA, 28 bp, synthetic construct
  source 1..28: mol_type = other DNA
tctatgagtgagaacacgcggtgtttgg

SEQ ID NO: 41521 - DNA, 28 bp, synthetic construct
  source 1..28: mol_type = other DNA
aacacgcggtgtttggttttttgcatgg

SEQ ID NO: 41522 - DNA, 28 bp, synthetic construct
  source 1..28: mol_type = other DNA
agagttcttaataagtgtactcaattgg

SEQ ID NO: 41523 - DNA, 28 bp, synthetic construct
  source 1..28: mol_type = other DNA
cttattaagaactctctagacatcttgg

SEQ ID NO: 41524 - DNA, 28 bp, synthetic construct
  source 1..28: mol_type = other DNA
ctctagacatcttggcactaaatgacgg

SEQ ID NO: 41525 - DNA, 28 bp, synthetic construct
  source 1..28: mol_type = other DNA
acattttactggacttttactgtcaggg

SEQ ID NO: 41526 - DNA, 28 bp, synthetic construct
  source 1..28: mol_type = other DNA
cacattttactggacttttactgtcagg

SEQ ID NO: 41527 - DNA, 28 bp, synthetic construct
  source 1..28: mol_type = other DNA
gtctgtgatcaggcacacattttactgg

SEQ ID NO: 41528 - DNA, 28 bp, synthetic construct
  source 1..28: mol_type = other DNA
ttgatataatgctatgtctgtgatcagg

SEQ ID NO: 41529 - DNA, 28 bp, synthetic construct
  source 1..28: mol_type = other DNA
gctttacatattcagagaaaaatgttgg

SEQ ID NO: 41530 - DNA, 28 bp, synthetic construct
  source 1..28: mol_type = other DNA
tttttctctgaatatgtaaagcttcagg

SEQ ID NO: 41531 - DNA, 28 bp, synthetic construct
  source 1..28: mol_type = other DNA
tctctgaatatgtaaagcttcaggcagg

SEQ ID NO: 41532 - DNA, 28 bp, synthetic construct
  source 1..28: mol_type = other DNA
atatgtaaagcttcaggcaggagtcagg

SEQ ID NO: 41533 - DNA, 28 bp, synthetic construct
  source 1..28: mol_type = other DNA
gggattacttgaatcttgtgaatagagg

SEQ ID NO: 41534 - DNA, 28 bp, synthetic construct
  source 1..28: mol_type = other DNA
tagtaagattgacagacagtgtggaggg

SEQ ID NO: 41535 - DNA, 28 bp, synthetic construct
  source 1..28: mol_type = other DNA
gtagtaagattgacagacagtgtggagg

SEQ ID NO: 41536 - DNA, 28 bp, synthetic construct
  source 1..28: mol_type = other DNA
actgtagtaagattgacagacagtgtgg

SEQ ID NO: 41537 - DNA, 28 bp, synthetic construct
  source 1..28: mol_type = other DNA
gtcattttgaagagtgagttaagtaggg

SEQ ID NO: 41538 - DNA, 28 bp, synthetic construct
  source 1..28: mol_type = other DNA
agtcattttgaagagtgagttaagtagg

SEQ ID NO: 41539 - DNA, 28 bp, synthetic construct
  source 1..28: mol_type = other DNA
tttggggacttgaggagcaaggagaagg

SEQ ID NO: 41540 - DNA, 28 bp, synthetic construct
  source 1..28: mol_type = other DNA
tgagattttggggacttgaggagcaagg

SEQ ID NO: 41541 - DNA, 28 bp, synthetic construct
  source 1..28: mol_type = other DNA
gaataaatgagattttggggacttgagg

SEQ ID NO: 41542 - DNA, 28 bp, synthetic construct
  source 1..28: mol_type = other DNA
gaatgaaagaataaatgagattttgggg

SEQ ID NO: 41543 - DNA, 28 bp, synthetic construct
  source 1..28: mol_type = other DNA
tgaatgaaagaataaatgagattttggg

SEQ ID NO: 41544 - DNA, 28 bp, synthetic construct
  source 1..28: mol_type = other DNA
ctgaatgaaagaataaatgagattttgg

SEQ ID NO: 41545 - DNA, 28 bp, synthetic construct
  source 1..28: mol_type = other DNA
tgattgcttctaacttctcaatgaaagg

SEQ ID NO: 41546 - DNA, 28 bp, synthetic construct
  source 1..28: mol_type = other DNA
gaagactctactacaaaggatacggtgg

SEQ ID NO: 41547 - DNA, 28 bp, synthetic construct
  source 1..28: mol_type = other DNA
ctagaagactctactacaaaggatacgg

SEQ ID NO: 41548 - DNA, 28 bp, synthetic construct
  source 1..28: mol_type = other DNA
gaatggctagaagactctactacaaagg

SEQ ID NO: 41549 - DNA, 28 bp, synthetic construct
  source 1..28: mol_type = other DNA
gaagtagagaatggatgttagggaatgg

SEQ ID NO: 41550 - DNA, 28 bp, synthetic construct
  source 1..28: mol_type = other DNA
tatgagaagtagagaatggatgttaggg

SEQ ID NO: 41551 - DNA, 28 bp, synthetic construct
  source 1..28: mol_type = other DNA
ttatgagaagtagagaatggatgttagg

SEQ ID NO: 41552 - DNA, 28 bp, synthetic construct
  source 1..28: mol_type = other DNA
ttcttctcttatgagaagtagagaatgg

SEQ ID NO: 41553 - DNA, 28 bp, synthetic construct
  source 1..28: mol_type = other DNA
ataagagaagaataacattttcagttgg

SEQ ID NO: 41554 - DNA, 28 bp, synthetic construct
  source 1..28: mol_type = other DNA
taagagaagaataacattttcagttggg

SEQ ID NO: 41555 - DNA, 28 bp, synthetic construct
  source 1..28: mol_type = other DNA
agaataacattttcagttgggcgcttgg

SEQ ID NO: 41556 - DNA, 28 bp, synthetic construct
  source 1..28: mol_type = other DNA
ggggctgggaaatttggtgtttgagggg

SEQ ID NO: 41557 - DNA, 28 bp, synthetic construct
  source 1..28: mol_type = other DNA
gggggctgggaaatttggtgtttgaggg

SEQ ID NO: 41558 - DNA, 28 bp, synthetic construct
  source 1..28: mol_type = other DNA
tgggggctgggaaatttggtgtttgagg

SEQ ID NO: 41559 - DNA, 28 bp, synthetic construct
  source 1..28: mol_type = other DNA
aagctacagtgggggctgggaaatttgg

SEQ ID NO: 41560 - DNA, 28 bp, synthetic construct
  source 1..28: mol_type = other DNA
atcactgcaagctacagtgggggctggg

SEQ ID NO: 41561 - DNA, 28 bp, synthetic construct
  source 1..28: mol_type = other DNA
catcactgcaagctacagtgggggctgg

SEQ ID NO: 41562 - DNA, 28 bp, synthetic construct
  source 1..28: mol_type = other DNA
acatcatcactgcaagctacagtggggg

SEQ ID NO: 41563 - DNA, 28 bp, synthetic construct
  source 1..28: mol_type = other DNA
cacatcatcactgcaagctacagtgggg

SEQ ID NO: 41564 - DNA, 28 bp, synthetic construct
  source 1..28: mol_type = other DNA
tcacatcatcactgcaagctacagtggg

SEQ ID NO: 41565 - DNA, 28 bp, synthetic construct
  source 1..28: mol_type = other DNA
atcacatcatcactgcaagctacagtgg

SEQ ID NO: 41566 - DNA, 28 bp, synthetic construct
  source 1..28: mol_type = other DNA
ttgcagtgatgatgtgattaaattaagg

SEQ ID NO: 41567 - DNA, 28 bp, synthetic construct
  source 1..28: mol_type = other DNA
aaggccaacgagatatgaacagaatagg

SEQ ID NO: 41568 - DNA, 28 bp, synthetic construct
  source 1..28: mol_type = other DNA
aggccaacgagatatgaacagaataggg

SEQ ID NO: 41569 - DNA, 28 bp, synthetic construct
  source 1..28: mol_type = other DNA
ggtccctattctgttcatatctcgttgg

SEQ ID NO: 41570 - DNA, 28 bp, synthetic construct
  source 1..28: mol_type = other DNA
tatgaacagaatagggaccatctctagg

SEQ ID NO: 41571 - DNA, 28 bp, synthetic construct
  source 1..28: mol_type = other DNA
tttcttaaagagcacaacctagagatgg

SEQ ID NO: 41572 - DNA, 28 bp, synthetic construct
  source 1..28: mol_type = other DNA
atctctaggttgtgctctttaagaaagg

SEQ ID NO: 41573 - DNA, 28 bp, synthetic construct
  source 1..28: mol_type = other DNA
aaagggaaaaagggggaagtgggagggg

SEQ ID NO: 41574 - DNA, 28 bp, synthetic construct
  source 1..28: mol_type = other DNA
caaagggaaaaagggggaagtgggaggg

SEQ ID NO: 41575 - DNA, 28 bp, synthetic construct
  source 1..28: mol_type = other DNA
tcaaagggaaaaagggggaagtgggagg

SEQ ID NO: 41576 - DNA, 28 bp, synthetic construct
  source 1..28: mol_type = other DNA
tagtcaaagggaaaaagggggaagtggg

SEQ ID NO: 41577 - DNA, 28 bp, synthetic construct
  source 1..28: mol_type = other DNA
ctagtcaaagggaaaaagggggaagtgg

SEQ ID NO: 41578 - DNA, 28 bp, synthetic construct
  source 1..28: mol_type = other DNA
tgaatactagtcaaagggaaaaaggggg

SEQ ID NO: 41579 - DNA, 28 bp, synthetic construct
  source 1..28: mol_type = other DNA
ctgaatactagtcaaagggaaaaagggg

SEQ ID NO: 41580 - DNA, 28 bp, synthetic construct
  source 1..28: mol_type = other DNA
actgaatactagtcaaagggaaaaaggg

SEQ ID NO: 41581 - DNA, 28 bp, synthetic construct
  source 1..28: mol_type = other DNA
gactgaatactagtcaaagggaaaaagg

SEQ ID NO: 41582 - DNA, 28 bp, synthetic construct
  source 1..28: mol_type = other DNA
ctatcatgactgaatactagtcaaaggg

SEQ ID NO: 41583 - DNA, 28 bp, synthetic construct
  source 1..28: mol_type = other DNA
gctatcatgactgaatactagtcaaagg

SEQ ID NO: 41584 - DNA, 28 bp, synthetic construct
  source 1..28: mol_type = other DNA
ttgactagtattcagtcatgatagcagg

SEQ ID NO: 41585 - DNA, 28 bp, synthetic construct
  source 1..28: mol_type = other DNA
agtattcagtcatgatagcaggagatgg

SEQ ID NO: 41586 - DNA, 28 bp, synthetic construct
  source 1..28: mol_type = other DNA
gcaggagatggaatagttcactttcagg

SEQ ID NO: 41587 - DNA, 28 bp, synthetic construct
  source 1..28: mol_type = other DNA
gccagcaagtgtaagctgcatgttgagg

SEQ ID NO: 41588 - DNA, 28 bp, synthetic construct
  source 1..28: mol_type = other DNA
acctcaacatgcagcttacacttgctgg

SEQ ID NO: 41589 - DNA, 28 bp, synthetic construct
  source 1..28: mol_type = other DNA
gcaagtgtaagctgcatgttgaggttgg

SEQ ID NO: 41590 - DNA, 28 bp, synthetic construct
  source 1..28: mol_type = other DNA
tgtaagctgcatgttgaggttggcatgg

SEQ ID NO: 41591 - DNA, 28 bp, synthetic construct
  source 1..28: mol_type = other DNA
gaggttggcatggcaacaagatagatgg

SEQ ID NO: 41592 - DNA, 28 bp, synthetic construct
  source 1..28: mol_type = other DNA
gcatggcaacaagatagatggagcctgg

SEQ ID NO: 41593 - DNA, 28 bp, synthetic construct
  source 1..28: mol_type = other DNA
gcagtggctccatacccaattatccagg

SEQ ID NO: 41594 - DNA, 28 bp, synthetic construct
  source 1..28: mol_type = other DNA
tcttttctccttcctccttatcgtatgg

SEQ ID NO: 41595 - DNA, 28 bp, synthetic construct
  source 1..28: mol_type = other DNA
cttttctccttcctccttatcgtatggg

SEQ ID NO: 41596 - DNA, 28 bp, synthetic construct
  source 1..28: mol_type = other DNA
ctccttcctccttatcgtatgggttagg

SEQ ID NO: 41597 - DNA, 28 bp, synthetic construct
  source 1..28: mol_type = other DNA
tgcctaacccatacgataaggaggaagg

SEQ ID NO: 41598 - DNA, 28 bp, synthetic construct
  source 1..28: mol_type = other DNA
tttttgcctaacccatacgataaggagg

SEQ ID NO: 41599 - DNA, 28 bp, synthetic construct
  source 1..28: mol_type = other DNA
ttgtttttgcctaacccatacgataagg

SEQ ID NO: 41600 - DNA, 28 bp, synthetic construct
  source 1..28: mol_type = other DNA
cagctgaaattttcttccagacagttgg

SEQ ID NO: 41601 - DNA, 28 bp, synthetic construct
  source 1..28: mol_type = other DNA
actcagaggtcacagtccaactgtctgg

SEQ ID NO: 41602 - DNA, 28 bp, synthetic construct
  source 1..28: mol_type = other DNA
gacctctgagtcctaccagctttgttgg

SEQ ID NO: 41603 - DNA, 28 bp, synthetic construct
  source 1..28: mol_type = other DNA
ctccaacaaagctggtaggactcagagg

SEQ ID NO: 41604 - DNA, 28 bp, synthetic construct
  source 1..28: mol_type = other DNA
atctggattctccaacaaagctggtagg

SEQ ID NO: 41605 - DNA, 28 bp, synthetic construct
  source 1..28: mol_type = other DNA
ctacatctggattctccaacaaagctgg

SEQ ID NO: 41606 - DNA, 28 bp, synthetic construct
  source 1..28: mol_type = other DNA
tggagaatccagatgtagatgagaacgg

SEQ ID NO: 41607 - DNA, 28 bp, synthetic construct
  source 1..28: mol_type = other DNA
aggcaacaccgttctcatctacatctgg

SEQ ID NO: 41608 - DNA, 28 bp, synthetic construct
  source 1..28: mol_type = other DNA
atgtagatgagaacggtgttgcctaagg

SEQ ID NO: 41609 - DNA, 28 bp, synthetic construct
  source 1..28: mol_type = other DNA
gttgcctaaggccacacttcaagccagg

SEQ ID NO: 41610 - DNA, 28 bp, synthetic construct
  source 1..28: mol_type = other DNA
cgggcctggcttgaagtgtggccttagg

SEQ ID NO: 41611 - DNA, 28 bp, synthetic construct
  source 1..28: mol_type = other DNA
aaatcaacgggcctggcttgaagtgtgg

SEQ ID NO: 41612 - DNA, 28 bp, synthetic construct
  source 1..28: mol_type = other DNA
gccaggcccgttgatttccaacttatgg

SEQ ID NO: 41613 - DNA, 28 bp, synthetic construct
  source 1..28: mol_type = other DNA
gccataagttggaaatcaacgggcctgg

SEQ ID NO: 41614 - DNA, 28 bp, synthetic construct
  source 1..28: mol_type = other DNA
aggaagccataagttggaaatcaacggg

SEQ ID NO: 41615 - DNA, 28 bp, synthetic construct
  source 1..28: mol_type = other DNA
taggaagccataagttggaaatcaacgg

SEQ ID NO: 41616 - DNA, 28 bp, synthetic construct
  source 1..28: mol_type = other DNA
cacactgctgtaggaagccataagttgg

SEQ ID NO: 41617 - DNA, 28 bp, synthetic construct
  source 1..28: mol_type = other DNA
caacttatggcttcctacagcagtgtgg

SEQ ID NO: 41618 - DNA, 28 bp, synthetic construct
  source 1..28: mol_type = other DNA
cctacagcagtgtggtcatgaagcctgg

SEQ ID NO: 41619 - DNA, 28 bp, synthetic construct
  source 1..28: mol_type = other DNA
agtgtggtcatgaagcctggaaaacagg

SEQ ID NO: 41620 - DNA, 28 bp, synthetic construct
  source 1..28: mol_type = other DNA
catgaagcctggaaaacaggaagatagg

SEQ ID NO: 41621 - DNA, 28 bp, synthetic construct
  source 1..28: mol_type = other DNA
tgtcactcctatcttcctgttttccagg

SEQ ID NO: 41622 - DNA, 28 bp, synthetic construct
  source 1..28: mol_type = other DNA
aacaggaagataggagtgacaaaagagg

SEQ ID NO: 41623 - DNA, 28 bp, synthetic construct
  source 1..28: mol_type = other DNA
acaggaagataggagtgacaaaagaggg

SEQ ID NO: 41624 - DNA, 28 bp, synthetic construct
  source 1..28: mol_type = other DNA
aagataggagtgacaaaagagggacagg

SEQ ID NO: 41625 - DNA, 28 bp, synthetic construct
  source 1..28: mol_type = other DNA
acaaaagagggacaggagtagaatgagg

SEQ ID NO: 41626 - DNA, 28 bp, synthetic construct
  source 1..28: mol_type = other DNA
gagggacaggagtagaatgaggcttagg

SEQ ID NO: 41627 - DNA, 28 bp, synthetic construct
  source 1..28: mol_type = other DNA
ttttcaaaagatgctcatttcattttgg

SEQ ID NO: 41628 - DNA, 28 bp, synthetic construct
  source 1..28: mol_type = other DNA
atgctcatttcattttggatgactatgg

SEQ ID NO: 41629 - DNA, 28 bp, synthetic construct
  source 1..28: mol_type = other DNA
catttcattttggatgactatggcaagg

SEQ ID NO: 41630 - DNA, 28 bp, synthetic construct
  source 1..28: mol_type = other DNA
tttggatgactatggcaaggaagagtgg

SEQ ID NO: 41631 - DNA, 28 bp, synthetic construct
  source 1..28: mol_type = other DNA
ggatgactatggcaaggaagagtggtgg

SEQ ID NO: 41632 - DNA, 28 bp, synthetic construct
  source 1..28: mol_type = other DNA
gtgatgactaacagtagcagtagacagg

SEQ ID NO: 41633 - DNA, 28 bp, synthetic construct
  source 1..28: mol_type = other DNA
catgtgactgtttttatgtattcattgg

SEQ ID NO: 41634 - DNA, 28 bp, synthetic construct
  source 1..28: mol_type = other DNA
tatgtattcattggtttaaattccctgg

SEQ ID NO: 41635 - DNA, 28 bp, synthetic construct
  source 1..28: mol_type = other DNA
aaagtgacatgtttctggagatccaggg

SEQ ID NO: 41636 - DNA, 28 bp, synthetic construct
  source 1..28: mol_type = other DNA
gaaagtgacatgtttctggagatccagg

SEQ ID NO: 41637 - DNA, 28 bp, synthetic construct
  source 1..28: mol_type = other DNA
tctccagaaacatgtcactttccactgg

SEQ ID NO: 41638 - DNA, 28 bp, synthetic construct
  source 1..28: mol_type = other DNA
ctccagaaacatgtcactttccactggg

SEQ ID NO: 41639 - DNA, 28 bp, synthetic construct
  source 1..28: mol_type = other DNA
tccagaaacatgtcactttccactgggg

SEQ ID NO: 41640 - DNA, 28 bp, synthetic construct
  source 1..28: mol_type = other DNA
cccccagtggaaagtgacatgtttctgg

SEQ ID NO: 41641 - DNA, 28 bp, synthetic construct
  source 1..28: mol_type = other DNA
taatcatgacacaaatttcccccagtgg

SEQ ID NO: 41642 - DNA, 28 bp, synthetic construct
  source 1..28: mol_type = other DNA
gtgattaacactgagaaaggaggagggg

SEQ ID NO: 41643 - DNA, 28 bp, synthetic construct
  source 1..28: mol_type = other DNA
ggtgattaacactgagaaaggaggaggg

SEQ ID NO: 41644 - DNA, 28 bp, synthetic construct
  source 1..28: mol_type = other DNA
aggtgattaacactgagaaaggaggagg

SEQ ID NO: 41645 - DNA, 28 bp, synthetic construct
  source 1..28: mol_type = other DNA
agaaggtgattaacactgagaaaggagg

SEQ ID NO: 41646 - DNA, 28 bp, synthetic construct
  source 1..28: mol_type = other DNA
aggagaaggtgattaacactgagaaagg

SEQ ID NO: 41647 - DNA, 28 bp, synthetic construct
  source 1..28: mol_type = other DNA
cattttaagtgctaattataggagaagg

SEQ ID NO: 41648 - DNA, 28 bp, synthetic construct
  source 1..28: mol_type = other DNA
ctttgacattttaagtgctaattatagg

SEQ ID NO: 41649 - DNA, 28 bp, synthetic construct
  source 1..28: mol_type = other DNA
ctataattagcacttaaaatgtcaaagg

SEQ ID NO: 41650 - DNA, 28 bp, synthetic construct
  source 1..28: mol_type = other DNA
gtcaaaggagaagaaattaattaacagg

SEQ ID NO: 41651 - DNA, 28 bp, synthetic construct
  source 1..28: mol_type = other DNA
attaacaggagtatccagtgcagcaagg

SEQ ID NO: 41652 - DNA, 28 bp, synthetic construct
  source 1..28: mol_type = other DNA
ggagtatccagtgcagcaaggctctagg

SEQ ID NO: 41653 - DNA, 28 bp, synthetic construct
  source 1..28: mol_type = other DNA
aatcagtcctagagccttgctgcactgg

SEQ ID NO: 41654 - DNA, 28 bp, synthetic construct
  source 1..28: mol_type = other DNA
cttccttaaatattttgagtgcttttgg

SEQ ID NO: 41655 - DNA, 28 bp, synthetic construct
  source 1..28: mol_type = other DNA
ttccttaaatattttgagtgcttttggg

SEQ ID NO: 41656 - DNA, 28 bp, synthetic construct
  source 1..28: mol_type = other DNA
ttcccaaaagcactcaaaatatttaagg

SEQ ID NO: 41657 - DNA, 28 bp, synthetic construct
  source 1..28: mol_type = other DNA
gttaaggatctttcaattagaagggagg

SEQ ID NO: 41658 - DNA, 28 bp, synthetic construct
  source 1..28: mol_type = other DNA
gtagttaaggatctttcaattagaaggg

SEQ ID NO: 41659 - DNA, 28 bp, synthetic construct
  source 1..28: mol_type = other DNA
tgtagttaaggatctttcaattagaagg

SEQ ID NO: 41660 - DNA, 28 bp, synthetic construct
  source 1..28: mol_type = other DNA
agatccttaactacaccctaagtcctgg

SEQ ID NO: 41661 - DNA, 28 bp, synthetic construct
  source 1..28: mol_type = other DNA
ccagccaggacttagggtgtagttaagg

SEQ ID NO: 41662 - DNA, 28 bp, synthetic construct
  source 1..28: mol_type = other DNA
taactacaccctaagtcctggctggtgg

SEQ ID NO: 41663 - DNA, 28 bp, synthetic construct
  source 1..28: mol_type = other DNA
acaccctaagtcctggctggtggccagg

SEQ ID NO: 41664 - DNA, 28 bp, synthetic construct
  source 1..28: mol_type = other DNA
caccctaagtcctggctggtggccaggg

SEQ ID NO: 41665 - DNA, 28 bp, synthetic construct
  source 1..28: mol_type = other DNA
accctaagtcctggctggtggccagggg

SEQ ID NO: 41666 - DNA, 28 bp, synthetic construct
  source 1..28: mol_type = other DNA
acccctggccaccagccaggacttaggg

SEQ ID NO: 41667 - DNA, 28 bp, synthetic construct
  source 1..28: mol_type = other DNA
cacccctggccaccagccaggacttagg

SEQ ID NO: 41668 - DNA, 28 bp, synthetic construct
  source 1..28: mol_type = other DNA
aagtcctggctggtggccaggggtgcgg

SEQ ID NO: 41669 - DNA, 28 bp, synthetic construct
  source 1..28: mol_type = other DNA
agtcctggctggtggccaggggtgcggg

SEQ ID NO: 41670 - DNA, 28 bp, synthetic construct
  source 1..28: mol_type = other DNA
gtcctggctggtggccaggggtgcgggg

SEQ ID NO: 41671 - DNA, 28 bp, synthetic construct
  source 1..28: mol_type = other DNA
agccccgcacccctggccaccagccagg

SEQ ID NO: 41672 - DNA, 28 bp, synthetic construct
  source 1..28: mol_type = other DNA
gtggccaggggtgcggggctgagtgagg

SEQ ID NO: 41673 - DNA, 28 bp, synthetic construct
  source 1..28: mol_type = other DNA
gccaggggtgcggggctgagtgaggcgg

SEQ ID NO: 41674 - DNA, 28 bp, synthetic construct
  source 1..28: mol_type = other DNA
gccgcctcactcagccccgcacccctgg

SEQ ID NO: 41675 - DNA, 28 bp, synthetic construct
  source 1..28: mol_type = other DNA
gtgcggggctgagtgaggcggcgtgtgg

SEQ ID NO: 41676 - DNA, 28 bp, synthetic construct
  source 1..28: mol_type = other DNA
gtggaaatcccttcttcaccatccttgg

SEQ ID NO: 41677 - DNA, 28 bp, synthetic construct
  source 1..28: mol_type = other DNA
tggaaatcccttcttcaccatccttggg

SEQ ID NO: 41678 - DNA, 28 bp, synthetic construct
  source 1..28: mol_type = other DNA
gaattttcccaaggatggtgaagaaggg

SEQ ID NO: 41679 - DNA, 28 bp, synthetic construct
  source 1..28: mol_type = other DNA
ggaattttcccaaggatggtgaagaagg

SEQ ID NO: 41680 - DNA, 28 bp, synthetic construct
  source 1..28: mol_type = other DNA
agtttggagggaattttcccaaggatgg

SEQ ID NO: 41681 - DNA, 28 bp, synthetic construct
  source 1..28: mol_type = other DNA
atccttgggaaaattccctccaaactgg

SEQ ID NO: 41682 - DNA, 28 bp, synthetic construct
  source 1..28: mol_type = other DNA
tccttgggaaaattccctccaaactggg

SEQ ID NO: 41683 - DNA, 28 bp, synthetic construct
  source 1..28: mol_type = other DNA
tcccagtttggagggaattttcccaagg

SEQ ID NO: 41684 - DNA, 28 bp, synthetic construct
  source 1..28: mol_type = other DNA
gggaaaattccctccaaactgggatagg

SEQ ID NO: 41685 - DNA, 28 bp, synthetic construct
  source 1..28: mol_type = other DNA
aaaattccctccaaactgggataggtgg

SEQ ID NO: 41686 - DNA, 28 bp, synthetic construct
  source 1..28: mol_type = other DNA
ctgttgccacctatcccagtttggaggg

SEQ ID NO: 41687 - DNA, 28 bp, synthetic construct
  source 1..28: mol_type = other DNA
tctgttgccacctatcccagtttggagg

SEQ ID NO: 41688 - DNA, 28 bp, synthetic construct
  source 1..28: mol_type = other DNA
tccaaactgggataggtggcaacagagg

SEQ ID NO: 41689 - DNA, 28 bp, synthetic construct
  source 1..28: mol_type = other DNA
acctctgttgccacctatcccagtttgg

SEQ ID NO: 41690 - DNA, 28 bp, synthetic construct
  source 1..28: mol_type = other DNA
actgggataggtggcaacagaggttcgg

SEQ ID NO: 41691 - DNA, 28 bp, synthetic construct
  source 1..28: mol_type = other DNA
gaggttcggaaacagcaagcgtcccagg

SEQ ID NO: 41692 - DNA, 28 bp, synthetic construct
  source 1..28: mol_type = other DNA
cagcaagcgtcccaggctgaatctgcgg

SEQ ID NO: 41693 - DNA, 28 bp, synthetic construct
  source 1..28: mol_type = other DNA
caagcgtcccaggctgaatctgcggagg

SEQ ID NO: 41694 - DNA, 28 bp, synthetic construct
  source 1..28: mol_type = other DNA
gcgtcccaggctgaatctgcggaggagg

SEQ ID NO: 41695 - DNA, 28 bp, synthetic construct
  source 1..28: mol_type = other DNA
tcttcctcctccgcagattcagcctggg

SEQ ID NO: 41696 - DNA, 28 bp, synthetic construct
  source 1..28: mol_type = other DNA
ctcttcctcctccgcagattcagcctgg

SEQ ID NO: 41697 - DNA, 28 bp, synthetic construct
  source 1..28: mol_type = other DNA
aggaagagatgaacctttcctgagctgg

SEQ ID NO: 41698 - DNA, 28 bp, synthetic construct
  source 1..28: mol_type = other DNA
ctggcacgcagtaccagctcaggaaagg

SEQ ID NO: 41699 - DNA, 28 bp, synthetic construct
  source 1..28: mol_type = other DNA
ctttcctgagctggtactgcgtgccagg

SEQ ID NO: 41700 - DNA, 28 bp, synthetic construct
  source 1..28: mol_type = other DNA
agttcctggcacgcagtaccagctcagg

SEQ ID NO: 41701 - DNA, 28 bp, synthetic construct
  source 1..28: mol_type = other DNA
gtactgcgtgccaggaactttagctcgg

SEQ ID NO: 41702 - DNA, 28 bp, synthetic construct
  source 1..28: mol_type = other DNA
tggcaaaataccgagctaaagttcctgg

SEQ ID NO: 41703 - DNA, 28 bp, synthetic construct
  source 1..28: mol_type = other DNA
tagtatcggttgtcttacaggattgtgg

SEQ ID NO: 41704 - DNA, 28 bp, synthetic construct
  source 1..28: mol_type = other DNA
gagatcatagtatcggttgtcttacagg

SEQ ID NO: 41705 - DNA, 28 bp, synthetic construct
  source 1..28: mol_type = other DNA
atctgtaaaatggagatcatagtatcgg

SEQ ID NO: 41706 - DNA, 28 bp, synthetic construct
  source 1..28: mol_type = other DNA
tactatgatctccattttacagatgagg

SEQ ID NO: 41707 - DNA, 28 bp, synthetic construct
  source 1..28: mol_type = other DNA
ctccattttacagatgaggacattgagg

SEQ ID NO: 41708 - DNA, 28 bp, synthetic construct
  source 1..28: mol_type = other DNA
agcctcaatgtcctcatctgtaaaatgg

SEQ ID NO: 41709 - DNA, 28 bp, synthetic construct
  source 1..28: mol_type = other DNA
cagatgaggacattgaggctcagcgtgg

SEQ ID NO: 41710 - DNA, 28 bp, synthetic construct
  source 1..28: mol_type = other DNA
ggctcagcgtggttgtgacttcctcagg

SEQ ID NO: 41711 - DNA, 28 bp, synthetic construct
  source 1..28: mol_type = other DNA
tttcattcagtggctgcgtgacctgagg

SEQ ID NO: 41712 - DNA, 28 bp, synthetic construct
  source 1..28: mol_type = other DNA
ttgaatctttggcgctttcattcagtgg

SEQ ID NO: 41713 - DNA, 28 bp, synthetic construct
  source 1..28: mol_type = other DNA
atgaaagcgccaaagattcaaactgagg

SEQ ID NO: 41714 - DNA, 28 bp, synthetic construct
  source 1..28: mol_type = other DNA
agaatcagacctcagtttgaatctttgg

SEQ ID NO: 41715 - DNA, 28 bp, synthetic construct
  source 1..28: mol_type = other DNA
ctgattctaaagctttgctctctcacgg

SEQ ID NO: 41716 - DNA, 28 bp, synthetic construct
  source 1..28: mol_type = other DNA
aaagctttgctctctcacggcatcctgg

SEQ ID NO: 41717 - DNA, 28 bp, synthetic construct
  source 1..28: mol_type = other DNA
cagatgaaggttgaaataggattccagg

SEQ ID NO: 41718 - DNA, 28 bp, synthetic construct
  source 1..28: mol_type = other DNA
ctggaatcctatttcaaccttcatctgg

SEQ ID NO: 41719 - DNA, 28 bp, synthetic construct
  source 1..28: mol_type = other DNA
taagagtccagatgaaggttgaaatagg

SEQ ID NO: 41720 - DNA, 28 bp, synthetic construct
  source 1..28: mol_type = other DNA
tgggctgggttaagagtccagatgaagg

SEQ ID NO: 41721 - DNA, 28 bp, synthetic construct
  source 1..28: mol_type = other DNA
aactgtagacgcttaggtttgggctggg

SEQ ID NO: 41722 - DNA, 28 bp, synthetic construct
  source 1..28: mol_type = other DNA
aaactgtagacgcttaggtttgggctgg

SEQ ID NO: 41723 - DNA, 28 bp, synthetic construct
  source 1..28: mol_type = other DNA
gtcaaaactgtagacgcttaggtttggg

SEQ ID NO: 41724 - DNA, 28 bp, synthetic construct
  source 1..28: mol_type = other DNA
tgtcaaaactgtagacgcttaggtttgg

SEQ ID NO: 41725 - DNA, 28 bp, synthetic construct
  source 1..28: mol_type = other DNA
tcagctgtcaaaactgtagacgcttagg

SEQ ID NO: 41726 - DNA, 28 bp, synthetic construct
  source 1..28: mol_type = other DNA
taagcgtctacagttttgacagctgagg

SEQ ID NO: 41727 - DNA, 28 bp, synthetic construct
  source 1..28: mol_type = other DNA
gcgtctacagttttgacagctgaggcgg

SEQ ID NO: 41728 - DNA, 28 bp, synthetic construct
  source 1..28: mol_type = other DNA
cgtctacagttttgacagctgaggcggg

SEQ ID NO: 41729 - DNA, 28 bp, synthetic construct
  source 1..28: mol_type = other DNA
agttttgacagctgaggcgggagcacgg

SEQ ID NO: 41730 - DNA, 28 bp, synthetic construct
  source 1..28: mol_type = other DNA
gttttgacagctgaggcgggagcacggg

SEQ ID NO: 41731 - DNA, 28 bp, synthetic construct
  source 1..28: mol_type = other DNA
ttgacagctgaggcgggagcacgggagg

SEQ ID NO: 41732 - DNA, 28 bp, synthetic construct
  source 1..28: mol_type = other DNA
acagctgaggcgggagcacgggaggcgg

SEQ ID NO: 41733 - DNA, 28 bp, synthetic construct
  source 1..28: mol_type = other DNA
gaggcgggagcacgggaggcggagctgg

SEQ ID NO: 41734 - DNA, 28 bp, synthetic construct
  source 1..28: mol_type = other DNA
gcgggagcacgggaggcggagctggtgg

SEQ ID NO: 41735 - DNA, 28 bp, synthetic construct
  source 1..28: mol_type = other DNA
ctggtggcagcgcagcgccccgccccgg

SEQ ID NO: 41736 - DNA, 28 bp, synthetic construct
  source 1..28: mol_type = other DNA
attggctgatgctggagccggggcgggg

SEQ ID NO: 41737 - DNA, 28 bp, synthetic construct
  source 1..28: mol_type = other DNA
cattggctgatgctggagccggggcggg

SEQ ID NO: 41738 - DNA, 28 bp, synthetic construct
  source 1..28: mol_type = other DNA
ccattggctgatgctggagccggggcgg

SEQ ID NO: 41739 - DNA, 28 bp, synthetic construct
  source 1..28: mol_type = other DNA
tcaccattggctgatgctggagccgggg

SEQ ID NO: 41740 - DNA, 28 bp, synthetic construct
  source 1..28: mol_type = other DNA
gtcaccattggctgatgctggagccggg

SEQ ID NO: 41741 - DNA, 28 bp, synthetic construct
  source 1..28: mol_type = other DNA
cgtcaccattggctgatgctggagccgg

SEQ ID NO: 41742 - DNA, 28 bp, synthetic construct
  source 1..28: mol_type = other DNA
gctccagcatcagccaatggtgacgcgg

SEQ ID NO: 41743 - DNA, 28 bp, synthetic construct
  source 1..28: mol_type = other DNA
gtgccgcgtcaccattggctgatgctgg

SEQ ID NO: 41744 - DNA, 28 bp, synthetic construct
  source 1..28: mol_type = other DNA
aaggctgtgggtgccgcgtcaccattgg

SEQ ID NO: 41745 - DNA, 28 bp, synthetic construct
  source 1..28: mol_type = other DNA
tcaagctgattgggcgaaaggctgtggg

SEQ ID NO: 41746 - DNA, 28 bp, synthetic construct
  source 1..28: mol_type = other DNA
ctcaagctgattgggcgaaaggctgtgg

SEQ ID NO: 41747 - DNA, 28 bp, synthetic construct
  source 1..28: mol_type = other DNA
gggaagctcaagctgattgggcgaaagg

SEQ ID NO: 41748 - DNA, 28 bp, synthetic construct
  source 1..28: mol_type = other DNA
tggaggcgggaagctcaagctgattggg

SEQ ID NO: 41749 - DNA, 28 bp, synthetic construct
  source 1..28: mol_type = other DNA
atggaggcgggaagctcaagctgattgg

SEQ ID NO: 41750 - DNA, 28 bp, synthetic construct
  source 1..28: mol_type = other DNA
gcagagaagagcggcggatggaggcggg

SEQ ID NO: 41751 - DNA, 28 bp, synthetic construct
  source 1..28: mol_type = other DNA
ggcagagaagagcggcggatggaggcgg

SEQ ID NO: 41752 - DNA, 28 bp, synthetic construct
  source 1..28: mol_type = other DNA
cggggcagagaagagcggcggatggagg

SEQ ID NO: 41753 - DNA, 28 bp, synthetic construct
  source 1..28: mol_type = other DNA
gggcggggcagagaagagcggcggatgg

SEQ ID NO: 41754 - DNA, 28 bp, synthetic construct
  source 1..28: mol_type = other DNA
gaaggggcggggcagagaagagcggcgg

SEQ ID NO: 41755 - DNA, 28 bp, synthetic construct
  source 1..28: mol_type = other DNA
agcgaaggggcggggcagagaagagcgg

SEQ ID NO: 41756 - DNA, 28 bp, synthetic construct
  source 1..28: mol_type = other DNA
ctgccccgccccttcgctttccctttgg

SEQ ID NO: 41757 - DNA, 28 bp, synthetic construct
  source 1..28: mol_type = other DNA
gaaccaaagggaaagcgaaggggcgggg

SEQ ID NO: 41758 - DNA, 28 bp, synthetic construct
  source 1..28: mol_type = other DNA
ggaaccaaagggaaagcgaaggggcggg

SEQ ID NO: 41759 - DNA, 28 bp, synthetic construct
  source 1..28: mol_type = other DNA
tggaaccaaagggaaagcgaaggggcgg

SEQ ID NO: 41760 - DNA, 28 bp, synthetic construct
  source 1..28: mol_type = other DNA
cggtggaaccaaagggaaagcgaagggg

SEQ ID NO: 41761 - DNA, 28 bp, synthetic construct
  source 1..28: mol_type = other DNA
tcggtggaaccaaagggaaagcgaaggg

SEQ ID NO: 41762 - DNA, 28 bp, synthetic construct
  source 1..28: mol_type = other DNA
ctcggtggaaccaaagggaaagcgaagg

SEQ ID NO: 41763 - DNA, 28 bp, synthetic construct
  source 1..28: mol_type = other DNA
ctctgtcaagctcggtggaaccaaaggg

SEQ ID NO: 41764 - DNA, 28 bp, synthetic construct
  source 1..28: mol_type = other DNA
gctctgtcaagctcggtggaaccaaagg

SEQ ID NO: 41765 - DNA, 28 bp, synthetic construct
  source 1..28: mol_type = other DNA
tttggttccaccgagcttgacagagcgg

SEQ ID NO: 41766 - DNA, 28 bp, synthetic construct
  source 1..28: mol_type = other DNA
ggactttccgctctgtcaagctcggtgg

SEQ ID NO: 41767 - DNA, 28 bp, synthetic construct
  source 1..28: mol_type = other DNA
aagggactttccgctctgtcaagctcgg

SEQ ID NO: 41768 - DNA, 28 bp, synthetic construct
  source 1..28: mol_type = other DNA
agcttgacagagcggaaagtcccttcgg

SEQ ID NO: 41769 - DNA, 28 bp, synthetic construct
  source 1..28: mol_type = other DNA
tgacagagcggaaagtcccttcggccgg

SEQ ID NO: 41770 - DNA, 28 bp, synthetic construct
  source 1..28: mol_type = other DNA
agcggaaagtcccttcggccggcgccgg

SEQ ID NO: 41771 - DNA, 28 bp, synthetic construct
  source 1..28: mol_type = other DNA
gcggaaagtcccttcggccggcgccggg

SEQ ID NO: 41772 - DNA, 28 bp, synthetic construct
  source 1..28: mol_type = other DNA
aaagtcccttcggccggcgccgggctgg

SEQ ID NO: 41773 - DNA, 28 bp, synthetic construct
  source 1..28: mol_type = other DNA
ggctgccagcccggcgccggccgaaggg

SEQ ID NO: 41774 - DNA, 28 bp, synthetic construct
  source 1..28: mol_type = other DNA
tggctgccagcccggcgccggccgaagg

SEQ ID NO: 41775 - DNA, 28 bp, synthetic construct
  source 1..28: mol_type = other DNA
cggccggcgccgggctggcagccattgg

SEQ ID NO: 41776 - DNA, 28 bp, synthetic construct
  source 1..28: mol_type = other DNA
ccggcgccgggctggcagccattggagg

SEQ ID NO: 41777 - DNA, 28 bp, synthetic construct
  source 1..28: mol_type = other DNA
cgccgggctggcagccattggaggaagg

SEQ ID NO: 41778 - DNA, 28 bp, synthetic construct
  source 1..28: mol_type = other DNA
gaccttcctccaatggctgccagcccgg

SEQ ID NO: 41779 - DNA, 28 bp, synthetic construct
  source 1..28: mol_type = other DNA
cagccattggaggaaggtctgtcacagg

SEQ ID NO: 41780 - DNA, 28 bp, synthetic construct
  source 1..28: mol_type = other DNA
agccattggaggaaggtctgtcacaggg

SEQ ID NO: 41781 - DNA, 28 bp, synthetic construct
  source 1..28: mol_type = other DNA
ctccctgtgacagaccttcctccaatgg

SEQ ID NO: 41782 - DNA, 28 bp, synthetic construct
  source 1..28: mol_type = other DNA
cattggaggaaggtctgtcacagggagg

SEQ ID NO: 41783 - DNA, 28 bp, synthetic construct
  source 1..28: mol_type = other DNA
ggtctgtcacagggaggcccaatcacgg

SEQ ID NO: 41784 - DNA, 28 bp, synthetic construct
  source 1..28: mol_type = other DNA
agggaggcccaatcacggcccgctcagg

SEQ ID NO: 41785 - DNA, 28 bp, synthetic construct
  source 1..28: mol_type = other DNA
ctgcgctcctgagcgggccgtgattggg

SEQ ID NO: 41786 - DNA, 28 bp, synthetic construct
  source 1..28: mol_type = other DNA
gctgcgctcctgagcgggccgtgattgg

SEQ ID NO: 41787 - DNA, 28 bp, synthetic construct
  source 1..28: mol_type = other DNA
tcacggcccgctcaggagcgcagctcgg

SEQ ID NO: 41788 - DNA, 28 bp, synthetic construct
  source 1..28: mol_type = other DNA
cgtaggccgagctgcgctcctgagcggg

SEQ ID NO: 41789 - DNA, 28 bp, synthetic construct
  source 1..28: mol_type = other DNA
tcgtaggccgagctgcgctcctgagcgg

SEQ ID NO: 41790 - DNA, 28 bp, synthetic construct
  source 1..28: mol_type = other DNA
tcaggagcgcagctcggcctacgattgg

SEQ ID NO: 41791 - DNA, 28 bp, synthetic construct
  source 1..28: mol_type = other DNA
cagctcggcctacgattggctagcgcgg

SEQ ID NO: 41792 - DNA, 28 bp, synthetic construct
  source 1..28: mol_type = other DNA
ctcggcctacgattggctagcgcggcgg

SEQ ID NO: 41793 - DNA, 28 bp, synthetic construct
  source 1..28: mol_type = other DNA
ggcagccgccgcgctagccaatcgtagg

SEQ ID NO: 41794 - DNA, 28 bp, synthetic construct
  source 1..28: mol_type = other DNA
aagagggagggagcgggggcggaggggg

SEQ ID NO: 41795 - DNA, 28 bp, synthetic construct
  source 1..28: mol_type = other DNA
gaagagggagggagcgggggcggagggg

SEQ ID NO: 41796 - DNA, 28 bp, synthetic construct
  source 1..28: mol_type = other DNA
ggaagagggagggagcgggggcggaggg

SEQ ID NO: 41797 - DNA, 28 bp, synthetic construct
  source 1..28: mol_type = other DNA
gggaagagggagggagcgggggcggagg

SEQ ID NO: 41798 - DNA, 28 bp, synthetic construct
  source 1..28: mol_type = other DNA
acagggaagagggagggagcgggggcgg

SEQ ID NO: 41799 - DNA, 28 bp, synthetic construct
  source 1..28: mol_type = other DNA
cgcacagggaagagggagggagcggggg

SEQ ID NO: 41800 - DNA, 28 bp, synthetic construct
  source 1..28: mol_type = other DNA
ccccgctccctccctcttccctgtgcgg

SEQ ID NO: 41801 - DNA, 28 bp, synthetic construct
  source 1..28: mol_type = other DNA
accgcacagggaagagggagggagcggg

SEQ ID NO: 41802 - DNA, 28 bp, synthetic construct
  source 1..28: mol_type = other DNA
aaccgcacagggaagagggagggagcgg

SEQ ID NO: 41803 - DNA, 28 bp, synthetic construct
  source 1..28: mol_type = other DNA
ctccctccctcttccctgtgcggttcgg

SEQ ID NO: 41804 - DNA, 28 bp, synthetic construct
  source 1..28: mol_type = other DNA
ctccgaaccgcacagggaagagggaggg

SEQ ID NO: 41805 - DNA, 28 bp, synthetic construct
  source 1..28: mol_type = other DNA
cctccgaaccgcacagggaagagggagg

SEQ ID NO: 41806 - DNA, 28 bp, synthetic construct
  source 1..28: mol_type = other DNA
ccctcttccctgtgcggttcggaggcgg

SEQ ID NO: 41807 - DNA, 28 bp, synthetic construct
  source 1..28: mol_type = other DNA
cctcttccctgtgcggttcggaggcggg

SEQ ID NO: 41808 - DNA, 28 bp, synthetic construct
  source 1..28: mol_type = other DNA
ctcttccctgtgcggttcggaggcgggg

SEQ ID NO: 41809 - DNA, 28 bp, synthetic construct
  source 1..28: mol_type = other DNA
tccctgtgcggttcggaggcggggcagg

SEQ ID NO: 41810 - DNA, 28 bp, synthetic construct
  source 1..28: mol_type = other DNA
acctgccccgcctccgaaccgcacaggg

SEQ ID NO: 41811 - DNA, 28 bp, synthetic construct
  source 1..28: mol_type = other DNA
cacctgccccgcctccgaaccgcacagg

SEQ ID NO: 41812 - DNA, 28 bp, synthetic construct
  source 1..28: mol_type = other DNA
ctgtgcggttcggaggcggggcaggtgg

SEQ ID NO: 41813 - DNA, 28 bp, synthetic construct
  source 1..28: mol_type = other DNA
tgtgcggttcggaggcggggcaggtggg

SEQ ID NO: 41814 - DNA, 28 bp, synthetic construct
  source 1..28: mol_type = other DNA
gtgcggttcggaggcggggcaggtgggg

SEQ ID NO: 41815 - DNA, 28 bp, synthetic construct
  source 1..28: mol_type = other DNA
tgcggttcggaggcggggcaggtggggg

SEQ ID NO: 41816 - DNA, 28 bp, synthetic construct
  source 1..28: mol_type = other DNA
ggttcggaggcggggcaggtgggggcgg

SEQ ID NO: 41817 - DNA, 28 bp, synthetic construct
  source 1..28: mol_type = other DNA
gttcggaggcggggcaggtgggggcggg

SEQ ID NO: 41818 - DNA, 28 bp, synthetic construct
  source 1..28: mol_type = other DNA
aggcggggcaggtgggggcgggcccagg

SEQ ID NO: 41819 - DNA, 28 bp, synthetic construct
  source 1..28: mol_type = other DNA
gcaggtgggggcgggcccaggtagcagg

SEQ ID NO: 41820 - DNA, 28 bp, synthetic construct
  source 1..28: mol_type = other DNA
tgggggcgggcccaggtagcaggtttgg

SEQ ID NO: 41821 - DNA, 28 bp, synthetic construct
  source 1..28: mol_type = other DNA
ggcccaggtagcaggtttggctgcgcgg

SEQ ID NO: 41822 - DNA, 28 bp, synthetic construct
  source 1..28: mol_type = other DNA
gcccaggtagcaggtttggctgcgcggg

SEQ ID NO: 41823 - DNA, 28 bp, synthetic construct
  source 1..28: mol_type = other DNA
ccccgcgcagccaaacctgctacctggg

SEQ ID NO: 41824 - DNA, 28 bp, synthetic construct
  source 1..28: mol_type = other DNA
cccccgcgcagccaaacctgctacctgg

SEQ ID NO: 41825 - DNA, 28 bp, synthetic construct
  source 1..28: mol_type = other DNA
gtttggctgcgcgggggccgcgcgtcgg

SEQ ID NO: 41826 - DNA, 28 bp, synthetic construct
  source 1..28: mol_type = other DNA
tggctgcgcgggggccgcgcgtcggagg

SEQ ID NO: 41827 - DNA, 28 bp, synthetic construct
  source 1..28: mol_type = other DNA
gggccgcgcgtcggaggtaaatactagg

SEQ ID NO: 41828 - DNA, 28 bp, synthetic construct
  source 1..28: mol_type = other DNA
ggccgcgcgtcggaggtaaatactaggg

SEQ ID NO: 41829 - DNA, 28 bp, synthetic construct
  source 1..28: mol_type = other DNA
cgccctagtatttacctccgacgcgcgg

SEQ ID NO: 41830 - DNA, 28 bp, synthetic construct
  source 1..28: mol_type = other DNA
cgcgcgtcggaggtaaatactagggcgg

SEQ ID NO: 41831 - DNA, 28 bp, synthetic construct
  source 1..28: mol_type = other DNA
gcgtcggaggtaaatactagggcggtgg

SEQ ID NO: 41832 - DNA, 28 bp, synthetic construct
  source 1..28: mol_type = other DNA
cgtcggaggtaaatactagggcggtggg

SEQ ID NO: 41833 - DNA, 28 bp, synthetic construct
  source 1..28: mol_type = other DNA
gaggtaaatactagggcggtgggtgtgg

SEQ ID NO: 41834 - DNA, 28 bp, synthetic construct
  source 1..28: mol_type = other DNA
aggtaaatactagggcggtgggtgtggg

SEQ ID NO: 41835 - DNA, 28 bp, synthetic construct
  source 1..28: mol_type = other DNA
ggtaaatactagggcggtgggtgtgggg

SEQ ID NO: 41836 - DNA, 28 bp, synthetic construct
  source 1..28: mol_type = other DNA
tactagggcggtgggtgtggggagccgg

SEQ ID NO: 41837 - DNA, 28 bp, synthetic construct
  source 1..28: mol_type = other DNA
actagggcggtgggtgtggggagccggg

SEQ ID NO: 41838 - DNA, 28 bp, synthetic construct
  source 1..28: mol_type = other DNA
ctagggcggtgggtgtggggagccgggg

SEQ ID NO: 41839 - DNA, 28 bp, synthetic construct
  source 1..28: mol_type = other DNA
ggcggtgggtgtggggagccggggccgg

SEQ ID NO: 41840 - DNA, 28 bp, synthetic construct
  source 1..28: mol_type = other DNA
tgggtgtggggagccggggccggcccgg

SEQ ID NO: 41841 - DNA, 28 bp, synthetic construct
  source 1..28: mol_type = other DNA
gggtgtggggagccggggccggcccggg

SEQ ID NO: 41842 - DNA, 28 bp, synthetic construct
  source 1..28: mol_type = other DNA
ggggagccggggccggcccgggacgcgg

SEQ ID NO: 41843 - DNA, 28 bp, synthetic construct
  source 1..28: mol_type = other DNA
gggagccggggccggcccgggacgcggg

SEQ ID NO: 41844 - DNA, 28 bp, synthetic construct
  source 1..28: mol_type = other DNA
gccggggccggcccgggacgcgggctgg

SEQ ID NO: 41845 - DNA, 28 bp, synthetic construct
  source 1..28: mol_type = other DNA
ccggggccggcccgggacgcgggctggg

SEQ ID NO: 41846 - DNA, 28 bp, synthetic construct
  source 1..28: mol_type = other DNA
cggggccggcccgggacgcgggctgggg

SEQ ID NO: 41847 - DNA, 28 bp, synthetic construct
  source 1..28: mol_type = other DNA
cggctccccagcccgcgtcccgggccgg

SEQ ID NO: 41848 - DNA, 28 bp, synthetic construct
  source 1..28: mol_type = other DNA
cggcccgggacgcgggctggggagccgg

SEQ ID NO: 41849 - DNA, 28 bp, synthetic construct
  source 1..28: mol_type = other DNA
ggcccgggacgcgggctggggagccggg

SEQ ID NO: 41850 - DNA, 28 bp, synthetic construct
  source 1..28: mol_type = other DNA
gcccgggacgcgggctggggagccgggg

SEQ ID NO: 41851 - DNA, 28 bp, synthetic construct
  source 1..28: mol_type = other DNA
gccccggctccccagcccgcgtcccggg

SEQ ID NO: 41852 - DNA, 28 bp, synthetic construct
  source 1..28: mol_type = other DNA
cgccccggctccccagcccgcgtcccgg

SEQ ID NO: 41853 - DNA, 28 bp, synthetic construct
  source 1..28: mol_type = other DNA
ggacgcgggctggggagccggggcgagg

SEQ ID NO: 41854 - DNA, 28 bp, synthetic construct
  source 1..28: mol_type = other DNA
gacgcgggctggggagccggggcgaggg

SEQ ID NO: 41855 - DNA, 28 bp, synthetic construct
  source 1..28: mol_type = other DNA
acgcgggctggggagccggggcgagggg

SEQ ID NO: 41856 - DNA, 28 bp, synthetic construct
  source 1..28: mol_type = other DNA
ggcggcggggcgtcgcccctcgccccgg

SEQ ID NO: 41857 - DNA, 28 bp, synthetic construct
  source 1..28: mol_type = other DNA
gcgaggggcgacgccccgccgcccgagg

SEQ ID NO: 41858 - DNA, 28 bp, synthetic construct
  source 1..28: mol_type = other DNA
gctcattcactaacctcgggcggcgggg

SEQ ID NO: 41859 - DNA, 28 bp, synthetic construct
  source 1..28: mol_type = other DNA
cgctcattcactaacctcgggcggcggg

SEQ ID NO: 41860 - DNA, 28 bp, synthetic construct
  source 1..28: mol_type = other DNA
ccgctcattcactaacctcgggcggcgg

SEQ ID NO: 41861 - DNA, 28 bp, synthetic construct
  source 1..28: mol_type = other DNA
cgccgcccgaggttagtgaatgagcggg

SEQ ID NO: 41862 - DNA, 28 bp, synthetic construct
  source 1..28: mol_type = other DNA
cgcccgctcattcactaacctcgggcgg

SEQ ID NO: 41863 - DNA, 28 bp, synthetic construct
  source 1..28: mol_type = other DNA
cgcccgaggttagtgaatgagcgggcgg

SEQ ID NO: 41864 - DNA, 28 bp, synthetic construct
  source 1..28: mol_type = other DNA
agccgcccgctcattcactaacctcggg

SEQ ID NO: 41865 - DNA, 28 bp, synthetic construct
  source 1..28: mol_type = other DNA
cagccgcccgctcattcactaacctcgg

SEQ ID NO: 41866 - DNA, 28 bp, synthetic construct
  source 1..28: mol_type = other DNA
cgaggttagtgaatgagcgggcggctgg

SEQ ID NO: 41867 - DNA, 28 bp, synthetic construct
  source 1..28: mol_type = other DNA
ggttagtgaatgagcgggcggctggcgg

SEQ ID NO: 41868 - DNA, 28 bp, synthetic construct
  source 1..28: mol_type = other DNA
agtgaatgagcgggcggctggcggccgg

SEQ ID NO: 41869 - DNA, 28 bp, synthetic construct
  source 1..28: mol_type = other DNA
gaatgagcgggcggctggcggccggcgg

SEQ ID NO: 41870 - DNA, 28 bp, synthetic construct
  source 1..28: mol_type = other DNA
aatgagcgggcggctggcggccggcggg

SEQ ID NO: 41871 - DNA, 28 bp, synthetic construct
  source 1..28: mol_type = other DNA
gagcgggcggctggcggccggcgggcgg

SEQ ID NO: 41872 - DNA, 28 bp, synthetic construct
  source 1..28: mol_type = other DNA
gggcggctggcggccggcgggcggccgg

SEQ ID NO: 41873 - DNA, 28 bp, synthetic construct
  source 1..28: mol_type = other DNA
cggccggcgggcggccggatcccctcgg

SEQ ID NO: 41874 - DNA, 28 bp, synthetic construct
  source 1..28: mol_type = other DNA
gcgccgaggggatccggccgcccgccgg

SEQ ID NO: 41875 - DNA, 28 bp, synthetic construct
  source 1..28: mol_type = other DNA
gccggatcccctcggcgcagccgcctgg

SEQ ID NO: 41876 - DNA, 28 bp, synthetic construct
  source 1..28: mol_type = other DNA
gccaggcggctgcgccgaggggatccgg

SEQ ID NO: 41877 - DNA, 28 bp, synthetic construct
  source 1..28: mol_type = other DNA
cccctcggcgcagccgcctggcctcagg

SEQ ID NO: 41878 - DNA, 28 bp, synthetic construct
  source 1..28: mol_type = other DNA
ccctcggcgcagccgcctggcctcaggg

SEQ ID NO: 41879 - DNA, 28 bp, synthetic construct
  source 1..28: mol_type = other DNA
gccctgaggccaggcggctgcgccgagg

SEQ ID NO: 41880 - DNA, 28 bp, synthetic construct
  source 1..28: mol_type = other DNA
cgcagccgcctggcctcagggcgtccgg

SEQ ID NO: 41881 - DNA, 28 bp, synthetic construct
  source 1..28: mol_type = other DNA
cggctccggacgccctgaggccaggcgg

SEQ ID NO: 41882 - DNA, 28 bp, synthetic construct
  source 1..28: mol_type = other DNA
cggcggctccggacgccctgaggccagg

SEQ ID NO: 41883 - DNA, 28 bp, synthetic construct
  source 1..28: mol_type = other DNA
ggcctcagggcgtccggagccgccgcgg

SEQ ID NO: 41884 - DNA, 28 bp, synthetic construct
  source 1..28: mol_type = other DNA
cgccgcggcggctccggacgccctgagg

SEQ ID NO: 41885 - DNA, 28 bp, synthetic construct
  source 1..28: mol_type = other DNA
cgtccggagccgccgcggcgaccatcgg

SEQ ID NO: 41886 - DNA, 28 bp, synthetic construct
  source 1..28: mol_type = other DNA
gtccggagccgccgcggcgaccatcggg

SEQ ID NO: 41887 - DNA, 28 bp, synthetic construct
  source 1..28: mol_type = other DNA
ggcccgatggtcgccgcggcggctccgg

SEQ ID NO: 41888 - DNA, 28 bp, synthetic construct
  source 1..28: mol_type = other DNA
gccgccgcggcgaccatcgggccctcgg

SEQ ID NO: 41889 - DNA, 28 bp, synthetic construct
  source 1..28: mol_type = other DNA
gccgagggcccgatggtcgccgcggcgg

SEQ ID NO: 41890 - DNA, 28 bp, synthetic construct
  source 1..28: mol_type = other DNA
ggcgccgagggcccgatggtcgccgcgg

SEQ ID NO: 41891 - DNA, 28 bp, synthetic construct
  source 1..28: mol_type = other DNA
gcggcgaccatcgggccctcggcgccgg

SEQ ID NO: 41892 - DNA, 28 bp, synthetic construct
  source 1..28: mol_type = other DNA
taacgggccggcgccgagggcccgatgg

SEQ ID NO: 41893 - DNA, 28 bp, synthetic construct
  source 1..28: mol_type = other DNA
cgggcaactaacgggccggcgccgaggg

SEQ ID NO: 41894 - DNA, 28 bp, synthetic construct
  source 1..28: mol_type = other DNA
ccgggcaactaacgggccggcgccgagg

SEQ ID NO: 41895 - DNA, 28 bp, synthetic construct
  source 1..28: mol_type = other DNA
ctcggcgccggcccgttagttgcccggg

SEQ ID NO: 41896 - DNA, 28 bp, synthetic construct
  source 1..28: mol_type = other DNA
gctcgggcccgggcaactaacgggccgg

SEQ ID NO: 41897 - DNA, 28 bp, synthetic construct
  source 1..28: mol_type = other DNA
gcccgttagttgcccgggcccgagccgg

SEQ ID NO: 41898 - DNA, 28 bp, synthetic construct
  source 1..28: mol_type = other DNA
gccggctcgggcccgggcaactaacggg

SEQ ID NO: 41899 - DNA, 28 bp, synthetic construct
  source 1..28: mol_type = other DNA
ggccggctcgggcccgggcaactaacgg

SEQ ID NO: 41900 - DNA, 28 bp, synthetic construct
  source 1..28: mol_type = other DNA
gttagttgcccgggcccgagccggccgg

SEQ ID NO: 41901 - DNA, 28 bp, synthetic construct
  source 1..28: mol_type = other DNA
ttagttgcccgggcccgagccggccggg

SEQ ID NO: 41902 - DNA, 28 bp, synthetic construct
  source 1..28: mol_type = other DNA
cccgggcccgagccggccgggcccgcgg

SEQ ID NO: 41903 - DNA, 28 bp, synthetic construct
  source 1..28: mol_type = other DNA
ccgggcccgagccggccgggcccgcggg

SEQ ID NO: 41904 - DNA, 28 bp, synthetic construct
  source 1..28: mol_type = other DNA
ggcaacccgcgggcccggccggctcggg

SEQ ID NO: 41905 - DNA, 28 bp, synthetic construct
  source 1..28: mol_type = other DNA
cggcaacccgcgggcccggccggctcgg

SEQ ID NO: 41906 - DNA, 28 bp, synthetic construct
  source 1..28: mol_type = other DNA
gggctcggcaacccgcgggcccggccgg

SEQ ID NO: 41907 - DNA, 28 bp, synthetic construct
  source 1..28: mol_type = other DNA
cagcgggctcggcaacccgcgggcccgg

SEQ ID NO: 41908 - DNA, 28 bp, synthetic construct
  source 1..28: mol_type = other DNA
gacgtcagcgggctcggcaacccgcggg

SEQ ID NO: 41909 - DNA, 28 bp, synthetic construct
  source 1..28: mol_type = other DNA
tgacgtcagcgggctcggcaacccgcgg

SEQ ID NO: 41910 - DNA, 28 bp, synthetic construct
  source 1..28: mol_type = other DNA
gttgccgagcccgctgacgtcagcccgg

SEQ ID NO: 41911 - DNA, 28 bp, synthetic construct
  source 1..28: mol_type = other DNA
ttgccgagcccgctgacgtcagcccggg

SEQ ID NO: 41912 - DNA, 28 bp, synthetic construct
  source 1..28: mol_type = other DNA
aaacccgggctgacgtcagcgggctcgg

SEQ ID NO: 41913 - DNA, 28 bp, synthetic construct
  source 1..28: mol_type = other DNA
gggggaaacccgggctgacgtcagcggg

SEQ ID NO: 41914 - DNA, 28 bp, synthetic construct
  source 1..28: mol_type = other DNA
ggggggaaacccgggctgacgtcagcgg

SEQ ID NO: 41915 - DNA, 28 bp, synthetic construct
  source 1..28: mol_type = other DNA
gtcagcccgggtttcccccccccaccgg

SEQ ID NO: 41916 - DNA, 28 bp, synthetic construct
  source 1..28: mol_type = other DNA
tcagcccgggtttcccccccccaccggg

SEQ ID NO: 41917 - DNA, 28 bp, synthetic construct
  source 1..28: mol_type = other DNA
cagcccgggtttcccccccccaccgggg

SEQ ID NO: 41918 - DNA, 28 bp, synthetic construct
  source 1..28: mol_type = other DNA
aagccccggtgggggggggaaacccggg

SEQ ID NO: 41919 - DNA, 28 bp, synthetic construct
  source 1..28: mol_type = other DNA
gaagccccggtgggggggggaaacccgg

SEQ ID NO: 41920 - DNA, 28 bp, synthetic construct
  source 1..28: mol_type = other DNA
gggatggggaagccccggtggggggggg

SEQ ID NO: 41921 - DNA, 28 bp, synthetic construct
  source 1..28: mol_type = other DNA
ggggatggggaagccccggtgggggggg

SEQ ID NO: 41922 - DNA, 28 bp, synthetic construct
  source 1..28: mol_type = other DNA
gggggatggggaagccccggtggggggg

SEQ ID NO: 41923 - DNA, 28 bp, synthetic construct
  source 1..28: mol_type = other DNA
cgggggatggggaagccccggtgggggg

SEQ ID NO: 41924 - DNA, 28 bp, synthetic construct
  source 1..28: mol_type = other DNA
tcgggggatggggaagccccggtggggg

SEQ ID NO: 41925 - DNA, 28 bp, synthetic construct
  source 1..28: mol_type = other DNA
ctcgggggatggggaagccccggtgggg

SEQ ID NO: 41926 - DNA, 28 bp, synthetic construct
  source 1..28: mol_type = other DNA
cctcgggggatggggaagccccggtggg

SEQ ID NO: 41927 - DNA, 28 bp, synthetic construct
  source 1..28: mol_type = other DNA
gcctcgggggatggggaagccccggtgg

SEQ ID NO: 41928 - DNA, 28 bp, synthetic construct
  source 1..28: mol_type = other DNA
gaagcctcgggggatggggaagccccgg

SEQ ID NO: 41929 - DNA, 28 bp, synthetic construct
  source 1..28: mol_type = other DNA
ggcttccccatcccccgaggcttcccgg

SEQ ID NO: 41930 - DNA, 28 bp, synthetic construct
  source 1..28: mol_type = other DNA
gcttccccatcccccgaggcttcccggg

SEQ ID NO: 41931 - DNA, 28 bp, synthetic construct
  source 1..28: mol_type = other DNA
tccccatcccccgaggcttcccgggagg

SEQ ID NO: 41932 - DNA, 28 bp, synthetic construct
  source 1..28: mol_type = other DNA
ccctcccgggaagcctcgggggatgggg

SEQ ID NO: 41933 - DNA, 28 bp, synthetic construct
  source 1..28: mol_type = other DNA
gccctcccgggaagcctcgggggatggg

SEQ ID NO: 41934 - DNA, 28 bp, synthetic construct
  source 1..28: mol_type = other DNA
agccctcccgggaagcctcgggggatgg

SEQ ID NO: 41935 - DNA, 28 bp, synthetic construct
  source 1..28: mol_type = other DNA
tcgcagccctcccgggaagcctcggggg

SEQ ID NO: 41936 - DNA, 28 bp, synthetic construct
  source 1..28: mol_type = other DNA
ctcgcagccctcccgggaagcctcgggg

SEQ ID NO: 41937 - DNA, 28 bp, synthetic construct
  source 1..28: mol_type = other DNA
actcgcagccctcccgggaagcctcggg

SEQ ID NO: 41938 - DNA, 28 bp, synthetic construct
  source 1..28: mol_type = other DNA
gactcgcagccctcccgggaagcctcgg

SEQ ID NO: 41939 - DNA, 28 bp, synthetic construct
  source 1..28: mol_type = other DNA
aggcttcccgggagggctgcgagtccgg

SEQ ID NO: 41940 - DNA, 28 bp, synthetic construct
  source 1..28: mol_type = other DNA
ggcttcccgggagggctgcgagtccggg

SEQ ID NO: 41941 - DNA, 28 bp, synthetic construct
  source 1..28: mol_type = other DNA
gcttcccgggagggctgcgagtccgggg

SEQ ID NO: 41942 - DNA, 28 bp, synthetic construct
  source 1..28: mol_type = other DNA
cgctccccggactcgcagccctcccggg

SEQ ID NO: 41943 - DNA, 28 bp, synthetic construct
  source 1..28: mol_type = other DNA
acgctccccggactcgcagccctcccgg

SEQ ID NO: 41944 - DNA, 28 bp, synthetic construct
  source 1..28: mol_type = other DNA
gagggctgcgagtccggggagcgtgcgg

SEQ ID NO: 41945 - DNA, 28 bp, synthetic construct
  source 1..28: mol_type = other DNA
agggctgcgagtccggggagcgtgcggg

SEQ ID NO: 41946 - DNA, 28 bp, synthetic construct
  source 1..28: mol_type = other DNA
gggctgcgagtccggggagcgtgcgggg

SEQ ID NO: 41947 - DNA, 28 bp, synthetic construct
  source 1..28: mol_type = other DNA
gatggtggcgaccccgcacgctccccgg

SEQ ID NO: 41948 - DNA, 28 bp, synthetic construct
  source 1..28: mol_type = other DNA
ggggagcgtgcggggtcgccaccatcgg

SEQ ID NO: 41949 - DNA, 28 bp, synthetic construct
  source 1..28: mol_type = other DNA
gggagcgtgcggggtcgccaccatcggg

SEQ ID NO: 41950 - DNA, 28 bp, synthetic construct
  source 1..28: mol_type = other DNA
gggtcgccaccatcgggacccccagagg

SEQ ID NO: 41951 - DNA, 28 bp, synthetic construct
  source 1..28: mol_type = other DNA
ctctctcctctgggggtcccgatggtgg

SEQ ID NO: 41952 - DNA, 28 bp, synthetic construct
  source 1..28: mol_type = other DNA
caccatcgggacccccagaggagagagg

SEQ ID NO: 41953 - DNA, 28 bp, synthetic construct
  source 1..28: mol_type = other DNA
gtcctctctcctctgggggtcccgatgg

SEQ ID NO: 41954 - DNA, 28 bp, synthetic construct
  source 1..28: mol_type = other DNA
cgggacccccagaggagagaggacttgg

SEQ ID NO: 41955 - DNA, 28 bp, synthetic construct
  source 1..28: mol_type = other DNA
gggacccccagaggagagaggacttggg

SEQ ID NO: 41956 - DNA, 28 bp, synthetic construct
  source 1..28: mol_type = other DNA
ggacccccagaggagagaggacttgggg

SEQ ID NO: 41957 - DNA, 28 bp, synthetic construct
  source 1..28: mol_type = other DNA
cccccagaggagagaggacttggggcgg

SEQ ID NO: 41958 - DNA, 28 bp, synthetic construct
  source 1..28: mol_type = other DNA
cccgccccaagtcctctctcctctgggg

SEQ ID NO: 41959 - DNA, 28 bp, synthetic construct
  source 1..28: mol_type = other DNA
tcccgccccaagtcctctctcctctggg

SEQ ID NO: 41960 - DNA, 28 bp, synthetic construct
  source 1..28: mol_type = other DNA
ctcccgccccaagtcctctctcctctgg

SEQ ID NO: 41961 - DNA, 28 bp, synthetic construct
  source 1..28: mol_type = other DNA
gagaggacttggggcgggagccgcgcgg

SEQ ID NO: 41962 - DNA, 28 bp, synthetic construct
  source 1..28: mol_type = other DNA
agaggacttggggcgggagccgcgcggg

SEQ ID NO: 41963 - DNA, 28 bp, synthetic construct
  source 1..28: mol_type = other DNA
ggcgggagggggacagcgtcccgcgcgg

SEQ ID NO: 41964 - DNA, 28 bp, synthetic construct
  source 1..28: mol_type = other DNA
tgtaaatggggtggggggcgggaggggg

SEQ ID NO: 41965 - DNA, 28 bp, synthetic construct
  source 1..28: mol_type = other DNA
ctgtaaatggggtggggggcgggagggg

SEQ ID NO: 41966 - DNA, 28 bp, synthetic construct
  source 1..28: mol_type = other DNA
tctgtaaatggggtggggggcgggaggg

SEQ ID NO: 41967 - DNA, 28 bp, synthetic construct
  source 1..28: mol_type = other DNA
atctgtaaatggggtggggggcgggagg

SEQ ID NO: 41968 - DNA, 28 bp, synthetic construct
  source 1..28: mol_type = other DNA
cccgccccccaccccatttacagattgg

SEQ ID NO: 41969 - DNA, 28 bp, synthetic construct
  source 1..28: mol_type = other DNA
ccgccccccaccccatttacagattggg

SEQ ID NO: 41970 - DNA, 28 bp, synthetic construct
  source 1..28: mol_type = other DNA
tctcccaatctgtaaatggggtgggggg

SEQ ID NO: 41971 - DNA, 28 bp, synthetic construct
  source 1..28: mol_type = other DNA
gtctcccaatctgtaaatggggtggggg

SEQ ID NO: 41972 - DNA, 28 bp, synthetic construct
  source 1..28: mol_type = other DNA
agtctcccaatctgtaaatggggtgggg

SEQ ID NO: 41973 - DNA, 28 bp, synthetic construct
  source 1..28: mol_type = other DNA
cagtctcccaatctgtaaatggggtggg

SEQ ID NO: 41974 - DNA, 28 bp, synthetic construct
  source 1..28: mol_type = other DNA
tcagtctcccaatctgtaaatggggtgg

SEQ ID NO: 41975 - DNA, 28 bp, synthetic construct
  source 1..28: mol_type = other DNA
accccatttacagattgggagactgagg

SEQ ID NO: 41976 - DNA, 28 bp, synthetic construct
  source 1..28: mol_type = other DNA
gcctcagtctcccaatctgtaaatgggg

SEQ ID NO: 41977 - DNA, 28 bp, synthetic construct
  source 1..28: mol_type = other DNA
tgcctcagtctcccaatctgtaaatggg

SEQ ID NO: 41978 - DNA, 28 bp, synthetic construct
  source 1..28: mol_type = other DNA
gtgcctcagtctcccaatctgtaaatgg

SEQ ID NO: 41979 - DNA, 28 bp, synthetic construct
  source 1..28: mol_type = other DNA
tttacagattgggagactgaggcacagg

SEQ ID NO: 41980 - DNA, 28 bp, synthetic construct
  source 1..28: mol_type = other DNA
attgggagactgaggcacaggccgctgg

SEQ ID NO: 41981 - DNA, 28 bp, synthetic construct
  source 1..28: mol_type = other DNA
gggagactgaggcacaggccgctggcgg

SEQ ID NO: 41982 - DNA, 28 bp, synthetic construct
  source 1..28: mol_type = other DNA
ggagactgaggcacaggccgctggcggg

SEQ ID NO: 41983 - DNA, 28 bp, synthetic construct
  source 1..28: mol_type = other DNA
ggcacaggccgctggcgggccccgacgg

SEQ ID NO: 41984 - DNA, 28 bp, synthetic construct
  source 1..28: mol_type = other DNA
ggccgctggcgggccccgacggccacgg

SEQ ID NO: 41985 - DNA, 28 bp, synthetic construct
  source 1..28: mol_type = other DNA
aaccgtggccgtcggggcccgccagcgg

SEQ ID NO: 41986 - DNA, 28 bp, synthetic construct
  source 1..28: mol_type = other DNA
gctggcgggccccgacggccacggttgg

SEQ ID NO: 41987 - DNA, 28 bp, synthetic construct
  source 1..28: mol_type = other DNA
ggccccgacggccacggttggcctcagg

SEQ ID NO: 41988 - DNA, 28 bp, synthetic construct
  source 1..28: mol_type = other DNA
ctcctgaggccaaccgtggccgtcgggg

SEQ ID NO: 41989 - DNA, 28 bp, synthetic construct
  source 1..28: mol_type = other DNA
gctcctgaggccaaccgtggccgtcggg

SEQ ID NO: 41990 - DNA, 28 bp, synthetic construct
  source 1..28: mol_type = other DNA
ggctcctgaggccaaccgtggccgtcgg

SEQ ID NO: 41991 - DNA, 28 bp, synthetic construct
  source 1..28: mol_type = other DNA
acggccacggttggcctcaggagcccgg

SEQ ID NO: 41992 - DNA, 28 bp, synthetic construct
  source 1..28: mol_type = other DNA
cggccacggttggcctcaggagcccggg

SEQ ID NO: 41993 - DNA, 28 bp, synthetic construct
  source 1..28: mol_type = other DNA
ggccacggttggcctcaggagcccgggg

SEQ ID NO: 41994 - DNA, 28 bp, synthetic construct
  source 1..28: mol_type = other DNA
agccccgggctcctgaggccaaccgtgg

SEQ ID NO: 41995 - DNA, 28 bp, synthetic construct
  source 1..28: mol_type = other DNA
taggaatcacagccccgggctcctgagg

SEQ ID NO: 41996 - DNA, 28 bp, synthetic construct
  source 1..28: mol_type = other DNA
cgcggtcggtaggaatcacagccccggg

SEQ ID NO: 41997 - DNA, 28 bp, synthetic construct
  source 1..28: mol_type = other DNA
gcgcggtcggtaggaatcacagccccgg

SEQ ID NO: 41998 - DNA, 28 bp, synthetic construct
  source 1..28: mol_type = other DNA
gctgtgattcctaccgaccgcgccgcgg

SEQ ID NO: 41999 - DNA, 28 bp, synthetic construct
  source 1..28: mol_type = other DNA
ctgtgattcctaccgaccgcgccgcggg

SEQ ID NO: 42000 - DNA, 28 bp, synthetic construct
  source 1..28: mol_type = other DNA
tgtgattcctaccgaccgcgccgcgggg

SEQ ID NO: 42001 - DNA, 28 bp, synthetic construct
  source 1..28: mol_type = other DNA
acgtacgccccgcggcgcggtcggtagg

SEQ ID NO: 42002 - DNA, 28 bp, synthetic construct
  source 1..28: mol_type = other DNA
cggtacgtacgccccgcggcgcggtcgg

SEQ ID NO: 42003 - DNA, 28 bp, synthetic construct
  source 1..28: mol_type = other DNA
cgatcggtacgtacgccccgcggcgcgg

SEQ ID NO: 42004 - DNA, 28 bp, synthetic construct
  source 1..28: mol_type = other DNA
aaaatcgatcggtacgtacgccccgcgg

SEQ ID NO: 42005 - DNA, 28 bp, synthetic construct
  source 1..28: mol_type = other DNA
ggggcgtacgtaccgatcgattttgcgg

SEQ ID NO: 42006 - DNA, 28 bp, synthetic construct
  source 1..28: mol_type = other DNA
gggcgtacgtaccgatcgattttgcggg

SEQ ID NO: 42007 - DNA, 28 bp, synthetic construct
  source 1..28: mol_type = other DNA
acgtaccgatcgattttgcgggtgttgg

SEQ ID NO: 42008 - DNA, 28 bp, synthetic construct
  source 1..28: mol_type = other DNA
taccgatcgattttgcgggtgttggtgg

SEQ ID NO: 42009 - DNA, 28 bp, synthetic construct
  source 1..28: mol_type = other DNA
agccaccaacacccgcaaaatcgatcgg

SEQ ID NO: 42010 - DNA, 28 bp, synthetic construct
  source 1..28: mol_type = other DNA
ttgcgggtgttggtggctcccgtccagg

SEQ ID NO: 42011 - DNA, 28 bp, synthetic construct
  source 1..28: mol_type = other DNA
ggtgttggtggctcccgtccaggaatgg

SEQ ID NO: 42012 - DNA, 28 bp, synthetic construct
  source 1..28: mol_type = other DNA
gtggctcccgtccaggaatggcagtcgg

SEQ ID NO: 42013 - DNA, 28 bp, synthetic construct
  source 1..28: mol_type = other DNA
tggctcccgtccaggaatggcagtcggg

SEQ ID NO: 42014 - DNA, 28 bp, synthetic construct
  source 1..28: mol_type = other DNA
ggctcccgtccaggaatggcagtcgggg

SEQ ID NO: 42015 - DNA, 28 bp, synthetic construct
  source 1..28: mol_type = other DNA
agaaccccgactgccattcctggacggg

SEQ ID NO: 42016 - DNA, 28 bp, synthetic construct
  source 1..28: mol_type = other DNA
cagaaccccgactgccattcctggacgg

SEQ ID NO: 42017 - DNA, 28 bp, synthetic construct
  source 1..28: mol_type = other DNA
cgtccaggaatggcagtcggggttctgg

SEQ ID NO: 42018 - DNA, 28 bp, synthetic construct
  source 1..28: mol_type = other DNA
aggccagaaccccgactgccattcctgg

SEQ ID NO: 42019 - DNA, 28 bp, synthetic construct
  source 1..28: mol_type = other DNA
gcagtcggggttctggccttgttaatgg

SEQ ID NO: 42020 - DNA, 28 bp, synthetic construct
  source 1..28: mol_type = other DNA
gaaaaagcagaacacgccattaacaagg

SEQ ID NO: 42021 - DNA, 28 bp, synthetic construct
  source 1..28: mol_type = other DNA
tttttctttcagtttccccctttctagg

SEQ ID NO: 42022 - DNA, 28 bp, synthetic construct
  source 1..28: mol_type = other DNA
ttttctttcagtttccccctttctaggg

SEQ ID NO: 42023 - DNA, 28 bp, synthetic construct
  source 1..28: mol_type = other DNA
tttcagtttccccctttctagggtgagg

SEQ ID NO: 42024 - DNA, 28 bp, synthetic construct
  source 1..28: mol_type = other DNA
agtttccccctttctagggtgaggatgg

SEQ ID NO: 42025 - DNA, 28 bp, synthetic construct
  source 1..28: mol_type = other DNA
tagaaccatcctcaccctagaaaggggg

SEQ ID NO: 42026 - DNA, 28 bp, synthetic construct
  source 1..28: mol_type = other DNA
gtagaaccatcctcaccctagaaagggg

SEQ ID NO: 42027 - DNA, 28 bp, synthetic construct
  source 1..28: mol_type = other DNA
tgtagaaccatcctcaccctagaaaggg

SEQ ID NO: 42028 - DNA, 28 bp, synthetic construct
  source 1..28: mol_type = other DNA
gtgtagaaccatcctcaccctagaaagg

SEQ ID NO: 42029 - DNA, 28 bp, synthetic construct
  source 1..28: mol_type = other DNA
gtgaggatggttctacacagccacccgg

SEQ ID NO: 42030 - DNA, 28 bp, synthetic construct
  source 1..28: mol_type = other DNA
agccacccggagttccttagttgaaagg

SEQ ID NO: 42031 - DNA, 28 bp, synthetic construct
  source 1..28: mol_type = other DNA
cacctttcaactaaggaactccgggtgg

SEQ ID NO: 42032 - DNA, 28 bp, synthetic construct
  source 1..28: mol_type = other DNA
gcgcacctttcaactaaggaactccggg

SEQ ID NO: 42033 - DNA, 28 bp, synthetic construct
  source 1..28: mol_type = other DNA
ggcgcacctttcaactaaggaactccgg

SEQ ID NO: 42034 - DNA, 28 bp, synthetic construct
  source 1..28: mol_type = other DNA
cacagcagggcgcacctttcaactaagg

SEQ ID NO: 42035 - DNA, 28 bp, synthetic construct
  source 1..28: mol_type = other DNA
gttgaaaggtgcgccctgctgtgacagg

SEQ ID NO: 42036 - DNA, 28 bp, synthetic construct
  source 1..28: mol_type = other DNA
taaagaaagaatacctgtcacagcaggg

SEQ ID NO: 42037 - DNA, 28 bp, synthetic construct
  source 1..28: mol_type = other DNA
ataaagaaagaatacctgtcacagcagg

SEQ ID NO: 42038 - DNA, 28 bp, synthetic construct
  source 1..28: mol_type = other DNA
tgtttttctttcatgttaacaatcgagg

SEQ ID NO: 42039 - DNA, 28 bp, synthetic construct
  source 1..28: mol_type = other DNA
gtttttctttcatgttaacaatcgaggg

SEQ ID NO: 42040 - DNA, 28 bp, synthetic construct
  source 1..28: mol_type = other DNA
tttttctttcatgttaacaatcgagggg

SEQ ID NO: 42041 - DNA, 28 bp, synthetic construct
  source 1..28: mol_type = other DNA
ttttctttcatgttaacaatcgaggggg

SEQ ID NO: 42042 - DNA, 28 bp, synthetic construct
  source 1..28: mol_type = other DNA
tttctttcatgttaacaatcgagggggg

SEQ ID NO: 42043 - DNA, 28 bp, synthetic construct
  source 1..28: mol_type = other DNA
ctttcatgttaacaatcgaggggggtgg

SEQ ID NO: 42044 - DNA, 28 bp, synthetic construct
  source 1..28: mol_type = other DNA
tttcatgttaacaatcgaggggggtggg

SEQ ID NO: 42045 - DNA, 28 bp, synthetic construct
  source 1..28: mol_type = other DNA
ttcatgttaacaatcgaggggggtgggg

SEQ ID NO: 42046 - DNA, 28 bp, synthetic construct
  source 1..28: mol_type = other DNA
tcatgttaacaatcgaggggggtggggg

SEQ ID NO: 42047 - DNA, 28 bp, synthetic construct
  source 1..28: mol_type = other DNA
catgttaacaatcgaggggggtgggggg

SEQ ID NO: 42048 - DNA, 28 bp, synthetic construct
  source 1..28: mol_type = other DNA
acaatcgaggggggtggggggcgaatgg

SEQ ID NO: 42049 - DNA, 28 bp, synthetic construct
  source 1..28: mol_type = other DNA
caatcgaggggggtggggggcgaatggg

SEQ ID NO: 42050 - DNA, 28 bp, synthetic construct
  source 1..28: mol_type = other DNA
aatcgaggggggtggggggcgaatgggg

SEQ ID NO: 42051 - DNA, 28 bp, synthetic construct
  source 1..28: mol_type = other DNA
atcgaggggggtggggggcgaatggggg

SEQ ID NO: 42052 - DNA, 28 bp, synthetic construct
  source 1..28: mol_type = other DNA
tcgaggggggtggggggcgaatgggggg

SEQ ID NO: 42053 - DNA, 28 bp, synthetic construct
  source 1..28: mol_type = other DNA
aggggggtggggggcgaatggggggcgg

SEQ ID NO: 42054 - DNA, 28 bp, synthetic construct
  source 1..28: mol_type = other DNA
ggggggtggggggcgaatggggggcggg

SEQ ID NO: 42055 - DNA, 28 bp, synthetic construct
  source 1..28: mol_type = other DNA
gggggtggggggcgaatggggggcgggg

SEQ ID NO: 42056 - DNA, 28 bp, synthetic construct
  source 1..28: mol_type = other DNA
ggggtggggggcgaatggggggcggggg

SEQ ID NO: 42057 - DNA, 28 bp, synthetic construct
  source 1..28: mol_type = other DNA
gcgggggcgaagtcatgaaatcttcagg

SEQ ID NO: 42058 - DNA, 28 bp, synthetic construct
  source 1..28: mol_type = other DNA
gcgaagtcatgaaatcttcaggagatgg

SEQ ID NO: 42059 - DNA, 28 bp, synthetic construct
  source 1..28: mol_type = other DNA
aatcttcaggagatggtgttgagtttgg

SEQ ID NO: 42060 - DNA, 28 bp, synthetic construct
  source 1..28: mol_type = other DNA
gatggtgttgagtttggtactcagctgg

SEQ ID NO: 42061 - DNA, 28 bp, synthetic construct
  source 1..28: mol_type = other DNA
atggtgttgagtttggtactcagctggg

SEQ ID NO: 42062 - DNA, 28 bp, synthetic construct
  source 1..28: mol_type = other DNA
aagttatcaggttatattgttcataagg

SEQ ID NO: 42063 - DNA, 28 bp, synthetic construct
  source 1..28: mol_type = other DNA
gtgtttttctgattctcaagttatcagg

SEQ ID NO: 42064 - DNA, 28 bp, synthetic construct
  source 1..28: mol_type = other DNA
agaatcagaaaaacactgcatcttctgg

SEQ ID NO: 42065 - DNA, 28 bp, synthetic construct
  source 1..28: mol_type = other DNA
atcagtagctacagaaaactaacaatgg

SEQ ID NO: 42066 - DNA, 28 bp, synthetic construct
  source 1..28: mol_type = other DNA
gtactatatgttgcctttcagaatgtgg

SEQ ID NO: 42067 - DNA, 28 bp, synthetic construct
  source 1..28: mol_type = other DNA
aagattacaattaccacattctgaaagg

SEQ ID NO: 42068 - DNA, 28 bp, synthetic construct
  source 1..28: mol_type = other DNA
ccatgaagacaatggaaagatgatcagg

SEQ ID NO: 42069 - DNA, 28 bp, synthetic construct
  source 1..28: mol_type = other DNA
atttatcaattttccatgaagacaatgg

SEQ ID NO: 42070 - DNA, 28 bp, synthetic construct
  source 1..28: mol_type = other DNA
tatttgtgccttccaactctcgtcttgg

SEQ ID NO: 42071 - DNA, 28 bp, synthetic construct
  source 1..28: mol_type = other DNA
tcattcaaccaagacgagagttggaagg

SEQ ID NO: 42072 - DNA, 28 bp, synthetic construct
  source 1..28: mol_type = other DNA
gaagtcattcaaccaagacgagagttgg

SEQ ID NO: 42073 - DNA, 28 bp, synthetic construct
  source 1..28: mol_type = other DNA
ttgatggtctggattctgagtaaagggg

SEQ ID NO: 42074 - DNA, 28 bp, synthetic construct
  source 1..28: mol_type = other DNA
gttgatggtctggattctgagtaaaggg

SEQ ID NO: 42075 - DNA, 28 bp, synthetic construct
  source 1..28: mol_type = other DNA
tgttgatggtctggattctgagtaaagg

SEQ ID NO: 42076 - DNA, 28 bp, synthetic construct
  source 1..28: mol_type = other DNA
tggttatctgagcttgttgatggtctgg

SEQ ID NO: 42077 - DNA, 28 bp, synthetic construct
  source 1..28: mol_type = other DNA
atttctggttatctgagcttgttgatgg

SEQ ID NO: 42078 - DNA, 28 bp, synthetic construct
  source 1..28: mol_type = other DNA
gttcacatagatttgaaaacatttctgg

SEQ ID NO: 42079 - DNA, 28 bp, synthetic construct
  source 1..28: mol_type = other DNA
ggacgctgatgaaggagaacagttcagg

SEQ ID NO: 42080 - DNA, 28 bp, synthetic construct
  source 1..28: mol_type = other DNA
tgttctccttcatcagcgtccttaaagg

SEQ ID NO: 42081 - DNA, 28 bp, synthetic construct
  source 1..28: mol_type = other DNA
tccttcatcagcgtccttaaaggaaagg

SEQ ID NO: 42082 - DNA, 28 bp, synthetic construct
  source 1..28: mol_type = other DNA
gcctttcctttaaggacgctgatgaagg

SEQ ID NO: 42083 - DNA, 28 bp, synthetic construct
  source 1..28: mol_type = other DNA
atttcatttgtgtgtatgtgtttactgg

SEQ ID NO: 42084 - DNA, 28 bp, synthetic construct
  source 1..28: mol_type = other DNA
taaagtttatttttgctttttcactagg

SEQ ID NO: 42085 - DNA, 28 bp, synthetic construct
  source 1..28: mol_type = other DNA
tttgatttcctttctttttacagcatgg

SEQ ID NO: 42086 - DNA, 28 bp, synthetic construct
  source 1..28: mol_type = other DNA
cgtggtgtccatgctgtaaaaagaaagg

SEQ ID NO: 42087 - DNA, 28 bp, synthetic construct
  source 1..28: mol_type = other DNA
acaccacgttgctgaaaacatgctttgg

SEQ ID NO: 42088 - DNA, 28 bp, synthetic construct
  source 1..28: mol_type = other DNA
caccacgttgctgaaaacatgctttggg

SEQ ID NO: 42089 - DNA, 28 bp, synthetic construct
  source 1..28: mol_type = other DNA
gtcccaaagcatgttttcagcaacgtgg

SEQ ID NO: 42090 - DNA, 28 bp, synthetic construct
  source 1..28: mol_type = other DNA
ggactgccactgaatttatcttttgcgg

SEQ ID NO: 42091 - DNA, 28 bp, synthetic construct
  source 1..28: mol_type = other DNA
ataaaaccgcaaaagataaattcagtgg

SEQ ID NO: 42092 - DNA, 28 bp, synthetic construct
  source 1..28: mol_type = other DNA
aacttcaaaatactaattcaaaaaaggg

SEQ ID NO: 42093 - DNA, 28 bp, synthetic construct
  source 1..28: mol_type = other DNA
taacttcaaaatactaattcaaaaaagg

SEQ ID NO: 42094 - DNA, 28 bp, synthetic construct
  source 1..28: mol_type = other DNA
ttgaagttaatatcacaatgagttcagg

SEQ ID NO: 42095 - DNA, 28 bp, synthetic construct
  source 1..28: mol_type = other DNA
taatatcacaatgagttcaggcttatgg

SEQ ID NO: 42096 - DNA, 28 bp, synthetic construct
  source 1..28: mol_type = other DNA
ccagtagggtgaagtgactttttcttgg

SEQ ID NO: 42097 - DNA, 28 bp, synthetic construct
  source 1..28: mol_type = other DNA
caagaaaaagtcacttcaccctactggg

SEQ ID NO: 42098 - DNA, 28 bp, synthetic construct
  source 1..28: mol_type = other DNA
agtcacttcaccctactgggaagagcgg

SEQ ID NO: 42099 - DNA, 28 bp, synthetic construct
  source 1..28: mol_type = other DNA
agtaaaaaatccgctcttcccagtaggg

SEQ ID NO: 42100 - DNA, 28 bp, synthetic construct
  source 1..28: mol_type = other DNA
aagtaaaaaatccgctcttcccagtagg

SEQ ID NO: 42101 - DNA, 28 bp, synthetic construct
  source 1..28: mol_type = other DNA
acacaaaagctccttaaagtaccgaagg

SEQ ID NO: 42102 - DNA, 28 bp, synthetic construct
  source 1..28: mol_type = other DNA
cacaaaagctccttaaagtaccgaaggg

SEQ ID NO: 42103 - DNA, 28 bp, synthetic construct
  source 1..28: mol_type = other DNA
tccttaaagtaccgaagggaagtatagg

SEQ ID NO: 42104 - DNA, 28 bp, synthetic construct
  source 1..28: mol_type = other DNA
tcctatacttcccttcggtactttaagg

SEQ ID NO: 42105 - DNA, 28 bp, synthetic construct
  source 1..28: mol_type = other DNA
gaatatactgtcctatacttcccttcgg

SEQ ID NO: 42106 - DNA, 28 bp, synthetic construct
  source 1..28: mol_type = other DNA
ggacagtatattcaagatcgttctgtgg

SEQ ID NO: 42107 - DNA, 28 bp, synthetic construct
  source 1..28: mol_type = other DNA
gacagtatattcaagatcgttctgtggg

SEQ ID NO: 42108 - DNA, 28 bp, synthetic construct
  source 1..28: mol_type = other DNA
acagtatattcaagatcgttctgtgggg

SEQ ID NO: 42109 - DNA, 28 bp, synthetic construct
  source 1..28: mol_type = other DNA
tcaagatcgttctgtggggcattcaagg

SEQ ID NO: 42110 - DNA, 28 bp, synthetic construct
  source 1..28: mol_type = other DNA
ggcattcaaggattccttctgcaaaagg

SEQ ID NO: 42111 - DNA, 28 bp, synthetic construct
  source 1..28: mol_type = other DNA
tctgatttttcttgccttttgcagaagg

SEQ ID NO: 42112 - DNA, 28 bp, synthetic construct
  source 1..28: mol_type = other DNA
ctgcaaaaggcaagaaaaatcagattgg

SEQ ID NO: 42113 - DNA, 28 bp, synthetic construct
  source 1..28: mol_type = other DNA
tttcatcaacaaagagaactgcatgagg

SEQ ID NO: 42114 - DNA, 28 bp, synthetic construct
  source 1..28: mol_type = other DNA
catgcagttctctttgttgatgaaaagg

SEQ ID NO: 42115 - DNA, 28 bp, synthetic construct
  source 1..28: mol_type = other DNA
aatgaaaagttcacagagttacttttgg

SEQ ID NO: 42116 - DNA, 28 bp, synthetic construct
  source 1..28: mol_type = other DNA
ttacttttggcaattaccaattgtgagg

SEQ ID NO: 42117 - DNA, 28 bp, synthetic construct
  source 1..28: mol_type = other DNA
tttggcaattaccaattgtgaggagagg

SEQ ID NO: 42118 - DNA, 28 bp, synthetic construct
  source 1..28: mol_type = other DNA
aacaggctgaacctctcctcacaattgg

SEQ ID NO: 42119 - DNA, 28 bp, synthetic construct
  source 1..28: mol_type = other DNA
acttagtctgtttctgtttttaaacagg

SEQ ID NO: 42120 - DNA, 28 bp, synthetic construct
  source 1..28: mol_type = other DNA
ttaaaaacagaaacagactaagtaaagg

SEQ ID NO: 42121 - DNA, 28 bp, synthetic construct
  source 1..28: mol_type = other DNA
ctaagtaaaggcctccaaatagacgtgg

SEQ ID NO: 42122 - DNA, 28 bp, synthetic construct
  source 1..28: mol_type = other DNA
taagtaaaggcctccaaatagacgtggg

SEQ ID NO: 42123 - DNA, 28 bp, synthetic construct
  source 1..28: mol_type = other DNA
cacaggacagcccacgtctatttggagg

SEQ ID NO: 42124 - DNA, 28 bp, synthetic construct
  source 1..28: mol_type = other DNA
tttcacaggacagcccacgtctatttgg

SEQ ID NO: 42125 - DNA, 28 bp, synthetic construct
  source 1..28: mol_type = other DNA
gtcctgtgaaagtacagctgagatctgg

SEQ ID NO: 42126 - DNA, 28 bp, synthetic construct
  source 1..28: mol_type = other DNA
tcctgtgaaagtacagctgagatctggg

SEQ ID NO: 42127 - DNA, 28 bp, synthetic construct
  source 1..28: mol_type = other DNA
cctgtgaaagtacagctgagatctgggg

SEQ ID NO: 42128 - DNA, 28 bp, synthetic construct
  source 1..28: mol_type = other DNA
tgagatctggggaagaaaaatttcctgg

SEQ ID NO: 42129 - DNA, 28 bp, synthetic construct
  source 1..28: mol_type = other DNA
aatttcctggagttgtacgcttcagagg

SEQ ID NO: 42130 - DNA, 28 bp, synthetic construct
  source 1..28: mol_type = other DNA
ggggtcctctgaagcgtacaactccagg

SEQ ID NO: 42131 - DNA, 28 bp, synthetic construct
  source 1..28: mol_type = other DNA
cttcagaggacccctgttagcagagagg

SEQ ID NO: 42132 - DNA, 28 bp, synthetic construct
  source 1..28: mol_type = other DNA
cggagactgtcctctctgctaacagggg

SEQ ID NO: 42133 - DNA, 28 bp, synthetic construct
  source 1..28: mol_type = other DNA
ccggagactgtcctctctgctaacaggg

SEQ ID NO: 42134 - DNA, 28 bp, synthetic construct
  source 1..28: mol_type = other DNA
tccggagactgtcctctctgctaacagg

SEQ ID NO: 42135 - DNA, 28 bp, synthetic construct
  source 1..28: mol_type = other DNA
agaggacagtctccggaatattctttgg

SEQ ID NO: 42136 - DNA, 28 bp, synthetic construct
  source 1..28: mol_type = other DNA
agcaattcaactccaaagaatattccgg

SEQ ID NO: 42137 - DNA, 28 bp, synthetic construct
  source 1..28: mol_type = other DNA
ggaatattctttggagttgaattgctgg

SEQ ID NO: 42138 - DNA, 28 bp, synthetic construct
  source 1..28: mol_type = other DNA
aacacaaacaaacacactactaaaatgg

SEQ ID NO: 42139 - DNA, 28 bp, synthetic construct
  source 1..28: mol_type = other DNA
cttgggaaaatttatttcgtatttaagg

SEQ ID NO: 42140 - DNA, 28 bp, synthetic construct
  source 1..28: mol_type = other DNA
tctagggatttcaggaaaatcactctgg

SEQ ID NO: 42141 - DNA, 28 bp, synthetic construct
  source 1..28: mol_type = other DNA
aaaaggggttcactctagggatttcagg

SEQ ID NO: 42142 - DNA, 28 bp, synthetic construct
  source 1..28: mol_type = other DNA
tccctagagtgaaccccttttcctatgg

SEQ ID NO: 42143 - DNA, 28 bp, synthetic construct
  source 1..28: mol_type = other DNA
tccataggaaaaggggttcactctaggg

SEQ ID NO: 42144 - DNA, 28 bp, synthetic construct
  source 1..28: mol_type = other DNA
atccataggaaaaggggttcactctagg

SEQ ID NO: 42145 - DNA, 28 bp, synthetic construct
  source 1..28: mol_type = other DNA
atagaaagacgatccataggaaaagggg

SEQ ID NO: 42146 - DNA, 28 bp, synthetic construct
  source 1..28: mol_type = other DNA
tatagaaagacgatccataggaaaaggg

SEQ ID NO: 42147 - DNA, 28 bp, synthetic construct
  source 1..28: mol_type = other DNA
atatagaaagacgatccataggaaaagg

SEQ ID NO: 42148 - DNA, 28 bp, synthetic construct
  source 1..28: mol_type = other DNA
aaatagatatagaaagacgatccatagg

SEQ ID NO: 42149 - DNA, 28 bp, synthetic construct
  source 1..28: mol_type = other DNA
ttctttcccttctctcttaaaaactagg

SEQ ID NO: 42150 - DNA, 28 bp, synthetic construct
  source 1..28: mol_type = other DNA
cttcttcctagtttttaagagagaaggg

SEQ ID NO: 42151 - DNA, 28 bp, synthetic construct
  source 1..28: mol_type = other DNA
ccttcttcctagtttttaagagagaagg

SEQ ID NO: 42152 - DNA, 28 bp, synthetic construct
  source 1..28: mol_type = other DNA
ctcttaaaaactaggaagaaggtcgtgg

SEQ ID NO: 42153 - DNA, 28 bp, synthetic construct
  source 1..28: mol_type = other DNA
aaaactaggaagaaggtcgtggtcaagg

SEQ ID NO: 42154 - DNA, 28 bp, synthetic construct
  source 1..28: mol_type = other DNA
aaggtcgtggtcaaggtttcactgacgg

SEQ ID NO: 42155 - DNA, 28 bp, synthetic construct
  source 1..28: mol_type = other DNA
aggtcgtggtcaaggtttcactgacggg

SEQ ID NO: 42156 - DNA, 28 bp, synthetic construct
  source 1..28: mol_type = other DNA
ggtcgtggtcaaggtttcactgacgggg

SEQ ID NO: 42157 - DNA, 28 bp, synthetic construct
  source 1..28: mol_type = other DNA
aaggtttcactgacggggtgtaccaagg

SEQ ID NO: 42158 - DNA, 28 bp, synthetic construct
  source 1..28: mol_type = other DNA
aggtttcactgacggggtgtaccaaggg

SEQ ID NO: 42159 - DNA, 28 bp, synthetic construct
  source 1..28: mol_type = other DNA
atcacactgaaaaagctgtttcccttgg

SEQ ID NO: 42160 - DNA, 28 bp, synthetic construct
  source 1..28: mol_type = other DNA
agctttttcagtgtgatgaagattgtgg

SEQ ID NO: 42161 - DNA, 28 bp, synthetic construct
  source 1..28: mol_type = other DNA
gaagattgtggcgtgtttgttgcattgg

SEQ ID NO: 42162 - DNA, 28 bp, synthetic construct
  source 1..28: mol_type = other DNA
ctcatagaagatgatgacactgcattgg

SEQ ID NO: 42163 - DNA, 28 bp, synthetic construct
  source 1..28: mol_type = other DNA
acactgcattggaaagtgattacgcagg

SEQ ID NO: 42164 - DNA, 28 bp, synthetic construct
  source 1..28: mol_type = other DNA
cattggaaagtgattacgcaggtcctgg

SEQ ID NO: 42165 - DNA, 28 bp, synthetic construct
  source 1..28: mol_type = other DNA
attggaaagtgattacgcaggtcctggg

SEQ ID NO: 42166 - DNA, 28 bp, synthetic construct
  source 1..28: mol_type = other DNA
ttggaaagtgattacgcaggtcctgggg

SEQ ID NO: 42167 - DNA, 28 bp, synthetic construct
  source 1..28: mol_type = other DNA
tacgcaggtcctggggacacaatgcagg

SEQ ID NO: 42168 - DNA, 28 bp, synthetic construct
  source 1..28: mol_type = other DNA
gaagttcgacctgcattgtgtccccagg

SEQ ID NO: 42169 - DNA, 28 bp, synthetic construct
  source 1..28: mol_type = other DNA
acaatgcaggtcgaacttcctcctttgg

SEQ ID NO: 42170 - DNA, 28 bp, synthetic construct
  source 1..28: mol_type = other DNA
aaactctggagtttatttccaaaggagg

SEQ ID NO: 42171 - DNA, 28 bp, synthetic construct
  source 1..28: mol_type = other DNA
aagaaactctggagtttatttccaaagg

SEQ ID NO: 42172 - DNA, 28 bp, synthetic construct
  source 1..28: mol_type = other DNA
gaaataaactccagagtttctttgaagg

SEQ ID NO: 42173 - DNA, 28 bp, synthetic construct
  source 1..28: mol_type = other DNA
taaactccagagtttctttgaaggttgg

SEQ ID NO: 42174 - DNA, 28 bp, synthetic construct
  source 1..28: mol_type = other DNA
gtttctccaaccttcaaagaaactctgg

SEQ ID NO: 42175 - DNA, 28 bp, synthetic construct
  source 1..28: mol_type = other DNA
tgaaggttggagaaacaatagaatctgg

SEQ ID NO: 42176 - DNA, 28 bp, synthetic construct
  source 1..28: mol_type = other DNA
cagttatattctgtgatgttttgccagg

SEQ ID NO: 42177 - DNA, 28 bp, synthetic construct
  source 1..28: mol_type = other DNA
atgttttgccaggaaaagaaagcttagg

SEQ ID NO: 42178 - DNA, 28 bp, synthetic construct
  source 1..28: mol_type = other DNA
caaaatatcctaagctttcttttcctgg

SEQ ID NO: 42179 - DNA, 28 bp, synthetic construct
  source 1..28: mol_type = other DNA
gaaaagaaagcttaggatattttgttgg

SEQ ID NO: 42180 - DNA, 28 bp, synthetic construct
  source 1..28: mol_type = other DNA
gaaagcttaggatattttgttggtgtgg

SEQ ID NO: 42181 - DNA, 28 bp, synthetic construct
  source 1..28: mol_type = other DNA
ttaggatattttgttggtgtggacatgg

SEQ ID NO: 42182 - DNA, 28 bp, synthetic construct
  source 1..28: mol_type = other DNA
tggtgtggacatggtaagaaaattttgg

SEQ ID NO: 42183 - DNA, 28 bp, synthetic construct
  source 1..28: mol_type = other DNA
taacatttaccaatgtaaaatattttgg

SEQ ID NO: 42184 - DNA, 28 bp, synthetic construct
  source 1..28: mol_type = other DNA
catttaccaatgtaaaatattttggagg

SEQ ID NO: 42185 - DNA, 28 bp, synthetic construct
  source 1..28: mol_type = other DNA
aagaatcctccaaaatattttacattgg

SEQ ID NO: 42186 - DNA, 28 bp, synthetic construct
  source 1..28: mol_type = other DNA
gtaaaatattttggaggattctttatgg

SEQ ID NO: 42187 - DNA, 28 bp, synthetic construct
  source 1..28: mol_type = other DNA
agacttccacatttacatttcattgagg

SEQ ID NO: 42188 - DNA, 28 bp, synthetic construct
  source 1..28: mol_type = other DNA
cttccacatttacatttcattgaggagg

SEQ ID NO: 42189 - DNA, 28 bp, synthetic construct
  source 1..28: mol_type = other DNA
aatcctcctcaatgaaatgtaaatgtgg

SEQ ID NO: 42190 - DNA, 28 bp, synthetic construct
  source 1..28: mol_type = other DNA
ttttaatgtttattatttaatttctagg

SEQ ID NO: 42191 - DNA, 28 bp, synthetic construct
  source 1..28: mol_type = other DNA
tatttaatttctaggataaccctattgg

SEQ ID NO: 42192 - DNA, 28 bp, synthetic construct
  source 1..28: mol_type = other DNA
tttctaggataaccctattggcaactgg

SEQ ID NO: 42193 - DNA, 28 bp, synthetic construct
  source 1..28: mol_type = other DNA
ttctaggataaccctattggcaactggg

SEQ ID NO: 42194 - DNA, 28 bp, synthetic construct
  source 1..28: mol_type = other DNA
aggataaccctattggcaactgggatgg

SEQ ID NO: 42195 - DNA, 28 bp, synthetic construct
  source 1..28: mol_type = other DNA
aaatcttccatcccagttgccaataggg

SEQ ID NO: 42196 - DNA, 28 bp, synthetic construct
  source 1..28: mol_type = other DNA
caaatcttccatcccagttgccaatagg

SEQ ID NO: 42197 - DNA, 28 bp, synthetic construct
  source 1..28: mol_type = other DNA
ttggcaactgggatggaagatttgatgg

SEQ ID NO: 42198 - DNA, 28 bp, synthetic construct
  source 1..28: mol_type = other DNA
tattgcacatcaatgatatcatcccagg

SEQ ID NO: 42199 - DNA, 28 bp, synthetic construct
  source 1..28: mol_type = other DNA
tgtataaaacaaagaaaacatacctggg

SEQ ID NO: 42200 - DNA, 28 bp, synthetic construct
  source 1..28: mol_type = other DNA
atgtataaaacaaagaaaacatacctgg

SEQ ID NO: 42201 - DNA, 28 bp, synthetic construct
  source 1..28: mol_type = other DNA
gttttctttgttttatacatttataagg

SEQ ID NO: 42202 - DNA, 28 bp, synthetic construct
  source 1..28: mol_type = other DNA
tttatttttttatatcaatatgttttgg

SEQ ID NO: 42203 - DNA, 28 bp, synthetic construct
  source 1..28: mol_type = other DNA
ttatttttttatatcaatatgttttggg

SEQ ID NO: 42204 - DNA, 28 bp, synthetic construct
  source 1..28: mol_type = other DNA
tatttttttatatcaatatgttttgggg

SEQ ID NO: 42205 - DNA, 28 bp, synthetic construct
  source 1..28: mol_type = other DNA
atttttttatatcaatatgttttggggg

SEQ ID NO: 42206 - DNA, 28 bp, synthetic construct
  source 1..28: mol_type = other DNA
ttatatcaatatgttttgggggaacagg

SEQ ID NO: 42207 - DNA, 28 bp, synthetic construct
  source 1..28: mol_type = other DNA
tatcaatatgttttgggggaacaggtgg

SEQ ID NO: 42208 - DNA, 28 bp, synthetic construct
  source 1..28: mol_type = other DNA
atgttttgggggaacaggtggtgtttgg

SEQ ID NO: 42209 - DNA, 28 bp, synthetic construct
  source 1..28: mol_type = other DNA
ggggaacaggtggtgtttggttacatgg

SEQ ID NO: 42210 - DNA, 28 bp, synthetic construct
  source 1..28: mol_type = other DNA
ttggttacatggataagttctttcgtgg

SEQ ID NO: 42211 - DNA, 28 bp, synthetic construct
  source 1..28: mol_type = other DNA
aggaaaagacttttcttaaaaaaagagg

SEQ ID NO: 42212 - DNA, 28 bp, synthetic construct
  source 1..28: mol_type = other DNA
ggaaaatttttacattttaaacacaagg

SEQ ID NO: 42213 - DNA, 28 bp, synthetic construct
  source 1..28: mol_type = other DNA
gatttgaggacagaaagaaagaaatagg

SEQ ID NO: 42214 - DNA, 28 bp, synthetic construct
  source 1..28: mol_type = other DNA
tttctttctgtcctcaaatccactgtgg

SEQ ID NO: 42215 - DNA, 28 bp, synthetic construct
  source 1..28: mol_type = other DNA
ttctttctgtcctcaaatccactgtggg

SEQ ID NO: 42216 - DNA, 28 bp, synthetic construct
  source 1..28: mol_type = other DNA
aacgatatcacccacagtggatttgagg

SEQ ID NO: 42217 - DNA, 28 bp, synthetic construct
  source 1..28: mol_type = other DNA
tcagcaaaaacgatatcacccacagtgg

SEQ ID NO: 42218 - DNA, 28 bp, synthetic construct
  source 1..28: mol_type = other DNA
gtttttgctgacacacagctttatcagg

SEQ ID NO: 42219 - DNA, 28 bp, synthetic construct
  source 1..28: mol_type = other DNA
caggtatgactcctaagtgtcgtgttgg

SEQ ID NO: 42220 - DNA, 28 bp, synthetic construct
  source 1..28: mol_type = other DNA
ctcctaagtgtcgtgttggactccacgg

SEQ ID NO: 42221 - DNA, 28 bp, synthetic construct
  source 1..28: mol_type = other DNA
atccgtggagtccaacacgacacttagg

SEQ ID NO: 42222 - DNA, 28 bp, synthetic construct
  source 1..28: mol_type = other DNA
tttgaaaaattcaacaatacatccgtgg

SEQ ID NO: 42223 - DNA, 28 bp, synthetic construct
  source 1..28: mol_type = other DNA
acggatgtattgttgaatttttcaaagg

SEQ ID NO: 42224 - DNA, 28 bp, synthetic construct
  source 1..28: mol_type = other DNA
aatactgatcaagggaatgtagaagagg

SEQ ID NO: 42225 - DNA, 28 bp, synthetic construct
  source 1..28: mol_type = other DNA
ttctacattcccttgatcagtatttagg

SEQ ID NO: 42226 - DNA, 28 bp, synthetic construct
  source 1..28: mol_type = other DNA
tagaatactcctaaatactgatcaaggg

SEQ ID NO: 42227 - DNA, 28 bp, synthetic construct
  source 1..28: mol_type = other DNA
atagaatactcctaaatactgatcaagg

SEQ ID NO: 42228 - DNA, 28 bp, synthetic construct
  source 1..28: mol_type = other DNA
taaaactaaaaattctgcctttttgtgg

SEQ ID NO: 42229 - DNA, 28 bp, synthetic construct
  source 1..28: mol_type = other DNA
aaaaattctgcctttttgtggaaagagg

SEQ ID NO: 42230 - DNA, 28 bp, synthetic construct
  source 1..28: mol_type = other DNA
aaaattctgcctttttgtggaaagaggg

SEQ ID NO: 42231 - DNA, 28 bp, synthetic construct
  source 1..28: mol_type = other DNA
ataaaaaaaccctctttccacaaaaagg

SEQ ID NO: 42232 - DNA, 28 bp, synthetic construct
  source 1..28: mol_type = other DNA
ggcaaattcttatagaagagaaacaagg

SEQ ID NO: 42233 - DNA, 28 bp, synthetic construct
  source 1..28: mol_type = other DNA
cagtaagcatgttttttaaagataaagg

SEQ ID NO: 42234 - DNA, 28 bp, synthetic construct
  source 1..28: mol_type = other DNA
cttactgtttcagagagtgtgacgcagg

SEQ ID NO: 42235 - DNA, 28 bp, synthetic construct
  source 1..28: mol_type = other DNA
tgtttcagagagtgtgacgcaggaaagg

SEQ ID NO: 42236 - DNA, 28 bp, synthetic construct
  source 1..28: mol_type = other DNA
ttcagagagtgtgacgcaggaaaggagg

SEQ ID NO: 42237 - DNA, 28 bp, synthetic construct
  source 1..28: mol_type = other DNA
ctcttgacataaaggcaagtttgggagg

SEQ ID NO: 42238 - DNA, 28 bp, synthetic construct
  source 1..28: mol_type = other DNA
ctcccaaacttgcctttatgtcaagagg

SEQ ID NO: 42239 - DNA, 28 bp, synthetic construct
  source 1..28: mol_type = other DNA
cacctcttgacataaaggcaagtttggg

SEQ ID NO: 42240 - DNA, 28 bp, synthetic construct
  source 1..28: mol_type = other DNA
acacctcttgacataaaggcaagtttgg

SEQ ID NO: 42241 - DNA, 28 bp, synthetic construct
  source 1..28: mol_type = other DNA
aacttgcctttatgtcaagaggtgttgg

SEQ ID NO: 42242 - DNA, 28 bp, synthetic construct
  source 1..28: mol_type = other DNA
acttgcctttatgtcaagaggtgttggg

SEQ ID NO: 42243 - DNA, 28 bp, synthetic construct
  source 1..28: mol_type = other DNA
cttgcctttatgtcaagaggtgttgggg

SEQ ID NO: 42244 - DNA, 28 bp, synthetic construct
  source 1..28: mol_type = other DNA
ttgtccccaacacctcttgacataaagg

SEQ ID NO: 42245 - DNA, 28 bp, synthetic construct
  source 1..28: mol_type = other DNA
ttatgtcaagaggtgttggggacaaagg

SEQ ID NO: 42246 - DNA, 28 bp, synthetic construct
  source 1..28: mol_type = other DNA
ggttcatccagtcataataaaccaaagg

SEQ ID NO: 42247 - DNA, 28 bp, synthetic construct
  source 1..28: mol_type = other DNA
cctgtagcctttggtttattatgactgg

SEQ ID NO: 42248 - DNA, 28 bp, synthetic construct
  source 1..28: mol_type = other DNA
cataataaaccaaaggctacaggtatgg

SEQ ID NO: 42249 - DNA, 28 bp, synthetic construct
  source 1..28: mol_type = other DNA
gctattaatccatacctgtagcctttgg

SEQ ID NO: 42250 - DNA, 28 bp, synthetic construct
  source 1..28: mol_type = other DNA
agttaggcattatgcaaattactaaagg

SEQ ID NO: 42251 - DNA, 28 bp, synthetic construct
  source 1..28: mol_type = other DNA
atcttttttaatgctatggcaagttagg

SEQ ID NO: 42252 - DNA, 28 bp, synthetic construct
  source 1..28: mol_type = other DNA
tagcttataatcttttttaatgctatgg

SEQ ID NO: 42253 - DNA, 28 bp, synthetic construct
  source 1..28: mol_type = other DNA
taaatgaaacttttcttgttcctatagg

SEQ ID NO: 42254 - DNA, 28 bp, synthetic construct
  source 1..28: mol_type = other DNA
ttcctataggatctacctcagaccctgg

SEQ ID NO: 42255 - DNA, 28 bp, synthetic construct
  source 1..28: mol_type = other DNA
ttccagggtctgaggtagatcctatagg

SEQ ID NO: 42256 - DNA, 28 bp, synthetic construct
  source 1..28: mol_type = other DNA
gatctgtttctatttccagggtctgagg

SEQ ID NO: 42257 - DNA, 28 bp, synthetic construct
  source 1..28: mol_type = other DNA
taattcagatctgtttctatttccaggg

SEQ ID NO: 42258 - DNA, 28 bp, synthetic construct
  source 1..28: mol_type = other DNA
ataattcagatctgtttctatttccagg

SEQ ID NO: 42259 - DNA, 28 bp, synthetic construct
  source 1..28: mol_type = other DNA
gatctgaattattttataccttaaatgg

SEQ ID NO: 42260 - DNA, 28 bp, synthetic construct
  source 1..28: mol_type = other DNA
atctgaattattttataccttaaatggg

SEQ ID NO: 42261 - DNA, 28 bp, synthetic construct
  source 1..28: mol_type = other DNA
tgtgagtcaacagaagacccatttaagg

SEQ ID NO: 42262 - DNA, 28 bp, synthetic construct
  source 1..28: mol_type = other DNA
accacaatccaaatcaaaaaatacatgg

SEQ ID NO: 42263 - DNA, 28 bp, synthetic construct
  source 1..28: mol_type = other DNA
accatgtattttttgatttggattgtgg

SEQ ID NO: 42264 - DNA, 28 bp, synthetic construct
  source 1..28: mol_type = other DNA
tcaatgtaccatgtattttttgatttgg

SEQ ID NO: 42265 - DNA, 28 bp, synthetic construct
  source 1..28: mol_type = other DNA
caaaaaatacatggtacattgatgaagg

SEQ ID NO: 42266 - DNA, 28 bp, synthetic construct
  source 1..28: mol_type = other DNA
tttttctctgatgagttagaaagaaagg

SEQ ID NO: 42267 - DNA, 28 bp, synthetic construct
  source 1..28: mol_type = other DNA
ttctttctaactcatcagagaaaaatgg

SEQ ID NO: 42268 - DNA, 28 bp, synthetic construct
  source 1..28: mol_type = other DNA
tttttatatcaatatttgtagtttttgg

SEQ ID NO: 42269 - DNA, 28 bp, synthetic construct
  source 1..28: mol_type = other DNA
gagtactattaatagcagggaggtcagg

SEQ ID NO: 42270 - DNA, 28 bp, synthetic construct
  source 1..28: mol_type = other DNA
tactattaatagcagggaggtcaggtgg

SEQ ID NO: 42271 - DNA, 28 bp, synthetic construct
  source 1..28: mol_type = other DNA
actattaatagcagggaggtcaggtggg

SEQ ID NO: 42272 - DNA, 28 bp, synthetic construct
  source 1..28: mol_type = other DNA
atagcagggaggtcaggtgggcagttgg

SEQ ID NO: 42273 - DNA, 28 bp, synthetic construct
  source 1..28: mol_type = other DNA
tatccttgaatacatttctgtaattagg

SEQ ID NO: 42274 - DNA, 28 bp, synthetic construct
  source 1..28: mol_type = other DNA
attcctaattacagaaatgtattcaagg

SEQ ID NO: 42275 - DNA, 28 bp, synthetic construct
  source 1..28: mol_type = other DNA
agatatctctgtaagagattttgcaggg

SEQ ID NO: 42276 - DNA, 28 bp, synthetic construct
  source 1..28: mol_type = other DNA
tagatatctctgtaagagattttgcagg

SEQ ID NO: 42277 - DNA, 28 bp, synthetic construct
  source 1..28: mol_type = other DNA
aggaggctggagtggtggtgaagaacgg

SEQ ID NO: 42278 - DNA, 28 bp, synthetic construct
  source 1..28: mol_type = other DNA
agttcacaggaggaggctggagtggtgg

SEQ ID NO: 42279 - DNA, 28 bp, synthetic construct
  source 1..28: mol_type = other DNA
gtgagttcacaggaggaggctggagtgg

SEQ ID NO: 42280 - DNA, 28 bp, synthetic construct
  source 1..28: mol_type = other DNA
ggtcagtgagttcacaggaggaggctgg

SEQ ID NO: 42281 - DNA, 28 bp, synthetic construct
  source 1..28: mol_type = other DNA
cggtggtcagtgagttcacaggaggagg

SEQ ID NO: 42282 - DNA, 28 bp, synthetic construct
  source 1..28: mol_type = other DNA
tctcggtggtcagtgagttcacaggagg

SEQ ID NO: 42283 - DNA, 28 bp, synthetic construct
  source 1..28: mol_type = other DNA
tgttctcggtggtcagtgagttcacagg

SEQ ID NO: 42284 - DNA, 28 bp, synthetic construct
  source 1..28: mol_type = other DNA
ggtaaagagtggaatctgttctcggtgg

SEQ ID NO: 42285 - DNA, 28 bp, synthetic construct
  source 1..28: mol_type = other DNA
aatggtaaagagtggaatctgttctcgg

SEQ ID NO: 42286 - DNA, 28 bp, synthetic construct
  source 1..28: mol_type = other DNA
cttggtgagactgaatggtaaagagtgg

SEQ ID NO: 42287 - DNA, 28 bp, synthetic construct
  source 1..28: mol_type = other DNA
tattgggcatcttggtgagactgaatgg

SEQ ID NO: 42288 - DNA, 28 bp, synthetic construct
  source 1..28: mol_type = other DNA
gtctcaccaagatgcccaataccaatgg

SEQ ID NO: 42289 - DNA, 28 bp, synthetic construct
  source 1..28: mol_type = other DNA
atacttccattggtattgggcatcttgg

SEQ ID NO: 42290 - DNA, 28 bp, synthetic construct
  source 1..28: mol_type = other DNA
agatgcccaataccaatggaagtattgg

SEQ ID NO: 42291 - DNA, 28 bp, synthetic construct
  source 1..28: mol_type = other DNA
tgtggccaatacttccattggtattggg

SEQ ID NO: 42292 - DNA, 28 bp, synthetic construct
  source 1..28: mol_type = other DNA
ctgtggccaatacttccattggtattgg

SEQ ID NO: 42293 - DNA, 28 bp, synthetic construct
  source 1..28: mol_type = other DNA
agtggactgtggccaatacttccattgg

SEQ ID NO: 42294 - DNA, 28 bp, synthetic construct
  source 1..28: mol_type = other DNA
ctgggctgacagagaaagtggactgtgg

SEQ ID NO: 42295 - DNA, 28 bp, synthetic construct
  source 1..28: mol_type = other DNA
ttacagactgggctgacagagaaagtgg

SEQ ID NO: 42296 - DNA, 28 bp, synthetic construct
  source 1..28: mol_type = other DNA
ctttctctgtcagcccagtctgtaatgg

SEQ ID NO: 42297 - DNA, 28 bp, synthetic construct
  source 1..28: mol_type = other DNA
gtgtttagctcttccattacagactggg

SEQ ID NO: 42298 - DNA, 28 bp, synthetic construct
  source 1..28: mol_type = other DNA
agtgtttagctcttccattacagactgg

SEQ ID NO: 42299 - DNA, 28 bp, synthetic construct
  source 1..28: mol_type = other DNA
gcacccgtccaagagagtccacccttgg

SEQ ID NO: 42300 - DNA, 28 bp, synthetic construct
  source 1..28: mol_type = other DNA
tggccaagggtggactctcttggacggg

SEQ ID NO: 42301 - DNA, 28 bp, synthetic construct
  source 1..28: mol_type = other DNA
atggccaagggtggactctcttggacgg

SEQ ID NO: 42302 - DNA, 28 bp, synthetic construct
  source 1..28: mol_type = other DNA
aggcatggccaagggtggactctcttgg

SEQ ID NO: 42303 - DNA, 28 bp, synthetic construct
  source 1..28: mol_type = other DNA
agagtccacccttggccatgcctcctgg

SEQ ID NO: 42304 - DNA, 28 bp, synthetic construct
  source 1..28: mol_type = other DNA
gagtccacccttggccatgcctcctggg

SEQ ID NO: 42305 - DNA, 28 bp, synthetic construct
  source 1..28: mol_type = other DNA
agttcccaggaggcatggccaagggtgg

SEQ ID NO: 42306 - DNA, 28 bp, synthetic construct
  source 1..28: mol_type = other DNA
gtgagttcccaggaggcatggccaaggg

SEQ ID NO: 42307 - DNA, 28 bp, synthetic construct
  source 1..28: mol_type = other DNA
tgtgagttcccaggaggcatggccaagg

SEQ ID NO: 42308 - DNA, 28 bp, synthetic construct
  source 1..28: mol_type = other DNA
tggccatgcctcctgggaactcacatgg

SEQ ID NO: 42309 - DNA, 28 bp, synthetic construct
  source 1..28: mol_type = other DNA
agaccatgtgagttcccaggaggcatgg

SEQ ID NO: 42310 - DNA, 28 bp, synthetic construct
  source 1..28: mol_type = other DNA
cttctagaccatgtgagttcccaggagg

SEQ ID NO: 42311 - DNA, 28 bp, synthetic construct
  source 1..28: mol_type = other DNA
cctgggaactcacatggtctagaagtgg

SEQ ID NO: 42312 - DNA, 28 bp, synthetic construct
  source 1..28: mol_type = other DNA
ctgggaactcacatggtctagaagtggg

SEQ ID NO: 42313 - DNA, 28 bp, synthetic construct
  source 1..28: mol_type = other DNA
tcacatggtctagaagtgggctcattgg

SEQ ID NO: 42314 - DNA, 28 bp, synthetic construct
  source 1..28: mol_type = other DNA
gaagtgggctcattggctgaagttaagg

SEQ ID NO: 42315 - DNA, 28 bp, synthetic construct
  source 1..28: mol_type = other DNA
aagttaaggagaaccctcctttctatgg

SEQ ID NO: 42316 - DNA, 28 bp, synthetic construct
  source 1..28: mol_type = other DNA
agttaaggagaaccctcctttctatggg

SEQ ID NO: 42317 - DNA, 28 bp, synthetic construct
  source 1..28: mol_type = other DNA
gttaaggagaaccctcctttctatgggg

SEQ ID NO: 42318 - DNA, 28 bp, synthetic construct
  source 1..28: mol_type = other DNA
ccctcctttctatggggtaatccgttgg

SEQ ID NO: 42319 - DNA, 28 bp, synthetic construct
  source 1..28: mol_type = other DNA
tccaacggattaccccatagaaaggagg

SEQ ID NO: 42320 - DNA, 28 bp, synthetic construct
  source 1..28: mol_type = other DNA
cgatccaacggattaccccatagaaagg

SEQ ID NO: 42321 - DNA, 28 bp, synthetic construct
  source 1..28: mol_type = other DNA
ctttctatggggtaatccgttggatcgg

SEQ ID NO: 42322 - DNA, 28 bp, synthetic construct
  source 1..28: mol_type = other DNA
taatccgttggatcggtcagccaccagg

SEQ ID NO: 42323 - DNA, 28 bp, synthetic construct
  source 1..28: mol_type = other DNA
cagtcctggtggctgaccgatccaacgg

SEQ ID NO: 42324 - DNA, 28 bp, synthetic construct
  source 1..28: mol_type = other DNA
cagcgagcacttcattcagtcctggtgg

SEQ ID NO: 42325 - DNA, 28 bp, synthetic construct
  source 1..28: mol_type = other DNA
caccaggactgaatgaagtgctcgctgg

SEQ ID NO: 42326 - DNA, 28 bp, synthetic construct
  source 1..28: mol_type = other DNA
gtccagcgagcacttcattcagtcctgg

SEQ ID NO: 42327 - DNA, 28 bp, synthetic construct
  source 1..28: mol_type = other DNA
ggactgaatgaagtgctcgctggactgg

SEQ ID NO: 42328 - DNA, 28 bp, synthetic construct
  source 1..28: mol_type = other DNA
aatgaagtgctcgctggactggaactgg

SEQ ID NO: 42329 - DNA, 28 bp, synthetic construct
  source 1..28: mol_type = other DNA
cacagagaaaaaaattgaaatttttggg

SEQ ID NO: 42330 - DNA, 28 bp, synthetic construct
  source 1..28: mol_type = other DNA
tcacagagaaaaaaattgaaatttttgg

SEQ ID NO: 42331 - DNA, 28 bp, synthetic construct
  source 1..28: mol_type = other DNA
aaaaatttcaatttttttctctgtgagg

SEQ ID NO: 42332 - DNA, 28 bp, synthetic construct
  source 1..28: mol_type = other DNA
acagtttgtcaaaaagcatataataggg

SEQ ID NO: 42333 - DNA, 28 bp, synthetic construct
  source 1..28: mol_type = other DNA
aacagtttgtcaaaaagcatataatagg

SEQ ID NO: 42334 - DNA, 28 bp, synthetic construct
  source 1..28: mol_type = other DNA
aggtgcgaagagggagtggtgagaaagg

SEQ ID NO: 42335 - DNA, 28 bp, synthetic construct
  source 1..28: mol_type = other DNA
ggtgcgaagagggagtggtgagaaaggg

SEQ ID NO: 42336 - DNA, 28 bp, synthetic construct
  source 1..28: mol_type = other DNA
tggtgagaaagggtatactagaaacagg

SEQ ID NO: 42337 - DNA, 28 bp, synthetic construct
  source 1..28: mol_type = other DNA
tacagagatagtatacaaagaactaagg

SEQ ID NO: 42338 - DNA, 28 bp, synthetic construct
  source 1..28: mol_type = other DNA
tagttctttgtatactatctctgtaagg

SEQ ID NO: 42339 - DNA, 28 bp, synthetic construct
  source 1..28: mol_type = other DNA
ctttgtatactatctctgtaaggcacgg

SEQ ID NO: 42340 - DNA, 28 bp, synthetic construct
  source 1..28: mol_type = other DNA
atgcatattgaagcatttctttttcagg

SEQ ID NO: 42341 - DNA, 28 bp, synthetic construct
  source 1..28: mol_type = other DNA
ttctttttcaggaagatgagtgtgcagg

SEQ ID NO: 42342 - DNA, 28 bp, synthetic construct
  source 1..28: mol_type = other DNA
caggaagatgagtgtgcaggctgtacgg

SEQ ID NO: 42343 - DNA, 28 bp, synthetic construct
  source 1..28: mol_type = other DNA
aagatgagtgtgcaggctgtacggatgg

SEQ ID NO: 42344 - DNA, 28 bp, synthetic construct
  source 1..28: mol_type = other DNA
caggctgtacggatggaaccttcagagg

SEQ ID NO: 42345 - DNA, 28 bp, synthetic construct
  source 1..28: mol_type = other DNA
tacggatggaaccttcagaggcactcgg

SEQ ID NO: 42346 - DNA, 28 bp, synthetic construct
  source 1..28: mol_type = other DNA
caggtgaaataccgagtgcctctgaagg

SEQ ID NO: 42347 - DNA, 28 bp, synthetic construct
  source 1..28: mol_type = other DNA
cggtatttcacctgtgccctgaagaagg

SEQ ID NO: 42348 - DNA, 28 bp, synthetic construct
  source 1..28: mol_type = other DNA
acaaacagcgccttcttcagggcacagg

SEQ ID NO: 42349 - DNA, 28 bp, synthetic construct
  source 1..28: mol_type = other DNA
agtttcacaaacagcgccttcttcaggg

SEQ ID NO: 42350 - DNA, 28 bp, synthetic construct
  source 1..28: mol_type = other DNA
cagtttcacaaacagcgccttcttcagg

SEQ ID NO: 42351 - DNA, 28 bp, synthetic construct
  source 1..28: mol_type = other DNA
gctgtttgtgaaactgaagagctgcagg

SEQ ID NO: 42352 - DNA, 28 bp, synthetic construct
  source 1..28: mol_type = other DNA
actgaagagctgcaggcctgactctagg

SEQ ID NO: 42353 - DNA, 28 bp, synthetic construct
  source 1..28: mol_type = other DNA
gctgcaatgatgcaaacctagagtcagg

SEQ ID NO: 42354 - DNA, 28 bp, synthetic construct
  source 1..28: mol_type = other DNA
gactctaggtttgcatcattgcagccgg

SEQ ID NO: 42355 - DNA, 28 bp, synthetic construct
  source 1..28: mol_type = other DNA
tacagcgctcaatctgattggaaaccgg

SEQ ID NO: 42356 - DNA, 28 bp, synthetic construct
  source 1..28: mol_type = other DNA
aaagagttacagcgctcaatctgattgg

SEQ ID NO: 42357 - DNA, 28 bp, synthetic construct
  source 1..28: mol_type = other DNA
atcagattgagcgctgtaactctttagg

SEQ ID NO: 42358 - DNA, 28 bp, synthetic construct
  source 1..28: mol_type = other DNA
tgagcgctgtaactctttaggtatttgg

SEQ ID NO: 42359 - DNA, 28 bp, synthetic construct
  source 1..28: mol_type = other DNA
gatgctttttgtttacttaacaacctgg

SEQ ID NO: 42360 - DNA, 28 bp, synthetic construct
  source 1..28: mol_type = other DNA
atgagattagaattagagtcattccagg

SEQ ID NO: 42361 - DNA, 28 bp, synthetic construct
  source 1..28: mol_type = other DNA
ttctaatctcatatcatgttatattagg

SEQ ID NO: 42362 - DNA, 28 bp, synthetic construct
  source 1..28: mol_type = other DNA
tctcatatcatgttatattaggtgatgg

SEQ ID NO: 42363 - DNA, 28 bp, synthetic construct
  source 1..28: mol_type = other DNA
acattttaaaatgaaaaaatatttatgg

SEQ ID NO: 42364 - DNA, 28 bp, synthetic construct
  source 1..28: mol_type = other DNA
cattttaaaatgaaaaaatatttatggg

SEQ ID NO: 42365 - DNA, 28 bp, synthetic construct
  source 1..28: mol_type = other DNA
tttttaaaaaaatcttttcagcatttgg

SEQ ID NO: 42366 - DNA, 28 bp, synthetic construct
  source 1..28: mol_type = other DNA
ttaaaaaaatcttttcagcatttggagg

SEQ ID NO: 42367 - DNA, 28 bp, synthetic construct
  source 1..28: mol_type = other DNA
gtagaagaaaatactccaccaaaaatgg

SEQ ID NO: 42368 - DNA, 28 bp, synthetic construct
  source 1..28: mol_type = other DNA
atactccaccaaaaatggaaaaagaagg

SEQ ID NO: 42369 - DNA, 28 bp, synthetic construct
  source 1..28: mol_type = other DNA
ccaccaaaaatggaaaaagaaggcttgg

SEQ ID NO: 42370 - DNA, 28 bp, synthetic construct
  source 1..28: mol_type = other DNA
tctccaagccttctttttccatttttgg

SEQ ID NO: 42371 - DNA, 28 bp, synthetic construct
  source 1..28: mol_type = other DNA
aaaaagaaggcttggagataatgattgg

SEQ ID NO: 42372 - DNA, 28 bp, synthetic construct
  source 1..28: mol_type = other DNA
aaaagaaggcttggagataatgattggg

SEQ ID NO: 42373 - DNA, 28 bp, synthetic construct
  source 1..28: mol_type = other DNA
tggagataatgattgggaagaagaaagg

SEQ ID NO: 42374 - DNA, 28 bp, synthetic construct
  source 1..28: mol_type = other DNA
atgattgggaagaagaaaggcatccagg

SEQ ID NO: 42375 - DNA, 28 bp, synthetic construct
  source 1..28: mol_type = other DNA
tgattgggaagaagaaaggcatccaggg

SEQ ID NO: 42376 - DNA, 28 bp, synthetic construct
  source 1..28: mol_type = other DNA
taagtaacaagaattgtaatgaccctgg

SEQ ID NO: 42377 - DNA, 28 bp, synthetic construct
  source 1..28: mol_type = other DNA
ttgttacttagactcaaccttattctgg

SEQ ID NO: 42378 - DNA, 28 bp, synthetic construct
  source 1..28: mol_type = other DNA
cattctttttaaacttaccagaataagg

SEQ ID NO: 42379 - DNA, 28 bp, synthetic construct
  source 1..28: mol_type = other DNA
ctggtaagtttaaaaagaatgcaatagg

SEQ ID NO: 42380 - DNA, 28 bp, synthetic construct
  source 1..28: mol_type = other DNA
tgcaataggtatagatagtgccatgagg

SEQ ID NO: 42381 - DNA, 28 bp, synthetic construct
  source 1..28: mol_type = other DNA
ataggtatagatagtgccatgaggcagg

SEQ ID NO: 42382 - DNA, 28 bp, synthetic construct
  source 1..28: mol_type = other DNA
taggtatagatagtgccatgaggcaggg

SEQ ID NO: 42383 - DNA, 28 bp, synthetic construct
  source 1..28: mol_type = other DNA
agtgccatgaggcagggacacataccgg

SEQ ID NO: 42384 - DNA, 28 bp, synthetic construct
  source 1..28: mol_type = other DNA
cacaccggtatgtgtccctgcctcatgg

SEQ ID NO: 42385 - DNA, 28 bp, synthetic construct
  source 1..28: mol_type = other DNA
ctcacacgcacacacacacacacaccgg

SEQ ID NO: 42386 - DNA, 28 bp, synthetic construct
  source 1..28: mol_type = other DNA
ttagaagaggaaaataagtaaagtctgg

SEQ ID NO: 42387 - DNA, 28 bp, synthetic construct
  source 1..28: mol_type = other DNA
aacagatttttaacagaattagaagagg

SEQ ID NO: 42388 - DNA, 28 bp, synthetic construct
  source 1..28: mol_type = other DNA
aaagcaaataagctgcaaaagaaaaagg

SEQ ID NO: 42389 - DNA, 28 bp, synthetic construct
  source 1..28: mol_type = other DNA
agcttatttgcttttagttctgttctgg

SEQ ID NO: 42390 - DNA, 28 bp, synthetic construct
  source 1..28: mol_type = other DNA
aatattctacatcgttcttttctttggg

SEQ ID NO: 42391 - DNA, 28 bp, synthetic construct
  source 1..28: mol_type = other DNA
taatattctacatcgttcttttctttgg

SEQ ID NO: 42392 - DNA, 28 bp, synthetic construct
  source 1..28: mol_type = other DNA
ttatagtgaaacccaagagctactgagg

SEQ ID NO: 42393 - DNA, 28 bp, synthetic construct
  source 1..28: mol_type = other DNA
acaatttctgtcctcagtagctcttggg

SEQ ID NO: 42394 - DNA, 28 bp, synthetic construct
  source 1..28: mol_type = other DNA
aacaatttctgtcctcagtagctcttgg

SEQ ID NO: 42395 - DNA, 28 bp, synthetic construct
  source 1..28: mol_type = other DNA
atttgttttctacttacattctcagagg

SEQ ID NO: 42396 - DNA, 28 bp, synthetic construct
  source 1..28: mol_type = other DNA
aacaaattgctattttgcctttacatgg

SEQ ID NO: 42397 - DNA, 28 bp, synthetic construct
  source 1..28: mol_type = other DNA
aaacagcaaatagaacaccatgtaaagg

SEQ ID NO: 42398 - DNA, 28 bp, synthetic construct
  source 1..28: mol_type = other DNA
acatggtgttctatttgctgttttctgg

SEQ ID NO: 42399 - DNA, 28 bp, synthetic construct
  source 1..28: mol_type = other DNA
taccttgtcttcatgtaataagagatgg

SEQ ID NO: 42400 - DNA, 28 bp, synthetic construct
  source 1..28: mol_type = other DNA
accttgtcttcatgtaataagagatggg

SEQ ID NO: 42401 - DNA, 28 bp, synthetic construct
  source 1..28: mol_type = other DNA
acccatctcttattacatgaagacaagg

SEQ ID NO: 42402 - DNA, 28 bp, synthetic construct
  source 1..28: mol_type = other DNA
agagatgggtgaaaattagttcttatgg

SEQ ID NO: 42403 - DNA, 28 bp, synthetic construct
  source 1..28: mol_type = other DNA
ctatcactcaggctggagtgtgcagtgg

SEQ ID NO: 42404 - DNA, 28 bp, synthetic construct
  source 1..28: mol_type = other DNA
tagagtctcactctatcactcaggctgg

SEQ ID NO: 42405 - DNA, 28 bp, synthetic construct
  source 1..28: mol_type = other DNA
gagatagagtctcactctatcactcagg

SEQ ID NO: 42406 - DNA, 28 bp, synthetic construct
  source 1..28: mol_type = other DNA
ttagtaaaaaactattaattgatattgg

SEQ ID NO: 42407 - DNA, 28 bp, synthetic construct
  source 1..28: mol_type = other DNA
taatagttttttactaacttagatatgg

SEQ ID NO: 42408 - DNA, 28 bp, synthetic construct
  source 1..28: mol_type = other DNA
gtgtgccacaaaaattatgaaactgagg

SEQ ID NO: 42409 - DNA, 28 bp, synthetic construct
  source 1..28: mol_type = other DNA
attttcctcagtttcataatttttgtgg

SEQ ID NO: 42410 - DNA, 28 bp, synthetic construct
  source 1..28: mol_type = other DNA
atgaaactgaggaaaatacttgaaaagg

SEQ ID NO: 42411 - DNA, 28 bp, synthetic construct
  source 1..28: mol_type = other DNA
aaactgaggaaaatacttgaaaaggtgg

SEQ ID NO: 42412 - DNA, 28 bp, synthetic construct
  source 1..28: mol_type = other DNA
ctgaggaaaatacttgaaaaggtggagg

SEQ ID NO: 42413 - DNA, 28 bp, synthetic construct
  source 1..28: mol_type = other DNA
tacttgaaaaggtggaggctgcatcagg

SEQ ID NO: 42414 - DNA, 28 bp, synthetic construct
  source 1..28: mol_type = other DNA
catcaggatttacctctgaagaaaaagg

SEQ ID NO: 42415 - DNA, 28 bp, synthetic construct
  source 1..28: mol_type = other DNA
ttaagatggtcacctttttcttcagagg

SEQ ID NO: 42416 - DNA, 28 bp, synthetic construct
  source 1..28: mol_type = other DNA
tatttttaacgcatataagttaagatgg

SEQ ID NO: 42417 - DNA, 28 bp, synthetic construct
  source 1..28: mol_type = other DNA
tagctgaaatgtgtgtctgtgtagttgg

SEQ ID NO: 42418 - DNA, 28 bp, synthetic construct
  source 1..28: mol_type = other DNA
agctgaaatgtgtgtctgtgtagttggg

SEQ ID NO: 42419 - DNA, 28 bp, synthetic construct
  source 1..28: mol_type = other DNA
gctgaaatgtgtgtctgtgtagttgggg

SEQ ID NO: 42420 - DNA, 28 bp, synthetic construct
  source 1..28: mol_type = other DNA
ctgaaatgtgtgtctgtgtagttggggg

SEQ ID NO: 42421 - DNA, 28 bp, synthetic construct
  source 1..28: mol_type = other DNA
tgaaatgtgtgtctgtgtagttgggggg

SEQ ID NO: 42422 - DNA, 28 bp, synthetic construct
  source 1..28: mol_type = other DNA
aaaatttaaaaatcaaataagtcacagg

SEQ ID NO: 42423 - DNA, 28 bp, synthetic construct
  source 1..28: mol_type = other DNA
tttttaaattttctcctagatcctgagg

SEQ ID NO: 42424 - DNA, 28 bp, synthetic construct
  source 1..28: mol_type = other DNA
aatattcaagaattcctcaggatctagg

SEQ ID NO: 42425 - DNA, 28 bp, synthetic construct
  source 1..28: mol_type = other DNA
gaaacagaatattcaagaattcctcagg

SEQ ID NO: 42426 - DNA, 28 bp, synthetic construct
  source 1..28: mol_type = other DNA
gaatattctgtttcatcatattttaagg

SEQ ID NO: 42427 - DNA, 28 bp, synthetic construct
  source 1..28: mol_type = other DNA
aatattctgtttcatcatattttaaggg

SEQ ID NO: 42428 - DNA, 28 bp, synthetic construct
  source 1..28: mol_type = other DNA
aagggtagaacctttgctaaaaataagg

SEQ ID NO: 42429 - DNA, 28 bp, synthetic construct
  source 1..28: mol_type = other DNA
ttaaaggttaccttatttttagcaaagg

SEQ ID NO: 42430 - DNA, 28 bp, synthetic construct
  source 1..28: mol_type = other DNA
aacctttaaattgttctagaagcattgg

SEQ ID NO: 42431 - DNA, 28 bp, synthetic construct
  source 1..28: mol_type = other DNA
ttccaatgcttctagaacaatttaaagg

SEQ ID NO: 42432 - DNA, 28 bp, synthetic construct
  source 1..28: mol_type = other DNA
tctggaaatcatgtctgttgaataatgg

SEQ ID NO: 42433 - DNA, 28 bp, synthetic construct
  source 1..28: mol_type = other DNA
caaatacaatattaagaaatcattctgg

SEQ ID NO: 42434 - DNA, 28 bp, synthetic construct
  source 1..28: mol_type = other DNA
tgatttcttaatattgtatttgtttagg

SEQ ID NO: 42435 - DNA, 28 bp, synthetic construct
  source 1..28: mol_type = other DNA
gatttcttaatattgtatttgtttaggg

SEQ ID NO: 42436 - DNA, 28 bp, synthetic construct
  source 1..28: mol_type = other DNA
attgtatttgtttagggctcttaatagg

SEQ ID NO: 42437 - DNA, 28 bp, synthetic construct
  source 1..28: mol_type = other DNA
atccaaagctacaccatcaattttatgg

SEQ ID NO: 42438 - DNA, 28 bp, synthetic construct
  source 1..28: mol_type = other DNA
aaccataaaattgatggtgtagctttgg

SEQ ID NO: 42439 - DNA, 28 bp, synthetic construct
  source 1..28: mol_type = other DNA
gagaacagaaaaaccataaaattgatgg

SEQ ID NO: 42440 - DNA, 28 bp, synthetic construct
  source 1..28: mol_type = other DNA
tggtttttctgttctcaaatactgctgg

SEQ ID NO: 42441 - DNA, 28 bp, synthetic construct
  source 1..28: mol_type = other DNA
ggtttttctgttctcaaatactgctggg

SEQ ID NO: 42442 - DNA, 28 bp, synthetic construct
  source 1..28: mol_type = other DNA
attttgatttaagcatttgataaatagg

SEQ ID NO: 42443 - DNA, 28 bp, synthetic construct
  source 1..28: mol_type = other DNA
tttctctgcgtgtttttagatcagcagg

SEQ ID NO: 42444 - DNA, 28 bp, synthetic construct
  source 1..28: mol_type = other DNA
cgtgtttttagatcagcaggtcaaaagg

SEQ ID NO: 42445 - DNA, 28 bp, synthetic construct
  source 1..28: mol_type = other DNA
gattgttacttctatcaaatttttatgg

SEQ ID NO: 42446 - DNA, 28 bp, synthetic construct
  source 1..28: mol_type = other DNA
tttttatggaaaaaaatgagaaagttgg

SEQ ID NO: 42447 - DNA, 28 bp, synthetic construct
  source 1..28: mol_type = other DNA
tcccacaattcagcagttgttagaatgg

SEQ ID NO: 42448 - DNA, 28 bp, synthetic construct
  source 1..28: mol_type = other DNA
accattctaacaactgctgaattgtggg

SEQ ID NO: 42449 - DNA, 28 bp, synthetic construct
  source 1..28: mol_type = other DNA
gaccattctaacaactgctgaattgtgg

SEQ ID NO: 42450 - DNA, 28 bp, synthetic construct
  source 1..28: mol_type = other DNA
atcaacagtaacctgaaatttgcagagg

SEQ ID NO: 42451 - DNA, 28 bp, synthetic construct
  source 1..28: mol_type = other DNA
agtatcactaacctctgcaaatttcagg

SEQ ID NO: 42452 - DNA, 28 bp, synthetic construct
  source 1..28: mol_type = other DNA
tgcagaggttagtgatactcacctgtgg

SEQ ID NO: 42453 - DNA, 28 bp, synthetic construct
  source 1..28: mol_type = other DNA
cacagactttcacataaaataccacagg

SEQ ID NO: 42454 - DNA, 28 bp, synthetic construct
  source 1..28: mol_type = other DNA
ctgtggtattttatgtgaaagtctgtgg

SEQ ID NO: 42455 - DNA, 28 bp, synthetic construct
  source 1..28: mol_type = other DNA
tgtggtattttatgtgaaagtctgtggg

SEQ ID NO: 42456 - DNA, 28 bp, synthetic construct
  source 1..28: mol_type = other DNA
aagtctgtgggagtcttaagactattgg

SEQ ID NO: 42457 - DNA, 28 bp, synthetic construct
  source 1..28: mol_type = other DNA
cctgtttcataggacaccaatattaagg

SEQ ID NO: 42458 - DNA, 28 bp, synthetic construct
  source 1..28: mol_type = other DNA
aaacaaaacagttctgccttaatattgg

SEQ ID NO: 42459 - DNA, 28 bp, synthetic construct
  source 1..28: mol_type = other DNA
ttttgtttgacagccatgactattttgg

SEQ ID NO: 42460 - DNA, 28 bp, synthetic construct
  source 1..28: mol_type = other DNA
acagccatgactattttggtttcatagg

SEQ ID NO: 42461 - DNA, 28 bp, synthetic construct
  source 1..28: mol_type = other DNA
cagccatgactattttggtttcataggg

SEQ ID NO: 42462 - DNA, 28 bp, synthetic construct
  source 1..28: mol_type = other DNA
tttccctatgaaaccaaaatagtcatgg

SEQ ID NO: 42463 - DNA, 28 bp, synthetic construct
  source 1..28: mol_type = other DNA
ttctaaaaatatctgtcttttttatagg

SEQ ID NO: 42464 - DNA, 28 bp, synthetic construct
  source 1..28: mol_type = other DNA
gaggcatctgaataatcagacatgatgg

SEQ ID NO: 42465 - DNA, 28 bp, synthetic construct
  source 1..28: mol_type = other DNA
gtctgattattcagatgcctcgatttgg

SEQ ID NO: 42466 - DNA, 28 bp, synthetic construct
  source 1..28: mol_type = other DNA
atagtttaaagtcttttccaaatcgagg

SEQ ID NO: 42467 - DNA, 28 bp, synthetic construct
  source 1..28: mol_type = other DNA
ctatttaaaaaaatttttccttctctgg

SEQ ID NO: 42468 - DNA, 28 bp, synthetic construct
  source 1..28: mol_type = other DNA
aatctgttatatttaattccagagaagg

SEQ ID NO: 42469 - DNA, 28 bp, synthetic construct
  source 1..28: mol_type = other DNA
atgagatttttttagtttgttttgttgg

SEQ ID NO: 42470 - DNA, 28 bp, synthetic construct
  source 1..28: mol_type = other DNA
tttttagtttgttttgttggttttgtgg

SEQ ID NO: 42471 - DNA, 28 bp, synthetic construct
  source 1..28: mol_type = other DNA
attgtcagataattctcatcagttgtgg

SEQ ID NO: 42472 - DNA, 28 bp, synthetic construct
  source 1..28: mol_type = other DNA
ttgtcagataattctcatcagttgtggg

SEQ ID NO: 42473 - DNA, 28 bp, synthetic construct
  source 1..28: mol_type = other DNA
catcagttgtgggttagactctaactgg

SEQ ID NO: 42474 - DNA, 28 bp, synthetic construct
  source 1..28: mol_type = other DNA
ctctaactggacacagtatttcccaagg

SEQ ID NO: 42475 - DNA, 28 bp, synthetic construct
  source 1..28: mol_type = other DNA
ggctcttcagatactgaattgccttggg

SEQ ID NO: 42476 - DNA, 28 bp, synthetic construct
  source 1..28: mol_type = other DNA
taggctttaaaaaggacaatgttcatgg

SEQ ID NO: 42477 - DNA, 28 bp, synthetic construct
  source 1..28: mol_type = other DNA
tgtaaagaaaagttaggctttaaaaagg

SEQ ID NO: 42478 - DNA, 28 bp, synthetic construct
  source 1..28: mol_type = other DNA
catgaagaagatgtaaagaaaagttagg

SEQ ID NO: 42479 - DNA, 28 bp, synthetic construct
  source 1..28: mol_type = other DNA
tgtgagaaggggaagggaagttaagagg

SEQ ID NO: 42480 - DNA, 28 bp, synthetic construct
  source 1..28: mol_type = other DNA
gggagctgaaatgtgagaaggggaaggg

SEQ ID NO: 42481 - DNA, 28 bp, synthetic construct
  source 1..28: mol_type = other DNA
tgggagctgaaatgtgagaaggggaagg

SEQ ID NO: 42482 - DNA, 28 bp, synthetic construct
  source 1..28: mol_type = other DNA
tgtctgggagctgaaatgtgagaagggg

SEQ ID NO: 42483 - DNA, 28 bp, synthetic construct
  source 1..28: mol_type = other DNA
ctgtctgggagctgaaatgtgagaaggg

SEQ ID NO: 42484 - DNA, 28 bp, synthetic construct
  source 1..28: mol_type = other DNA
actgtctgggagctgaaatgtgagaagg

SEQ ID NO: 42485 - DNA, 28 bp, synthetic construct
  source 1..28: mol_type = other DNA
tcacatttcagctcccagacagtgccgg

SEQ ID NO: 42486 - DNA, 28 bp, synthetic construct
  source 1..28: mol_type = other DNA
cagctcccagacagtgccggatatgtgg

SEQ ID NO: 42487 - DNA, 28 bp, synthetic construct
  source 1..28: mol_type = other DNA
ctcccagacagtgccggatatgtggagg

SEQ ID NO: 42488 - DNA, 28 bp, synthetic construct
  source 1..28: mol_type = other DNA
tcccagacagtgccggatatgtggaggg

SEQ ID NO: 42489 - DNA, 28 bp, synthetic construct
  source 1..28: mol_type = other DNA
gccctccacatatccggcactgtctggg

SEQ ID NO: 42490 - DNA, 28 bp, synthetic construct
  source 1..28: mol_type = other DNA
agccctccacatatccggcactgtctgg

SEQ ID NO: 42491 - DNA, 28 bp, synthetic construct
  source 1..28: mol_type = other DNA
atacattgcaagccctccacatatccgg

SEQ ID NO: 42492 - DNA, 28 bp, synthetic construct
  source 1..28: mol_type = other DNA
gagtgtagagaatgctacgacgatccgg

SEQ ID NO: 42493 - DNA, 28 bp, synthetic construct
  source 1..28: mol_type = other DNA
gctacgacgatccggacatctcagctgg

SEQ ID NO: 42494 - DNA, 28 bp, synthetic construct
  source 1..28: mol_type = other DNA
gcttgatttttccagctgagatgtccgg

SEQ ID NO: 42495 - DNA, 28 bp, synthetic construct
  source 1..28: mol_type = other DNA
gaagggaagctcacttgagtgttgcagg

SEQ ID NO: 42496 - DNA, 28 bp, synthetic construct
  source 1..28: mol_type = other DNA
ctcaagtgagcttcccttcacttaatgg

SEQ ID NO: 42497 - DNA, 28 bp, synthetic construct
  source 1..28: mol_type = other DNA
aacaaaagtttatccattaagtgaaggg

SEQ ID NO: 42498 - DNA, 28 bp, synthetic construct
  source 1..28: mol_type = other DNA
caacaaaagtttatccattaagtgaagg

SEQ ID NO: 42499 - DNA, 28 bp, synthetic construct
  source 1..28: mol_type = other DNA
atagttgaaaacacaatgctcgttttgg

SEQ ID NO: 42500 - DNA, 28 bp, synthetic construct
  source 1..28: mol_type = other DNA
gaaagttttttaaaatcataattaacgg

SEQ ID NO: 42501 - DNA, 28 bp, synthetic construct
  source 1..28: mol_type = other DNA
tctgttaaaaatacaaaaattagctggg

SEQ ID NO: 42502 - DNA, 28 bp, synthetic construct
  source 1..28: mol_type = other DNA
ctctgttaaaaatacaaaaattagctgg

SEQ ID NO: 42503 - DNA, 28 bp, synthetic construct
  source 1..28: mol_type = other DNA
taatttttgtatttttaacagagacagg

SEQ ID NO: 42504 - DNA, 28 bp, synthetic construct
  source 1..28: mol_type = other DNA
aatttttgtatttttaacagagacaggg

SEQ ID NO: 42505 - DNA, 28 bp, synthetic construct
  source 1..28: mol_type = other DNA
gagacagggtttcaccatcttgatcagg

SEQ ID NO: 42506 - DNA, 28 bp, synthetic construct
  source 1..28: mol_type = other DNA
cagggtttcaccatcttgatcaggctgg

SEQ ID NO: 42507 - DNA, 28 bp, synthetic construct
  source 1..28: mol_type = other DNA
gagttcaagaccagcctgatcaagatgg

SEQ ID NO: 42508 - DNA, 28 bp, synthetic construct
  source 1..28: mol_type = other DNA
tcctgacctcgtgatccaccagcctcgg

SEQ ID NO: 42509 - DNA, 28 bp, synthetic construct
  source 1..28: mol_type = other DNA
gccgaggctggtggatcacgaggtcagg

SEQ ID NO: 42510 - DNA, 28 bp, synthetic construct
  source 1..28: mol_type = other DNA
attaggccgaggctggtggatcacgagg

SEQ ID NO: 42511 - DNA, 28 bp, synthetic construct
  source 1..28: mol_type = other DNA
aagaatgtcattaggccgaggctggtgg

SEQ ID NO: 42512 - DNA, 28 bp, synthetic construct
  source 1..28: mol_type = other DNA
gaaaagaatgtcattaggccgaggctgg

SEQ ID NO: 42513 - DNA, 28 bp, synthetic construct
  source 1..28: mol_type = other DNA
cctcggcctaatgacattcttttcatgg

SEQ ID NO: 42514 - DNA, 28 bp, synthetic construct
  source 1..28: mol_type = other DNA
aatggaccatgaaaagaatgtcattagg

SEQ ID NO: 42515 - DNA, 28 bp, synthetic construct
  source 1..28: mol_type = other DNA
tgacattcttttcatggtccattttagg

SEQ ID NO: 42516 - DNA, 28 bp, synthetic construct
  source 1..28: mol_type = other DNA
tcttcggatgaaggtggacctaaaatgg

SEQ ID NO: 42517 - DNA, 28 bp, synthetic construct
  source 1..28: mol_type = other DNA
attttaggtccaccttcatccgaagagg

SEQ ID NO: 42518 - DNA, 28 bp, synthetic construct
  source 1..28: mol_type = other DNA
atgattcagcctcttcggatgaaggtgg

SEQ ID NO: 42519 - DNA, 28 bp, synthetic construct
  source 1..28: mol_type = other DNA
tttatgattcagcctcttcggatgaagg

SEQ ID NO: 42520 - DNA, 28 bp, synthetic construct
  source 1..28: mol_type = other DNA
ggttatatttatgattcagcctcttcgg

SEQ ID NO: 42521 - DNA, 28 bp, synthetic construct
  source 1..28: mol_type = other DNA
gggtaagtctttgggaagtgacactggg

SEQ ID NO: 42522 - DNA, 28 bp, synthetic construct
  source 1..28: mol_type = other DNA
cgggtaagtctttgggaagtgacactgg

SEQ ID NO: 42523 - DNA, 28 bp, synthetic construct
  source 1..28: mol_type = other DNA
gtcacttcccaaagacttacccgactgg

SEQ ID NO: 42524 - DNA, 28 bp, synthetic construct
  source 1..28: mol_type = other DNA
tcacttcccaaagacttacccgactggg

SEQ ID NO: 42525 - DNA, 28 bp, synthetic construct
  source 1..28: mol_type = other DNA
tcccaaagacttacccgactgggactgg

SEQ ID NO: 42526 - DNA, 28 bp, synthetic construct
  source 1..28: mol_type = other DNA
tccagtcccagtcgggtaagtctttggg

SEQ ID NO: 42527 - DNA, 28 bp, synthetic construct
  source 1..28: mol_type = other DNA
ctccagtcccagtcgggtaagtctttgg

SEQ ID NO: 42528 - DNA, 28 bp, synthetic construct
  source 1..28: mol_type = other DNA
acttacccgactgggactggagacacgg

SEQ ID NO: 42529 - DNA, 28 bp, synthetic construct
  source 1..28: mol_type = other DNA
tgcagccgtgtctccagtcccagtcggg

SEQ ID NO: 42530 - DNA, 28 bp, synthetic construct
  source 1..28: mol_type = other DNA
atgcagccgtgtctccagtcccagtcgg

SEQ ID NO: 42531 - DNA, 28 bp, synthetic construct
  source 1..28: mol_type = other DNA
cacggctgcatcccttgccagaatatgg

SEQ ID NO: 42532 - DNA, 28 bp, synthetic construct
  source 1..28: mol_type = other DNA
agcaaataactccatattctggcaaggg

SEQ ID NO: 42533 - DNA, 28 bp, synthetic construct
  source 1..28: mol_type = other DNA
cagcaaataactccatattctggcaagg

SEQ ID NO: 42534 - DNA, 28 bp, synthetic construct
  source 1..28: mol_type = other DNA
gagaacagcaaataactccatattctgg

SEQ ID NO: 42535 - DNA, 28 bp, synthetic construct
  source 1..28: mol_type = other DNA
gccactatgttgcttttgtgaagtatgg

SEQ ID NO: 42536 - DNA, 28 bp, synthetic construct
  source 1..28: mol_type = other DNA
cccatacttcacaaaagcaacatagtgg

SEQ ID NO: 42537 - DNA, 28 bp, synthetic construct
  source 1..28: mol_type = other DNA
tatgttgcttttgtgaagtatgggaagg

SEQ ID NO: 42538 - DNA, 28 bp, synthetic construct
  source 1..28: mol_type = other DNA
gaagtatgggaaggacgattctgcctgg

SEQ ID NO: 42539 - DNA, 28 bp, synthetic construct
  source 1..28: mol_type = other DNA
tctgcctggctcttctttgacagcatgg

SEQ ID NO: 42540 - DNA, 28 bp, synthetic construct
  source 1..28: mol_type = other DNA
tcggccatgctgtcaaagaagagccagg

SEQ ID NO: 42541 - DNA, 28 bp, synthetic construct
  source 1..28: mol_type = other DNA
gctcttctttgacagcatggccgatcgg

SEQ ID NO: 42542 - DNA, 28 bp, synthetic construct
  source 1..28: mol_type = other DNA
ctcttctttgacagcatggccgatcggg

SEQ ID NO: 42543 - DNA, 28 bp, synthetic construct
  source 1..28: mol_type = other DNA
tctttgacagcatggccgatcgggatgg

SEQ ID NO: 42544 - DNA, 28 bp, synthetic construct
  source 1..28: mol_type = other DNA
aaggcgttttcagtaccatcccgatcgg

SEQ ID NO: 42545 - DNA, 28 bp, synthetic construct
  source 1..28: mol_type = other DNA
actgaaaacgcctttcttctgcatgtgg

SEQ ID NO: 42546 - DNA, 28 bp, synthetic construct
  source 1..28: mol_type = other DNA
aacgcctttcttctgcatgtggcacagg

SEQ ID NO: 42547 - DNA, 28 bp, synthetic construct
  source 1..28: mol_type = other DNA
acgcctttcttctgcatgtggcacaggg

SEQ ID NO: 42548 - DNA, 28 bp, synthetic construct
  source 1..28: mol_type = other DNA
gaaccctgtgccacatgcagaagaaagg

SEQ ID NO: 42549 - DNA, 28 bp, synthetic construct
  source 1..28: mol_type = other DNA
ttcttctgcatgtggcacagggttctgg

SEQ ID NO: 42550 - DNA, 28 bp, synthetic construct
  source 1..28: mol_type = other DNA
tgtggcacagggttctggtttgtagtgg

SEQ ID NO: 42551 - DNA, 28 bp, synthetic construct
  source 1..28: mol_type = other DNA
gtggcacagggttctggtttgtagtggg

SEQ ID NO: 42552 - DNA, 28 bp, synthetic construct
  source 1..28: mol_type = other DNA
tggtttgtagtgggacagtttgtagtgg

SEQ ID NO: 42553 - DNA, 28 bp, synthetic construct
  source 1..28: mol_type = other DNA
ggtttgtagtgggacagtttgtagtggg

SEQ ID NO: 42554 - DNA, 28 bp, synthetic construct
  source 1..28: mol_type = other DNA
tttctcagaaaatatcactcagaacagg

SEQ ID NO: 42555 - DNA, 28 bp, synthetic construct
  source 1..28: mol_type = other DNA
tgatattttctgagaaaatcctttcagg

SEQ ID NO: 42556 - DNA, 28 bp, synthetic construct
  source 1..28: mol_type = other DNA
tgagaaaatcctttcaggattattctgg

SEQ ID NO: 42557 - DNA, 28 bp, synthetic construct
  source 1..28: mol_type = other DNA
cttttagagcctgaaattagctttttgg

SEQ ID NO: 42558 - DNA, 28 bp, synthetic construct
  source 1..28: mol_type = other DNA
ctatcatttccaaaaagctaatttcagg

SEQ ID NO: 42559 - DNA, 28 bp, synthetic construct
  source 1..28: mol_type = other DNA
ctgaaattagctttttggaaatgatagg

SEQ ID NO: 42560 - DNA, 28 bp, synthetic construct
  source 1..28: mol_type = other DNA
ggaaatgataggattataaaatcactgg

SEQ ID NO: 42561 - DNA, 28 bp, synthetic construct
  source 1..28: mol_type = other DNA
ataggattataaaatcactggcaaaagg

SEQ ID NO: 42562 - DNA, 28 bp, synthetic construct
  source 1..28: mol_type = other DNA
taggattataaaatcactggcaaaaggg

SEQ ID NO: 42563 - DNA, 28 bp, synthetic construct
  source 1..28: mol_type = other DNA
tggcacagaggaagaactctttataggg

SEQ ID NO: 42564 - DNA, 28 bp, synthetic construct
  source 1..28: mol_type = other DNA
atggcacagaggaagaactctttatagg

SEQ ID NO: 42565 - DNA, 28 bp, synthetic construct
  source 1..28: mol_type = other DNA
ataaagagttcttcctctgtgccatagg

SEQ ID NO: 42566 - DNA, 28 bp, synthetic construct
  source 1..28: mol_type = other DNA
aagagttcttcctctgtgccataggtgg

SEQ ID NO: 42567 - DNA, 28 bp, synthetic construct
  source 1..28: mol_type = other DNA
tcctctgtgccataggtggtcagaatgg

SEQ ID NO: 42568 - DNA, 28 bp, synthetic construct
  source 1..28: mol_type = other DNA
gccattctgaccacctatggcacagagg

SEQ ID NO: 42569 - DNA, 28 bp, synthetic construct
  source 1..28: mol_type = other DNA
atgttgaagccattctgaccacctatgg

SEQ ID NO: 42570 - DNA, 28 bp, synthetic construct
  source 1..28: mol_type = other DNA
ctacttctgggcatggggtgacttgagg

SEQ ID NO: 42571 - DNA, 28 bp, synthetic construct
  source 1..28: mol_type = other DNA
ctcaagtcaccccatgcccagaagtagg

SEQ ID NO: 42572 - DNA, 28 bp, synthetic construct
  source 1..28: mol_type = other DNA
aagtactctcctacttctgggcatgggg

SEQ ID NO: 42573 - DNA, 28 bp, synthetic construct
  source 1..28: mol_type = other DNA
caagtactctcctacttctgggcatggg

SEQ ID NO: 42574 - DNA, 28 bp, synthetic construct
  source 1..28: mol_type = other DNA
tcaagtactctcctacttctgggcatgg

SEQ ID NO: 42575 - DNA, 28 bp, synthetic construct
  source 1..28: mol_type = other DNA
catcttcaagtactctcctacttctggg

SEQ ID NO: 42576 - DNA, 28 bp, synthetic construct
  source 1..28: mol_type = other DNA
acatcttcaagtactctcctacttctgg

SEQ ID NO: 42577 - DNA, 28 bp, synthetic construct
  source 1..28: mol_type = other DNA
gtaggagagtacttgaagatgtctctgg

SEQ ID NO: 42578 - DNA, 28 bp, synthetic construct
  source 1..28: mol_type = other DNA
atgtctctggaagacctgcattccttgg

SEQ ID NO: 42579 - DNA, 28 bp, synthetic construct
  source 1..28: mol_type = other DNA
ggaagacctgcattccttggactccagg

SEQ ID NO: 42580 - DNA, 28 bp, synthetic construct
  source 1..28: mol_type = other DNA
gattctcctggagtccaaggaatgcagg

SEQ ID NO: 42581 - DNA, 28 bp, synthetic construct
  source 1..28: mol_type = other DNA
attccttggactccaggagaatccaagg

SEQ ID NO: 42582 - DNA, 28 bp, synthetic construct
  source 1..28: mol_type = other DNA
cagccttggattctcctggagtccaagg

SEQ ID NO: 42583 - DNA, 28 bp, synthetic construct
  source 1..28: mol_type = other DNA
cttcgtgcacagccttggattctcctgg

SEQ ID NO: 42584 - DNA, 28 bp, synthetic construct
  source 1..28: mol_type = other DNA
acaaagcagtcttcgtgcacagccttgg

SEQ ID NO: 42585 - DNA, 28 bp, synthetic construct
  source 1..28: mol_type = other DNA
tttgtacaaactcattgttggactctgg

SEQ ID NO: 42586 - DNA, 28 bp, synthetic construct
  source 1..28: mol_type = other DNA
ccaacaatgagtttgtacaaataactgg

SEQ ID NO: 42587 - DNA, 28 bp, synthetic construct
  source 1..28: mol_type = other DNA
caacaatgagtttgtacaaataactggg

SEQ ID NO: 42588 - DNA, 28 bp, synthetic construct
  source 1..28: mol_type = other DNA
aacaatgagtttgtacaaataactgggg

SEQ ID NO: 42589 - DNA, 28 bp, synthetic construct
  source 1..28: mol_type = other DNA
agtttgtacaaataactggggtcatcgg

SEQ ID NO: 42590 - DNA, 28 bp, synthetic construct
  source 1..28: mol_type = other DNA
gtttgtacaaataactggggtcatcggg

SEQ ID NO: 42591 - DNA, 28 bp, synthetic construct
  source 1..28: mol_type = other DNA
tacaaataactggggtcatcgggaaagg

SEQ ID NO: 42592 - DNA, 28 bp, synthetic construct
  source 1..28: mol_type = other DNA
tcatcgggaaaggcaaagaaactgaagg

SEQ ID NO: 42593 - DNA, 28 bp, synthetic construct
  source 1..28: mol_type = other DNA
tcctaacgttgcatcttattcgagctgg

SEQ ID NO: 42594 - DNA, 28 bp, synthetic construct
  source 1..28: mol_type = other DNA
gccagctcgaataagatgcaacgttagg

SEQ ID NO: 42595 - DNA, 28 bp, synthetic construct
  source 1..28: mol_type = other DNA
tggcagttctgttcacgtccattgccgg

SEQ ID NO: 42596 - DNA, 28 bp, synthetic construct
  source 1..28: mol_type = other DNA
ttctgttcacgtccattgccggcaatgg

SEQ ID NO: 42597 - DNA, 28 bp, synthetic construct
  source 1..28: mol_type = other DNA
ccacaaagacatccattgccggcaatgg

SEQ ID NO: 42598 - DNA, 28 bp, synthetic construct
  source 1..28: mol_type = other DNA
tcatcaccacaaagacatccattgccgg

SEQ ID NO: 42599 - DNA, 28 bp, synthetic construct
  source 1..28: mol_type = other DNA
ctttgtggtgatgatccttcagaaaagg

SEQ ID NO: 42600 - DNA, 28 bp, synthetic construct
  source 1..28: mol_type = other DNA
tttaaacagaggcatccttttctgaagg

SEQ ID NO: 42601 - DNA, 28 bp, synthetic construct
  source 1..28: mol_type = other DNA
acaaaagcaatttgtttttaaacagagg

SEQ ID NO: 42602 - DNA, 28 bp, synthetic construct
  source 1..28: mol_type = other DNA
aaaatgcttcttattaaatacttcaggg

SEQ ID NO: 42603 - DNA, 28 bp, synthetic construct
  source 1..28: mol_type = other DNA
caaaatgcttcttattaaatacttcagg

SEQ ID NO: 42604 - DNA, 28 bp, synthetic construct
  source 1..28: mol_type = other DNA
tgcactctagaaagtatgtttgtgttgg

SEQ ID NO: 42605 - DNA, 28 bp, synthetic construct
  source 1..28: mol_type = other DNA
atcaatgcacttaacttaaagcttcagg

SEQ ID NO: 42606 - DNA, 28 bp, synthetic construct
  source 1..28: mol_type = other DNA
aagtgcattgatcatatgatatttttgg

SEQ ID NO: 42607 - DNA, 28 bp, synthetic construct
  source 1..28: mol_type = other DNA
ttttggaagcatacaattttaattgtgg

SEQ ID NO: 42608 - DNA, 28 bp, synthetic construct
  source 1..28: mol_type = other DNA
atttacattctcaatggactaaaagagg

SEQ ID NO: 42609 - DNA, 28 bp, synthetic construct
  source 1..28: mol_type = other DNA
aagacacatttatttacattctcaatgg

SEQ ID NO: 42610 - DNA, 28 bp, synthetic construct
  source 1..28: mol_type = other DNA
aatgtaaataaatgtgtcttctttatgg

SEQ ID NO: 42611 - DNA, 28 bp, synthetic construct
  source 1..28: mol_type = other DNA
ataaatgtgtcttctttatggaccaagg

SEQ ID NO: 42612 - DNA, 28 bp, synthetic construct
  source 1..28: mol_type = other DNA
caaaagaaaaatgatttcatatccttgg

SEQ ID NO: 42613 - DNA, 28 bp, synthetic construct
  source 1..28: mol_type = other DNA
gaaatcatttttcttttgtagctaacgg

SEQ ID NO: 42614 - DNA, 28 bp, synthetic construct
  source 1..28: mol_type = other DNA
tcttttgtagctaacggttgccttgagg

SEQ ID NO: 42615 - DNA, 28 bp, synthetic construct
  source 1..28: mol_type = other DNA
cggttgccttgaggaagaaataatttgg

SEQ ID NO: 42616 - DNA, 28 bp, synthetic construct
  source 1..28: mol_type = other DNA
ataaaaccaaattatttcttcctcaagg

SEQ ID NO: 42617 - DNA, 28 bp, synthetic construct
  source 1..28: mol_type = other DNA
tcaaactcagtacatctctaataactgg

SEQ ID NO: 42618 - DNA, 28 bp, synthetic construct
  source 1..28: mol_type = other DNA
catgcaagatcagcagtatatagaaagg

SEQ ID NO: 42619 - DNA, 28 bp, synthetic construct
  source 1..28: mol_type = other DNA
cagtttttctgtgtttctgcaatagtgg

SEQ ID NO: 42620 - DNA, 28 bp, synthetic construct
  source 1..28: mol_type = other DNA
cagaaaaatacttaaattcccttaatgg

SEQ ID NO: 42621 - DNA, 28 bp, synthetic construct
  source 1..28: mol_type = other DNA
aacaaatagaaaacaacaccattaaggg

SEQ ID NO: 42622 - DNA, 28 bp, synthetic construct
  source 1..28: mol_type = other DNA
gaacaaatagaaaacaacaccattaagg

SEQ ID NO: 42623 - DNA, 28 bp, synthetic construct
  source 1..28: mol_type = other DNA
taatggtgttgttttctatttgttctgg

SEQ ID NO: 42624 - DNA, 28 bp, synthetic construct
  source 1..28: mol_type = other DNA
aaatcacttcaaaaatggacatttgggg

SEQ ID NO: 42625 - DNA, 28 bp, synthetic construct
  source 1..28: mol_type = other DNA
aaaatcacttcaaaaatggacatttggg

SEQ ID NO: 42626 - DNA, 28 bp, synthetic construct
  source 1..28: mol_type = other DNA
gaaaatcacttcaaaaatggacatttgg

SEQ ID NO: 42627 - DNA, 28 bp, synthetic construct
  source 1..28: mol_type = other DNA
atgtccatttttgaagtgattttcctgg

SEQ ID NO: 42628 - DNA, 28 bp, synthetic construct
  source 1..28: mol_type = other DNA
tccatttttgaagtgattttcctggagg

SEQ ID NO: 42629 - DNA, 28 bp, synthetic construct
  source 1..28: mol_type = other DNA
tcctccaggaaaatcacttcaaaaatgg

SEQ ID NO: 42630 - DNA, 28 bp, synthetic construct
  source 1..28: mol_type = other DNA
tttgaagtgattttcctggaggattagg

SEQ ID NO: 42631 - DNA, 28 bp, synthetic construct
  source 1..28: mol_type = other DNA
ttgaagtgattttcctggaggattaggg

SEQ ID NO: 42632 - DNA, 28 bp, synthetic construct
  source 1..28: mol_type = other DNA
caactgctaaataccctaatcctccagg

SEQ ID NO: 42633 - DNA, 28 bp, synthetic construct
  source 1..28: mol_type = other DNA
ttcatagtagttactgtcagctaacagg

SEQ ID NO: 42634 - DNA, 28 bp, synthetic construct
  source 1..28: mol_type = other DNA
ttactgtcagctaacaggttttttaagg

SEQ ID NO: 42635 - DNA, 28 bp, synthetic construct
  source 1..28: mol_type = other DNA
aaggcttttaactattaatattttatgg

SEQ ID NO: 42636 - DNA, 28 bp, synthetic construct
  source 1..28: mol_type = other DNA
ttttaactattaatattttatggaatgg

SEQ ID NO: 42637 - DNA, 28 bp, synthetic construct
  source 1..28: mol_type = other DNA
tttaactattaatattttatggaatggg

SEQ ID NO: 42638 - DNA, 28 bp, synthetic construct
  source 1..28: mol_type = other DNA
ttaactattaatattttatggaatgggg

SEQ ID NO: 42639 - DNA, 28 bp, synthetic construct
  source 1..28: mol_type = other DNA
gggcaaagtaaattgatgaaagaattgg

SEQ ID NO: 42640 - DNA, 28 bp, synthetic construct
  source 1..28: mol_type = other DNA
tttcttatggactgtatgtttgtaaagg

SEQ ID NO: 42641 - DNA, 28 bp, synthetic construct
  source 1..28: mol_type = other DNA
catacagtccataagaaaatgaatttgg

SEQ ID NO: 42642 - DNA, 28 bp, synthetic construct
  source 1..28: mol_type = other DNA
tctatatgccaaattcattttcttatgg

SEQ ID NO: 42643 - DNA, 28 bp, synthetic construct
  source 1..28: mol_type = other DNA
ggcatatagaattattacaatttcctgg

SEQ ID NO: 42644 - DNA, 28 bp, synthetic construct
  source 1..28: mol_type = other DNA
gcatatagaattattacaatttcctggg

SEQ ID NO: 42645 - DNA, 28 bp, synthetic construct
  source 1..28: mol_type = other DNA
aattattacaatttcctgggagagatgg

SEQ ID NO: 42646 - DNA, 28 bp, synthetic construct
  source 1..28: mol_type = other DNA
agaggtttaaatatccatctctcccagg

SEQ ID NO: 42647 - DNA, 28 bp, synthetic construct
  source 1..28: mol_type = other DNA
tagacagtcttgtctaaaataatagagg

SEQ ID NO: 42648 - DNA, 28 bp, synthetic construct
  source 1..28: mol_type = other DNA
actacactgaatttaatgggagtactgg

SEQ ID NO: 42649 - DNA, 28 bp, synthetic construct
  source 1..28: mol_type = other DNA
caagtgaaactacactgaatttaatggg

SEQ ID NO: 42650 - DNA, 28 bp, synthetic construct
  source 1..28: mol_type = other DNA
tcaagtgaaactacactgaatttaatgg

SEQ ID NO: 42651 - DNA, 28 bp, synthetic construct
  source 1..28: mol_type = other DNA
atttctacttactttaatcagaaggagg

SEQ ID NO: 42652 - DNA, 28 bp, synthetic construct
  source 1..28: mol_type = other DNA
tccttctgattaaagtaagtagaaatgg

SEQ ID NO: 42653 - DNA, 28 bp, synthetic construct
  source 1..28: mol_type = other DNA
cccatttctacttactttaatcagaagg

SEQ ID NO: 42654 - DNA, 28 bp, synthetic construct
  source 1..28: mol_type = other DNA
gccatagtgtgtgtttagaccacagcgg

SEQ ID NO: 42655 - DNA, 28 bp, synthetic construct
  source 1..28: mol_type = other DNA
tccgctgtggtctaaacacacactatgg

SEQ ID NO: 42656 - DNA, 28 bp, synthetic construct
  source 1..28: mol_type = other DNA
tagaccacagcggatgttgtagaccagg

SEQ ID NO: 42657 - DNA, 28 bp, synthetic construct
  source 1..28: mol_type = other DNA
tggtcctggtctacaacatccgctgtgg

SEQ ID NO: 42658 - DNA, 28 bp, synthetic construct
  source 1..28: mol_type = other DNA
cactgacatgtatcatctatggtcctgg

SEQ ID NO: 42659 - DNA, 28 bp, synthetic construct
  source 1..28: mol_type = other DNA
ccacagcactgacatgtatcatctatgg

SEQ ID NO: 42660 - DNA, 28 bp, synthetic construct
  source 1..28: mol_type = other DNA
tgtgcattctctgagtgttgttttgtgg

SEQ ID NO: 42661 - DNA, 28 bp, synthetic construct
  source 1..28: mol_type = other DNA
tttctgcacagttagaaagtcattcagg

SEQ ID NO: 42662 - DNA, 28 bp, synthetic construct
  source 1..28: mol_type = other DNA
tgaatgactttctaactgtgcagaaagg

SEQ ID NO: 42663 - DNA, 28 bp, synthetic construct
  source 1..28: mol_type = other DNA
ataaaatatttaatgtgacaaaaagtgg

SEQ ID NO: 42664 - DNA, 28 bp, synthetic construct
  source 1..28: mol_type = other DNA
acaaaccctgcaattacttttttaaagg

SEQ ID NO: 42665 - DNA, 28 bp, synthetic construct
  source 1..28: mol_type = other DNA
aagtgcctttaaaaaagtaattgcaggg

SEQ ID NO: 42666 - DNA, 28 bp, synthetic construct
  source 1..28: mol_type = other DNA
aaagtgcctttaaaaaagtaattgcagg

SEQ ID NO: 42667 - DNA, 28 bp, synthetic construct
  source 1..28: mol_type = other DNA
cttttttaaaggcacttttactctttgg

SEQ ID NO: 42668 - DNA, 28 bp, synthetic construct
  source 1..28: mol_type = other DNA
ataaagctagtaaatattagcaaaatgg

SEQ ID NO: 42669 - DNA, 28 bp, synthetic construct
  source 1..28: mol_type = other DNA
tttactagctttataaattacagtaagg

SEQ ID NO: 42670 - DNA, 28 bp, synthetic construct
  source 1..28: mol_type = other DNA
tgaaaaagtacatatattttgcacaagg

SEQ ID NO: 42671 - DNA, 28 bp, synthetic construct
  source 1..28: mol_type = other DNA
acaaggttttatactgctaagtgcttgg

SEQ ID NO: 42672 - DNA, 28 bp, synthetic construct
  source 1..28: mol_type = other DNA
ggttttatactgctaagtgcttggttgg

SEQ ID NO: 42673 - DNA, 28 bp, synthetic construct
  source 1..28: mol_type = other DNA
gttttatactgctaagtgcttggttggg

SEQ ID NO: 42674 - DNA, 28 bp, synthetic construct
  source 1..28: mol_type = other DNA
ttttatactgctaagtgcttggttgggg

SEQ ID NO: 42675 - DNA, 28 bp, synthetic construct
  source 1..28: mol_type = other DNA
tatactgctaagtgcttggttggggtgg

SEQ ID NO: 42676 - DNA, 28 bp, synthetic construct
  source 1..28: mol_type = other DNA
ggggtggtgagatgatgattagatcagg

SEQ ID NO: 42677 - DNA, 28 bp, synthetic construct
  source 1..28: mol_type = other DNA
gggtggtgagatgatgattagatcaggg

SEQ ID NO: 42678 - DNA, 28 bp, synthetic construct
  source 1..28: mol_type = other DNA
ggtggtgagatgatgattagatcagggg

SEQ ID NO: 42679 - DNA, 28 bp, synthetic construct
  source 1..28: mol_type = other DNA
tgagatgatgattagatcaggggtgagg

SEQ ID NO: 42680 - DNA, 28 bp, synthetic construct
  source 1..28: mol_type = other DNA
gatcaggggtgaggctgagagactctgg

SEQ ID NO: 42681 - DNA, 28 bp, synthetic construct
  source 1..28: mol_type = other DNA
atcaggggtgaggctgagagactctggg

SEQ ID NO: 42682 - DNA, 28 bp, synthetic construct
  source 1..28: mol_type = other DNA
ggtgaggctgagagactctgggtttagg

SEQ ID NO: 42683 - DNA, 28 bp, synthetic construct
  source 1..28: mol_type = other DNA
gtgaggctgagagactctgggtttaggg

SEQ ID NO: 42684 - DNA, 28 bp, synthetic construct
  source 1..28: mol_type = other DNA
gggctagccctgcctccatctcccttgg

SEQ ID NO: 42685 - DNA, 28 bp, synthetic construct
  source 1..28: mol_type = other DNA
ggctagccctgcctccatctcccttggg

SEQ ID NO: 42686 - DNA, 28 bp, synthetic construct
  source 1..28: mol_type = other DNA
attttacccaagggagatggaggcaggg

SEQ ID NO: 42687 - DNA, 28 bp, synthetic construct
  source 1..28: mol_type = other DNA
cattttacccaagggagatggaggcagg

SEQ ID NO: 42688 - DNA, 28 bp, synthetic construct
  source 1..28: mol_type = other DNA
cctccatctcccttgggtaaaatgaagg

SEQ ID NO: 42689 - DNA, 28 bp, synthetic construct
  source 1..28: mol_type = other DNA
ctccatctcccttgggtaaaatgaaggg

SEQ ID NO: 42690 - DNA, 28 bp, synthetic construct
  source 1..28: mol_type = other DNA
cacccttcattttacccaagggagatgg

SEQ ID NO: 42691 - DNA, 28 bp, synthetic construct
  source 1..28: mol_type = other DNA
tctcccttgggtaaaatgaagggtgtgg

SEQ ID NO: 42692 - DNA, 28 bp, synthetic construct
  source 1..28: mol_type = other DNA
ctcccttgggtaaaatgaagggtgtggg

SEQ ID NO: 42693 - DNA, 28 bp, synthetic construct
  source 1..28: mol_type = other DNA
tcccttgggtaaaatgaagggtgtgggg

SEQ ID NO: 42694 - DNA, 28 bp, synthetic construct
  source 1..28: mol_type = other DNA
accccacacccttcattttacccaaggg

SEQ ID NO: 42695 - DNA, 28 bp, synthetic construct
  source 1..28: mol_type = other DNA
taccccacacccttcattttacccaagg

SEQ ID NO: 42696 - DNA, 28 bp, synthetic construct
  source 1..28: mol_type = other DNA
aagggtgtggggtaaaagatgcataagg

SEQ ID NO: 42697 - DNA, 28 bp, synthetic construct
  source 1..28: mol_type = other DNA
acttctaggctgtcagagctagaaaagg

SEQ ID NO: 42698 - DNA, 28 bp, synthetic construct
  source 1..28: mol_type = other DNA
tttattacagggtgattggacttctagg

SEQ ID NO: 42699 - DNA, 28 bp, synthetic construct
  source 1..28: mol_type = other DNA
caacacatatttattacagggtgattgg

SEQ ID NO: 42700 - DNA, 28 bp, synthetic construct
  source 1..28: mol_type = other DNA
cttcattcaacacatatttattacaggg

SEQ ID NO: 42701 - DNA, 28 bp, synthetic construct
  source 1..28: mol_type = other DNA
tcttcattcaacacatatttattacagg

SEQ ID NO: 42702 - DNA, 28 bp, synthetic construct
  source 1..28: mol_type = other DNA
aataaatatgtgttgaatgaagaaatgg

SEQ ID NO: 42703 - DNA, 28 bp, synthetic construct
  source 1..28: mol_type = other DNA
ataaatatgtgttgaatgaagaaatggg

SEQ ID NO: 42704 - DNA, 28 bp, synthetic construct
  source 1..28: mol_type = other DNA
atgtgattttaaaaaattgactacctgg

SEQ ID NO: 42705 - DNA, 28 bp, synthetic construct
  source 1..28: mol_type = other DNA
tgattttaaaaaattgactacctggagg

SEQ ID NO: 42706 - DNA, 28 bp, synthetic construct
  source 1..28: mol_type = other DNA
aaattgactacctggaggaatgattagg

SEQ ID NO: 42707 - DNA, 28 bp, synthetic construct
  source 1..28: mol_type = other DNA
catttagattcctaatcattcctccagg

SEQ ID NO: 42708 - DNA, 28 bp, synthetic construct
  source 1..28: mol_type = other DNA
taggaatctaaatgaagccagccctcgg

SEQ ID NO: 42709 - DNA, 28 bp, synthetic construct
  source 1..28: mol_type = other DNA
aatgaagccagccctcggtatctgcagg

SEQ ID NO: 42710 - DNA, 28 bp, synthetic construct
  source 1..28: mol_type = other DNA
tgagaaacctgcagataccgagggctgg

SEQ ID NO: 42711 - DNA, 28 bp, synthetic construct
  source 1..28: mol_type = other DNA
tggatgagaaacctgcagataccgaggg

SEQ ID NO: 42712 - DNA, 28 bp, synthetic construct
  source 1..28: mol_type = other DNA
atggatgagaaacctgcagataccgagg

SEQ ID NO: 42713 - DNA, 28 bp, synthetic construct
  source 1..28: mol_type = other DNA
tcggtatctgcaggtttctcatccatgg

SEQ ID NO: 42714 - DNA, 28 bp, synthetic construct
  source 1..28: mol_type = other DNA
atccatggattcaaccaactgcaaatgg

SEQ ID NO: 42715 - DNA, 28 bp, synthetic construct
  source 1..28: mol_type = other DNA
ttccatttgcagttggttgaatccatgg

SEQ ID NO: 42716 - DNA, 28 bp, synthetic construct
  source 1..28: mol_type = other DNA
aaaaatcgtattttccatttgcagttgg

SEQ ID NO: 42717 - DNA, 28 bp, synthetic construct
  source 1..28: mol_type = other DNA
ggaaaatacgattttttttaaaaaaagg

SEQ ID NO: 42718 - DNA, 28 bp, synthetic construct
  source 1..28: mol_type = other DNA
aatacgattttttttaaaaaaaggatgg

SEQ ID NO: 42719 - DNA, 28 bp, synthetic construct
  source 1..28: mol_type = other DNA
gaaaaaagtctgtacatgttcaatacgg

SEQ ID NO: 42720 - DNA, 28 bp, synthetic construct
  source 1..28: mol_type = other DNA
tctttatgtagcatttacatttattagg

SEQ ID NO: 42721 - DNA, 28 bp, synthetic construct
  source 1..28: mol_type = other DNA
tagagattatttaattaaaatatacagg

SEQ ID NO: 42722 - DNA, 28 bp, synthetic construct
  source 1..28: mol_type = other DNA
agattatttaattaaaatatacaggagg

SEQ ID NO: 42723 - DNA, 28 bp, synthetic construct
  source 1..28: mol_type = other DNA
tgcaaattctgtaccattttgtatcagg

SEQ ID NO: 42724 - DNA, 28 bp, synthetic construct
  source 1..28: mol_type = other DNA
gcaaattctgtaccattttgtatcaggg

SEQ ID NO: 42725 - DNA, 28 bp, synthetic construct
  source 1..28: mol_type = other DNA
agatgctcaattccctgatacaaaatgg

SEQ ID NO: 42726 - DNA, 28 bp, synthetic construct
  source 1..28: mol_type = other DNA
cagggaattgagcatcttcagatgttgg

SEQ ID NO: 42727 - DNA, 28 bp, synthetic construct
  source 1..28: mol_type = other DNA
agcatcttcagatgttggtatctgcagg

SEQ ID NO: 42728 - DNA, 28 bp, synthetic construct
  source 1..28: mol_type = other DNA
gcatcttcagatgttggtatctgcaggg

SEQ ID NO: 42729 - DNA, 28 bp, synthetic construct
  source 1..28: mol_type = other DNA
cagatgttggtatctgcagggatcctgg

SEQ ID NO: 42730 - DNA, 28 bp, synthetic construct
  source 1..28: mol_type = other DNA
ttagtatctgcaggggtttggttccagg

SEQ ID NO: 42731 - DNA, 28 bp, synthetic construct
  source 1..28: mol_type = other DNA
tggaaccaaacccctgcagatactaagg

SEQ ID NO: 42732 - DNA, 28 bp, synthetic construct
  source 1..28: mol_type = other DNA
ggaaccaaacccctgcagatactaaggg

SEQ ID NO: 42733 - DNA, 28 bp, synthetic construct
  source 1..28: mol_type = other DNA
tcagcccttagtatctgcaggggtttgg

SEQ ID NO: 42734 - DNA, 28 bp, synthetic construct
  source 1..28: mol_type = other DNA
gatcgtcagcccttagtatctgcagggg

SEQ ID NO: 42735 - DNA, 28 bp, synthetic construct
  source 1..28: mol_type = other DNA
agatcgtcagcccttagtatctgcaggg

SEQ ID NO: 42736 - DNA, 28 bp, synthetic construct
  source 1..28: mol_type = other DNA
tagatcgtcagcccttagtatctgcagg

SEQ ID NO: 42737 - DNA, 28 bp, synthetic construct
  source 1..28: mol_type = other DNA
tgcagatactaagggctgacgatctagg

SEQ ID NO: 42738 - DNA, 28 bp, synthetic construct
  source 1..28: mol_type = other DNA
taagggctgacgatctaggtaagactgg

SEQ ID NO: 42739 - DNA, 28 bp, synthetic construct
  source 1..28: mol_type = other DNA
tctaggtaagactggatttaacagttgg

SEQ ID NO: 42740 - DNA, 28 bp, synthetic construct
  source 1..28: mol_type = other DNA
taacagttggaaaaaaaaaaaaaaaagg

SEQ ID NO: 42741 - DNA, 28 bp, synthetic construct
  source 1..28: mol_type = other DNA
tattttgttttaatttctacaggaaagg

SEQ ID NO: 42742 - DNA, 28 bp, synthetic construct
  source 1..28: mol_type = other DNA
atttgtattttgttttaatttctacagg

SEQ ID NO: 42743 - DNA, 28 bp, synthetic construct
  source 1..28: mol_type = other DNA
agaaattaaaacaaaatacaaattgagg

SEQ ID NO: 42744 - DNA, 28 bp, synthetic construct
  source 1..28: mol_type = other DNA
acaaattgaggaagctctgctacccagg

SEQ ID NO: 42745 - DNA, 28 bp, synthetic construct
  source 1..28: mol_type = other DNA
ggaagctctgctacccaggctgtcatgg

SEQ ID NO: 42746 - DNA, 28 bp, synthetic construct
  source 1..28: mol_type = other DNA
ttcaagttctctaccatgacagcctggg

SEQ ID NO: 42747 - DNA, 28 bp, synthetic construct
  source 1..28: mol_type = other DNA
cttcaagttctctaccatgacagcctgg

SEQ ID NO: 42748 - DNA, 28 bp, synthetic construct
  source 1..28: mol_type = other DNA
gtagagaacttgaagaagacctgtttgg

SEQ ID NO: 42749 - DNA, 28 bp, synthetic construct
  source 1..28: mol_type = other DNA
agaacttgaagaagacctgtttggatgg

SEQ ID NO: 42750 - DNA, 28 bp, synthetic construct
  source 1..28: mol_type = other DNA
aagaagacctgtttggatggacacctgg

SEQ ID NO: 42751 - DNA, 28 bp, synthetic construct
  source 1..28: mol_type = other DNA
tttgaaaccaggtgtccatccaaacagg

SEQ ID NO: 42752 - DNA, 28 bp, synthetic construct
  source 1..28: mol_type = other DNA
ggatggacacctggtttcaaaagtcagg

SEQ ID NO: 42753 - DNA, 28 bp, synthetic construct
  source 1..28: mol_type = other DNA
gacacctggtttcaaaagtcaggtgtgg

SEQ ID NO: 42754 - DNA, 28 bp, synthetic construct
  source 1..28: mol_type = other DNA
gtctccacacctgacttttgaaaccagg

SEQ ID NO: 42755 - DNA, 28 bp, synthetic construct
  source 1..28: mol_type = other DNA
aaagtcaggtgtggagactgttaaatgg

SEQ ID NO: 42756 - DNA, 28 bp, synthetic construct
  source 1..28: mol_type = other DNA
aagtcaggtgtggagactgttaaatggg

SEQ ID NO: 42757 - DNA, 28 bp, synthetic construct
  source 1..28: mol_type = other DNA
tcaggtgtggagactgttaaatgggagg

SEQ ID NO: 42758 - DNA, 28 bp, synthetic construct
  source 1..28: mol_type = other DNA
caggtgtggagactgttaaatgggaggg

SEQ ID NO: 42759 - DNA, 28 bp, synthetic construct
  source 1..28: mol_type = other DNA
gagggcctcatccataaatgatttctgg

SEQ ID NO: 42760 - DNA, 28 bp, synthetic construct
  source 1..28: mol_type = other DNA
cgttgccagaaatcatttatggatgagg

SEQ ID NO: 42761 - DNA, 28 bp, synthetic construct
  source 1..28: mol_type = other DNA
agaagacgttgccagaaatcatttatgg

SEQ ID NO: 42762 - DNA, 28 bp, synthetic construct
  source 1..28: mol_type = other DNA
aatgatttctggcaacgtcttcttcagg

SEQ ID NO: 42763 - DNA, 28 bp, synthetic construct
  source 1..28: mol_type = other DNA
gatttctggcaacgtcttcttcaggtgg

SEQ ID NO: 42764 - DNA, 28 bp, synthetic construct
  source 1..28: mol_type = other DNA
agcttgacgtctttttaatgttacttgg

SEQ ID NO: 42765 - DNA, 28 bp, synthetic construct
  source 1..28: mol_type = other DNA
gcttgacgtctttttaatgttacttggg

SEQ ID NO: 42766 - DNA, 28 bp, synthetic construct
  source 1..28: mol_type = other DNA
cttgacgtctttttaatgttacttgggg

SEQ ID NO: 42767 - DNA, 28 bp, synthetic construct
  source 1..28: mol_type = other DNA
gacgtctttttaatgttacttggggagg

SEQ ID NO: 42768 - DNA, 28 bp, synthetic construct
  source 1..28: mol_type = other DNA
acgtctttttaatgttacttggggaggg

SEQ ID NO: 42769 - DNA, 28 bp, synthetic construct
  source 1..28: mol_type = other DNA
ttacttggggagggagtgctcattaagg

SEQ ID NO: 42770 - DNA, 28 bp, synthetic construct
  source 1..28: mol_type = other DNA
tacttggggagggagtgctcattaaggg

SEQ ID NO: 42771 - DNA, 28 bp, synthetic construct
  source 1..28: mol_type = other DNA
gagggagtgctcattaagggatgccagg

SEQ ID NO: 42772 - DNA, 28 bp, synthetic construct
  source 1..28: mol_type = other DNA
agggagtgctcattaagggatgccaggg

SEQ ID NO: 42773 - DNA, 28 bp, synthetic construct
  source 1..28: mol_type = other DNA
cattaagggatgccagggccagctctgg

SEQ ID NO: 42774 - DNA, 28 bp, synthetic construct
  source 1..28: mol_type = other DNA
taagggatgccagggccagctctggtgg

SEQ ID NO: 42775 - DNA, 28 bp, synthetic construct
  source 1..28: mol_type = other DNA
tgccagggccagctctggtggttcctgg

SEQ ID NO: 42776 - DNA, 28 bp, synthetic construct
  source 1..28: mol_type = other DNA
gccagggccagctctggtggttcctggg

SEQ ID NO: 42777 - DNA, 28 bp, synthetic construct
  source 1..28: mol_type = other DNA
ccagggccagctctggtggttcctgggg

SEQ ID NO: 42778 - DNA, 28 bp, synthetic construct
  source 1..28: mol_type = other DNA
gggccagctctggtggttcctggggagg

SEQ ID NO: 42779 - DNA, 28 bp, synthetic construct
  source 1..28: mol_type = other DNA
cagcctccccaggaaccaccagagctgg

SEQ ID NO: 42780 - DNA, 28 bp, synthetic construct
  source 1..28: mol_type = other DNA
aagcagggaaggacgcagcctccccagg

SEQ ID NO: 42781 - DNA, 28 bp, synthetic construct
  source 1..28: mol_type = other DNA
tccttccctgcttctgcatgtcatgagg

SEQ ID NO: 42782 - DNA, 28 bp, synthetic construct
  source 1..28: mol_type = other DNA
gcctcatgacatgcagaagcagggaagg

SEQ ID NO: 42783 - DNA, 28 bp, synthetic construct
  source 1..28: mol_type = other DNA
tgctgcctcatgacatgcagaagcaggg

SEQ ID NO: 42784 - DNA, 28 bp, synthetic construct
  source 1..28: mol_type = other DNA
ctgctgcctcatgacatgcagaagcagg

SEQ ID NO: 42785 - DNA, 28 bp, synthetic construct
  source 1..28: mol_type = other DNA
ctgcttctgcatgtcatgaggcagcagg

SEQ ID NO: 42786 - DNA, 28 bp, synthetic construct
  source 1..28: mol_type = other DNA
ttctgcatgtcatgaggcagcaggaagg

SEQ ID NO: 42787 - DNA, 28 bp, synthetic construct
  source 1..28: mol_type = other DNA
aggtttcccctgcacctgtctgtcctgg

SEQ ID NO: 42788 - DNA, 28 bp, synthetic construct
  source 1..28: mol_type = other DNA
agggagccaggacagacaggtgcagggg

SEQ ID NO: 42789 - DNA, 28 bp, synthetic construct
  source 1..28: mol_type = other DNA
gagggagccaggacagacaggtgcaggg

SEQ ID NO: 42790 - DNA, 28 bp, synthetic construct
  source 1..28: mol_type = other DNA
agagggagccaggacagacaggtgcagg

SEQ ID NO: 42791 - DNA, 28 bp, synthetic construct
  source 1..28: mol_type = other DNA
tgcacctgtctgtcctggctccctctgg

SEQ ID NO: 42792 - DNA, 28 bp, synthetic construct
  source 1..28: mol_type = other DNA
gcacctgtctgtcctggctccctctggg

SEQ ID NO: 42793 - DNA, 28 bp, synthetic construct
  source 1..28: mol_type = other DNA
ctacccagagggagccaggacagacagg

SEQ ID NO: 42794 - DNA, 28 bp, synthetic construct
  source 1..28: mol_type = other DNA
agtagggggctacccagagggagccagg

SEQ ID NO: 42795 - DNA, 28 bp, synthetic construct
  source 1..28: mol_type = other DNA
acagaacagtagggggctacccagaggg

SEQ ID NO: 42796 - DNA, 28 bp, synthetic construct
  source 1..28: mol_type = other DNA
cacagaacagtagggggctacccagagg

SEQ ID NO: 42797 - DNA, 28 bp, synthetic construct
  source 1..28: mol_type = other DNA
ctgtgctgaagcacagaacagtaggggg

SEQ ID NO: 42798 - DNA, 28 bp, synthetic construct
  source 1..28: mol_type = other DNA
gctgtgctgaagcacagaacagtagggg

SEQ ID NO: 42799 - DNA, 28 bp, synthetic construct
  source 1..28: mol_type = other DNA
ggctgtgctgaagcacagaacagtaggg

SEQ ID NO: 42800 - DNA, 28 bp, synthetic construct
  source 1..28: mol_type = other DNA
aggctgtgctgaagcacagaacagtagg

SEQ ID NO: 42801 - DNA, 28 bp, synthetic construct
  source 1..28: mol_type = other DNA
tactgttctgtgcttcagcacagcctgg

SEQ ID NO: 42802 - DNA, 28 bp, synthetic construct
  source 1..28: mol_type = other DNA
cttcagcacagcctggtttgtcaagagg

SEQ ID NO: 42803 - DNA, 28 bp, synthetic construct
  source 1..28: mol_type = other DNA
cctggtttgtcaagaggcacatagttgg

SEQ ID NO: 42804 - DNA, 28 bp, synthetic construct
  source 1..28: mol_type = other DNA
ctggtttgtcaagaggcacatagttggg

SEQ ID NO: 42805 - DNA, 28 bp, synthetic construct
  source 1..28: mol_type = other DNA
tggtttgtcaagaggcacatagttgggg

SEQ ID NO: 42806 - DNA, 28 bp, synthetic construct
  source 1..28: mol_type = other DNA
ttgtcaagaggcacatagttggggctgg

SEQ ID NO: 42807 - DNA, 28 bp, synthetic construct
  source 1..28: mol_type = other DNA
tgtcaagaggcacatagttggggctggg

SEQ ID NO: 42808 - DNA, 28 bp, synthetic construct
  source 1..28: mol_type = other DNA
ggcacatagttggggctgggctgcatgg

SEQ ID NO: 42809 - DNA, 28 bp, synthetic construct
  source 1..28: mol_type = other DNA
tagttggggctgggctgcatggcacagg

SEQ ID NO: 42810 - DNA, 28 bp, synthetic construct
  source 1..28: mol_type = other DNA
agttggggctgggctgcatggcacaggg

SEQ ID NO: 42811 - DNA, 28 bp, synthetic construct
  source 1..28: mol_type = other DNA
gttggggctgggctgcatggcacagggg

SEQ ID NO: 42812 - DNA, 28 bp, synthetic construct
  source 1..28: mol_type = other DNA
atggcacaggggcttatgtgcctgctgg

SEQ ID NO: 42813 - DNA, 28 bp, synthetic construct
  source 1..28: mol_type = other DNA
taaggctgaaaattaaataaccagcagg

SEQ ID NO: 42814 - DNA, 28 bp, synthetic construct
  source 1..28: mol_type = other DNA
acaggaaaatattaaagaaaacttaagg

SEQ ID NO: 42815 - DNA, 28 bp, synthetic construct
  source 1..28: mol_type = other DNA
taagttttctttaatattttcctgttgg

SEQ ID NO: 42816 - DNA, 28 bp, synthetic construct
  source 1..28: mol_type = other DNA
taatattttcctgttggctatttaaagg

SEQ ID NO: 42817 - DNA, 28 bp, synthetic construct
  source 1..28: mol_type = other DNA
tttcctgttggctatttaaaggttttgg

SEQ ID NO: 42818 - DNA, 28 bp, synthetic construct
  source 1..28: mol_type = other DNA
taaccaaaacctttaaatagccaacagg

SEQ ID NO: 42819 - DNA, 28 bp, synthetic construct
  source 1..28: mol_type = other DNA
tacattgtcatcttgattgtagataagg

SEQ ID NO: 42820 - DNA, 28 bp, synthetic construct
  source 1..28: mol_type = other DNA
taattgaattatcttatttataacacgg

SEQ ID NO: 42821 - DNA, 28 bp, synthetic construct
  source 1..28: mol_type = other DNA
acacacacatatttatttggaggtgagg

SEQ ID NO: 42822 - DNA, 28 bp, synthetic construct
  source 1..28: mol_type = other DNA
cacagacacacacatatttatttggagg

SEQ ID NO: 42823 - DNA, 28 bp, synthetic construct
  source 1..28: mol_type = other DNA
acacacagacacacacatatttatttgg

SEQ ID NO: 42824 - DNA, 28 bp, synthetic construct
  source 1..28: mol_type = other DNA
gtctgtgtgtgtgtatatatgtatgtgg

SEQ ID NO: 42825 - DNA, 28 bp, synthetic construct
  source 1..28: mol_type = other DNA
tgtgtgtgtgtatatatgtatgtggcgg

SEQ ID NO: 42826 - DNA, 28 bp, synthetic construct
  source 1..28: mol_type = other DNA
gtgtgtatatatgtatgtggcggagagg

SEQ ID NO: 42827 - DNA, 28 bp, synthetic construct
  source 1..28: mol_type = other DNA
tgtgtatatatgtatgtggcggagaggg

SEQ ID NO: 42828 - DNA, 28 bp, synthetic construct
  source 1..28: mol_type = other DNA
atgtatgtggcggagagggagagagtgg

SEQ ID NO: 42829 - DNA, 28 bp, synthetic construct
  source 1..28: mol_type = other DNA
tgtatgtggcggagagggagagagtggg

SEQ ID NO: 42830 - DNA, 28 bp, synthetic construct
  source 1..28: mol_type = other DNA
gtatgtggcggagagggagagagtgggg

SEQ ID NO: 42831 - DNA, 28 bp, synthetic construct
  source 1..28: mol_type = other DNA
gtggcggagagggagagagtggggaagg

SEQ ID NO: 42832 - DNA, 28 bp, synthetic construct
  source 1..28: mol_type = other DNA
gagagcagtgttatcatacatagagagg

SEQ ID NO: 42833 - DNA, 28 bp, synthetic construct
  source 1..28: mol_type = other DNA
ctttataaagctgacagtgagggatggg

SEQ ID NO: 42834 - DNA, 28 bp, synthetic construct
  source 1..28: mol_type = other DNA
ccatccctcactgtcagctttataaagg

SEQ ID NO: 42835 - DNA, 28 bp, synthetic construct
  source 1..28: mol_type = other DNA
aactcctttataaagctgacagtgaggg

SEQ ID NO: 42836 - DNA, 28 bp, synthetic construct
  source 1..28: mol_type = other DNA
aaactcctttataaagctgacagtgagg

SEQ ID NO: 42837 - DNA, 28 bp, synthetic construct
  source 1..28: mol_type = other DNA
gtcttataaaacattcttctgtggatgg

SEQ ID NO: 42838 - DNA, 28 bp, synthetic construct
  source 1..28: mol_type = other DNA
ccacagaagaatgttttataagactagg

SEQ ID NO: 42839 - DNA, 28 bp, synthetic construct
  source 1..28: mol_type = other DNA
agactaggaaaacacgttgaaaactagg

SEQ ID NO: 42840 - DNA, 28 bp, synthetic construct
  source 1..28: mol_type = other DNA
actaaatatgttgttactgttgctaagg

SEQ ID NO: 42841 - DNA, 28 bp, synthetic construct
  source 1..28: mol_type = other DNA
aaggattttctccttagaataatttagg

SEQ ID NO: 42842 - DNA, 28 bp, synthetic construct
  source 1..28: mol_type = other DNA
tttttaaaaatcctaaattattctaagg

SEQ ID NO: 42843 - DNA, 28 bp, synthetic construct
  source 1..28: mol_type = other DNA
ctgtttgccaaatgctgtagataaatgg

SEQ ID NO: 42844 - DNA, 28 bp, synthetic construct
  source 1..28: mol_type = other DNA
aatctggccatttatctacagcatttgg

SEQ ID NO: 42845 - DNA, 28 bp, synthetic construct
  source 1..28: mol_type = other DNA
aaatggccagattcttcctatccctagg

SEQ ID NO: 42846 - DNA, 28 bp, synthetic construct
  source 1..28: mol_type = other DNA
aggaatcctagggataggaagaatctgg

SEQ ID NO: 42847 - DNA, 28 bp, synthetic construct
  source 1..28: mol_type = other DNA
aaaataataaaggaatcctagggatagg

SEQ ID NO: 42848 - DNA, 28 bp, synthetic construct
  source 1..28: mol_type = other DNA
gaaaaaaaataataaaggaatcctaggg

SEQ ID NO: 42849 - DNA, 28 bp, synthetic construct
  source 1..28: mol_type = other DNA
tgaaaaaaaataataaaggaatcctagg

SEQ ID NO: 42850 - DNA, 28 bp, synthetic construct
  source 1..28: mol_type = other DNA
caaaatctgtgaaaaaaaataataaagg

SEQ ID NO: 42851 - DNA, 28 bp, synthetic construct
  source 1..28: mol_type = other DNA
ttttttttcacagattttgagaacaagg

SEQ ID NO: 42852 - DNA, 28 bp, synthetic construct
  source 1..28: mol_type = other DNA
tttttttcacagattttgagaacaaggg

SEQ ID NO: 42853 - DNA, 28 bp, synthetic construct
  source 1..28: mol_type = other DNA
ttttttcacagattttgagaacaagggg

SEQ ID NO: 42854 - DNA, 28 bp, synthetic construct
  source 1..28: mol_type = other DNA
tttttcacagattttgagaacaaggggg

SEQ ID NO: 42855 - DNA, 28 bp, synthetic construct
  source 1..28: mol_type = other DNA
ttgagaacaagggggagagatagtatgg

SEQ ID NO: 42856 - DNA, 28 bp, synthetic construct
  source 1..28: mol_type = other DNA
tgacaacacagttctataagattaatgg

SEQ ID NO: 42857 - DNA, 28 bp, synthetic construct
  source 1..28: mol_type = other DNA
acccaaattcctgcttgtttgaacatgg

SEQ ID NO: 42858 - DNA, 28 bp, synthetic construct
  source 1..28: mol_type = other DNA
gccatgttcaaacaagcaggaatttggg

SEQ ID NO: 42859 - DNA, 28 bp, synthetic construct
  source 1..28: mol_type = other DNA
tgccatgttcaaacaagcaggaatttgg

SEQ ID NO: 42860 - DNA, 28 bp, synthetic construct
  source 1..28: mol_type = other DNA
atgaagatgccatgttcaaacaagcagg

SEQ ID NO: 42861 - DNA, 28 bp, synthetic construct
  source 1..28: mol_type = other DNA
ttgaacatggcatcttcatagattcagg

SEQ ID NO: 42862 - DNA, 28 bp, synthetic construct
  source 1..28: mol_type = other DNA
ttcaggattcactaccctctatagctgg

SEQ ID NO: 42863 - DNA, 28 bp, synthetic construct
  source 1..28: mol_type = other DNA
ataattttcaagatccagctatagaggg

SEQ ID NO: 42864 - DNA, 28 bp, synthetic construct
  source 1..28: mol_type = other DNA
gataattttcaagatccagctatagagg

SEQ ID NO: 42865 - DNA, 28 bp, synthetic construct
  source 1..28: mol_type = other DNA
ctatagctggatcttgaaaattatctgg

SEQ ID NO: 42866 - DNA, 28 bp, synthetic construct
  source 1..28: mol_type = other DNA
ctggccagataattttgcatctgcttgg

SEQ ID NO: 42867 - DNA, 28 bp, synthetic construct
  source 1..28: mol_type = other DNA
tcatccaagcagatgcaaaattatctgg

SEQ ID NO: 42868 - DNA, 28 bp, synthetic construct
  source 1..28: mol_type = other DNA
ggatgattgtagactgagatgtgagtgg

SEQ ID NO: 42869 - DNA, 28 bp, synthetic construct
  source 1..28: mol_type = other DNA
tgattgtagactgagatgtgagtggagg

SEQ ID NO: 42870 - DNA, 28 bp, synthetic construct
  source 1..28: mol_type = other DNA
taactgccaaccaagaagtatttatcgg

SEQ ID NO: 42871 - DNA, 28 bp, synthetic construct
  source 1..28: mol_type = other DNA
aagtgtccgataaatacttcttggttgg

SEQ ID NO: 42872 - DNA, 28 bp, synthetic construct
  source 1..28: mol_type = other DNA
tagtaagtgtccgataaatacttcttgg

SEQ ID NO: 42873 - DNA, 28 bp, synthetic construct
  source 1..28: mol_type = other DNA
aagaagtatttatcggacacttactagg

SEQ ID NO: 42874 - DNA, 28 bp, synthetic construct
  source 1..28: mol_type = other DNA
tttatcggacacttactaggtgcctagg

SEQ ID NO: 42875 - DNA, 28 bp, synthetic construct
  source 1..28: mol_type = other DNA
tactaggtgcctaggattgtatcagagg

SEQ ID NO: 42876 - DNA, 28 bp, synthetic construct
  source 1..28: mol_type = other DNA
actaggtgcctaggattgtatcagaggg

SEQ ID NO: 42877 - DNA, 28 bp, synthetic construct
  source 1..28: mol_type = other DNA
ttcatattccctctgatacaatcctagg

SEQ ID NO: 42878 - DNA, 28 bp, synthetic construct
  source 1..28: mol_type = other DNA
tctgtcgttaaaactaggtagggcaggg

SEQ ID NO: 42879 - DNA, 28 bp, synthetic construct
  source 1..28: mol_type = other DNA
ttctgtcgttaaaactaggtagggcagg

SEQ ID NO: 42880 - DNA, 28 bp, synthetic construct
  source 1..28: mol_type = other DNA
gatattctgtcgttaaaactaggtaggg

SEQ ID NO: 42881 - DNA, 28 bp, synthetic construct
  source 1..28: mol_type = other DNA
agatattctgtcgttaaaactaggtagg

SEQ ID NO: 42882 - DNA, 28 bp, synthetic construct
  source 1..28: mol_type = other DNA
taatagatattctgtcgttaaaactagg

SEQ ID NO: 42883 - DNA, 28 bp, synthetic construct
  source 1..28: mol_type = other DNA
gttttaacgacagaatatctattaaagg

SEQ ID NO: 42884 - DNA, 28 bp, synthetic construct
  source 1..28: mol_type = other DNA
tatctattaaaggctacttagctgaagg

SEQ ID NO: 42885 - DNA, 28 bp, synthetic construct
  source 1..28: mol_type = other DNA
atctattaaaggctacttagctgaaggg

SEQ ID NO: 42886 - DNA, 28 bp, synthetic construct
  source 1..28: mol_type = other DNA
ttaaaggctacttagctgaagggtaagg

SEQ ID NO: 42887 - DNA, 28 bp, synthetic construct
  source 1..28: mol_type = other DNA
taaaggctacttagctgaagggtaaggg

SEQ ID NO: 42888 - DNA, 28 bp, synthetic construct
  source 1..28: mol_type = other DNA
tacttagctgaagggtaagggtgacagg

SEQ ID NO: 42889 - DNA, 28 bp, synthetic construct
  source 1..28: mol_type = other DNA
gctgaagggtaagggtgacaggtctagg

SEQ ID NO: 42890 - DNA, 28 bp, synthetic construct
  source 1..28: mol_type = other DNA
ctgaagggtaagggtgacaggtctaggg

SEQ ID NO: 42891 - DNA, 28 bp, synthetic construct
  source 1..28: mol_type = other DNA
tgaagggtaagggtgacaggtctagggg

SEQ ID NO: 42892 - DNA, 28 bp, synthetic construct
  source 1..28: mol_type = other DNA
agggtgacaggtctaggggaagctttgg

SEQ ID NO: 42893 - DNA, 28 bp, synthetic construct
  source 1..28: mol_type = other DNA
gggtgacaggtctaggggaagctttggg

SEQ ID NO: 42894 - DNA, 28 bp, synthetic construct
  source 1..28: mol_type = other DNA
tgacaggtctaggggaagctttgggagg

SEQ ID NO: 42895 - DNA, 28 bp, synthetic construct
  source 1..28: mol_type = other DNA
caggtctaggggaagctttgggaggtgg

SEQ ID NO: 42896 - DNA, 28 bp, synthetic construct
  source 1..28: mol_type = other DNA
aggtggtgtgctgtgacagaaaaagtgg

SEQ ID NO: 42897 - DNA, 28 bp, synthetic construct
  source 1..28: mol_type = other DNA
gctgtgacagaaaaagtggcagagtagg

SEQ ID NO: 42898 - DNA, 28 bp, synthetic construct
  source 1..28: mol_type = other DNA
ctgtgacagaaaaagtggcagagtaggg

SEQ ID NO: 42899 - DNA, 28 bp, synthetic construct
  source 1..28: mol_type = other DNA
agtgacagaaacagggctagaatgcagg

SEQ ID NO: 42900 - DNA, 28 bp, synthetic construct
  source 1..28: mol_type = other DNA
gtgtacagagcaagtgacagaaacaggg

SEQ ID NO: 42901 - DNA, 28 bp, synthetic construct
  source 1..28: mol_type = other DNA
agtgtacagagcaagtgacagaaacagg

SEQ ID NO: 42902 - DNA, 28 bp, synthetic construct
  source 1..28: mol_type = other DNA
gcagaggaggaaactaaagctcaagagg

SEQ ID NO: 42903 - DNA, 28 bp, synthetic construct
  source 1..28: mol_type = other DNA
ttagtttcctcctctgcataatgagagg

SEQ ID NO: 42904 - DNA, 28 bp, synthetic construct
  source 1..28: mol_type = other DNA
tagtttcctcctctgcataatgagaggg

SEQ ID NO: 42905 - DNA, 28 bp, synthetic construct
  source 1..28: mol_type = other DNA
gtctaaccctctcattatgcagaggagg

SEQ ID NO: 42906 - DNA, 28 bp, synthetic construct
  source 1..28: mol_type = other DNA
gtagtctaaccctctcattatgcagagg

SEQ ID NO: 42907 - DNA, 28 bp, synthetic construct
  source 1..28: mol_type = other DNA
gagagggttagactactgaattgtatgg

SEQ ID NO: 42908 - DNA, 28 bp, synthetic construct
  source 1..28: mol_type = other DNA
agagggttagactactgaattgtatggg

SEQ ID NO: 42909 - DNA, 28 bp, synthetic construct
  source 1..28: mol_type = other DNA
tgtatgggaaaaaaatacaaattcctgg

SEQ ID NO: 42910 - DNA, 28 bp, synthetic construct
  source 1..28: mol_type = other DNA
gtatgggaaaaaaatacaaattcctggg

SEQ ID NO: 42911 - DNA, 28 bp, synthetic construct
  source 1..28: mol_type = other DNA
aaaaaaatacaaattcctgggtcctagg

SEQ ID NO: 42912 - DNA, 28 bp, synthetic construct
  source 1..28: mol_type = other DNA
attcagcaggcatggcctaggacccagg

SEQ ID NO: 42913 - DNA, 28 bp, synthetic construct
  source 1..28: mol_type = other DNA
cagtcggattcagcaggcatggcctagg

SEQ ID NO: 42914 - DNA, 28 bp, synthetic construct
  source 1..28: mol_type = other DNA
ccatgcctgctgaatccgactgttcagg

SEQ ID NO: 42915 - DNA, 28 bp, synthetic construct
  source 1..28: mol_type = other DNA
ctcttcctgaacagtcggattcagcagg

SEQ ID NO: 42916 - DNA, 28 bp, synthetic construct
  source 1..28: mol_type = other DNA
ctgctgaatccgactgttcaggaagagg

SEQ ID NO: 42917 - DNA, 28 bp, synthetic construct
  source 1..28: mol_type = other DNA
aatccgactgttcaggaagaggcctagg

SEQ ID NO: 42918 - DNA, 28 bp, synthetic construct
  source 1..28: mol_type = other DNA
tttcctaggcctcttcctgaacagtcgg

SEQ ID NO: 42919 - DNA, 28 bp, synthetic construct
  source 1..28: mol_type = other DNA
caggaagaggcctaggaaatctgtgagg

SEQ ID NO: 42920 - DNA, 28 bp, synthetic construct
  source 1..28: mol_type = other DNA
aggaagaggcctaggaaatctgtgaggg

SEQ ID NO: 42921 - DNA, 28 bp, synthetic construct
  source 1..28: mol_type = other DNA
ctggggattccctcacagatttcctagg

SEQ ID NO: 42922 - DNA, 28 bp, synthetic construct
  source 1..28: mol_type = other DNA
ctaggaaatctgtgagggaatccccagg

SEQ ID NO: 42923 - DNA, 28 bp, synthetic construct
  source 1..28: mol_type = other DNA
taggaaatctgtgagggaatccccaggg

SEQ ID NO: 42924 - DNA, 28 bp, synthetic construct
  source 1..28: mol_type = other DNA
aggaaatctgtgagggaatccccagggg

SEQ ID NO: 42925 - DNA, 28 bp, synthetic construct
  source 1..28: mol_type = other DNA
cctggctggtcacgagattcccctgggg

SEQ ID NO: 42926 - DNA, 28 bp, synthetic construct
  source 1..28: mol_type = other DNA
acctggctggtcacgagattcccctggg

SEQ ID NO: 42927 - DNA, 28 bp, synthetic construct
  source 1..28: mol_type = other DNA
cacctggctggtcacgagattcccctgg

SEQ ID NO: 42928 - DNA, 28 bp, synthetic construct
  source 1..28: mol_type = other DNA
ccagccaggtgtgaaatctgctaactgg

SEQ ID NO: 42929 - DNA, 28 bp, synthetic construct
  source 1..28: mol_type = other DNA
tcttccagttagcagatttcacacctgg

SEQ ID NO: 42930 - DNA, 28 bp, synthetic construct
  source 1..28: mol_type = other DNA
gcttccttcactttttgtgattttgtgg

SEQ ID NO: 42931 - DNA, 28 bp, synthetic construct
  source 1..28: mol_type = other DNA
atgaccacaaaatcacaaaaagtgaagg

SEQ ID NO: 42932 - DNA, 28 bp, synthetic construct
  source 1..28: mol_type = other DNA
gttactgtattattctacgtaaatgtgg

SEQ ID NO: 42933 - DNA, 28 bp, synthetic construct
  source 1..28: mol_type = other DNA
ttactgtattattctacgtaaatgtggg

SEQ ID NO: 42934 - DNA, 28 bp, synthetic construct
  source 1..28: mol_type = other DNA
attattctacgtaaatgtgggtacttgg

SEQ ID NO: 42935 - DNA, 28 bp, synthetic construct
  source 1..28: mol_type = other DNA
cctcaacctgctgtttgtttcctagagg

SEQ ID NO: 42936 - DNA, 28 bp, synthetic construct
  source 1..28: mol_type = other DNA
ctaacacctctaggaaacaaacagcagg

SEQ ID NO: 42937 - DNA, 28 bp, synthetic construct
  source 1..28: mol_type = other DNA
gtatttaaagactactaacacctctagg

SEQ ID NO: 42938 - DNA, 28 bp, synthetic construct
  source 1..28: mol_type = other DNA
tctttaaatacaagtaagacttaagagg

SEQ ID NO: 42939 - DNA, 28 bp, synthetic construct
  source 1..28: mol_type = other DNA
aagaggatatttgatgttatttacctgg

SEQ ID NO: 42940 - DNA, 28 bp, synthetic construct
  source 1..28: mol_type = other DNA
taaataaaaggggaagaaaatatccagg

SEQ ID NO: 42941 - DNA, 28 bp, synthetic construct
  source 1..28: mol_type = other DNA
ttttcttccccttttatttatttagagg

SEQ ID NO: 42942 - DNA, 28 bp, synthetic construct
  source 1..28: mol_type = other DNA
tcaatttcctctaaataaataaaagggg

SEQ ID NO: 42943 - DNA, 28 bp, synthetic construct
  source 1..28: mol_type = other DNA
ctcaatttcctctaaataaataaaaggg

SEQ ID NO: 42944 - DNA, 28 bp, synthetic construct
  source 1..28: mol_type = other DNA
tctcaatttcctctaaataaataaaagg

SEQ ID NO: 42945 - DNA, 28 bp, synthetic construct
  source 1..28: mol_type = other DNA
tttatttagaggaaattgagattctagg

SEQ ID NO: 42946 - DNA, 28 bp, synthetic construct
  source 1..28: mol_type = other DNA
ccaaaaaaatgaaaacaaaattctaagg

SEQ ID NO: 42947 - DNA, 28 bp, synthetic construct
  source 1..28: mol_type = other DNA
taaattttcattataaagtagcaaatgg

SEQ ID NO: 42948 - DNA, 28 bp, synthetic construct
  source 1..28: mol_type = other DNA
ttataatgaaaatttaaaaattatatgg

SEQ ID NO: 42949 - DNA, 28 bp, synthetic construct
  source 1..28: mol_type = other DNA
tataatgaaaatttaaaaattatatggg

SEQ ID NO: 42950 - DNA, 28 bp, synthetic construct
  source 1..28: mol_type = other DNA
aaaattatatgggaagatttttctctgg

SEQ ID NO: 42951 - DNA, 28 bp, synthetic construct
  source 1..28: mol_type = other DNA
aaattatatgggaagatttttctctggg

SEQ ID NO: 42952 - DNA, 28 bp, synthetic construct
  source 1..28: mol_type = other DNA
taacaaatccttgtcataaagtaagagg

SEQ ID NO: 42953 - DNA, 28 bp, synthetic construct
  source 1..28: mol_type = other DNA
taaaaagacctcttactttatgacaagg

SEQ ID NO: 42954 - DNA, 28 bp, synthetic construct
  source 1..28: mol_type = other DNA
ataaagtaagaggtctttttaaagtagg

SEQ ID NO: 42955 - DNA, 28 bp, synthetic construct
  source 1..28: mol_type = other DNA
agtaagaggtctttttaaagtaggtagg

SEQ ID NO: 42956 - DNA, 28 bp, synthetic construct
  source 1..28: mol_type = other DNA
gtctttttaaagtaggtaggctataagg

SEQ ID NO: 42957 - DNA, 28 bp, synthetic construct
  source 1..28: mol_type = other DNA
agaaaggagtattattttaaattacagg

SEQ ID NO: 42958 - DNA, 28 bp, synthetic construct
  source 1..28: mol_type = other DNA
aatttaaaataatactcctttctctagg

SEQ ID NO: 42959 - DNA, 28 bp, synthetic construct
  source 1..28: mol_type = other DNA
atttaaaataatactcctttctctaggg

SEQ ID NO: 42960 - DNA, 28 bp, synthetic construct
  source 1..28: mol_type = other DNA
aaataatactcctttctctagggtttgg

SEQ ID NO: 42961 - DNA, 28 bp, synthetic construct
  source 1..28: mol_type = other DNA
gagaattgcaccaaaccctagagaaagg

SEQ ID NO: 42962 - DNA, 28 bp, synthetic construct
  source 1..28: mol_type = other DNA
ggaattcaaatgttatcttcattaatgg

SEQ ID NO: 42963 - DNA, 28 bp, synthetic construct
  source 1..28: mol_type = other DNA
agataacatttgaattccccaaagcagg

SEQ ID NO: 42964 - DNA, 28 bp, synthetic construct
  source 1..28: mol_type = other DNA
acatttgaattccccaaagcaggtgagg

SEQ ID NO: 42965 - DNA, 28 bp, synthetic construct
  source 1..28: mol_type = other DNA
gaattccccaaagcaggtgaggagtcgg

SEQ ID NO: 42966 - DNA, 28 bp, synthetic construct
  source 1..28: mol_type = other DNA
aattccccaaagcaggtgaggagtcggg

SEQ ID NO: 42967 - DNA, 28 bp, synthetic construct
  source 1..28: mol_type = other DNA
attccccaaagcaggtgaggagtcgggg

SEQ ID NO: 42968 - DNA, 28 bp, synthetic construct
  source 1..28: mol_type = other DNA
cctccccgactcctcacctgctttgggg

SEQ ID NO: 42969 - DNA, 28 bp, synthetic construct
  source 1..28: mol_type = other DNA
tcctccccgactcctcacctgctttggg

SEQ ID NO: 42970 - DNA, 28 bp, synthetic construct
  source 1..28: mol_type = other DNA
ctcctccccgactcctcacctgctttgg

SEQ ID NO: 42971 - DNA, 28 bp, synthetic construct
  source 1..28: mol_type = other DNA
ttaaaatgaaaactcactgcaaaagagg

SEQ ID NO: 42972 - DNA, 28 bp, synthetic construct
  source 1..28: mol_type = other DNA
aaatgaaaactcactgcaaaagaggagg

SEQ ID NO: 42973 - DNA, 28 bp, synthetic construct
  source 1..28: mol_type = other DNA
aaactcactgcaaaagaggaggcagagg

SEQ ID NO: 42974 - DNA, 28 bp, synthetic construct
  source 1..28: mol_type = other DNA
ctgcaaaagaggaggcagaggaagaagg

SEQ ID NO: 42975 - DNA, 28 bp, synthetic construct
  source 1..28: mol_type = other DNA
gtaaaccccttaaagcagatgtgtgtgg

SEQ ID NO: 42976 - DNA, 28 bp, synthetic construct
  source 1..28: mol_type = other DNA
taaaccccttaaagcagatgtgtgtggg

SEQ ID NO: 42977 - DNA, 28 bp, synthetic construct
  source 1..28: mol_type = other DNA
aaaccccttaaagcagatgtgtgtgggg

SEQ ID NO: 42978 - DNA, 28 bp, synthetic construct
  source 1..28: mol_type = other DNA
aggccccacacacatctgctttaagggg

SEQ ID NO: 42979 - DNA, 28 bp, synthetic construct
  source 1..28: mol_type = other DNA
aaggccccacacacatctgctttaaggg

SEQ ID NO: 42980 - DNA, 28 bp, synthetic construct
  source 1..28: mol_type = other DNA
taaggccccacacacatctgctttaagg

SEQ ID NO: 42981 - DNA, 28 bp, synthetic construct
  source 1..28: mol_type = other DNA
atgtgtgtggggccttatgaagaccagg

SEQ ID NO: 42982 - DNA, 28 bp, synthetic construct
  source 1..28: mol_type = other DNA
gggccttatgaagaccaggattctgcgg

SEQ ID NO: 42983 - DNA, 28 bp, synthetic construct
  source 1..28: mol_type = other DNA
ggccttatgaagaccaggattctgcggg

SEQ ID NO: 42984 - DNA, 28 bp, synthetic construct
  source 1..28: mol_type = other DNA
cacccgcagaatcctggtcttcataagg

SEQ ID NO: 42985 - DNA, 28 bp, synthetic construct
  source 1..28: mol_type = other DNA
tgaagaccaggattctgcgggtgtcagg

SEQ ID NO: 42986 - DNA, 28 bp, synthetic construct
  source 1..28: mol_type = other DNA
gaagaccaggattctgcgggtgtcaggg

SEQ ID NO: 42987 - DNA, 28 bp, synthetic construct
  source 1..28: mol_type = other DNA
aagaccaggattctgcgggtgtcagggg

SEQ ID NO: 42988 - DNA, 28 bp, synthetic construct
  source 1..28: mol_type = other DNA
caatcccctgacacccgcagaatcctgg

SEQ ID NO: 42989 - DNA, 28 bp, synthetic construct
  source 1..28: mol_type = other DNA
gggattgcccctcttgacagagactagg

SEQ ID NO: 42990 - DNA, 28 bp, synthetic construct
  source 1..28: mol_type = other DNA
ggattgcccctcttgacagagactaggg

SEQ ID NO: 42991 - DNA, 28 bp, synthetic construct
  source 1..28: mol_type = other DNA
ctaaaaccctagtctctgtcaagagggg

SEQ ID NO: 42992 - DNA, 28 bp, synthetic construct
  source 1..28: mol_type = other DNA
tctaaaaccctagtctctgtcaagaggg

SEQ ID NO: 42993 - DNA, 28 bp, synthetic construct
  source 1..28: mol_type = other DNA
gtctaaaaccctagtctctgtcaagagg

SEQ ID NO: 42994 - DNA, 28 bp, synthetic construct
  source 1..28: mol_type = other DNA
tgacagagactagggttttagactgagg

SEQ ID NO: 42995 - DNA, 28 bp, synthetic construct
  source 1..28: mol_type = other DNA
agggttttagactgaggcttcctgcagg

SEQ ID NO: 42996 - DNA, 28 bp, synthetic construct
  source 1..28: mol_type = other DNA
gggttttagactgaggcttcctgcaggg

SEQ ID NO: 42997 - DNA, 28 bp, synthetic construct
  source 1..28: mol_type = other DNA
gagaagggcaatgcgaacaccctgcagg

SEQ ID NO: 42998 - DNA, 28 bp, synthetic construct
  source 1..28: mol_type = other DNA
gaaaggtctgaaggggaacggagaaggg

SEQ ID NO: 42999 - DNA, 28 bp, synthetic construct
  source 1..28: mol_type = other DNA
agaaaggtctgaaggggaacggagaagg

SEQ ID NO: 43000 - DNA, 28 bp, synthetic construct
  source 1..28: mol_type = other DNA
ttctccgttccccttcagacctttctgg

SEQ ID NO: 43001 - DNA, 28 bp, synthetic construct
  source 1..28: mol_type = other DNA
tctccgttccccttcagacctttctggg

SEQ ID NO: 43002 - DNA, 28 bp, synthetic construct
  source 1..28: mol_type = other DNA
ctccgttccccttcagacctttctgggg

SEQ ID NO: 43003 - DNA, 28 bp, synthetic construct
  source 1..28: mol_type = other DNA
ctccccagaaaggtctgaaggggaacgg

SEQ ID NO: 43004 - DNA, 28 bp, synthetic construct
  source 1..28: mol_type = other DNA
ctcttctccccagaaaggtctgaagggg

SEQ ID NO: 43005 - DNA, 28 bp, synthetic construct
  source 1..28: mol_type = other DNA
cctcttctccccagaaaggtctgaaggg

SEQ ID NO: 43006 - DNA, 28 bp, synthetic construct
  source 1..28: mol_type = other DNA
acctcttctccccagaaaggtctgaagg

SEQ ID NO: 43007 - DNA, 28 bp, synthetic construct
  source 1..28: mol_type = other DNA
ttcagacctttctggggagaagaggtgg

SEQ ID NO: 43008 - DNA, 28 bp, synthetic construct
  source 1..28: mol_type = other DNA
tcagacctttctggggagaagaggtggg

SEQ ID NO: 43009 - DNA, 28 bp, synthetic construct
  source 1..28: mol_type = other DNA
gacctttctggggagaagaggtgggagg

SEQ ID NO: 43010 - DNA, 28 bp, synthetic construct
  source 1..28: mol_type = other DNA
ctcctcccacctcttctccccagaaagg

SEQ ID NO: 43011 - DNA, 28 bp, synthetic construct
  source 1..28: mol_type = other DNA
ctttctggggagaagaggtgggaggagg

SEQ ID NO: 43012 - DNA, 28 bp, synthetic construct
  source 1..28: mol_type = other DNA
tttctggggagaagaggtgggaggaggg

SEQ ID NO: 43013 - DNA, 28 bp, synthetic construct
  source 1..28: mol_type = other DNA
ttctggggagaagaggtgggaggagggg

SEQ ID NO: 43014 - DNA, 28 bp, synthetic construct
  source 1..28: mol_type = other DNA
agactgttcatcttattctgaatcctgg

SEQ ID NO: 43015 - DNA, 28 bp, synthetic construct
  source 1..28: mol_type = other DNA
ttattctgaatcctggagcagctgaagg

SEQ ID NO: 43016 - DNA, 28 bp, synthetic construct
  source 1..28: mol_type = other DNA
tcaagagaaaaccttcagctgctccagg

SEQ ID NO: 43017 - DNA, 28 bp, synthetic construct
  source 1..28: mol_type = other DNA
gcagctgaaggttttctcttgagtcagg

SEQ ID NO: 43018 - DNA, 28 bp, synthetic construct
  source 1..28: mol_type = other DNA
ggttttctcttgagtcaggatgcagtgg

SEQ ID NO: 43019 - DNA, 28 bp, synthetic construct
  source 1..28: mol_type = other DNA
gtggtaatgcattaaccagcaagtgtgg

SEQ ID NO: 43020 - DNA, 28 bp, synthetic construct
  source 1..28: mol_type = other DNA
atgcattaaccagcaagtgtggccaagg

SEQ ID NO: 43021 - DNA, 28 bp, synthetic construct
  source 1..28: mol_type = other DNA
tttcattatccttggccacacttgctgg

SEQ ID NO: 43022 - DNA, 28 bp, synthetic construct
  source 1..28: mol_type = other DNA
agtgtggccaaggataatgaaaaagtgg

SEQ ID NO: 43023 - DNA, 28 bp, synthetic construct
  source 1..28: mol_type = other DNA
gtgtggccaaggataatgaaaaagtggg

SEQ ID NO: 43024 - DNA, 28 bp, synthetic construct
  source 1..28: mol_type = other DNA
gccaaggataatgaaaaagtgggaaagg

SEQ ID NO: 43025 - DNA, 28 bp, synthetic construct
  source 1..28: mol_type = other DNA
tcctttcccactttttcattatccttgg

SEQ ID NO: 43026 - DNA, 28 bp, synthetic construct
  source 1..28: mol_type = other DNA
aggataatgaaaaagtgggaaaggaagg

SEQ ID NO: 43027 - DNA, 28 bp, synthetic construct
  source 1..28: mol_type = other DNA
ctggatgctacaatcagggaggaggagg

SEQ ID NO: 43028 - DNA, 28 bp, synthetic construct
  source 1..28: mol_type = other DNA
ctgctggatgctacaatcagggaggagg

SEQ ID NO: 43029 - DNA, 28 bp, synthetic construct
  source 1..28: mol_type = other DNA
agactgctggatgctacaatcagggagg

SEQ ID NO: 43030 - DNA, 28 bp, synthetic construct
  source 1..28: mol_type = other DNA
cagagactgctggatgctacaatcaggg

SEQ ID NO: 43031 - DNA, 28 bp, synthetic construct
  source 1..28: mol_type = other DNA
acagagactgctggatgctacaatcagg

SEQ ID NO: 43032 - DNA, 28 bp, synthetic construct
  source 1..28: mol_type = other DNA
gtagcatccagcagtctctgtagccagg

SEQ ID NO: 43033 - DNA, 28 bp, synthetic construct
  source 1..28: mol_type = other DNA
tgagtaacctggctacagagactgctgg

SEQ ID NO: 43034 - DNA, 28 bp, synthetic construct
  source 1..28: mol_type = other DNA
aatcaaatgtggttcttgagtaacctgg

SEQ ID NO: 43035 - DNA, 28 bp, synthetic construct
  source 1..28: mol_type = other DNA
tactcaagaaccacatttgatttcctgg

SEQ ID NO: 43036 - DNA, 28 bp, synthetic construct
  source 1..28: mol_type = other DNA
aggcaaagggccaggaaatcaaatgtgg

SEQ ID NO: 43037 - DNA, 28 bp, synthetic construct
  source 1..28: mol_type = other DNA
catttgatttcctggccctttgccttgg

SEQ ID NO: 43038 - DNA, 28 bp, synthetic construct
  source 1..28: mol_type = other DNA
tcctggccctttgccttggcagtgatgg

SEQ ID NO: 43039 - DNA, 28 bp, synthetic construct
  source 1..28: mol_type = other DNA
gccatcactgccaaggcaaagggccagg

SEQ ID NO: 43040 - DNA, 28 bp, synthetic construct
  source 1..28: mol_type = other DNA
aaaatgccatcactgccaaggcaaaggg

SEQ ID NO: 43041 - DNA, 28 bp, synthetic construct
  source 1..28: mol_type = other DNA
aaaaatgccatcactgccaaggcaaagg

SEQ ID NO: 43042 - DNA, 28 bp, synthetic construct
  source 1..28: mol_type = other DNA
tgaaataaaaatgccatcactgccaagg

SEQ ID NO: 43043 - DNA, 28 bp, synthetic construct
  source 1..28: mol_type = other DNA
aaagtcttcatttatttttataacatgg

SEQ ID NO: 43044 - DNA, 28 bp, synthetic construct
  source 1..28: mol_type = other DNA
aagtcttcatttatttttataacatggg

SEQ ID NO: 43045 - DNA, 28 bp, synthetic construct
  source 1..28: mol_type = other DNA
ttcatttatttttataacatgggttagg

SEQ ID NO: 43046 - DNA, 28 bp, synthetic construct
  source 1..28: mol_type = other DNA
tcatttatttttataacatgggttaggg

SEQ ID NO: 43047 - DNA, 28 bp, synthetic construct
  source 1..28: mol_type = other DNA
atttttataacatgggttagggagaagg

SEQ ID NO: 43048 - DNA, 28 bp, synthetic construct
  source 1..28: mol_type = other DNA
tttttataacatgggttagggagaaggg

SEQ ID NO: 43049 - DNA, 28 bp, synthetic construct
  source 1..28: mol_type = other DNA
atgggttagggagaagggccacaaatgg

SEQ ID NO: 43050 - DNA, 28 bp, synthetic construct
  source 1..28: mol_type = other DNA
ggttagggagaagggccacaaatggagg

SEQ ID NO: 43051 - DNA, 28 bp, synthetic construct
  source 1..28: mol_type = other DNA
gttagggagaagggccacaaatggaggg

SEQ ID NO: 43052 - DNA, 28 bp, synthetic construct
  source 1..28: mol_type = other DNA
cttgaaaggacaatccctccatttgtgg

SEQ ID NO: 43053 - DNA, 28 bp, synthetic construct
  source 1..28: mol_type = other DNA
tttatctgaagctgtggtgcttgaaagg

SEQ ID NO: 43054 - DNA, 28 bp, synthetic construct
  source 1..28: mol_type = other DNA
aaagtactaattttatctgaagctgtgg

SEQ ID NO: 43055 - DNA, 28 bp, synthetic construct
  source 1..28: mol_type = other DNA
tccactttaacttaaaaaattctagagg

SEQ ID NO: 43056 - DNA, 28 bp, synthetic construct
  source 1..28: mol_type = other DNA
ccactttaacttaaaaaattctagaggg

SEQ ID NO: 43057 - DNA, 28 bp, synthetic construct
  source 1..28: mol_type = other DNA
ttaaaaaattctagagggattatattgg

SEQ ID NO: 43058 - DNA, 28 bp, synthetic construct
  source 1..28: mol_type = other DNA
attatattggagactcaactgcccttgg

SEQ ID NO: 43059 - DNA, 28 bp, synthetic construct
  source 1..28: mol_type = other DNA
ctgcccttggttttagtttataaaatgg

SEQ ID NO: 43060 - DNA, 28 bp, synthetic construct
  source 1..28: mol_type = other DNA
aggccattttataaactaaaaccaaggg

SEQ ID NO: 43061 - DNA, 28 bp, synthetic construct
  source 1..28: mol_type = other DNA
taggccattttataaactaaaaccaagg

SEQ ID NO: 43062 - DNA, 28 bp, synthetic construct
  source 1..28: mol_type = other DNA
tagtttataaaatggcctagtactgtgg

SEQ ID NO: 43063 - DNA, 28 bp, synthetic construct
  source 1..28: mol_type = other DNA
tctaaaattaaaattccacagtactagg

SEQ ID NO: 43064 - DNA, 28 bp, synthetic construct
  source 1..28: mol_type = other DNA
actcacatcccatctgaaacttcccagg

SEQ ID NO: 43065 - DNA, 28 bp, synthetic construct
  source 1..28: mol_type = other DNA
ctcacatcccatctgaaacttcccaggg

SEQ ID NO: 43066 - DNA, 28 bp, synthetic construct
  source 1..28: mol_type = other DNA
tcacatcccatctgaaacttcccagggg

SEQ ID NO: 43067 - DNA, 28 bp, synthetic construct
  source 1..28: mol_type = other DNA
cccatctgaaacttcccaggggagttgg

SEQ ID NO: 43068 - DNA, 28 bp, synthetic construct
  source 1..28: mol_type = other DNA
cccaactcccctgggaagtttcagatgg

SEQ ID NO: 43069 - DNA, 28 bp, synthetic construct
  source 1..28: mol_type = other DNA
atctactaagaatcccaactcccctggg

SEQ ID NO: 43070 - DNA, 28 bp, synthetic construct
  source 1..28: mol_type = other DNA
aatctactaagaatcccaactcccctgg

SEQ ID NO: 43071 - DNA, 28 bp, synthetic construct
  source 1..28: mol_type = other DNA
aggggagttgggattcttagtagattgg

SEQ ID NO: 43072 - DNA, 28 bp, synthetic construct
  source 1..28: mol_type = other DNA
tgggattcttagtagattggtagaaagg

SEQ ID NO: 43073 - DNA, 28 bp, synthetic construct
  source 1..28: mol_type = other DNA
gggattcttagtagattggtagaaaggg

SEQ ID NO: 43074 - DNA, 28 bp, synthetic construct
  source 1..28: mol_type = other DNA
ggattcttagtagattggtagaaagggg

SEQ ID NO: 43075 - DNA, 28 bp, synthetic construct
  source 1..28: mol_type = other DNA
cattttctactgcatttcccatttttgg

SEQ ID NO: 43076 - DNA, 28 bp, synthetic construct
  source 1..28: mol_type = other DNA
acatgctgaacaagataccaaaaatggg

SEQ ID NO: 43077 - DNA, 28 bp, synthetic construct
  source 1..28: mol_type = other DNA
aacatgctgaacaagataccaaaaatgg

SEQ ID NO: 43078 - DNA, 28 bp, synthetic construct
  source 1..28: mol_type = other DNA
tcttaaagaatgttctcataaatatagg

SEQ ID NO: 43079 - DNA, 28 bp, synthetic construct
  source 1..28: mol_type = other DNA
tgataggaaggggtattctatgtggtgg

SEQ ID NO: 43080 - DNA, 28 bp, synthetic construct
  source 1..28: mol_type = other DNA
agctgataggaaggggtattctatgtgg

SEQ ID NO: 43081 - DNA, 28 bp, synthetic construct
  source 1..28: mol_type = other DNA
taaatcagagcgagctgataggaagggg

SEQ ID NO: 43082 - DNA, 28 bp, synthetic construct
  source 1..28: mol_type = other DNA
ctaaatcagagcgagctgataggaaggg

SEQ ID NO: 43083 - DNA, 28 bp, synthetic construct
  source 1..28: mol_type = other DNA
gctaaatcagagcgagctgataggaagg

SEQ ID NO: 43084 - DNA, 28 bp, synthetic construct
  source 1..28: mol_type = other DNA
taaggctaaatcagagcgagctgatagg

SEQ ID NO: 43085 - DNA, 28 bp, synthetic construct
  source 1..28: mol_type = other DNA
atctctaaaaaatttaacaaaattaagg

SEQ ID NO: 43086 - DNA, 28 bp, synthetic construct
  source 1..28: mol_type = other DNA
tttagagatgaatgaagtgctgctgtgg

SEQ ID NO: 43087 - DNA, 28 bp, synthetic construct
  source 1..28: mol_type = other DNA
ctgtatcattaaaattacatttttatgg

SEQ ID NO: 43088 - DNA, 28 bp, synthetic construct
  source 1..28: mol_type = other DNA
ccttccctcaaagaaatccaggaaaagg

SEQ ID NO: 43089 - DNA, 28 bp, synthetic construct
  source 1..28: mol_type = other DNA
tgtagaataaaaatgcaaagttcactgg

SEQ ID NO: 43090 - DNA, 28 bp, synthetic construct
  source 1..28: mol_type = other DNA
aactttgcatttttattctacatagtgg

SEQ ID NO: 43091 - DNA, 28 bp, synthetic construct
  source 1..28: mol_type = other DNA
catagtggttctccatgtttttaccagg

SEQ ID NO: 43092 - DNA, 28 bp, synthetic construct
  source 1..28: mol_type = other DNA
gttctccatgtttttaccaggaatatgg

SEQ ID NO: 43093 - DNA, 28 bp, synthetic construct
  source 1..28: mol_type = other DNA
tgctaccatattcctggtaaaaacatgg

SEQ ID NO: 43094 - DNA, 28 bp, synthetic construct
  source 1..28: mol_type = other DNA
tttaccaggaatatggtagcatcacagg

SEQ ID NO: 43095 - DNA, 28 bp, synthetic construct
  source 1..28: mol_type = other DNA
aatgcctgtgatgctaccatattcctgg

SEQ ID NO: 43096 - DNA, 28 bp, synthetic construct
  source 1..28: mol_type = other DNA
ttttttgcatagatttaaaatgaagtgg

SEQ ID NO: 43097 - DNA, 28 bp, synthetic construct
  source 1..28: mol_type = other DNA
agtggaaaaaatttcacccatcctttgg

SEQ ID NO: 43098 - DNA, 28 bp, synthetic construct
  source 1..28: mol_type = other DNA
cttctatcaaacatctccaaaggatggg

SEQ ID NO: 43099 - DNA, 28 bp, synthetic construct
  source 1..28: mol_type = other DNA
gcttctatcaaacatctccaaaggatgg

SEQ ID NO: 43100 - DNA, 28 bp, synthetic construct
  source 1..28: mol_type = other DNA
ttcagcttctatcaaacatctccaaagg

SEQ ID NO: 43101 - DNA, 28 bp, synthetic construct
  source 1..28: mol_type = other DNA
tttcacacagtactaacgaagaggtggg

SEQ ID NO: 43102 - DNA, 28 bp, synthetic construct
  source 1..28: mol_type = other DNA
atttcacacagtactaacgaagaggtgg

SEQ ID NO: 43103 - DNA, 28 bp, synthetic construct
  source 1..28: mol_type = other DNA
cctcttcgttagtactgtgtgaaattgg

SEQ ID NO: 43104 - DNA, 28 bp, synthetic construct
  source 1..28: mol_type = other DNA
tgtgaaattggctgtgatgtgctcgtgg

SEQ ID NO: 43105 - DNA, 28 bp, synthetic construct
  source 1..28: mol_type = other DNA
ttggctgtgatgtgctcgtggttgaagg

SEQ ID NO: 43106 - DNA, 28 bp, synthetic construct
  source 1..28: mol_type = other DNA
tggctgtgatgtgctcgtggttgaaggg

SEQ ID NO: 43107 - DNA, 28 bp, synthetic construct
  source 1..28: mol_type = other DNA
tgaagggtatgtagtcagcaacccctgg

SEQ ID NO: 43108 - DNA, 28 bp, synthetic construct
  source 1..28: mol_type = other DNA
catgttattctctgcttatttccagggg

SEQ ID NO: 43109 - DNA, 28 bp, synthetic construct
  source 1..28: mol_type = other DNA
tcatgttattctctgcttatttccaggg

SEQ ID NO: 43110 - DNA, 28 bp, synthetic construct
  source 1..28: mol_type = other DNA
ctcatgttattctctgcttatttccagg

SEQ ID NO: 43111 - DNA, 28 bp, synthetic construct
  source 1..28: mol_type = other DNA
ctggaaataagcagagaataacatgagg

SEQ ID NO: 43112 - DNA, 28 bp, synthetic construct
  source 1..28: mol_type = other DNA
agcagagaataacatgaggtgactgtgg

SEQ ID NO: 43113 - DNA, 28 bp, synthetic construct
  source 1..28: mol_type = other DNA
tgcatgtaaccacctccatcccccaagg

SEQ ID NO: 43114 - DNA, 28 bp, synthetic construct
  source 1..28: mol_type = other DNA
gcatgtaaccacctccatcccccaaggg

SEQ ID NO: 43115 - DNA, 28 bp, synthetic construct
  source 1..28: mol_type = other DNA
cactgcatcccttgggggatggaggtgg

SEQ ID NO: 43116 - DNA, 28 bp, synthetic construct
  source 1..28: mol_type = other DNA
gctcactgcatcccttgggggatggagg

SEQ ID NO: 43117 - DNA, 28 bp, synthetic construct
  source 1..28: mol_type = other DNA
ctagctcactgcatcccttgggggatgg

SEQ ID NO: 43118 - DNA, 28 bp, synthetic construct
  source 1..28: mol_type = other DNA
gcatctagctcactgcatcccttggggg

SEQ ID NO: 43119 - DNA, 28 bp, synthetic construct
  source 1..28: mol_type = other DNA
tgcatctagctcactgcatcccttgggg

SEQ ID NO: 43120 - DNA, 28 bp, synthetic construct
  source 1..28: mol_type = other DNA
ctgcatctagctcactgcatcccttggg

SEQ ID NO: 43121 - DNA, 28 bp, synthetic construct
  source 1..28: mol_type = other DNA
actgcatctagctcactgcatcccttgg

SEQ ID NO: 43122 - DNA, 28 bp, synthetic construct
  source 1..28: mol_type = other DNA
cagtgaacccattaaatgtttttaaagg

SEQ ID NO: 43123 - DNA, 28 bp, synthetic construct
  source 1..28: mol_type = other DNA
ttttactcctttaaaaacatttaatggg

SEQ ID NO: 43124 - DNA, 28 bp, synthetic construct
  source 1..28: mol_type = other DNA
attttactcctttaaaaacatttaatgg

SEQ ID NO: 43125 - DNA, 28 bp, synthetic construct
  source 1..28: mol_type = other DNA
attaaagaatgtagccttcagactatgg

SEQ ID NO: 43126 - DNA, 28 bp, synthetic construct
  source 1..28: mol_type = other DNA
ataggcgttatcttccatagtctgaagg

SEQ ID NO: 43127 - DNA, 28 bp, synthetic construct
  source 1..28: mol_type = other DNA
atgaaggtgagggaagaaaagacatagg

SEQ ID NO: 43128 - DNA, 28 bp, synthetic construct
  source 1..28: mol_type = other DNA
cttttcttccctcaccttcattcaaagg

SEQ ID NO: 43129 - DNA, 28 bp, synthetic construct
  source 1..28: mol_type = other DNA
gtgtaacacctttgaatgaaggtgaggg

SEQ ID NO: 43130 - DNA, 28 bp, synthetic construct
  source 1..28: mol_type = other DNA
ggtgtaacacctttgaatgaaggtgagg

SEQ ID NO: 43131 - DNA, 28 bp, synthetic construct
  source 1..28: mol_type = other DNA
ttagtggtgtaacacctttgaatgaagg

SEQ ID NO: 43132 - DNA, 28 bp, synthetic construct
  source 1..28: mol_type = other DNA
acaagacatactggcagtttcttagtgg

SEQ ID NO: 43133 - DNA, 28 bp, synthetic construct
  source 1..28: mol_type = other DNA
ggaaaatgttaatcacaagacatactgg

SEQ ID NO: 43134 - DNA, 28 bp, synthetic construct
  source 1..28: mol_type = other DNA
gtcgtctcttctatcaacaatatcgcgg

SEQ ID NO: 43135 - DNA, 28 bp, synthetic construct
  source 1..28: mol_type = other DNA
gatattgttgatagaagagacgacaagg

SEQ ID NO: 43136 - DNA, 28 bp, synthetic construct
  source 1..28: mol_type = other DNA
acgacaaggccccaagatgtcattgtgg

SEQ ID NO: 43137 - DNA, 28 bp, synthetic construct
  source 1..28: mol_type = other DNA
gatttgaaaccacaatgacatcttgggg

SEQ ID NO: 43138 - DNA, 28 bp, synthetic construct
  source 1..28: mol_type = other DNA
agatttgaaaccacaatgacatcttggg

SEQ ID NO: 43139 - DNA, 28 bp, synthetic construct
  source 1..28: mol_type = other DNA
tagatttgaaaccacaatgacatcttgg

SEQ ID NO: 43140 - DNA, 28 bp, synthetic construct
  source 1..28: mol_type = other DNA
ttatatatgattaacatctcactttagg

SEQ ID NO: 43141 - DNA, 28 bp, synthetic construct
  source 1..28: mol_type = other DNA
tatgattaacatctcactttaggtcagg

SEQ ID NO: 43142 - DNA, 28 bp, synthetic construct
  source 1..28: mol_type = other DNA
atgattaacatctcactttaggtcaggg

SEQ ID NO: 43143 - DNA, 28 bp, synthetic construct
  source 1..28: mol_type = other DNA
atctcactttaggtcagggaataagcgg

SEQ ID NO: 43144 - DNA, 28 bp, synthetic construct
  source 1..28: mol_type = other DNA
ggtcagggaataagcggtaagatgaagg

SEQ ID NO: 43145 - DNA, 28 bp, synthetic construct
  source 1..28: mol_type = other DNA
gtcagggaataagcggtaagatgaaggg

SEQ ID NO: 43146 - DNA, 28 bp, synthetic construct
  source 1..28: mol_type = other DNA
ttagttaattaattttttagagacaagg

SEQ ID NO: 43147 - DNA, 28 bp, synthetic construct
  source 1..28: mol_type = other DNA
tattaaataaaaatctgttatcaaaagg

SEQ ID NO: 43148 - DNA, 28 bp, synthetic construct
  source 1..28: mol_type = other DNA
atctgttatcaaaaggaaaaaaattagg

SEQ ID NO: 43149 - DNA, 28 bp, synthetic construct
  source 1..28: mol_type = other DNA
tcaaaaggaaaaaaattaggaaaacagg

SEQ ID NO: 43150 - DNA, 28 bp, synthetic construct
  source 1..28: mol_type = other DNA
aaggaaaaaaattaggaaaacaggatgg

SEQ ID NO: 43151 - DNA, 28 bp, synthetic construct
  source 1..28: mol_type = other DNA
ttaggaaaacaggatggataaaaaatgg

SEQ ID NO: 43152 - DNA, 28 bp, synthetic construct
  source 1..28: mol_type = other DNA
taggaaaacaggatggataaaaaatggg

SEQ ID NO: 43153 - DNA, 28 bp, synthetic construct
  source 1..28: mol_type = other DNA
tggataaaaaatgggaattcagatcagg

SEQ ID NO: 43154 - DNA, 28 bp, synthetic construct
  source 1..28: mol_type = other DNA
acaaatgtcattcatcattctctcaagg

SEQ ID NO: 43155 - DNA, 28 bp, synthetic construct
  source 1..28: mol_type = other DNA
acatttgtaatactcacttgaacatagg

SEQ ID NO: 43156 - DNA, 28 bp, synthetic construct
  source 1..28: mol_type = other DNA
aggatttttgcgctgtgcttcctctagg

SEQ ID NO: 43157 - DNA, 28 bp, synthetic construct
  source 1..28: mol_type = other DNA
gggtcagtgttacttgttgtcctagagg

SEQ ID NO: 43158 - DNA, 28 bp, synthetic construct
  source 1..28: mol_type = other DNA
gacccacttttcacactaacattgatgg

SEQ ID NO: 43159 - DNA, 28 bp, synthetic construct
  source 1..28: mol_type = other DNA
gaccatcaatgttagtgtgaaaagtggg

SEQ ID NO: 43160 - DNA, 28 bp, synthetic construct
  source 1..28: mol_type = other DNA
agaccatcaatgttagtgtgaaaagtgg

SEQ ID NO: 43161 - DNA, 28 bp, synthetic construct
  source 1..28: mol_type = other DNA
gaagagcagctcaacccccctcagctgg

SEQ ID NO: 43162 - DNA, 28 bp, synthetic construct
  source 1..28: mol_type = other DNA
tcaacccccctcagctggttatttatgg

SEQ ID NO: 43163 - DNA, 28 bp, synthetic construct
  source 1..28: mol_type = other DNA
tacaccataaataaccagctgagggggg

SEQ ID NO: 43164 - DNA, 28 bp, synthetic construct
  source 1..28: mol_type = other DNA
atacaccataaataaccagctgaggggg

SEQ ID NO: 43165 - DNA, 28 bp, synthetic construct
  source 1..28: mol_type = other DNA
tatacaccataaataaccagctgagggg

SEQ ID NO: 43166 - DNA, 28 bp, synthetic construct
  source 1..28: mol_type = other DNA
atatacaccataaataaccagctgaggg

SEQ ID NO: 43167 - DNA, 28 bp, synthetic construct
  source 1..28: mol_type = other DNA
catatacaccataaataaccagctgagg

SEQ ID NO: 43168 - DNA, 28 bp, synthetic construct
  source 1..28: mol_type = other DNA
tatatgacagtgatgttagatgcagagg

SEQ ID NO: 43169 - DNA, 28 bp, synthetic construct
  source 1..28: mol_type = other DNA
atgacagtgatgttagatgcagaggtgg

SEQ ID NO: 43170 - DNA, 28 bp, synthetic construct
  source 1..28: mol_type = other DNA
tgacagtgatgttagatgcagaggtggg

SEQ ID NO: 43171 - DNA, 28 bp, synthetic construct
  source 1..28: mol_type = other DNA
gacagtgatgttagatgcagaggtgggg

SEQ ID NO: 43172 - DNA, 28 bp, synthetic construct
  source 1..28: mol_type = other DNA
tgatgttagatgcagaggtggggccagg

SEQ ID NO: 43173 - DNA, 28 bp, synthetic construct
  source 1..28: mol_type = other DNA
gatgttagatgcagaggtggggccaggg

SEQ ID NO: 43174 - DNA, 28 bp, synthetic construct
  source 1..28: mol_type = other DNA
tagatgcagaggtggggccagggccagg

SEQ ID NO: 43175 - DNA, 28 bp, synthetic construct
  source 1..28: mol_type = other DNA
agatgcagaggtggggccagggccaggg

SEQ ID NO: 43176 - DNA, 28 bp, synthetic construct
  source 1..28: mol_type = other DNA
gaggtggggccagggccagggttgctgg

SEQ ID NO: 43177 - DNA, 28 bp, synthetic construct
  source 1..28: mol_type = other DNA
aggtggggccagggccagggttgctggg

SEQ ID NO: 43178 - DNA, 28 bp, synthetic construct
  source 1..28: mol_type = other DNA
caactctacccagcaaccctggccctgg

SEQ ID NO: 43179 - DNA, 28 bp, synthetic construct
  source 1..28: mol_type = other DNA
cagggccagggttgctgggtagagttgg

SEQ ID NO: 43180 - DNA, 28 bp, synthetic construct
  source 1..28: mol_type = other DNA
tacaaccaactctacccagcaaccctgg

SEQ ID NO: 43181 - DNA, 28 bp, synthetic construct
  source 1..28: mol_type = other DNA
gttggttgtacctcatgatctgtgaagg

SEQ ID NO: 43182 - DNA, 28 bp, synthetic construct
  source 1..28: mol_type = other DNA
ttggttgtacctcatgatctgtgaaggg

SEQ ID NO: 43183 - DNA, 28 bp, synthetic construct
  source 1..28: mol_type = other DNA
acctcatgatctgtgaagggcaaagagg

SEQ ID NO: 43184 - DNA, 28 bp, synthetic construct
  source 1..28: mol_type = other DNA
gcctctttgcccttcacagatcatgagg

SEQ ID NO: 43185 - DNA, 28 bp, synthetic construct
  source 1..28: mol_type = other DNA
aagaggccacatttgtcaaagattatgg

SEQ ID NO: 43186 - DNA, 28 bp, synthetic construct
  source 1..28: mol_type = other DNA
agaggccacatttgtcaaagattatggg

SEQ ID NO: 43187 - DNA, 28 bp, synthetic construct
  source 1..28: mol_type = other DNA
gaggccacatttgtcaaagattatgggg

SEQ ID NO: 43188 - DNA, 28 bp, synthetic construct
  source 1..28: mol_type = other DNA
caaaccccataatctttgacaaatgtgg

SEQ ID NO: 43189 - DNA, 28 bp, synthetic construct
  source 1..28: mol_type = other DNA
tcaaagattatggggtttgtatcatagg

SEQ ID NO: 43190 - DNA, 28 bp, synthetic construct
  source 1..28: mol_type = other DNA
atcataggtgcaaaatctctgttattgg

SEQ ID NO: 43191 - DNA, 28 bp, synthetic construct
  source 1..28: mol_type = other DNA
cactactttctcaaaatgtcttctgggg

SEQ ID NO: 43192 - DNA, 28 bp, synthetic construct
  source 1..28: mol_type = other DNA
tcactactttctcaaaatgtcttctggg

SEQ ID NO: 43193 - DNA, 28 bp, synthetic construct
  source 1..28: mol_type = other DNA
ctcactactttctcaaaatgtcttctgg

SEQ ID NO: 43194 - DNA, 28 bp, synthetic construct
  source 1..28: mol_type = other DNA
atgtactctgcccacatgggaataatgg

SEQ ID NO: 43195 - DNA, 28 bp, synthetic construct
  source 1..28: mol_type = other DNA
cttgtaatgtccattattcccatgtggg

SEQ ID NO: 43196 - DNA, 28 bp, synthetic construct
  source 1..28: mol_type = other DNA
gcttgtaatgtccattattcccatgtgg

SEQ ID NO: 43197 - DNA, 28 bp, synthetic construct
  source 1..28: mol_type = other DNA
tgtggatcaatgttaagtggcatatagg

SEQ ID NO: 43198 - DNA, 28 bp, synthetic construct
  source 1..28: mol_type = other DNA
aaatgacatgtggatcaatgttaagtgg

SEQ ID NO: 43199 - DNA, 28 bp, synthetic construct
  source 1..28: mol_type = other DNA
ttaacattgatccacatgtcatttctgg

SEQ ID NO: 43200 - DNA, 28 bp, synthetic construct
  source 1..28: mol_type = other DNA
agcaacttatgccagaaatgacatgtgg

SEQ ID NO: 43201 - DNA, 28 bp, synthetic construct
  source 1..28: mol_type = other DNA
gcataagttgctgctttatgacataagg

SEQ ID NO: 43202 - DNA, 28 bp, synthetic construct
  source 1..28: mol_type = other DNA
agttgctgctttatgacataaggagagg

SEQ ID NO: 43203 - DNA, 28 bp, synthetic construct
  source 1..28: mol_type = other DNA
tgctgctttatgacataaggagaggtgg

SEQ ID NO: 43204 - DNA, 28 bp, synthetic construct
  source 1..28: mol_type = other DNA
cataaggagaggtggatgtcttaccagg

SEQ ID NO: 43205 - DNA, 28 bp, synthetic construct
  source 1..28: mol_type = other DNA
tgtcttaccaggactacaagtgacctgg

SEQ ID NO: 43206 - DNA, 28 bp, synthetic construct
  source 1..28: mol_type = other DNA
gtcttaccaggactacaagtgacctggg

SEQ ID NO: 43207 - DNA, 28 bp, synthetic construct
  source 1..28: mol_type = other DNA
tcttaccaggactacaagtgacctgggg

SEQ ID NO: 43208 - DNA, 28 bp, synthetic construct
  source 1..28: mol_type = other DNA
atgtgccccaggtcacttgtagtcctgg

SEQ ID NO: 43209 - DNA, 28 bp, synthetic construct
  source 1..28: mol_type = other DNA
actacaagtgacctggggcacatctagg

SEQ ID NO: 43210 - DNA, 28 bp, synthetic construct
  source 1..28: mol_type = other DNA
ggcaagacatacctagatgtgccccagg

SEQ ID NO: 43211 - DNA, 28 bp, synthetic construct
  source 1..28: mol_type = other DNA
cacatctaggtatgtcttgcctttcagg

SEQ ID NO: 43212 - DNA, 28 bp, synthetic construct
  source 1..28: mol_type = other DNA
acatctaggtatgtcttgcctttcaggg

SEQ ID NO: 43213 - DNA, 28 bp, synthetic construct
  source 1..28: mol_type = other DNA
ctaggtatgtcttgcctttcagggaagg

SEQ ID NO: 43214 - DNA, 28 bp, synthetic construct
  source 1..28: mol_type = other DNA
taggtatgtcttgcctttcagggaaggg

SEQ ID NO: 43215 - DNA, 28 bp, synthetic construct
  source 1..28: mol_type = other DNA
gtatgtcttgcctttcagggaagggagg

SEQ ID NO: 43216 - DNA, 28 bp, synthetic construct
  source 1..28: mol_type = other DNA
ttgctcaaatcctcccttccctgaaagg

SEQ ID NO: 43217 - DNA, 28 bp, synthetic construct
  source 1..28: mol_type = other DNA
ttcagggaagggaggatttgagcaatgg

SEQ ID NO: 43218 - DNA, 28 bp, synthetic construct
  source 1..28: mol_type = other DNA
gaagggaggatttgagcaatggacatgg

SEQ ID NO: 43219 - DNA, 28 bp, synthetic construct
  source 1..28: mol_type = other DNA
aagggaggatttgagcaatggacatggg

SEQ ID NO: 43220 - DNA, 28 bp, synthetic construct
  source 1..28: mol_type = other DNA
agggaggatttgagcaatggacatgggg

SEQ ID NO: 43221 - DNA, 28 bp, synthetic construct
  source 1..28: mol_type = other DNA
gatttgagcaatggacatggggttgtgg

SEQ ID NO: 43222 - DNA, 28 bp, synthetic construct
  source 1..28: mol_type = other DNA
tatgatactcaatgagattaagcagggg

SEQ ID NO: 43223 - DNA, 28 bp, synthetic construct
  source 1..28: mol_type = other DNA
atatgatactcaatgagattaagcaggg

SEQ ID NO: 43224 - DNA, 28 bp, synthetic construct
  source 1..28: mol_type = other DNA
gatatgatactcaatgagattaagcagg

SEQ ID NO: 43225 - DNA, 28 bp, synthetic construct
  source 1..28: mol_type = other DNA
aaggaatggaactgcaagaagactacgg

SEQ ID NO: 43226 - DNA, 28 bp, synthetic construct
  source 1..28: mol_type = other DNA
tcttgcagttccattcctttttagatgg

SEQ ID NO: 43227 - DNA, 28 bp, synthetic construct
  source 1..28: mol_type = other DNA
agttccattcctttttagatggctcagg

SEQ ID NO: 43228 - DNA, 28 bp, synthetic construct
  source 1..28: mol_type = other DNA
aacacctgagccatctaaaaaggaatgg

SEQ ID NO: 43229 - DNA, 28 bp, synthetic construct
  source 1..28: mol_type = other DNA
tctgtaacacctgagccatctaaaaagg

SEQ ID NO: 43230 - DNA, 28 bp, synthetic construct
  source 1..28: mol_type = other DNA
tggctcaggtgttacagagagagcctgg

SEQ ID NO: 43231 - DNA, 28 bp, synthetic construct
  source 1..28: mol_type = other DNA
ggctcaggtgttacagagagagcctggg

SEQ ID NO: 43232 - DNA, 28 bp, synthetic construct
  source 1..28: mol_type = other DNA
caggtgttacagagagagcctgggaagg

SEQ ID NO: 43233 - DNA, 28 bp, synthetic construct
  source 1..28: mol_type = other DNA
tctctctctttctgtcttccttcccagg

SEQ ID NO: 43234 - DNA, 28 bp, synthetic construct
  source 1..28: mol_type = other DNA
acagaaagagagagaaagagtaattagg

SEQ ID NO: 43235 - DNA, 28 bp, synthetic construct
  source 1..28: mol_type = other DNA
agagtaattaggcatagctgagagttgg

SEQ ID NO: 43236 - DNA, 28 bp, synthetic construct
  source 1..28: mol_type = other DNA
aagagataaacttgatcactaatcatgg

SEQ ID NO: 43237 - DNA, 28 bp, synthetic construct
  source 1..28: mol_type = other DNA
agaatatatctcaggtcatactagctgg

SEQ ID NO: 43238 - DNA, 28 bp, synthetic construct
  source 1..28: mol_type = other DNA
tttcacagagatgttagtagaagcctgg

SEQ ID NO: 43239 - DNA, 28 bp, synthetic construct
  source 1..28: mol_type = other DNA
gcctggcctcttgattctgcaatccagg

SEQ ID NO: 43240 - DNA, 28 bp, synthetic construct
  source 1..28: mol_type = other DNA
gcctggattgcagaatcaagaggccagg

SEQ ID NO: 43241 - DNA, 28 bp, synthetic construct
  source 1..28: mol_type = other DNA
aataagcctggattgcagaatcaagagg

SEQ ID NO: 43242 - DNA, 28 bp, synthetic construct
  source 1..28: mol_type = other DNA
tcttgattctgcaatccaggcttattgg

SEQ ID NO: 43243 - DNA, 28 bp, synthetic construct
  source 1..28: mol_type = other DNA
gattctgcaatccaggcttattggcagg

SEQ ID NO: 43244 - DNA, 28 bp, synthetic construct
  source 1..28: mol_type = other DNA
ttggttgggttcctgccaataagcctgg

SEQ ID NO: 43245 - DNA, 28 bp, synthetic construct
  source 1..28: mol_type = other DNA
aaacacgtgctggatgctcttggttggg

SEQ ID NO: 43246 - DNA, 28 bp, synthetic construct
  source 1..28: mol_type = other DNA
taaacacgtgctggatgctcttggttgg

SEQ ID NO: 43247 - DNA, 28 bp, synthetic construct
  source 1..28: mol_type = other DNA
caggtaaacacgtgctggatgctcttgg

SEQ ID NO: 43248 - DNA, 28 bp, synthetic construct
  source 1..28: mol_type = other DNA
agcatccagcacgtgtttacctgcatgg

SEQ ID NO: 43249 - DNA, 28 bp, synthetic construct
  source 1..28: mol_type = other DNA
ccagcacgtgtttacctgcatggcgagg

SEQ ID NO: 43250 - DNA, 28 bp, synthetic construct
  source 1..28: mol_type = other DNA
atctacagtactggcctcgccatgcagg

SEQ ID NO: 43251 - DNA, 28 bp, synthetic construct
  source 1..28: mol_type = other DNA
gcatcattggagacatctacagtactgg

SEQ ID NO: 43252 - DNA, 28 bp, synthetic construct
  source 1..28: mol_type = other DNA
tgaagatcaaagataatggcatcattgg

SEQ ID NO: 43253 - DNA, 28 bp, synthetic construct
  source 1..28: mol_type = other DNA
aaatcagcatgaagatcaaagataatgg

SEQ ID NO: 43254 - DNA, 28 bp, synthetic construct
  source 1..28: mol_type = other DNA
tttggtcaggtactaaaggatattgtgg

SEQ ID NO: 43255 - DNA, 28 bp, synthetic construct
  source 1..28: mol_type = other DNA
aatatcctttagtacctgaccaaacagg

SEQ ID NO: 43256 - DNA, 28 bp, synthetic construct
  source 1..28: mol_type = other DNA
atatcctttagtacctgaccaaacaggg

SEQ ID NO: 43257 - DNA, 28 bp, synthetic construct
  source 1..28: mol_type = other DNA
agatccctgtttggtcaggtactaaagg

SEQ ID NO: 43258 - DNA, 28 bp, synthetic construct
  source 1..28: mol_type = other DNA
gaaggttacagatccctgtttggtcagg

SEQ ID NO: 43259 - DNA, 28 bp, synthetic construct
  source 1..28: mol_type = other DNA
cagaggaaggttacagatccctgtttgg

SEQ ID NO: 43260 - DNA, 28 bp, synthetic construct
  source 1..28: mol_type = other DNA
atctgtaaccttcctctgaacctacagg

SEQ ID NO: 43261 - DNA, 28 bp, synthetic construct
  source 1..28: mol_type = other DNA
tctgtaaccttcctctgaacctacaggg

SEQ ID NO: 43262 - DNA, 28 bp, synthetic construct
  source 1..28: mol_type = other DNA
acaagatccctgtaggttcagaggaagg

SEQ ID NO: 43263 - DNA, 28 bp, synthetic construct
  source 1..28: mol_type = other DNA
tacaacaagatccctgtaggttcagagg

SEQ ID NO: 43264 - DNA, 28 bp, synthetic construct
  source 1..28: mol_type = other DNA
cctgtatgtacaacaagatccctgtagg

SEQ ID NO: 43265 - DNA, 28 bp, synthetic construct
  source 1..28: mol_type = other DNA
ttgttgtacatacaggtcagagccaagg

SEQ ID NO: 43266 - DNA, 28 bp, synthetic construct
  source 1..28: mol_type = other DNA
acagacacaggagcaatggcaaccttgg

SEQ ID NO: 43267 - DNA, 28 bp, synthetic construct
  source 1..28: mol_type = other DNA
ctgtcattcacagacacaggagcaatgg

SEQ ID NO: 43268 - DNA, 28 bp, synthetic construct
  source 1..28: mol_type = other DNA
ttgctcctgtgtctgtgaatgacagagg

SEQ ID NO: 43269 - DNA, 28 bp, synthetic construct
  source 1..28: mol_type = other DNA
tgctcctgtgtctgtgaatgacagaggg

SEQ ID NO: 43270 - DNA, 28 bp, synthetic construct
  source 1..28: mol_type = other DNA
tataccctctgtcattcacagacacagg

SEQ ID NO: 43271 - DNA, 28 bp, synthetic construct
  source 1..28: mol_type = other DNA
gttcatattgctgtgatggtgactatgg

SEQ ID NO: 43272 - DNA, 28 bp, synthetic construct
  source 1..28: mol_type = other DNA
atgttagctgttcatattgctgtgatgg

SEQ ID NO: 43273 - DNA, 28 bp, synthetic construct
  source 1..28: mol_type = other DNA
catttattgtgtgcttattatattctgg

SEQ ID NO: 43274 - DNA, 28 bp, synthetic construct
  source 1..28: mol_type = other DNA
ttgttctgaggagcaaataaaatcatgg

SEQ ID NO: 43275 - DNA, 28 bp, synthetic construct
  source 1..28: mol_type = other DNA
gttcacatccttagctcctcctccatgg

SEQ ID NO: 43276 - DNA, 28 bp, synthetic construct
  source 1..28: mol_type = other DNA
ttcacatccttagctcctcctccatggg

SEQ ID NO: 43277 - DNA, 28 bp, synthetic construct
  source 1..28: mol_type = other DNA
agagcgtcccatggaggaggagctaagg

SEQ ID NO: 43278 - DNA, 28 bp, synthetic construct
  source 1..28: mol_type = other DNA
gacaaaggagagcgtcccatggaggagg

SEQ ID NO: 43279 - DNA, 28 bp, synthetic construct
  source 1..28: mol_type = other DNA
agtgacaaaggagagcgtcccatggagg

SEQ ID NO: 43280 - DNA, 28 bp, synthetic construct
  source 1..28: mol_type = other DNA
ggaagtgacaaaggagagcgtcccatgg

SEQ ID NO: 43281 - DNA, 28 bp, synthetic construct
  source 1..28: mol_type = other DNA
ggtggagctggcagggaagtgacaaagg

SEQ ID NO: 43282 - DNA, 28 bp, synthetic construct
  source 1..28: mol_type = other DNA
cgtgaactgaatggtggagctggcaggg

SEQ ID NO: 43283 - DNA, 28 bp, synthetic construct
  source 1..28: mol_type = other DNA
tcgtgaactgaatggtggagctggcagg

SEQ ID NO: 43284 - DNA, 28 bp, synthetic construct
  source 1..28: mol_type = other DNA
ggcatcgtgaactgaatggtggagctgg

SEQ ID NO: 43285 - DNA, 28 bp, synthetic construct
  source 1..28: mol_type = other DNA
atcagaggcatcgtgaactgaatggtgg

SEQ ID NO: 43286 - DNA, 28 bp, synthetic construct
  source 1..28: mol_type = other DNA
aacatcagaggcatcgtgaactgaatgg

SEQ ID NO: 43287 - DNA, 28 bp, synthetic construct
  source 1..28: mol_type = other DNA
cacgatgcctctgatgttcccagctcgg

SEQ ID NO: 43288 - DNA, 28 bp, synthetic construct
  source 1..28: mol_type = other DNA
acgatgcctctgatgttcccagctcggg

SEQ ID NO: 43289 - DNA, 28 bp, synthetic construct
  source 1..28: mol_type = other DNA
cgatgcctctgatgttcccagctcgggg

SEQ ID NO: 43290 - DNA, 28 bp, synthetic construct
  source 1..28: mol_type = other DNA
cactaccccgagctgggaacatcagagg

SEQ ID NO: 43291 - DNA, 28 bp, synthetic construct
  source 1..28: mol_type = other DNA
ctctgatgttcccagctcggggtagtgg

SEQ ID NO: 43292 - DNA, 28 bp, synthetic construct
  source 1..28: mol_type = other DNA
gagtaggtcaccactaccccgagctggg

SEQ ID NO: 43293 - DNA, 28 bp, synthetic construct
  source 1..28: mol_type = other DNA
tgagtaggtcaccactaccccgagctgg

SEQ ID NO: 43294 - DNA, 28 bp, synthetic construct
  source 1..28: mol_type = other DNA
gtggtgacctactcacctacattgaagg

SEQ ID NO: 43295 - DNA, 28 bp, synthetic construct
  source 1..28: mol_type = other DNA
tggtgacctactcacctacattgaaggg

SEQ ID NO: 43296 - DNA, 28 bp, synthetic construct
  source 1..28: mol_type = other DNA
acctactcacctacattgaagggagagg

SEQ ID NO: 43297 - DNA, 28 bp, synthetic construct
  source 1..28: mol_type = other DNA
tcctctcccttcaatgtaggtgagtagg

SEQ ID NO: 43298 - DNA, 28 bp, synthetic construct
  source 1..28: mol_type = other DNA
tcacctacattgaagggagaggagttgg

SEQ ID NO: 43299 - DNA, 28 bp, synthetic construct
  source 1..28: mol_type = other DNA
tggccaactcctctcccttcaatgtagg

SEQ ID NO: 43300 - DNA, 28 bp, synthetic construct
  source 1..28: mol_type = other DNA
attgaagggagaggagttggccagcagg

SEQ ID NO: 43301 - DNA, 28 bp, synthetic construct
  source 1..28: mol_type = other DNA
ttgaagggagaggagttggccagcaggg

SEQ ID NO: 43302 - DNA, 28 bp, synthetic construct
  source 1..28: mol_type = other DNA
ggagaggagttggccagcagggtcttgg

SEQ ID NO: 43303 - DNA, 28 bp, synthetic construct
  source 1..28: mol_type = other DNA
gttggccagcagggtcttggcaaagcgg

SEQ ID NO: 43304 - DNA, 28 bp, synthetic construct
  source 1..28: mol_type = other DNA
gccagcagggtcttggcaaagcggacgg

SEQ ID NO: 43305 - DNA, 28 bp, synthetic construct
  source 1..28: mol_type = other DNA
gccgtccgctttgccaagaccctgctgg

SEQ ID NO: 43306 - DNA, 28 bp, synthetic construct
  source 1..28: mol_type = other DNA
gggtcttggcaaagcggacggctatcgg

SEQ ID NO: 43307 - DNA, 28 bp, synthetic construct
  source 1..28: mol_type = other DNA
ttggcaaagcggacggctatcggcaagg

SEQ ID NO: 43308 - DNA, 28 bp, synthetic construct
  source 1..28: mol_type = other DNA
cggcaaggtcgcctcagagttcttctgg

SEQ ID NO: 43309 - DNA, 28 bp, synthetic construct
  source 1..28: mol_type = other DNA
ttggcactgtgccagaagaactctgagg

SEQ ID NO: 43310 - DNA, 28 bp, synthetic construct
  source 1..28: mol_type = other DNA
tggcacagtgccaagatcgctagactgg

SEQ ID NO: 43311 - DNA, 28 bp, synthetic construct
  source 1..28: mol_type = other DNA
ggcacagtgccaagatcgctagactggg

SEQ ID NO: 43312 - DNA, 28 bp, synthetic construct
  source 1..28: mol_type = other DNA
ttctatgggcccagtctagcgatcttgg

SEQ ID NO: 43313 - DNA, 28 bp, synthetic construct
  source 1..28: mol_type = other DNA
aagatcgctagactgggcccatagaagg

SEQ ID NO: 43314 - DNA, 28 bp, synthetic construct
  source 1..28: mol_type = other DNA
caacgctgaagcatcagccttctatggg

SEQ ID NO: 43315 - DNA, 28 bp, synthetic construct
  source 1..28: mol_type = other DNA
ccaacgctgaagcatcagccttctatgg

SEQ ID NO: 43316 - DNA, 28 bp, synthetic construct
  source 1..28: mol_type = other DNA
catagaaggctgatgcttcagcgttggg

SEQ ID NO: 43317 - DNA, 28 bp, synthetic construct
  source 1..28: mol_type = other DNA
atagaaggctgatgcttcagcgttgggg

SEQ ID NO: 43318 - DNA, 28 bp, synthetic construct
  source 1..28: mol_type = other DNA
gatgcttcagcgttggggcctccgaagg

SEQ ID NO: 43319 - DNA, 28 bp, synthetic construct
  source 1..28: mol_type = other DNA
atgcttcagcgttggggcctccgaaggg

SEQ ID NO: 43320 - DNA, 28 bp, synthetic construct
  source 1..28: mol_type = other DNA
tgcttcagcgttggggcctccgaagggg

SEQ ID NO: 43321 - DNA, 28 bp, synthetic construct
  source 1..28: mol_type = other DNA
gatgaaggttctctatccccttcggagg

SEQ ID NO: 43322 - DNA, 28 bp, synthetic construct
  source 1..28: mol_type = other DNA
tctgatgaaggttctctatccccttcgg

SEQ ID NO: 43323 - DNA, 28 bp, synthetic construct
  source 1..28: mol_type = other DNA
atcgtggtgactgtgagtctgatgaagg

SEQ ID NO: 43324 - DNA, 28 bp, synthetic construct
  source 1..28: mol_type = other DNA
catcagactcacagtcaccacgatgagg

SEQ ID NO: 43325 - DNA, 28 bp, synthetic construct
  source 1..28: mol_type = other DNA
accacgatgaggacatttgcaaagaagg

SEQ ID NO: 43326 - DNA, 28 bp, synthetic construct
  source 1..28: mol_type = other DNA
tccttctttgcaaatgtcctcatcgtgg

SEQ ID NO: 43327 - DNA, 28 bp, synthetic construct
  source 1..28: mol_type = other DNA
agaaggaaaagccaagcctttgaaaagg

SEQ ID NO: 43328 - DNA, 28 bp, synthetic construct
  source 1..28: mol_type = other DNA
tctagcaatttccttttcaaaggcttgg

SEQ ID NO: 43329 - DNA, 28 bp, synthetic construct
  source 1..28: mol_type = other DNA
ggttttctagcaatttccttttcaaagg

SEQ ID NO: 43330 - DNA, 28 bp, synthetic construct
  source 1..28: mol_type = other DNA
tgggggtggagagaaaggcaagttaggg

SEQ ID NO: 43331 - DNA, 28 bp, synthetic construct
  source 1..28: mol_type = other DNA
gtgggggtggagagaaaggcaagttagg

SEQ ID NO: 43332 - DNA, 28 bp, synthetic construct
  source 1..28: mol_type = other DNA
aggaaaagggtgggggtggagagaaagg

SEQ ID NO: 43333 - DNA, 28 bp, synthetic construct
  source 1..28: mol_type = other DNA
tctccacccccacccttttcctttctgg

SEQ ID NO: 43334 - DNA, 28 bp, synthetic construct
  source 1..28: mol_type = other DNA
ctccacccccacccttttcctttctggg

SEQ ID NO: 43335 - DNA, 28 bp, synthetic construct
  source 1..28: mol_type = other DNA
aacccagaaaggaaaagggtgggggtgg

SEQ ID NO: 43336 - DNA, 28 bp, synthetic construct
  source 1..28: mol_type = other DNA
ttaaacccagaaaggaaaagggtggggg

SEQ ID NO: 43337 - DNA, 28 bp, synthetic construct
  source 1..28: mol_type = other DNA
tttaaacccagaaaggaaaagggtgggg

SEQ ID NO: 43338 - DNA, 28 bp, synthetic construct
  source 1..28: mol_type = other DNA
ttttaaacccagaaaggaaaagggtggg

SEQ ID NO: 43339 - DNA, 28 bp, synthetic construct
  source 1..28: mol_type = other DNA
attttaaacccagaaaggaaaagggtgg

SEQ ID NO: 43340 - DNA, 28 bp, synthetic construct
  source 1..28: mol_type = other DNA
agaattttaaacccagaaaggaaaaggg

SEQ ID NO: 43341 - DNA, 28 bp, synthetic construct
  source 1..28: mol_type = other DNA
aagaattttaaacccagaaaggaaaagg

SEQ ID NO: 43342 - DNA, 28 bp, synthetic construct
  source 1..28: mol_type = other DNA
tttcctttctgggtttaaaattcttagg

SEQ ID NO: 43343 - DNA, 28 bp, synthetic construct
  source 1..28: mol_type = other DNA
ttacctaagaattttaaacccagaaagg

SEQ ID NO: 43344 - DNA, 28 bp, synthetic construct
  source 1..28: mol_type = other DNA
ggaagggagaaaagagtcaggcatatgg

SEQ ID NO: 43345 - DNA, 28 bp, synthetic construct
  source 1..28: mol_type = other DNA
cctgactggaagggagaaaagagtcagg

SEQ ID NO: 43346 - DNA, 28 bp, synthetic construct
  source 1..28: mol_type = other DNA
tttctcccttccagtcaggtcttactgg

SEQ ID NO: 43347 - DNA, 28 bp, synthetic construct
  source 1..28: mol_type = other DNA
tcccttccagtcaggtcttactggaagg

SEQ ID NO: 43348 - DNA, 28 bp, synthetic construct
  source 1..28: mol_type = other DNA
accttccagtaagacctgactggaaggg

SEQ ID NO: 43349 - DNA, 28 bp, synthetic construct
  source 1..28: mol_type = other DNA
caccttccagtaagacctgactggaagg

SEQ ID NO: 43350 - DNA, 28 bp, synthetic construct
  source 1..28: mol_type = other DNA
tgggcaccttccagtaagacctgactgg

SEQ ID NO: 43351 - DNA, 28 bp, synthetic construct
  source 1..28: mol_type = other DNA
attctacaaagacaaatggagaactggg

SEQ ID NO: 43352 - DNA, 28 bp, synthetic construct
  source 1..28: mol_type = other DNA
cattctacaaagacaaatggagaactgg

SEQ ID NO: 43353 - DNA, 28 bp, synthetic construct
  source 1..28: mol_type = other DNA
cagttctccatttgtctttgtagaatgg

SEQ ID NO: 43354 - DNA, 28 bp, synthetic construct
  source 1..28: mol_type = other DNA
aaagtatccattctacaaagacaaatgg

SEQ ID NO: 43355 - DNA, 28 bp, synthetic construct
  source 1..28: mol_type = other DNA
tttgtagaatggatactttatccccagg

SEQ ID NO: 43356 - DNA, 28 bp, synthetic construct
  source 1..28: mol_type = other DNA
ttgtagaatggatactttatccccaggg

SEQ ID NO: 43357 - DNA, 28 bp, synthetic construct
  source 1..28: mol_type = other DNA
aatggatactttatccccagggtctcgg

SEQ ID NO: 43358 - DNA, 28 bp, synthetic construct
  source 1..28: mol_type = other DNA
gatactttatccccagggtctcggcagg

SEQ ID NO: 43359 - DNA, 28 bp, synthetic construct
  source 1..28: mol_type = other DNA
actttatccccagggtctcggcaggagg

SEQ ID NO: 43360 - DNA, 28 bp, synthetic construct
  source 1..28: mol_type = other DNA
ttatccccagggtctcggcaggaggagg

SEQ ID NO: 43361 - DNA, 28 bp, synthetic construct
  source 1..28: mol_type = other DNA
ctcacctcctcctgccgagaccctgggg

SEQ ID NO: 43362 - DNA, 28 bp, synthetic construct
  source 1..28: mol_type = other DNA
cctcacctcctcctgccgagaccctggg

SEQ ID NO: 43363 - DNA, 28 bp, synthetic construct
  source 1..28: mol_type = other DNA
ccagggtctcggcaggaggaggtgaggg

SEQ ID NO: 43364 - DNA, 28 bp, synthetic construct
  source 1..28: mol_type = other DNA
cggcaggaggaggtgagggccatgatgg

SEQ ID NO: 43365 - DNA, 28 bp, synthetic construct
  source 1..28: mol_type = other DNA
ggaggaggtgagggccatgatggtgagg

SEQ ID NO: 43366 - DNA, 28 bp, synthetic construct
  source 1..28: mol_type = other DNA
attgggcagctcggcctcaccatcatgg

SEQ ID NO: 43367 - DNA, 28 bp, synthetic construct
  source 1..28: mol_type = other DNA
atgatggtgaggccgagctgcccaatgg

SEQ ID NO: 43368 - DNA, 28 bp, synthetic construct
  source 1..28: mol_type = other DNA
ctgcagatctaaccattgggcagctcgg

SEQ ID NO: 43369 - DNA, 28 bp, synthetic construct
  source 1..28: mol_type = other DNA
tctcttctctgcagatctaaccattggg

SEQ ID NO: 43370 - DNA, 28 bp, synthetic construct
  source 1..28: mol_type = other DNA
ttctcttctctgcagatctaaccattgg

SEQ ID NO: 43371 - DNA, 28 bp, synthetic construct
  source 1..28: mol_type = other DNA
tagatctgcagagaagagaacacaacgg

SEQ ID NO: 43372 - DNA, 28 bp, synthetic construct
  source 1..28: mol_type = other DNA
acaacggttagacagagacatcctcagg

SEQ ID NO: 43373 - DNA, 28 bp, synthetic construct
  source 1..28: mol_type = other DNA
caacggttagacagagacatcctcaggg

SEQ ID NO: 43374 - DNA, 28 bp, synthetic construct
  source 1..28: mol_type = other DNA
aacggttagacagagacatcctcagggg

SEQ ID NO: 43375 - DNA, 28 bp, synthetic construct
  source 1..28: mol_type = other DNA
agacatcctcaggggacagctctccagg

SEQ ID NO: 43376 - DNA, 28 bp, synthetic construct
  source 1..28: mol_type = other DNA
ctggctcctggagagctgtcccctgagg

SEQ ID NO: 43377 - DNA, 28 bp, synthetic construct
  source 1..28: mol_type = other DNA
aagcagagaactcatcactggctcctgg

SEQ ID NO: 43378 - DNA, 28 bp, synthetic construct
  source 1..28: mol_type = other DNA
agataaaaagcagagaactcatcactgg

SEQ ID NO: 43379 - DNA, 28 bp, synthetic construct
  source 1..28: mol_type = other DNA
gtttgggtagtttatttacagtcagagg

SEQ ID NO: 43380 - DNA, 28 bp, synthetic construct
  source 1..28: mol_type = other DNA
gtttatttacagtcagaggcagcattgg

SEQ ID NO: 43381 - DNA, 28 bp, synthetic construct
  source 1..28: mol_type = other DNA
tttatttacagtcagaggcagcattggg

SEQ ID NO: 43382 - DNA, 28 bp, synthetic construct
  source 1..28: mol_type = other DNA
ttatttacagtcagaggcagcattgggg

SEQ ID NO: 43383 - DNA, 28 bp, synthetic construct
  source 1..28: mol_type = other DNA
tttacagtcagaggcagcattggggtgg

SEQ ID NO: 43384 - DNA, 28 bp, synthetic construct
  source 1..28: mol_type = other DNA
ttacagtcagaggcagcattggggtggg

SEQ ID NO: 43385 - DNA, 28 bp, synthetic construct
  source 1..28: mol_type = other DNA
agtcagaggcagcattggggtgggaagg

SEQ ID NO: 43386 - DNA, 28 bp, synthetic construct
  source 1..28: mol_type = other DNA
cattggggtgggaaggacgctgagttgg

SEQ ID NO: 43387 - DNA, 28 bp, synthetic construct
  source 1..28: mol_type = other DNA
gtgggaaggacgctgagttggaatctgg

SEQ ID NO: 43388 - DNA, 28 bp, synthetic construct
  source 1..28: mol_type = other DNA
ggaaggacgctgagttggaatctggagg

SEQ ID NO: 43389 - DNA, 28 bp, synthetic construct
  source 1..28: mol_type = other DNA
aggacgctgagttggaatctggaggtgg

SEQ ID NO: 43390 - DNA, 28 bp, synthetic construct
  source 1..28: mol_type = other DNA
aggtggtatgtgatgtgtgagattcagg

SEQ ID NO: 43391 - DNA, 28 bp, synthetic construct
  source 1..28: mol_type = other DNA
ggtggtatgtgatgtgtgagattcaggg

SEQ ID NO: 43392 - DNA, 28 bp, synthetic construct
  source 1..28: mol_type = other DNA
gtgtgagattcagggagagtgcgagcgg

SEQ ID NO: 43393 - DNA, 28 bp, synthetic construct
  source 1..28: mol_type = other DNA
tcagatgtctcaccgttgttgtcgctgg

SEQ ID NO: 43394 - DNA, 28 bp, synthetic construct
  source 1..28: mol_type = other DNA
accgttgttgtcgctggacatgagctgg

SEQ ID NO: 43395 - DNA, 28 bp, synthetic construct
  source 1..28: mol_type = other DNA
accagctcatgtccagcgacaacaacgg

SEQ ID NO: 43396 - DNA, 28 bp, synthetic construct
  source 1..28: mol_type = other DNA
gtcgctggacatgagctggtaagtcagg

SEQ ID NO: 43397 - DNA, 28 bp, synthetic construct
  source 1..28: mol_type = other DNA
catgagctggtaagtcaggagcttctgg

SEQ ID NO: 43398 - DNA, 28 bp, synthetic construct
  source 1..28: mol_type = other DNA
atgagctggtaagtcaggagcttctggg

SEQ ID NO: 43399 - DNA, 28 bp, synthetic construct
  source 1..28: mol_type = other DNA
aggagcttctgggccttcaagttgtagg

SEQ ID NO: 43400 - DNA, 28 bp, synthetic construct
  source 1..28: mol_type = other DNA
ttctgggccttcaagttgtaggctccgg

SEQ ID NO: 43401 - DNA, 28 bp, synthetic construct
  source 1..28: mol_type = other DNA
aatctggccggagcctacaacttgaagg

SEQ ID NO: 43402 - DNA, 28 bp, synthetic construct
  source 1..28: mol_type = other DNA
aagttgtaggctccggccagattcatgg

SEQ ID NO: 43403 - DNA, 28 bp, synthetic construct
  source 1..28: mol_type = other DNA
ggctccggccagattcatggcaatcagg

SEQ ID NO: 43404 - DNA, 28 bp, synthetic construct
  source 1..28: mol_type = other DNA
gcatcctgattgccatgaatctggccgg

SEQ ID NO: 43405 - DNA, 28 bp, synthetic construct
  source 1..28: mol_type = other DNA
gccagattcatggcaatcaggatgctgg

SEQ ID NO: 43406 - DNA, 28 bp, synthetic construct
  source 1..28: mol_type = other DNA
ccagattcatggcaatcaggatgctggg

SEQ ID NO: 43407 - DNA, 28 bp, synthetic construct
  source 1..28: mol_type = other DNA
cagattcatggcaatcaggatgctgggg

SEQ ID NO: 43408 - DNA, 28 bp, synthetic construct
  source 1..28: mol_type = other DNA
tcatggcaatcaggatgctggggtttgg

SEQ ID NO: 43409 - DNA, 28 bp, synthetic construct
  source 1..28: mol_type = other DNA
catggcaatcaggatgctggggtttggg

SEQ ID NO: 43410 - DNA, 28 bp, synthetic construct
  source 1..28: mol_type = other DNA
gcaatcaggatgctggggtttgggtagg

SEQ ID NO: 43411 - DNA, 28 bp, synthetic construct
  source 1..28: mol_type = other DNA
ggaatacaagtactcatggagaactcgg

SEQ ID NO: 43412 - DNA, 28 bp, synthetic construct
  source 1..28: mol_type = other DNA
ttggtcaatggaatacaagtactcatgg

SEQ ID NO: 43413 - DNA, 28 bp, synthetic construct
  source 1..28: mol_type = other DNA
atgagtacttgtattccattgaccaagg

SEQ ID NO: 43414 - DNA, 28 bp, synthetic construct
  source 1..28: mol_type = other DNA
tgagtacttgtattccattgaccaaggg

SEQ ID NO: 43415 - DNA, 28 bp, synthetic construct
  source 1..28: mol_type = other DNA
ccattgaccaagggctcctgtgctgagg

SEQ ID NO: 43416 - DNA, 28 bp, synthetic construct
  source 1..28: mol_type = other DNA
cattgaccaagggctcctgtgctgaggg

SEQ ID NO: 43417 - DNA, 28 bp, synthetic construct
  source 1..28: mol_type = other DNA
accaagggctcctgtgctgagggaacgg

SEQ ID NO: 43418 - DNA, 28 bp, synthetic construct
  source 1..28: mol_type = other DNA
gccgttccctcagcacaggagcccttgg

SEQ ID NO: 43419 - DNA, 28 bp, synthetic construct
  source 1..28: mol_type = other DNA
ctcttctcagccgttccctcagcacagg

SEQ ID NO: 43420 - DNA, 28 bp, synthetic construct
  source 1..28: mol_type = other DNA
ctgtgctgagggaacggctgagaagagg

SEQ ID NO: 43421 - DNA, 28 bp, synthetic construct
  source 1..28: mol_type = other DNA
gaatgagggttagaaggtgagtaaatgg

SEQ ID NO: 43422 - DNA, 28 bp, synthetic construct
  source 1..28: mol_type = other DNA
tttttgagaaggaatgagggttagaagg

SEQ ID NO: 43423 - DNA, 28 bp, synthetic construct
  source 1..28: mol_type = other DNA
ggataatgtttttgagaaggaatgaggg

SEQ ID NO: 43424 - DNA, 28 bp, synthetic construct
  source 1..28: mol_type = other DNA
gggataatgtttttgagaaggaatgagg

SEQ ID NO: 43425 - DNA, 28 bp, synthetic construct
  source 1..28: mol_type = other DNA
agacacggggataatgtttttgagaagg

SEQ ID NO: 43426 - DNA, 28 bp, synthetic construct
  source 1..28: mol_type = other DNA
agaaagaaaaagcatcaaagacacgggg

SEQ ID NO: 43427 - DNA, 28 bp, synthetic construct
  source 1..28: mol_type = other DNA
aagaaagaaaaagcatcaaagacacggg

SEQ ID NO: 43428 - DNA, 28 bp, synthetic construct
  source 1..28: mol_type = other DNA
aaagaaagaaaaagcatcaaagacacgg

SEQ ID NO: 43429 - DNA, 28 bp, synthetic construct
  source 1..28: mol_type = other DNA
gcaatcactataggaattccaaaatggg

SEQ ID NO: 43430 - DNA, 28 bp, synthetic construct
  source 1..28: mol_type = other DNA
agcaatcactataggaattccaaaatgg

SEQ ID NO: 43431 - DNA, 28 bp, synthetic construct
  source 1..28: mol_type = other DNA
agtggttgaaaatagcaatcactatagg

SEQ ID NO: 43432 - DNA, 28 bp, synthetic construct
  source 1..28: mol_type = other DNA
gctattttcaaccactcagtgtcagagg

SEQ ID NO: 43433 - DNA, 28 bp, synthetic construct
  source 1..28: mol_type = other DNA
aggggctgtgacctctgacactgagtgg

SEQ ID NO: 43434 - DNA, 28 bp, synthetic construct
  source 1..28: mol_type = other DNA
tgtcagaggtcacagccccttccccagg

SEQ ID NO: 43435 - DNA, 28 bp, synthetic construct
  source 1..28: mol_type = other DNA
gtcagaggtcacagccccttccccaggg

SEQ ID NO: 43436 - DNA, 28 bp, synthetic construct
  source 1..28: mol_type = other DNA
cagggaagcagttgccctggggaagggg

SEQ ID NO: 43437 - DNA, 28 bp, synthetic construct
  source 1..28: mol_type = other DNA
tcagggaagcagttgccctggggaaggg

SEQ ID NO: 43438 - DNA, 28 bp, synthetic construct
  source 1..28: mol_type = other DNA
gtcagggaagcagttgccctggggaagg

SEQ ID NO: 43439 - DNA, 28 bp, synthetic construct
  source 1..28: mol_type = other DNA
ggaggtcagggaagcagttgccctgggg

SEQ ID NO: 43440 - DNA, 28 bp, synthetic construct
  source 1..28: mol_type = other DNA
aggaggtcagggaagcagttgccctggg

SEQ ID NO: 43441 - DNA, 28 bp, synthetic construct
  source 1..28: mol_type = other DNA
aaggaggtcagggaagcagttgccctgg

SEQ ID NO: 43442 - DNA, 28 bp, synthetic construct
  source 1..28: mol_type = other DNA
agggcaactgcttccctgacctccttgg

SEQ ID NO: 43443 - DNA, 28 bp, synthetic construct
  source 1..28: mol_type = other DNA
gtatgatgtttttccaaggaggtcaggg

SEQ ID NO: 43444 - DNA, 28 bp, synthetic construct
  source 1..28: mol_type = other DNA
agtatgatgtttttccaaggaggtcagg

SEQ ID NO: 43445 - DNA, 28 bp, synthetic construct
  source 1..28: mol_type = other DNA
ctgtgagtatgatgtttttccaaggagg

SEQ ID NO: 43446 - DNA, 28 bp, synthetic construct
  source 1..28: mol_type = other DNA
atgctgtgagtatgatgtttttccaagg

SEQ ID NO: 43447 - DNA, 28 bp, synthetic construct
  source 1..28: mol_type = other DNA
aacatcatactcacagcatgaactctgg

SEQ ID NO: 43448 - DNA, 28 bp, synthetic construct
  source 1..28: mol_type = other DNA
acatcatactcacagcatgaactctggg

SEQ ID NO: 43449 - DNA, 28 bp, synthetic construct
  source 1..28: mol_type = other DNA
atactcacagcatgaactctgggtctgg

SEQ ID NO: 43450 - DNA, 28 bp, synthetic construct
  source 1..28: mol_type = other DNA
tactcacagcatgaactctgggtctggg

SEQ ID NO: 43451 - DNA, 28 bp, synthetic construct
  source 1..28: mol_type = other DNA
actagtcccagctgtagcccagagaagg

SEQ ID NO: 43452 - DNA, 28 bp, synthetic construct
  source 1..28: mol_type = other DNA
cccagctgtagcccagagaaggctcagg

SEQ ID NO: 43453 - DNA, 28 bp, synthetic construct
  source 1..28: mol_type = other DNA
tcctgagccttctctgggctacagctgg

SEQ ID NO: 43454 - DNA, 28 bp, synthetic construct
  source 1..28: mol_type = other DNA
agctgtagcccagagaaggctcaggagg

SEQ ID NO: 43455 - DNA, 28 bp, synthetic construct
  source 1..28: mol_type = other DNA
agcccagagaaggctcaggaggtagagg

SEQ ID NO: 43456 - DNA, 28 bp, synthetic construct
  source 1..28: mol_type = other DNA
gcccagagaaggctcaggaggtagaggg

SEQ ID NO: 43457 - DNA, 28 bp, synthetic construct
  source 1..28: mol_type = other DNA
gccctctacctcctgagccttctctggg

SEQ ID NO: 43458 - DNA, 28 bp, synthetic construct
  source 1..28: mol_type = other DNA
tgccctctacctcctgagccttctctgg

SEQ ID NO: 43459 - DNA, 28 bp, synthetic construct
  source 1..28: mol_type = other DNA
aggctcaggaggtagagggcaaaccagg

SEQ ID NO: 43460 - DNA, 28 bp, synthetic construct
  source 1..28: mol_type = other DNA
acatagacgagagagtgagatggcctgg

SEQ ID NO: 43461 - DNA, 28 bp, synthetic construct
  source 1..28: mol_type = other DNA
gagagacatagacgagagagtgagatgg

SEQ ID NO: 43462 - DNA, 28 bp, synthetic construct
  source 1..28: mol_type = other DNA
tctctcgtctatgtctctcatccacagg

SEQ ID NO: 43463 - DNA, 28 bp, synthetic construct
  source 1..28: mol_type = other DNA
atccacaggtaccgcgatttgcaagtgg

SEQ ID NO: 43464 - DNA, 28 bp, synthetic construct
  source 1..28: mol_type = other DNA
ttccacttgcaaatcgcggtacctgtgg

SEQ ID NO: 43465 - DNA, 28 bp, synthetic construct
  source 1..28: mol_type = other DNA
aaagaaatattccacttgcaaatcgcgg

SEQ ID NO: 43466 - DNA, 28 bp, synthetic construct
  source 1..28: mol_type = other DNA
aacaaagggaagcacatataagagaagg

SEQ ID NO: 43467 - DNA, 28 bp, synthetic construct
  source 1..28: mol_type = other DNA
ggttggggacagattatttaacaaaggg

SEQ ID NO: 43468 - DNA, 28 bp, synthetic construct
  source 1..28: mol_type = other DNA
gggttggggacagattatttaacaaagg

SEQ ID NO: 43469 - DNA, 28 bp, synthetic construct
  source 1..28: mol_type = other DNA
ggggcagttaggagaggctgggttgggg

SEQ ID NO: 43470 - DNA, 28 bp, synthetic construct
  source 1..28: mol_type = other DNA
aggggcagttaggagaggctgggttggg

SEQ ID NO: 43471 - DNA, 28 bp, synthetic construct
  source 1..28: mol_type = other DNA
caggggcagttaggagaggctgggttgg

SEQ ID NO: 43472 - DNA, 28 bp, synthetic construct
  source 1..28: mol_type = other DNA
agcacaggggcagttaggagaggctggg

SEQ ID NO: 43473 - DNA, 28 bp, synthetic construct
  source 1..28: mol_type = other DNA
cagcacaggggcagttaggagaggctgg

SEQ ID NO: 43474 - DNA, 28 bp, synthetic construct
  source 1..28: mol_type = other DNA
aggtcagcacaggggcagttaggagagg

SEQ ID NO: 43475 - DNA, 28 bp, synthetic construct
  source 1..28: mol_type = other DNA
aggagaggtcagcacaggggcagttagg

SEQ ID NO: 43476 - DNA, 28 bp, synthetic construct
  source 1..28: mol_type = other DNA
atcaggaaaggagaggtcagcacagggg

SEQ ID NO: 43477 - DNA, 28 bp, synthetic construct
  source 1..28: mol_type = other DNA
tatcaggaaaggagaggtcagcacaggg

SEQ ID NO: 43478 - DNA, 28 bp, synthetic construct
  source 1..28: mol_type = other DNA
gtatcaggaaaggagaggtcagcacagg

SEQ ID NO: 43479 - DNA, 28 bp, synthetic construct
  source 1..28: mol_type = other DNA
ttacttacttgtatcaggaaaggagagg

SEQ ID NO: 43480 - DNA, 28 bp, synthetic construct
  source 1..28: mol_type = other DNA
aaaatttacttacttgtatcaggaaagg

SEQ ID NO: 43481 - DNA, 28 bp, synthetic construct
  source 1..28: mol_type = other DNA
aaatgaaaatttacttacttgtatcagg

SEQ ID NO: 43482 - DNA, 28 bp, synthetic construct
  source 1..28: mol_type = other DNA
aagtttaccgactatagaccctccaagg

SEQ ID NO: 43483 - DNA, 28 bp, synthetic construct
  source 1..28: mol_type = other DNA
tcagacaccttggagggtctatagtcgg

SEQ ID NO: 43484 - DNA, 28 bp, synthetic construct
  source 1..28: mol_type = other DNA
actatagaccctccaaggtgtctgaagg

SEQ ID NO: 43485 - DNA, 28 bp, synthetic construct
  source 1..28: mol_type = other DNA
agaagtcaccttcagacaccttggaggg

SEQ ID NO: 43486 - DNA, 28 bp, synthetic construct
  source 1..28: mol_type = other DNA
tagaagtcaccttcagacaccttggagg

SEQ ID NO: 43487 - DNA, 28 bp, synthetic construct
  source 1..28: mol_type = other DNA
tccaaggtgtctgaaggtgacttctagg

SEQ ID NO: 43488 - DNA, 28 bp, synthetic construct
  source 1..28: mol_type = other DNA
acctagaagtcaccttcagacaccttgg

SEQ ID NO: 43489 - DNA, 28 bp, synthetic construct
  source 1..28: mol_type = other DNA
aggttgcacagtcatatgagaaacctgg

SEQ ID NO: 43490 - DNA, 28 bp, synthetic construct
  source 1..28: mol_type = other DNA
ggttgcacagtcatatgagaaacctggg

SEQ ID NO: 43491 - DNA, 28 bp, synthetic construct
  source 1..28: mol_type = other DNA
gttgcacagtcatatgagaaacctgggg

SEQ ID NO: 43492 - DNA, 28 bp, synthetic construct
  source 1..28: mol_type = other DNA
cacagtcatatgagaaacctggggctgg

SEQ ID NO: 43493 - DNA, 28 bp, synthetic construct
  source 1..28: mol_type = other DNA
acagtcatatgagaaacctggggctggg

SEQ ID NO: 43494 - DNA, 28 bp, synthetic construct
  source 1..28: mol_type = other DNA
aaacctggggctgggtatgcagtgaagg

SEQ ID NO: 43495 - DNA, 28 bp, synthetic construct
  source 1..28: mol_type = other DNA
ttgccttcactgcatacccagccccagg

SEQ ID NO: 43496 - DNA, 28 bp, synthetic construct
  source 1..28: mol_type = other DNA
atgttgagaaaatgtcctttaccaaagg

SEQ ID NO: 43497 - DNA, 28 bp, synthetic construct
  source 1..28: mol_type = other DNA
gagaaaatgtcctttaccaaaggcctgg

SEQ ID NO: 43498 - DNA, 28 bp, synthetic construct
  source 1..28: mol_type = other DNA
agaaaatgtcctttaccaaaggcctggg

SEQ ID NO: 43499 - DNA, 28 bp, synthetic construct
  source 1..28: mol_type = other DNA
gatgtctgacccaggcctttggtaaagg

SEQ ID NO: 43500 - DNA, 28 bp, synthetic construct
  source 1..28: mol_type = other DNA
ttaccaaaggcctgggtcagacatcagg

SEQ ID NO: 43501 - DNA, 28 bp, synthetic construct
  source 1..28: mol_type = other DNA
cttcctgatgtctgacccaggcctttgg

SEQ ID NO: 43502 - DNA, 28 bp, synthetic construct
  source 1..28: mol_type = other DNA
ggcctgggtcagacatcaggaagtttgg

SEQ ID NO: 43503 - DNA, 28 bp, synthetic construct
  source 1..28: mol_type = other DNA
atccaaacttcctgatgtctgacccagg

SEQ ID NO: 43504 - DNA, 28 bp, synthetic construct
  source 1..28: mol_type = other DNA
gattggatacaataagggctagaagagg

SEQ ID NO: 43505 - DNA, 28 bp, synthetic construct
  source 1..28: mol_type = other DNA
cccttattgtatccaatcagttaccagg

SEQ ID NO: 43506 - DNA, 28 bp, synthetic construct
  source 1..28: mol_type = other DNA
gcctggtaactgattggatacaataagg

SEQ ID NO: 43507 - DNA, 28 bp, synthetic construct
  source 1..28: mol_type = other DNA
actaaaaagcagcctggtaactgattgg

SEQ ID NO: 43508 - DNA, 28 bp, synthetic construct
  source 1..28: mol_type = other DNA
gtgaagtagttactaaaaagcagcctgg

SEQ ID NO: 43509 - DNA, 28 bp, synthetic construct
  source 1..28: mol_type = other DNA
ggctgctttttagtaactacttcactgg

SEQ ID NO: 43510 - DNA, 28 bp, synthetic construct
  source 1..28: mol_type = other DNA
gctgctttttagtaactacttcactggg

SEQ ID NO: 43511 - DNA, 28 bp, synthetic construct
  source 1..28: mol_type = other DNA
tttagtaactacttcactgggatttagg

SEQ ID NO: 43512 - DNA, 28 bp, synthetic construct
  source 1..28: mol_type = other DNA
cttcactgggatttaggccattcatagg

SEQ ID NO: 43513 - DNA, 28 bp, synthetic construct
  source 1..28: mol_type = other DNA
cataaaatgagctgatgcctatgaatgg

SEQ ID NO: 43514 - DNA, 28 bp, synthetic construct
  source 1..28: mol_type = other DNA
aggacatgttgtaaagcaggtgtctagg

SEQ ID NO: 43515 - DNA, 28 bp, synthetic construct
  source 1..28: mol_type = other DNA
cacctgctttacaacatgtccttttagg

SEQ ID NO: 43516 - DNA, 28 bp, synthetic construct
  source 1..28: mol_type = other DNA
agcctaaaaggacatgttgtaaagcagg

SEQ ID NO: 43517 - DNA, 28 bp, synthetic construct
  source 1..28: mol_type = other DNA
ttacaacatgtccttttaggctctcagg

SEQ ID NO: 43518 - DNA, 28 bp, synthetic construct
  source 1..28: mol_type = other DNA
aacatgtccttttaggctctcaggcagg

SEQ ID NO: 43519 - DNA, 28 bp, synthetic construct
  source 1..28: mol_type = other DNA
acatgtccttttaggctctcaggcaggg

SEQ ID NO: 43520 - DNA, 28 bp, synthetic construct
  source 1..28: mol_type = other DNA
gcagatccctgcctgagagcctaaaagg

SEQ ID NO: 43521 - DNA, 28 bp, synthetic construct
  source 1..28: mol_type = other DNA
ttaggctctcaggcagggatctgccagg

SEQ ID NO: 43522 - DNA, 28 bp, synthetic construct
  source 1..28: mol_type = other DNA
aggcagggatctgccaggtgacatctgg

SEQ ID NO: 43523 - DNA, 28 bp, synthetic construct
  source 1..28: mol_type = other DNA
taatttcacaaagccagatgtcacctgg

SEQ ID NO: 43524 - DNA, 28 bp, synthetic construct
  source 1..28: mol_type = other DNA
ctttgtgaaattaatgatgtctacctgg

SEQ ID NO: 43525 - DNA, 28 bp, synthetic construct
  source 1..28: mol_type = other DNA
gaaattaatgatgtctacctggacctgg

SEQ ID NO: 43526 - DNA, 28 bp, synthetic construct
  source 1..28: mol_type = other DNA
agagtctaggctagaatccaggtccagg

SEQ ID NO: 43527 - DNA, 28 bp, synthetic construct
  source 1..28: mol_type = other DNA
cttcaaagagtctaggctagaatccagg

SEQ ID NO: 43528 - DNA, 28 bp, synthetic construct
  source 1..28: mol_type = other DNA
aaagtcaaacaacttcaaagagtctagg

SEQ ID NO: 43529 - DNA, 28 bp, synthetic construct
  source 1..28: mol_type = other DNA
agactctttgaagttgtttgactttagg

SEQ ID NO: 43530 - DNA, 28 bp, synthetic construct
  source 1..28: mol_type = other DNA
aagttgtttgactttaggcaagaaatgg

SEQ ID NO: 43531 - DNA, 28 bp, synthetic construct
  source 1..28: mol_type = other DNA
ttgactttaggcaagaaatggacctcgg

SEQ ID NO: 43532 - DNA, 28 bp, synthetic construct
  source 1..28: mol_type = other DNA
gaaatggacctcggtttcccagaaatgg

SEQ ID NO: 43533 - DNA, 28 bp, synthetic construct
  source 1..28: mol_type = other DNA
aaacaaaaccatttctgggaaaccgagg

SEQ ID NO: 43534 - DNA, 28 bp, synthetic construct
  source 1..28: mol_type = other DNA
agagaaatcaaacaaaaccatttctggg

SEQ ID NO: 43535 - DNA, 28 bp, synthetic construct
  source 1..28: mol_type = other DNA
aagagaaatcaaacaaaaccatttctgg

SEQ ID NO: 43536 - DNA, 28 bp, synthetic construct
  source 1..28: mol_type = other DNA
tttgtttgatttctctttccttatctgg

SEQ ID NO: 43537 - DNA, 28 bp, synthetic construct
  source 1..28: mol_type = other DNA
ttgagatggcttttatctccagataagg

SEQ ID NO: 43538 - DNA, 28 bp, synthetic construct
  source 1..28: mol_type = other DNA
atctgaaagctttgggtgtttgagatgg

SEQ ID NO: 43539 - DNA, 28 bp, synthetic construct
  source 1..28: mol_type = other DNA
ttaaaagataatatctgaaagctttggg

SEQ ID NO: 43540 - DNA, 28 bp, synthetic construct
  source 1..28: mol_type = other DNA
tttaaaagataatatctgaaagctttgg

SEQ ID NO: 43541 - DNA, 28 bp, synthetic construct
  source 1..28: mol_type = other DNA
acacatctgaaatatgtattcttaatgg

SEQ ID NO: 43542 - DNA, 28 bp, synthetic construct
  source 1..28: mol_type = other DNA
ataatgcaaattatacttctttataagg

SEQ ID NO: 43543 - DNA, 28 bp, synthetic construct
  source 1..28: mol_type = other DNA
taatgcaaattatacttctttataaggg

SEQ ID NO: 43544 - DNA, 28 bp, synthetic construct
  source 1..28: mol_type = other DNA
cttctttataagggagaactgaaaatgg

SEQ ID NO: 43545 - DNA, 28 bp, synthetic construct
  source 1..28: mol_type = other DNA
aatggtatgttgaaattataaagaaagg

SEQ ID NO: 43546 - DNA, 28 bp, synthetic construct
  source 1..28: mol_type = other DNA
ccttaaaatgagctactttacatgcagg

SEQ ID NO: 43547 - DNA, 28 bp, synthetic construct
  source 1..28: mol_type = other DNA
ctgcatgtaaagtagctcattttaaggg

SEQ ID NO: 43548 - DNA, 28 bp, synthetic construct
  source 1..28: mol_type = other DNA
tgcatgtaaagtagctcattttaagggg

SEQ ID NO: 43549 - DNA, 28 bp, synthetic construct
  source 1..28: mol_type = other DNA
ctcattttaaggggatattctccagtgg

SEQ ID NO: 43550 - DNA, 28 bp, synthetic construct
  source 1..28: mol_type = other DNA
acttttatgctaagatgggcgccactgg

SEQ ID NO: 43551 - DNA, 28 bp, synthetic construct
  source 1..28: mol_type = other DNA
agggctttgacttttatgctaagatggg

SEQ ID NO: 43552 - DNA, 28 bp, synthetic construct
  source 1..28: mol_type = other DNA
aagggctttgacttttatgctaagatgg

SEQ ID NO: 43553 - DNA, 28 bp, synthetic construct
  source 1..28: mol_type = other DNA
tctaaggtcttataggtcatgaaaaggg

SEQ ID NO: 43554 - DNA, 28 bp, synthetic construct
  source 1..28: mol_type = other DNA
ttctaaggtcttataggtcatgaaaagg

SEQ ID NO: 43555 - DNA, 28 bp, synthetic construct
  source 1..28: mol_type = other DNA
atgacctataagaccttagaagatctgg

SEQ ID NO: 43556 - DNA, 28 bp, synthetic construct
  source 1..28: mol_type = other DNA
ggagccagatcttctaaggtcttatagg

SEQ ID NO: 43557 - DNA, 28 bp, synthetic construct
  source 1..28: mol_type = other DNA
ataagaccttagaagatctggctcctgg

SEQ ID NO: 43558 - DNA, 28 bp, synthetic construct
  source 1..28: mol_type = other DNA
aggaaaccaggagccagatcttctaagg

SEQ ID NO: 43559 - DNA, 28 bp, synthetic construct
  source 1..28: mol_type = other DNA
tggagctgaggtcagaaaggaaaccagg

SEQ ID NO: 43560 - DNA, 28 bp, synthetic construct
  source 1..28: mol_type = other DNA
tggtttcctttctgacctcagctccagg

SEQ ID NO: 43561 - DNA, 28 bp, synthetic construct
  source 1..28: mol_type = other DNA
aaaacgcctggagctgaggtcagaaagg

SEQ ID NO: 43562 - DNA, 28 bp, synthetic construct
  source 1..28: mol_type = other DNA
gcaaaggggaaaacgcctggagctgagg

SEQ ID NO: 43563 - DNA, 28 bp, synthetic construct
  source 1..28: mol_type = other DNA
cggtgtgagcaaaggggaaaacgcctgg

SEQ ID NO: 43564 - DNA, 28 bp, synthetic construct
  source 1..28: mol_type = other DNA
tgtgatgggagcggtgtgagcaaagggg

SEQ ID NO: 43565 - DNA, 28 bp, synthetic construct
  source 1..28: mol_type = other DNA
gtgtgatgggagcggtgtgagcaaaggg

SEQ ID NO: 43566 - DNA, 28 bp, synthetic construct
  source 1..28: mol_type = other DNA
tgtgtgatgggagcggtgtgagcaaagg

SEQ ID NO: 43567 - DNA, 28 bp, synthetic construct
  source 1..28: mol_type = other DNA
cacaagaagttctgtgtgatgggagcgg

SEQ ID NO: 43568 - DNA, 28 bp, synthetic construct
  source 1..28: mol_type = other DNA
aggggcacaagaagttctgtgtgatggg

SEQ ID NO: 43569 - DNA, 28 bp, synthetic construct
  source 1..28: mol_type = other DNA
aaggggcacaagaagttctgtgtgatgg

SEQ ID NO: 43570 - DNA, 28 bp, synthetic construct
  source 1..28: mol_type = other DNA
tgcaaaggtagctgatgtgttcaagggg

SEQ ID NO: 43571 - DNA, 28 bp, synthetic construct
  source 1..28: mol_type = other DNA
gtgcaaaggtagctgatgtgttcaaggg

SEQ ID NO: 43572 - DNA, 28 bp, synthetic construct
  source 1..28: mol_type = other DNA
tgtgcaaaggtagctgatgtgttcaagg

SEQ ID NO: 43573 - DNA, 28 bp, synthetic construct
  source 1..28: mol_type = other DNA
gggctgagggggacatcatgtgcaaagg

SEQ ID NO: 43574 - DNA, 28 bp, synthetic construct
  source 1..28: mol_type = other DNA
ttgcacatgatgtccccctcagcccagg

SEQ ID NO: 43575 - DNA, 28 bp, synthetic construct
  source 1..28: mol_type = other DNA
aaaagaagagggtcctgggctgaggggg

SEQ ID NO: 43576 - DNA, 28 bp, synthetic construct
  source 1..28: mol_type = other DNA
taaaagaagagggtcctgggctgagggg

SEQ ID NO: 43577 - DNA, 28 bp, synthetic construct
  source 1..28: mol_type = other DNA
ttaaaagaagagggtcctgggctgaggg

SEQ ID NO: 43578 - DNA, 28 bp, synthetic construct
  source 1..28: mol_type = other DNA
tttaaaagaagagggtcctgggctgagg

SEQ ID NO: 43579 - DNA, 28 bp, synthetic construct
  source 1..28: mol_type = other DNA
aggctatttaaaagaagagggtcctggg

SEQ ID NO: 43580 - DNA, 28 bp, synthetic construct
  source 1..28: mol_type = other DNA
gaggctatttaaaagaagagggtcctgg

SEQ ID NO: 43581 - DNA, 28 bp, synthetic construct
  source 1..28: mol_type = other DNA
gaccctcttcttttaaatagcctcatgg

SEQ ID NO: 43582 - DNA, 28 bp, synthetic construct
  source 1..28: mol_type = other DNA
caccatgaggctatttaaaagaagaggg

SEQ ID NO: 43583 - DNA, 28 bp, synthetic construct
  source 1..28: mol_type = other DNA
ccaccatgaggctatttaaaagaagagg

SEQ ID NO: 43584 - DNA, 28 bp, synthetic construct
  source 1..28: mol_type = other DNA
tgaaggatgtgaggaagccaccatgagg

SEQ ID NO: 43585 - DNA, 28 bp, synthetic construct
  source 1..28: mol_type = other DNA
tctgagcagagacatgaaggatgtgagg

SEQ ID NO: 43586 - DNA, 28 bp, synthetic construct
  source 1..28: mol_type = other DNA
tcacatccttcatgtctctgctcagagg

SEQ ID NO: 43587 - DNA, 28 bp, synthetic construct
  source 1..28: mol_type = other DNA
agcttacctctgagcagagacatgaagg

SEQ ID NO: 43588 - DNA, 28 bp, synthetic construct
  source 1..28: mol_type = other DNA
ggtaagcttttagagacgccttcccagg

SEQ ID NO: 43589 - DNA, 28 bp, synthetic construct
  source 1..28: mol_type = other DNA
ggatcttatgtagggtggcctgggaagg

SEQ ID NO: 43590 - DNA, 28 bp, synthetic construct
  source 1..28: mol_type = other DNA
tgtaggatcttatgtagggtggcctggg

SEQ ID NO: 43591 - DNA, 28 bp, synthetic construct
  source 1..28: mol_type = other DNA
atgtaggatcttatgtagggtggcctgg

SEQ ID NO: 43592 - DNA, 28 bp, synthetic construct
  source 1..28: mol_type = other DNA
tgaggatgtaggatcttatgtagggtgg

SEQ ID NO: 43593 - DNA, 28 bp, synthetic construct
  source 1..28: mol_type = other DNA
aggtgaggatgtaggatcttatgtaggg

SEQ ID NO: 43594 - DNA, 28 bp, synthetic construct
  source 1..28: mol_type = other DNA
gaggtgaggatgtaggatcttatgtagg

SEQ ID NO: 43595 - DNA, 28 bp, synthetic construct
  source 1..28: mol_type = other DNA
ggggtgtcagtggaggtgaggatgtagg

SEQ ID NO: 43596 - DNA, 28 bp, synthetic construct
  source 1..28: mol_type = other DNA
ggcatgaggggtgtcagtggaggtgagg

SEQ ID NO: 43597 - DNA, 28 bp, synthetic construct
  source 1..28: mol_type = other DNA
cgaggggcatgaggggtgtcagtggagg

SEQ ID NO: 43598 - DNA, 28 bp, synthetic construct
  source 1..28: mol_type = other DNA
aggcgaggggcatgaggggtgtcagtgg

SEQ ID NO: 43599 - DNA, 28 bp, synthetic construct
  source 1..28: mol_type = other DNA
agttatagcaggcgaggggcatgagggg

SEQ ID NO: 43600 - DNA, 28 bp, synthetic construct
  source 1..28: mol_type = other DNA
gagttatagcaggcgaggggcatgaggg

SEQ ID NO: 43601 - DNA, 28 bp, synthetic construct
  source 1..28: mol_type = other DNA
tgagttatagcaggcgaggggcatgagg

SEQ ID NO: 43602 - DNA, 28 bp, synthetic construct
  source 1..28: mol_type = other DNA
agggcaatgagttatagcaggcgagggg

SEQ ID NO: 43603 - DNA, 28 bp, synthetic construct
  source 1..28: mol_type = other DNA
gagggcaatgagttatagcaggcgaggg

SEQ ID NO: 43604 - DNA, 28 bp, synthetic construct
  source 1..28: mol_type = other DNA
agagggcaatgagttatagcaggcgagg

SEQ ID NO: 43605 - DNA, 28 bp, synthetic construct
  source 1..28: mol_type = other DNA
gcgacagagggcaatgagttatagcagg

SEQ ID NO: 43606 - DNA, 28 bp, synthetic construct
  source 1..28: mol_type = other DNA
attgccctctgtcgcactaagtgtgtgg

SEQ ID NO: 43607 - DNA, 28 bp, synthetic construct
  source 1..28: mol_type = other DNA
acaaccacacacttagtgcgacagaggg

SEQ ID NO: 43608 - DNA, 28 bp, synthetic construct
  source 1..28: mol_type = other DNA
aacaaccacacacttagtgcgacagagg

SEQ ID NO: 43609 - DNA, 28 bp, synthetic construct
  source 1..28: mol_type = other DNA
tccctactagaatgtctgctccacgagg

SEQ ID NO: 43610 - DNA, 28 bp, synthetic construct
  source 1..28: mol_type = other DNA
ccctcgtggagcagacattctagtaggg

SEQ ID NO: 43611 - DNA, 28 bp, synthetic construct
  source 1..28: mol_type = other DNA
tccctcgtggagcagacattctagtagg

SEQ ID NO: 43612 - DNA, 28 bp, synthetic construct
  source 1..28: mol_type = other DNA
tactagaatgtctgctccacgagggagg

SEQ ID NO: 43613 - DNA, 28 bp, synthetic construct
  source 1..28: mol_type = other DNA
actagaatgtctgctccacgagggaggg

SEQ ID NO: 43614 - DNA, 28 bp, synthetic construct
  source 1..28: mol_type = other DNA
ctagaatgtctgctccacgagggagggg

SEQ ID NO: 43615 - DNA, 28 bp, synthetic construct
  source 1..28: mol_type = other DNA
ccacgagggaggggctttgtctctttgg

SEQ ID NO: 43616 - DNA, 28 bp, synthetic construct
  source 1..28: mol_type = other DNA
gagctaggtagtgttgtaagggctaagg

SEQ ID NO: 43617 - DNA, 28 bp, synthetic construct
  source 1..28: mol_type = other DNA
tactgtgagctaggtagtgttgtaaggg

SEQ ID NO: 43618 - DNA, 28 bp, synthetic construct
  source 1..28: mol_type = other DNA
ctactgtgagctaggtagtgttgtaagg

SEQ ID NO: 43619 - DNA, 28 bp, synthetic construct
  source 1..28: mol_type = other DNA
aagtattttatttctactgtgagctagg

SEQ ID NO: 43620 - DNA, 28 bp, synthetic construct
  source 1..28: mol_type = other DNA
tgaattaatgagcaaatgtaagacatgg

SEQ ID NO: 43621 - DNA, 28 bp, synthetic construct
  source 1..28: mol_type = other DNA
gaattaatgagcaaatgtaagacatggg

SEQ ID NO: 43622 - DNA, 28 bp, synthetic construct
  source 1..28: mol_type = other DNA
gggtaataaagcattttttcccccttgg

SEQ ID NO: 43623 - DNA, 28 bp, synthetic construct
  source 1..28: mol_type = other DNA
ggtaataaagcattttttcccccttggg

SEQ ID NO: 43624 - DNA, 28 bp, synthetic construct
  source 1..28: mol_type = other DNA
agcattttttcccccttgggaaacatgg

SEQ ID NO: 43625 - DNA, 28 bp, synthetic construct
  source 1..28: mol_type = other DNA
gcattttttcccccttgggaaacatggg

SEQ ID NO: 43626 - DNA, 28 bp, synthetic construct
  source 1..28: mol_type = other DNA
caaaactcacccatgtttcccaaggggg

SEQ ID NO: 43627 - DNA, 28 bp, synthetic construct
  source 1..28: mol_type = other DNA
acaaaactcacccatgtttcccaagggg

SEQ ID NO: 43628 - DNA, 28 bp, synthetic construct
  source 1..28: mol_type = other DNA
cacaaaactcacccatgtttcccaaggg

SEQ ID NO: 43629 - DNA, 28 bp, synthetic construct
  source 1..28: mol_type = other DNA
tcacaaaactcacccatgtttcccaagg

SEQ ID NO: 43630 - DNA, 28 bp, synthetic construct
  source 1..28: mol_type = other DNA
ggtgagttttgtgagatgagagcacagg

SEQ ID NO: 43631 - DNA, 28 bp, synthetic construct
  source 1..28: mol_type = other DNA
gtgagttttgtgagatgagagcacaggg

SEQ ID NO: 43632 - DNA, 28 bp, synthetic construct
  source 1..28: mol_type = other DNA
tgagatgagagcacagggtacatactgg

SEQ ID NO: 43633 - DNA, 28 bp, synthetic construct
  source 1..28: mol_type = other DNA
gagatgagagcacagggtacatactggg

SEQ ID NO: 43634 - DNA, 28 bp, synthetic construct
  source 1..28: mol_type = other DNA
agatgagagcacagggtacatactgggg

SEQ ID NO: 43635 - DNA, 28 bp, synthetic construct
  source 1..28: mol_type = other DNA
gcacagggtacatactggggtgtgctgg

SEQ ID NO: 43636 - DNA, 28 bp, synthetic construct
  source 1..28: mol_type = other DNA
ggggtgtgctggacaacttctaacatgg

SEQ ID NO: 43637 - DNA, 28 bp, synthetic construct
  source 1..28: mol_type = other DNA
atgaataccgggaggtgaaaacacaggg

SEQ ID NO: 43638 - DNA, 28 bp, synthetic construct
  source 1..28: mol_type = other DNA
catgaataccgggaggtgaaaacacagg

SEQ ID NO: 43639 - DNA, 28 bp, synthetic construct
  source 1..28: mol_type = other DNA
aaacattattcagataaaatattatagg

SEQ ID NO: 43640 - DNA, 28 bp, synthetic construct
  source 1..28: mol_type = other DNA
gtggagtttgtattttgcatactcaagg

SEQ ID NO: 43641 - DNA, 28 bp, synthetic construct
  source 1..28: mol_type = other DNA
actacaaagtaaaatgaacattttgtgg

SEQ ID NO: 43642 - DNA, 28 bp, synthetic construct
  source 1..28: mol_type = other DNA
ttaaatttatattacatatttattaagg

SEQ ID NO: 43643 - DNA, 28 bp, synthetic construct
  source 1..28: mol_type = other DNA
tttatattacatatttattaaggcaagg

SEQ ID NO: 43644 - DNA, 28 bp, synthetic construct
  source 1..28: mol_type = other DNA
tagaaaaacacatttgttctgcttaagg

SEQ ID NO: 43645 - DNA, 28 bp, synthetic construct
  source 1..28: mol_type = other DNA
acatttgttctgcttaaggcatacttgg

SEQ ID NO: 43646 - DNA, 28 bp, synthetic construct
  source 1..28: mol_type = other DNA
catttgttctgcttaaggcatacttggg

SEQ ID NO: 43647 - DNA, 28 bp, synthetic construct
  source 1..28: mol_type = other DNA
ttcagatgtgcaataatttgtacaatgg

SEQ ID NO: 43648 - DNA, 28 bp, synthetic construct
  source 1..28: mol_type = other DNA
tatgcagacagtctgttatgcactgtgg

SEQ ID NO: 43649 - DNA, 28 bp, synthetic construct
  source 1..28: mol_type = other DNA
cataaaaatgctaaagaagtaaaccagg

SEQ ID NO: 43650 - DNA, 28 bp, synthetic construct
  source 1..28: mol_type = other DNA
gtaaaccaggtatattacctgacttagg

SEQ ID NO: 43651 - DNA, 28 bp, synthetic construct
  source 1..28: mol_type = other DNA
tatgacctaagtcaggtaatatacctgg

SEQ ID NO: 43652 - DNA, 28 bp, synthetic construct
  source 1..28: mol_type = other DNA
ccgatcaacatttatgacctaagtcagg

SEQ ID NO: 43653 - DNA, 28 bp, synthetic construct
  source 1..28: mol_type = other DNA
tttcaaactgctgcatactttgacaagg

SEQ ID NO: 43654 - DNA, 28 bp, synthetic construct
  source 1..28: mol_type = other DNA
aaagtatgcagcagtttgaaaactttgg

SEQ ID NO: 43655 - DNA, 28 bp, synthetic construct
  source 1..28: mol_type = other DNA
gtttgaaaactttggcttccttgtttgg

SEQ ID NO: 43656 - DNA, 28 bp, synthetic construct
  source 1..28: mol_type = other DNA
gtcttggttctaaaggtaccaaacaagg

SEQ ID NO: 43657 - DNA, 28 bp, synthetic construct
  source 1..28: mol_type = other DNA
ggtgcttggtgagtcttggttctaaagg

SEQ ID NO: 43658 - DNA, 28 bp, synthetic construct
  source 1..28: mol_type = other DNA
ctaaatgatggtgcttggtgagtcttgg

SEQ ID NO: 43659 - DNA, 28 bp, synthetic construct
  source 1..28: mol_type = other DNA
caagactcaccaagcaccatcatttagg

SEQ ID NO: 43660 - DNA, 28 bp, synthetic construct
  source 1..28: mol_type = other DNA
tttaaatagcctaaatgatggtgcttgg

SEQ ID NO: 43661 - DNA, 28 bp, synthetic construct
  source 1..28: mol_type = other DNA
aaacatgtttaaatagcctaaatgatgg

SEQ ID NO: 43662 - DNA, 28 bp, synthetic construct
  source 1..28: mol_type = other DNA
atgttagaagaagaggaagaaattcagg

SEQ ID NO: 43663 - DNA, 28 bp, synthetic construct
  source 1..28: mol_type = other DNA
tcctcttcttctaacatcataataatgg

SEQ ID NO: 43664 - DNA, 28 bp, synthetic construct
  source 1..28: mol_type = other DNA
gccattattatgatgttagaagaagagg

SEQ ID NO: 43665 - DNA, 28 bp, synthetic construct
  source 1..28: mol_type = other DNA
taacatcataataatggcttttagaagg

SEQ ID NO: 43666 - DNA, 28 bp, synthetic construct
  source 1..28: mol_type = other DNA
gcttttagaaggtaaagagaatacaagg

SEQ ID NO: 43667 - DNA, 28 bp, synthetic construct
  source 1..28: mol_type = other DNA
ttatattgcatcaatacacaattcaagg

SEQ ID NO: 43668 - DNA, 28 bp, synthetic construct
  source 1..28: mol_type = other DNA
tatattgcatcaatacacaattcaaggg

SEQ ID NO: 43669 - DNA, 28 bp, synthetic construct
  source 1..28: mol_type = other DNA
atcaatacacaattcaagggaattctgg

SEQ ID NO: 43670 - DNA, 28 bp, synthetic construct
  source 1..28: mol_type = other DNA
ttctggtcttccctcccccaactcacgg

SEQ ID NO: 43671 - DNA, 28 bp, synthetic construct
  source 1..28: mol_type = other DNA
taaattatatccgtgagttgggggaggg

SEQ ID NO: 43672 - DNA, 28 bp, synthetic construct
  source 1..28: mol_type = other DNA
ataaattatatccgtgagttgggggagg

SEQ ID NO: 43673 - DNA, 28 bp, synthetic construct
  source 1..28: mol_type = other DNA
ggtataaattatatccgtgagttggggg

SEQ ID NO: 43674 - DNA, 28 bp, synthetic construct
  source 1..28: mol_type = other DNA
gggtataaattatatccgtgagttgggg

SEQ ID NO: 43675 - DNA, 28 bp, synthetic construct
  source 1..28: mol_type = other DNA
agggtataaattatatccgtgagttggg

SEQ ID NO: 43676 - DNA, 28 bp, synthetic construct
  source 1..28: mol_type = other DNA
cagggtataaattatatccgtgagttgg

SEQ ID NO: 43677 - DNA, 28 bp, synthetic construct
  source 1..28: mol_type = other DNA
gggtgactggaagttgtggatatcaggg

SEQ ID NO: 43678 - DNA, 28 bp, synthetic construct
  source 1..28: mol_type = other DNA
ggggtgactggaagttgtggatatcagg

SEQ ID NO: 43679 - DNA, 28 bp, synthetic construct
  source 1..28: mol_type = other DNA
tatccacaacttccagtcacccccttgg

SEQ ID NO: 43680 - DNA, 28 bp, synthetic construct
  source 1..28: mol_type = other DNA
atgccaagggggtgactggaagttgtgg

SEQ ID NO: 43681 - DNA, 28 bp, synthetic construct
  source 1..28: mol_type = other DNA
acttacaaaatgccaagggggtgactgg

SEQ ID NO: 43682 - DNA, 28 bp, synthetic construct
  source 1..28: mol_type = other DNA
cacccccttggcattttgtaagtccagg

SEQ ID NO: 43683 - DNA, 28 bp, synthetic construct
  source 1..28: mol_type = other DNA
ttcctggacttacaaaatgccaaggggg

SEQ ID NO: 43684 - DNA, 28 bp, synthetic construct
  source 1..28: mol_type = other DNA
attcctggacttacaaaatgccaagggg

SEQ ID NO: 43685 - DNA, 28 bp, synthetic construct
  source 1..28: mol_type = other DNA
tattcctggacttacaaaatgccaaggg

SEQ ID NO: 43686 - DNA, 28 bp, synthetic construct
  source 1..28: mol_type = other DNA
atattcctggacttacaaaatgccaagg

SEQ ID NO: 43687 - DNA, 28 bp, synthetic construct
  source 1..28: mol_type = other DNA
tttgtaagtccaggaatattcaagtcgg

SEQ ID NO: 43688 - DNA, 28 bp, synthetic construct
  source 1..28: mol_type = other DNA
attctaaatccgacttgaatattcctgg

SEQ ID NO: 43689 - DNA, 28 bp, synthetic construct
  source 1..28: mol_type = other DNA
ggaatattcaagtcggatttagaattgg

SEQ ID NO: 43690 - DNA, 28 bp, synthetic construct
  source 1..28: mol_type = other DNA
tcaaagaacagatggggtctgtgactgg

SEQ ID NO: 43691 - DNA, 28 bp, synthetic construct
  source 1..28: mol_type = other DNA
aaagacaaaaatcaaagaacagatgggg

SEQ ID NO: 43692 - DNA, 28 bp, synthetic construct
  source 1..28: mol_type = other DNA
aaaagacaaaaatcaaagaacagatggg

SEQ ID NO: 43693 - DNA, 28 bp, synthetic construct
  source 1..28: mol_type = other DNA
caaaagacaaaaatcaaagaacagatgg

SEQ ID NO: 43694 - DNA, 28 bp, synthetic construct
  source 1..28: mol_type = other DNA
catctgttctttgatttttgtcttttgg

SEQ ID NO: 43695 - DNA, 28 bp, synthetic construct
  source 1..28: mol_type = other DNA
tgtgagtggataatcaggaaaaatgagg

SEQ ID NO: 43696 - DNA, 28 bp, synthetic construct
  source 1..28: mol_type = other DNA
tgagtcatcttgtgagtggataatcagg

SEQ ID NO: 43697 - DNA, 28 bp, synthetic construct
  source 1..28: mol_type = other DNA
ttatccactcacaagatgactcagttgg

SEQ ID NO: 43698 - DNA, 28 bp, synthetic construct
  source 1..28: mol_type = other DNA
tatccactcacaagatgactcagttggg

SEQ ID NO: 43699 - DNA, 28 bp, synthetic construct
  source 1..28: mol_type = other DNA
gttcccaactgagtcatcttgtgagtgg

SEQ ID NO: 43700 - DNA, 28 bp, synthetic construct
  source 1..28: mol_type = other DNA
acttgaccatgattgtagtgctttctgg

SEQ ID NO: 43701 - DNA, 28 bp, synthetic construct
  source 1..28: mol_type = other DNA
gaccatgattgtagtgctttctggctgg

SEQ ID NO: 43702 - DNA, 28 bp, synthetic construct
  source 1..28: mol_type = other DNA
accatgattgtagtgctttctggctggg

SEQ ID NO: 43703 - DNA, 28 bp, synthetic construct
  source 1..28: mol_type = other DNA
gcccagccagaaagcactacaatcatgg

SEQ ID NO: 43704 - DNA, 28 bp, synthetic construct
  source 1..28: mol_type = other DNA
tttctggctgggctccttccctcatcgg

SEQ ID NO: 43705 - DNA, 28 bp, synthetic construct
  source 1..28: mol_type = other DNA
ttctggctgggctccttccctcatcggg

SEQ ID NO: 43706 - DNA, 28 bp, synthetic construct
  source 1..28: mol_type = other DNA
ttcacactgtcttcccgatgagggaagg

SEQ ID NO: 43707 - DNA, 28 bp, synthetic construct
  source 1..28: mol_type = other DNA
acttttcacactgtcttcccgatgaggg

SEQ ID NO: 43708 - DNA, 28 bp, synthetic construct
  source 1..28: mol_type = other DNA
tacttttcacactgtcttcccgatgagg

SEQ ID NO: 43709 - DNA, 28 bp, synthetic construct
  source 1..28: mol_type = other DNA
aagtaaaaaatactgaattctcttctgg

SEQ ID NO: 43710 - DNA, 28 bp, synthetic construct
  source 1..28: mol_type = other DNA
aatactgaattctcttctggcagtgtgg

SEQ ID NO: 43711 - DNA, 28 bp, synthetic construct
  source 1..28: mol_type = other DNA
atactgaattctcttctggcagtgtggg

SEQ ID NO: 43712 - DNA, 28 bp, synthetic construct
  source 1..28: mol_type = other DNA
ggcagtgtgggtcatatccactgtctgg

SEQ ID NO: 43713 - DNA, 28 bp, synthetic construct
  source 1..28: mol_type = other DNA
gcagtgtgggtcatatccactgtctggg

SEQ ID NO: 43714 - DNA, 28 bp, synthetic construct
  source 1..28: mol_type = other DNA
agaggcatttttaaatcccagacagtgg

SEQ ID NO: 43715 - DNA, 28 bp, synthetic construct
  source 1..28: mol_type = other DNA
atttaaaaatgcctcttcatgtgtaagg

SEQ ID NO: 43716 - DNA, 28 bp, synthetic construct
  source 1..28: mol_type = other DNA
aaaatgcctcttcatgtgtaaggcgagg

SEQ ID NO: 43717 - DNA, 28 bp, synthetic construct
  source 1..28: mol_type = other DNA
atgcctcttcatgtgtaaggcgaggtgg

SEQ ID NO: 43718 - DNA, 28 bp, synthetic construct
  source 1..28: mol_type = other DNA
ggaccacctcgccttacacatgaagagg

SEQ ID NO: 43719 - DNA, 28 bp, synthetic construct
  source 1..28: mol_type = other DNA
atgtgtaaggcgaggtggtccgacctgg

SEQ ID NO: 43720 - DNA, 28 bp, synthetic construct
  source 1..28: mol_type = other DNA
gaggtggtccgacctggaaaatgctcgg

SEQ ID NO: 43721 - DNA, 28 bp, synthetic construct
  source 1..28: mol_type = other DNA
aaatgcgaccgagcattttccaggtcgg

SEQ ID NO: 43722 - DNA, 28 bp, synthetic construct
  source 1..28: mol_type = other DNA
ccaaaaatgcgaccgagcattttccagg

SEQ ID NO: 43723 - DNA, 28 bp, synthetic construct
  source 1..28: mol_type = other DNA
aaatgctcggtcgcatttttggcactgg

SEQ ID NO: 43724 - DNA, 28 bp, synthetic construct
  source 1..28: mol_type = other DNA
ctcggtcgcatttttggcactggaacgg

SEQ ID NO: 43725 - DNA, 28 bp, synthetic construct
  source 1..28: mol_type = other DNA
tcggtcgcatttttggcactggaacggg

SEQ ID NO: 43726 - DNA, 28 bp, synthetic construct
  source 1..28: mol_type = other DNA
gtcgcatttttggcactggaacgggcgg

SEQ ID NO: 43727 - DNA, 28 bp, synthetic construct
  source 1..28: mol_type = other DNA
gaacgggcggtgccccgtgtgtttacgg

SEQ ID NO: 43728 - DNA, 28 bp, synthetic construct
  source 1..28: mol_type = other DNA
tgccccgtgtgtttacggtagtgcctgg

SEQ ID NO: 43729 - DNA, 28 bp, synthetic construct
  source 1..28: mol_type = other DNA
gaccaggcactaccgtaaacacacgggg

SEQ ID NO: 43730 - DNA, 28 bp, synthetic construct
  source 1..28: mol_type = other DNA
tgaccaggcactaccgtaaacacacggg

SEQ ID NO: 43731 - DNA, 28 bp, synthetic construct
  source 1..28: mol_type = other DNA
ctgaccaggcactaccgtaaacacacgg

SEQ ID NO: 43732 - DNA, 28 bp, synthetic construct
  source 1..28: mol_type = other DNA
gtagtgcctggtcagttcatctgagcgg

SEQ ID NO: 43733 - DNA, 28 bp, synthetic construct
  source 1..28: mol_type = other DNA
tagtgcctggtcagttcatctgagcggg

SEQ ID NO: 43734 - DNA, 28 bp, synthetic construct
  source 1..28: mol_type = other DNA
attcgcccgctcagatgaactgaccagg

SEQ ID NO: 43735 - DNA, 28 bp, synthetic construct
  source 1..28: mol_type = other DNA
ccatccacagccgtcccagtcacagtgg

SEQ ID NO: 43736 - DNA, 28 bp, synthetic construct
  source 1..28: mol_type = other DNA
cttaccactgtgactgggacggctgtgg

SEQ ID NO: 43737 - DNA, 28 bp, synthetic construct
  source 1..28: mol_type = other DNA
cacagccgtcccagtcacagtggtaagg

SEQ ID NO: 43738 - DNA, 28 bp, synthetic construct
  source 1..28: mol_type = other DNA
agaaaccttaccactgtgactgggacgg

SEQ ID NO: 43739 - DNA, 28 bp, synthetic construct
  source 1..28: mol_type = other DNA
ggtgagaaaccttaccactgtgactggg

SEQ ID NO: 43740 - DNA, 28 bp, synthetic construct
  source 1..28: mol_type = other DNA
aggtgagaaaccttaccactgtgactgg

SEQ ID NO: 43741 - DNA, 28 bp, synthetic construct
  source 1..28: mol_type = other DNA
cagtggtaaggtttctcacctgtaaagg

SEQ ID NO: 43742 - DNA, 28 bp, synthetic construct
  source 1..28: mol_type = other DNA
aattttttttttcttttacctttacagg

SEQ ID NO: 43743 - DNA, 28 bp, synthetic construct
  source 1..28: mol_type = other DNA
aagaatcgccccttttaaaaactgaagg

SEQ ID NO: 43744 - DNA, 28 bp, synthetic construct
  source 1..28: mol_type = other DNA
ctatctggccttcagtttttaaaagggg

SEQ ID NO: 43745 - DNA, 28 bp, synthetic construct
  source 1..28: mol_type = other DNA
actatctggccttcagtttttaaaaggg

SEQ ID NO: 43746 - DNA, 28 bp, synthetic construct
  source 1..28: mol_type = other DNA
tactatctggccttcagtttttaaaagg

SEQ ID NO: 43747 - DNA, 28 bp, synthetic construct
  source 1..28: mol_type = other DNA
atagggtcagagttggtttactatctgg

SEQ ID NO: 43748 - DNA, 28 bp, synthetic construct
  source 1..28: mol_type = other DNA
gatttctttaggatagggtcagagttgg

SEQ ID NO: 43749 - DNA, 28 bp, synthetic construct
  source 1..28: mol_type = other DNA
ctctgaccctatcctaaagaaatccagg

SEQ ID NO: 43750 - DNA, 28 bp, synthetic construct
  source 1..28: mol_type = other DNA
gacattcctggatttctttaggataggg

SEQ ID NO: 43751 - DNA, 28 bp, synthetic construct
  source 1..28: mol_type = other DNA
agacattcctggatttctttaggatagg

SEQ ID NO: 43752 - DNA, 28 bp, synthetic construct
  source 1..28: mol_type = other DNA
agtgtccactggtagcctatggggctgg

SEQ ID NO: 43753 - DNA, 28 bp, synthetic construct
  source 1..28: mol_type = other DNA
agcttccagccccataggctaccagtgg

SEQ ID NO: 43754 - DNA, 28 bp, synthetic construct
  source 1..28: mol_type = other DNA
tagcctatggggctggaagctaacctgg

SEQ ID NO: 43755 - DNA, 28 bp, synthetic construct
  source 1..28: mol_type = other DNA
agcctatggggctggaagctaacctggg

SEQ ID NO: 43756 - DNA, 28 bp, synthetic construct
  source 1..28: mol_type = other DNA
ttcccaggttagcttccagccccatagg

SEQ ID NO: 43757 - DNA, 28 bp, synthetic construct
  source 1..28: mol_type = other DNA
ggctggaagctaacctgggaagtcaagg

SEQ ID NO: 43758 - DNA, 28 bp, synthetic construct
  source 1..28: mol_type = other DNA
tggaagctaacctgggaagtcaaggagg

SEQ ID NO: 43759 - DNA, 28 bp, synthetic construct
  source 1..28: mol_type = other DNA
aacctgggaagtcaaggaggcactgagg

SEQ ID NO: 43760 - DNA, 28 bp, synthetic construct
  source 1..28: mol_type = other DNA
ctcctcagtgcctccttgacttcccagg

SEQ ID NO: 43761 - DNA, 28 bp, synthetic construct
  source 1..28: mol_type = other DNA
caaggaggcactgaggagtgtccactgg

SEQ ID NO: 43762 - DNA, 28 bp, synthetic construct
  source 1..28: mol_type = other DNA
ctgaggagtgtccactggtagcctatgg

SEQ ID NO: 43763 - DNA, 28 bp, synthetic construct
  source 1..28: mol_type = other DNA
tgaggagtgtccactggtagcctatggg

SEQ ID NO: 43764 - DNA, 28 bp, synthetic construct
  source 1..28: mol_type = other DNA
gaggagtgtccactggtagcctatgggg

SEQ ID NO: 43765 - DNA, 28 bp, synthetic construct
  source 1..28: mol_type = other DNA
agtgtccactggtagcctatggggctgg

SEQ ID NO: 43766 - DNA, 28 bp, synthetic construct
  source 1..28: mol_type = other DNA
agcttccagccccataggctaccagtgg

SEQ ID NO: 43767 - DNA, 28 bp, synthetic construct
  source 1..28: mol_type = other DNA
gaggggggttagcttccagccccatagg

SEQ ID NO: 43768 - DNA, 28 bp, synthetic construct
  source 1..28: mol_type = other DNA
gggggacaaactgcagaagggagggggg

SEQ ID NO: 43769 - DNA, 28 bp, synthetic construct
  source 1..28: mol_type = other DNA
agggggacaaactgcagaagggaggggg

SEQ ID NO: 43770 - DNA, 28 bp, synthetic construct
  source 1..28: mol_type = other DNA
tagggggacaaactgcagaagggagggg

SEQ ID NO: 43771 - DNA, 28 bp, synthetic construct
  source 1..28: mol_type = other DNA
gtagggggacaaactgcagaagggaggg

SEQ ID NO: 43772 - DNA, 28 bp, synthetic construct
  source 1..28: mol_type = other DNA
ggtagggggacaaactgcagaagggagg

SEQ ID NO: 43773 - DNA, 28 bp, synthetic construct
  source 1..28: mol_type = other DNA
acaggtagggggacaaactgcagaaggg

SEQ ID NO: 43774 - DNA, 28 bp, synthetic construct
  source 1..28: mol_type = other DNA
cacaggtagggggacaaactgcagaagg

SEQ ID NO: 43775 - DNA, 28 bp, synthetic construct
  source 1..28: mol_type = other DNA
tctgcagtttgtccccctacctgtgtgg

SEQ ID NO: 43776 - DNA, 28 bp, synthetic construct
  source 1..28: mol_type = other DNA
ctgcagtttgtccccctacctgtgtggg

SEQ ID NO: 43777 - DNA, 28 bp, synthetic construct
  source 1..28: mol_type = other DNA
tgtccccctacctgtgtgggttcgcagg

SEQ ID NO: 43778 - DNA, 28 bp, synthetic construct
  source 1..28: mol_type = other DNA
acacctgcgaacccacacaggtaggggg

SEQ ID NO: 43779 - DNA, 28 bp, synthetic construct
  source 1..28: mol_type = other DNA
cacacctgcgaacccacacaggtagggg

SEQ ID NO: 43780 - DNA, 28 bp, synthetic construct
  source 1..28: mol_type = other DNA
gcacacctgcgaacccacacaggtaggg

SEQ ID NO: 43781 - DNA, 28 bp, synthetic construct
  source 1..28: mol_type = other DNA
ggcacacctgcgaacccacacaggtagg

SEQ ID NO: 43782 - DNA, 28 bp, synthetic construct
  source 1..28: mol_type = other DNA
tcaaggcacacctgcgaacccacacagg

SEQ ID NO: 43783 - DNA, 28 bp, synthetic construct
  source 1..28: mol_type = other DNA
gtgggttcgcaggtgtgccttgagatgg

SEQ ID NO: 43784 - DNA, 28 bp, synthetic construct
  source 1..28: mol_type = other DNA
tgggttcgcaggtgtgccttgagatggg

SEQ ID NO: 43785 - DNA, 28 bp, synthetic construct
  source 1..28: mol_type = other DNA
gccttgagatgggaactctttgtgtagg

SEQ ID NO: 43786 - DNA, 28 bp, synthetic construct
  source 1..28: mol_type = other DNA
acctacacaaagagttcccatctcaagg

SEQ ID NO: 43787 - DNA, 28 bp, synthetic construct
  source 1..28: mol_type = other DNA
gccgcagcccgcgtaatcacaagtgtgg

SEQ ID NO: 43788 - DNA, 28 bp, synthetic construct
  source 1..28: mol_type = other DNA
ccgcagcccgcgtaatcacaagtgtggg

SEQ ID NO: 43789 - DNA, 28 bp, synthetic construct
  source 1..28: mol_type = other DNA
cagcccgcgtaatcacaagtgtgggtgg

SEQ ID NO: 43790 - DNA, 28 bp, synthetic construct
  source 1..28: mol_type = other DNA
cccgcgtaatcacaagtgtgggtggcgg

SEQ ID NO: 43791 - DNA, 28 bp, synthetic construct
  source 1..28: mol_type = other DNA
accgccacccacacttgtgattacgcgg

SEQ ID NO: 43792 - DNA, 28 bp, synthetic construct
  source 1..28: mol_type = other DNA
acaagtgtgggtggcggtccttttccgg

SEQ ID NO: 43793 - DNA, 28 bp, synthetic construct
  source 1..28: mol_type = other DNA
caagtgtgggtggcggtccttttccggg

SEQ ID NO: 43794 - DNA, 28 bp, synthetic construct
  source 1..28: mol_type = other DNA
aagtgtgggtggcggtccttttccgggg

SEQ ID NO: 43795 - DNA, 28 bp, synthetic construct
  source 1..28: mol_type = other DNA
gggaagacgatcgtggccccggaaaagg

SEQ ID NO: 43796 - DNA, 28 bp, synthetic construct
  source 1..28: mol_type = other DNA
aaagaggggaagacgatcgtggccccgg

SEQ ID NO: 43797 - DNA, 28 bp, synthetic construct
  source 1..28: mol_type = other DNA
ggggccacgatcgtcttcccctctttgg

SEQ ID NO: 43798 - DNA, 28 bp, synthetic construct
  source 1..28: mol_type = other DNA
caagccaaagaggggaagacgatcgtgg

SEQ ID NO: 43799 - DNA, 28 bp, synthetic construct
  source 1..28: mol_type = other DNA
cacgatcgtcttcccctctttggcttgg

SEQ ID NO: 43800 - DNA, 28 bp, synthetic construct
  source 1..28: mol_type = other DNA
acgatcgtcttcccctctttggcttggg

SEQ ID NO: 43801 - DNA, 28 bp, synthetic construct
  source 1..28: mol_type = other DNA
ttcccctctttggcttgggctcctctgg

SEQ ID NO: 43802 - DNA, 28 bp, synthetic construct
  source 1..28: mol_type = other DNA
tgccagaggagcccaagccaaagagggg

SEQ ID NO: 43803 - DNA, 28 bp, synthetic construct
  source 1..28: mol_type = other DNA
atgccagaggagcccaagccaaagaggg

SEQ ID NO: 43804 - DNA, 28 bp, synthetic construct
  source 1..28: mol_type = other DNA
catgccagaggagcccaagccaaagagg

SEQ ID NO: 43805 - DNA, 28 bp, synthetic construct
  source 1..28: mol_type = other DNA
tttggcttgggctcctctggcatgcagg

SEQ ID NO: 43806 - DNA, 28 bp, synthetic construct
  source 1..28: mol_type = other DNA
ttgggctcctctggcatgcaggaaccgg

SEQ ID NO: 43807 - DNA, 28 bp, synthetic construct
  source 1..28: mol_type = other DNA
tgggctcctctggcatgcaggaaccggg

SEQ ID NO: 43808 - DNA, 28 bp, synthetic construct
  source 1..28: mol_type = other DNA
gctcctctggcatgcaggaaccgggtgg

SEQ ID NO: 43809 - DNA, 28 bp, synthetic construct
  source 1..28: mol_type = other DNA
atgccacccggttcctgcatgccagagg

SEQ ID NO: 43810 - DNA, 28 bp, synthetic construct
  source 1..28: mol_type = other DNA
gcaggaaccgggtggcatgagctctagg

SEQ ID NO: 43811 - DNA, 28 bp, synthetic construct
  source 1..28: mol_type = other DNA
caggaaccgggtggcatgagctctaggg

SEQ ID NO: 43812 - DNA, 28 bp, synthetic construct
  source 1..28: mol_type = other DNA
aggaaccgggtggcatgagctctagggg

SEQ ID NO: 43813 - DNA, 28 bp, synthetic construct
  source 1..28: mol_type = other DNA
cttcacccctagagctcatgccacccgg

SEQ ID NO: 43814 - DNA, 28 bp, synthetic construct
  source 1..28: mol_type = other DNA
gtggcatgagctctaggggtgaagaagg

SEQ ID NO: 43815 - DNA, 28 bp, synthetic construct
  source 1..28: mol_type = other DNA
gcatgagctctaggggtgaagaaggtgg

SEQ ID NO: 43816 - DNA, 28 bp, synthetic construct
  source 1..28: mol_type = other DNA
catgagctctaggggtgaagaaggtggg

SEQ ID NO: 43817 - DNA, 28 bp, synthetic construct
  source 1..28: mol_type = other DNA
atgagctctaggggtgaagaaggtgggg

SEQ ID NO: 43818 - DNA, 28 bp, synthetic construct
  source 1..28: mol_type = other DNA
gagcatcatcccgtgtgtcccgaagtgg

SEQ ID NO: 43819 - DNA, 28 bp, synthetic construct
  source 1..28: mol_type = other DNA
agcatcatcccgtgtgtcccgaagtggg

SEQ ID NO: 43820 - DNA, 28 bp, synthetic construct
  source 1..28: mol_type = other DNA
gcatcatcccgtgtgtcccgaagtgggg

SEQ ID NO: 43821 - DNA, 28 bp, synthetic construct
  source 1..28: mol_type = other DNA
gtgctggccccacttcgggacacacggg

SEQ ID NO: 43822 - DNA, 28 bp, synthetic construct
  source 1..28: mol_type = other DNA
tgtgctggccccacttcgggacacacgg

SEQ ID NO: 43823 - DNA, 28 bp, synthetic construct
  source 1..28: mol_type = other DNA
gtcccgaagtggggccagcacacacagg

SEQ ID NO: 43824 - DNA, 28 bp, synthetic construct
  source 1..28: mol_type = other DNA
tcccgaagtggggccagcacacacaggg

SEQ ID NO: 43825 - DNA, 28 bp, synthetic construct
  source 1..28: mol_type = other DNA
gccctgtgtgtgctggccccacttcggg

SEQ ID NO: 43826 - DNA, 28 bp, synthetic construct
  source 1..28: mol_type = other DNA
agccctgtgtgtgctggccccacttcgg

SEQ ID NO: 43827 - DNA, 28 bp, synthetic construct
  source 1..28: mol_type = other DNA
tcgggctggggagccctgtgtgtgctgg

SEQ ID NO: 43828 - DNA, 28 bp, synthetic construct
  source 1..28: mol_type = other DNA
ctccccagcccgagctacaaatccccgg

SEQ ID NO: 43829 - DNA, 28 bp, synthetic construct
  source 1..28: mol_type = other DNA
tccccagcccgagctacaaatccccggg

SEQ ID NO: 43830 - DNA, 28 bp, synthetic construct
  source 1..28: mol_type = other DNA
tcccggggatttgtagctcgggctgggg

SEQ ID NO: 43831 - DNA, 28 bp, synthetic construct
  source 1..28: mol_type = other DNA
gtcccggggatttgtagctcgggctggg

SEQ ID NO: 43832 - DNA, 28 bp, synthetic construct
  source 1..28: mol_type = other DNA
agtcccggggatttgtagctcgggctgg

SEQ ID NO: 43833 - DNA, 28 bp, synthetic construct
  source 1..28: mol_type = other DNA
ggtcagtcccggggatttgtagctcggg

SEQ ID NO: 43834 - DNA, 28 bp, synthetic construct
  source 1..28: mol_type = other DNA
aggtcagtcccggggatttgtagctcgg

SEQ ID NO: 43835 - DNA, 28 bp, synthetic construct
  source 1..28: mol_type = other DNA
agctacaaatccccgggactgaccttgg

SEQ ID NO: 43836 - DNA, 28 bp, synthetic construct
  source 1..28: mol_type = other DNA
aaatccccgggactgaccttggtaatgg

SEQ ID NO: 43837 - DNA, 28 bp, synthetic construct
  source 1..28: mol_type = other DNA
cgctccattaccaaggtcagtcccgggg

SEQ ID NO: 43838 - DNA, 28 bp, synthetic construct
  source 1..28: mol_type = other DNA
ccgctccattaccaaggtcagtcccggg

SEQ ID NO: 43839 - DNA, 28 bp, synthetic construct
  source 1..28: mol_type = other DNA
gccgctccattaccaaggtcagtcccgg

SEQ ID NO: 43840 - DNA, 28 bp, synthetic construct
  source 1..28: mol_type = other DNA
gggactgaccttggtaatggagcggcgg

SEQ ID NO: 43841 - DNA, 28 bp, synthetic construct
  source 1..28: mol_type = other DNA
ggactgaccttggtaatggagcggcggg

SEQ ID NO: 43842 - DNA, 28 bp, synthetic construct
  source 1..28: mol_type = other DNA
cgcaagtcccgccgctccattaccaagg

SEQ ID NO: 43843 - DNA, 28 bp, synthetic construct
  source 1..28: mol_type = other DNA
cttggtaatggagcggcgggacttgcgg

SEQ ID NO: 43844 - DNA, 28 bp, synthetic construct
  source 1..28: mol_type = other DNA
ggcgggacttgcggctgcatctgatcgg

SEQ ID NO: 43845 - DNA, 28 bp, synthetic construct
  source 1..28: mol_type = other DNA
gcgggacttgcggctgcatctgatcggg

SEQ ID NO: 43846 - DNA, 28 bp, synthetic construct
  source 1..28: mol_type = other DNA
gacttgcggctgcatctgatcgggcagg

SEQ ID NO: 43847 - DNA, 28 bp, synthetic construct
  source 1..28: mol_type = other DNA
tgcggctgcatctgatcgggcaggaagg

SEQ ID NO: 43848 - DNA, 28 bp, synthetic construct
  source 1..28: mol_type = other DNA
gctgcatctgatcgggcaggaaggatgg

SEQ ID NO: 43849 - DNA, 28 bp, synthetic construct
  source 1..28: mol_type = other DNA
ctgcatctgatcgggcaggaaggatggg

SEQ ID NO: 43850 - DNA, 28 bp, synthetic construct
  source 1..28: mol_type = other DNA
tgatcgggcaggaaggatgggtaattgg

SEQ ID NO: 43851 - DNA, 28 bp, synthetic construct
  source 1..28: mol_type = other DNA
gatcgggcaggaaggatgggtaattggg

SEQ ID NO: 43852 - DNA, 28 bp, synthetic construct
  source 1..28: mol_type = other DNA
gcaggaaggatgggtaattgggccccgg

SEQ ID NO: 43853 - DNA, 28 bp, synthetic construct
  source 1..28: mol_type = other DNA
caggaaggatgggtaattgggccccggg

SEQ ID NO: 43854 - DNA, 28 bp, synthetic construct
  source 1..28: mol_type = other DNA
gaaggatgggtaattgggccccgggtgg

SEQ ID NO: 43855 - DNA, 28 bp, synthetic construct
  source 1..28: mol_type = other DNA
aaggatgggtaattgggccccgggtggg

SEQ ID NO: 43856 - DNA, 28 bp, synthetic construct
  source 1..28: mol_type = other DNA
aggatgggtaattgggccccgggtgggg

SEQ ID NO: 43857 - DNA, 28 bp, synthetic construct
  source 1..28: mol_type = other DNA
tgggtaattgggccccgggtggggatgg

SEQ ID NO: 43858 - DNA, 28 bp, synthetic construct
  source 1..28: mol_type = other DNA
ttgggccccgggtggggatggaagccgg

SEQ ID NO: 43859 - DNA, 28 bp, synthetic construct
  source 1..28: mol_type = other DNA
tgggccccgggtggggatggaagccggg

SEQ ID NO: 43860 - DNA, 28 bp, synthetic construct
  source 1..28: mol_type = other DNA
gccccgggtggggatggaagccgggagg

SEQ ID NO: 43861 - DNA, 28 bp, synthetic construct
  source 1..28: mol_type = other DNA
tcctcccggcttccatccccacccgggg

SEQ ID NO: 43862 - DNA, 28 bp, synthetic construct
  source 1..28: mol_type = other DNA
ttcctcccggcttccatccccacccggg

SEQ ID NO: 43863 - DNA, 28 bp, synthetic construct
  source 1..28: mol_type = other DNA
cttcctcccggcttccatccccacccgg

SEQ ID NO: 43864 - DNA, 28 bp, synthetic construct
  source 1..28: mol_type = other DNA
ggtggggatggaagccgggaggaagcgg

SEQ ID NO: 43865 - DNA, 28 bp, synthetic construct
  source 1..28: mol_type = other DNA
gggatggaagccgggaggaagcggcagg

SEQ ID NO: 43866 - DNA, 28 bp, synthetic construct
  source 1..28: mol_type = other DNA
ggatggaagccgggaggaagcggcaggg

SEQ ID NO: 43867 - DNA, 28 bp, synthetic construct
  source 1..28: mol_type = other DNA
ggaagccgggaggaagcggcagggcagg

SEQ ID NO: 43868 - DNA, 28 bp, synthetic construct
  source 1..28: mol_type = other DNA
gaagccgggaggaagcggcagggcaggg

SEQ ID NO: 43869 - DNA, 28 bp, synthetic construct
  source 1..28: mol_type = other DNA
gtcaccctgccctgccgcttcctcccgg

SEQ ID NO: 43870 - DNA, 28 bp, synthetic construct
  source 1..28: mol_type = other DNA
ggtcttgaggaagtgctgagcagcaggg

SEQ ID NO: 43871 - DNA, 28 bp, synthetic construct
  source 1..28: mol_type = other DNA
gggtcttgaggaagtgctgagcagcagg

SEQ ID NO: 43872 - DNA, 28 bp, synthetic construct
  source 1..28: mol_type = other DNA
gctgctcagcacttcctcaagacccagg

SEQ ID NO: 43873 - DNA, 28 bp, synthetic construct
  source 1..28: mol_type = other DNA
ctgctcagcacttcctcaagacccaggg

SEQ ID NO: 43874 - DNA, 28 bp, synthetic construct
  source 1..28: mol_type = other DNA
tcagcacttcctcaagacccagggtcgg

SEQ ID NO: 43875 - DNA, 28 bp, synthetic construct
  source 1..28: mol_type = other DNA
cagcacttcctcaagacccagggtcggg

SEQ ID NO: 43876 - DNA, 28 bp, synthetic construct
  source 1..28: mol_type = other DNA
agcacttcctcaagacccagggtcgggg

SEQ ID NO: 43877 - DNA, 28 bp, synthetic construct
  source 1..28: mol_type = other DNA
aggactaccccgaccctgggtcttgagg

SEQ ID NO: 43878 - DNA, 28 bp, synthetic construct
  source 1..28: mol_type = other DNA
agacccagggtcggggtagtcctgctgg

SEQ ID NO: 43879 - DNA, 28 bp, synthetic construct
  source 1..28: mol_type = other DNA
gacccagggtcggggtagtcctgctggg

SEQ ID NO: 43880 - DNA, 28 bp, synthetic construct
  source 1..28: mol_type = other DNA
acccagggtcggggtagtcctgctgggg

SEQ ID NO: 43881 - DNA, 28 bp, synthetic construct
  source 1..28: mol_type = other DNA
tccccagcaggactaccccgaccctggg

SEQ ID NO: 43882 - DNA, 28 bp, synthetic construct
  source 1..28: mol_type = other DNA
ctccccagcaggactaccccgaccctgg

SEQ ID NO: 43883 - DNA, 28 bp, synthetic construct
  source 1..28: mol_type = other DNA
agtcctgctggggagctgccgccccagg

SEQ ID NO: 43884 - DNA, 28 bp, synthetic construct
  source 1..28: mol_type = other DNA
gtcctgctggggagctgccgccccaggg

SEQ ID NO: 43885 - DNA, 28 bp, synthetic construct
  source 1..28: mol_type = other DNA
tcctgctggggagctgccgccccagggg

SEQ ID NO: 43886 - DNA, 28 bp, synthetic construct
  source 1..28: mol_type = other DNA
cctgctggggagctgccgccccaggggg

SEQ ID NO: 43887 - DNA, 28 bp, synthetic construct
  source 1..28: mol_type = other DNA
ggctgcacacgacttccccctggggcgg

SEQ ID NO: 43888 - DNA, 28 bp, synthetic construct
  source 1..28: mol_type = other DNA
gccccagggggaagtcgtgtgcagccgg

SEQ ID NO: 43889 - DNA, 28 bp, synthetic construct
  source 1..28: mol_type = other DNA
gccggctgcacacgacttccccctgggg

SEQ ID NO: 43890 - DNA, 28 bp, synthetic construct
  source 1..28: mol_type = other DNA
ggccggctgcacacgacttccccctggg

SEQ ID NO: 43891 - DNA, 28 bp, synthetic construct
  source 1..28: mol_type = other DNA
cggccggctgcacacgacttccccctgg

SEQ ID NO: 43892 - DNA, 28 bp, synthetic construct
  source 1..28: mol_type = other DNA
cagggggaagtcgtgtgcagccggccgg

SEQ ID NO: 43893 - DNA, 28 bp, synthetic construct
  source 1..28: mol_type = other DNA
ggggaagtcgtgtgcagccggccggtgg

SEQ ID NO: 43894 - DNA, 28 bp, synthetic construct
  source 1..28: mol_type = other DNA
cagccggccggtggccattgctgagagg

SEQ ID NO: 43895 - DNA, 28 bp, synthetic construct
  source 1..28: mol_type = other DNA
agccggccggtggccattgctgagaggg

SEQ ID NO: 43896 - DNA, 28 bp, synthetic construct
  source 1..28: mol_type = other DNA
gccggccggtggccattgctgagagggg

SEQ ID NO: 43897 - DNA, 28 bp, synthetic construct
  source 1..28: mol_type = other DNA
ccccctctcagcaatggccaccggccgg

SEQ ID NO: 43898 - DNA, 28 bp, synthetic construct
  source 1..28: mol_type = other DNA
tggaccccctctcagcaatggccaccgg

SEQ ID NO: 43899 - DNA, 28 bp, synthetic construct
  source 1..28: mol_type = other DNA
tgggcgctggaccccctctcagcaatgg

SEQ ID NO: 43900 - DNA, 28 bp, synthetic construct
  source 1..28: mol_type = other DNA
gctgagagggggtccagcgcccaagtgg

SEQ ID NO: 43901 - DNA, 28 bp, synthetic construct
  source 1..28: mol_type = other DNA
ctgagagggggtccagcgcccaagtggg

SEQ ID NO: 43902 - DNA, 28 bp, synthetic construct
  source 1..28: mol_type = other DNA
tctcttcgtgcacccacttgggcgctgg

SEQ ID NO: 43903 - DNA, 28 bp, synthetic construct
  source 1..28: mol_type = other DNA
aggcggtctcttcgtgcacccacttggg

SEQ ID NO: 43904 - DNA, 28 bp, synthetic construct
  source 1..28: mol_type = other DNA
gaggcggtctcttcgtgcacccacttgg

SEQ ID NO: 43905 - DNA, 28 bp, synthetic construct
  source 1..28: mol_type = other DNA
gaagagaccgcctcctgcttgatcttgg

SEQ ID NO: 43906 - DNA, 28 bp, synthetic construct
  source 1..28: mol_type = other DNA
aagagaccgcctcctgcttgatcttggg

SEQ ID NO: 43907 - DNA, 28 bp, synthetic construct
  source 1..28: mol_type = other DNA
agagaccgcctcctgcttgatcttgggg

SEQ ID NO: 43908 - DNA, 28 bp, synthetic construct
  source 1..28: mol_type = other DNA
acgtgccccaagatcaagcaggaggcgg

SEQ ID NO: 43909 - DNA, 28 bp, synthetic construct
  source 1..28: mol_type = other DNA
cgcacgtgccccaagatcaagcaggagg

SEQ ID NO: 43910 - DNA, 28 bp, synthetic construct
  source 1..28: mol_type = other DNA
cctgcttgatcttggggcacgtgcgcgg

SEQ ID NO: 43911 - DNA, 28 bp, synthetic construct
  source 1..28: mol_type = other DNA
gcttgatcttggggcacgtgcgcggcgg

SEQ ID NO: 43912 - DNA, 28 bp, synthetic construct
  source 1..28: mol_type = other DNA
cacgtgcgcggcggcccgccgttgtagg

SEQ ID NO: 43913 - DNA, 28 bp, synthetic construct
  source 1..28: mol_type = other DNA
acgtgcgcggcggcccgccgttgtaggg

SEQ ID NO: 43914 - DNA, 28 bp, synthetic construct
  source 1..28: mol_type = other DNA
ggtggtggtggcgccctacaacggcggg

SEQ ID NO: 43915 - DNA, 28 bp, synthetic construct
  source 1..28: mol_type = other DNA
cggtggtggtggcgccctacaacggcgg

SEQ ID NO: 43916 - DNA, 28 bp, synthetic construct
  source 1..28: mol_type = other DNA
cgccgttgtagggcgccaccaccaccgg

SEQ ID NO: 43917 - DNA, 28 bp, synthetic construct
  source 1..28: mol_type = other DNA
gccgttgtagggcgccaccaccaccggg

SEQ ID NO: 43918 - DNA, 28 bp, synthetic construct
  source 1..28: mol_type = other DNA
acccggtggtggtggcgccctacaacgg

SEQ ID NO: 43919 - DNA, 28 bp, synthetic construct
  source 1..28: mol_type = other DNA
gttgtagggcgccaccaccaccgggtgg

SEQ ID NO: 43920 - DNA, 28 bp, synthetic construct
  source 1..28: mol_type = other DNA
cctgacggcagccacccggtggtggtgg

SEQ ID NO: 43921 - DNA, 28 bp, synthetic construct
  source 1..28: mol_type = other DNA
caccaccaccgggtggctgccgtcaggg

SEQ ID NO: 43922 - DNA, 28 bp, synthetic construct
  source 1..28: mol_type = other DNA
agccctgacggcagccacccggtggtgg

SEQ ID NO: 43923 - DNA, 28 bp, synthetic construct
  source 1..28: mol_type = other DNA
ggcagccctgacggcagccacccggtgg

SEQ ID NO: 43924 - DNA, 28 bp, synthetic construct
  source 1..28: mol_type = other DNA
aaaggcagccctgacggcagccacccgg

SEQ ID NO: 43925 - DNA, 28 bp, synthetic construct
  source 1..28: mol_type = other DNA
tcagcgtcagcaaaggcagccctgacgg

SEQ ID NO: 43926 - DNA, 28 bp, synthetic construct
  source 1..28: mol_type = other DNA
tgcctttgctgacgctgatgaccgacgg

SEQ ID NO: 43927 - DNA, 28 bp, synthetic construct
  source 1..28: mol_type = other DNA
gcctttgctgacgctgatgaccgacggg

SEQ ID NO: 43928 - DNA, 28 bp, synthetic construct
  source 1..28: mol_type = other DNA
gcccgtcggtcatcagcgtcagcaaagg

SEQ ID NO: 43929 - DNA, 28 bp, synthetic construct
  source 1..28: mol_type = other DNA
cctggcagcgagtacggcagcccgtcgg

SEQ ID NO: 43930 - DNA, 28 bp, synthetic construct
  source 1..28: mol_type = other DNA
cgacgggctgccgtactcgctgccaggg

SEQ ID NO: 43931 - DNA, 28 bp, synthetic construct
  source 1..28: mol_type = other DNA
gacgggctgccgtactcgctgccagggg

SEQ ID NO: 43932 - DNA, 28 bp, synthetic construct
  source 1..28: mol_type = other DNA
cgctgagcgcccctggcagcgagtacgg

SEQ ID NO: 43933 - DNA, 28 bp, synthetic construct
  source 1..28: mol_type = other DNA
tgctgaaggcgtcgctgagcgcccctgg

SEQ ID NO: 43934 - DNA, 28 bp, synthetic construct
  source 1..28: mol_type = other DNA
gggctgatgggcaagttcgtgctgaagg

SEQ ID NO: 43935 - DNA, 28 bp, synthetic construct
  source 1..28: mol_type = other DNA
cgaacttgcccatcagcccgccacctgg

SEQ ID NO: 43936 - DNA, 28 bp, synthetic construct
  source 1..28: mol_type = other DNA
acttgcccatcagcccgccacctggcgg

SEQ ID NO: 43937 - DNA, 28 bp, synthetic construct
  source 1..28: mol_type = other DNA
cgcagccgccaggtggcgggctgatggg

SEQ ID NO: 43938 - DNA, 28 bp, synthetic construct
  source 1..28: mol_type = other DNA
ccatcagcccgccacctggcggctgcgg

SEQ ID NO: 43939 - DNA, 28 bp, synthetic construct
  source 1..28: mol_type = other DNA
gcagcagccgcagccgccaggtggcggg

SEQ ID NO: 43940 - DNA, 28 bp, synthetic construct
  source 1..28: mol_type = other DNA
cgcagcagccgcagccgccaggtggcgg

SEQ ID NO: 43941 - DNA, 28 bp, synthetic construct
  source 1..28: mol_type = other DNA
cgccacctggcggctgcggctgctgcgg

SEQ ID NO: 43942 - DNA, 28 bp, synthetic construct
  source 1..28: mol_type = other DNA
cgccgcagcagccgcagccgccaggtgg

SEQ ID NO: 43943 - DNA, 28 bp, synthetic construct
  source 1..28: mol_type = other DNA
cacctggcggctgcggctgctgcggcgg

SEQ ID NO: 43944 - DNA, 28 bp, synthetic construct
  source 1..28: mol_type = other DNA
ttccgccgcagcagccgcagccgccagg

SEQ ID NO: 43945 - DNA, 28 bp, synthetic construct
  source 1..28: mol_type = other DNA
gcggctgctgcggcggaatgtacaccgg

SEQ ID NO: 43946 - DNA, 28 bp, synthetic construct
  source 1..28: mol_type = other DNA
cggctgctgcggcggaatgtacaccggg

SEQ ID NO: 43947 - DNA, 28 bp, synthetic construct
  source 1..28: mol_type = other DNA
gcggaatgtacaccgggtccaattctgg

SEQ ID NO: 43948 - DNA, 28 bp, synthetic construct
  source 1..28: mol_type = other DNA
gtacaccgggtccaattctggccgcagg

SEQ ID NO: 43949 - DNA, 28 bp, synthetic construct
  source 1..28: mol_type = other DNA
gagctcctgcggccagaattggacccgg

SEQ ID NO: 43950 - DNA, 28 bp, synthetic construct
  source 1..28: mol_type = other DNA
gggtccaattctggccgcaggagctcgg

SEQ ID NO: 43951 - DNA, 28 bp, synthetic construct
  source 1..28: mol_type = other DNA
gtggccgagctcctgcggccagaattgg

SEQ ID NO: 43952 - DNA, 28 bp, synthetic construct
  source 1..28: mol_type = other DNA
gggcggcttcgtggccgagctcctgcgg

SEQ ID NO: 43953 - DNA, 28 bp, synthetic construct
  source 1..28: mol_type = other DNA
aggagctcggccacgaagccgcccgagg

SEQ ID NO: 43954 - DNA, 28 bp, synthetic construct
  source 1..28: mol_type = other DNA
ggagctcggccacgaagccgcccgaggg

SEQ ID NO: 43955 - DNA, 28 bp, synthetic construct
  source 1..28: mol_type = other DNA
gagctcggccacgaagccgcccgagggg

SEQ ID NO: 43956 - DNA, 28 bp, synthetic construct
  source 1..28: mol_type = other DNA
gacgtgagcccctcgggcggcttcgtgg

SEQ ID NO: 43957 - DNA, 28 bp, synthetic construct
  source 1..28: mol_type = other DNA
acatcaacgacgtgagcccctcgggcgg

SEQ ID NO: 43958 - DNA, 28 bp, synthetic construct
  source 1..28: mol_type = other DNA
cggacatcaacgacgtgagcccctcggg

SEQ ID NO: 43959 - DNA, 28 bp, synthetic construct
  source 1..28: mol_type = other DNA
gcggacatcaacgacgtgagcccctcgg

SEQ ID NO: 43960 - DNA, 28 bp, synthetic construct
  source 1..28: mol_type = other DNA
ggggctcacgtcgttgatgtccgccagg

SEQ ID NO: 43961 - DNA, 28 bp, synthetic construct
  source 1..28: mol_type = other DNA
acgtcgttgatgtccgccaggttgaagg

SEQ ID NO: 43962 - DNA, 28 bp, synthetic construct
  source 1..28: mol_type = other DNA
cgtcgttgatgtccgccaggttgaaggg

SEQ ID NO: 43963 - DNA, 28 bp, synthetic construct
  source 1..28: mol_type = other DNA
tgtccgccaggttgaagggagccgtcgg

SEQ ID NO: 43964 - DNA, 28 bp, synthetic construct
  source 1..28: mol_type = other DNA
cctccgacggctcccttcaacctggcgg

SEQ ID NO: 43965 - DNA, 28 bp, synthetic construct
  source 1..28: mol_type = other DNA
cgccaggttgaagggagccgtcggaggg

SEQ ID NO: 43966 - DNA, 28 bp, synthetic construct
  source 1..28: mol_type = other DNA
gccaggttgaagggagccgtcggagggg

SEQ ID NO: 43967 - DNA, 28 bp, synthetic construct
  source 1..28: mol_type = other DNA
ccaggttgaagggagccgtcggaggggg

SEQ ID NO: 43968 - DNA, 28 bp, synthetic construct
  source 1..28: mol_type = other DNA
ttgaagggagccgtcggagggggagcgg

SEQ ID NO: 43969 - DNA, 28 bp, synthetic construct
  source 1..28: mol_type = other DNA
ggcagggagtccgctccccctccgacgg

SEQ ID NO: 43970 - DNA, 28 bp, synthetic construct
  source 1..28: mol_type = other DNA
agggggagcggactccctgccatagagg

SEQ ID NO: 43971 - DNA, 28 bp, synthetic construct
  source 1..28: mol_type = other DNA
gggagcggactccctgccatagaggagg

SEQ ID NO: 43972 - DNA, 28 bp, synthetic construct
  source 1..28: mol_type = other DNA
acgggcggaggcctcctctatggcaggg

SEQ ID NO: 43973 - DNA, 28 bp, synthetic construct
  source 1..28: mol_type = other DNA
cacgggcggaggcctcctctatggcagg

SEQ ID NO: 43974 - DNA, 28 bp, synthetic construct
  source 1..28: mol_type = other DNA
gcggcacgggcggaggcctcctctatgg

SEQ ID NO: 43975 - DNA, 28 bp, synthetic construct
  source 1..28: mol_type = other DNA
agaggaggcctccgcccgtgccgcccgg

SEQ ID NO: 43976 - DNA, 28 bp, synthetic construct
  source 1..28: mol_type = other DNA
gcgtggcgccgggcggcacgggcggagg

SEQ ID NO: 43977 - DNA, 28 bp, synthetic construct
  source 1..28: mol_type = other DNA
cgggcgtggcgccgggcggcacgggcgg

SEQ ID NO: 43978 - DNA, 28 bp, synthetic construct
  source 1..28: mol_type = other DNA
cgcccgtgccgcccggcgccacgcccgg

SEQ ID NO: 43979 - DNA, 28 bp, synthetic construct
  source 1..28: mol_type = other DNA
gcccgtgccgcccggcgccacgcccggg

SEQ ID NO: 43980 - DNA, 28 bp, synthetic construct
  source 1..28: mol_type = other DNA
acccgggcgtggcgccgggcggcacggg

SEQ ID NO: 43981 - DNA, 28 bp, synthetic construct
  source 1..28: mol_type = other DNA
gacccgggcgtggcgccgggcggcacgg

SEQ ID NO: 43982 - DNA, 28 bp, synthetic construct
  source 1..28: mol_type = other DNA
ggaacgacccgggcgtggcgccgggcgg

SEQ ID NO: 43983 - DNA, 28 bp, synthetic construct
  source 1..28: mol_type = other DNA
cccggcgccacgcccgggtcgttcccgg

SEQ ID NO: 43984 - DNA, 28 bp, synthetic construct
  source 1..28: mol_type = other DNA
gccgggaacgacccgggcgtggcgccgg

SEQ ID NO: 43985 - DNA, 28 bp, synthetic construct
  source 1..28: mol_type = other DNA
cgccacgcccgggtcgttcccggcccgg

SEQ ID NO: 43986 - DNA, 28 bp, synthetic construct
  source 1..28: mol_type = other DNA
atccgggccgggaacgacccgggcgtgg

SEQ ID NO: 43987 - DNA, 28 bp, synthetic construct
  source 1..28: mol_type = other DNA
cgcccgggtcgttcccggcccggatcgg

SEQ ID NO: 43988 - DNA, 28 bp, synthetic construct
  source 1..28: mol_type = other DNA
atccgatccgggccgggaacgacccggg

SEQ ID NO: 43989 - DNA, 28 bp, synthetic construct
  source 1..28: mol_type = other DNA
tatccgatccgggccgggaacgacccgg

SEQ ID NO: 43990 - DNA, 28 bp, synthetic construct
  source 1..28: mol_type = other DNA
gggtcgttcccggcccggatcggatagg

SEQ ID NO: 43991 - DNA, 28 bp, synthetic construct
  source 1..28: mol_type = other DNA
cagcttcacctatccgatccgggccggg

SEQ ID NO: 43992 - DNA, 28 bp, synthetic construct
  source 1..28: mol_type = other DNA
gcagcttcacctatccgatccgggccgg

SEQ ID NO: 43993 - DNA, 28 bp, synthetic construct
  source 1..28: mol_type = other DNA
gcccggatcggataggtgaagctgcagg

SEQ ID NO: 43994 - DNA, 28 bp, synthetic construct
  source 1..28: mol_type = other DNA
acctgcagcttcacctatccgatccggg

SEQ ID NO: 43995 - DNA, 28 bp, synthetic construct
  source 1..28: mol_type = other DNA
cacctgcagcttcacctatccgatccgg

SEQ ID NO: 43996 - DNA, 28 bp, synthetic construct
  source 1..28: mol_type = other DNA
cggatcggataggtgaagctgcaggtgg

SEQ ID NO: 43997 - DNA, 28 bp, synthetic construct
  source 1..28: mol_type = other DNA
atcggataggtgaagctgcaggtggagg

SEQ ID NO: 43998 - DNA, 28 bp, synthetic construct
  source 1..28: mol_type = other DNA
tcggataggtgaagctgcaggtggaggg

SEQ ID NO: 43999 - DNA, 28 bp, synthetic construct
  source 1..28: mol_type = other DNA
gtgaagctgcaggtggagggcgcgctgg

SEQ ID NO: 44000 - DNA, 28 bp, synthetic construct
  source 1..28: mol_type = other DNA
agctgcaggtggagggcgcgctggcagg

SEQ ID NO: 44001 - DNA, 28 bp, synthetic construct
  source 1..28: mol_type = other DNA
gctgcaggtggagggcgcgctggcaggg

SEQ ID NO: 44002 - DNA, 28 bp, synthetic construct
  source 1..28: mol_type = other DNA
gcgcgctggcagggccgctgctcgacgg

SEQ ID NO: 44003 - DNA, 28 bp, synthetic construct
  source 1..28: mol_type = other DNA
ccgctgctcgacggcgacgacgaagagg

SEQ ID NO: 44004 - DNA, 28 bp, synthetic construct
  source 1..28: mol_type = other DNA
ctgctcgacggcgacgacgaagaggagg

SEQ ID NO: 44005 - DNA, 28 bp, synthetic construct
  source 1..28: mol_type = other DNA
gacgaagaggaggctgacgctgacgagg

SEQ ID NO: 44006 - DNA, 28 bp, synthetic construct
  source 1..28: mol_type = other DNA
gaggaggctgacgctgacgaggacacgg

SEQ ID NO: 44007 - DNA, 28 bp, synthetic construct
  source 1..28: mol_type = other DNA
gaggctgacgctgacgaggacacggtgg

SEQ ID NO: 44008 - DNA, 28 bp, synthetic construct
  source 1..28: mol_type = other DNA
gctgacgctgacgaggacacggtggcgg

SEQ ID NO: 44009 - DNA, 28 bp, synthetic construct
  source 1..28: mol_type = other DNA
aggacacggtggcggccactgactccgg

SEQ ID NO: 44010 - DNA, 28 bp, synthetic construct
  source 1..28: mol_type = other DNA
acacggtggcggccactgactccggagg

SEQ ID NO: 44011 - DNA, 28 bp, synthetic construct
  source 1..28: mol_type = other DNA
ggtggcggccactgactccggaggatgg

SEQ ID NO: 44012 - DNA, 28 bp, synthetic construct
  source 1..28: mol_type = other DNA
gtggcggccactgactccggaggatggg

SEQ ID NO: 44013 - DNA, 28 bp, synthetic construct
  source 1..28: mol_type = other DNA
tcgctgacccatcctccggagtcagtgg

SEQ ID NO: 44014 - DNA, 28 bp, synthetic construct
  source 1..28: mol_type = other DNA
gactccggaggatgggtcagcgaattgg

SEQ ID NO: 44015 - DNA, 28 bp, synthetic construct
  source 1..28: mol_type = other DNA
ctctccaattcgctgacccatcctccgg

SEQ ID NO: 44016 - DNA, 28 bp, synthetic construct
  source 1..28: mol_type = other DNA
cagcgaattggagagaataaagtccagg

SEQ ID NO: 44017 - DNA, 28 bp, synthetic construct
  source 1..28: mol_type = other DNA
attggagagaataaagtccaggtccagg

SEQ ID NO: 44018 - DNA, 28 bp, synthetic construct
  source 1..28: mol_type = other DNA
gaggagttcaacgatctcctggacctgg

SEQ ID NO: 44019 - DNA, 28 bp, synthetic construct
  source 1..28: mol_type = other DNA
aggtccaggagatcgttgaactcctcgg

SEQ ID NO: 44020 - DNA, 28 bp, synthetic construct
  source 1..28: mol_type = other DNA
gagaccgaggagttcaacgatctcctgg

SEQ ID NO: 44021 - DNA, 28 bp, synthetic construct
  source 1..28: mol_type = other DNA
cgttgaactcctcggtctctctccgagg

SEQ ID NO: 44022 - DNA, 28 bp, synthetic construct
  source 1..28: mol_type = other DNA
gaactcctcggtctctctccgaggtagg

SEQ ID NO: 44023 - DNA, 28 bp, synthetic construct
  source 1..28: mol_type = other DNA
aactcctcggtctctctccgaggtaggg

SEQ ID NO: 44024 - DNA, 28 bp, synthetic construct
  source 1..28: mol_type = other DNA
actcctcggtctctctccgaggtagggg

SEQ ID NO: 44025 - DNA, 28 bp, synthetic construct
  source 1..28: mol_type = other DNA
gcgcccctacctcggagagagaccgagg

SEQ ID NO: 44026 - DNA, 28 bp, synthetic construct
  source 1..28: mol_type = other DNA
ggtctctctccgaggtaggggcgccagg

SEQ ID NO: 44027 - DNA, 28 bp, synthetic construct
  source 1..28: mol_type = other DNA
cggtagcaacctggcgcccctacctcgg

SEQ ID NO: 44028 - DNA, 28 bp, synthetic construct
  source 1..28: mol_type = other DNA
ggtgcggcttgcggcggtagcaacctgg

SEQ ID NO: 44029 - DNA, 28 bp, synthetic construct
  source 1..28: mol_type = other DNA
aggttgctaccgccgcaagccgcaccgg

SEQ ID NO: 44030 - DNA, 28 bp, synthetic construct
  source 1..28: mol_type = other DNA
gcggcggagccggtgcggcttgcggcgg

SEQ ID NO: 44031 - DNA, 28 bp, synthetic construct
  source 1..28: mol_type = other DNA
agagcggcggagccggtgcggcttgcgg

SEQ ID NO: 44032 - DNA, 28 bp, synthetic construct
  source 1..28: mol_type = other DNA
agccgcaccggctccgccgctctccagg

SEQ ID NO: 44033 - DNA, 28 bp, synthetic construct
  source 1..28: mol_type = other DNA
gacctggagagcggcggagccggtgcgg

SEQ ID NO: 44034 - DNA, 28 bp, synthetic construct
  source 1..28: mol_type = other DNA
ccacagacctggagagcggcggagccgg

SEQ ID NO: 44035 - DNA, 28 bp, synthetic construct
  source 1..28: mol_type = other DNA
ccgccgctctccaggtctgtggccacgg

SEQ ID NO: 44036 - DNA, 28 bp, synthetic construct
  source 1..28: mol_type = other DNA
cgaccgtggccacagacctggagagcgg

SEQ ID NO: 44037 - DNA, 28 bp, synthetic construct
  source 1..28: mol_type = other DNA
gcggcggcgaccgtggccacagacctgg

SEQ ID NO: 44038 - DNA, 28 bp, synthetic construct
  source 1..28: mol_type = other DNA
gtctgtggccacggtcgccgccgccagg

SEQ ID NO: 44039 - DNA, 28 bp, synthetic construct
  source 1..28: mol_type = other DNA
gccacggtcgccgccgccaggtcatagg

SEQ ID NO: 44040 - DNA, 28 bp, synthetic construct
  source 1..28: mol_type = other DNA
ccctatgacctggcggcggcgaccgtgg

SEQ ID NO: 44041 - DNA, 28 bp, synthetic construct
  source 1..28: mol_type = other DNA
cacggtcgccgccgccaggtcatagggg

SEQ ID NO: 44042 - DNA, 28 bp, synthetic construct
  source 1..28: mol_type = other DNA
ggtcgccgccgccaggtcataggggcgg

SEQ ID NO: 44043 - DNA, 28 bp, synthetic construct
  source 1..28: mol_type = other DNA
gccgccgccaggtcataggggcggccgg

SEQ ID NO: 44044 - DNA, 28 bp, synthetic construct
  source 1..28: mol_type = other DNA
ccgccgccaggtcataggggcggccggg

SEQ ID NO: 44045 - DNA, 28 bp, synthetic construct
  source 1..28: mol_type = other DNA
cttcccggccgcccctatgacctggcgg

SEQ ID NO: 44046 - DNA, 28 bp, synthetic construct
  source 1..28: mol_type = other DNA
gtgcttcccggccgcccctatgacctgg

SEQ ID NO: 44047 - DNA, 28 bp, synthetic construct
  source 1..28: mol_type = other DNA
ggtcataggggcggccgggaagcactgg

SEQ ID NO: 44048 - DNA, 28 bp, synthetic construct
  source 1..28: mol_type = other DNA
gtcataggggcggccgggaagcactggg

SEQ ID NO: 44049 - DNA, 28 bp, synthetic construct
  source 1..28: mol_type = other DNA
tcataggggcggccgggaagcactgggg

SEQ ID NO: 44050 - DNA, 28 bp, synthetic construct
  source 1..28: mol_type = other DNA
cataggggcggccgggaagcactggggg

SEQ ID NO: 44051 - DNA, 28 bp, synthetic construct
  source 1..28: mol_type = other DNA
tgaagcgacttcccccagtgcttcccgg

SEQ ID NO: 44052 - DNA, 28 bp, synthetic construct
  source 1..28: mol_type = other DNA
aagcactgggggaagtcgcttcatgtgg

SEQ ID NO: 44053 - DNA, 28 bp, synthetic construct
  source 1..28: mol_type = other DNA
agcactgggggaagtcgcttcatgtggg

SEQ ID NO: 44054 - DNA, 28 bp, synthetic construct
  source 1..28: mol_type = other DNA
gggagagctcctcccgccagcgctgcgg

SEQ ID NO: 44055 - DNA, 28 bp, synthetic construct
  source 1..28: mol_type = other DNA
ggagagctcctcccgccagcgctgcggg

SEQ ID NO: 44056 - DNA, 28 bp, synthetic construct
  source 1..28: mol_type = other DNA
gagagctcctcccgccagcgctgcgggg

SEQ ID NO: 44057 - DNA, 28 bp, synthetic construct
  source 1..28: mol_type = other DNA
ctcctcccgccagcgctgcggggacagg

SEQ ID NO: 44058 - DNA, 28 bp, synthetic construct
  source 1..28: mol_type = other DNA
tcctcccgccagcgctgcggggacaggg

SEQ ID NO: 44059 - DNA, 28 bp, synthetic construct
  source 1..28: mol_type = other DNA
gccctgtccccgcagcgctggcgggagg

SEQ ID NO: 44060 - DNA, 28 bp, synthetic construct
  source 1..28: mol_type = other DNA
tcccgccagcgctgcggggacagggcgg

SEQ ID NO: 44061 - DNA, 28 bp, synthetic construct
  source 1..28: mol_type = other DNA
cccgccagcgctgcggggacagggcggg

SEQ ID NO: 44062 - DNA, 28 bp, synthetic construct
  source 1..28: mol_type = other DNA
tcccgccctgtccccgcagcgctggcgg

SEQ ID NO: 44063 - DNA, 28 bp, synthetic construct
  source 1..28: mol_type = other DNA
ctctcccgccctgtccccgcagcgctgg

SEQ ID NO: 44064 - DNA, 28 bp, synthetic construct
  source 1..28: mol_type = other DNA
ggacagggcgggagagacctgtcagtgg

SEQ ID NO: 44065 - DNA, 28 bp, synthetic construct
  source 1..28: mol_type = other DNA
cagggcgggagagacctgtcagtggtgg

SEQ ID NO: 44066 - DNA, 28 bp, synthetic construct
  source 1..28: mol_type = other DNA
gtggcaacaggggaccaccactgacagg

SEQ ID NO: 44067 - DNA, 28 bp, synthetic construct
  source 1..28: mol_type = other DNA
acgtcagtatgtcgggtggcaacagggg

SEQ ID NO: 44068 - DNA, 28 bp, synthetic construct
  source 1..28: mol_type = other DNA
cacgtcagtatgtcgggtggcaacaggg

SEQ ID NO: 44069 - DNA, 28 bp, synthetic construct
  source 1..28: mol_type = other DNA
gcacgtcagtatgtcgggtggcaacagg

SEQ ID NO: 44070 - DNA, 28 bp, synthetic construct
  source 1..28: mol_type = other DNA
gttgccacccgacatactgacgtgctgg

SEQ ID NO: 44071 - DNA, 28 bp, synthetic construct
  source 1..28: mol_type = other DNA
gccacccgacatactgacgtgctggcgg

SEQ ID NO: 44072 - DNA, 28 bp, synthetic construct
  source 1..28: mol_type = other DNA
cccgccagcacgtcagtatgtcgggtgg

SEQ ID NO: 44073 - DNA, 28 bp, synthetic construct
  source 1..28: mol_type = other DNA
tggcccgccagcacgtcagtatgtcggg

SEQ ID NO: 44074 - DNA, 28 bp, synthetic construct
  source 1..28: mol_type = other DNA
gtggcccgccagcacgtcagtatgtcgg

SEQ ID NO: 44075 - DNA, 28 bp, synthetic construct
  source 1..28: mol_type = other DNA
catgtctgggcggtgcagtcgcgcgtgg

SEQ ID NO: 44076 - DNA, 28 bp, synthetic construct
  source 1..28: mol_type = other DNA
cacgcgcgactgcaccgcccagacatgg

SEQ ID NO: 44077 - DNA, 28 bp, synthetic construct
  source 1..28: mol_type = other DNA
acgcgcgactgcaccgcccagacatggg

SEQ ID NO: 44078 - DNA, 28 bp, synthetic construct
  source 1..28: mol_type = other DNA
cgcgcgactgcaccgcccagacatgggg

SEQ ID NO: 44079 - DNA, 28 bp, synthetic construct
  source 1..28: mol_type = other DNA
gactgcaccgcccagacatggggactgg

SEQ ID NO: 44080 - DNA, 28 bp, synthetic construct
  source 1..28: mol_type = other DNA
caccgcccagacatggggactggtcagg

SEQ ID NO: 44081 - DNA, 28 bp, synthetic construct
  source 1..28: mol_type = other DNA
tgcctgaccagtccccatgtctgggcgg

SEQ ID NO: 44082 - DNA, 28 bp, synthetic construct
  source 1..28: mol_type = other DNA
gcccagacatggggactggtcaggcagg

SEQ ID NO: 44083 - DNA, 28 bp, synthetic construct
  source 1..28: mol_type = other DNA
tcctgcctgaccagtccccatgtctggg

SEQ ID NO: 44084 - DNA, 28 bp, synthetic construct
  source 1..28: mol_type = other DNA
ttcctgcctgaccagtccccatgtctgg

SEQ ID NO: 44085 - DNA, 28 bp, synthetic construct
  source 1..28: mol_type = other DNA
acgagggtaaggagcggccaccgcgcgg

SEQ ID NO: 44086 - DNA, 28 bp, synthetic construct
  source 1..28: mol_type = other DNA
gtggccgctccttaccctcgttcagtgg

SEQ ID NO: 44087 - DNA, 28 bp, synthetic construct
  source 1..28: mol_type = other DNA
agagccactgaacgagggtaaggagcgg

SEQ ID NO: 44088 - DNA, 28 bp, synthetic construct
  source 1..28: mol_type = other DNA
ctccttaccctcgttcagtggctcttgg

SEQ ID NO: 44089 - DNA, 28 bp, synthetic construct
  source 1..28: mol_type = other DNA
caccaagagccactgaacgagggtaagg

SEQ ID NO: 44090 - DNA, 28 bp, synthetic construct
  source 1..28: mol_type = other DNA
ggggtcaccaagagccactgaacgaggg

SEQ ID NO: 44091 - DNA, 28 bp, synthetic construct
  source 1..28: mol_type = other DNA
tggggtcaccaagagccactgaacgagg

SEQ ID NO: 44092 - DNA, 28 bp, synthetic construct
  source 1..28: mol_type = other DNA
cgttcagtggctcttggtgaccccaagg

SEQ ID NO: 44093 - DNA, 28 bp, synthetic construct
  source 1..28: mol_type = other DNA
tgtggtgggggcgggcggagccttgggg

SEQ ID NO: 44094 - DNA, 28 bp, synthetic construct
  source 1..28: mol_type = other DNA
gtgtggtgggggcgggcggagccttggg

SEQ ID NO: 44095 - DNA, 28 bp, synthetic construct
  source 1..28: mol_type = other DNA
ggtgtggtgggggcgggcggagccttgg

SEQ ID NO: 44096 - DNA, 28 bp, synthetic construct
  source 1..28: mol_type = other DNA
ttttcgtgggtgtggtgggggcgggcgg

SEQ ID NO: 44097 - DNA, 28 bp, synthetic construct
  source 1..28: mol_type = other DNA
gggttttcgtgggtgtggtgggggcggg

SEQ ID NO: 44098 - DNA, 28 bp, synthetic construct
  source 1..28: mol_type = other DNA
tgggttttcgtgggtgtggtgggggcgg

SEQ ID NO: 44099 - DNA, 28 bp, synthetic construct
  source 1..28: mol_type = other DNA
cggtgggttttcgtgggtgtggtggggg

SEQ ID NO: 44100 - DNA, 28 bp, synthetic construct
  source 1..28: mol_type = other DNA
ccccaccacacccacgaaaacccaccgg

SEQ ID NO: 44101 - DNA, 28 bp, synthetic construct
  source 1..28: mol_type = other DNA
cccaccacacccacgaaaacccaccggg

SEQ ID NO: 44102 - DNA, 28 bp, synthetic construct
  source 1..28: mol_type = other DNA
gcccggtgggttttcgtgggtgtggtgg

SEQ ID NO: 44103 - DNA, 28 bp, synthetic construct
  source 1..28: mol_type = other DNA
aacgcccggtgggttttcgtgggtgtgg

SEQ ID NO: 44104 - DNA, 28 bp, synthetic construct
  source 1..28: mol_type = other DNA
cccacgaaaacccaccgggcgttcccgg

SEQ ID NO: 44105 - DNA, 28 bp, synthetic construct
  source 1..28: mol_type = other DNA
gccgggaacgcccggtgggttttcgtgg

SEQ ID NO: 44106 - DNA, 28 bp, synthetic construct
  source 1..28: mol_type = other DNA
acgaaaacccaccgggcgttcccggcgg

SEQ ID NO: 44107 - DNA, 28 bp, synthetic construct
  source 1..28: mol_type = other DNA
aacccaccgggcgttcccggcggcccgg

SEQ ID NO: 44108 - DNA, 28 bp, synthetic construct
  source 1..28: mol_type = other DNA
ctccgggccgccgggaacgcccggtggg

SEQ ID NO: 44109 - DNA, 28 bp, synthetic construct
  source 1..28: mol_type = other DNA
gctccgggccgccgggaacgcccggtgg

SEQ ID NO: 44110 - DNA, 28 bp, synthetic construct
  source 1..28: mol_type = other DNA
atcgctccgggccgccgggaacgcccgg

SEQ ID NO: 44111 - DNA, 28 bp, synthetic construct
  source 1..28: mol_type = other DNA
aacgtgagtatcgctccgggccgccggg

SEQ ID NO: 44112 - DNA, 28 bp, synthetic construct
  source 1..28: mol_type = other DNA
taacgtgagtatcgctccgggccgccgg

SEQ ID NO: 44113 - DNA, 28 bp, synthetic construct
  source 1..28: mol_type = other DNA
ggcccggagcgatactcacgttattcgg

SEQ ID NO: 44114 - DNA, 28 bp, synthetic construct
  source 1..28: mol_type = other DNA
gcccggagcgatactcacgttattcggg

SEQ ID NO: 44115 - DNA, 28 bp, synthetic construct
  source 1..28: mol_type = other DNA
ccccgaataacgtgagtatcgctccggg

SEQ ID NO: 44116 - DNA, 28 bp, synthetic construct
  source 1..28: mol_type = other DNA
gccccgaataacgtgagtatcgctccgg

SEQ ID NO: 44117 - DNA, 28 bp, synthetic construct
  source 1..28: mol_type = other DNA
gaagggagaagacactgcgtcaagcagg

SEQ ID NO: 44118 - DNA, 28 bp, synthetic construct
  source 1..28: mol_type = other DNA
gacgcagtgtcttctcccttcccgccgg

SEQ ID NO: 44119 - DNA, 28 bp, synthetic construct
  source 1..28: mol_type = other DNA
acgcagtgtcttctcccttcccgccggg

SEQ ID NO: 44120 - DNA, 28 bp, synthetic construct
  source 1..28: mol_type = other DNA
acgttcgcgtctggcccggcgggaaggg

SEQ ID NO: 44121 - DNA, 28 bp, synthetic construct
  source 1..28: mol_type = other DNA
cacgttcgcgtctggcccggcgggaagg

SEQ ID NO: 44122 - DNA, 28 bp, synthetic construct
  source 1..28: mol_type = other DNA
cttcccgccgggccagacgcgaacgtgg

SEQ ID NO: 44123 - DNA, 28 bp, synthetic construct
  source 1..28: mol_type = other DNA
tctccacgttcgcgtctggcccggcggg

SEQ ID NO: 44124 - DNA, 28 bp, synthetic construct
  source 1..28: mol_type = other DNA
ttctccacgttcgcgtctggcccggcgg

SEQ ID NO: 44125 - DNA, 28 bp, synthetic construct
  source 1..28: mol_type = other DNA
tctttctccacgttcgcgtctggcccgg

SEQ ID NO: 44126 - DNA, 28 bp, synthetic construct
  source 1..28: mol_type = other DNA
ggccagacgcgaacgtggagaaagatgg

SEQ ID NO: 44127 - DNA, 28 bp, synthetic construct
  source 1..28: mol_type = other DNA
gccagacgcgaacgtggagaaagatggg

SEQ ID NO: 44128 - DNA, 28 bp, synthetic construct
  source 1..28: mol_type = other DNA
tcccatctttctccacgttcgcgtctgg

SEQ ID NO: 44129 - DNA, 28 bp, synthetic construct
  source 1..28: mol_type = other DNA
cgctgacagccatgtcagactcgccagg

SEQ ID NO: 44130 - DNA, 28 bp, synthetic construct
  source 1..28: mol_type = other DNA
tgacagccatgtcagactcgccaggtgg

SEQ ID NO: 44131 - DNA, 28 bp, synthetic construct
  source 1..28: mol_type = other DNA
aggcagccacctggcgagtctgacatgg

SEQ ID NO: 44132 - DNA, 28 bp, synthetic construct
  source 1..28: mol_type = other DNA
ctcgccaggtggctgcctgcgagcaagg

SEQ ID NO: 44133 - DNA, 28 bp, synthetic construct
  source 1..28: mol_type = other DNA
cctgccttgctcgcaggcagccacctgg

SEQ ID NO: 44134 - DNA, 28 bp, synthetic construct
  source 1..28: mol_type = other DNA
caggtggctgcctgcgagcaaggcaggg

SEQ ID NO: 44135 - DNA, 28 bp, synthetic construct
  source 1..28: mol_type = other DNA
ggctgcctgcgagcaaggcagggagcgg

SEQ ID NO: 44136 - DNA, 28 bp, synthetic construct
  source 1..28: mol_type = other DNA
tgtctccgctccctgccttgctcgcagg

SEQ ID NO: 44137 - DNA, 28 bp, synthetic construct
  source 1..28: mol_type = other DNA
tgcgagcaaggcagggagcggagacagg

SEQ ID NO: 44138 - DNA, 28 bp, synthetic construct
  source 1..28: mol_type = other DNA
ggcagggagcggagacaggagagtcagg

SEQ ID NO: 44139 - DNA, 28 bp, synthetic construct
  source 1..28: mol_type = other DNA
gcagggagcggagacaggagagtcaggg

SEQ ID NO: 44140 - DNA, 28 bp, synthetic construct
  source 1..28: mol_type = other DNA
cagggagcggagacaggagagtcagggg

SEQ ID NO: 44141 - DNA, 28 bp, synthetic construct
  source 1..28: mol_type = other DNA
ggagcggagacaggagagtcaggggcgg

SEQ ID NO: 44142 - DNA, 28 bp, synthetic construct
  source 1..28: mol_type = other DNA
agacaggagagtcaggggcggctttcgg

SEQ ID NO: 44143 - DNA, 28 bp, synthetic construct
  source 1..28: mol_type = other DNA
caggggcggctttcggccgtcgttccgg

SEQ ID NO: 44144 - DNA, 28 bp, synthetic construct
  source 1..28: mol_type = other DNA
cggccgtcgttccggcgcgtcccaccgg

SEQ ID NO: 44145 - DNA, 28 bp, synthetic construct
  source 1..28: mol_type = other DNA
ggaccggtgggacgcgccggaacgacgg

SEQ ID NO: 44146 - DNA, 28 bp, synthetic construct
  source 1..28: mol_type = other DNA
aggggtgaggaccggtgggacgcgccgg

SEQ ID NO: 44147 - DNA, 28 bp, synthetic construct
  source 1..28: mol_type = other DNA
ggagcagggaggggtgaggaccggtggg

SEQ ID NO: 44148 - DNA, 28 bp, synthetic construct
  source 1..28: mol_type = other DNA
gggagcagggaggggtgaggaccggtgg

SEQ ID NO: 44149 - DNA, 28 bp, synthetic construct
  source 1..28: mol_type = other DNA
gctgggagcagggaggggtgaggaccgg

SEQ ID NO: 44150 - DNA, 28 bp, synthetic construct
  source 1..28: mol_type = other DNA
gcggcgctgggagcagggaggggtgagg

SEQ ID NO: 44151 - DNA, 28 bp, synthetic construct
  source 1..28: mol_type = other DNA
ggcgcgcggcgctgggagcagggagggg

SEQ ID NO: 44152 - DNA, 28 bp, synthetic construct
  source 1..28: mol_type = other DNA
aggcgcgcggcgctgggagcagggaggg

SEQ ID NO: 44153 - DNA, 28 bp, synthetic construct
  source 1..28: mol_type = other DNA
gaggcgcgcggcgctgggagcagggagg

SEQ ID NO: 44154 - DNA, 28 bp, synthetic construct
  source 1..28: mol_type = other DNA
ggtgaggcgcgcggcgctgggagcaggg

SEQ ID NO: 44155 - DNA, 28 bp, synthetic construct
  source 1..28: mol_type = other DNA
aggtgaggcgcgcggcgctgggagcagg

SEQ ID NO: 44156 - DNA, 28 bp, synthetic construct
  source 1..28: mol_type = other DNA
tgaggtaggtgaggcgcgcggcgctggg

SEQ ID NO: 44157 - DNA, 28 bp, synthetic construct
  source 1..28: mol_type = other DNA
atgaggtaggtgaggcgcgcggcgctgg

SEQ ID NO: 44158 - DNA, 28 bp, synthetic construct
  source 1..28: mol_type = other DNA
acattaatgaggtaggtgaggcgcgcgg

SEQ ID NO: 44159 - DNA, 28 bp, synthetic construct
  source 1..28: mol_type = other DNA
gcgcgcctcacctacctcattaatgtgg

SEQ ID NO: 44160 - DNA, 28 bp, synthetic construct
  source 1..28: mol_type = other DNA
cgcgcctcacctacctcattaatgtggg

SEQ ID NO: 44161 - DNA, 28 bp, synthetic construct
  source 1..28: mol_type = other DNA
gcgcctcacctacctcattaatgtgggg

SEQ ID NO: 44162 - DNA, 28 bp, synthetic construct
  source 1..28: mol_type = other DNA
cgcctcacctacctcattaatgtggggg

SEQ ID NO: 44163 - DNA, 28 bp, synthetic construct
  source 1..28: mol_type = other DNA
ggcccccacattaatgaggtaggtgagg

SEQ ID NO: 44164 - DNA, 28 bp, synthetic construct
  source 1..28: mol_type = other DNA
ttctgggcccccacattaatgaggtagg

SEQ ID NO: 44165 - DNA, 28 bp, synthetic construct
  source 1..28: mol_type = other DNA
tacctcattaatgtgggggcccagaagg

SEQ ID NO: 44166 - DNA, 28 bp, synthetic construct
  source 1..28: mol_type = other DNA
gaccttctgggcccccacattaatgagg

SEQ ID NO: 44167 - DNA, 28 bp, synthetic construct
  source 1..28: mol_type = other DNA
ttaatgtgggggcccagaaggtcctcgg

SEQ ID NO: 44168 - DNA, 28 bp, synthetic construct
  source 1..28: mol_type = other DNA
tgcttcgggctgccgaggaccttctggg

SEQ ID NO: 44169 - DNA, 28 bp, synthetic construct
  source 1..28: mol_type = other DNA
ctgcttcgggctgccgaggaccttctgg

SEQ ID NO: 44170 - DNA, 28 bp, synthetic construct
  source 1..28: mol_type = other DNA
aaggtcctcggcagcccgaagcagctgg

SEQ ID NO: 44171 - DNA, 28 bp, synthetic construct
  source 1..28: mol_type = other DNA
aggtcctcggcagcccgaagcagctggg

SEQ ID NO: 44172 - DNA, 28 bp, synthetic construct
  source 1..28: mol_type = other DNA
ggtcctcggcagcccgaagcagctgggg

SEQ ID NO: 44173 - DNA, 28 bp, synthetic construct
  source 1..28: mol_type = other DNA
gtgccccagctgcttcgggctgccgagg

SEQ ID NO: 44174 - DNA, 28 bp, synthetic construct
  source 1..28: mol_type = other DNA
ggggttcaggtgccccagctgcttcggg

SEQ ID NO: 44175 - DNA, 28 bp, synthetic construct
  source 1..28: mol_type = other DNA
tggggttcaggtgccccagctgcttcgg

SEQ ID NO: 44176 - DNA, 28 bp, synthetic construct
  source 1..28: mol_type = other DNA
cttctcttcgttgactttggggttcagg

SEQ ID NO: 44177 - DNA, 28 bp, synthetic construct
  source 1..28: mol_type = other DNA
tcgtttcttctcttcgttgactttgggg

SEQ ID NO: 44178 - DNA, 28 bp, synthetic construct
  source 1..28: mol_type = other DNA
ttcgtttcttctcttcgttgactttggg

SEQ ID NO: 44179 - DNA, 28 bp, synthetic construct
  source 1..28: mol_type = other DNA
cttcgtttcttctcttcgttgactttgg

SEQ ID NO: 44180 - DNA, 28 bp, synthetic construct
  source 1..28: mol_type = other DNA
gaagccaaaacccaaaaccccaaattgg

SEQ ID NO: 44181 - DNA, 28 bp, synthetic construct
  source 1..28: mol_type = other DNA
tcggccaatttggggttttgggttttgg

SEQ ID NO: 44182 - DNA, 28 bp, synthetic construct
  source 1..28: mol_type = other DNA
aggatctcggccaatttggggttttggg

SEQ ID NO: 44183 - DNA, 28 bp, synthetic construct
  source 1..28: mol_type = other DNA
aaggatctcggccaatttggggttttgg

SEQ ID NO: 44184 - DNA, 28 bp, synthetic construct
  source 1..28: mol_type = other DNA
aagaagaaggatctcggccaatttgggg

SEQ ID NO: 44185 - DNA, 28 bp, synthetic construct
  source 1..28: mol_type = other DNA
aaagaagaaggatctcggccaatttggg

SEQ ID NO: 44186 - DNA, 28 bp, synthetic construct
  source 1..28: mol_type = other DNA
caaagaagaaggatctcggccaatttgg

SEQ ID NO: 44187 - DNA, 28 bp, synthetic construct
  source 1..28: mol_type = other DNA
caaattggccgagatccttcttctttgg

SEQ ID NO: 44188 - DNA, 28 bp, synthetic construct
  source 1..28: mol_type = other DNA
tatttaatccaaagaagaaggatctcgg

SEQ ID NO: 44189 - DNA, 28 bp, synthetic construct
  source 1..28: mol_type = other DNA
caagttatatttaatccaaagaagaagg

SEQ ID NO: 44190 - DNA, 28 bp, synthetic construct
  source 1..28: mol_type = other DNA
cttcttctttggattaaatataacttgg

SEQ ID NO: 44191 - DNA, 28 bp, synthetic construct
  source 1..28: mol_type = other DNA
cttttctaagaacttttgtatacaaagg

SEQ ID NO: 44192 - DNA, 28 bp, synthetic construct
  source 1..28: mol_type = other DNA
taaacgcaaaaatagacaatcagcaagg

SEQ ID NO: 44193 - DNA, 28 bp, synthetic construct
  source 1..28: mol_type = other DNA
tagacaatcagcaaggcgagtaagtagg

SEQ ID NO: 44194 - DNA, 28 bp, synthetic construct
  source 1..28: mol_type = other DNA
aatcagcaaggcgagtaagtaggtccgg

SEQ ID NO: 44195 - DNA, 28 bp, synthetic construct
  source 1..28: mol_type = other DNA
cagcaaggcgagtaagtaggtccggtgg

SEQ ID NO: 44196 - DNA, 28 bp, synthetic construct
  source 1..28: mol_type = other DNA
aaggcgagtaagtaggtccggtggccgg

SEQ ID NO: 44197 - DNA, 28 bp, synthetic construct
  source 1..28: mol_type = other DNA
aggcgagtaagtaggtccggtggccggg

SEQ ID NO: 44198 - DNA, 28 bp, synthetic construct
  source 1..28: mol_type = other DNA
gtggaagagagcgcagcccggccaccgg

SEQ ID NO: 44199 - DNA, 28 bp, synthetic construct
  source 1..28: mol_type = other DNA
ctgctgagtggaagagagcgcagcccgg

SEQ ID NO: 44200 - DNA, 28 bp, synthetic construct
  source 1..28: mol_type = other DNA
gacagtggtgggggacgctgctgagtgg

SEQ ID NO: 44201 - DNA, 28 bp, synthetic construct
  source 1..28: mol_type = other DNA
tcagcagcgtcccccaccactgtcgcgg

SEQ ID NO: 44202 - DNA, 28 bp, synthetic construct
  source 1..28: mol_type = other DNA
ctcgaggcgaccgcgacagtggtggggg

SEQ ID NO: 44203 - DNA, 28 bp, synthetic construct
  source 1..28: mol_type = other DNA
actcgaggcgaccgcgacagtggtgggg

SEQ ID NO: 44204 - DNA, 28 bp, synthetic construct
  source 1..28: mol_type = other DNA
cactcgaggcgaccgcgacagtggtggg

SEQ ID NO: 44205 - DNA, 28 bp, synthetic construct
  source 1..28: mol_type = other DNA
gcactcgaggcgaccgcgacagtggtgg

SEQ ID NO: 44206 - DNA, 28 bp, synthetic construct
  source 1..28: mol_type = other DNA
gcagcactcgaggcgaccgcgacagtgg

SEQ ID NO: 44207 - DNA, 28 bp, synthetic construct
  source 1..28: mol_type = other DNA
gtcgcggtcgcctcgagtgctgccgtgg

SEQ ID NO: 44208 - DNA, 28 bp, synthetic construct
  source 1..28: mol_type = other DNA
tcgcggtcgcctcgagtgctgccgtggg

SEQ ID NO: 44209 - DNA, 28 bp, synthetic construct
  source 1..28: mol_type = other DNA
tcgcctcgagtgctgccgtgggcgcagg

SEQ ID NO: 44210 - DNA, 28 bp, synthetic construct
  source 1..28: mol_type = other DNA
cgcctcgagtgctgccgtgggcgcaggg

SEQ ID NO: 44211 - DNA, 28 bp, synthetic construct
  source 1..28: mol_type = other DNA
gcctcgagtgctgccgtgggcgcagggg

SEQ ID NO: 44212 - DNA, 28 bp, synthetic construct
  source 1..28: mol_type = other DNA
gcccctgcgcccacggcagcactcgagg

SEQ ID NO: 44213 - DNA, 28 bp, synthetic construct
  source 1..28: mol_type = other DNA
agtgctgccgtgggcgcaggggctgtgg

SEQ ID NO: 44214 - DNA, 28 bp, synthetic construct
  source 1..28: mol_type = other DNA
ctgccgtgggcgcaggggctgtggccgg

SEQ ID NO: 44215 - DNA, 28 bp, synthetic construct
  source 1..28: mol_type = other DNA
tgccgtgggcgcaggggctgtggccggg

SEQ ID NO: 44216 - DNA, 28 bp, synthetic construct
  source 1..28: mol_type = other DNA
gccgtgggcgcaggggctgtggccgggg

SEQ ID NO: 44217 - DNA, 28 bp, synthetic construct
  source 1..28: mol_type = other DNA
gccccggccacagcccctgcgcccacgg

SEQ ID NO: 44218 - DNA, 28 bp, synthetic construct
  source 1..28: mol_type = other DNA
gtgggcgcaggggctgtggccggggcgg

SEQ ID NO: 44219 - DNA, 28 bp, synthetic construct
  source 1..28: mol_type = other DNA
ggcgcaggggctgtggccggggcggtgg

SEQ ID NO: 44220 - DNA, 28 bp, synthetic construct
  source 1..28: mol_type = other DNA
gcgcaggggctgtggccggggcggtggg

SEQ ID NO: 44221 - DNA, 28 bp, synthetic construct
  source 1..28: mol_type = other DNA
caggggctgtggccggggcggtgggcgg

SEQ ID NO: 44222 - DNA, 28 bp, synthetic construct
  source 1..28: mol_type = other DNA
aggggctgtggccggggcggtgggcggg

SEQ ID NO: 44223 - DNA, 28 bp, synthetic construct
  source 1..28: mol_type = other DNA
ggctgtggccggggcggtgggcgggcgg

SEQ ID NO: 44224 - DNA, 28 bp, synthetic construct
  source 1..28: mol_type = other DNA
tggcggcaccgcccgcccaccgccccgg

SEQ ID NO: 44225 - DNA, 28 bp, synthetic construct
  source 1..28: mol_type = other DNA
ggggcggtgggcgggcggtgccgccagg

SEQ ID NO: 44226 - DNA, 28 bp, synthetic construct
  source 1..28: mol_type = other DNA
ggcgggcggtgccgccaggtgagactgg

SEQ ID NO: 44227 - DNA, 28 bp, synthetic construct
  source 1..28: mol_type = other DNA
tgccgccaggtgagactggctgccgtgg

SEQ ID NO: 44228 - DNA, 28 bp, synthetic construct
  source 1..28: mol_type = other DNA
cgccacggcagccagtctcacctggcgg

SEQ ID NO: 44229 - DNA, 28 bp, synthetic construct
  source 1..28: mol_type = other DNA
ccgcgccacggcagccagtctcacctgg

SEQ ID NO: 44230 - DNA, 28 bp, synthetic construct
  source 1..28: mol_type = other DNA
gctgccgtggcgcggagctgcgaactgg

SEQ ID NO: 44231 - DNA, 28 bp, synthetic construct
  source 1..28: mol_type = other DNA
ccgaccagttcgcagctccgcgccacgg

SEQ ID NO: 44232 - DNA, 28 bp, synthetic construct
  source 1..28: mol_type = other DNA
tggcgcggagctgcgaactggtcggcgg

SEQ ID NO: 44233 - DNA, 28 bp, synthetic construct
  source 1..28: mol_type = other DNA
gagctgcgaactggtcggcggcgcaagg

SEQ ID NO: 44234 - DNA, 28 bp, synthetic construct
  source 1..28: mol_type = other DNA
gcgaactggtcggcggcgcaaggcgcgg

SEQ ID NO: 44235 - DNA, 28 bp, synthetic construct
  source 1..28: mol_type = other DNA
ggtcggcggcgcaaggcgcggactccgg

SEQ ID NO: 44236 - DNA, 28 bp, synthetic construct
  source 1..28: mol_type = other DNA
aaggcgcggactccggtgagttgtgtgg

SEQ ID NO: 44237 - DNA, 28 bp, synthetic construct
  source 1..28: mol_type = other DNA
tccggtgagttgtgtggagcgcgcgcgg

SEQ ID NO: 44238 - DNA, 28 bp, synthetic construct
  source 1..28: mol_type = other DNA
gccgcgcgcgctccacacaactcaccgg

SEQ ID NO: 44239 - DNA, 28 bp, synthetic construct
  source 1..28: mol_type = other DNA
gagttgtgtggagcgcgcgcggccatgg

SEQ ID NO: 44240 - DNA, 28 bp, synthetic construct
  source 1..28: mol_type = other DNA
agttgtgtggagcgcgcgcggccatggg

SEQ ID NO: 44241 - DNA, 28 bp, synthetic construct
  source 1..28: mol_type = other DNA
tgtggagcgcgcgcggccatgggcgcgg

SEQ ID NO: 44242 - DNA, 28 bp, synthetic construct
  source 1..28: mol_type = other DNA
gtggagcgcgcgcggccatgggcgcggg

SEQ ID NO: 44243 - DNA, 28 bp, synthetic construct
  source 1..28: mol_type = other DNA
cgcgcgcggccatgggcgcgggccacgg

SEQ ID NO: 44244 - DNA, 28 bp, synthetic construct
  source 1..28: mol_type = other DNA
gcgcgcggccatgggcgcgggccacggg

SEQ ID NO: 44245 - DNA, 28 bp, synthetic construct
  source 1..28: mol_type = other DNA
cgcggccatgggcgcgggccacgggcgg

SEQ ID NO: 44246 - DNA, 28 bp, synthetic construct
  source 1..28: mol_type = other DNA
gcggccatgggcgcgggccacgggcggg

SEQ ID NO: 44247 - DNA, 28 bp, synthetic construct
  source 1..28: mol_type = other DNA
gccatgggcgcgggccacgggcgggtgg

SEQ ID NO: 44248 - DNA, 28 bp, synthetic construct
  source 1..28: mol_type = other DNA
cccacccgcccgtggcccgcgcccatgg

SEQ ID NO: 44249 - DNA, 28 bp, synthetic construct
  source 1..28: mol_type = other DNA
tgggcgcgggccacgggcgggtgggagg

SEQ ID NO: 44250 - DNA, 28 bp, synthetic construct
  source 1..28: mol_type = other DNA
gggcgcgggccacgggcgggtgggaggg

SEQ ID NO: 44251 - DNA, 28 bp, synthetic construct
  source 1..28: mol_type = other DNA
cgcgggccacgggcgggtgggagggtgg

SEQ ID NO: 44252 - DNA, 28 bp, synthetic construct
  source 1..28: mol_type = other DNA
gcgggccacgggcgggtgggagggtggg

SEQ ID NO: 44253 - DNA, 28 bp, synthetic construct
  source 1..28: mol_type = other DNA
cgggccacgggcgggtgggagggtgggg

SEQ ID NO: 44254 - DNA, 28 bp, synthetic construct
  source 1..28: mol_type = other DNA
gggccacgggcgggtgggagggtggggg

SEQ ID NO: 44255 - DNA, 28 bp, synthetic construct
  source 1..28: mol_type = other DNA
ggccacgggcgggtgggagggtgggggg

SEQ ID NO: 44256 - DNA, 28 bp, synthetic construct
  source 1..28: mol_type = other DNA
ggccccccaccctcccacccgcccgtgg

SEQ ID NO: 44257 - DNA, 28 bp, synthetic construct
  source 1..28: mol_type = other DNA
ggcgggtgggagggtggggggccagagg

SEQ ID NO: 44258 - DNA, 28 bp, synthetic construct
  source 1..28: mol_type = other DNA
gcgggtgggagggtggggggccagaggg

SEQ ID NO: 44259 - DNA, 28 bp, synthetic construct
  source 1..28: mol_type = other DNA
cgggtgggagggtggggggccagagggg

SEQ ID NO: 44260 - DNA, 28 bp, synthetic construct
  source 1..28: mol_type = other DNA
gtgggagggtggggggccagaggggcgg

SEQ ID NO: 44261 - DNA, 28 bp, synthetic construct
  source 1..28: mol_type = other DNA
tgggagggtggggggccagaggggcggg

SEQ ID NO: 44262 - DNA, 28 bp, synthetic construct
  source 1..28: mol_type = other DNA
gggagggtggggggccagaggggcgggg

SEQ ID NO: 44263 - DNA, 28 bp, synthetic construct
  source 1..28: mol_type = other DNA
ggagggtggggggccagaggggcggggg

SEQ ID NO: 44264 - DNA, 28 bp, synthetic construct
  source 1..28: mol_type = other DNA
gggtggggggccagaggggcgggggagg

SEQ ID NO: 44265 - DNA, 28 bp, synthetic construct
  source 1..28: mol_type = other DNA
ggtggggggccagaggggcgggggaggg

SEQ ID NO: 44266 - DNA, 28 bp, synthetic construct
  source 1..28: mol_type = other DNA
gccagaggggcgggggagggtcactcgg

SEQ ID NO: 44267 - DNA, 28 bp, synthetic construct
  source 1..28: mol_type = other DNA
gccgagtgaccctcccccgcccctctgg

SEQ ID NO: 44268 - DNA, 28 bp, synthetic construct
  source 1..28: mol_type = other DNA
agaggggcgggggagggtcactcggcgg

SEQ ID NO: 44269 - DNA, 28 bp, synthetic construct
  source 1..28: mol_type = other DNA
cgggggagggtcactcggcggctcccgg

SEQ ID NO: 44270 - DNA, 28 bp, synthetic construct
  source 1..28: mol_type = other DNA
ggcggtggcgggcggcggcggcaccggg

SEQ ID NO: 44271 - DNA, 28 bp, synthetic construct
  source 1..28: mol_type = other DNA
aggcggtggcgggcggcggcggcaccgg

SEQ ID NO: 44272 - DNA, 28 bp, synthetic construct
  source 1..28: mol_type = other DNA
gagcagaggcggtggcgggcggcggcgg

SEQ ID NO: 44273 - DNA, 28 bp, synthetic construct
  source 1..28: mol_type = other DNA
ggggagcagaggcggtggcgggcggcgg

SEQ ID NO: 44274 - DNA, 28 bp, synthetic construct
  source 1..28: mol_type = other DNA
cgcggggagcagaggcggtggcgggcgg

SEQ ID NO: 44275 - DNA, 28 bp, synthetic construct
  source 1..28: mol_type = other DNA
gcgcgcggggagcagaggcggtggcggg

SEQ ID NO: 44276 - DNA, 28 bp, synthetic construct
  source 1..28: mol_type = other DNA
ggcgcgcggggagcagaggcggtggcgg

SEQ ID NO: 44277 - DNA, 28 bp, synthetic construct
  source 1..28: mol_type = other DNA
gcgggcgcgcggggagcagaggcggtgg

SEQ ID NO: 44278 - DNA, 28 bp, synthetic construct
  source 1..28: mol_type = other DNA
tctgcgggcgcgcggggagcagaggcgg

SEQ ID NO: 44279 - DNA, 28 bp, synthetic construct
  source 1..28: mol_type = other DNA
gtgtctgcgggcgcgcggggagcagagg

SEQ ID NO: 44280 - DNA, 28 bp, synthetic construct
  source 1..28: mol_type = other DNA
gaacgaacgtgtctgcgggcgcgcgggg

SEQ ID NO: 44281 - DNA, 28 bp, synthetic construct
  source 1..28: mol_type = other DNA
agaacgaacgtgtctgcgggcgcgcggg

SEQ ID NO: 44282 - DNA, 28 bp, synthetic construct
  source 1..28: mol_type = other DNA
gagaacgaacgtgtctgcgggcgcgcgg

SEQ ID NO: 44283 - DNA, 28 bp, synthetic construct
  source 1..28: mol_type = other DNA
cgcccgcagacacgttcgttctctctgg

SEQ ID NO: 44284 - DNA, 28 bp, synthetic construct
  source 1..28: mol_type = other DNA
gaccagagagaacgaacgtgtctgcggg

SEQ ID NO: 44285 - DNA, 28 bp, synthetic construct
  source 1..28: mol_type = other DNA
cgaccagagagaacgaacgtgtctgcgg

SEQ ID NO: 44286 - DNA, 28 bp, synthetic construct
  source 1..28: mol_type = other DNA
cgcagacacgttcgttctctctggtcgg

SEQ ID NO: 44287 - DNA, 28 bp, synthetic construct
  source 1..28: mol_type = other DNA
gcagacacgttcgttctctctggtcggg

SEQ ID NO: 44288 - DNA, 28 bp, synthetic construct
  source 1..28: mol_type = other DNA
tcgttctctctggtcgggaaactgccgg

SEQ ID NO: 44289 - DNA, 28 bp, synthetic construct
  source 1..28: mol_type = other DNA
ctctggtcgggaaactgccggccgccgg

SEQ ID NO: 44290 - DNA, 28 bp, synthetic construct
  source 1..28: mol_type = other DNA
taagtaaggaacgcgcgccggcggccgg

SEQ ID NO: 44291 - DNA, 28 bp, synthetic construct
  source 1..28: mol_type = other DNA
gttataagtaaggaacgcgcgccggcgg

SEQ ID NO: 44292 - DNA, 28 bp, synthetic construct
  source 1..28: mol_type = other DNA
gaagttataagtaaggaacgcgcgccgg

SEQ ID NO: 44293 - DNA, 28 bp, synthetic construct
  source 1..28: mol_type = other DNA
gctgtagcgaaggaagttataagtaagg

SEQ ID NO: 44294 - DNA, 28 bp, synthetic construct
  source 1..28: mol_type = other DNA
aaggcggaggaaaaggctgtagcgaagg

SEQ ID NO: 44295 - DNA, 28 bp, synthetic construct
  source 1..28: mol_type = other DNA
ggggcatgggagaaggcggaggaaaagg

SEQ ID NO: 44296 - DNA, 28 bp, synthetic construct
  source 1..28: mol_type = other DNA
aggggcggggcatgggagaaggcggagg

SEQ ID NO: 44297 - DNA, 28 bp, synthetic construct
  source 1..28: mol_type = other DNA
gggaggggcggggcatgggagaaggcgg

SEQ ID NO: 44298 - DNA, 28 bp, synthetic construct
  source 1..28: mol_type = other DNA
aaagggaggggcggggcatgggagaagg

SEQ ID NO: 44299 - DNA, 28 bp, synthetic construct
  source 1..28: mol_type = other DNA
gagaagaaagggaggggcggggcatggg

SEQ ID NO: 44300 - DNA, 28 bp, synthetic construct
  source 1..28: mol_type = other DNA
agagaagaaagggaggggcggggcatgg

SEQ ID NO: 44301 - DNA, 28 bp, synthetic construct
  source 1..28: mol_type = other DNA
ggcggagagaagaaagggaggggcgggg

SEQ ID NO: 44302 - DNA, 28 bp, synthetic construct
  source 1..28: mol_type = other DNA
gggcggagagaagaaagggaggggcggg

SEQ ID NO: 44303 - DNA, 28 bp, synthetic construct
  source 1..28: mol_type = other DNA
ggggcggagagaagaaagggaggggcgg

SEQ ID NO: 44304 - DNA, 28 bp, synthetic construct
  source 1..28: mol_type = other DNA
gggggggcggagagaagaaagggagggg

SEQ ID NO: 44305 - DNA, 28 bp, synthetic construct
  source 1..28: mol_type = other DNA
ggggggggcggagagaagaaagggaggg

SEQ ID NO: 44306 - DNA, 28 bp, synthetic construct
  source 1..28: mol_type = other DNA
cggggggggcggagagaagaaagggagg

SEQ ID NO: 44307 - DNA, 28 bp, synthetic construct
  source 1..28: mol_type = other DNA
cctcggggggggcggagagaagaaaggg

SEQ ID NO: 44308 - DNA, 28 bp, synthetic construct
  source 1..28: mol_type = other DNA
gcctcggggggggcggagagaagaaagg

SEQ ID NO: 44309 - DNA, 28 bp, synthetic construct
  source 1..28: mol_type = other DNA
cgatggaagggagcctcggggggggcgg

SEQ ID NO: 44310 - DNA, 28 bp, synthetic construct
  source 1..28: mol_type = other DNA
caacgatggaagggagcctcgggggggg

SEQ ID NO: 44311 - DNA, 28 bp, synthetic construct
  source 1..28: mol_type = other DNA
gcaacgatggaagggagcctcggggggg

SEQ ID NO: 44312 - DNA, 28 bp, synthetic construct
  source 1..28: mol_type = other DNA
agcaacgatggaagggagcctcgggggg

SEQ ID NO: 44313 - DNA, 28 bp, synthetic construct
  source 1..28: mol_type = other DNA
tagcaacgatggaagggagcctcggggg

SEQ ID NO: 44314 - DNA, 28 bp, synthetic construct
  source 1..28: mol_type = other DNA
atagcaacgatggaagggagcctcgggg

SEQ ID NO: 44315 - DNA, 28 bp, synthetic construct
  source 1..28: mol_type = other DNA
catagcaacgatggaagggagcctcggg

SEQ ID NO: 44316 - DNA, 28 bp, synthetic construct
  source 1..28: mol_type = other DNA
ccgaggctcccttccatcgttgctatgg

SEQ ID NO: 44317 - DNA, 28 bp, synthetic construct
  source 1..28: mol_type = other DNA
tttagctgccatagcaacgatggaaggg

SEQ ID NO: 44318 - DNA, 28 bp, synthetic construct
  source 1..28: mol_type = other DNA
atttagctgccatagcaacgatggaagg

SEQ ID NO: 44319 - DNA, 28 bp, synthetic construct
  source 1..28: mol_type = other DNA
gttgatttagctgccatagcaacgatgg

SEQ ID NO: 44320 - DNA, 28 bp, synthetic construct
  source 1..28: mol_type = other DNA
gctatggcagctaaatcaacaaactcgg

SEQ ID NO: 44321 - DNA, 28 bp, synthetic construct
  source 1..28: mol_type = other DNA
gctaaatcaacaaactcggcgcacgtgg

SEQ ID NO: 44322 - DNA, 28 bp, synthetic construct
  source 1..28: mol_type = other DNA
ctaaatcaacaaactcggcgcacgtggg

SEQ ID NO: 44323 - DNA, 28 bp, synthetic construct
  source 1..28: mol_type = other DNA
taaatcaacaaactcggcgcacgtgggg

SEQ ID NO: 44324 - DNA, 28 bp, synthetic construct
  source 1..28: mol_type = other DNA
aaatcaacaaactcggcgcacgtggggg

SEQ ID NO: 44325 - DNA, 28 bp, synthetic construct
  source 1..28: mol_type = other DNA
tcaacaaactcggcgcacgtgggggcgg

SEQ ID NO: 44326 - DNA, 28 bp, synthetic construct
  source 1..28: mol_type = other DNA
caacaaactcggcgcacgtgggggcggg

SEQ ID NO: 44327 - DNA, 28 bp, synthetic construct
  source 1..28: mol_type = other DNA
aacaaactcggcgcacgtgggggcgggg

SEQ ID NO: 44328 - DNA, 28 bp, synthetic construct
  source 1..28: mol_type = other DNA
acaaactcggcgcacgtgggggcggggg

SEQ ID NO: 44329 - DNA, 28 bp, synthetic construct
  source 1..28: mol_type = other DNA
aactcggcgcacgtgggggcgggggagg

SEQ ID NO: 44330 - DNA, 28 bp, synthetic construct
  source 1..28: mol_type = other DNA
actcggcgcacgtgggggcgggggaggg

SEQ ID NO: 44331 - DNA, 28 bp, synthetic construct
  source 1..28: mol_type = other DNA
ctcggcgcacgtgggggcgggggagggg

SEQ ID NO: 44332 - DNA, 28 bp, synthetic construct
  source 1..28: mol_type = other DNA
gcgcacgtgggggcgggggaggggaagg

SEQ ID NO: 44333 - DNA, 28 bp, synthetic construct
  source 1..28: mol_type = other DNA
cacgtgggggcgggggaggggaaggagg

SEQ ID NO: 44334 - DNA, 28 bp, synthetic construct
  source 1..28: mol_type = other DNA
acgtgggggcgggggaggggaaggaggg

SEQ ID NO: 44335 - DNA, 28 bp, synthetic construct
  source 1..28: mol_type = other DNA
cgtgggggcgggggaggggaaggagggg

SEQ ID NO: 44336 - DNA, 28 bp, synthetic construct
  source 1..28: mol_type = other DNA
gggcgggggaggggaaggaggggcgcgg

SEQ ID NO: 44337 - DNA, 28 bp, synthetic construct
  source 1..28: mol_type = other DNA
ggcgggggaggggaaggaggggcgcggg

SEQ ID NO: 44338 - DNA, 28 bp, synthetic construct
  source 1..28: mol_type = other DNA
gggggaggggaaggaggggcgcgggcgg

SEQ ID NO: 44339 - DNA, 28 bp, synthetic construct
  source 1..28: mol_type = other DNA
ggggaggggaaggaggggcgcgggcggg

SEQ ID NO: 44340 - DNA, 28 bp, synthetic construct
  source 1..28: mol_type = other DNA
gggaggggaaggaggggcgcgggcgggg

SEQ ID NO: 44341 - DNA, 28 bp, synthetic construct
  source 1..28: mol_type = other DNA
ggggaaggaggggcgcgggcggggctgg

SEQ ID NO: 44342 - DNA, 28 bp, synthetic construct
  source 1..28: mol_type = other DNA
gggaaggaggggcgcgggcggggctggg

SEQ ID NO: 44343 - DNA, 28 bp, synthetic construct
  source 1..28: mol_type = other DNA
aggaggggcgcgggcggggctgggccgg

SEQ ID NO: 44344 - DNA, 28 bp, synthetic construct
  source 1..28: mol_type = other DNA
ggaggggcgcgggcggggctgggccggg

SEQ ID NO: 44345 - DNA, 28 bp, synthetic construct
  source 1..28: mol_type = other DNA
gctgggccgggccgtgacgccagccagg

SEQ ID NO: 44346 - DNA, 28 bp, synthetic construct
  source 1..28: mol_type = other DNA
cagctgcctggctggcgtcacggcccgg

SEQ ID NO: 44347 - DNA, 28 bp, synthetic construct
  source 1..28: mol_type = other DNA
cgggccgtgacgccagccaggcagctgg

SEQ ID NO: 44348 - DNA, 28 bp, synthetic construct
  source 1..28: mol_type = other DNA
gccgtgacgccagccaggcagctggcgg

SEQ ID NO: 44349 - DNA, 28 bp, synthetic construct
  source 1..28: mol_type = other DNA
cccgccagctgcctggctggcgtcacgg

SEQ ID NO: 44350 - DNA, 28 bp, synthetic construct
  source 1..28: mol_type = other DNA
gacgccagccaggcagctggcgggctgg

SEQ ID NO: 44351 - DNA, 28 bp, synthetic construct
  source 1..28: mol_type = other DNA
ggctccagcccgccagctgcctggctgg

SEQ ID NO: 44352 - DNA, 28 bp, synthetic construct
  source 1..28: mol_type = other DNA
gctcggctccagcccgccagctgcctgg

SEQ ID NO: 44353 - DNA, 28 bp, synthetic construct
  source 1..28: mol_type = other DNA
tggcgggctggagccgagctgacgccgg

SEQ ID NO: 44354 - DNA, 28 bp, synthetic construct
  source 1..28: mol_type = other DNA
cgggctggagccgagctgacgccggcgg

SEQ ID NO: 44355 - DNA, 28 bp, synthetic construct
  source 1..28: mol_type = other DNA
ggagccgagctgacgccggcggcagtgg

SEQ ID NO: 44356 - DNA, 28 bp, synthetic construct
  source 1..28: mol_type = other DNA
gacaccactgccgccggcgtcagctcgg

SEQ ID NO: 44357 - DNA, 28 bp, synthetic construct
  source 1..28: mol_type = other DNA
gagctgacgccggcggcagtggtgtcgg

SEQ ID NO: 44358 - DNA, 28 bp, synthetic construct
  source 1..28: mol_type = other DNA
ctgacgccggcggcagtggtgtcggcgg

SEQ ID NO: 44359 - DNA, 28 bp, synthetic construct
  source 1..28: mol_type = other DNA
acgccggcggcagtggtgtcggcggcgg

SEQ ID NO: 44360 - DNA, 28 bp, synthetic construct
  source 1..28: mol_type = other DNA
ccgccgccgccgacaccactgccgccgg

SEQ ID NO: 44361 - DNA, 28 bp, synthetic construct
  source 1..28: mol_type = other DNA
gcggcagtggtgtcggcggcggcggcgg

SEQ ID NO: 44362 - DNA, 28 bp, synthetic construct
  source 1..28: mol_type = other DNA
ggcggcggcggcgtccgccccagcgcgg

SEQ ID NO: 44363 - DNA, 28 bp, synthetic construct
  source 1..28: mol_type = other DNA
gcggcggcggcgtccgccccagcgcggg

SEQ ID NO: 44364 - DNA, 28 bp, synthetic construct
  source 1..28: mol_type = other DNA
cggcggcggcgtccgccccagcgcgggg

SEQ ID NO: 44365 - DNA, 28 bp, synthetic construct
  source 1..28: mol_type = other DNA
ggcgtccgccccagcgcggggcgcgagg

SEQ ID NO: 44366 - DNA, 28 bp, synthetic construct
  source 1..28: mol_type = other DNA
cggttcctcgcgccccgcgctggggcgg

SEQ ID NO: 44367 - DNA, 28 bp, synthetic construct
  source 1..28: mol_type = other DNA
cgccccagcgcggggcgcgaggaaccgg

SEQ ID NO: 44368 - DNA, 28 bp, synthetic construct
  source 1..28: mol_type = other DNA
gccccagcgcggggcgcgaggaaccggg

SEQ ID NO: 44369 - DNA, 28 bp, synthetic construct
  source 1..28: mol_type = other DNA
gcccggttcctcgcgccccgcgctgggg

SEQ ID NO: 44370 - DNA, 28 bp, synthetic construct
  source 1..28: mol_type = other DNA
cgcccggttcctcgcgccccgcgctggg

SEQ ID NO: 44371 - DNA, 28 bp, synthetic construct
  source 1..28: mol_type = other DNA
gcgcccggttcctcgcgccccgcgctgg

SEQ ID NO: 44372 - DNA, 28 bp, synthetic construct
  source 1..28: mol_type = other DNA
gcgcggggcgcgaggaaccgggcgcagg

SEQ ID NO: 44373 - DNA, 28 bp, synthetic construct
  source 1..28: mol_type = other DNA
gggcgcgaggaaccgggcgcaggttcgg

SEQ ID NO: 44374 - DNA, 28 bp, synthetic construct
  source 1..28: mol_type = other DNA
gtcgcgcagcgaccgaacctgcgcccgg

SEQ ID NO: 44375 - DNA, 28 bp, synthetic construct
  source 1..28: mol_type = other DNA
gcgcaggttcggtcgctgcgcgaccagg

SEQ ID NO: 44376 - DNA, 28 bp, synthetic construct
  source 1..28: mol_type = other DNA
cgcaggttcggtcgctgcgcgaccaggg

SEQ ID NO: 44377 - DNA, 28 bp, synthetic construct
  source 1..28: mol_type = other DNA
ccagggccgtactcaccgccattgtcgg

SEQ ID NO: 44378 - DNA, 28 bp, synthetic construct
  source 1..28: mol_type = other DNA
agggagccgacaatggcggtgagtacgg

SEQ ID NO: 44379 - DNA, 28 bp, synthetic construct
  source 1..28: mol_type = other DNA
gtactcaccgccattgtcggctccctgg

SEQ ID NO: 44380 - DNA, 28 bp, synthetic construct
  source 1..28: mol_type = other DNA
tactcaccgccattgtcggctccctggg

SEQ ID NO: 44381 - DNA, 28 bp, synthetic construct
  source 1..28: mol_type = other DNA
ttcgaacccagggagccgacaatggcgg

SEQ ID NO: 44382 - DNA, 28 bp, synthetic construct
  source 1..28: mol_type = other DNA
ggcttcgaacccagggagccgacaatgg

SEQ ID NO: 44383 - DNA, 28 bp, synthetic construct
  source 1..28: mol_type = other DNA
ccagtcttcgcgggcttcgaacccaggg

SEQ ID NO: 44384 - DNA, 28 bp, synthetic construct
  source 1..28: mol_type = other DNA
accagtcttcgcgggcttcgaacccagg

SEQ ID NO: 44385 - DNA, 28 bp, synthetic construct
  source 1..28: mol_type = other DNA
tgggttcgaagcccgcgaagactggtgg

SEQ ID NO: 44386 - DNA, 28 bp, synthetic construct
  source 1..28: mol_type = other DNA
gggttcgaagcccgcgaagactggtggg

SEQ ID NO: 44387 - DNA, 28 bp, synthetic construct
  source 1..28: mol_type = other DNA
ggttcgaagcccgcgaagactggtgggg

SEQ ID NO: 44388 - DNA, 28 bp, synthetic construct
  source 1..28: mol_type = other DNA
agcccgcgaagactggtggggtcagcgg

SEQ ID NO: 44389 - DNA, 28 bp, synthetic construct
  source 1..28: mol_type = other DNA
gcccgcgaagactggtggggtcagcggg

SEQ ID NO: 44390 - DNA, 28 bp, synthetic construct
  source 1..28: mol_type = other DNA
gcccgctgaccccaccagtcttcgcggg

SEQ ID NO: 44391 - DNA, 28 bp, synthetic construct
  source 1..28: mol_type = other DNA
cgcccgctgaccccaccagtcttcgcgg

SEQ ID NO: 44392 - DNA, 28 bp, synthetic construct
  source 1..28: mol_type = other DNA
cgcgaagactggtggggtcagcgggcgg

SEQ ID NO: 44393 - DNA, 28 bp, synthetic construct
  source 1..28: mol_type = other DNA
agactggtggggtcagcgggcggcacgg

SEQ ID NO: 44394 - DNA, 28 bp, synthetic construct
  source 1..28: mol_type = other DNA
gcaagcgcgtatgctagcaggggtgcgg

SEQ ID NO: 44395 - DNA, 28 bp, synthetic construct
  source 1..28: mol_type = other DNA
gcgcggcaagcgcgtatgctagcagggg

SEQ ID NO: 44396 - DNA, 28 bp, synthetic construct
  source 1..28: mol_type = other DNA
agcgcggcaagcgcgtatgctagcaggg

SEQ ID NO: 44397 - DNA, 28 bp, synthetic construct
  source 1..28: mol_type = other DNA
cagcgcggcaagcgcgtatgctagcagg

SEQ ID NO: 44398 - DNA, 28 bp, synthetic construct
  source 1..28: mol_type = other DNA
cgcgcttgccgcgctgtctgcgcgctgg

SEQ ID NO: 44399 - DNA, 28 bp, synthetic construct
  source 1..28: mol_type = other DNA
gctcttctccagcgcgcagacagcgcgg

SEQ ID NO: 44400 - DNA, 28 bp, synthetic construct
  source 1..28: mol_type = other DNA
gagatggagggctggatgagtcacgcgg

SEQ ID NO: 44401 - DNA, 28 bp, synthetic construct
  source 1..28: mol_type = other DNA
agagagggagggggagatggagggctgg

SEQ ID NO: 44402 - DNA, 28 bp, synthetic construct
  source 1..28: mol_type = other DNA
gcgcagagagggagggggagatggaggg

SEQ ID NO: 44403 - DNA, 28 bp, synthetic construct
  source 1..28: mol_type = other DNA
agcgcagagagggagggggagatggagg

SEQ ID NO: 44404 - DNA, 28 bp, synthetic construct
  source 1..28: mol_type = other DNA
gcgagcgcagagagggagggggagatgg

SEQ ID NO: 44405 - DNA, 28 bp, synthetic construct
  source 1..28: mol_type = other DNA
tctccccctccctctctgcgctcgcagg

SEQ ID NO: 44406 - DNA, 28 bp, synthetic construct
  source 1..28: mol_type = other DNA
actcctgcgagcgcagagagggaggggg

SEQ ID NO: 44407 - DNA, 28 bp, synthetic construct
  source 1..28: mol_type = other DNA
gactcctgcgagcgcagagagggagggg

SEQ ID NO: 44408 - DNA, 28 bp, synthetic construct
  source 1..28: mol_type = other DNA
ggactcctgcgagcgcagagagggaggg

SEQ ID NO: 44409 - DNA, 28 bp, synthetic construct
  source 1..28: mol_type = other DNA
cggactcctgcgagcgcagagagggagg

SEQ ID NO: 44410 - DNA, 28 bp, synthetic construct
  source 1..28: mol_type = other DNA
gagcggactcctgcgagcgcagagaggg

SEQ ID NO: 44411 - DNA, 28 bp, synthetic construct
  source 1..28: mol_type = other DNA
agagcggactcctgcgagcgcagagagg

SEQ ID NO: 44412 - DNA, 28 bp, synthetic construct
  source 1..28: mol_type = other DNA
cggcactggcgctgagcgacgagagcgg

SEQ ID NO: 44413 - DNA, 28 bp, synthetic construct
  source 1..28: mol_type = other DNA
cgctctcgtcgctcagcgccagtgccgg

SEQ ID NO: 44414 - DNA, 28 bp, synthetic construct
  source 1..28: mol_type = other DNA
tctcgtcgctcagcgccagtgccggtgg

SEQ ID NO: 44415 - DNA, 28 bp, synthetic construct
  source 1..28: mol_type = other DNA
cgtcgctcagcgccagtgccggtggcgg

SEQ ID NO: 44416 - DNA, 28 bp, synthetic construct
  source 1..28: mol_type = other DNA
tcagcgccagtgccggtggcggtgccgg

SEQ ID NO: 44417 - DNA, 28 bp, synthetic construct
  source 1..28: mol_type = other DNA
cgagcgccggcaccgccaccggcactgg

SEQ ID NO: 44418 - DNA, 28 bp, synthetic construct
  source 1..28: mol_type = other DNA
cagtgccggtggcggtgccggcgctcgg

SEQ ID NO: 44419 - DNA, 28 bp, synthetic construct
  source 1..28: mol_type = other DNA
tcaggccgagcgccggcaccgccaccgg

SEQ ID NO: 44420 - DNA, 28 bp, synthetic construct
  source 1..28: mol_type = other DNA
tgccggcgctcggcctgacctcgcacgg

SEQ ID NO: 44421 - DNA, 28 bp, synthetic construct
  source 1..28: mol_type = other DNA
aaccgtgcgaggtcaggccgagcgccgg

SEQ ID NO: 44422 - DNA, 28 bp, synthetic construct
  source 1..28: mol_type = other DNA
cggcctgacctcgcacggttcctcgcgg

SEQ ID NO: 44423 - DNA, 28 bp, synthetic construct
  source 1..28: mol_type = other DNA
ggcctgacctcgcacggttcctcgcggg

SEQ ID NO: 44424 - DNA, 28 bp, synthetic construct
  source 1..28: mol_type = other DNA
ggcccgcgaggaaccgtgcgaggtcagg

SEQ ID NO: 44425 - DNA, 28 bp, synthetic construct
  source 1..28: mol_type = other DNA
agaagggcccgcgaggaaccgtgcgagg

SEQ ID NO: 44426 - DNA, 28 bp, synthetic construct
  source 1..28: mol_type = other DNA
cggttcctcgcgggcccttctgctgagg

SEQ ID NO: 44427 - DNA, 28 bp, synthetic construct
  source 1..28: mol_type = other DNA
ggttcctcgcgggcccttctgctgaggg

SEQ ID NO: 44428 - DNA, 28 bp, synthetic construct
  source 1..28: mol_type = other DNA
gttcctcgcgggcccttctgctgagggg

SEQ ID NO: 44429 - DNA, 28 bp, synthetic construct
  source 1..28: mol_type = other DNA
cctcgcgggcccttctgctgaggggtgg

SEQ ID NO: 44430 - DNA, 28 bp, synthetic construct
  source 1..28: mol_type = other DNA
ctcgcgggcccttctgctgaggggtggg

SEQ ID NO: 44431 - DNA, 28 bp, synthetic construct
  source 1..28: mol_type = other DNA
tcgcgggcccttctgctgaggggtgggg

SEQ ID NO: 44432 - DNA, 28 bp, synthetic construct
  source 1..28: mol_type = other DNA
cgcgggcccttctgctgaggggtggggg

SEQ ID NO: 44433 - DNA, 28 bp, synthetic construct
  source 1..28: mol_type = other DNA
gcgggcccttctgctgaggggtgggggg

SEQ ID NO: 44434 - DNA, 28 bp, synthetic construct
  source 1..28: mol_type = other DNA
tagcgccccccacccctcagcagaaggg

SEQ ID NO: 44435 - DNA, 28 bp, synthetic construct
  source 1..28: mol_type = other DNA
ctagcgccccccacccctcagcagaagg

SEQ ID NO: 44436 - DNA, 28 bp, synthetic construct
  source 1..28: mol_type = other DNA
cttctgctgaggggtggggggcgctagg

SEQ ID NO: 44437 - DNA, 28 bp, synthetic construct
  source 1..28: mol_type = other DNA
ttctgctgaggggtggggggcgctaggg

SEQ ID NO: 44438 - DNA, 28 bp, synthetic construct
  source 1..28: mol_type = other DNA
tctgctgaggggtggggggcgctagggg

SEQ ID NO: 44439 - DNA, 28 bp, synthetic construct
  source 1..28: mol_type = other DNA
tgaggggtggggggcgctaggggtgtgg

SEQ ID NO: 44440 - DNA, 28 bp, synthetic construct
  source 1..28: mol_type = other DNA
ggtggggggcgctaggggtgtggagagg

SEQ ID NO: 44441 - DNA, 28 bp, synthetic construct
  source 1..28: mol_type = other DNA
ggggggcgctaggggtgtggagaggagg

SEQ ID NO: 44442 - DNA, 28 bp, synthetic construct
  source 1..28: mol_type = other DNA
gtgcccagcactgtgcagcgtgaactgg

SEQ ID NO: 44443 - DNA, 28 bp, synthetic construct
  source 1..28: mol_type = other DNA
tgcccagcactgtgcagcgtgaactggg

SEQ ID NO: 44444 - DNA, 28 bp, synthetic construct
  source 1..28: mol_type = other DNA
ctcccagttcacgctgcacagtgctggg

SEQ ID NO: 44445 - DNA, 28 bp, synthetic construct
  source 1..28: mol_type = other DNA
gctcccagttcacgctgcacagtgctgg

SEQ ID NO: 44446 - DNA, 28 bp, synthetic construct
  source 1..28: mol_type = other DNA
agcgtgaactgggagcctcaagagaagg

SEQ ID NO: 44447 - DNA, 28 bp, synthetic construct
  source 1..28: mol_type = other DNA
actgggagcctcaagagaaggccagagg

SEQ ID NO: 44448 - DNA, 28 bp, synthetic construct
  source 1..28: mol_type = other DNA
ggaacactcctctggccttctcttgagg

SEQ ID NO: 44449 - DNA, 28 bp, synthetic construct
  source 1..28: mol_type = other DNA
agagaaggccagaggagtgttccgccgg

SEQ ID NO: 44450 - DNA, 28 bp, synthetic construct
  source 1..28: mol_type = other DNA
gagaaggccagaggagtgttccgccggg

SEQ ID NO: 44451 - DNA, 28 bp, synthetic construct
  source 1..28: mol_type = other DNA
gccagaggagtgttccgccgggaacagg

SEQ ID NO: 44452 - DNA, 28 bp, synthetic construct
  source 1..28: mol_type = other DNA
gcctgttcccggcggaacactcctctgg

SEQ ID NO: 44453 - DNA, 28 bp, synthetic construct
  source 1..28: mol_type = other DNA
agaggagtgttccgccgggaacaggcgg

SEQ ID NO: 44454 - DNA, 28 bp, synthetic construct
  source 1..28: mol_type = other DNA
tgttccgccgggaacaggcggaaagagg

SEQ ID NO: 44455 - DNA, 28 bp, synthetic construct
  source 1..28: mol_type = other DNA
cgtgcctctttccgcctgttcccggcgg

SEQ ID NO: 44456 - DNA, 28 bp, synthetic construct
  source 1..28: mol_type = other DNA
attcgtgcctctttccgcctgttcccgg

SEQ ID NO: 44457 - DNA, 28 bp, synthetic construct
  source 1..28: mol_type = other DNA
gggaacaggcggaaagaggcacgaatgg

SEQ ID NO: 44458 - DNA, 28 bp, synthetic construct
  source 1..28: mol_type = other DNA
ggaacaggcggaaagaggcacgaatggg

SEQ ID NO: 44459 - DNA, 28 bp, synthetic construct
  source 1..28: mol_type = other DNA
gaacaggcggaaagaggcacgaatgggg

SEQ ID NO: 44460 - DNA, 28 bp, synthetic construct
  source 1..28: mol_type = other DNA
ggaaagaggcacgaatggggagttatgg

SEQ ID NO: 44461 - DNA, 28 bp, synthetic construct
  source 1..28: mol_type = other DNA
gttttgatactttaaatagcgagaaagg

SEQ ID NO: 44462 - DNA, 28 bp, synthetic construct
  source 1..28: mol_type = other DNA
ttttgatactttaaatagcgagaaaggg

SEQ ID NO: 44463 - DNA, 28 bp, synthetic construct
  source 1..28: mol_type = other DNA
tttaaatagcgagaaagggagtgaaagg

SEQ ID NO: 44464 - DNA, 28 bp, synthetic construct
  source 1..28: mol_type = other DNA
ttaaatagcgagaaagggagtgaaaggg

SEQ ID NO: 44465 - DNA, 28 bp, synthetic construct
  source 1..28: mol_type = other DNA
gtgaaagggctcaagatttactcagagg

SEQ ID NO: 44466 - DNA, 28 bp, synthetic construct
  source 1..28: mol_type = other DNA
ggctcaagatttactcagaggcataagg

SEQ ID NO: 44467 - DNA, 28 bp, synthetic construct
  source 1..28: mol_type = other DNA
gctcaagatttactcagaggcataaggg

SEQ ID NO: 44468 - DNA, 28 bp, synthetic construct
  source 1..28: mol_type = other DNA
tactcagaggcataagggagagaagagg

SEQ ID NO: 44469 - DNA, 28 bp, synthetic construct
  source 1..28: mol_type = other DNA
actcagaggcataagggagagaagaggg

SEQ ID NO: 44470 - DNA, 28 bp, synthetic construct
  source 1..28: mol_type = other DNA
cataagggagagaagagggactgtgagg

SEQ ID NO: 44471 - DNA, 28 bp, synthetic construct
  source 1..28: mol_type = other DNA
gggagagaagagggactgtgaggcgcgg

SEQ ID NO: 44472 - DNA, 28 bp, synthetic construct
  source 1..28: mol_type = other DNA
aaaaaggaaagggcttcgagatggctgg

SEQ ID NO: 44473 - DNA, 28 bp, synthetic construct
  source 1..28: mol_type = other DNA
aaaaaaaaaggaaagggcttcgagatgg

SEQ ID NO: 44474 - DNA, 28 bp, synthetic construct
  source 1..28: mol_type = other DNA
aaaaaagaaagaaaaaaaaaggaaaggg

SEQ ID NO: 44475 - DNA, 28 bp, synthetic construct
  source 1..28: mol_type = other DNA
aaaaaaagaaagaaaaaaaaaggaaagg

SEQ ID NO: 44476 - DNA, 28 bp, synthetic construct
  source 1..28: mol_type = other DNA
aaaaaaaaaaaagaaagaaaaaaaaagg

SEQ ID NO: 44477 - DNA, 28 bp, synthetic construct
  source 1..28: mol_type = other DNA
cagagtctcgctgtgtcgcccaagctgg

SEQ ID NO: 44478 - DNA, 28 bp, synthetic construct
  source 1..28: mol_type = other DNA
ctgtgtcgcccaagctggaatgcagtgg

SEQ ID NO: 44479 - DNA, 28 bp, synthetic construct
  source 1..28: mol_type = other DNA
agatcgtgccactgcattccagcttggg

SEQ ID NO: 44480 - DNA, 28 bp, synthetic construct
  source 1..28: mol_type = other DNA
gagatcgtgccactgcattccagcttgg

SEQ ID NO: 44481 - DNA, 28 bp, synthetic construct
  source 1..28: mol_type = other DNA
agaatcgcttggacgcaggaggcggagg

SEQ ID NO: 44482 - DNA, 28 bp, synthetic construct
  source 1..28: mol_type = other DNA
aggagaatcgcttggacgcaggaggcgg

SEQ ID NO: 44483 - DNA, 28 bp, synthetic construct
  source 1..28: mol_type = other DNA
cgcaggagaatcgcttggacgcaggagg

SEQ ID NO: 44484 - DNA, 28 bp, synthetic construct
  source 1..28: mol_type = other DNA
tgacgcaggagaatcgcttggacgcagg

SEQ ID NO: 44485 - DNA, 28 bp, synthetic construct
  source 1..28: mol_type = other DNA
gggaggctgacgcaggagaatcgcttgg

SEQ ID NO: 44486 - DNA, 28 bp, synthetic construct
  source 1..28: mol_type = other DNA
tctcctgcgtcagcctcccgagtagcgg

SEQ ID NO: 44487 - DNA, 28 bp, synthetic construct
  source 1..28: mol_type = other DNA
ctcctgcgtcagcctcccgagtagcggg

SEQ ID NO: 44488 - DNA, 28 bp, synthetic construct
  source 1..28: mol_type = other DNA
tcctgcgtcagcctcccgagtagcgggg

SEQ ID NO: 44489 - DNA, 28 bp, synthetic construct
  source 1..28: mol_type = other DNA
tccccgctactcgggaggctgacgcagg

SEQ ID NO: 44490 - DNA, 28 bp, synthetic construct
  source 1..28: mol_type = other DNA
cagcctcccgagtagcggggattacagg

SEQ ID NO: 44491 - DNA, 28 bp, synthetic construct
  source 1..28: mol_type = other DNA
acgcctgtaatccccgctactcgggagg

SEQ ID NO: 44492 - DNA, 28 bp, synthetic construct
  source 1..28: mol_type = other DNA
cgcacgcctgtaatccccgctactcggg

SEQ ID NO: 44493 - DNA, 28 bp, synthetic construct
  source 1..28: mol_type = other DNA
gcgcacgcctgtaatccccgctactcgg

SEQ ID NO: 44494 - DNA, 28 bp, synthetic construct
  source 1..28: mol_type = other DNA
ggattacaggcgtgcgccacgacgccgg

SEQ ID NO: 44495 - DNA, 28 bp, synthetic construct
  source 1..28: mol_type = other DNA
aaaatacaaaaattagccggcgtcgtgg

SEQ ID NO: 44496 - DNA, 28 bp, synthetic construct
  source 1..28: mol_type = other DNA
cgccggctaatttttgtatttttcgtgg

SEQ ID NO: 44497 - DNA, 28 bp, synthetic construct
  source 1..28: mol_type = other DNA
ctccacgaaaaatacaaaaattagccgg

SEQ ID NO: 44498 - DNA, 28 bp, synthetic construct
  source 1..28: mol_type = other DNA
ctaatttttgtatttttcgtggagacgg

SEQ ID NO: 44499 - DNA, 28 bp, synthetic construct
  source 1..28: mol_type = other DNA
taatttttgtatttttcgtggagacggg

SEQ ID NO: 44500 - DNA, 28 bp, synthetic construct
  source 1..28: mol_type = other DNA
aatttttgtatttttcgtggagacgggg

SEQ ID NO: 44501 - DNA, 28 bp, synthetic construct
  source 1..28: mol_type = other DNA
tcgtggagacggggtttcaccatgttgg

SEQ ID NO: 44502 - DNA, 28 bp, synthetic construct
  source 1..28: mol_type = other DNA
gagacggggtttcaccatgttggccagg

SEQ ID NO: 44503 - DNA, 28 bp, synthetic construct
  source 1..28: mol_type = other DNA
cggggtttcaccatgttggccaggcagg

SEQ ID NO: 44504 - DNA, 28 bp, synthetic construct
  source 1..28: mol_type = other DNA
gtgttcgagacctgcctggccaacatgg

SEQ ID NO: 44505 - DNA, 28 bp, synthetic construct
  source 1..28: mol_type = other DNA
tgaggtcaggtgttcgagacctgcctgg

SEQ ID NO: 44506 - DNA, 28 bp, synthetic construct
  source 1..28: mol_type = other DNA
cgaggcaggctgatcacttgaggtcagg

SEQ ID NO: 44507 - DNA, 28 bp, synthetic construct
  source 1..28: mol_type = other DNA
ctgacctcaagtgatcagcctgcctcgg

SEQ ID NO: 44508 - DNA, 28 bp, synthetic construct
  source 1..28: mol_type = other DNA
gaggccgaggcaggctgatcacttgagg

SEQ ID NO: 44509 - DNA, 28 bp, synthetic construct
  source 1..28: mol_type = other DNA
agcctgcctcggcctcccgaagtgctgg

SEQ ID NO: 44510 - DNA, 28 bp, synthetic construct
  source 1..28: mol_type = other DNA
gcctgcctcggcctcccgaagtgctggg

SEQ ID NO: 44511 - DNA, 28 bp, synthetic construct
  source 1..28: mol_type = other DNA
tcccagcacttcgggaggccgaggcagg

SEQ ID NO: 44512 - DNA, 28 bp, synthetic construct
  source 1..28: mol_type = other DNA
gtaatcccagcacttcgggaggccgagg

SEQ ID NO: 44513 - DNA, 28 bp, synthetic construct
  source 1..28: mol_type = other DNA
cggcctcccgaagtgctgggattacagg

SEQ ID NO: 44514 - DNA, 28 bp, synthetic construct
  source 1..28: mol_type = other DNA
acgcctgtaatcccagcacttcgggagg

SEQ ID NO: 44515 - DNA, 28 bp, synthetic construct
  source 1..28: mol_type = other DNA
ctcacgcctgtaatcccagcacttcggg

SEQ ID NO: 44516 - DNA, 28 bp, synthetic construct
  source 1..28: mol_type = other DNA
gctcacgcctgtaatcccagcacttcgg

SEQ ID NO: 44517 - DNA, 28 bp, synthetic construct
  source 1..28: mol_type = other DNA
tttagtcatcaaatattacaggcagtgg

SEQ ID NO: 44518 - DNA, 28 bp, synthetic construct
  source 1..28: mol_type = other DNA
gtgcaatttagtcatcaaatattacagg

SEQ ID NO: 44519 - DNA, 28 bp, synthetic construct
  source 1..28: mol_type = other DNA
agtgagtgtttaattcttctttaatggg

SEQ ID NO: 44520 - DNA, 28 bp, synthetic construct
  source 1..28: mol_type = other DNA
cagtgagtgtttaattcttctttaatgg

SEQ ID NO: 44521 - DNA, 28 bp, synthetic construct
  source 1..28: mol_type = other DNA
gccacgcactctcctttccactttatgg

SEQ ID NO: 44522 - DNA, 28 bp, synthetic construct
  source 1..28: mol_type = other DNA
tccataaagtggaaaggagagtgcgtgg

SEQ ID NO: 44523 - DNA, 28 bp, synthetic construct
  source 1..28: mol_type = other DNA
tcaatttctcatccataaagtggaaagg

SEQ ID NO: 44524 - DNA, 28 bp, synthetic construct
  source 1..28: mol_type = other DNA
atgactcaatttctcatccataaagtgg

SEQ ID NO: 44525 - DNA, 28 bp, synthetic construct
  source 1..28: mol_type = other DNA
atggatgagaaattgagtcataaagagg

SEQ ID NO: 44526 - DNA, 28 bp, synthetic construct
  source 1..28: mol_type = other DNA
gaaattgagtcataaagaggtgaaatgg

SEQ ID NO: 44527 - DNA, 28 bp, synthetic construct
  source 1..28: mol_type = other DNA
cataaagaggtgaaatggccagtaaagg

SEQ ID NO: 44528 - DNA, 28 bp, synthetic construct
  source 1..28: mol_type = other DNA
aggtgaaatggccagtaaaggtcaaagg

SEQ ID NO: 44529 - DNA, 28 bp, synthetic construct
  source 1..28: mol_type = other DNA
gaacgagttgtcctttgacctttactgg

SEQ ID NO: 44530 - DNA, 28 bp, synthetic construct
  source 1..28: mol_type = other DNA
aaggtcaaaggacaactcgttccttcgg

SEQ ID NO: 44531 - DNA, 28 bp, synthetic construct
  source 1..28: mol_type = other DNA
aaaggacaactcgttccttcggctcagg

SEQ ID NO: 44532 - DNA, 28 bp, synthetic construct
  source 1..28: mol_type = other DNA
caactcgttccttcggctcaggctccgg

SEQ ID NO: 44533 - DNA, 28 bp, synthetic construct
  source 1..28: mol_type = other DNA
aactcgttccttcggctcaggctccggg

SEQ ID NO: 44534 - DNA, 28 bp, synthetic construct
  source 1..28: mol_type = other DNA
cgttccttcggctcaggctccgggtagg

SEQ ID NO: 44535 - DNA, 28 bp, synthetic construct
  source 1..28: mol_type = other DNA
ctgacctacccggagcctgagccgaagg

SEQ ID NO: 44536 - DNA, 28 bp, synthetic construct
  source 1..28: mol_type = other DNA
cttcggctcaggctccgggtaggtcagg

SEQ ID NO: 44537 - DNA, 28 bp, synthetic construct
  source 1..28: mol_type = other DNA
ctccgggtaggtcaggcccccctaaagg

SEQ ID NO: 44538 - DNA, 28 bp, synthetic construct
  source 1..28: mol_type = other DNA
tccgggtaggtcaggcccccctaaaggg

SEQ ID NO: 44539 - DNA, 28 bp, synthetic construct
  source 1..28: mol_type = other DNA
tccctttaggggggcctgacctacccgg

SEQ ID NO: 44540 - DNA, 28 bp, synthetic construct
  source 1..28: mol_type = other DNA
tcaggcccccctaaagggacttccctgg

SEQ ID NO: 44541 - DNA, 28 bp, synthetic construct
  source 1..28: mol_type = other DNA
caggcccccctaaagggacttccctggg

SEQ ID NO: 44542 - DNA, 28 bp, synthetic construct
  source 1..28: mol_type = other DNA
acttcccagggaagtccctttagggggg

SEQ ID NO: 44543 - DNA, 28 bp, synthetic construct
  source 1..28: mol_type = other DNA
cacttcccagggaagtccctttaggggg

SEQ ID NO: 44544 - DNA, 28 bp, synthetic construct
  source 1..28: mol_type = other DNA
tcacttcccagggaagtccctttagggg

SEQ ID NO: 44545 - DNA, 28 bp, synthetic construct
  source 1..28: mol_type = other DNA
gtcacttcccagggaagtccctttaggg

SEQ ID NO: 44546 - DNA, 28 bp, synthetic construct
  source 1..28: mol_type = other DNA
ggtcacttcccagggaagtccctttagg

SEQ ID NO: 44547 - DNA, 28 bp, synthetic construct
  source 1..28: mol_type = other DNA
cttccctgggaagtgaccatgtgccagg

SEQ ID NO: 44548 - DNA, 28 bp, synthetic construct
  source 1..28: mol_type = other DNA
cttcctggcacatggtcacttcccaggg

SEQ ID NO: 44549 - DNA, 28 bp, synthetic construct
  source 1..28: mol_type = other DNA
acttcctggcacatggtcacttcccagg

SEQ ID NO: 44550 - DNA, 28 bp, synthetic construct
  source 1..28: mol_type = other DNA
tgggaagtgaccatgtgccaggaagtgg

SEQ ID NO: 44551 - DNA, 28 bp, synthetic construct
  source 1..28: mol_type = other DNA
ccgcatcgctccacttcctggcacatgg

SEQ ID NO: 44552 - DNA, 28 bp, synthetic construct
  source 1..28: mol_type = other DNA
tgtgccaggaagtggagcgatgcggtgg

SEQ ID NO: 44553 - DNA, 28 bp, synthetic construct
  source 1..28: mol_type = other DNA
gtgccaggaagtggagcgatgcggtggg

SEQ ID NO: 44554 - DNA, 28 bp, synthetic construct
  source 1..28: mol_type = other DNA
gatcccaccgcatcgctccacttcctgg

SEQ ID NO: 44555 - DNA, 28 bp, synthetic construct
  source 1..28: mol_type = other DNA
gctcggtgtgcactttttgagagctagg

SEQ ID NO: 44556 - DNA, 28 bp, synthetic construct
  source 1..28: mol_type = other DNA
aaaaagtgcacaccgagcccgccgcagg

SEQ ID NO: 44557 - DNA, 28 bp, synthetic construct
  source 1..28: mol_type = other DNA
tgggcaaggacgcctgcggcgggctcgg

SEQ ID NO: 44558 - DNA, 28 bp, synthetic construct
  source 1..28: mol_type = other DNA
cccggtgggcaaggacgcctgcggcggg

SEQ ID NO: 44559 - DNA, 28 bp, synthetic construct
  source 1..28: mol_type = other DNA
tcccggtgggcaaggacgcctgcggcgg

SEQ ID NO: 44560 - DNA, 28 bp, synthetic construct
  source 1..28: mol_type = other DNA
ccttcccggtgggcaaggacgcctgcgg

SEQ ID NO: 44561 - DNA, 28 bp, synthetic construct
  source 1..28: mol_type = other DNA
gaaatcccagctactcgggaggctgagg

SEQ ID NO: 44562 - DNA, 28 bp, synthetic construct
  source 1..28: mol_type = other DNA
tcccagctactcgggaggctgaggtagg

SEQ ID NO: 44563 - DNA, 28 bp, synthetic construct
  source 1..28: mol_type = other DNA
cagctactcgggaggctgaggtaggagg

SEQ ID NO: 44564 - DNA, 28 bp, synthetic construct
  source 1..28: mol_type = other DNA
agctactcgggaggctgaggtaggaggg

SEQ ID NO: 44565 - DNA, 28 bp, synthetic construct
  source 1..28: mol_type = other DNA
tgaggtaggagggttgcttaagcccagg

SEQ ID NO: 44566 - DNA, 28 bp, synthetic construct
  source 1..28: mol_type = other DNA
taagcccaggagttcaagaccagcctgg

SEQ ID NO: 44567 - DNA, 28 bp, synthetic construct
  source 1..28: mol_type = other DNA
ttgtccaggctggtcttgaactcctggg

SEQ ID NO: 44568 - DNA, 28 bp, synthetic construct
  source 1..28: mol_type = other DNA
gttgtccaggctggtcttgaactcctgg

SEQ ID NO: 44569 - DNA, 28 bp, synthetic construct
  source 1..28: mol_type = other DNA
cagggtctcactatgttgtccaggctgg

SEQ ID NO: 44570 - DNA, 28 bp, synthetic construct
  source 1..28: mol_type = other DNA
gagacagggtctcactatgttgtccagg

SEQ ID NO: 44571 - DNA, 28 bp, synthetic construct
  source 1..28: mol_type = other DNA
tctactctttttgctgtttgagacaggg

SEQ ID NO: 44572 - DNA, 28 bp, synthetic construct
  source 1..28: mol_type = other DNA
atctactctttttgctgtttgagacagg

SEQ ID NO: 44573 - DNA, 28 bp, synthetic construct
  source 1..28: mol_type = other DNA
aacagcaaaaagagtagatctcctttgg

SEQ ID NO: 44574 - DNA, 28 bp, synthetic construct
  source 1..28: mol_type = other DNA
gtagatctcctttggttctaacaagagg

SEQ ID NO: 44575 - DNA, 28 bp, synthetic construct
  source 1..28: mol_type = other DNA
tagatctcctttggttctaacaagaggg

SEQ ID NO: 44576 - DNA, 28 bp, synthetic construct
  source 1..28: mol_type = other DNA
agatctcctttggttctaacaagagggg

SEQ ID NO: 44577 - DNA, 28 bp, synthetic construct
  source 1..28: mol_type = other DNA
tcacatcccctcttgttagaaccaaagg

SEQ ID NO: 44578 - DNA, 28 bp, synthetic construct
  source 1..28: mol_type = other DNA
acgaaaagacagcagagtggacagtggg

SEQ ID NO: 44579 - DNA, 28 bp, synthetic construct
  source 1..28: mol_type = other DNA
cacgaaaagacagcagagtggacagtgg

SEQ ID NO: 44580 - DNA, 28 bp, synthetic construct
  source 1..28: mol_type = other DNA
tccactctgctgtcttttcgtgcctcgg

SEQ ID NO: 44581 - DNA, 28 bp, synthetic construct
  source 1..28: mol_type = other DNA
accgaggcacgaaaagacagcagagtgg

SEQ ID NO: 44582 - DNA, 28 bp, synthetic construct
  source 1..28: mol_type = other DNA
cctcggtgtccccaagctgctgcccagg

SEQ ID NO: 44583 - DNA, 28 bp, synthetic construct
  source 1..28: mol_type = other DNA
ccttgggctcctgggcagcagcttgggg

SEQ ID NO: 44584 - DNA, 28 bp, synthetic construct
  source 1..28: mol_type = other DNA
cccaagctgctgcccaggagcccaaggg

SEQ ID NO: 44585 - DNA, 28 bp, synthetic construct
  source 1..28: mol_type = other DNA
acccttgggctcctgggcagcagcttgg

SEQ ID NO: 44586 - DNA, 28 bp, synthetic construct
  source 1..28: mol_type = other DNA
aagctgctgcccaggagcccaagggtgg

SEQ ID NO: 44587 - DNA, 28 bp, synthetic construct
  source 1..28: mol_type = other DNA
agctgctgcccaggagcccaagggtggg

SEQ ID NO: 44588 - DNA, 28 bp, synthetic construct
  source 1..28: mol_type = other DNA
aaagactgcccacccttgggctcctggg

SEQ ID NO: 44589 - DNA, 28 bp, synthetic construct
  source 1..28: mol_type = other DNA
caaagactgcccacccttgggctcctgg

SEQ ID NO: 44590 - DNA, 28 bp, synthetic construct
  source 1..28: mol_type = other DNA
tgtcagacaaagactgcccacccttggg

SEQ ID NO: 44591 - DNA, 28 bp, synthetic construct
  source 1..28: mol_type = other DNA
gtgtcagacaaagactgcccacccttgg

SEQ ID NO: 44592 - DNA, 28 bp, synthetic construct
  source 1..28: mol_type = other DNA
agggtgggcagtctttgtctgacacagg

SEQ ID NO: 44593 - DNA, 28 bp, synthetic construct
  source 1..28: mol_type = other DNA
acaggaaccccttcacttcacatttagg

SEQ ID NO: 44594 - DNA, 28 bp, synthetic construct
  source 1..28: mol_type = other DNA
caggaaccccttcacttcacatttaggg

SEQ ID NO: 44595 - DNA, 28 bp, synthetic construct
  source 1..28: mol_type = other DNA
aggaaccccttcacttcacatttagggg

SEQ ID NO: 44596 - DNA, 28 bp, synthetic construct
  source 1..28: mol_type = other DNA
tcaatcccctaaatgtgaagtgaagggg

SEQ ID NO: 44597 - DNA, 28 bp, synthetic construct
  source 1..28: mol_type = other DNA
ctcaatcccctaaatgtgaagtgaaggg

SEQ ID NO: 44598 - DNA, 28 bp, synthetic construct
  source 1..28: mol_type = other DNA
ccttcacttcacatttaggggattgagg

SEQ ID NO: 44599 - DNA, 28 bp, synthetic construct
  source 1..28: mol_type = other DNA
tcacatttaggggattgaggcctagtgg

SEQ ID NO: 44600 - DNA, 28 bp, synthetic construct
  source 1..28: mol_type = other DNA
ttaggggattgaggcctagtggagcagg

SEQ ID NO: 44601 - DNA, 28 bp, synthetic construct
  source 1..28: mol_type = other DNA
taggggattgaggcctagtggagcaggg

SEQ ID NO: 44602 - DNA, 28 bp, synthetic construct
  source 1..28: mol_type = other DNA
gcctagtggagcagggactcacccacgg

SEQ ID NO: 44603 - DNA, 28 bp, synthetic construct
  source 1..28: mol_type = other DNA
gccgtgggtgagtccctgctccactagg

SEQ ID NO: 44604 - DNA, 28 bp, synthetic construct
  source 1..28: mol_type = other DNA
agcagggactcacccacggccacacagg

SEQ ID NO: 44605 - DNA, 28 bp, synthetic construct
  source 1..28: mol_type = other DNA
gcagggactcacccacggccacacaggg

SEQ ID NO: 44606 - DNA, 28 bp, synthetic construct
  source 1..28: mol_type = other DNA
cagggactcacccacggccacacagggg

SEQ ID NO: 44607 - DNA, 28 bp, synthetic construct
  source 1..28: mol_type = other DNA
agggactcacccacggccacacaggggg

SEQ ID NO: 44608 - DNA, 28 bp, synthetic construct
  source 1..28: mol_type = other DNA
taattctgaccccctgtgtggccgtggg

SEQ ID NO: 44609 - DNA, 28 bp, synthetic construct
  source 1..28: mol_type = other DNA
gtaattctgaccccctgtgtggccgtgg

SEQ ID NO: 44610 - DNA, 28 bp, synthetic construct
  source 1..28: mol_type = other DNA
tcaacagtaattctgaccccctgtgtgg

SEQ ID NO: 44611 - DNA, 28 bp, synthetic construct
  source 1..28: mol_type = other DNA
acacagggggtcagaattactgttgagg

SEQ ID NO: 44612 - DNA, 28 bp, synthetic construct
  source 1..28: mol_type = other DNA
ttggaactgaaacaattctggattctgg

SEQ ID NO: 44613 - DNA, 28 bp, synthetic construct
  source 1..28: mol_type = other DNA
atccagaattgtttcagttccaaccagg

SEQ ID NO: 44614 - DNA, 28 bp, synthetic construct
  source 1..28: mol_type = other DNA
ttcctggttggaactgaaacaattctgg

SEQ ID NO: 44615 - DNA, 28 bp, synthetic construct
  source 1..28: mol_type = other DNA
agaattgtttcagttccaaccaggaagg

SEQ ID NO: 44616 - DNA, 28 bp, synthetic construct
  source 1..28: mol_type = other DNA
gaattgtttcagttccaaccaggaaggg

SEQ ID NO: 44617 - DNA, 28 bp, synthetic construct
  source 1..28: mol_type = other DNA
aattgtttcagttccaaccaggaagggg

SEQ ID NO: 44618 - DNA, 28 bp, synthetic construct
  source 1..28: mol_type = other DNA
tttgggaaacaaaccccttcctggttgg

SEQ ID NO: 44619 - DNA, 28 bp, synthetic construct
  source 1..28: mol_type = other DNA
aggttttgggaaacaaaccccttcctgg

SEQ ID NO: 44620 - DNA, 28 bp, synthetic construct
  source 1..28: mol_type = other DNA
aaggggtggggtagggacaggttttggg

SEQ ID NO: 44621 - DNA, 28 bp, synthetic construct
  source 1..28: mol_type = other DNA
gaaggggtggggtagggacaggttttgg

SEQ ID NO: 44622 - DNA, 28 bp, synthetic construct
  source 1..28: mol_type = other DNA
acctgtccctaccccaccccttctttgg

SEQ ID NO: 44623 - DNA, 28 bp, synthetic construct
  source 1..28: mol_type = other DNA
gccaaagaaggggtggggtagggacagg

SEQ ID NO: 44624 - DNA, 28 bp, synthetic construct
  source 1..28: mol_type = other DNA
gtccctaccccaccccttctttggcagg

SEQ ID NO: 44625 - DNA, 28 bp, synthetic construct
  source 1..28: mol_type = other DNA
cgcctgccaaagaaggggtggggtaggg

SEQ ID NO: 44626 - DNA, 28 bp, synthetic construct
  source 1..28: mol_type = other DNA
cctaccccaccccttctttggcaggcgg

SEQ ID NO: 44627 - DNA, 28 bp, synthetic construct
  source 1..28: mol_type = other DNA
tactccgcctgccaaagaaggggtgggg

SEQ ID NO: 44628 - DNA, 28 bp, synthetic construct
  source 1..28: mol_type = other DNA
ctactccgcctgccaaagaaggggtggg

SEQ ID NO: 44629 - DNA, 28 bp, synthetic construct
  source 1..28: mol_type = other DNA
gctactccgcctgccaaagaaggggtgg

SEQ ID NO: 44630 - DNA, 28 bp, synthetic construct
  source 1..28: mol_type = other DNA
acagctactccgcctgccaaagaagggg

SEQ ID NO: 44631 - DNA, 28 bp, synthetic construct
  source 1..28: mol_type = other DNA
gacagctactccgcctgccaaagaaggg

SEQ ID NO: 44632 - DNA, 28 bp, synthetic construct
  source 1..28: mol_type = other DNA
cgacagctactccgcctgccaaagaagg

SEQ ID NO: 44633 - DNA, 28 bp, synthetic construct
  source 1..28: mol_type = other DNA
ggcaggcggagtagctgtcgccctcagg

SEQ ID NO: 44634 - DNA, 28 bp, synthetic construct
  source 1..28: mol_type = other DNA
gcaggcggagtagctgtcgccctcaggg

SEQ ID NO: 44635 - DNA, 28 bp, synthetic construct
  source 1..28: mol_type = other DNA
ggcggagtagctgtcgccctcagggtgg

SEQ ID NO: 44636 - DNA, 28 bp, synthetic construct
  source 1..28: mol_type = other DNA
ccctcagggtggcccagagcagtgctgg

SEQ ID NO: 44637 - DNA, 28 bp, synthetic construct
  source 1..28: mol_type = other DNA
cctcagggtggcccagagcagtgctggg

SEQ ID NO: 44638 - DNA, 28 bp, synthetic construct
  source 1..28: mol_type = other DNA
ctcagggtggcccagagcagtgctgggg

SEQ ID NO: 44639 - DNA, 28 bp, synthetic construct
  source 1..28: mol_type = other DNA
tcagggtggcccagagcagtgctggggg

SEQ ID NO: 44640 - DNA, 28 bp, synthetic construct
  source 1..28: mol_type = other DNA
tcatctctacccccagcactgctctggg

SEQ ID NO: 44641 - DNA, 28 bp, synthetic construct
  source 1..28: mol_type = other DNA
ttcatctctacccccagcactgctctgg

SEQ ID NO: 44642 - DNA, 28 bp, synthetic construct
  source 1..28: mol_type = other DNA
agagcagtgctgggggtagagatgaagg

SEQ ID NO: 44643 - DNA, 28 bp, synthetic construct
  source 1..28: mol_type = other DNA
gtgccttgtgaagacactgccaagaagg

SEQ ID NO: 44644 - DNA, 28 bp, synthetic construct
  source 1..28: mol_type = other DNA
tgccttgtgaagacactgccaagaaggg

SEQ ID NO: 44645 - DNA, 28 bp, synthetic construct
  source 1..28: mol_type = other DNA
gccttgtgaagacactgccaagaagggg

SEQ ID NO: 44646 - DNA, 28 bp, synthetic construct
  source 1..28: mol_type = other DNA
accccttcttggcagtgtcttcacaagg

SEQ ID NO: 44647 - DNA, 28 bp, synthetic construct
  source 1..28: mol_type = other DNA
ttgtgaagacactgccaagaaggggtgg

SEQ ID NO: 44648 - DNA, 28 bp, synthetic construct
  source 1..28: mol_type = other DNA
tgtgaagacactgccaagaaggggtggg

SEQ ID NO: 44649 - DNA, 28 bp, synthetic construct
  source 1..28: mol_type = other DNA
gtgaagacactgccaagaaggggtgggg

SEQ ID NO: 44650 - DNA, 28 bp, synthetic construct
  source 1..28: mol_type = other DNA
tcttggaagttgccccaccccttcttgg

SEQ ID NO: 44651 - DNA, 28 bp, synthetic construct
  source 1..28: mol_type = other DNA
aagaaggggtggggcaacttccaagagg

SEQ ID NO: 44652 - DNA, 28 bp, synthetic construct
  source 1..28: mol_type = other DNA
ttgggcttcttggtgctcttcctcttgg

SEQ ID NO: 44653 - DNA, 28 bp, synthetic construct
  source 1..28: mol_type = other DNA
agcaccaagaagcccaaaccccagacgg

SEQ ID NO: 44654 - DNA, 28 bp, synthetic construct
  source 1..28: mol_type = other DNA
gtttccgtctggggtttgggcttcttgg

SEQ ID NO: 44655 - DNA, 28 bp, synthetic construct
  source 1..28: mol_type = other DNA
tacatttggtttccgtctggggtttggg

SEQ ID NO: 44656 - DNA, 28 bp, synthetic construct
  source 1..28: mol_type = other DNA
atacatttggtttccgtctggggtttgg

SEQ ID NO: 44657 - DNA, 28 bp, synthetic construct
  source 1..28: mol_type = other DNA
agaaaatacatttggtttccgtctgggg

SEQ ID NO: 44658 - DNA, 28 bp, synthetic construct
  source 1..28: mol_type = other DNA
cagaaaatacatttggtttccgtctggg

SEQ ID NO: 44659 - DNA, 28 bp, synthetic construct
  source 1..28: mol_type = other DNA
ccagaaaatacatttggtttccgtctgg

SEQ ID NO: 44660 - DNA, 28 bp, synthetic construct
  source 1..28: mol_type = other DNA
cagacggaaaccaaatgtattttctggg

SEQ ID NO: 44661 - DNA, 28 bp, synthetic construct
  source 1..28: mol_type = other DNA
ccaaatgtattttctgggccctgagagg

SEQ ID NO: 44662 - DNA, 28 bp, synthetic construct
  source 1..28: mol_type = other DNA
attttctgggccctgagaggatatttgg

SEQ ID NO: 44663 - DNA, 28 bp, synthetic construct
  source 1..28: mol_type = other DNA
ggccctgagaggatatttggaacaatgg

SEQ ID NO: 44664 - DNA, 28 bp, synthetic construct
  source 1..28: mol_type = other DNA
ctccattgttccaaatatcctctcaggg

SEQ ID NO: 44665 - DNA, 28 bp, synthetic construct
  source 1..28: mol_type = other DNA
cctgagaggatatttggaacaatggagg

SEQ ID NO: 44666 - DNA, 28 bp, synthetic construct
  source 1..28: mol_type = other DNA
gagaggatatttggaacaatggaggtgg

SEQ ID NO: 44667 - DNA, 28 bp, synthetic construct
  source 1..28: mol_type = other DNA
agaggatatttggaacaatggaggtggg

SEQ ID NO: 44668 - DNA, 28 bp, synthetic construct
  source 1..28: mol_type = other DNA
tatttggaacaatggaggtgggatgagg

SEQ ID NO: 44669 - DNA, 28 bp, synthetic construct
  source 1..28: mol_type = other DNA
atttggaacaatggaggtgggatgaggg

SEQ ID NO: 44670 - DNA, 28 bp, synthetic construct
  source 1..28: mol_type = other DNA
ggaggtgggatgagggaagttaaaaagg

SEQ ID NO: 44671 - DNA, 28 bp, synthetic construct
  source 1..28: mol_type = other DNA
gaggtgggatgagggaagttaaaaaggg

SEQ ID NO: 44672 - DNA, 28 bp, synthetic construct
  source 1..28: mol_type = other DNA
tgatatccttagaaaaaaaaaatacagg

SEQ ID NO: 44673 - DNA, 28 bp, synthetic construct
  source 1..28: mol_type = other DNA
ttaaagcctgtattttttttttctaagg

SEQ ID NO: 44674 - DNA, 28 bp, synthetic construct
  source 1..28: mol_type = other DNA
ttaagtttgacttttgtttctctgaagg

SEQ ID NO: 44675 - DNA, 28 bp, synthetic construct
  source 1..28: mol_type = other DNA
gaaggatgtttgtgtaactttctgaagg

SEQ ID NO: 44676 - DNA, 28 bp, synthetic construct
  source 1..28: mol_type = other DNA
gatgtttgtgtaactttctgaaggcagg

SEQ ID NO: 44677 - DNA, 28 bp, synthetic construct
  source 1..28: mol_type = other DNA
catctgacaagcttcacagagtgctggg

SEQ ID NO: 44678 - DNA, 28 bp, synthetic construct
  source 1..28: mol_type = other DNA
gcatctgacaagcttcacagagtgctgg

SEQ ID NO: 44679 - DNA, 28 bp, synthetic construct
  source 1..28: mol_type = other DNA
tgagacagagtctgctctgttgcccagg

SEQ ID NO: 44680 - DNA, 28 bp, synthetic construct
  source 1..28: mol_type = other DNA
acagagtctgctctgttgcccaggctgg

SEQ ID NO: 44681 - DNA, 28 bp, synthetic construct
  source 1..28: mol_type = other DNA
ctctgttgcccaggctggagtgcagtgg

SEQ ID NO: 44682 - DNA, 28 bp, synthetic construct
  source 1..28: mol_type = other DNA
agatcgcgccactgcactccagcctggg

SEQ ID NO: 44683 - DNA, 28 bp, synthetic construct
  source 1..28: mol_type = other DNA
aagatcgcgccactgcactccagcctgg

SEQ ID NO: 44684 - DNA, 28 bp, synthetic construct
  source 1..28: mol_type = other DNA
aggctggagtgcagtggcgcgatcttgg

SEQ ID NO: 44685 - DNA, 28 bp, synthetic construct
  source 1..28: mol_type = other DNA
ttggctcactgcagcctccatctcccgg

SEQ ID NO: 44686 - DNA, 28 bp, synthetic construct
  source 1..28: mol_type = other DNA
tggctcactgcagcctccatctcccggg

SEQ ID NO: 44687 - DNA, 28 bp, synthetic construct
  source 1..28: mol_type = other DNA
agaatcgcttgaacccgggagatggagg

SEQ ID NO: 44688 - DNA, 28 bp, synthetic construct
  source 1..28: mol_type = other DNA
aggagaatcgcttgaacccgggagatgg

SEQ ID NO: 44689 - DNA, 28 bp, synthetic construct
  source 1..28: mol_type = other DNA
cgaggcaggagaatcgcttgaacccggg

SEQ ID NO: 44690 - DNA, 28 bp, synthetic construct
  source 1..28: mol_type = other DNA
ccgaggcaggagaatcgcttgaacccgg

SEQ ID NO: 44691 - DNA, 28 bp, synthetic construct
  source 1..28: mol_type = other DNA
ctcctgcctcggcctcccgaatagctgg

SEQ ID NO: 44692 - DNA, 28 bp, synthetic construct
  source 1..28: mol_type = other DNA
tcctgcctcggcctcccgaatagctggg

SEQ ID NO: 44693 - DNA, 28 bp, synthetic construct
  source 1..28: mol_type = other DNA
tcccagctattcgggaggccgaggcagg

SEQ ID NO: 44694 - DNA, 28 bp, synthetic construct
  source 1..28: mol_type = other DNA
gtaatcccagctattcgggaggccgagg

SEQ ID NO: 44695 - DNA, 28 bp, synthetic construct
  source 1..28: mol_type = other DNA
cggcctcccgaatagctgggattactgg

SEQ ID NO: 44696 - DNA, 28 bp, synthetic construct
  source 1..28: mol_type = other DNA
acaccagtaatcccagctattcgggagg

SEQ ID NO: 44697 - DNA, 28 bp, synthetic construct
  source 1..28: mol_type = other DNA
cacacaccagtaatcccagctattcggg

SEQ ID NO: 44698 - DNA, 28 bp, synthetic construct
  source 1..28: mol_type = other DNA
gcacacaccagtaatcccagctattcgg

SEQ ID NO: 44699 - DNA, 28 bp, synthetic construct
  source 1..28: mol_type = other DNA
acaaaaaaaatttagctgggtatggtgg

SEQ ID NO: 44700 - DNA, 28 bp, synthetic construct
  source 1..28: mol_type = other DNA
aatacaaaaaaaatttagctgggtatgg

SEQ ID NO: 44701 - DNA, 28 bp, synthetic construct
  source 1..28: mol_type = other DNA
ctaaaaatacaaaaaaaatttagctggg

SEQ ID NO: 44702 - DNA, 28 bp, synthetic construct
  source 1..28: mol_type = other DNA
actaaaaatacaaaaaaaatttagctgg

SEQ ID NO: 44703 - DNA, 28 bp, synthetic construct
  source 1..28: mol_type = other DNA
attttttttgtatttttagtagagacgg

SEQ ID NO: 44704 - DNA, 28 bp, synthetic construct
  source 1..28: mol_type = other DNA
ttttttttgtatttttagtagagacggg

SEQ ID NO: 44705 - DNA, 28 bp, synthetic construct
  source 1..28: mol_type = other DNA
tttttttgtatttttagtagagacgggg

SEQ ID NO: 44706 - DNA, 28 bp, synthetic construct
  source 1..28: mol_type = other DNA
gagacggggtttcaccatattgaccagg

SEQ ID NO: 44707 - DNA, 28 bp, synthetic construct
  source 1..28: mol_type = other DNA
cggggtttcaccatattgaccaggctgg

SEQ ID NO: 44708 - DNA, 28 bp, synthetic construct
  source 1..28: mol_type = other DNA
gagttcgagaccagcctggtcaatatgg

SEQ ID NO: 44709 - DNA, 28 bp, synthetic construct
  source 1..28: mol_type = other DNA
tgaggtcaggagttcgagaccagcctgg

SEQ ID NO: 44710 - DNA, 28 bp, synthetic construct
  source 1..28: mol_type = other DNA
aggctggtctcgaactcctgacctcagg

SEQ ID NO: 44711 - DNA, 28 bp, synthetic construct
  source 1..28: mol_type = other DNA
caaagcaggcagatcacctgaggtcagg

SEQ ID NO: 44712 - DNA, 28 bp, synthetic construct
  source 1..28: mol_type = other DNA
ctgacctcaggtgatctgcctgctttgg

SEQ ID NO: 44713 - DNA, 28 bp, synthetic construct
  source 1..28: mol_type = other DNA
gaggccaaagcaggcagatcacctgagg

SEQ ID NO: 44714 - DNA, 28 bp, synthetic construct
  source 1..28: mol_type = other DNA
tgcctgctttggcctcccaaagtgctgg

SEQ ID NO: 44715 - DNA, 28 bp, synthetic construct
  source 1..28: mol_type = other DNA
gcctgctttggcctcccaaagtgctggg

SEQ ID NO: 44716 - DNA, 28 bp, synthetic construct
  source 1..28: mol_type = other DNA
tcccagcactttgggaggccaaagcagg

SEQ ID NO: 44717 - DNA, 28 bp, synthetic construct
  source 1..28: mol_type = other DNA
tggcctcccaaagtgctgggattgcagg

SEQ ID NO: 44718 - DNA, 28 bp, synthetic construct
  source 1..28: mol_type = other DNA
atgcctgcaatcccagcactttgggagg

SEQ ID NO: 44719 - DNA, 28 bp, synthetic construct
  source 1..28: mol_type = other DNA
ctcatgcctgcaatcccagcactttggg

SEQ ID NO: 44720 - DNA, 28 bp, synthetic construct
  source 1..28: mol_type = other DNA
gctcatgcctgcaatcccagcactttgg

SEQ ID NO: 44721 - DNA, 28 bp, synthetic construct
  source 1..28: mol_type = other DNA
gattgcaggcatgagctaccacgcctgg

SEQ ID NO: 44722 - DNA, 28 bp, synthetic construct
  source 1..28: mol_type = other DNA
gcatgagctaccacgcctggccattagg

SEQ ID NO: 44723 - DNA, 28 bp, synthetic construct
  source 1..28: mol_type = other DNA
aaaaacagcacctaatggccaggcgtgg

SEQ ID NO: 44724 - DNA, 28 bp, synthetic construct
  source 1..28: mol_type = other DNA
tctataaaaacagcacctaatggccagg

SEQ ID NO: 44725 - DNA, 28 bp, synthetic construct
  source 1..28: mol_type = other DNA
ctgaatctataaaaacagcacctaatgg

SEQ ID NO: 44726 - DNA, 28 bp, synthetic construct
  source 1..28: mol_type = other DNA
cattaggtgctgtttttatagattcagg

SEQ ID NO: 44727 - DNA, 28 bp, synthetic construct
  source 1..28: mol_type = other DNA
attaggtgctgtttttatagattcaggg

SEQ ID NO: 44728 - DNA, 28 bp, synthetic construct
  source 1..28: mol_type = other DNA
tgctgtttttatagattcagggctttgg

SEQ ID NO: 44729 - DNA, 28 bp, synthetic construct
  source 1..28: mol_type = other DNA
ttttatagattcagggctttggagctgg

SEQ ID NO: 44730 - DNA, 28 bp, synthetic construct
  source 1..28: mol_type = other DNA
tttatagattcagggctttggagctggg

SEQ ID NO: 44731 - DNA, 28 bp, synthetic construct
  source 1..28: mol_type = other DNA
tagattcagggctttggagctgggaagg

SEQ ID NO: 44732 - DNA, 28 bp, synthetic construct
  source 1..28: mol_type = other DNA
tcaagtagtctcctcactttatagttgg

SEQ ID NO: 44733 - DNA, 28 bp, synthetic construct
  source 1..28: mol_type = other DNA
tctcctcactttatagttggtgaaatgg

SEQ ID NO: 44734 - DNA, 28 bp, synthetic construct
  source 1..28: mol_type = other DNA
cctccatttcaccaactataaagtgagg

SEQ ID NO: 44735 - DNA, 28 bp, synthetic construct
  source 1..28: mol_type = other DNA
tatagttggtgaaatggaggctgagagg

SEQ ID NO: 44736 - DNA, 28 bp, synthetic construct
  source 1..28: mol_type = other DNA
agttggtgaaatggaggctgagaggtgg

SEQ ID NO: 44737 - DNA, 28 bp, synthetic construct
  source 1..28: mol_type = other DNA
gttggtgaaatggaggctgagaggtggg

SEQ ID NO: 44738 - DNA, 28 bp, synthetic construct
  source 1..28: mol_type = other DNA
ttggtgaaatggaggctgagaggtgggg

SEQ ID NO: 44739 - DNA, 28 bp, synthetic construct
  source 1..28: mol_type = other DNA
tggtgaaatggaggctgagaggtggggg

SEQ ID NO: 44740 - DNA, 28 bp, synthetic construct
  source 1..28: mol_type = other DNA
ggtgaaatggaggctgagaggtgggggg

SEQ ID NO: 44741 - DNA, 28 bp, synthetic construct
  source 1..28: mol_type = other DNA
ggctgagaggtggggggcctgcttgagg

SEQ ID NO: 44742 - DNA, 28 bp, synthetic construct
  source 1..28: mol_type = other DNA
ggggcctgcttgaggtcacacagtgagg

SEQ ID NO: 44743 - DNA, 28 bp, synthetic construct
  source 1..28: mol_type = other DNA
gctgcctcactgtgtgacctcaagcagg

SEQ ID NO: 44744 - DNA, 28 bp, synthetic construct
  source 1..28: mol_type = other DNA
ttgaggtcacacagtgaggcagccgagg

SEQ ID NO: 44745 - DNA, 28 bp, synthetic construct
  source 1..28: mol_type = other DNA
tcacacagtgaggcagccgaggtcttgg

SEQ ID NO: 44746 - DNA, 28 bp, synthetic construct
  source 1..28: mol_type = other DNA
caacacataggaagatccaagacctcgg

SEQ ID NO: 44747 - DNA, 28 bp, synthetic construct
  source 1..28: mol_type = other DNA
cttggatcttcctatgtgttgcaagagg

SEQ ID NO: 44748 - DNA, 28 bp, synthetic construct
  source 1..28: mol_type = other DNA
agatggacagcctcttgcaacacatagg

SEQ ID NO: 44749 - DNA, 28 bp, synthetic construct
  source 1..28: mol_type = other DNA
ctgtccatcttgacttaccacctcctgg

SEQ ID NO: 44750 - DNA, 28 bp, synthetic construct
  source 1..28: mol_type = other DNA
tgtccatcttgacttaccacctcctggg

SEQ ID NO: 44751 - DNA, 28 bp, synthetic construct
  source 1..28: mol_type = other DNA
ggtcccaggaggtggtaagtcaagatgg

SEQ ID NO: 44752 - DNA, 28 bp, synthetic construct
  source 1..28: mol_type = other DNA
tcttgacttaccacctcctgggacctgg

SEQ ID NO: 44753 - DNA, 28 bp, synthetic construct
  source 1..28: mol_type = other DNA
gacttaccacctcctgggacctggctgg

SEQ ID NO: 44754 - DNA, 28 bp, synthetic construct
  source 1..28: mol_type = other DNA
accacctcctgggacctggctggcatgg

SEQ ID NO: 44755 - DNA, 28 bp, synthetic construct
  source 1..28: mol_type = other DNA
ccacctcctgggacctggctggcatggg

SEQ ID NO: 44756 - DNA, 28 bp, synthetic construct
  source 1..28: mol_type = other DNA
cacctcctgggacctggctggcatgggg

SEQ ID NO: 44757 - DNA, 28 bp, synthetic construct
  source 1..28: mol_type = other DNA
acctcctgggacctggctggcatggggg

SEQ ID NO: 44758 - DNA, 28 bp, synthetic construct
  source 1..28: mol_type = other DNA
gcccccatgccagccaggtcccaggagg

SEQ ID NO: 44759 - DNA, 28 bp, synthetic construct
  source 1..28: mol_type = other DNA
ccagcccccatgccagccaggtcccagg

SEQ ID NO: 44760 - DNA, 28 bp, synthetic construct
  source 1..28: mol_type = other DNA
ctgggacctggctggcatgggggctggg

SEQ ID NO: 44761 - DNA, 28 bp, synthetic construct
  source 1..28: mol_type = other DNA
ggacctggctggcatgggggctgggcgg

SEQ ID NO: 44762 - DNA, 28 bp, synthetic construct
  source 1..28: mol_type = other DNA
tgaccgcccagcccccatgccagccagg

SEQ ID NO: 44763 - DNA, 28 bp, synthetic construct
  source 1..28: mol_type = other DNA
catgggggctgggcggtcactgatgagg

SEQ ID NO: 44764 - DNA, 28 bp, synthetic construct
  source 1..28: mol_type = other DNA
atgggggctgggcggtcactgatgaggg

SEQ ID NO: 44765 - DNA, 28 bp, synthetic construct
  source 1..28: mol_type = other DNA
tgggggctgggcggtcactgatgagggg

SEQ ID NO: 44766 - DNA, 28 bp, synthetic construct
  source 1..28: mol_type = other DNA
ttcccttcaaaatgctcattgctgctgg

SEQ ID NO: 44767 - DNA, 28 bp, synthetic construct
  source 1..28: mol_type = other DNA
tcccttcaaaatgctcattgctgctggg

SEQ ID NO: 44768 - DNA, 28 bp, synthetic construct
  source 1..28: mol_type = other DNA
cccttcaaaatgctcattgctgctgggg

SEQ ID NO: 44769 - DNA, 28 bp, synthetic construct
  source 1..28: mol_type = other DNA
tccccagcagcaatgagcattttgaagg

SEQ ID NO: 44770 - DNA, 28 bp, synthetic construct
  source 1..28: mol_type = other DNA
caaaatgctcattgctgctggggatagg

SEQ ID NO: 44771 - DNA, 28 bp, synthetic construct
  source 1..28: mol_type = other DNA
gctcattgctgctggggataggataagg

SEQ ID NO: 44772 - DNA, 28 bp, synthetic construct
  source 1..28: mol_type = other DNA
ttgctgctggggataggataaggccagg

SEQ ID NO: 44773 - DNA, 28 bp, synthetic construct
  source 1..28: mol_type = other DNA
gctggggataggataaggccaggtctgg

SEQ ID NO: 44774 - DNA, 28 bp, synthetic construct
  source 1..28: mol_type = other DNA
gataggataaggccaggtctggtcttgg

SEQ ID NO: 44775 - DNA, 28 bp, synthetic construct
  source 1..28: mol_type = other DNA
ataggataaggccaggtctggtcttggg

SEQ ID NO: 44776 - DNA, 28 bp, synthetic construct
  source 1..28: mol_type = other DNA
ggctcatcttgcccaagaccagacctgg

SEQ ID NO: 44777 - DNA, 28 bp, synthetic construct
  source 1..28: mol_type = other DNA
ctggtcttgggcaagatgagcccactgg

SEQ ID NO: 44778 - DNA, 28 bp, synthetic construct
  source 1..28: mol_type = other DNA
gtcttgggcaagatgagcccactggtgg

SEQ ID NO: 44779 - DNA, 28 bp, synthetic construct
  source 1..28: mol_type = other DNA
tcttgggcaagatgagcccactggtggg

SEQ ID NO: 44780 - DNA, 28 bp, synthetic construct
  source 1..28: mol_type = other DNA
cttgggcaagatgagcccactggtgggg

SEQ ID NO: 44781 - DNA, 28 bp, synthetic construct
  source 1..28: mol_type = other DNA
caagatgagcccactggtggggagaagg

SEQ ID NO: 44782 - DNA, 28 bp, synthetic construct
  source 1..28: mol_type = other DNA
ccatctcagccttctccccaccagtggg

SEQ ID NO: 44783 - DNA, 28 bp, synthetic construct
  source 1..28: mol_type = other DNA
accatctcagccttctccccaccagtgg

SEQ ID NO: 44784 - DNA, 28 bp, synthetic construct
  source 1..28: mol_type = other DNA
ggggagaaggctgagatggtacacctgg

SEQ ID NO: 44785 - DNA, 28 bp, synthetic construct
  source 1..28: mol_type = other DNA
gcatctggatgagggtggcattaccagg

SEQ ID NO: 44786 - DNA, 28 bp, synthetic construct
  source 1..28: mol_type = other DNA
gtaatgccaccctcatccagatgccagg

SEQ ID NO: 44787 - DNA, 28 bp, synthetic construct
  source 1..28: mol_type = other DNA
gctgggcctggcatctggatgagggtgg

SEQ ID NO: 44788 - DNA, 28 bp, synthetic construct
  source 1..28: mol_type = other DNA
acagctgggcctggcatctggatgaggg

SEQ ID NO: 44789 - DNA, 28 bp, synthetic construct
  source 1..28: mol_type = other DNA
cacagctgggcctggcatctggatgagg

SEQ ID NO: 44790 - DNA, 28 bp, synthetic construct
  source 1..28: mol_type = other DNA
acggtgcacagctgggcctggcatctgg

SEQ ID NO: 44791 - DNA, 28 bp, synthetic construct
  source 1..28: mol_type = other DNA
tgggcagacggtgcacagctgggcctgg

SEQ ID NO: 44792 - DNA, 28 bp, synthetic construct
  source 1..28: mol_type = other DNA
gctgctgggcagacggtgcacagctggg

SEQ ID NO: 44793 - DNA, 28 bp, synthetic construct
  source 1..28: mol_type = other DNA
agctgctgggcagacggtgcacagctgg

SEQ ID NO: 44794 - DNA, 28 bp, synthetic construct
  source 1..28: mol_type = other DNA
agctgtgcaccgtctgcccagcagctgg

SEQ ID NO: 44795 - DNA, 28 bp, synthetic construct
  source 1..28: mol_type = other DNA
gctgtgcaccgtctgcccagcagctggg

SEQ ID NO: 44796 - DNA, 28 bp, synthetic construct
  source 1..28: mol_type = other DNA
tcacagctcccagctgctgggcagacgg

SEQ ID NO: 44797 - DNA, 28 bp, synthetic construct
  source 1..28: mol_type = other DNA
gtgtgactcacagctcccagctgctggg

SEQ ID NO: 44798 - DNA, 28 bp, synthetic construct
  source 1..28: mol_type = other DNA
ggtgtgactcacagctcccagctgctgg

SEQ ID NO: 44799 - DNA, 28 bp, synthetic construct
  source 1..28: mol_type = other DNA
gctgggagctgtgagtcacacccagtgg

SEQ ID NO: 44800 - DNA, 28 bp, synthetic construct
  source 1..28: mol_type = other DNA
tgtgagtcacacccagtggatacagagg

SEQ ID NO: 44801 - DNA, 28 bp, synthetic construct
  source 1..28: mol_type = other DNA
tcacacccagtggatacagaggcgcagg

SEQ ID NO: 44802 - DNA, 28 bp, synthetic construct
  source 1..28: mol_type = other DNA
aatggcctgcgcctctgtatccactggg

SEQ ID NO: 44803 - DNA, 28 bp, synthetic construct
  source 1..28: mol_type = other DNA
caatggcctgcgcctctgtatccactgg

SEQ ID NO: 44804 - DNA, 28 bp, synthetic construct
  source 1..28: mol_type = other DNA
gaacagaatgaatcacggcacacaatgg

SEQ ID NO: 44805 - DNA, 28 bp, synthetic construct
  source 1..28: mol_type = other DNA
tgtgccgtgattcattctgttctcccgg

SEQ ID NO: 44806 - DNA, 28 bp, synthetic construct
  source 1..28: mol_type = other DNA
ggggccgggagaacagaatgaatcacgg

SEQ ID NO: 44807 - DNA, 28 bp, synthetic construct
  source 1..28: mol_type = other DNA
attcattctgttctcccggccccgaagg

SEQ ID NO: 44808 - DNA, 28 bp, synthetic construct
  source 1..28: mol_type = other DNA
ttcattctgttctcccggccccgaaggg

SEQ ID NO: 44809 - DNA, 28 bp, synthetic construct
  source 1..28: mol_type = other DNA
ttctcccggccccgaagggatgacgagg

SEQ ID NO: 44810 - DNA, 28 bp, synthetic construct
  source 1..28: mol_type = other DNA
agggcctcgtcatcccttcggggccggg

SEQ ID NO: 44811 - DNA, 28 bp, synthetic construct
  source 1..28: mol_type = other DNA
cagggcctcgtcatcccttcggggccgg

SEQ ID NO: 44812 - DNA, 28 bp, synthetic construct
  source 1..28: mol_type = other DNA
tgctcagggcctcgtcatcccttcgggg

SEQ ID NO: 44813 - DNA, 28 bp, synthetic construct
  source 1..28: mol_type = other DNA
gtgctcagggcctcgtcatcccttcggg

SEQ ID NO: 44814 - DNA, 28 bp, synthetic construct
  source 1..28: mol_type = other DNA
ggtgctcagggcctcgtcatcccttcgg

SEQ ID NO: 44815 - DNA, 28 bp, synthetic construct
  source 1..28: mol_type = other DNA
aggcgtgggcatggatcggtgctcaggg

SEQ ID NO: 44816 - DNA, 28 bp, synthetic construct
  source 1..28: mol_type = other DNA
caggcgtgggcatggatcggtgctcagg

SEQ ID NO: 44817 - DNA, 28 bp, synthetic construct
  source 1..28: mol_type = other DNA
gagcaccgatccatgcccacgcctgtgg

SEQ ID NO: 44818 - DNA, 28 bp, synthetic construct
  source 1..28: mol_type = other DNA
ttcatccacaggcgtgggcatggatcgg

SEQ ID NO: 44819 - DNA, 28 bp, synthetic construct
  source 1..28: mol_type = other DNA
cagctttcatccacaggcgtgggcatgg

SEQ ID NO: 44820 - DNA, 28 bp, synthetic construct
  source 1..28: mol_type = other DNA
catatcagctttcatccacaggcgtggg

SEQ ID NO: 44821 - DNA, 28 bp, synthetic construct
  source 1..28: mol_type = other DNA
tcatatcagctttcatccacaggcgtgg

SEQ ID NO: 44822 - DNA, 28 bp, synthetic construct
  source 1..28: mol_type = other DNA
acgcctgtggatgaaagctgatatgagg

SEQ ID NO: 44823 - DNA, 28 bp, synthetic construct
  source 1..28: mol_type = other DNA
cctgtggatgaaagctgatatgaggagg

SEQ ID NO: 44824 - DNA, 28 bp, synthetic construct
  source 1..28: mol_type = other DNA
gatgaaagctgatatgaggaggcccagg

SEQ ID NO: 44825 - DNA, 28 bp, synthetic construct
  source 1..28: mol_type = other DNA
atgaaagctgatatgaggaggcccaggg

SEQ ID NO: 44826 - DNA, 28 bp, synthetic construct
  source 1..28: mol_type = other DNA
tgaaagctgatatgaggaggcccagggg

SEQ ID NO: 44827 - DNA, 28 bp, synthetic construct
  source 1..28: mol_type = other DNA
gatatgaggaggcccaggggacctgagg

SEQ ID NO: 44828 - DNA, 28 bp, synthetic construct
  source 1..28: mol_type = other DNA
atatgaggaggcccaggggacctgaggg

SEQ ID NO: 44829 - DNA, 28 bp, synthetic construct
  source 1..28: mol_type = other DNA
ggaggcccaggggacctgagggagtcgg

SEQ ID NO: 44830 - DNA, 28 bp, synthetic construct
  source 1..28: mol_type = other DNA
gggagccgactccctcaggtcccctggg

SEQ ID NO: 44831 - DNA, 28 bp, synthetic construct
  source 1..28: mol_type = other DNA
agggagccgactccctcaggtcccctgg

SEQ ID NO: 44832 - DNA, 28 bp, synthetic construct
  source 1..28: mol_type = other DNA
ggtagcagagggagccgactccctcagg

SEQ ID NO: 44833 - DNA, 28 bp, synthetic construct
  source 1..28: mol_type = other DNA
tactcaagagacaggaggtagcagaggg

SEQ ID NO: 44834 - DNA, 28 bp, synthetic construct
  source 1..28: mol_type = other DNA
atactcaagagacaggaggtagcagagg

SEQ ID NO: 44835 - DNA, 28 bp, synthetic construct
  source 1..28: mol_type = other DNA
gatcacaggatactcaagagacaggagg

SEQ ID NO: 44836 - DNA, 28 bp, synthetic construct
  source 1..28: mol_type = other DNA
cacgatcacaggatactcaagagacagg

SEQ ID NO: 44837 - DNA, 28 bp, synthetic construct
  source 1..28: mol_type = other DNA
gtgggaatggacaggtcacgatcacagg

SEQ ID NO: 44838 - DNA, 28 bp, synthetic construct
  source 1..28: mol_type = other DNA
gtgacctgtccattcccaccagtgcagg

SEQ ID NO: 44839 - DNA, 28 bp, synthetic construct
  source 1..28: mol_type = other DNA
tgacctgtccattcccaccagtgcaggg

SEQ ID NO: 44840 - DNA, 28 bp, synthetic construct
  source 1..28: mol_type = other DNA
gacctgtccattcccaccagtgcagggg

SEQ ID NO: 44841 - DNA, 28 bp, synthetic construct
  source 1..28: mol_type = other DNA
gacccctgcactggtgggaatggacagg

SEQ ID NO: 44842 - DNA, 28 bp, synthetic construct
  source 1..28: mol_type = other DNA
tcatggacccctgcactggtgggaatgg

SEQ ID NO: 44843 - DNA, 28 bp, synthetic construct
  source 1..28: mol_type = other DNA
ggggctcatggacccctgcactggtggg

SEQ ID NO: 44844 - DNA, 28 bp, synthetic construct
  source 1..28: mol_type = other DNA
gggggctcatggacccctgcactggtgg

SEQ ID NO: 44845 - DNA, 28 bp, synthetic construct
  source 1..28: mol_type = other DNA
tttgggggctcatggacccctgcactgg

SEQ ID NO: 44846 - DNA, 28 bp, synthetic construct
  source 1..28: mol_type = other DNA
agtgcaggggtccatgagcccccaaagg

SEQ ID NO: 44847 - DNA, 28 bp, synthetic construct
  source 1..28: mol_type = other DNA
aactcactgcacctttgggggctcatgg

SEQ ID NO: 44848 - DNA, 28 bp, synthetic construct
  source 1..28: mol_type = other DNA
agcccccaaaggtgcagtgagttgtagg

SEQ ID NO: 44849 - DNA, 28 bp, synthetic construct
  source 1..28: mol_type = other DNA
tgcctacaactcactgcacctttggggg

SEQ ID NO: 44850 - DNA, 28 bp, synthetic construct
  source 1..28: mol_type = other DNA
atgcctacaactcactgcacctttgggg

SEQ ID NO: 44851 - DNA, 28 bp, synthetic construct
  source 1..28: mol_type = other DNA
aatgcctacaactcactgcacctttggg

SEQ ID NO: 44852 - DNA, 28 bp, synthetic construct
  source 1..28: mol_type = other DNA
aaatgcctacaactcactgcacctttgg

SEQ ID NO: 44853 - DNA, 28 bp, synthetic construct
  source 1..28: mol_type = other DNA
ttctttttctgaagaaagagtttgttgg

SEQ ID NO: 44854 - DNA, 28 bp, synthetic construct
  source 1..28: mol_type = other DNA
ttgttggtttcatcagatcatcagaagg

SEQ ID NO: 44855 - DNA, 28 bp, synthetic construct
  source 1..28: mol_type = other DNA
tggtttcatcagatcatcagaaggctgg

SEQ ID NO: 44856 - DNA, 28 bp, synthetic construct
  source 1..28: mol_type = other DNA
ggtttcatcagatcatcagaaggctggg

SEQ ID NO: 44857 - DNA, 28 bp, synthetic construct
  source 1..28: mol_type = other DNA
atcatcagaaggctgggtgtccctgtgg

SEQ ID NO: 44858 - DNA, 28 bp, synthetic construct
  source 1..28: mol_type = other DNA
gctgggtgtccctgtggagtgctgacgg

SEQ ID NO: 44859 - DNA, 28 bp, synthetic construct
  source 1..28: mol_type = other DNA
ctgggtgtccctgtggagtgctgacggg

SEQ ID NO: 44860 - DNA, 28 bp, synthetic construct
  source 1..28: mol_type = other DNA
tgggtgtccctgtggagtgctgacgggg

SEQ ID NO: 44861 - DNA, 28 bp, synthetic construct
  source 1..28: mol_type = other DNA
cacacggccccgtcagcactccacaggg

SEQ ID NO: 44862 - DNA, 28 bp, synthetic construct
  source 1..28: mol_type = other DNA
gcacacggccccgtcagcactccacagg

SEQ ID NO: 44863 - DNA, 28 bp, synthetic construct
  source 1..28: mol_type = other DNA
agtgctgacggggccgtgtgcactgcgg

SEQ ID NO: 44864 - DNA, 28 bp, synthetic construct
  source 1..28: mol_type = other DNA
gtgctgacggggccgtgtgcactgcggg

SEQ ID NO: 44865 - DNA, 28 bp, synthetic construct
  source 1..28: mol_type = other DNA
acagaaacgtggagcaaaaagcactggg

SEQ ID NO: 44866 - DNA, 28 bp, synthetic construct
  source 1..28: mol_type = other DNA
aacagaaacgtggagcaaaaagcactgg

SEQ ID NO: 44867 - DNA, 28 bp, synthetic construct
  source 1..28: mol_type = other DNA
agacaacagctagagaacagaaacgtgg

SEQ ID NO: 44868 - DNA, 28 bp, synthetic construct
  source 1..28: mol_type = other DNA
ctgttgtctgtgtcctagagaaagccgg

SEQ ID NO: 44869 - DNA, 28 bp, synthetic construct
  source 1..28: mol_type = other DNA
tgttgtctgtgtcctagagaaagccggg

SEQ ID NO: 44870 - DNA, 28 bp, synthetic construct
  source 1..28: mol_type = other DNA
ggggcaagtgggcccggctttctctagg

SEQ ID NO: 44871 - DNA, 28 bp, synthetic construct
  source 1..28: mol_type = other DNA
ggggagaggtgggggcaagtgggcccgg

SEQ ID NO: 44872 - DNA, 28 bp, synthetic construct
  source 1..28: mol_type = other DNA
aaggtggggagaggtgggggcaagtggg

SEQ ID NO: 44873 - DNA, 28 bp, synthetic construct
  source 1..28: mol_type = other DNA
gaaggtggggagaggtgggggcaagtgg

SEQ ID NO: 44874 - DNA, 28 bp, synthetic construct
  source 1..28: mol_type = other DNA
gggggcagaaggtggggagaggtggggg

SEQ ID NO: 44875 - DNA, 28 bp, synthetic construct
  source 1..28: mol_type = other DNA
agggggcagaaggtggggagaggtgggg

SEQ ID NO: 44876 - DNA, 28 bp, synthetic construct
  source 1..28: mol_type = other DNA
gagggggcagaaggtggggagaggtggg

SEQ ID NO: 44877 - DNA, 28 bp, synthetic construct
  source 1..28: mol_type = other DNA
ggagggggcagaaggtggggagaggtgg

SEQ ID NO: 44878 - DNA, 28 bp, synthetic construct
  source 1..28: mol_type = other DNA
gggggagggggcagaaggtggggagagg

SEQ ID NO: 44879 - DNA, 28 bp, synthetic construct
  source 1..28: mol_type = other DNA
tggcagggggagggggcagaaggtgggg

SEQ ID NO: 44880 - DNA, 28 bp, synthetic construct
  source 1..28: mol_type = other DNA
ctggcagggggagggggcagaaggtggg

SEQ ID NO: 44881 - DNA, 28 bp, synthetic construct
  source 1..28: mol_type = other DNA
gctggcagggggagggggcagaaggtgg

SEQ ID NO: 44882 - DNA, 28 bp, synthetic construct
  source 1..28: mol_type = other DNA
gcagctggcagggggagggggcagaagg

SEQ ID NO: 44883 - DNA, 28 bp, synthetic construct
  source 1..28: mol_type = other DNA
tggaggcgcagctggcagggggaggggg

SEQ ID NO: 44884 - DNA, 28 bp, synthetic construct
  source 1..28: mol_type = other DNA
atggaggcgcagctggcagggggagggg

SEQ ID NO: 44885 - DNA, 28 bp, synthetic construct
  source 1..28: mol_type = other DNA
catggaggcgcagctggcagggggaggg

SEQ ID NO: 44886 - DNA, 28 bp, synthetic construct
  source 1..28: mol_type = other DNA
acatggaggcgcagctggcagggggagg

SEQ ID NO: 44887 - DNA, 28 bp, synthetic construct
  source 1..28: mol_type = other DNA
cttacatggaggcgcagctggcaggggg

SEQ ID NO: 44888 - DNA, 28 bp, synthetic construct
  source 1..28: mol_type = other DNA
acttacatggaggcgcagctggcagggg

SEQ ID NO: 44889 - DNA, 28 bp, synthetic construct
  source 1..28: mol_type = other DNA
tacttacatggaggcgcagctggcaggg

SEQ ID NO: 44890 - DNA, 28 bp, synthetic construct
  source 1..28: mol_type = other DNA
gtacttacatggaggcgcagctggcagg

SEQ ID NO: 44891 - DNA, 28 bp, synthetic construct
  source 1..28: mol_type = other DNA
caaagtacttacatggaggcgcagctgg

SEQ ID NO: 44892 - DNA, 28 bp, synthetic construct
  source 1..28: mol_type = other DNA
taagggactcaaagtacttacatggagg

SEQ ID NO: 44893 - DNA, 28 bp, synthetic construct
  source 1..28: mol_type = other DNA
tgttaagggactcaaagtacttacatgg

SEQ ID NO: 44894 - DNA, 28 bp, synthetic construct
  source 1..28: mol_type = other DNA
gtactttgagtcccttaacaccccaagg

SEQ ID NO: 44895 - DNA, 28 bp, synthetic construct
  source 1..28: mol_type = other DNA
agtcccttaacaccccaaggcgtgttgg

SEQ ID NO: 44896 - DNA, 28 bp, synthetic construct
  source 1..28: mol_type = other DNA
ccaccaacacgccttggggtgttaaggg

SEQ ID NO: 44897 - DNA, 28 bp, synthetic construct
  source 1..28: mol_type = other DNA
gccaccaacacgccttggggtgttaagg

SEQ ID NO: 44898 - DNA, 28 bp, synthetic construct
  source 1..28: mol_type = other DNA
aaaagctggccaccaacacgccttgggg

SEQ ID NO: 44899 - DNA, 28 bp, synthetic construct
  source 1..28: mol_type = other DNA
caaaagctggccaccaacacgccttggg

SEQ ID NO: 44900 - DNA, 28 bp, synthetic construct
  source 1..28: mol_type = other DNA
acaaaagctggccaccaacacgccttgg

SEQ ID NO: 44901 - DNA, 28 bp, synthetic construct
  source 1..28: mol_type = other DNA
tggggcttgtcatcacgacaaaagctgg

SEQ ID NO: 44902 - DNA, 28 bp, synthetic construct
  source 1..28: mol_type = other DNA
tgatgacaagccccagcaagtctacagg

SEQ ID NO: 44903 - DNA, 28 bp, synthetic construct
  source 1..28: mol_type = other DNA
gatgacaagccccagcaagtctacaggg

SEQ ID NO: 44904 - DNA, 28 bp, synthetic construct
  source 1..28: mol_type = other DNA
caagccccagcaagtctacagggactgg

SEQ ID NO: 44905 - DNA, 28 bp, synthetic construct
  source 1..28: mol_type = other DNA
gcagccagtccctgtagacttgctgggg

SEQ ID NO: 44906 - DNA, 28 bp, synthetic construct
  source 1..28: mol_type = other DNA
agcagccagtccctgtagacttgctggg

SEQ ID NO: 44907 - DNA, 28 bp, synthetic construct
  source 1..28: mol_type = other DNA
aagcagccagtccctgtagacttgctgg

SEQ ID NO: 44908 - DNA, 28 bp, synthetic construct
  source 1..28: mol_type = other DNA
tctacagggactggctgctttcatgtgg

SEQ ID NO: 44909 - DNA, 28 bp, synthetic construct
  source 1..28: mol_type = other DNA
ctacagggactggctgctttcatgtggg

SEQ ID NO: 44910 - DNA, 28 bp, synthetic construct
  source 1..28: mol_type = other DNA
gactggctgctttcatgtgggccctcgg

SEQ ID NO: 44911 - DNA, 28 bp, synthetic construct
  source 1..28: mol_type = other DNA
atgtgggccctcggtgaagcctccttgg

SEQ ID NO: 44912 - DNA, 28 bp, synthetic construct
  source 1..28: mol_type = other DNA
gctgagaccaaggaggcttcaccgaggg

SEQ ID NO: 44913 - DNA, 28 bp, synthetic construct
  source 1..28: mol_type = other DNA
tgctgagaccaaggaggcttcaccgagg

SEQ ID NO: 44914 - DNA, 28 bp, synthetic construct
  source 1..28: mol_type = other DNA
tcggtgaagcctccttggtctcagcagg

SEQ ID NO: 44915 - DNA, 28 bp, synthetic construct
  source 1..28: mol_type = other DNA
aacacagggcctgctgagaccaaggagg

SEQ ID NO: 44916 - DNA, 28 bp, synthetic construct
  source 1..28: mol_type = other DNA
tacaacacagggcctgctgagaccaagg

SEQ ID NO: 44917 - DNA, 28 bp, synthetic construct
  source 1..28: mol_type = other DNA
cagcaggccctgtgttgtacccaccagg

SEQ ID NO: 44918 - DNA, 28 bp, synthetic construct
  source 1..28: mol_type = other DNA
ctagaggcctggtgggtacaacacaggg

SEQ ID NO: 44919 - DNA, 28 bp, synthetic construct
  source 1..28: mol_type = other DNA
cctgtgttgtacccaccaggcctctagg

SEQ ID NO: 44920 - DNA, 28 bp, synthetic construct
  source 1..28: mol_type = other DNA
gtacccaccaggcctctaggagattagg

SEQ ID NO: 44921 - DNA, 28 bp, synthetic construct
  source 1..28: mol_type = other DNA
tacccaccaggcctctaggagattaggg

SEQ ID NO: 44922 - DNA, 28 bp, synthetic construct
  source 1..28: mol_type = other DNA
acccaccaggcctctaggagattagggg

SEQ ID NO: 44923 - DNA, 28 bp, synthetic construct
  source 1..28: mol_type = other DNA
ccccctaatctcctagaggcctggtggg

SEQ ID NO: 44924 - DNA, 28 bp, synthetic construct
  source 1..28: mol_type = other DNA
gccccctaatctcctagaggcctggtgg

SEQ ID NO: 44925 - DNA, 28 bp, synthetic construct
  source 1..28: mol_type = other DNA
gaagccccctaatctcctagaggcctgg

SEQ ID NO: 44926 - DNA, 28 bp, synthetic construct
  source 1..28: mol_type = other DNA
ccacagaagccccctaatctcctagagg

SEQ ID NO: 44927 - DNA, 28 bp, synthetic construct
  source 1..28: mol_type = other DNA
attagggggcttctgtggctccagatgg

SEQ ID NO: 44928 - DNA, 28 bp, synthetic construct
  source 1..28: mol_type = other DNA
aggaagggaaaagctttgagccatctgg

SEQ ID NO: 44929 - DNA, 28 bp, synthetic construct
  source 1..28: mol_type = other DNA
gtgggctagggataacacagaggaaggg

SEQ ID NO: 44930 - DNA, 28 bp, synthetic construct
  source 1..28: mol_type = other DNA
ggtgggctagggataacacagaggaagg

SEQ ID NO: 44931 - DNA, 28 bp, synthetic construct
  source 1..28: mol_type = other DNA
tcctctgtgttatccctagcccacctgg

SEQ ID NO: 44932 - DNA, 28 bp, synthetic construct
  source 1..28: mol_type = other DNA
gccaggtgggctagggataacacagagg

SEQ ID NO: 44933 - DNA, 28 bp, synthetic construct
  source 1..28: mol_type = other DNA
gtgaggacggaagccaggtgggctaggg

SEQ ID NO: 44934 - DNA, 28 bp, synthetic construct
  source 1..28: mol_type = other DNA
agtgaggacggaagccaggtgggctagg

SEQ ID NO: 44935 - DNA, 28 bp, synthetic construct
  source 1..28: mol_type = other DNA
tagcccacctggcttccgtcctcactgg

SEQ ID NO: 44936 - DNA, 28 bp, synthetic construct
  source 1..28: mol_type = other DNA
tggccagtgaggacggaagccaggtggg

SEQ ID NO: 44937 - DNA, 28 bp, synthetic construct
  source 1..28: mol_type = other DNA
gtggccagtgaggacggaagccaggtgg

SEQ ID NO: 44938 - DNA, 28 bp, synthetic construct
  source 1..28: mol_type = other DNA
acctggcttccgtcctcactggccacgg

SEQ ID NO: 44939 - DNA, 28 bp, synthetic construct
  source 1..28: mol_type = other DNA
cctggcttccgtcctcactggccacggg

SEQ ID NO: 44940 - DNA, 28 bp, synthetic construct
  source 1..28: mol_type = other DNA
ctggcttccgtcctcactggccacgggg

SEQ ID NO: 44941 - DNA, 28 bp, synthetic construct
  source 1..28: mol_type = other DNA
ttccgtcctcactggccacggggcttgg

SEQ ID NO: 44942 - DNA, 28 bp, synthetic construct
  source 1..28: mol_type = other DNA
tccgtcctcactggccacggggcttggg

SEQ ID NO: 44943 - DNA, 28 bp, synthetic construct
  source 1..28: mol_type = other DNA
ccgtcctcactggccacggggcttgggg

SEQ ID NO: 44944 - DNA, 28 bp, synthetic construct
  source 1..28: mol_type = other DNA
cgtcctcactggccacggggcttggggg

SEQ ID NO: 44945 - DNA, 28 bp, synthetic construct
  source 1..28: mol_type = other DNA
aatcccccaagccccgtggccagtgagg

SEQ ID NO: 44946 - DNA, 28 bp, synthetic construct
  source 1..28: mol_type = other DNA
gagactgaaaatcccccaagccccgtgg

SEQ ID NO: 44947 - DNA, 28 bp, synthetic construct
  source 1..28: mol_type = other DNA
gcttgggggattttcagtctctccaagg

SEQ ID NO: 44948 - DNA, 28 bp, synthetic construct
  source 1..28: mol_type = other DNA
gggattttcagtctctccaaggctctgg

SEQ ID NO: 44949 - DNA, 28 bp, synthetic construct
  source 1..28: mol_type = other DNA
tccaaggctctggcatcttccagagtgg

SEQ ID NO: 44950 - DNA, 28 bp, synthetic construct
  source 1..28: mol_type = other DNA
ccaaggctctggcatcttccagagtggg

SEQ ID NO: 44951 - DNA, 28 bp, synthetic construct
  source 1..28: mol_type = other DNA
ggcatcttccagagtgggctagtcttgg

SEQ ID NO: 44952 - DNA, 28 bp, synthetic construct
  source 1..28: mol_type = other DNA
tggacactccaagactagcccactctgg

SEQ ID NO: 44953 - DNA, 28 bp, synthetic construct
  source 1..28: mol_type = other DNA
gtggtgacagaaagaatggctcagatgg

SEQ ID NO: 44954 - DNA, 28 bp, synthetic construct
  source 1..28: mol_type = other DNA
gagccattctttctgtcaccactgctgg

SEQ ID NO: 44955 - DNA, 28 bp, synthetic construct
  source 1..28: mol_type = other DNA
agccattctttctgtcaccactgctggg

SEQ ID NO: 44956 - DNA, 28 bp, synthetic construct
  source 1..28: mol_type = other DNA
ggcccagcagtggtgacagaaagaatgg

SEQ ID NO: 44957 - DNA, 28 bp, synthetic construct
  source 1..28: mol_type = other DNA
tgtcaccactgctgggcctgcctgctgg

SEQ ID NO: 44958 - DNA, 28 bp, synthetic construct
  source 1..28: mol_type = other DNA
gtcaccactgctgggcctgcctgctggg

SEQ ID NO: 44959 - DNA, 28 bp, synthetic construct
  source 1..28: mol_type = other DNA
aaggcccagcaggcaggcccagcagtgg

SEQ ID NO: 44960 - DNA, 28 bp, synthetic construct
  source 1..28: mol_type = other DNA
ctgctgggcctgcctgctgggccttagg

SEQ ID NO: 44961 - DNA, 28 bp, synthetic construct
  source 1..28: mol_type = other DNA
agaagtcacctaaggcccagcaggcagg

SEQ ID NO: 44962 - DNA, 28 bp, synthetic construct
  source 1..28: mol_type = other DNA
ctcaagaagtcacctaaggcccagcagg

SEQ ID NO: 44963 - DNA, 28 bp, synthetic construct
  source 1..28: mol_type = other DNA
gctgggccttaggtgacttcttgagagg

SEQ ID NO: 44964 - DNA, 28 bp, synthetic construct
  source 1..28: mol_type = other DNA
gggccttaggtgacttcttgagaggtgg

SEQ ID NO: 44965 - DNA, 28 bp, synthetic construct
  source 1..28: mol_type = other DNA
tggccacctctcaagaagtcacctaagg

SEQ ID NO: 44966 - DNA, 28 bp, synthetic construct
  source 1..28: mol_type = other DNA
agaggtggccaaagctgctaatccctgg

SEQ ID NO: 44967 - DNA, 28 bp, synthetic construct
  source 1..28: mol_type = other DNA
gtggccaaagctgctaatccctggaagg

SEQ ID NO: 44968 - DNA, 28 bp, synthetic construct
  source 1..28: mol_type = other DNA
tggccaaagctgctaatccctggaaggg

SEQ ID NO: 44969 - DNA, 28 bp, synthetic construct
  source 1..28: mol_type = other DNA
ggccaaagctgctaatccctggaagggg

SEQ ID NO: 44970 - DNA, 28 bp, synthetic construct
  source 1..28: mol_type = other DNA
agccccttccagggattagcagctttgg

SEQ ID NO: 44971 - DNA, 28 bp, synthetic construct
  source 1..28: mol_type = other DNA
ctgctaatccctggaaggggctcctagg

SEQ ID NO: 44972 - DNA, 28 bp, synthetic construct
  source 1..28: mol_type = other DNA
agggaaatcctaggagccccttccaggg

SEQ ID NO: 44973 - DNA, 28 bp, synthetic construct
  source 1..28: mol_type = other DNA
cagggaaatcctaggagccccttccagg

SEQ ID NO: 44974 - DNA, 28 bp, synthetic construct
  source 1..28: mol_type = other DNA
ggaaggggctcctaggatttccctgtgg

SEQ ID NO: 44975 - DNA, 28 bp, synthetic construct
  source 1..28: mol_type = other DNA
ggggctcctaggatttccctgtggctgg

SEQ ID NO: 44976 - DNA, 28 bp, synthetic construct
  source 1..28: mol_type = other DNA
ctcctaggatttccctgtggctggcagg

SEQ ID NO: 44977 - DNA, 28 bp, synthetic construct
  source 1..28: mol_type = other DNA
gtcctgccagccacagggaaatcctagg

SEQ ID NO: 44978 - DNA, 28 bp, synthetic construct
  source 1..28: mol_type = other DNA
atttccctgtggctggcaggacccttgg

SEQ ID NO: 44979 - DNA, 28 bp, synthetic construct
  source 1..28: mol_type = other DNA
gtggccaagggtcctgccagccacaggg

SEQ ID NO: 44980 - DNA, 28 bp, synthetic construct
  source 1..28: mol_type = other DNA
ggtggccaagggtcctgccagccacagg

SEQ ID NO: 44981 - DNA, 28 bp, synthetic construct
  source 1..28: mol_type = other DNA
ctggcaggacccttggccacccacgtgg

SEQ ID NO: 44982 - DNA, 28 bp, synthetic construct
  source 1..28: mol_type = other DNA
catgtcacaccacgtgggtggccaaggg

SEQ ID NO: 44983 - DNA, 28 bp, synthetic construct
  source 1..28: mol_type = other DNA
tcatgtcacaccacgtgggtggccaagg

SEQ ID NO: 44984 - DNA, 28 bp, synthetic construct
  source 1..28: mol_type = other DNA
ttggccacccacgtggtgtgacatgagg

SEQ ID NO: 44985 - DNA, 28 bp, synthetic construct
  source 1..28: mol_type = other DNA
ggctcctcatgtcacaccacgtgggtgg

SEQ ID NO: 44986 - DNA, 28 bp, synthetic construct
  source 1..28: mol_type = other DNA
cccacgtggtgtgacatgaggagcctgg

SEQ ID NO: 44987 - DNA, 28 bp, synthetic construct
  source 1..28: mol_type = other DNA
tccaggctcctcatgtcacaccacgtgg

SEQ ID NO: 44988 - DNA, 28 bp, synthetic construct
  source 1..28: mol_type = other DNA
aggatggaggttgggctggctttccagg

SEQ ID NO: 44989 - DNA, 28 bp, synthetic construct
  source 1..28: mol_type = other DNA
tggggcttaaggatggaggttgggctgg

SEQ ID NO: 44990 - DNA, 28 bp, synthetic construct
  source 1..28: mol_type = other DNA
tacgtggggcttaaggatggaggttggg

SEQ ID NO: 44991 - DNA, 28 bp, synthetic construct
  source 1..28: mol_type = other DNA
atacgtggggcttaaggatggaggttgg

SEQ ID NO: 44992 - DNA, 28 bp, synthetic construct
  source 1..28: mol_type = other DNA
gtttatacgtggggcttaaggatggagg

SEQ ID NO: 44993 - DNA, 28 bp, synthetic construct
  source 1..28: mol_type = other DNA
tatgtttatacgtggggcttaaggatgg

SEQ ID NO: 44994 - DNA, 28 bp, synthetic construct
  source 1..28: mol_type = other DNA
aaggtatgtttatacgtggggcttaagg

SEQ ID NO: 44995 - DNA, 28 bp, synthetic construct
  source 1..28: mol_type = other DNA
aaaaaaaaaggtatgtttatacgtgggg

SEQ ID NO: 44996 - DNA, 28 bp, synthetic construct
  source 1..28: mol_type = other DNA
aaaaaaaaaaggtatgtttatacgtggg

SEQ ID NO: 44997 - DNA, 28 bp, synthetic construct
  source 1..28: mol_type = other DNA
aaaaaaaaaaaggtatgtttatacgtgg

SEQ ID NO: 44998 - DNA, 28 bp, synthetic construct
  source 1..28: mol_type = other DNA
agagctgcagttaaaaaaaaaaaaaagg

SEQ ID NO: 44999 - DNA, 28 bp, synthetic construct
  source 1..28: mol_type = other DNA
cagagcctgcagttctactgttgtcagg

SEQ ID NO: 45000 - DNA, 28 bp, synthetic construct
  source 1..28: mol_type = other DNA
ggcaacctgacaacagtagaactgcagg

SEQ ID NO: 45001 - DNA, 28 bp, synthetic construct
  source 1..28: mol_type = other DNA
ttgtcaggttgccttgtgctctccttgg

SEQ ID NO: 45002 - DNA, 28 bp, synthetic construct
  source 1..28: mol_type = other DNA
cttagaggatgccaaggagagcacaagg

SEQ ID NO: 45003 - DNA, 28 bp, synthetic construct
  source 1..28: mol_type = other DNA
gtgctctccttggcatcctctaagaagg

SEQ ID NO: 45004 - DNA, 28 bp, synthetic construct
  source 1..28: mol_type = other DNA
gtatttgccttcttagaggatgccaagg

SEQ ID NO: 45005 - DNA, 28 bp, synthetic construct
  source 1..28: mol_type = other DNA
gctgaaaaggtatttgccttcttagagg

SEQ ID NO: 45006 - DNA, 28 bp, synthetic construct
  source 1..28: mol_type = other DNA
ctaagaaggcaaataccttttcagctgg

SEQ ID NO: 45007 - DNA, 28 bp, synthetic construct
  source 1..28: mol_type = other DNA
taagaaggcaaataccttttcagctggg

SEQ ID NO: 45008 - DNA, 28 bp, synthetic construct
  source 1..28: mol_type = other DNA
aatgcttaaaagcacccagctgaaaagg

SEQ ID NO: 45009 - DNA, 28 bp, synthetic construct
  source 1..28: mol_type = other DNA
gcatttgctgtcaagaagcaagccctgg

SEQ ID NO: 45010 - DNA, 28 bp, synthetic construct
  source 1..28: mol_type = other DNA
gtcaagaagcaagccctggccagcctgg

SEQ ID NO: 45011 - DNA, 28 bp, synthetic construct
  source 1..28: mol_type = other DNA
cactggaaaagggccaggctggccaggg

SEQ ID NO: 45012 - DNA, 28 bp, synthetic construct
  source 1..28: mol_type = other DNA
acactggaaaagggccaggctggccagg

SEQ ID NO: 45013 - DNA, 28 bp, synthetic construct
  source 1..28: mol_type = other DNA
acagaacactggaaaagggccaggctgg

SEQ ID NO: 45014 - DNA, 28 bp, synthetic construct
  source 1..28: mol_type = other DNA
tcacacagaacactggaaaagggccagg

SEQ ID NO: 45015 - DNA, 28 bp, synthetic construct
  source 1..28: mol_type = other DNA
cacggtcacacagaacactggaaaaggg

SEQ ID NO: 45016 - DNA, 28 bp, synthetic construct
  source 1..28: mol_type = other DNA
ccacggtcacacagaacactggaaaagg

SEQ ID NO: 45017 - DNA, 28 bp, synthetic construct
  source 1..28: mol_type = other DNA
acttggccacggtcacacagaacactgg

SEQ ID NO: 45018 - DNA, 28 bp, synthetic construct
  source 1..28: mol_type = other DNA
ccagagaagagaagcaacttggccacgg

SEQ ID NO: 45019 - DNA, 28 bp, synthetic construct
  source 1..28: mol_type = other DNA
cgtggccaagttgcttctcttctctggg

SEQ ID NO: 45020 - DNA, 28 bp, synthetic construct
  source 1..28: mol_type = other DNA
cgagacccagagaagagaagcaacttgg

SEQ ID NO: 45021 - DNA, 28 bp, synthetic construct
  source 1..28: mol_type = other DNA
gacccttttcagctctagcactttgagg

SEQ ID NO: 45022 - DNA, 28 bp, synthetic construct
  source 1..28: mol_type = other DNA
agcctcaaagtgctagagctgaaaaggg

SEQ ID NO: 45023 - DNA, 28 bp, synthetic construct
  source 1..28: mol_type = other DNA
gagcctcaaagtgctagagctgaaaagg

SEQ ID NO: 45024 - DNA, 28 bp, synthetic construct
  source 1..28: mol_type = other DNA
gctctagcactttgaggctccagcatgg

SEQ ID NO: 45025 - DNA, 28 bp, synthetic construct
  source 1..28: mol_type = other DNA
gtgtggagggtgtaagaatccatgctgg

SEQ ID NO: 45026 - DNA, 28 bp, synthetic construct
  source 1..28: mol_type = other DNA
attcttacaccctccacacctttgccgg

SEQ ID NO: 45027 - DNA, 28 bp, synthetic construct
  source 1..28: mol_type = other DNA
gaaaggtgaccggcaaaggtgtggaggg

SEQ ID NO: 45028 - DNA, 28 bp, synthetic construct
  source 1..28: mol_type = other DNA
agaaaggtgaccggcaaaggtgtggagg

SEQ ID NO: 45029 - DNA, 28 bp, synthetic construct
  source 1..28: mol_type = other DNA
ggaagaaaggtgaccggcaaaggtgtgg

SEQ ID NO: 45030 - DNA, 28 bp, synthetic construct
  source 1..28: mol_type = other DNA
gagaaggaagaaaggtgaccggcaaagg

SEQ ID NO: 45031 - DNA, 28 bp, synthetic construct
  source 1..28: mol_type = other DNA
cctgcagagaaggaagaaaggtgaccgg

SEQ ID NO: 45032 - DNA, 28 bp, synthetic construct
  source 1..28: mol_type = other DNA
cggtcacctttcttccttctctgcaggg

SEQ ID NO: 45033 - DNA, 28 bp, synthetic construct
  source 1..28: mol_type = other DNA
tcacctttcttccttctctgcagggtgg

SEQ ID NO: 45034 - DNA, 28 bp, synthetic construct
  source 1..28: mol_type = other DNA
cacctttcttccttctctgcagggtggg

SEQ ID NO: 45035 - DNA, 28 bp, synthetic construct
  source 1..28: mol_type = other DNA
acctttcttccttctctgcagggtgggg

SEQ ID NO: 45036 - DNA, 28 bp, synthetic construct
  source 1..28: mol_type = other DNA
gccccaccctgcagagaaggaagaaagg

SEQ ID NO: 45037 - DNA, 28 bp, synthetic construct
  source 1..28: mol_type = other DNA
cttccttctctgcagggtggggcacagg

SEQ ID NO: 45038 - DNA, 28 bp, synthetic construct
  source 1..28: mol_type = other DNA
ttccttctctgcagggtggggcacaggg

SEQ ID NO: 45039 - DNA, 28 bp, synthetic construct
  source 1..28: mol_type = other DNA
ttccctgtgccccaccctgcagagaagg

SEQ ID NO: 45040 - DNA, 28 bp, synthetic construct
  source 1..28: mol_type = other DNA
ttctctgcagggtggggcacagggaagg

SEQ ID NO: 45041 - DNA, 28 bp, synthetic construct
  source 1..28: mol_type = other DNA
tctctgcagggtggggcacagggaaggg

SEQ ID NO: 45042 - DNA, 28 bp, synthetic construct
  source 1..28: mol_type = other DNA
gcagggtggggcacagggaagggcctgg

SEQ ID NO: 45043 - DNA, 28 bp, synthetic construct
  source 1..28: mol_type = other DNA
acagggaagggcctggcagctgagctgg

SEQ ID NO: 45044 - DNA, 28 bp, synthetic construct
  source 1..28: mol_type = other DNA
cagggaagggcctggcagctgagctggg

SEQ ID NO: 45045 - DNA, 28 bp, synthetic construct
  source 1..28: mol_type = other DNA
ggaagggcctggcagctgagctgggtgg

SEQ ID NO: 45046 - DNA, 28 bp, synthetic construct
  source 1..28: mol_type = other DNA
gaagggcctggcagctgagctgggtggg

SEQ ID NO: 45047 - DNA, 28 bp, synthetic construct
  source 1..28: mol_type = other DNA
aagggcctggcagctgagctgggtgggg

SEQ ID NO: 45048 - DNA, 28 bp, synthetic construct
  source 1..28: mol_type = other DNA
cctggcagctgagctgggtggggccagg

SEQ ID NO: 45049 - DNA, 28 bp, synthetic construct
  source 1..28: mol_type = other DNA
ctggcagctgagctgggtggggccaggg

SEQ ID NO: 45050 - DNA, 28 bp, synthetic construct
  source 1..28: mol_type = other DNA
tggcagctgagctgggtggggccagggg

SEQ ID NO: 45051 - DNA, 28 bp, synthetic construct
  source 1..28: mol_type = other DNA
gtctatgatgctggcttttggcccctgg

SEQ ID NO: 45052 - DNA, 28 bp, synthetic construct
  source 1..28: mol_type = other DNA
gaaaagtgtctatgatgctggcttttgg

SEQ ID NO: 45053 - DNA, 28 bp, synthetic construct
  source 1..28: mol_type = other DNA
ctggagggaaaagtgtctatgatgctgg

SEQ ID NO: 45054 - DNA, 28 bp, synthetic construct
  source 1..28: mol_type = other DNA
catcatagacacttttccctccagctgg

SEQ ID NO: 45055 - DNA, 28 bp, synthetic construct
  source 1..28: mol_type = other DNA
atcatagacacttttccctccagctggg

SEQ ID NO: 45056 - DNA, 28 bp, synthetic construct
  source 1..28: mol_type = other DNA
ggaaggactggtatgcccagctggaggg

SEQ ID NO: 45057 - DNA, 28 bp, synthetic construct
  source 1..28: mol_type = other DNA
aggaaggactggtatgcccagctggagg

SEQ ID NO: 45058 - DNA, 28 bp, synthetic construct
  source 1..28: mol_type = other DNA
aagaggaaggactggtatgcccagctgg

SEQ ID NO: 45059 - DNA, 28 bp, synthetic construct
  source 1..28: mol_type = other DNA
cataccagtccttcctcttcttctcagg

SEQ ID NO: 45060 - DNA, 28 bp, synthetic construct
  source 1..28: mol_type = other DNA
ctgtcctgagaagaagaggaaggactgg

SEQ ID NO: 45061 - DNA, 28 bp, synthetic construct
  source 1..28: mol_type = other DNA
cagtccttcctcttcttctcaggacagg

SEQ ID NO: 45062 - DNA, 28 bp, synthetic construct
  source 1..28: mol_type = other DNA
tccttcctcttcttctcaggacaggtgg

SEQ ID NO: 45063 - DNA, 28 bp, synthetic construct
  source 1..28: mol_type = other DNA
cccacctgtcctgagaagaagaggaagg

SEQ ID NO: 45064 - DNA, 28 bp, synthetic construct
  source 1..28: mol_type = other DNA
cttcctcttcttctcaggacaggtgggg

SEQ ID NO: 45065 - DNA, 28 bp, synthetic construct
  source 1..28: mol_type = other DNA
tttccccacctgtcctgagaagaagagg

SEQ ID NO: 45066 - DNA, 28 bp, synthetic construct
  source 1..28: mol_type = other DNA
cttctcaggacaggtggggaaactgagg

SEQ ID NO: 45067 - DNA, 28 bp, synthetic construct
  source 1..28: mol_type = other DNA
caggacaggtggggaaactgaggtctgg

SEQ ID NO: 45068 - DNA, 28 bp, synthetic construct
  source 1..28: mol_type = other DNA
gacaggtggggaaactgaggtctggagg

SEQ ID NO: 45069 - DNA, 28 bp, synthetic construct
  source 1..28: mol_type = other DNA
acaggtggggaaactgaggtctggaggg

SEQ ID NO: 45070 - DNA, 28 bp, synthetic construct
  source 1..28: mol_type = other DNA
caggtggggaaactgaggtctggagggg

SEQ ID NO: 45071 - DNA, 28 bp, synthetic construct
  source 1..28: mol_type = other DNA
aggtggggaaactgaggtctggaggggg

SEQ ID NO: 45072 - DNA, 28 bp, synthetic construct
  source 1..28: mol_type = other DNA
ggggaaactgaggtctggagggggaagg

SEQ ID NO: 45073 - DNA, 28 bp, synthetic construct
  source 1..28: mol_type = other DNA
gggaaactgaggtctggagggggaaggg

SEQ ID NO: 45074 - DNA, 28 bp, synthetic construct
  source 1..28: mol_type = other DNA
actgaggtctggagggggaagggccagg

SEQ ID NO: 45075 - DNA, 28 bp, synthetic construct
  source 1..28: mol_type = other DNA
ctgaggtctggagggggaagggccaggg

SEQ ID NO: 45076 - DNA, 28 bp, synthetic construct
  source 1..28: mol_type = other DNA
ggtctggagggggaagggccagggctgg

SEQ ID NO: 45077 - DNA, 28 bp, synthetic construct
  source 1..28: mol_type = other DNA
agggggaagggccagggctggaaccagg

SEQ ID NO: 45078 - DNA, 28 bp, synthetic construct
  source 1..28: mol_type = other DNA
gataactgggtcctggttccagccctgg

SEQ ID NO: 45079 - DNA, 28 bp, synthetic construct
  source 1..28: mol_type = other DNA
actggcaataaggataactgggtcctgg

SEQ ID NO: 45080 - DNA, 28 bp, synthetic construct
  source 1..28: mol_type = other DNA
gcactcactggcaataaggataactggg

SEQ ID NO: 45081 - DNA, 28 bp, synthetic construct
  source 1..28: mol_type = other DNA
agcactcactggcaataaggataactgg

SEQ ID NO: 45082 - DNA, 28 bp, synthetic construct
  source 1..28: mol_type = other DNA
gcaggaggagcactcactggcaataagg

SEQ ID NO: 45083 - DNA, 28 bp, synthetic construct
  source 1..28: mol_type = other DNA
tgccagtgagtgctcctcctgctgttgg

SEQ ID NO: 45084 - DNA, 28 bp, synthetic construct
  source 1..28: mol_type = other DNA
agccaacagcaggaggagcactcactgg

SEQ ID NO: 45085 - DNA, 28 bp, synthetic construct
  source 1..28: mol_type = other DNA
aagagaggtagcagccaacagcaggagg

SEQ ID NO: 45086 - DNA, 28 bp, synthetic construct
  source 1..28: mol_type = other DNA
ctcaagagaggtagcagccaacagcagg

SEQ ID NO: 45087 - DNA, 28 bp, synthetic construct
  source 1..28: mol_type = other DNA
gctgttggctgctacctctcttgagagg

SEQ ID NO: 45088 - DNA, 28 bp, synthetic construct
  source 1..28: mol_type = other DNA
ctgttggctgctacctctcttgagaggg

SEQ ID NO: 45089 - DNA, 28 bp, synthetic construct
  source 1..28: mol_type = other DNA
gtgggtcttctgaccctctcaagagagg

SEQ ID NO: 45090 - DNA, 28 bp, synthetic construct
  source 1..28: mol_type = other DNA
gagggtcagaagacccactagcatgagg

SEQ ID NO: 45091 - DNA, 28 bp, synthetic construct
  source 1..28: mol_type = other DNA
agggtcagaagacccactagcatgaggg

SEQ ID NO: 45092 - DNA, 28 bp, synthetic construct
  source 1..28: mol_type = other DNA
cagaagacccactagcatgagggtcagg

SEQ ID NO: 45093 - DNA, 28 bp, synthetic construct
  source 1..28: mol_type = other DNA
agaagacccactagcatgagggtcaggg

SEQ ID NO: 45094 - DNA, 28 bp, synthetic construct
  source 1..28: mol_type = other DNA
gcatgtccctgaccctcatgctagtggg

SEQ ID NO: 45095 - DNA, 28 bp, synthetic construct
  source 1..28: mol_type = other DNA
agcatgtccctgaccctcatgctagtgg

SEQ ID NO: 45096 - DNA, 28 bp, synthetic construct
  source 1..28: mol_type = other DNA
cagggacatgctttttcctttcccgtgg

SEQ ID NO: 45097 - DNA, 28 bp, synthetic construct
  source 1..28: mol_type = other DNA
gacatgctttttcctttcccgtggaagg

SEQ ID NO: 45098 - DNA, 28 bp, synthetic construct
  source 1..28: mol_type = other DNA
ttcctttcccgtggaaggctcctccagg

SEQ ID NO: 45099 - DNA, 28 bp, synthetic construct
  source 1..28: mol_type = other DNA
tgcctggaggagccttccacgggaaagg

SEQ ID NO: 45100 - DNA, 28 bp, synthetic construct
  source 1..28: mol_type = other DNA
tttcccgtggaaggctcctccaggcagg

SEQ ID NO: 45101 - DNA, 28 bp, synthetic construct
  source 1..28: mol_type = other DNA
ttcccgtggaaggctcctccaggcaggg

SEQ ID NO: 45102 - DNA, 28 bp, synthetic construct
  source 1..28: mol_type = other DNA
agccctgcctggaggagccttccacggg

SEQ ID NO: 45103 - DNA, 28 bp, synthetic construct
  source 1..28: mol_type = other DNA
aagccctgcctggaggagccttccacgg

SEQ ID NO: 45104 - DNA, 28 bp, synthetic construct
  source 1..28: mol_type = other DNA
gtggaaggctcctccaggcagggcttgg

SEQ ID NO: 45105 - DNA, 28 bp, synthetic construct
  source 1..28: mol_type = other DNA
tggaaggctcctccaggcagggcttggg

SEQ ID NO: 45106 - DNA, 28 bp, synthetic construct
  source 1..28: mol_type = other DNA
ggctcctccaggcagggcttgggtgagg

SEQ ID NO: 45107 - DNA, 28 bp, synthetic construct
  source 1..28: mol_type = other DNA
cctgcctcacccaagccctgcctggagg

SEQ ID NO: 45108 - DNA, 28 bp, synthetic construct
  source 1..28: mol_type = other DNA
tcgcctgcctcacccaagccctgcctgg

SEQ ID NO: 45109 - DNA, 28 bp, synthetic construct
  source 1..28: mol_type = other DNA
aggcagggcttgggtgaggcaggcgagg

SEQ ID NO: 45110 - DNA, 28 bp, synthetic construct
  source 1..28: mol_type = other DNA
ttgggtgaggcaggcgaggtgccagtgg

SEQ ID NO: 45111 - DNA, 28 bp, synthetic construct
  source 1..28: mol_type = other DNA
ggcaggcgaggtgccagtggttccctgg

SEQ ID NO: 45112 - DNA, 28 bp, synthetic construct
  source 1..28: mol_type = other DNA
gcaggcgaggtgccagtggttccctggg

SEQ ID NO: 45113 - DNA, 28 bp, synthetic construct
  source 1..28: mol_type = other DNA
cgaggtgccagtggttccctgggcacgg

SEQ ID NO: 45114 - DNA, 28 bp, synthetic construct
  source 1..28: mol_type = other DNA
gaggtgccagtggttccctgggcacggg

SEQ ID NO: 45115 - DNA, 28 bp, synthetic construct
  source 1..28: mol_type = other DNA
aggtgccagtggttccctgggcacgggg

SEQ ID NO: 45116 - DNA, 28 bp, synthetic construct
  source 1..28: mol_type = other DNA
ttctgccccgtgcccagggaaccactgg

SEQ ID NO: 45117 - DNA, 28 bp, synthetic construct
  source 1..28: mol_type = other DNA
tggttccctgggcacggggcagaatcgg

SEQ ID NO: 45118 - DNA, 28 bp, synthetic construct
  source 1..28: mol_type = other DNA
ttccctgggcacggggcagaatcggagg

SEQ ID NO: 45119 - DNA, 28 bp, synthetic construct
  source 1..28: mol_type = other DNA
ctcctccgattctgccccgtgcccaggg

SEQ ID NO: 45120 - DNA, 28 bp, synthetic construct
  source 1..28: mol_type = other DNA
cctgggcacggggcagaatcggaggagg

SEQ ID NO: 45121 - DNA, 28 bp, synthetic construct
  source 1..28: mol_type = other DNA
atcggaggaggacatcctctttctgagg

SEQ ID NO: 45122 - DNA, 28 bp, synthetic construct
  source 1..28: mol_type = other DNA
ggaggacatcctctttctgaggttaagg

SEQ ID NO: 45123 - DNA, 28 bp, synthetic construct
  source 1..28: mol_type = other DNA
ggacatcctctttctgaggttaaggagg

SEQ ID NO: 45124 - DNA, 28 bp, synthetic construct
  source 1..28: mol_type = other DNA
atcctctttctgaggttaaggaggtagg

SEQ ID NO: 45125 - DNA, 28 bp, synthetic construct
  source 1..28: mol_type = other DNA
tcctctttctgaggttaaggaggtaggg

SEQ ID NO: 45126 - DNA, 28 bp, synthetic construct
  source 1..28: mol_type = other DNA
cctctttctgaggttaaggaggtagggg

SEQ ID NO: 45127 - DNA, 28 bp, synthetic construct
  source 1..28: mol_type = other DNA
tttctgaggttaaggaggtaggggctgg

SEQ ID NO: 45128 - DNA, 28 bp, synthetic construct
  source 1..28: mol_type = other DNA
ctgaggttaaggaggtaggggctggagg

SEQ ID NO: 45129 - DNA, 28 bp, synthetic construct
  source 1..28: mol_type = other DNA
gaggtaggggctggaggccttgacaagg

SEQ ID NO: 45130 - DNA, 28 bp, synthetic construct
  source 1..28: mol_type = other DNA
aggtaggggctggaggccttgacaaggg

SEQ ID NO: 45131 - DNA, 28 bp, synthetic construct
  source 1..28: mol_type = other DNA
taggggctggaggccttgacaagggagg

SEQ ID NO: 45132 - DNA, 28 bp, synthetic construct
  source 1..28: mol_type = other DNA
gggctggaggccttgacaagggaggtgg

SEQ ID NO: 45133 - DNA, 28 bp, synthetic construct
  source 1..28: mol_type = other DNA
ggccttgacaagggaggtggcatgaagg

SEQ ID NO: 45134 - DNA, 28 bp, synthetic construct
  source 1..28: mol_type = other DNA
gccttgacaagggaggtggcatgaaggg

SEQ ID NO: 45135 - DNA, 28 bp, synthetic construct
  source 1..28: mol_type = other DNA
ccttgacaagggaggtggcatgaagggg

SEQ ID NO: 45136 - DNA, 28 bp, synthetic construct
  source 1..28: mol_type = other DNA
acaagggaggtggcatgaaggggcgtgg

SEQ ID NO: 45137 - DNA, 28 bp, synthetic construct
  source 1..28: mol_type = other DNA
agggaggtggcatgaaggggcgtggagg

SEQ ID NO: 45138 - DNA, 28 bp, synthetic construct
  source 1..28: mol_type = other DNA
ggcatgaaggggcgtggaggtttctagg

SEQ ID NO: 45139 - DNA, 28 bp, synthetic construct
  source 1..28: mol_type = other DNA
aggggcgtggaggtttctaggaacgtgg

SEQ ID NO: 45140 - DNA, 28 bp, synthetic construct
  source 1..28: mol_type = other DNA
gcgtggaggtttctaggaacgtggttgg

SEQ ID NO: 45141 - DNA, 28 bp, synthetic construct
  source 1..28: mol_type = other DNA
tggaggtttctaggaacgtggttggtgg

SEQ ID NO: 45142 - DNA, 28 bp, synthetic construct
  source 1..28: mol_type = other DNA
tttctaggaacgtggttggtggcgcagg

SEQ ID NO: 45143 - DNA, 28 bp, synthetic construct
  source 1..28: mol_type = other DNA
ttctaggaacgtggttggtggcgcaggg

SEQ ID NO: 45144 - DNA, 28 bp, synthetic construct
  source 1..28: mol_type = other DNA
cgtggttggtggcgcagggtgctctagg

SEQ ID NO: 45145 - DNA, 28 bp, synthetic construct
  source 1..28: mol_type = other DNA
gtggttggtggcgcagggtgctctaggg

SEQ ID NO: 45146 - DNA, 28 bp, synthetic construct
  source 1..28: mol_type = other DNA
ggaaggcagaagcaagggagggaggtgg

SEQ ID NO: 45147 - DNA, 28 bp, synthetic construct
  source 1..28: mol_type = other DNA
aagggaaggcagaagcaagggagggagg

SEQ ID NO: 45148 - DNA, 28 bp, synthetic construct
  source 1..28: mol_type = other DNA
agaaagggaaggcagaagcaagggaggg

SEQ ID NO: 45149 - DNA, 28 bp, synthetic construct
  source 1..28: mol_type = other DNA
gagaaagggaaggcagaagcaagggagg

SEQ ID NO: 45150 - DNA, 28 bp, synthetic construct
  source 1..28: mol_type = other DNA
caggagaaagggaaggcagaagcaaggg

SEQ ID NO: 45151 - DNA, 28 bp, synthetic construct
  source 1..28: mol_type = other DNA
ccaggagaaagggaaggcagaagcaagg

SEQ ID NO: 45152 - DNA, 28 bp, synthetic construct
  source 1..28: mol_type = other DNA
cttgcttctgccttccctttctcctggg

SEQ ID NO: 45153 - DNA, 28 bp, synthetic construct
  source 1..28: mol_type = other DNA
ttgcttctgccttccctttctcctgggg

SEQ ID NO: 45154 - DNA, 28 bp, synthetic construct
  source 1..28: mol_type = other DNA
cttctgccttccctttctcctggggagg

SEQ ID NO: 45155 - DNA, 28 bp, synthetic construct
  source 1..28: mol_type = other DNA
ttctgccttccctttctcctggggaggg

SEQ ID NO: 45156 - DNA, 28 bp, synthetic construct
  source 1..28: mol_type = other DNA
tctgccttccctttctcctggggagggg

SEQ ID NO: 45157 - DNA, 28 bp, synthetic construct
  source 1..28: mol_type = other DNA
cagtcccctccccaggagaaagggaagg

SEQ ID NO: 45158 - DNA, 28 bp, synthetic construct
  source 1..28: mol_type = other DNA
cttccctttctcctggggaggggactgg

SEQ ID NO: 45159 - DNA, 28 bp, synthetic construct
  source 1..28: mol_type = other DNA
ttccctttctcctggggaggggactggg

SEQ ID NO: 45160 - DNA, 28 bp, synthetic construct
  source 1..28: mol_type = other DNA
ggcccagtcccctccccaggagaaaggg

SEQ ID NO: 45161 - DNA, 28 bp, synthetic construct
  source 1..28: mol_type = other DNA
tggcccagtcccctccccaggagaaagg

SEQ ID NO: 45162 - DNA, 28 bp, synthetic construct
  source 1..28: mol_type = other DNA
ttactgttggcccagtcccctccccagg

SEQ ID NO: 45163 - DNA, 28 bp, synthetic construct
  source 1..28: mol_type = other DNA
gggccaacagtaatgccatttttcctgg

SEQ ID NO: 45164 - DNA, 28 bp, synthetic construct
  source 1..28: mol_type = other DNA
gggccaggaaaaatggcattactgttgg

SEQ ID NO: 45165 - DNA, 28 bp, synthetic construct
  source 1..28: mol_type = other DNA
acagtaatgccatttttcctggccctgg

SEQ ID NO: 45166 - DNA, 28 bp, synthetic construct
  source 1..28: mol_type = other DNA
cagtaatgccatttttcctggccctggg

SEQ ID NO: 45167 - DNA, 28 bp, synthetic construct
  source 1..28: mol_type = other DNA
tgccatttttcctggccctgggattagg

SEQ ID NO: 45168 - DNA, 28 bp, synthetic construct
  source 1..28: mol_type = other DNA
cacctaatcccagggccaggaaaaatgg

SEQ ID NO: 45169 - DNA, 28 bp, synthetic construct
  source 1..28: mol_type = other DNA
cacggctgcacctaatcccagggccagg

SEQ ID NO: 45170 - DNA, 28 bp, synthetic construct
  source 1..28: mol_type = other DNA
cttaacacggctgcacctaatcccaggg

SEQ ID NO: 45171 - DNA, 28 bp, synthetic construct
  source 1..28: mol_type = other DNA
ccttaacacggctgcacctaatcccagg

SEQ ID NO: 45172 - DNA, 28 bp, synthetic construct
  source 1..28: mol_type = other DNA
gattaggtgcagccgtgttaaggagagg

SEQ ID NO: 45173 - DNA, 28 bp, synthetic construct
  source 1..28: mol_type = other DNA
ccgtgttaaggagaggacattcgagagg

SEQ ID NO: 45174 - DNA, 28 bp, synthetic construct
  source 1..28: mol_type = other DNA
cgtgttaaggagaggacattcgagaggg

SEQ ID NO: 45175 - DNA, 28 bp, synthetic construct
  source 1..28: mol_type = other DNA
taaggagaggacattcgagagggcgtgg

SEQ ID NO: 45176 - DNA, 28 bp, synthetic construct
  source 1..28: mol_type = other DNA
ttcgagagggcgtggcgaagtgaagagg

SEQ ID NO: 45177 - DNA, 28 bp, synthetic construct
  source 1..28: mol_type = other DNA
tgaagaggaacctcacgccactgcctgg

SEQ ID NO: 45178 - DNA, 28 bp, synthetic construct
  source 1..28: mol_type = other DNA
aacctcacgccactgcctggagctccgg

SEQ ID NO: 45179 - DNA, 28 bp, synthetic construct
  source 1..28: mol_type = other DNA
caccggagctccaggcagtggcgtgagg

SEQ ID NO: 45180 - DNA, 28 bp, synthetic construct
  source 1..28: mol_type = other DNA
ctcacgccactgcctggagctccggtgg

SEQ ID NO: 45181 - DNA, 28 bp, synthetic construct
  source 1..28: mol_type = other DNA
tcacgccactgcctggagctccggtggg

SEQ ID NO: 45182 - DNA, 28 bp, synthetic construct
  source 1..28: mol_type = other DNA
ccagacccaccggagctccaggcagtgg

SEQ ID NO: 45183 - DNA, 28 bp, synthetic construct
  source 1..28: mol_type = other DNA
cactgcctggagctccggtgggtctggg

SEQ ID NO: 45184 - DNA, 28 bp, synthetic construct
  source 1..28: mol_type = other DNA
cctggagctccggtgggtctgggtctgg

SEQ ID NO: 45185 - DNA, 28 bp, synthetic construct
  source 1..28: mol_type = other DNA
agacaatgaccagacccagacccaccgg

SEQ ID NO: 45186 - DNA, 28 bp, synthetic construct
  source 1..28: mol_type = other DNA
ggtctgggtctggtcattgtctcgctgg

SEQ ID NO: 45187 - DNA, 28 bp, synthetic construct
  source 1..28: mol_type = other DNA
tcctgtccactctgaccactgtccctgg

SEQ ID NO: 45188 - DNA, 28 bp, synthetic construct
  source 1..28: mol_type = other DNA
gccagggacagtggtcagagtggacagg

SEQ ID NO: 45189 - DNA, 28 bp, synthetic construct
  source 1..28: mol_type = other DNA
agggggccagggacagtggtcagagtgg

SEQ ID NO: 45190 - DNA, 28 bp, synthetic construct
  source 1..28: mol_type = other DNA
ggacagggcagggggccagggacagtgg

SEQ ID NO: 45191 - DNA, 28 bp, synthetic construct
  source 1..28: mol_type = other DNA
aaggactggacagggcagggggccaggg

SEQ ID NO: 45192 - DNA, 28 bp, synthetic construct
  source 1..28: mol_type = other DNA
gaaggactggacagggcagggggccagg

SEQ ID NO: 45193 - DNA, 28 bp, synthetic construct
  source 1..28: mol_type = other DNA
gccccctgccctgtccagtccttccagg

SEQ ID NO: 45194 - DNA, 28 bp, synthetic construct
  source 1..28: mol_type = other DNA
acctggaaggactggacagggcaggggg

SEQ ID NO: 45195 - DNA, 28 bp, synthetic construct
  source 1..28: mol_type = other DNA
gacctggaaggactggacagggcagggg

SEQ ID NO: 45196 - DNA, 28 bp, synthetic construct
  source 1..28: mol_type = other DNA
ggacctggaaggactggacagggcaggg

SEQ ID NO: 45197 - DNA, 28 bp, synthetic construct
  source 1..28: mol_type = other DNA
tggacctggaaggactggacagggcagg

SEQ ID NO: 45198 - DNA, 28 bp, synthetic construct
  source 1..28: mol_type = other DNA
cagatggacctggaaggactggacaggg

SEQ ID NO: 45199 - DNA, 28 bp, synthetic construct
  source 1..28: mol_type = other DNA
tcagatggacctggaaggactggacagg

SEQ ID NO: 45200 - DNA, 28 bp, synthetic construct
  source 1..28: mol_type = other DNA
cacactcagatggacctggaaggactgg

SEQ ID NO: 45201 - DNA, 28 bp, synthetic construct
  source 1..28: mol_type = other DNA
acacacacactcagatggacctggaagg

SEQ ID NO: 45202 - DNA, 28 bp, synthetic construct
  source 1..28: mol_type = other DNA
acacacacacacactcagatggacctgg

SEQ ID NO: 45203 - DNA, 28 bp, synthetic construct
  source 1..28: mol_type = other DNA
acacacacacacacacacactcagatgg

SEQ ID NO: 45204 - DNA, 28 bp, synthetic construct
  source 1..28: mol_type = other DNA
aaatgcaagtacggctgccgaaccaagg

SEQ ID NO: 45205 - DNA, 28 bp, synthetic construct
  source 1..28: mol_type = other DNA
ttggttcggcagccgtacttgcatttgg

SEQ ID NO: 45206 - DNA, 28 bp, synthetic construct
  source 1..28: mol_type = other DNA
tggttcggcagccgtacttgcatttggg

SEQ ID NO: 45207 - DNA, 28 bp, synthetic construct
  source 1..28: mol_type = other DNA
gccgtacttgcatttgggcattcctagg

SEQ ID NO: 45208 - DNA, 28 bp, synthetic construct
  source 1..28: mol_type = other DNA
acctaggaatgcccaaatgcaagtacgg

SEQ ID NO: 45209 - DNA, 28 bp, synthetic construct
  source 1..28: mol_type = other DNA
actgtggacacacaggagctgacctagg

SEQ ID NO: 45210 - DNA, 28 bp, synthetic construct
  source 1..28: mol_type = other DNA
agggttcagctaactgtggacacacagg

SEQ ID NO: 45211 - DNA, 28 bp, synthetic construct
  source 1..28: mol_type = other DNA
gcgggcttcagggttcagctaactgtgg

SEQ ID NO: 45212 - DNA, 28 bp, synthetic construct
  source 1..28: mol_type = other DNA
caggagcgtcagagtgcgggcttcaggg

SEQ ID NO: 45213 - DNA, 28 bp, synthetic construct
  source 1..28: mol_type = other DNA
acaggagcgtcagagtgcgggcttcagg

SEQ ID NO: 45214 - DNA, 28 bp, synthetic construct
  source 1..28: mol_type = other DNA
ggagagaacaggagcgtcagagtgcggg

SEQ ID NO: 45215 - DNA, 28 bp, synthetic construct
  source 1..28: mol_type = other DNA
tggagagaacaggagcgtcagagtgcgg

SEQ ID NO: 45216 - DNA, 28 bp, synthetic construct
  source 1..28: mol_type = other DNA
taaggctgtggagagtggagagaacagg

SEQ ID NO: 45217 - DNA, 28 bp, synthetic construct
  source 1..28: mol_type = other DNA
tccactctccacagccttagccccgtgg

SEQ ID NO: 45218 - DNA, 28 bp, synthetic construct
  source 1..28: mol_type = other DNA
ccactctccacagccttagccccgtggg

SEQ ID NO: 45219 - DNA, 28 bp, synthetic construct
  source 1..28: mol_type = other DNA
cgtggggcccacggggctaaggctgtgg

SEQ ID NO: 45220 - DNA, 28 bp, synthetic construct
  source 1..28: mol_type = other DNA
cacagccttagccccgtgggccccacgg

SEQ ID NO: 45221 - DNA, 28 bp, synthetic construct
  source 1..28: mol_type = other DNA
tcactccgtggggcccacggggctaagg

SEQ ID NO: 45222 - DNA, 28 bp, synthetic construct
  source 1..28: mol_type = other DNA
agccccgtgggccccacggagtgagcgg

SEQ ID NO: 45223 - DNA, 28 bp, synthetic construct
  source 1..28: mol_type = other DNA
tgccgctcactccgtggggcccacgggg

SEQ ID NO: 45224 - DNA, 28 bp, synthetic construct
  source 1..28: mol_type = other DNA
atgccgctcactccgtggggcccacggg

SEQ ID NO: 45225 - DNA, 28 bp, synthetic construct
  source 1..28: mol_type = other DNA
catgccgctcactccgtggggcccacgg

SEQ ID NO: 45226 - DNA, 28 bp, synthetic construct
  source 1..28: mol_type = other DNA
ggtgctgcatgccgctcactccgtgggg

SEQ ID NO: 45227 - DNA, 28 bp, synthetic construct
  source 1..28: mol_type = other DNA
gggtgctgcatgccgctcactccgtggg

SEQ ID NO: 45228 - DNA, 28 bp, synthetic construct
  source 1..28: mol_type = other DNA
ggggtgctgcatgccgctcactccgtgg

SEQ ID NO: 45229 - DNA, 28 bp, synthetic construct
  source 1..28: mol_type = other DNA
cggagtgagcggcatgcagcacccccgg

SEQ ID NO: 45230 - DNA, 28 bp, synthetic construct
  source 1..28: mol_type = other DNA
ggagtgagcggcatgcagcacccccggg

SEQ ID NO: 45231 - DNA, 28 bp, synthetic construct
  source 1..28: mol_type = other DNA
acccccgggcctgtccagtgtcctctgg

SEQ ID NO: 45232 - DNA, 28 bp, synthetic construct
  source 1..28: mol_type = other DNA
gccagaggacactggacaggcccggggg

SEQ ID NO: 45233 - DNA, 28 bp, synthetic construct
  source 1..28: mol_type = other DNA
ggccagaggacactggacaggcccgggg

SEQ ID NO: 45234 - DNA, 28 bp, synthetic construct
  source 1..28: mol_type = other DNA
aggccagaggacactggacaggcccggg

SEQ ID NO: 45235 - DNA, 28 bp, synthetic construct
  source 1..28: mol_type = other DNA
caggccagaggacactggacaggcccgg

SEQ ID NO: 45236 - DNA, 28 bp, synthetic construct
  source 1..28: mol_type = other DNA
ggcagcaggccagaggacactggacagg

SEQ ID NO: 45237 - DNA, 28 bp, synthetic construct
  source 1..28: mol_type = other DNA
tgcagggcagcaggccagaggacactgg

SEQ ID NO: 45238 - DNA, 28 bp, synthetic construct
  source 1..28: mol_type = other DNA
ctgggggtgcagggcagcaggccagagg

SEQ ID NO: 45239 - DNA, 28 bp, synthetic construct
  source 1..28: mol_type = other DNA
tggcctgctgccctgcacccccagaagg

SEQ ID NO: 45240 - DNA, 28 bp, synthetic construct
  source 1..28: mol_type = other DNA
gggccttctgggggtgcagggcagcagg

SEQ ID NO: 45241 - DNA, 28 bp, synthetic construct
  source 1..28: mol_type = other DNA
ggcgtcagggccttctgggggtgcaggg

SEQ ID NO: 45242 - DNA, 28 bp, synthetic construct
  source 1..28: mol_type = other DNA
gggcgtcagggccttctgggggtgcagg

SEQ ID NO: 45243 - DNA, 28 bp, synthetic construct
  source 1..28: mol_type = other DNA
gcacccccagaaggccctgacgccctgg

SEQ ID NO: 45244 - DNA, 28 bp, synthetic construct
  source 1..28: mol_type = other DNA
cacccccagaaggccctgacgccctggg

SEQ ID NO: 45245 - DNA, 28 bp, synthetic construct
  source 1..28: mol_type = other DNA
acccccagaaggccctgacgccctgggg

SEQ ID NO: 45246 - DNA, 28 bp, synthetic construct
  source 1..28: mol_type = other DNA
gccccagggcgtcagggccttctggggg

SEQ ID NO: 45247 - DNA, 28 bp, synthetic construct
  source 1..28: mol_type = other DNA
tgccccagggcgtcagggccttctgggg

SEQ ID NO: 45248 - DNA, 28 bp, synthetic construct
  source 1..28: mol_type = other DNA
gtgccccagggcgtcagggccttctggg

SEQ ID NO: 45249 - DNA, 28 bp, synthetic construct
  source 1..28: mol_type = other DNA
agtgccccagggcgtcagggccttctgg

SEQ ID NO: 45250 - DNA, 28 bp, synthetic construct
  source 1..28: mol_type = other DNA
agagcagaagtgccccagggcgtcaggg

SEQ ID NO: 45251 - DNA, 28 bp, synthetic construct
  source 1..28: mol_type = other DNA
cagagcagaagtgccccagggcgtcagg

SEQ ID NO: 45252 - DNA, 28 bp, synthetic construct
  source 1..28: mol_type = other DNA
gccctggggcacttctgctctgcacagg

SEQ ID NO: 45253 - DNA, 28 bp, synthetic construct
  source 1..28: mol_type = other DNA
tcctgtgcagagcagaagtgccccaggg

SEQ ID NO: 45254 - DNA, 28 bp, synthetic construct
  source 1..28: mol_type = other DNA
gtcctgtgcagagcagaagtgccccagg

SEQ ID NO: 45255 - DNA, 28 bp, synthetic construct
  source 1..28: mol_type = other DNA
cacttctgctctgcacaggaccacgcgg

SEQ ID NO: 45256 - DNA, 28 bp, synthetic construct
  source 1..28: mol_type = other DNA
acttctgctctgcacaggaccacgcggg

SEQ ID NO: 45257 - DNA, 28 bp, synthetic construct
  source 1..28: mol_type = other DNA
cttctgctctgcacaggaccacgcgggg

SEQ ID NO: 45258 - DNA, 28 bp, synthetic construct
  source 1..28: mol_type = other DNA
ttctgctctgcacaggaccacgcggggg

SEQ ID NO: 45259 - DNA, 28 bp, synthetic construct
  source 1..28: mol_type = other DNA
cacaggaccacgcgggggtttgccatgg

SEQ ID NO: 45260 - DNA, 28 bp, synthetic construct
  source 1..28: mol_type = other DNA
tatgtcaccatggcaaacccccgcgtgg

SEQ ID NO: 45261 - DNA, 28 bp, synthetic construct
  source 1..28: mol_type = other DNA
gcgggggtttgccatggtgacataaagg

SEQ ID NO: 45262 - DNA, 28 bp, synthetic construct
  source 1..28: mol_type = other DNA
cgggggtttgccatggtgacataaaggg

SEQ ID NO: 45263 - DNA, 28 bp, synthetic construct
  source 1..28: mol_type = other DNA
gggggtttgccatggtgacataaagggg

SEQ ID NO: 45264 - DNA, 28 bp, synthetic construct
  source 1..28: mol_type = other DNA
tttgccatggtgacataaaggggcgcgg

SEQ ID NO: 45265 - DNA, 28 bp, synthetic construct
  source 1..28: mol_type = other DNA
gccatggtgacataaaggggcgcggagg

SEQ ID NO: 45266 - DNA, 28 bp, synthetic construct
  source 1..28: mol_type = other DNA
tcctccgcgcccctttatgtcaccatgg

SEQ ID NO: 45267 - DNA, 28 bp, synthetic construct
  source 1..28: mol_type = other DNA
tggtgacataaaggggcgcggaggaagg

SEQ ID NO: 45268 - DNA, 28 bp, synthetic construct
  source 1..28: mol_type = other DNA
gacataaaggggcgcggaggaaggaagg

SEQ ID NO: 45269 - DNA, 28 bp, synthetic construct
  source 1..28: mol_type = other DNA
ggaaggaaggagcgtgaccagcctgtgg

SEQ ID NO: 45270 - DNA, 28 bp, synthetic construct
  source 1..28: mol_type = other DNA
gtgaccagcctgtggactgcgcccctgg

SEQ ID NO: 45271 - DNA, 28 bp, synthetic construct
  source 1..28: mol_type = other DNA
ccagccaggggcgcagtccacaggctgg

SEQ ID NO: 45272 - DNA, 28 bp, synthetic construct
  source 1..28: mol_type = other DNA
cagcctgtggactgcgcccctggctggg

SEQ ID NO: 45273 - DNA, 28 bp, synthetic construct
  source 1..28: mol_type = other DNA
cctcccagccaggggcgcagtccacagg

SEQ ID NO: 45274 - DNA, 28 bp, synthetic construct
  source 1..28: mol_type = other DNA
tggactgcgcccctggctgggaggaagg

SEQ ID NO: 45275 - DNA, 28 bp, synthetic construct
  source 1..28: mol_type = other DNA
tgcgcccctggctgggaggaaggactgg

SEQ ID NO: 45276 - DNA, 28 bp, synthetic construct
  source 1..28: mol_type = other DNA
gcgcccctggctgggaggaaggactggg

SEQ ID NO: 45277 - DNA, 28 bp, synthetic construct
  source 1..28: mol_type = other DNA
cgcccctggctgggaggaaggactgggg

SEQ ID NO: 45278 - DNA, 28 bp, synthetic construct
  source 1..28: mol_type = other DNA
gcccctggctgggaggaaggactggggg

SEQ ID NO: 45279 - DNA, 28 bp, synthetic construct
  source 1..28: mol_type = other DNA
gcccccagtccttcctcccagccagggg

SEQ ID NO: 45280 - DNA, 28 bp, synthetic construct
  source 1..28: mol_type = other DNA
ggcccccagtccttcctcccagccaggg

SEQ ID NO: 45281 - DNA, 28 bp, synthetic construct
  source 1..28: mol_type = other DNA
gggcccccagtccttcctcccagccagg

SEQ ID NO: 45282 - DNA, 28 bp, synthetic construct
  source 1..28: mol_type = other DNA
gtggggcactgggagtggaggatctggg

SEQ ID NO: 45283 - DNA, 28 bp, synthetic construct
  source 1..28: mol_type = other DNA
tgtggggcactgggagtggaggatctgg

SEQ ID NO: 45284 - DNA, 28 bp, synthetic construct
  source 1..28: mol_type = other DNA
gatcctccactcccagtgccccacaagg

SEQ ID NO: 45285 - DNA, 28 bp, synthetic construct
  source 1..28: mol_type = other DNA
atcctccactcccagtgccccacaaggg

SEQ ID NO: 45286 - DNA, 28 bp, synthetic construct
  source 1..28: mol_type = other DNA
cgcccttgtggggcactgggagtggagg

SEQ ID NO: 45287 - DNA, 28 bp, synthetic construct
  source 1..28: mol_type = other DNA
cgacgcccttgtggggcactgggagtgg

SEQ ID NO: 45288 - DNA, 28 bp, synthetic construct
  source 1..28: mol_type = other DNA
ggaagcgacgcccttgtggggcactggg

SEQ ID NO: 45289 - DNA, 28 bp, synthetic construct
  source 1..28: mol_type = other DNA
aggaagcgacgcccttgtggggcactgg

SEQ ID NO: 45290 - DNA, 28 bp, synthetic construct
  source 1..28: mol_type = other DNA
agacttaggaagcgacgcccttgtgggg

SEQ ID NO: 45291 - DNA, 28 bp, synthetic construct
  source 1..28: mol_type = other DNA
gagacttaggaagcgacgcccttgtggg

SEQ ID NO: 45292 - DNA, 28 bp, synthetic construct
  source 1..28: mol_type = other DNA
agagacttaggaagcgacgcccttgtgg

SEQ ID NO: 45293 - DNA, 28 bp, synthetic construct
  source 1..28: mol_type = other DNA
gcttcctaagtctctgtgaatttgttgg

SEQ ID NO: 45294 - DNA, 28 bp, synthetic construct
  source 1..28: mol_type = other DNA
ctgaccaacaaattcacagagacttagg

SEQ ID NO: 45295 - DNA, 28 bp, synthetic construct
  source 1..28: mol_type = other DNA
aagtctctgtgaatttgttggtcagtgg

SEQ ID NO: 45296 - DNA, 28 bp, synthetic construct
  source 1..28: mol_type = other DNA
gacgattctcgtgtctcctcctgtgtgg

SEQ ID NO: 45297 - DNA, 28 bp, synthetic construct
  source 1..28: mol_type = other DNA
acgattctcgtgtctcctcctgtgtggg

SEQ ID NO: 45298 - DNA, 28 bp, synthetic construct
  source 1..28: mol_type = other DNA
cgattctcgtgtctcctcctgtgtgggg

SEQ ID NO: 45299 - DNA, 28 bp, synthetic construct
  source 1..28: mol_type = other DNA
tcgtgtctcctcctgtgtggggccttgg

SEQ ID NO: 45300 - DNA, 28 bp, synthetic construct
  source 1..28: mol_type = other DNA
cgtgtctcctcctgtgtggggccttggg

SEQ ID NO: 45301 - DNA, 28 bp, synthetic construct
  source 1..28: mol_type = other DNA
gtgtctcctcctgtgtggggccttgggg

SEQ ID NO: 45302 - DNA, 28 bp, synthetic construct
  source 1..28: mol_type = other DNA
tggctaccccaaggccccacacaggagg

SEQ ID NO: 45303 - DNA, 28 bp, synthetic construct
  source 1..28: mol_type = other DNA
tcctgtgtggggccttggggtagccagg

SEQ ID NO: 45304 - DNA, 28 bp, synthetic construct
  source 1..28: mol_type = other DNA
cctgtgtggggccttggggtagccaggg

SEQ ID NO: 45305 - DNA, 28 bp, synthetic construct
  source 1..28: mol_type = other DNA
tgtggggccttggggtagccagggcagg

SEQ ID NO: 45306 - DNA, 28 bp, synthetic construct
  source 1..28: mol_type = other DNA
gggccttggggtagccagggcaggccgg

SEQ ID NO: 45307 - DNA, 28 bp, synthetic construct
  source 1..28: mol_type = other DNA
ggccttggggtagccagggcaggccggg

SEQ ID NO: 45308 - DNA, 28 bp, synthetic construct
  source 1..28: mol_type = other DNA
ggcccggcctgccctggctaccccaagg

SEQ ID NO: 45309 - DNA, 28 bp, synthetic construct
  source 1..28: mol_type = other DNA
gggtagccagggcaggccgggcctccgg

SEQ ID NO: 45310 - DNA, 28 bp, synthetic construct
  source 1..28: mol_type = other DNA
tagccagggcaggccgggcctccggtgg

SEQ ID NO: 45311 - DNA, 28 bp, synthetic construct
  source 1..28: mol_type = other DNA
tggccaccggaggcccggcctgccctgg

SEQ ID NO: 45312 - DNA, 28 bp, synthetic construct
  source 1..28: mol_type = other DNA
gggcaggccgggcctccggtggccaagg

SEQ ID NO: 45313 - DNA, 28 bp, synthetic construct
  source 1..28: mol_type = other DNA
gccgggcctccggtggccaaggtctcgg

SEQ ID NO: 45314 - DNA, 28 bp, synthetic construct
  source 1..28: mol_type = other DNA
tccgagaccttggccaccggaggcccgg

SEQ ID NO: 45315 - DNA, 28 bp, synthetic construct
  source 1..28: mol_type = other DNA
gggcctccggtggccaaggtctcggagg

SEQ ID NO: 45316 - DNA, 28 bp, synthetic construct
  source 1..28: mol_type = other DNA
tggcctccgagaccttggccaccggagg

SEQ ID NO: 45317 - DNA, 28 bp, synthetic construct
  source 1..28: mol_type = other DNA
tccggtggccaaggtctcggaggccagg

SEQ ID NO: 45318 - DNA, 28 bp, synthetic construct
  source 1..28: mol_type = other DNA
tcctggcctccgagaccttggccaccgg

SEQ ID NO: 45319 - DNA, 28 bp, synthetic construct
  source 1..28: mol_type = other DNA
gcaggcatcctggcctccgagaccttgg

SEQ ID NO: 45320 - DNA, 28 bp, synthetic construct
  source 1..28: mol_type = other DNA
gtctcggaggccaggatgcctgccctgg

SEQ ID NO: 45321 - DNA, 28 bp, synthetic construct
  source 1..28: mol_type = other DNA
cggaggcatgccagggcaggcatcctgg

SEQ ID NO: 45322 - DNA, 28 bp, synthetic construct
  source 1..28: mol_type = other DNA
caggatgcctgccctggcatgcctccgg

SEQ ID NO: 45323 - DNA, 28 bp, synthetic construct
  source 1..28: mol_type = other DNA
gatgcctgccctggcatgcctccggagg

SEQ ID NO: 45324 - DNA, 28 bp, synthetic construct
  source 1..28: mol_type = other DNA
acagcctccggaggcatgccagggcagg

SEQ ID NO: 45325 - DNA, 28 bp, synthetic construct
  source 1..28: mol_type = other DNA
cgacacagcctccggaggcatgccaggg

SEQ ID NO: 45326 - DNA, 28 bp, synthetic construct
  source 1..28: mol_type = other DNA
cctggcatgcctccggaggctgtgtcgg

SEQ ID NO: 45327 - DNA, 28 bp, synthetic construct
  source 1..28: mol_type = other DNA
ggacacgtgccgacacagcctccggagg

SEQ ID NO: 45328 - DNA, 28 bp, synthetic construct
  source 1..28: mol_type = other DNA
cggggacacgtgccgacacagcctccgg

SEQ ID NO: 45329 - DNA, 28 bp, synthetic construct
  source 1..28: mol_type = other DNA
aggctgtgtcggcacgtgtccccgcagg

SEQ ID NO: 45330 - DNA, 28 bp, synthetic construct
  source 1..28: mol_type = other DNA
aacagcaggaaaaggacagcctgcgggg

SEQ ID NO: 45331 - DNA, 28 bp, synthetic construct
  source 1..28: mol_type = other DNA
gaacagcaggaaaaggacagcctgcggg

SEQ ID NO: 45332 - DNA, 28 bp, synthetic construct
  source 1..28: mol_type = other DNA
tgaacagcaggaaaaggacagcctgcgg

SEQ ID NO: 45333 - DNA, 28 bp, synthetic construct
  source 1..28: mol_type = other DNA
caggcagaagatgaacagcaggaaaagg

SEQ ID NO: 45334 - DNA, 28 bp, synthetic construct
  source 1..28: mol_type = other DNA
gctgaacaggcagaagatgaacagcagg

SEQ ID NO: 45335 - DNA, 28 bp, synthetic construct
  source 1..28: mol_type = other DNA
ttctgcctgttcagcgttttcatctcgg

SEQ ID NO: 45336 - DNA, 28 bp, synthetic construct
  source 1..28: mol_type = other DNA
gtaggccgagatgaaaacgctgaacagg

SEQ ID NO: 45337 - DNA, 28 bp, synthetic construct
  source 1..28: mol_type = other DNA
ttttcatctcggcctactacctatatgg

SEQ ID NO: 45338 - DNA, 28 bp, synthetic construct
  source 1..28: mol_type = other DNA
catctcggcctactacctatatggctgg

SEQ ID NO: 45339 - DNA, 28 bp, synthetic construct
  source 1..28: mol_type = other DNA
cctcgcttccagccatataggtagtagg

SEQ ID NO: 45340 - DNA, 28 bp, synthetic construct
  source 1..28: mol_type = other DNA
tacctatatggctggaagcgaggcctgg

SEQ ID NO: 45341 - DNA, 28 bp, synthetic construct
  source 1..28: mol_type = other DNA
ctccaggcctcgcttccagccatatagg

SEQ ID NO: 45342 - DNA, 28 bp, synthetic construct
  source 1..28: mol_type = other DNA
ggctggaagcgaggcctggagccctcgg

SEQ ID NO: 45343 - DNA, 28 bp, synthetic construct
  source 1..28: mol_type = other DNA
tggaagcgaggcctggagccctcggcgg

SEQ ID NO: 45344 - DNA, 28 bp, synthetic construct
  source 1..28: mol_type = other DNA
ctcgggggcatccgccgagggctccagg

SEQ ID NO: 45345 - DNA, 28 bp, synthetic construct
  source 1..28: mol_type = other DNA
agtcaggctcgggggcatccgccgaggg

SEQ ID NO: 45346 - DNA, 28 bp, synthetic construct
  source 1..28: mol_type = other DNA
cagtcaggctcgggggcatccgccgagg

SEQ ID NO: 45347 - DNA, 28 bp, synthetic construct
  source 1..28: mol_type = other DNA
cggcggatgcccccgagcctgactgcgg

SEQ ID NO: 45348 - DNA, 28 bp, synthetic construct
  source 1..28: mol_type = other DNA
ggcggatgcccccgagcctgactgcggg

SEQ ID NO: 45349 - DNA, 28 bp, synthetic construct
  source 1..28: mol_type = other DNA
gcggatgcccccgagcctgactgcgggg

SEQ ID NO: 45350 - DNA, 28 bp, synthetic construct
  source 1..28: mol_type = other DNA
ggcgggtccccgcagtcaggctcggggg

SEQ ID NO: 45351 - DNA, 28 bp, synthetic construct
  source 1..28: mol_type = other DNA
cggcgggtccccgcagtcaggctcgggg

SEQ ID NO: 45352 - DNA, 28 bp, synthetic construct
  source 1..28: mol_type = other DNA
gcggcgggtccccgcagtcaggctcggg

SEQ ID NO: 45353 - DNA, 28 bp, synthetic construct
  source 1..28: mol_type = other DNA
ggcggcgggtccccgcagtcaggctcgg

SEQ ID NO: 45354 - DNA, 28 bp, synthetic construct
  source 1..28: mol_type = other DNA
ccacaggcggcgggtccccgcagtcagg

SEQ ID NO: 45355 - DNA, 28 bp, synthetic construct
  source 1..28: mol_type = other DNA
caggcgactgggggccacaggcggcggg

SEQ ID NO: 45356 - DNA, 28 bp, synthetic construct
  source 1..28: mol_type = other DNA
gcaggcgactgggggccacaggcggcgg

SEQ ID NO: 45357 - DNA, 28 bp, synthetic construct
  source 1..28: mol_type = other DNA
gcagcaggcgactgggggccacaggcgg

SEQ ID NO: 45358 - DNA, 28 bp, synthetic construct
  source 1..28: mol_type = other DNA
gtggcagcaggcgactgggggccacagg

SEQ ID NO: 45359 - DNA, 28 bp, synthetic construct
  source 1..28: mol_type = other DNA
ggcttgagtggcagcaggcgactggggg

SEQ ID NO: 45360 - DNA, 28 bp, synthetic construct
  source 1..28: mol_type = other DNA
aggcttgagtggcagcaggcgactgggg

SEQ ID NO: 45361 - DNA, 28 bp, synthetic construct
  source 1..28: mol_type = other DNA
caggcttgagtggcagcaggcgactggg

SEQ ID NO: 45362 - DNA, 28 bp, synthetic construct
  source 1..28: mol_type = other DNA
acaggcttgagtggcagcaggcgactgg

SEQ ID NO: 45363 - DNA, 28 bp, synthetic construct
  source 1..28: mol_type = other DNA
cgcctgctgccactcaagcctgtgcagg

SEQ ID NO: 45364 - DNA, 28 bp, synthetic construct
  source 1..28: mol_type = other DNA
tgcctgcacaggcttgagtggcagcagg

SEQ ID NO: 45365 - DNA, 28 bp, synthetic construct
  source 1..28: mol_type = other DNA
gggtggctgcctgcacaggcttgagtgg

SEQ ID NO: 45366 - DNA, 28 bp, synthetic construct
  source 1..28: mol_type = other DNA
tgcgggaaggggtggctgcctgcacagg

SEQ ID NO: 45367 - DNA, 28 bp, synthetic construct
  source 1..28: mol_type = other DNA
gccaccccttcccgcacagacccgttgg

SEQ ID NO: 45368 - DNA, 28 bp, synthetic construct
  source 1..28: mol_type = other DNA
accaacgggtctgtgcgggaaggggtgg

SEQ ID NO: 45369 - DNA, 28 bp, synthetic construct
  source 1..28: mol_type = other DNA
agcaccaacgggtctgtgcgggaagggg

SEQ ID NO: 45370 - DNA, 28 bp, synthetic construct
  source 1..28: mol_type = other DNA
cagcaccaacgggtctgtgcgggaaggg

SEQ ID NO: 45371 - DNA, 28 bp, synthetic construct
  source 1..28: mol_type = other DNA
ccagcaccaacgggtctgtgcgggaagg

SEQ ID NO: 45372 - DNA, 28 bp, synthetic construct
  source 1..28: mol_type = other DNA
aagaccagcaccaacgggtctgtgcggg

SEQ ID NO: 45373 - DNA, 28 bp, synthetic construct
  source 1..28: mol_type = other DNA
aaagaccagcaccaacgggtctgtgcgg

SEQ ID NO: 45374 - DNA, 28 bp, synthetic construct
  source 1..28: mol_type = other DNA
acagacccgttggtgctggtctttgtgg

SEQ ID NO: 45375 - DNA, 28 bp, synthetic construct
  source 1..28: mol_type = other DNA
gctctccacaaagaccagcaccaacggg

SEQ ID NO: 45376 - DNA, 28 bp, synthetic construct
  source 1..28: mol_type = other DNA
ggctctccacaaagaccagcaccaacgg

SEQ ID NO: 45377 - DNA, 28 bp, synthetic construct
  source 1..28: mol_type = other DNA
tttgtggagagcctctactcgcaactgg

SEQ ID NO: 45378 - DNA, 28 bp, synthetic construct
  source 1..28: mol_type = other DNA
ttgtggagagcctctactcgcaactggg

SEQ ID NO: 45379 - DNA, 28 bp, synthetic construct
  source 1..28: mol_type = other DNA
gagagcctctactcgcaactgggccagg

SEQ ID NO: 45380 - DNA, 28 bp, synthetic construct
  source 1..28: mol_type = other DNA
agcctctactcgcaactgggccaggagg

SEQ ID NO: 45381 - DNA, 28 bp, synthetic construct
  source 1..28: mol_type = other DNA
cacctcctggcccagttgcgagtagagg

SEQ ID NO: 45382 - DNA, 28 bp, synthetic construct
  source 1..28: mol_type = other DNA
ctctactcgcaactgggccaggaggtgg

SEQ ID NO: 45383 - DNA, 28 bp, synthetic construct
  source 1..28: mol_type = other DNA
tactcgcaactgggccaggaggtggtgg

SEQ ID NO: 45384 - DNA, 28 bp, synthetic construct
  source 1..28: mol_type = other DNA
ctgggccaggaggtggtggccatcctgg

SEQ ID NO: 45385 - DNA, 28 bp, synthetic construct
  source 1..28: mol_type = other DNA
ggactccaggatggccaccacctcctgg

SEQ ID NO: 45386 - DNA, 28 bp, synthetic construct
  source 1..28: mol_type = other DNA
tatttgaagcggctggactccaggatgg

SEQ ID NO: 45387 - DNA, 28 bp, synthetic construct
  source 1..28: mol_type = other DNA
gcggtatttgaagcggctggactccagg

SEQ ID NO: 45388 - DNA, 28 bp, synthetic construct
  source 1..28: mol_type = other DNA
atctctgtgcggtatttgaagcggctgg

SEQ ID NO: 45389 - DNA, 28 bp, synthetic construct
  source 1..28: mol_type = other DNA
cgcaatctctgtgcggtatttgaagcgg

SEQ ID NO: 45390 - DNA, 28 bp, synthetic construct
  source 1..28: mol_type = other DNA
ttcaaataccgcacagagattgcgccgg

SEQ ID NO: 45391 - DNA, 28 bp, synthetic construct
  source 1..28: mol_type = other DNA
tcaaataccgcacagagattgcgccggg

SEQ ID NO: 45392 - DNA, 28 bp, synthetic construct
  source 1..28: mol_type = other DNA
taccgcacagagattgcgccgggcaagg

SEQ ID NO: 45393 - DNA, 28 bp, synthetic construct
  source 1..28: mol_type = other DNA
accgcacagagattgcgccgggcaaggg

SEQ ID NO: 45394 - DNA, 28 bp, synthetic construct
  source 1..28: mol_type = other DNA
acccttgcccggcgcaatctctgtgcgg

SEQ ID NO: 45395 - DNA, 28 bp, synthetic construct
  source 1..28: mol_type = other DNA
tgagcgtgggcatgtcacccttgcccgg

SEQ ID NO: 45396 - DNA, 28 bp, synthetic construct
  source 1..28: mol_type = other DNA
ggtgacatgcccacgctcactgacaagg

SEQ ID NO: 45397 - DNA, 28 bp, synthetic construct
  source 1..28: mol_type = other DNA
gtgacatgcccacgctcactgacaaggg

SEQ ID NO: 45398 - DNA, 28 bp, synthetic construct
  source 1..28: mol_type = other DNA
tgcccacgctcactgacaagggccgtgg

SEQ ID NO: 45399 - DNA, 28 bp, synthetic construct
  source 1..28: mol_type = other DNA
ggccacggcccttgtcagtgagcgtggg

SEQ ID NO: 45400 - DNA, 28 bp, synthetic construct
  source 1..28: mol_type = other DNA
cggccacggcccttgtcagtgagcgtgg

SEQ ID NO: 45401 - DNA, 28 bp, synthetic construct
  source 1..28: mol_type = other DNA
atagatgatgagggcgaagcggccacgg

SEQ ID NO: 45402 - DNA, 28 bp, synthetic construct
  source 1..28: mol_type = other DNA
gttctcatagatgatgagggcgaagcgg

SEQ ID NO: 45403 - DNA, 28 bp, synthetic construct
  source 1..28: mol_type = other DNA
ttgaggatgttctcatagatgatgaggg

SEQ ID NO: 45404 - DNA, 28 bp, synthetic construct
  source 1..28: mol_type = other DNA
cttgaggatgttctcatagatgatgagg

SEQ ID NO: 45405 - DNA, 28 bp, synthetic construct
  source 1..28: mol_type = other DNA
gagaacatcctcaagtatgtcaacctgg

SEQ ID NO: 45406 - DNA, 28 bp, synthetic construct
  source 1..28: mol_type = other DNA
cctcaagtatgtcaacctggacgcctgg

SEQ ID NO: 45407 - DNA, 28 bp, synthetic construct
  source 1..28: mol_type = other DNA
gtatgtcaacctggacgcctggaaccgg

SEQ ID NO: 45408 - DNA, 28 bp, synthetic construct
  source 1..28: mol_type = other DNA
tatgtcaacctggacgcctggaaccggg

SEQ ID NO: 45409 - DNA, 28 bp, synthetic construct
  source 1..28: mol_type = other DNA
cagcagctcccggttccaggcgtccagg

SEQ ID NO: 45410 - DNA, 28 bp, synthetic construct
  source 1..28: mol_type = other DNA
ctggacgcctggaaccgggagctgctgg

SEQ ID NO: 45411 - DNA, 28 bp, synthetic construct
  source 1..28: mol_type = other DNA
tacttgtccagcagctcccggttccagg

SEQ ID NO: 45412 - DNA, 28 bp, synthetic construct
  source 1..28: mol_type = other DNA
cacacagtacttgtccagcagctcccgg

SEQ ID NO: 45413 - DNA, 28 bp, synthetic construct
  source 1..28: mol_type = other DNA
cgggagctgctggacaagtactgtgtgg

SEQ ID NO: 45414 - DNA, 28 bp, synthetic construct
  source 1..28: mol_type = other DNA
tgctggacaagtactgtgtggcctacgg

SEQ ID NO: 45415 - DNA, 28 bp, synthetic construct
  source 1..28: mol_type = other DNA
gacaagtactgtgtggcctacggcgtgg

SEQ ID NO: 45416 - DNA, 28 bp, synthetic construct
  source 1..28: mol_type = other DNA
acaagtactgtgtggcctacggcgtggg

SEQ ID NO: 45417 - DNA, 28 bp, synthetic construct
  source 1..28: mol_type = other DNA
gtgtggcctacggcgtgggcatcattgg

SEQ ID NO: 45418 - DNA, 28 bp, synthetic construct
  source 1..28: mol_type = other DNA
aagaagccaatgatgcccacgccgtagg

SEQ ID NO: 45419 - DNA, 28 bp, synthetic construct
  source 1..28: mol_type = other DNA
ggcgtgggcatcattggcttcttcaagg

SEQ ID NO: 45420 - DNA, 28 bp, synthetic construct
  source 1..28: mol_type = other DNA
ggcttcttcaaggtacacaagaagcagg

SEQ ID NO: 45421 - DNA, 28 bp, synthetic construct
  source 1..28: mol_type = other DNA
gcttcttcaaggtacacaagaagcaggg

SEQ ID NO: 45422 - DNA, 28 bp, synthetic construct
  source 1..28: mol_type = other DNA
tgcagagggggctctgaactgctcgggg

SEQ ID NO: 45423 - DNA, 28 bp, synthetic construct
  source 1..28: mol_type = other DNA
ctgcagagggggctctgaactgctcggg

SEQ ID NO: 45424 - DNA, 28 bp, synthetic construct
  source 1..28: mol_type = other DNA
gctgcagagggggctctgaactgctcgg

SEQ ID NO: 45425 - DNA, 28 bp, synthetic construct
  source 1..28: mol_type = other DNA
gaattcaggcactgagctgcagaggggg

SEQ ID NO: 45426 - DNA, 28 bp, synthetic construct
  source 1..28: mol_type = other DNA
agaattcaggcactgagctgcagagggg

SEQ ID NO: 45427 - DNA, 28 bp, synthetic construct
  source 1..28: mol_type = other DNA
gagaattcaggcactgagctgcagaggg

SEQ ID NO: 45428 - DNA, 28 bp, synthetic construct
  source 1..28: mol_type = other DNA
tgagaattcaggcactgagctgcagagg

SEQ ID NO: 45429 - DNA, 28 bp, synthetic construct
  source 1..28: mol_type = other DNA
gtgcctgaattctcatttgtgaaatagg

SEQ ID NO: 45430 - DNA, 28 bp, synthetic construct
  source 1..28: mol_type = other DNA
acacctatttcacaaatgagaattcagg

SEQ ID NO: 45431 - DNA, 28 bp, synthetic construct
  source 1..28: mol_type = other DNA
attctcatttgtgaaataggtgtaatgg

SEQ ID NO: 45432 - DNA, 28 bp, synthetic construct
  source 1..28: mol_type = other DNA
aggtgtaatggtagcacccgcctcctgg

SEQ ID NO: 45433 - DNA, 28 bp, synthetic construct
  source 1..28: mol_type = other DNA
ggtgtaatggtagcacccgcctcctggg

SEQ ID NO: 45434 - DNA, 28 bp, synthetic construct
  source 1..28: mol_type = other DNA
gtgtaatggtagcacccgcctcctgggg

SEQ ID NO: 45435 - DNA, 28 bp, synthetic construct
  source 1..28: mol_type = other DNA
ggtagcacccgcctcctggggttgttgg

SEQ ID NO: 45436 - DNA, 28 bp, synthetic construct
  source 1..28: mol_type = other DNA
gtagcacccgcctcctggggttgttggg

SEQ ID NO: 45437 - DNA, 28 bp, synthetic construct
  source 1..28: mol_type = other DNA
gcacccgcctcctggggttgttgggagg

SEQ ID NO: 45438 - DNA, 28 bp, synthetic construct
  source 1..28: mol_type = other DNA
cacccgcctcctggggttgttgggaggg

SEQ ID NO: 45439 - DNA, 28 bp, synthetic construct
  source 1..28: mol_type = other DNA
aaccctcccaacaaccccaggaggcggg

SEQ ID NO: 45440 - DNA, 28 bp, synthetic construct
  source 1..28: mol_type = other DNA
taaccctcccaacaaccccaggaggcgg

SEQ ID NO: 45441 - DNA, 28 bp, synthetic construct
  source 1..28: mol_type = other DNA
atttaaccctcccaacaaccccaggagg

SEQ ID NO: 45442 - DNA, 28 bp, synthetic construct
  source 1..28: mol_type = other DNA
ctcatttaaccctcccaacaaccccagg

SEQ ID NO: 45443 - DNA, 28 bp, synthetic construct
  source 1..28: mol_type = other DNA
atcaatattcaccaacattcatggaggg

SEQ ID NO: 45444 - DNA, 28 bp, synthetic construct
  source 1..28: mol_type = other DNA
tatcaatattcaccaacattcatggagg

SEQ ID NO: 45445 - DNA, 28 bp, synthetic construct
  source 1..28: mol_type = other DNA
tggtatcaatattcaccaacattcatgg

SEQ ID NO: 45446 - DNA, 28 bp, synthetic construct
  source 1..28: mol_type = other DNA
ttggtgaatattgataccactgttatgg

SEQ ID NO: 45447 - DNA, 28 bp, synthetic construct
  source 1..28: mol_type = other DNA
gtctctcacatgtggaccataacagtgg

SEQ ID NO: 45448 - DNA, 28 bp, synthetic construct
  source 1..28: mol_type = other DNA
tccacatgtgagagactgtgtcctttgg

SEQ ID NO: 45449 - DNA, 28 bp, synthetic construct
  source 1..28: mol_type = other DNA
ccacatgtgagagactgtgtcctttggg

SEQ ID NO: 45450 - DNA, 28 bp, synthetic construct
  source 1..28: mol_type = other DNA
cacatgtgagagactgtgtcctttgggg

SEQ ID NO: 45451 - DNA, 28 bp, synthetic construct
  source 1..28: mol_type = other DNA
tgagagactgtgtcctttggggttctgg

SEQ ID NO: 45452 - DNA, 28 bp, synthetic construct
  source 1..28: mol_type = other DNA
agaactgtcacatccagaaccccaaagg

SEQ ID NO: 45453 - DNA, 28 bp, synthetic construct
  source 1..28: mol_type = other DNA
ccccttcctgccctccattgactgcagg

SEQ ID NO: 45454 - DNA, 28 bp, synthetic construct
  source 1..28: mol_type = other DNA
gcctgcagtcaatggagggcaggaaggg

SEQ ID NO: 45455 - DNA, 28 bp, synthetic construct
  source 1..28: mol_type = other DNA
ggcctgcagtcaatggagggcaggaagg

SEQ ID NO: 45456 - DNA, 28 bp, synthetic construct
  source 1..28: mol_type = other DNA
cattggcctgcagtcaatggagggcagg

SEQ ID NO: 45457 - DNA, 28 bp, synthetic construct
  source 1..28: mol_type = other DNA
ttctcattggcctgcagtcaatggaggg

SEQ ID NO: 45458 - DNA, 28 bp, synthetic construct
  source 1..28: mol_type = other DNA
gttctcattggcctgcagtcaatggagg

SEQ ID NO: 45459 - DNA, 28 bp, synthetic construct
  source 1..28: mol_type = other DNA
gctgttctcattggcctgcagtcaatgg

SEQ ID NO: 45460 - DNA, 28 bp, synthetic construct
  source 1..28: mol_type = other DNA
tgcgcactcagcaggctgttctcattgg

SEQ ID NO: 45461 - DNA, 28 bp, synthetic construct
  source 1..28: mol_type = other DNA
aacagcctgctgagtgcgcagctcaagg

SEQ ID NO: 45462 - DNA, 28 bp, synthetic construct
  source 1..28: mol_type = other DNA
acagcctgctgagtgcgcagctcaaggg

SEQ ID NO: 45463 - DNA, 28 bp, synthetic construct
  source 1..28: mol_type = other DNA
gaagcccttgagctgcgcactcagcagg

SEQ ID NO: 45464 - DNA, 28 bp, synthetic construct
  source 1..28: mol_type = other DNA
ttccccctgttcctgcactcaaacctgg

SEQ ID NO: 45465 - DNA, 28 bp, synthetic construct
  source 1..28: mol_type = other DNA
tccccctgttcctgcactcaaacctggg

SEQ ID NO: 45466 - DNA, 28 bp, synthetic construct
  source 1..28: mol_type = other DNA
gcccaggtttgagtgcaggaacaggggg

SEQ ID NO: 45467 - DNA, 28 bp, synthetic construct
  source 1..28: mol_type = other DNA
ggcccaggtttgagtgcaggaacagggg

SEQ ID NO: 45468 - DNA, 28 bp, synthetic construct
  source 1..28: mol_type = other DNA
aggcccaggtttgagtgcaggaacaggg

SEQ ID NO: 45469 - DNA, 28 bp, synthetic construct
  source 1..28: mol_type = other DNA
caggcccaggtttgagtgcaggaacagg

SEQ ID NO: 45470 - DNA, 28 bp, synthetic construct
  source 1..28: mol_type = other DNA
ttcctgcactcaaacctgggcctgaagg

SEQ ID NO: 45471 - DNA, 28 bp, synthetic construct
  source 1..28: mol_type = other DNA
gtccttcaggcccaggtttgagtgcagg

SEQ ID NO: 45472 - DNA, 28 bp, synthetic construct
  source 1..28: mol_type = other DNA
gttgatgctgcagtccttcaggcccagg

SEQ ID NO: 45473 - DNA, 28 bp, synthetic construct
  source 1..28: mol_type = other DNA
cttggggttgatgctgcagtccttcagg

SEQ ID NO: 45474 - DNA, 28 bp, synthetic construct
  source 1..28: mol_type = other DNA
cgtcacgtagagcagcggggacttgggg

SEQ ID NO: 45475 - DNA, 28 bp, synthetic construct
  source 1..28: mol_type = other DNA
gcgtcacgtagagcagcggggacttggg

SEQ ID NO: 45476 - DNA, 28 bp, synthetic construct
  source 1..28: mol_type = other DNA
cgcgtcacgtagagcagcggggacttgg

SEQ ID NO: 45477 - DNA, 28 bp, synthetic construct
  source 1..28: mol_type = other DNA
ctaggtcgcgtcacgtagagcagcgggg

SEQ ID NO: 45478 - DNA, 28 bp, synthetic construct
  source 1..28: mol_type = other DNA
gctaggtcgcgtcacgtagagcagcggg

SEQ ID NO: 45479 - DNA, 28 bp, synthetic construct
  source 1..28: mol_type = other DNA
cgctaggtcgcgtcacgtagagcagcgg

SEQ ID NO: 45480 - DNA, 28 bp, synthetic construct
  source 1..28: mol_type = other DNA
ctgctctacgtgacgcgacctagcgagg

SEQ ID NO: 45481 - DNA, 28 bp, synthetic construct
  source 1..28: mol_type = other DNA
ctctacgtgacgcgacctagcgaggtgg

SEQ ID NO: 45482 - DNA, 28 bp, synthetic construct
  source 1..28: mol_type = other DNA
tgacgcgacctagcgaggtggagaaagg

SEQ ID NO: 45483 - DNA, 28 bp, synthetic construct
  source 1..28: mol_type = other DNA
ggagcacacctttctccacctcgctagg

SEQ ID NO: 45484 - DNA, 28 bp, synthetic construct
  source 1..28: mol_type = other DNA
gcgaggtggagaaaggtgtgctccccgg

SEQ ID NO: 45485 - DNA, 28 bp, synthetic construct
  source 1..28: mol_type = other DNA
gtggagaaaggtgtgctccccggcgagg

SEQ ID NO: 45486 - DNA, 28 bp, synthetic construct
  source 1..28: mol_type = other DNA
gaaaggtgtgctccccggcgaggactgg

SEQ ID NO: 45487 - DNA, 28 bp, synthetic construct
  source 1..28: mol_type = other DNA
ggtgtgctccccggcgaggactggacgg

SEQ ID NO: 45488 - DNA, 28 bp, synthetic construct
  source 1..28: mol_type = other DNA
ctggaaaaccgtccagtcctcgccgggg

SEQ ID NO: 45489 - DNA, 28 bp, synthetic construct
  source 1..28: mol_type = other DNA
actggaaaaccgtccagtcctcgccggg

SEQ ID NO: 45490 - DNA, 28 bp, synthetic construct
  source 1..28: mol_type = other DNA
gactggaaaaccgtccagtcctcgccgg

SEQ ID NO: 45491 - DNA, 28 bp, synthetic construct
  source 1..28: mol_type = other DNA
tggctcataggtggagtgatttgactgg

SEQ ID NO: 45492 - DNA, 28 bp, synthetic construct
  source 1..28: mol_type = other DNA
cactccacctatgagccagtgctgctgg

SEQ ID NO: 45493 - DNA, 28 bp, synthetic construct
  source 1..28: mol_type = other DNA
ttggccagcagcactggctcataggtgg

SEQ ID NO: 45494 - DNA, 28 bp, synthetic construct
  source 1..28: mol_type = other DNA
gtcttggccagcagcactggctcatagg

SEQ ID NO: 45495 - DNA, 28 bp, synthetic construct
  source 1..28: mol_type = other DNA
acgagcgcgtcttggccagcagcactgg

SEQ ID NO: 45496 - DNA, 28 bp, synthetic construct
  source 1..28: mol_type = other DNA
gggatggactcagacgagcgcgtcttgg

SEQ ID NO: 45497 - DNA, 28 bp, synthetic construct
  source 1..28: mol_type = other DNA
cgctcgtctgagtccatcccacacctgg

SEQ ID NO: 45498 - DNA, 28 bp, synthetic construct
  source 1..28: mol_type = other DNA
gctcgtctgagtccatcccacacctggg

SEQ ID NO: 45499 - DNA, 28 bp, synthetic construct
  source 1..28: mol_type = other DNA
ccggcgtctgcgcccaggtgtgggatgg

SEQ ID NO: 45500 - DNA, 28 bp, synthetic construct
  source 1..28: mol_type = other DNA
caggccggcgtctgcgcccaggtgtggg

SEQ ID NO: 45501 - DNA, 28 bp, synthetic construct
  source 1..28: mol_type = other DNA
gcaggccggcgtctgcgcccaggtgtgg

SEQ ID NO: 45502 - DNA, 28 bp, synthetic construct
  source 1..28: mol_type = other DNA
agcatgcaggccggcgtctgcgcccagg

SEQ ID NO: 45503 - DNA, 28 bp, synthetic construct
  source 1..28: mol_type = other DNA
gtggcgtgcagtgcagcatgcaggccgg

SEQ ID NO: 45504 - DNA, 28 bp, synthetic construct
  source 1..28: mol_type = other DNA
cacagtggcgtgcagtgcagcatgcagg

SEQ ID NO: 45505 - DNA, 28 bp, synthetic construct
  source 1..28: mol_type = other DNA
ctgcatgctgcactgcacgccactgtgg

SEQ ID NO: 45506 - DNA, 28 bp, synthetic construct
  source 1..28: mol_type = other DNA
gctgcactgcacgccactgtggtccagg

SEQ ID NO: 45507 - DNA, 28 bp, synthetic construct
  source 1..28: mol_type = other DNA
ctgcacgccactgtggtccaggacctgg

SEQ ID NO: 45508 - DNA, 28 bp, synthetic construct
  source 1..28: mol_type = other DNA
tgcacgccactgtggtccaggacctggg

SEQ ID NO: 45509 - DNA, 28 bp, synthetic construct
  source 1..28: mol_type = other DNA
tgcaggcccaggtcctggaccacagtgg

SEQ ID NO: 45510 - DNA, 28 bp, synthetic construct
  source 1..28: mol_type = other DNA
tggtccaggacctgggcctgcacgacgg

SEQ ID NO: 45511 - DNA, 28 bp, synthetic construct
  source 1..28: mol_type = other DNA
gatgccgtcgtgcaggcccaggtcctgg

SEQ ID NO: 45512 - DNA, 28 bp, synthetic construct
  source 1..28: mol_type = other DNA
gcgctggatgccgtcgtgcaggcccagg

SEQ ID NO: 45513 - DNA, 28 bp, synthetic construct
  source 1..28: mol_type = other DNA
cagcacgcgctggatgccgtcgtgcagg

SEQ ID NO: 45514 - DNA, 28 bp, synthetic construct
  source 1..28: mol_type = other DNA
acgacggcatccagcgcgtgctgtttgg

SEQ ID NO: 45515 - DNA, 28 bp, synthetic construct
  source 1..28: mol_type = other DNA
caggttgttgccaaacagcacgcgctgg

SEQ ID NO: 45516 - DNA, 28 bp, synthetic construct
  source 1..28: mol_type = other DNA
gctgtttggcaacaacctgaacttctgg

SEQ ID NO: 45517 - DNA, 28 bp, synthetic construct
  source 1..28: mol_type = other DNA
gacaagcttgtgcagccagaagttcagg

SEQ ID NO: 45518 - DNA, 28 bp, synthetic construct
  source 1..28: mol_type = other DNA
ttctggctgcacaagcttgtcttcgtgg

SEQ ID NO: 45519 - DNA, 28 bp, synthetic construct
  source 1..28: mol_type = other DNA
cacaagcttgtcttcgtggatgccgtgg

SEQ ID NO: 45520 - DNA, 28 bp, synthetic construct
  source 1..28: mol_type = other DNA
ttcgtggatgccgtggccttcctcacgg

SEQ ID NO: 45521 - DNA, 28 bp, synthetic construct
  source 1..28: mol_type = other DNA
tcgtggatgccgtggccttcctcacggg

SEQ ID NO: 45522 - DNA, 28 bp, synthetic construct
  source 1..28: mol_type = other DNA
cgtggatgccgtggccttcctcacgggg

SEQ ID NO: 45523 - DNA, 28 bp, synthetic construct
  source 1..28: mol_type = other DNA
aggcgcttccccgtgaggaaggccacgg

SEQ ID NO: 45524 - DNA, 28 bp, synthetic construct
  source 1..28: mol_type = other DNA
agggagaggcgcttccccgtgaggaagg

SEQ ID NO: 45525 - DNA, 28 bp, synthetic construct
  source 1..28: mol_type = other DNA
tggcagggagaggcgcttccccgtgagg

SEQ ID NO: 45526 - DNA, 28 bp, synthetic construct
  source 1..28: mol_type = other DNA
acggggaagcgcctctccctgccattgg

SEQ ID NO: 45527 - DNA, 28 bp, synthetic construct
  source 1..28: mol_type = other DNA
gatgtagcggtccaatggcagggagagg

SEQ ID NO: 45528 - DNA, 28 bp, synthetic construct
  source 1..28: mol_type = other DNA
tccctgccattggaccgctacatcctgg

SEQ ID NO: 45529 - DNA, 28 bp, synthetic construct
  source 1..28: mol_type = other DNA
accaggatgtagcggtccaatggcaggg

SEQ ID NO: 45530 - DNA, 28 bp, synthetic construct
  source 1..28: mol_type = other DNA
caccaggatgtagcggtccaatggcagg

SEQ ID NO: 45531 - DNA, 28 bp, synthetic construct
  source 1..28: mol_type = other DNA
ctgccattggaccgctacatcctggtgg

SEQ ID NO: 45532 - DNA, 28 bp, synthetic construct
  source 1..28: mol_type = other DNA
tgtccaccaggatgtagcggtccaatgg

SEQ ID NO: 45533 - DNA, 28 bp, synthetic construct
  source 1..28: mol_type = other DNA
gtcatcaatgtccaccaggatgtagcgg

SEQ ID NO: 45534 - DNA, 28 bp, synthetic construct
  source 1..28: mol_type = other DNA
cacgaagatgtcatcaatgtccaccagg

SEQ ID NO: 45535 - DNA, 28 bp, synthetic construct
  source 1..28: mol_type = other DNA
ctggtggacattgatgacatcttcgtgg

SEQ ID NO: 45536 - DNA, 28 bp, synthetic construct
  source 1..28: mol_type = other DNA
tggtggacattgatgacatcttcgtggg

SEQ ID NO: 45537 - DNA, 28 bp, synthetic construct
  source 1..28: mol_type = other DNA
gacattgatgacatcttcgtgggcaagg

SEQ ID NO: 45538 - DNA, 28 bp, synthetic construct
  source 1..28: mol_type = other DNA
attgatgacatcttcgtgggcaaggagg

SEQ ID NO: 45539 - DNA, 28 bp, synthetic construct
  source 1..28: mol_type = other DNA
ttgatgacatcttcgtgggcaaggaggg

SEQ ID NO: 45540 - DNA, 28 bp, synthetic construct
  source 1..28: mol_type = other DNA
gtgggcaaggagggcacacgcatgaagg

SEQ ID NO: 45541 - DNA, 28 bp, synthetic construct
  source 1..28: mol_type = other DNA
ggcaaggagggcacacgcatgaaggtgg

SEQ ID NO: 45542 - DNA, 28 bp, synthetic construct
  source 1..28: mol_type = other DNA
aaggagggcacacgcatgaaggtggagg

SEQ ID NO: 45543 - DNA, 28 bp, synthetic construct
  source 1..28: mol_type = other DNA
acacgcatgaaggtggaggacgtgaagg

SEQ ID NO: 45544 - DNA, 28 bp, synthetic construct
  source 1..28: mol_type = other DNA
catgaaggtggaggacgtgaaggtatgg

SEQ ID NO: 45545 - DNA, 28 bp, synthetic construct
  source 1..28: mol_type = other DNA
aaggtggaggacgtgaaggtatggccgg

SEQ ID NO: 45546 - DNA, 28 bp, synthetic construct
  source 1..28: mol_type = other DNA
aggtggaggacgtgaaggtatggccggg

SEQ ID NO: 45547 - DNA, 28 bp, synthetic construct
  source 1..28: mol_type = other DNA
ggtggaggacgtgaaggtatggccgggg

SEQ ID NO: 45548 - DNA, 28 bp, synthetic construct
  source 1..28: mol_type = other DNA
gtggaggacgtgaaggtatggccggggg

SEQ ID NO: 45549 - DNA, 28 bp, synthetic construct
  source 1..28: mol_type = other DNA
gaaggtatggccgggggtgctagaccgg

SEQ ID NO: 45550 - DNA, 28 bp, synthetic construct
  source 1..28: mol_type = other DNA
aaggtatggccgggggtgctagaccggg

SEQ ID NO: 45551 - DNA, 28 bp, synthetic construct
  source 1..28: mol_type = other DNA
atggccgggggtgctagaccgggcaagg

SEQ ID NO: 45552 - DNA, 28 bp, synthetic construct
  source 1..28: mol_type = other DNA
cctgccttgcccggtctagcacccccgg

SEQ ID NO: 45553 - DNA, 28 bp, synthetic construct
  source 1..28: mol_type = other DNA
ggggtgctagaccgggcaaggcaggtgg

SEQ ID NO: 45554 - DNA, 28 bp, synthetic construct
  source 1..28: mol_type = other DNA
gggtgctagaccgggcaaggcaggtggg

SEQ ID NO: 45555 - DNA, 28 bp, synthetic construct
  source 1..28: mol_type = other DNA
ggtgctagaccgggcaaggcaggtgggg

SEQ ID NO: 45556 - DNA, 28 bp, synthetic construct
  source 1..28: mol_type = other DNA
tagaccgggcaaggcaggtggggcctgg

SEQ ID NO: 45557 - DNA, 28 bp, synthetic construct
  source 1..28: mol_type = other DNA
cttgccaggccccacctgccttgcccgg

SEQ ID NO: 45558 - DNA, 28 bp, synthetic construct
  source 1..28: mol_type = other DNA
tggggcctggcaagcttcagccttcagg

SEQ ID NO: 45559 - DNA, 28 bp, synthetic construct
  source 1..28: mol_type = other DNA
gggcacctgaaggctgaagcttgccagg

SEQ ID NO: 45560 - DNA, 28 bp, synthetic construct
  source 1..28: mol_type = other DNA
gcttcagccttcaggtgccccatcgtgg

SEQ ID NO: 45561 - DNA, 28 bp, synthetic construct
  source 1..28: mol_type = other DNA
cttcagccttcaggtgccccatcgtggg

SEQ ID NO: 45562 - DNA, 28 bp, synthetic construct
  source 1..28: mol_type = other DNA
ggcacacccacgatggggcacctgaagg

SEQ ID NO: 45563 - DNA, 28 bp, synthetic construct
  source 1..28: mol_type = other DNA
atgcagacagggcacacccacgatgggg

SEQ ID NO: 45564 - DNA, 28 bp, synthetic construct
  source 1..28: mol_type = other DNA
gatgcagacagggcacacccacgatggg

SEQ ID NO: 45565 - DNA, 28 bp, synthetic construct
  source 1..28: mol_type = other DNA
agatgcagacagggcacacccacgatgg

SEQ ID NO: 45566 - DNA, 28 bp, synthetic construct
  source 1..28: mol_type = other DNA
tgccctgtctgcatctcccctatgctgg

SEQ ID NO: 45567 - DNA, 28 bp, synthetic construct
  source 1..28: mol_type = other DNA
gccctgtctgcatctcccctatgctggg

SEQ ID NO: 45568 - DNA, 28 bp, synthetic construct
  source 1..28: mol_type = other DNA
tcccagcataggggagatgcagacaggg

SEQ ID NO: 45569 - DNA, 28 bp, synthetic construct
  source 1..28: mol_type = other DNA
ctcccagcataggggagatgcagacagg

SEQ ID NO: 45570 - DNA, 28 bp, synthetic construct
  source 1..28: mol_type = other DNA
gtcttttaagtaactcccagcatagggg

SEQ ID NO: 45571 - DNA, 28 bp, synthetic construct
  source 1..28: mol_type = other DNA
tgtcttttaagtaactcccagcataggg

SEQ ID NO: 45572 - DNA, 28 bp, synthetic construct
  source 1..28: mol_type = other DNA
ctgtcttttaagtaactcccagcatagg

SEQ ID NO: 45573 - DNA, 28 bp, synthetic construct
  source 1..28: mol_type = other DNA
caaaaattataaagaatgtcaaggacgg

SEQ ID NO: 45574 - DNA, 28 bp, synthetic construct
  source 1..28: mol_type = other DNA
tgttcaaaaattataaagaatgtcaagg

SEQ ID NO: 45575 - DNA, 28 bp, synthetic construct
  source 1..28: mol_type = other DNA
tgacattctttataatttttgaacaagg

SEQ ID NO: 45576 - DNA, 28 bp, synthetic construct
  source 1..28: mol_type = other DNA
gacattctttataatttttgaacaaggg

SEQ ID NO: 45577 - DNA, 28 bp, synthetic construct
  source 1..28: mol_type = other DNA
ttccacgttttttcactgccctcagtgg

SEQ ID NO: 45578 - DNA, 28 bp, synthetic construct
  source 1..28: mol_type = other DNA
tccacgttttttcactgccctcagtggg

SEQ ID NO: 45579 - DNA, 28 bp, synthetic construct
  source 1..28: mol_type = other DNA
tcccactgagggcagtgaaaaaacgtgg

SEQ ID NO: 45580 - DNA, 28 bp, synthetic construct
  source 1..28: mol_type = other DNA
tttcactgccctcagtgggaaaagcagg

SEQ ID NO: 45581 - DNA, 28 bp, synthetic construct
  source 1..28: mol_type = other DNA
ttcactgccctcagtgggaaaagcaggg

SEQ ID NO: 45582 - DNA, 28 bp, synthetic construct
  source 1..28: mol_type = other DNA
aggagctccctgcttttcccactgaggg

SEQ ID NO: 45583 - DNA, 28 bp, synthetic construct
  source 1..28: mol_type = other DNA
caggagctccctgcttttcccactgagg

SEQ ID NO: 45584 - DNA, 28 bp, synthetic construct
  source 1..28: mol_type = other DNA
ctcagtgggaaaagcagggagctcctgg

SEQ ID NO: 45585 - DNA, 28 bp, synthetic construct
  source 1..28: mol_type = other DNA
agaaaggaatgagtgagggaaagccagg

SEQ ID NO: 45586 - DNA, 28 bp, synthetic construct
  source 1..28: mol_type = other DNA
aggcaggggagaaaggaatgagtgaggg

SEQ ID NO: 45587 - DNA, 28 bp, synthetic construct
  source 1..28: mol_type = other DNA
caggcaggggagaaaggaatgagtgagg

SEQ ID NO: 45588 - DNA, 28 bp, synthetic construct
  source 1..28: mol_type = other DNA
cattcctttctcccctgcctgtcctagg

SEQ ID NO: 45589 - DNA, 28 bp, synthetic construct
  source 1..28: mol_type = other DNA
agggcctaggacaggcaggggagaaagg

SEQ ID NO: 45590 - DNA, 28 bp, synthetic construct
  source 1..28: mol_type = other DNA
gtcaaacagggcctaggacaggcagggg

SEQ ID NO: 45591 - DNA, 28 bp, synthetic construct
  source 1..28: mol_type = other DNA
tgtcaaacagggcctaggacaggcaggg

SEQ ID NO: 45592 - DNA, 28 bp, synthetic construct
  source 1..28: mol_type = other DNA
gtgtcaaacagggcctaggacaggcagg

SEQ ID NO: 45593 - DNA, 28 bp, synthetic construct
  source 1..28: mol_type = other DNA
ctgtgtgtcaaacagggcctaggacagg

SEQ ID NO: 45594 - DNA, 28 bp, synthetic construct
  source 1..28: mol_type = other DNA
tcgttctgtgtgtcaaacagggcctagg

SEQ ID NO: 45595 - DNA, 28 bp, synthetic construct
  source 1..28: mol_type = other DNA
cgtagttcgttctgtgtgtcaaacaggg

SEQ ID NO: 45596 - DNA, 28 bp, synthetic construct
  source 1..28: mol_type = other DNA
gcgtagttcgttctgtgtgtcaaacagg

SEQ ID NO: 45597 - DNA, 28 bp, synthetic construct
  source 1..28: mol_type = other DNA
cacatcccaaacttcaccttcaacctgg

SEQ ID NO: 45598 - DNA, 28 bp, synthetic construct
  source 1..28: mol_type = other DNA
acatcccaaacttcaccttcaacctggg

SEQ ID NO: 45599 - DNA, 28 bp, synthetic construct
  source 1..28: mol_type = other DNA
gtagcccaggttgaaggtgaagtttggg

SEQ ID NO: 45600 - DNA, 28 bp, synthetic construct
  source 1..28: mol_type = other DNA
agtagcccaggttgaaggtgaagtttgg

SEQ ID NO: 45601 - DNA, 28 bp, synthetic construct
  source 1..28: mol_type = other DNA
acttcaccttcaacctgggctactcagg

SEQ ID NO: 45602 - DNA, 28 bp, synthetic construct
  source 1..28: mol_type = other DNA
cttcaccttcaacctgggctactcaggg

SEQ ID NO: 45603 - DNA, 28 bp, synthetic construct
  source 1..28: mol_type = other DNA
aatttccctgagtagcccaggttgaagg

SEQ ID NO: 45604 - DNA, 28 bp, synthetic construct
  source 1..28: mol_type = other DNA
gtggaagaatttccctgagtagcccagg

SEQ ID NO: 45605 - DNA, 28 bp, synthetic construct
  source 1..28: mol_type = other DNA
gctactcagggaaattcttccacacagg

SEQ ID NO: 45606 - DNA, 28 bp, synthetic construct
  source 1..28: mol_type = other DNA
agggaaattcttccacacaggtaagtgg

SEQ ID NO: 45607 - DNA, 28 bp, synthetic construct
  source 1..28: mol_type = other DNA
gggaaattcttccacacaggtaagtggg

SEQ ID NO: 45608 - DNA, 28 bp, synthetic construct
  source 1..28: mol_type = other DNA
gcaggggcaggcccacttacctgtgtgg

SEQ ID NO: 45609 - DNA, 28 bp, synthetic construct
  source 1..28: mol_type = other DNA
ggaagttgctagtgagggcaggggcagg

SEQ ID NO: 45610 - DNA, 28 bp, synthetic construct
  source 1..28: mol_type = other DNA
gcccctgccctcactagcaacttccagg

SEQ ID NO: 45611 - DNA, 28 bp, synthetic construct
  source 1..28: mol_type = other DNA
tcctggaagttgctagtgagggcagggg

SEQ ID NO: 45612 - DNA, 28 bp, synthetic construct
  source 1..28: mol_type = other DNA
gtcctggaagttgctagtgagggcaggg

SEQ ID NO: 45613 - DNA, 28 bp, synthetic construct
  source 1..28: mol_type = other DNA
agtcctggaagttgctagtgagggcagg

SEQ ID NO: 45614 - DNA, 28 bp, synthetic construct
  source 1..28: mol_type = other DNA
gaggagtcctggaagttgctagtgaggg

SEQ ID NO: 45615 - DNA, 28 bp, synthetic construct
  source 1..28: mol_type = other DNA
tgaggagtcctggaagttgctagtgagg

SEQ ID NO: 45616 - DNA, 28 bp, synthetic construct
  source 1..28: mol_type = other DNA
tgagggtttgggtgctgaggagtcctgg

SEQ ID NO: 45617 - DNA, 28 bp, synthetic construct
  source 1..28: mol_type = other DNA
gggtgctttgagggtttgggtgctgagg

SEQ ID NO: 45618 - DNA, 28 bp, synthetic construct
  source 1..28: mol_type = other DNA
tcatggatgggtgctttgagggtttggg

SEQ ID NO: 45619 - DNA, 28 bp, synthetic construct
  source 1..28: mol_type = other DNA
ctcatggatgggtgctttgagggtttgg

SEQ ID NO: 45620 - DNA, 28 bp, synthetic construct
  source 1..28: mol_type = other DNA
caaaccctcaaagcacccatccatgagg

SEQ ID NO: 45621 - DNA, 28 bp, synthetic construct
  source 1..28: mol_type = other DNA
aaaccctcaaagcacccatccatgaggg

SEQ ID NO: 45622 - DNA, 28 bp, synthetic construct
  source 1..28: mol_type = other DNA
ctgccctcatggatgggtgctttgaggg

SEQ ID NO: 45623 - DNA, 28 bp, synthetic construct
  source 1..28: mol_type = other DNA
gctgccctcatggatgggtgctttgagg

SEQ ID NO: 45624 - DNA, 28 bp, synthetic construct
  source 1..28: mol_type = other DNA
tcaaagcacccatccatgagggcagcgg

SEQ ID NO: 45625 - DNA, 28 bp, synthetic construct
  source 1..28: mol_type = other DNA
caaagcacccatccatgagggcagcggg

SEQ ID NO: 45626 - DNA, 28 bp, synthetic construct
  source 1..28: mol_type = other DNA
agcacccatccatgagggcagcgggtgg

SEQ ID NO: 45627 - DNA, 28 bp, synthetic construct
  source 1..28: mol_type = other DNA
gcacccatccatgagggcagcgggtggg

SEQ ID NO: 45628 - DNA, 28 bp, synthetic construct
  source 1..28: mol_type = other DNA
aaacccacccgctgccctcatggatggg

SEQ ID NO: 45629 - DNA, 28 bp, synthetic construct
  source 1..28: mol_type = other DNA
taaacccacccgctgccctcatggatgg

SEQ ID NO: 45630 - DNA, 28 bp, synthetic construct
  source 1..28: mol_type = other DNA
ccatgagggcagcgggtgggtttactgg

SEQ ID NO: 45631 - DNA, 28 bp, synthetic construct
  source 1..28: mol_type = other DNA
gggtgggtttactggcccacattagagg

SEQ ID NO: 45632 - DNA, 28 bp, synthetic construct
  source 1..28: mol_type = other DNA
gtttactggcccacattagaggcagagg

SEQ ID NO: 45633 - DNA, 28 bp, synthetic construct
  source 1..28: mol_type = other DNA
caggagctgcctggaagagttatctggg

SEQ ID NO: 45634 - DNA, 28 bp, synthetic construct
  source 1..28: mol_type = other DNA
ccaggagctgcctggaagagttatctgg

SEQ ID NO: 45635 - DNA, 28 bp, synthetic construct
  source 1..28: mol_type = other DNA
cagataactcttccaggcagctcctggg

SEQ ID NO: 45636 - DNA, 28 bp, synthetic construct
  source 1..28: mol_type = other DNA
ataactcttccaggcagctcctgggtgg

SEQ ID NO: 45637 - DNA, 28 bp, synthetic construct
  source 1..28: mol_type = other DNA
taactcttccaggcagctcctgggtggg

SEQ ID NO: 45638 - DNA, 28 bp, synthetic construct
  source 1..28: mol_type = other DNA
ttccaggcagctcctgggtgggctctgg

SEQ ID NO: 45639 - DNA, 28 bp, synthetic construct
  source 1..28: mol_type = other DNA
ggccagagcccacccaggagctgcctgg

SEQ ID NO: 45640 - DNA, 28 bp, synthetic construct
  source 1..28: mol_type = other DNA
gggagagcatggccagagcccacccagg

SEQ ID NO: 45641 - DNA, 28 bp, synthetic construct
  source 1..28: mol_type = other DNA
gctctggccatgctctcccatccccagg

SEQ ID NO: 45642 - DNA, 28 bp, synthetic construct
  source 1..28: mol_type = other DNA
gccatgctctcccatccccaggcacagg

SEQ ID NO: 45643 - DNA, 28 bp, synthetic construct
  source 1..28: mol_type = other DNA
gcctgtgcctggggatgggagagcatgg

SEQ ID NO: 45644 - DNA, 28 bp, synthetic construct
  source 1..28: mol_type = other DNA
ctctcccatccccaggcacaggcccagg

SEQ ID NO: 45645 - DNA, 28 bp, synthetic construct
  source 1..28: mol_type = other DNA
ctaacctgggcctgtgcctggggatggg

SEQ ID NO: 45646 - DNA, 28 bp, synthetic construct
  source 1..28: mol_type = other DNA
tctaacctgggcctgtgcctggggatgg

SEQ ID NO: 45647 - DNA, 28 bp, synthetic construct
  source 1..28: mol_type = other DNA
atccccaggcacaggcccaggttagagg

SEQ ID NO: 45648 - DNA, 28 bp, synthetic construct
  source 1..28: mol_type = other DNA
tccccaggcacaggcccaggttagaggg

SEQ ID NO: 45649 - DNA, 28 bp, synthetic construct
  source 1..28: mol_type = other DNA
gccctctaacctgggcctgtgcctgggg

SEQ ID NO: 45650 - DNA, 28 bp, synthetic construct
  source 1..28: mol_type = other DNA
ggccctctaacctgggcctgtgcctggg

SEQ ID NO: 45651 - DNA, 28 bp, synthetic construct
  source 1..28: mol_type = other DNA
aggccctctaacctgggcctgtgcctgg

SEQ ID NO: 45652 - DNA, 28 bp, synthetic construct
  source 1..28: mol_type = other DNA
cacaggcccaggttagagggcctcatgg

SEQ ID NO: 45653 - DNA, 28 bp, synthetic construct
  source 1..28: mol_type = other DNA
actgggccatgaggccctctaacctggg

SEQ ID NO: 45654 - DNA, 28 bp, synthetic construct
  source 1..28: mol_type = other DNA
cactgggccatgaggccctctaacctgg

SEQ ID NO: 45655 - DNA, 28 bp, synthetic construct
  source 1..28: mol_type = other DNA
caggttagagggcctcatggcccagtgg

SEQ ID NO: 45656 - DNA, 28 bp, synthetic construct
  source 1..28: mol_type = other DNA
aggttagagggcctcatggcccagtggg

SEQ ID NO: 45657 - DNA, 28 bp, synthetic construct
  source 1..28: mol_type = other DNA
ttagagggcctcatggcccagtgggtgg

SEQ ID NO: 45658 - DNA, 28 bp, synthetic construct
  source 1..28: mol_type = other DNA
gctcagaaccacccactgggccatgagg

SEQ ID NO: 45659 - DNA, 28 bp, synthetic construct
  source 1..28: mol_type = other DNA
cacaggcagctcagaaccacccactggg

SEQ ID NO: 45660 - DNA, 28 bp, synthetic construct
  source 1..28: mol_type = other DNA
acacaggcagctcagaaccacccactgg

SEQ ID NO: 45661 - DNA, 28 bp, synthetic construct
  source 1..28: mol_type = other DNA
ggttctgagctgcctgtgttgctgcagg

SEQ ID NO: 45662 - DNA, 28 bp, synthetic construct
  source 1..28: mol_type = other DNA
tcagcattggtacctgcagcaacacagg

SEQ ID NO: 45663 - DNA, 28 bp, synthetic construct
  source 1..28: mol_type = other DNA
tgtgttgctgcaggtaccaatgctgagg

SEQ ID NO: 45664 - DNA, 28 bp, synthetic construct
  source 1..28: mol_type = other DNA
ctgcaggtaccaatgctgaggacgctgg

SEQ ID NO: 45665 - DNA, 28 bp, synthetic construct
  source 1..28: mol_type = other DNA
tgcaggtaccaatgctgaggacgctggg

SEQ ID NO: 45666 - DNA, 28 bp, synthetic construct
  source 1..28: mol_type = other DNA
gcaggtaccaatgctgaggacgctgggg

SEQ ID NO: 45667 - DNA, 28 bp, synthetic construct
  source 1..28: mol_type = other DNA
agatcatccccagcgtcctcagcattgg

SEQ ID NO: 45668 - DNA, 28 bp, synthetic construct
  source 1..28: mol_type = other DNA
gatgatctgctgctgtcgtatgtgaagg

SEQ ID NO: 45669 - DNA, 28 bp, synthetic construct
  source 1..28: mol_type = other DNA
gctgctgtcgtatgtgaaggagttctgg

SEQ ID NO: 45670 - DNA, 28 bp, synthetic construct
  source 1..28: mol_type = other DNA
gctgtcgtatgtgaaggagttctggtgg

SEQ ID NO: 45671 - DNA, 28 bp, synthetic construct
  source 1..28: mol_type = other DNA
ggagttctggtggttcccccacatgtgg

SEQ ID NO: 45672 - DNA, 28 bp, synthetic construct
  source 1..28: mol_type = other DNA
gggctgcatgtggctccacatgtggggg

SEQ ID NO: 45673 - DNA, 28 bp, synthetic construct
  source 1..28: mol_type = other DNA
ggggctgcatgtggctccacatgtgggg

SEQ ID NO: 45674 - DNA, 28 bp, synthetic construct
  source 1..28: mol_type = other DNA
tggggctgcatgtggctccacatgtggg

SEQ ID NO: 45675 - DNA, 28 bp, synthetic construct
  source 1..28: mol_type = other DNA
gtggggctgcatgtggctccacatgtgg

SEQ ID NO: 45676 - DNA, 28 bp, synthetic construct
  source 1..28: mol_type = other DNA
gttgtggaaaaggtggggctgcatgtgg

SEQ ID NO: 45677 - DNA, 28 bp, synthetic construct
  source 1..28: mol_type = other DNA
acacggactggttgtggaaaaggtgggg

SEQ ID NO: 45678 - DNA, 28 bp, synthetic construct
  source 1..28: mol_type = other DNA
aacacggactggttgtggaaaaggtggg

SEQ ID NO: 45679 - DNA, 28 bp, synthetic construct
  source 1..28: mol_type = other DNA
caacacggactggttgtggaaaaggtgg

SEQ ID NO: 45680 - DNA, 28 bp, synthetic construct
  source 1..28: mol_type = other DNA
caccttttccacaaccagtccgtgttgg

SEQ ID NO: 45681 - DNA, 28 bp, synthetic construct
  source 1..28: mol_type = other DNA
ggccaacacggactggttgtggaaaagg

SEQ ID NO: 45682 - DNA, 28 bp, synthetic construct
  source 1..28: mol_type = other DNA
ctgctcggccaacacggactggttgtgg

SEQ ID NO: 45683 - DNA, 28 bp, synthetic construct
  source 1..28: mol_type = other DNA
aaccagtccgtgttggccgagcagatgg

SEQ ID NO: 45684 - DNA, 28 bp, synthetic construct
  source 1..28: mol_type = other DNA
ggccatctgctcggccaacacggactgg

SEQ ID NO: 45685 - DNA, 28 bp, synthetic construct
  source 1..28: mol_type = other DNA
ttcaaggccatctgctcggccaacacgg

SEQ ID NO: 45686 - DNA, 28 bp, synthetic construct
  source 1..28: mol_type = other DNA
aacttcttgttcaaggccatctgctcgg

SEQ ID NO: 45687 - DNA, 28 bp, synthetic construct
  source 1..28: mol_type = other DNA
ctcacgacagcgaacttcttgttcaagg

SEQ ID NO: 45688 - DNA, 28 bp, synthetic construct
  source 1..28: mol_type = other DNA
cgctgtcgtgagtaagattccttgcagg

SEQ ID NO: 45689 - DNA, 28 bp, synthetic construct
  source 1..28: mol_type = other DNA
gctgtcgtgagtaagattccttgcaggg

SEQ ID NO: 45690 - DNA, 28 bp, synthetic construct
  source 1..28: mol_type = other DNA
gagtaagattccttgcagggcagagcgg

SEQ ID NO: 45691 - DNA, 28 bp, synthetic construct
  source 1..28: mol_type = other DNA
agtaagattccttgcagggcagagcggg

SEQ ID NO: 45692 - DNA, 28 bp, synthetic construct
  source 1..28: mol_type = other DNA
gtaagattccttgcagggcagagcgggg

SEQ ID NO: 45693 - DNA, 28 bp, synthetic construct
  source 1..28: mol_type = other DNA
agattccttgcagggcagagcggggcgg

SEQ ID NO: 45694 - DNA, 28 bp, synthetic construct
  source 1..28: mol_type = other DNA
gattccttgcagggcagagcggggcggg

SEQ ID NO: 45695 - DNA, 28 bp, synthetic construct
  source 1..28: mol_type = other DNA
ttagcccgccccgctctgccctgcaagg

SEQ ID NO: 45696 - DNA, 28 bp, synthetic construct
  source 1..28: mol_type = other DNA
ttgcagggcagagcggggcgggctaagg

SEQ ID NO: 45697 - DNA, 28 bp, synthetic construct
  source 1..28: mol_type = other DNA
tgcagggcagagcggggcgggctaaggg

SEQ ID NO: 45698 - DNA, 28 bp, synthetic construct
  source 1..28: mol_type = other DNA
gggcagagcggggcgggctaagggctgg

SEQ ID NO: 45699 - DNA, 28 bp, synthetic construct
  source 1..28: mol_type = other DNA
ggcagagcggggcgggctaagggctggg

SEQ ID NO: 45700 - DNA, 28 bp, synthetic construct
  source 1..28: mol_type = other DNA
gagcggggcgggctaagggctgggctgg

SEQ ID NO: 45701 - DNA, 28 bp, synthetic construct
  source 1..28: mol_type = other DNA
cggggcgggctaagggctgggctggagg

SEQ ID NO: 45702 - DNA, 28 bp, synthetic construct
  source 1..28: mol_type = other DNA
gggctgggctggaggtccagactgctgg

SEQ ID NO: 45703 - DNA, 28 bp, synthetic construct
  source 1..28: mol_type = other DNA
caaaagcagcaagaggccagcagtctgg

SEQ ID NO: 45704 - DNA, 28 bp, synthetic construct
  source 1..28: mol_type = other DNA
cagagcagactgcaaaagcagcaagagg

SEQ ID NO: 45705 - DNA, 28 bp, synthetic construct
  source 1..28: mol_type = other DNA
ttgctgcttttgcagtctgctctgacgg

SEQ ID NO: 45706 - DNA, 28 bp, synthetic construct
  source 1..28: mol_type = other DNA
tctgacggatttttactaacacctctgg

SEQ ID NO: 45707 - DNA, 28 bp, synthetic construct
  source 1..28: mol_type = other DNA
ctgacggatttttactaacacctctggg

SEQ ID NO: 45708 - DNA, 28 bp, synthetic construct
  source 1..28: mol_type = other DNA
ggatttttactaacacctctgggccagg

SEQ ID NO: 45709 - DNA, 28 bp, synthetic construct
  source 1..28: mol_type = other DNA
gatttttactaacacctctgggccaggg

SEQ ID NO: 45710 - DNA, 28 bp, synthetic construct
  source 1..28: mol_type = other DNA
tcagaggttaggtcggcatggctgctgg

SEQ ID NO: 45711 - DNA, 28 bp, synthetic construct
  source 1..28: mol_type = other DNA
agagaaatcagaggttaggtcggcatgg

SEQ ID NO: 45712 - DNA, 28 bp, synthetic construct
  source 1..28: mol_type = other DNA
gggagagagaaatcagaggttaggtcgg

SEQ ID NO: 45713 - DNA, 28 bp, synthetic construct
  source 1..28: mol_type = other DNA
gaatgggagagagaaatcagaggttagg

SEQ ID NO: 45714 - DNA, 28 bp, synthetic construct
  source 1..28: mol_type = other DNA
ttgtagaatgggagagagaaatcagagg

SEQ ID NO: 45715 - DNA, 28 bp, synthetic construct
  source 1..28: mol_type = other DNA
ctgatttctctctcccattctacaaagg

SEQ ID NO: 45716 - DNA, 28 bp, synthetic construct
  source 1..28: mol_type = other DNA
tgatttctctctcccattctacaaaggg

SEQ ID NO: 45717 - DNA, 28 bp, synthetic construct
  source 1..28: mol_type = other DNA
gatttctctctcccattctacaaagggg

SEQ ID NO: 45718 - DNA, 28 bp, synthetic construct
  source 1..28: mol_type = other DNA
atttctctctcccattctacaaaggggg

SEQ ID NO: 45719 - DNA, 28 bp, synthetic construct
  source 1..28: mol_type = other DNA
tttctctctcccattctacaaagggggg

SEQ ID NO: 45720 - DNA, 28 bp, synthetic construct
  source 1..28: mol_type = other DNA
tctcccattctacaaaggggggataagg

SEQ ID NO: 45721 - DNA, 28 bp, synthetic construct
  source 1..28: mol_type = other DNA
gggccttatcccccctttgtagaatggg

SEQ ID NO: 45722 - DNA, 28 bp, synthetic construct
  source 1..28: mol_type = other DNA
tgggccttatcccccctttgtagaatgg

SEQ ID NO: 45723 - DNA, 28 bp, synthetic construct
  source 1..28: mol_type = other DNA
tctacaaaggggggataaggcccaaagg

SEQ ID NO: 45724 - DNA, 28 bp, synthetic construct
  source 1..28: mol_type = other DNA
ctacaaaggggggataaggcccaaaggg

SEQ ID NO: 45725 - DNA, 28 bp, synthetic construct
  source 1..28: mol_type = other DNA
tacaaaggggggataaggcccaaagggg

SEQ ID NO: 45726 - DNA, 28 bp, synthetic construct
  source 1..28: mol_type = other DNA
aaggggggataaggcccaaaggggaagg

SEQ ID NO: 45727 - DNA, 28 bp, synthetic construct
  source 1..28: mol_type = other DNA
gtgagcataggggtccttcccctttggg

SEQ ID NO: 45728 - DNA, 28 bp, synthetic construct
  source 1..28: mol_type = other DNA
ggtgagcataggggtccttcccctttgg

SEQ ID NO: 45729 - DNA, 28 bp, synthetic construct
  source 1..28: mol_type = other DNA
aggggaaggacccctatgctcaccctgg

SEQ ID NO: 45730 - DNA, 28 bp, synthetic construct
  source 1..28: mol_type = other DNA
aaggacccctatgctcaccctggcctgg

SEQ ID NO: 45731 - DNA, 28 bp, synthetic construct
  source 1..28: mol_type = other DNA
gatgaccaggccagggtgagcatagggg

SEQ ID NO: 45732 - DNA, 28 bp, synthetic construct
  source 1..28: mol_type = other DNA
ggatgaccaggccagggtgagcataggg

SEQ ID NO: 45733 - DNA, 28 bp, synthetic construct
  source 1..28: mol_type = other DNA
aggatgaccaggccagggtgagcatagg

SEQ ID NO: 45734 - DNA, 28 bp, synthetic construct
  source 1..28: mol_type = other DNA
accctggcctggtcatcctctccctagg

SEQ ID NO: 45735 - DNA, 28 bp, synthetic construct
  source 1..28: mol_type = other DNA
tcctagggagaggatgaccaggccaggg

SEQ ID NO: 45736 - DNA, 28 bp, synthetic construct
  source 1..28: mol_type = other DNA
ctcctagggagaggatgaccaggccagg

SEQ ID NO: 45737 - DNA, 28 bp, synthetic construct
  source 1..28: mol_type = other DNA
cctggtcatcctctccctaggagcatgg

SEQ ID NO: 45738 - DNA, 28 bp, synthetic construct
  source 1..28: mol_type = other DNA
gtgggaatgccatgctcctagggagagg

SEQ ID NO: 45739 - DNA, 28 bp, synthetic construct
  source 1..28: mol_type = other DNA
tgtctgtgggaatgccatgctcctaggg

SEQ ID NO: 45740 - DNA, 28 bp, synthetic construct
  source 1..28: mol_type = other DNA
atgtctgtgggaatgccatgctcctagg

SEQ ID NO: 45741 - DNA, 28 bp, synthetic construct
  source 1..28: mol_type = other DNA
taggagcatggcattcccacagacatgg

SEQ ID NO: 45742 - DNA, 28 bp, synthetic construct
  source 1..28: mol_type = other DNA
aggagcatggcattcccacagacatggg

SEQ ID NO: 45743 - DNA, 28 bp, synthetic construct
  source 1..28: mol_type = other DNA
ggagcatggcattcccacagacatgggg

SEQ ID NO: 45744 - DNA, 28 bp, synthetic construct
  source 1..28: mol_type = other DNA
attcccacagacatggggtatgcagtgg

SEQ ID NO: 45745 - DNA, 28 bp, synthetic construct
  source 1..28: mol_type = other DNA
gcgccactgcataccccatgtctgtggg

SEQ ID NO: 45746 - DNA, 28 bp, synthetic construct
  source 1..28: mol_type = other DNA
ggcgccactgcataccccatgtctgtgg

SEQ ID NO: 45747 - DNA, 28 bp, synthetic construct
  source 1..28: mol_type = other DNA
gggtatgcagtggcgccccaccactcgg

SEQ ID NO: 45748 - DNA, 28 bp, synthetic construct
  source 1..28: mol_type = other DNA
ggtatgcagtggcgccccaccactcggg

SEQ ID NO: 45749 - DNA, 28 bp, synthetic construct
  source 1..28: mol_type = other DNA
gcacggggtacacgcccgagtggtgggg

SEQ ID NO: 45750 - DNA, 28 bp, synthetic construct
  source 1..28: mol_type = other DNA
tgcacggggtacacgcccgagtggtggg

SEQ ID NO: 45751 - DNA, 28 bp, synthetic construct
  source 1..28: mol_type = other DNA
gtgcacggggtacacgcccgagtggtgg

SEQ ID NO: 45752 - DNA, 28 bp, synthetic construct
  source 1..28: mol_type = other DNA
cacgtgcacggggtacacgcccgagtgg

SEQ ID NO: 45753 - DNA, 28 bp, synthetic construct
  source 1..28: mol_type = other DNA
taccccgtgcacgtgcagctgtacgagg

SEQ ID NO: 45754 - DNA, 28 bp, synthetic construct
  source 1..28: mol_type = other DNA
agcctcgtacagctgcacgtgcacgggg

SEQ ID NO: 45755 - DNA, 28 bp, synthetic construct
  source 1..28: mol_type = other DNA
aagcctcgtacagctgcacgtgcacggg

SEQ ID NO: 45756 - DNA, 28 bp, synthetic construct
  source 1..28: mol_type = other DNA
caagcctcgtacagctgcacgtgcacgg

SEQ ID NO: 45757 - DNA, 28 bp, synthetic construct
  source 1..28: mol_type = other DNA
cgtgcacgtgcagctgtacgaggcttgg

SEQ ID NO: 45758 - DNA, 28 bp, synthetic construct
  source 1..28: mol_type = other DNA
gtgcagctgtacgaggcttggaagcagg

SEQ ID NO: 45759 - DNA, 28 bp, synthetic construct
  source 1..28: mol_type = other DNA
gctgtacgaggcttggaagcaggtgtgg

SEQ ID NO: 45760 - DNA, 28 bp, synthetic construct
  source 1..28: mol_type = other DNA
gtgtggagcatccgcgtgaccagcacgg

SEQ ID NO: 45761 - DNA, 28 bp, synthetic construct
  source 1..28: mol_type = other DNA
tggagcatccgcgtgaccagcacggagg

SEQ ID NO: 45762 - DNA, 28 bp, synthetic construct
  source 1..28: mol_type = other DNA
ggggtactcctccgtgctggtcacgcgg

SEQ ID NO: 45763 - DNA, 28 bp, synthetic construct
  source 1..28: mol_type = other DNA
ttcaggtgggggtactcctccgtgctgg

SEQ ID NO: 45764 - DNA, 28 bp, synthetic construct
  source 1..28: mol_type = other DNA
gcggtagcgggctggcttcaggtggggg

SEQ ID NO: 45765 - DNA, 28 bp, synthetic construct
  source 1..28: mol_type = other DNA
ggcggtagcgggctggcttcaggtgggg

SEQ ID NO: 45766 - DNA, 28 bp, synthetic construct
  source 1..28: mol_type = other DNA
cggcggtagcgggctggcttcaggtggg

SEQ ID NO: 45767 - DNA, 28 bp, synthetic construct
  source 1..28: mol_type = other DNA
acggcggtagcgggctggcttcaggtgg

SEQ ID NO: 45768 - DNA, 28 bp, synthetic construct
  source 1..28: mol_type = other DNA
acctgaagccagcccgctaccgccgtgg

SEQ ID NO: 45769 - DNA, 28 bp, synthetic construct
  source 1..28: mol_type = other DNA
gccacggcggtagcgggctggcttcagg

SEQ ID NO: 45770 - DNA, 28 bp, synthetic construct
  source 1..28: mol_type = other DNA
ggatgaagccacggcggtagcgggctgg

SEQ ID NO: 45771 - DNA, 28 bp, synthetic construct
  source 1..28: mol_type = other DNA
ttgtggatgaagccacggcggtagcggg

SEQ ID NO: 45772 - DNA, 28 bp, synthetic construct
  source 1..28: mol_type = other DNA
attgtggatgaagccacggcggtagcgg

SEQ ID NO: 45773 - DNA, 28 bp, synthetic construct
  source 1..28: mol_type = other DNA
gctaccgccgtggcttcatccacaatgg

SEQ ID NO: 45774 - DNA, 28 bp, synthetic construct
  source 1..28: mol_type = other DNA
gatgccattgtggatgaagccacggcgg

SEQ ID NO: 45775 - DNA, 28 bp, synthetic construct
  source 1..28: mol_type = other DNA
catgatgccattgtggatgaagccacgg

SEQ ID NO: 45776 - DNA, 28 bp, synthetic construct
  source 1..28: mol_type = other DNA
cgtggcttcatccacaatggcatcatgg

SEQ ID NO: 45777 - DNA, 28 bp, synthetic construct
  source 1..28: mol_type = other DNA
tcatccacaatggcatcatggtgagtgg

SEQ ID NO: 45778 - DNA, 28 bp, synthetic construct
  source 1..28: mol_type = other DNA
catccacaatggcatcatggtgagtggg

SEQ ID NO: 45779 - DNA, 28 bp, synthetic construct
  source 1..28: mol_type = other DNA
gggcccactcaccatgatgccattgtgg

SEQ ID NO: 45780 - DNA, 28 bp, synthetic construct
  source 1..28: mol_type = other DNA
aatggcatcatggtgagtgggcccctgg

SEQ ID NO: 45781 - DNA, 28 bp, synthetic construct
  source 1..28: mol_type = other DNA
atggtgagtgggcccctggaagcccagg

SEQ ID NO: 45782 - DNA, 28 bp, synthetic construct
  source 1..28: mol_type = other DNA
gtgagtgggcccctggaagcccaggagg

SEQ ID NO: 45783 - DNA, 28 bp, synthetic construct
  source 1..28: mol_type = other DNA
agtgggcccctggaagcccaggaggtgg

SEQ ID NO: 45784 - DNA, 28 bp, synthetic construct
  source 1..28: mol_type = other DNA
gtgggcccctggaagcccaggaggtggg

SEQ ID NO: 45785 - DNA, 28 bp, synthetic construct
  source 1..28: mol_type = other DNA
attctcccacctcctgggcttccagggg

SEQ ID NO: 45786 - DNA, 28 bp, synthetic construct
  source 1..28: mol_type = other DNA
cattctcccacctcctgggcttccaggg

SEQ ID NO: 45787 - DNA, 28 bp, synthetic construct
  source 1..28: mol_type = other DNA
ccattctcccacctcctgggcttccagg

SEQ ID NO: 45788 - DNA, 28 bp, synthetic construct
  source 1..28: mol_type = other DNA
tgtgctctccattctcccacctcctggg

SEQ ID NO: 45789 - DNA, 28 bp, synthetic construct
  source 1..28: mol_type = other DNA
ctgtgctctccattctcccacctcctgg

SEQ ID NO: 45790 - DNA, 28 bp, synthetic construct
  source 1..28: mol_type = other DNA
tgtcatgtgtgtgcatacgctgtcctgg

SEQ ID NO: 45791 - DNA, 28 bp, synthetic construct
  source 1..28: mol_type = other DNA
tgtgcatacgctgtcctggtaagcacgg

SEQ ID NO: 45792 - DNA, 28 bp, synthetic construct
  source 1..28: mol_type = other DNA
tacgctgtcctggtaagcacggctctgg

SEQ ID NO: 45793 - DNA, 28 bp, synthetic construct
  source 1..28: mol_type = other DNA
cctggtaagcacggctctggtttgctgg

SEQ ID NO: 45794 - DNA, 28 bp, synthetic construct
  source 1..28: mol_type = other DNA
aagcacggctctggtttgctggcttagg

SEQ ID NO: 45795 - DNA, 28 bp, synthetic construct
  source 1..28: mol_type = other DNA
agcacggctctggtttgctggcttaggg

SEQ ID NO: 45796 - DNA, 28 bp, synthetic construct
  source 1..28: mol_type = other DNA
gcacggctctggtttgctggcttagggg

SEQ ID NO: 45797 - DNA, 28 bp, synthetic construct
  source 1..28: mol_type = other DNA
cgaccacatggagactgcctttctgagg

SEQ ID NO: 45798 - DNA, 28 bp, synthetic construct
  source 1..28: mol_type = other DNA
gctcctcagaaaggcagtctccatgtgg

SEQ ID NO: 45799 - DNA, 28 bp, synthetic construct
  source 1..28: mol_type = other DNA
ggagactgcctttctgaggagcagctgg

SEQ ID NO: 45800 - DNA, 28 bp, synthetic construct
  source 1..28: mol_type = other DNA
gagactgcctttctgaggagcagctggg

SEQ ID NO: 45801 - DNA, 28 bp, synthetic construct
  source 1..28: mol_type = other DNA
aagaaggcccagctgctcctcagaaagg

SEQ ID NO: 45802 - DNA, 28 bp, synthetic construct
  source 1..28: mol_type = other DNA
ggagcagctgggccttcttcctctgagg

SEQ ID NO: 45803 - DNA, 28 bp, synthetic construct
  source 1..28: mol_type = other DNA
gggaggactcttcctcagaggaagaagg

SEQ ID NO: 45804 - DNA, 28 bp, synthetic construct
  source 1..28: mol_type = other DNA
gggtggtgggaggactcttcctcagagg

SEQ ID NO: 45805 - DNA, 28 bp, synthetic construct
  source 1..28: mol_type = other DNA
gtcctcccaccaccctcatgccagaagg

SEQ ID NO: 45806 - DNA, 28 bp, synthetic construct
  source 1..28: mol_type = other DNA
tgccttctggcatgagggtggtgggagg

SEQ ID NO: 45807 - DNA, 28 bp, synthetic construct
  source 1..28: mol_type = other DNA
tggtgccttctggcatgagggtggtggg

SEQ ID NO: 45808 - DNA, 28 bp, synthetic construct
  source 1..28: mol_type = other DNA
atggtgccttctggcatgagggtggtgg

SEQ ID NO: 45809 - DNA, 28 bp, synthetic construct
  source 1..28: mol_type = other DNA
gctatggtgccttctggcatgagggtgg

SEQ ID NO: 45810 - DNA, 28 bp, synthetic construct
  source 1..28: mol_type = other DNA
ggagctatggtgccttctggcatgaggg

SEQ ID NO: 45811 - DNA, 28 bp, synthetic construct
  source 1..28: mol_type = other DNA
aggagctatggtgccttctggcatgagg

SEQ ID NO: 45812 - DNA, 28 bp, synthetic construct
  source 1..28: mol_type = other DNA
gggggagaggagctatggtgccttctgg

SEQ ID NO: 45813 - DNA, 28 bp, synthetic construct
  source 1..28: mol_type = other DNA
aggagggggtgggggagaggagctatgg

SEQ ID NO: 45814 - DNA, 28 bp, synthetic construct
  source 1..28: mol_type = other DNA
agctcctctcccccaccccctcctcagg

SEQ ID NO: 45815 - DNA, 28 bp, synthetic construct
  source 1..28: mol_type = other DNA
agaacctgaggagggggtgggggagagg

SEQ ID NO: 45816 - DNA, 28 bp, synthetic construct
  source 1..28: mol_type = other DNA
gtgggagaacctgaggagggggtggggg

SEQ ID NO: 45817 - DNA, 28 bp, synthetic construct
  source 1..28: mol_type = other DNA
cgtgggagaacctgaggagggggtgggg

SEQ ID NO: 45818 - DNA, 28 bp, synthetic construct
  source 1..28: mol_type = other DNA
cccaccccctcctcaggttctcccacgg

SEQ ID NO: 45819 - DNA, 28 bp, synthetic construct
  source 1..28: mol_type = other DNA
gccgtgggagaacctgaggagggggtgg

SEQ ID NO: 45820 - DNA, 28 bp, synthetic construct
  source 1..28: mol_type = other DNA
tctgccgtgggagaacctgaggaggggg

SEQ ID NO: 45821 - DNA, 28 bp, synthetic construct
  source 1..28: mol_type = other DNA
gtctgccgtgggagaacctgaggagggg

SEQ ID NO: 45822 - DNA, 28 bp, synthetic construct
  source 1..28: mol_type = other DNA
ggtctgccgtgggagaacctgaggaggg

SEQ ID NO: 45823 - DNA, 28 bp, synthetic construct
  source 1..28: mol_type = other DNA
aggtctgccgtgggagaacctgaggagg

SEQ ID NO: 45824 - DNA, 28 bp, synthetic construct
  source 1..28: mol_type = other DNA
cgcaggtctgccgtgggagaacctgagg

SEQ ID NO: 45825 - DNA, 28 bp, synthetic construct
  source 1..28: mol_type = other DNA
ctcaggttctcccacggcagacctgcgg

SEQ ID NO: 45826 - DNA, 28 bp, synthetic construct
  source 1..28: mol_type = other DNA
tgtgaagaggccgcaggtctgccgtggg

SEQ ID NO: 45827 - DNA, 28 bp, synthetic construct
  source 1..28: mol_type = other DNA
gtgtgaagaggccgcaggtctgccgtgg

SEQ ID NO: 45828 - DNA, 28 bp, synthetic construct
  source 1..28: mol_type = other DNA
aagatggtgtgtgtgaagaggccgcagg

SEQ ID NO: 45829 - DNA, 28 bp, synthetic construct
  source 1..28: mol_type = other DNA
gttgtagaagatggtgtgtgtgaagagg

SEQ ID NO: 45830 - DNA, 28 bp, synthetic construct
  source 1..28: mol_type = other DNA
acaccatcttctacaacgagtaccctgg

SEQ ID NO: 45831 - DNA, 28 bp, synthetic construct
  source 1..28: mol_type = other DNA
ccgccagggtactcgttgtagaagatgg

SEQ ID NO: 45832 - DNA, 28 bp, synthetic construct
  source 1..28: mol_type = other DNA
gagtaccctggcggctccagtgagctgg

SEQ ID NO: 45833 - DNA, 28 bp, synthetic construct
  source 1..28: mol_type = other DNA
cttgtccagctcactggagccgccaggg

SEQ ID NO: 45834 - DNA, 28 bp, synthetic construct
  source 1..28: mol_type = other DNA
tcttgtccagctcactggagccgccagg

SEQ ID NO: 45835 - DNA, 28 bp, synthetic construct
  source 1..28: mol_type = other DNA
ccgttgatgatcttgtccagctcactgg

SEQ ID NO: 45836 - DNA, 28 bp, synthetic construct
  source 1..28: mol_type = other DNA
cagtgagctggacaagatcatcaacggg

SEQ ID NO: 45837 - DNA, 28 bp, synthetic construct
  source 1..28: mol_type = other DNA
agtgagctggacaagatcatcaacgggg

SEQ ID NO: 45838 - DNA, 28 bp, synthetic construct
  source 1..28: mol_type = other DNA
gtgagctggacaagatcatcaacggggg

SEQ ID NO: 45839 - DNA, 28 bp, synthetic construct
  source 1..28: mol_type = other DNA
actcacaggattgaggagcacggtgagg

SEQ ID NO: 45840 - DNA, 28 bp, synthetic construct
  source 1..28: mol_type = other DNA
ggagcactcacaggattgaggagcacgg

SEQ ID NO: 45841 - DNA, 28 bp, synthetic construct
  source 1..28: mol_type = other DNA
gggctgtggagcactcacaggattgagg

SEQ ID NO: 45842 - DNA, 28 bp, synthetic construct
  source 1..28: mol_type = other DNA
aatcctgtgagtgctccacagcccatgg

SEQ ID NO: 45843 - DNA, 28 bp, synthetic construct
  source 1..28: mol_type = other DNA
cagccatgggctgtggagcactcacagg

SEQ ID NO: 45844 - DNA, 28 bp, synthetic construct
  source 1..28: mol_type = other DNA
tgagtgctccacagcccatggctgctgg

SEQ ID NO: 45845 - DNA, 28 bp, synthetic construct
  source 1..28: mol_type = other DNA
ccacagcccatggctgctggtgagaagg

SEQ ID NO: 45846 - DNA, 28 bp, synthetic construct
  source 1..28: mol_type = other DNA
cacagcccatggctgctggtgagaaggg

SEQ ID NO: 45847 - DNA, 28 bp, synthetic construct
  source 1..28: mol_type = other DNA
acagcccatggctgctggtgagaagggg

SEQ ID NO: 45848 - DNA, 28 bp, synthetic construct
  source 1..28: mol_type = other DNA
gcagccccttctcaccagcagccatggg

SEQ ID NO: 45849 - DNA, 28 bp, synthetic construct
  source 1..28: mol_type = other DNA
agcagccccttctcaccagcagccatgg

SEQ ID NO: 45850 - DNA, 28 bp, synthetic construct
  source 1..28: mol_type = other DNA
tgcacagcctgtctgcagctgacacagg

SEQ ID NO: 45851 - DNA, 28 bp, synthetic construct
  source 1..28: mol_type = other DNA
caggaagcctgtgtcagctgcagacagg

SEQ ID NO: 45852 - DNA, 28 bp, synthetic construct
  source 1..28: mol_type = other DNA
ctgtctgcagctgacacaggcttcctgg

SEQ ID NO: 45853 - DNA, 28 bp, synthetic construct
  source 1..28: mol_type = other DNA
cagctgacacaggcttcctggagccagg

SEQ ID NO: 45854 - DNA, 28 bp, synthetic construct
  source 1..28: mol_type = other DNA
gacacaggcttcctggagccaggaaagg

SEQ ID NO: 45855 - DNA, 28 bp, synthetic construct
  source 1..28: mol_type = other DNA
acacaggcttcctggagccaggaaaggg

SEQ ID NO: 45856 - DNA, 28 bp, synthetic construct
  source 1..28: mol_type = other DNA
caggcttcctggagccaggaaagggtgg

SEQ ID NO: 45857 - DNA, 28 bp, synthetic construct
  source 1..28: mol_type = other DNA
ttcctggagccaggaaagggtggagagg

SEQ ID NO: 45858 - DNA, 28 bp, synthetic construct
  source 1..28: mol_type = other DNA
tgcctctccaccctttcctggctccagg

SEQ ID NO: 45859 - DNA, 28 bp, synthetic construct
  source 1..28: mol_type = other DNA
tcactcatgcctctccaccctttcctgg

SEQ ID NO: 45860 - DNA, 28 bp, synthetic construct
  source 1..28: mol_type = other DNA
gggtggagaggcatgagtgagtgcctgg

SEQ ID NO: 45861 - DNA, 28 bp, synthetic construct
  source 1..28: mol_type = other DNA
gaggcatgagtgagtgcctggcagttgg

SEQ ID NO: 45862 - DNA, 28 bp, synthetic construct
  source 1..28: mol_type = other DNA
aggcatgagtgagtgcctggcagttggg

SEQ ID NO: 45863 - DNA, 28 bp, synthetic construct
  source 1..28: mol_type = other DNA
agcttgcaaggctcctgatgaccagtgg

SEQ ID NO: 45864 - DNA, 28 bp, synthetic construct
  source 1..28: mol_type = other DNA
tggtcatcaggagccttgcaagctaagg

SEQ ID NO: 45865 - DNA, 28 bp, synthetic construct
  source 1..28: mol_type = other DNA
catcaggagccttgcaagctaaggcagg

SEQ ID NO: 45866 - DNA, 28 bp, synthetic construct
  source 1..28: mol_type = other DNA
atcaggagccttgcaagctaaggcaggg

SEQ ID NO: 45867 - DNA, 28 bp, synthetic construct
  source 1..28: mol_type = other DNA
ccttctgaccctgccttagcttgcaagg

SEQ ID NO: 45868 - DNA, 28 bp, synthetic construct
  source 1..28: mol_type = other DNA
cttgcaagctaaggcagggtcagaaggg

SEQ ID NO: 45869 - DNA, 28 bp, synthetic construct
  source 1..28: mol_type = other DNA
aaggcagggtcagaagggtcagagttgg

SEQ ID NO: 45870 - DNA, 28 bp, synthetic construct
  source 1..28: mol_type = other DNA
gcagggtcagaagggtcagagttggcgg

SEQ ID NO: 45871 - DNA, 28 bp, synthetic construct
  source 1..28: mol_type = other DNA
gtcagaagggtcagagttggcggtgagg

SEQ ID NO: 45872 - DNA, 28 bp, synthetic construct
  source 1..28: mol_type = other DNA
tcagaagggtcagagttggcggtgaggg

SEQ ID NO: 45873 - DNA, 28 bp, synthetic construct
  source 1..28: mol_type = other DNA
gaagggtcagagttggcggtgagggtgg

SEQ ID NO: 45874 - DNA, 28 bp, synthetic construct
  source 1..28: mol_type = other DNA
gcggtgagggtggctcagacactgatgg

SEQ ID NO: 45875 - DNA, 28 bp, synthetic construct
  source 1..28: mol_type = other DNA
cggtgagggtggctcagacactgatggg

SEQ ID NO: 45876 - DNA, 28 bp, synthetic construct
  source 1..28: mol_type = other DNA
gccctgcctctctcctcccctcccctgg

SEQ ID NO: 45877 - DNA, 28 bp, synthetic construct
  source 1..28: mol_type = other DNA
tccaggggaggggaggagagaggcaggg

SEQ ID NO: 45878 - DNA, 28 bp, synthetic construct
  source 1..28: mol_type = other DNA
ctccaggggaggggaggagagaggcagg

SEQ ID NO: 45879 - DNA, 28 bp, synthetic construct
  source 1..28: mol_type = other DNA
tctgctccaggggaggggaggagagagg

SEQ ID NO: 45880 - DNA, 28 bp, synthetic construct
  source 1..28: mol_type = other DNA
atgctgatctgctccaggggaggggagg

SEQ ID NO: 45881 - DNA, 28 bp, synthetic construct
  source 1..28: mol_type = other DNA
aagatgctgatctgctccaggggagggg

SEQ ID NO: 45882 - DNA, 28 bp, synthetic construct
  source 1..28: mol_type = other DNA
gaagatgctgatctgctccaggggaggg

SEQ ID NO: 45883 - DNA, 28 bp, synthetic construct
  source 1..28: mol_type = other DNA
tgaagatgctgatctgctccaggggagg

SEQ ID NO: 45884 - DNA, 28 bp, synthetic construct
  source 1..28: mol_type = other DNA
tcatgaagatgctgatctgctccagggg

SEQ ID NO: 45885 - DNA, 28 bp, synthetic construct
  source 1..28: mol_type = other DNA
gtcatgaagatgctgatctgctccaggg

SEQ ID NO: 45886 - DNA, 28 bp, synthetic construct
  source 1..28: mol_type = other DNA
cgtcatgaagatgctgatctgctccagg

SEQ ID NO: 45887 - DNA, 28 bp, synthetic construct
  source 1..28: mol_type = other DNA
tcttcatgacgcacctgtccaactatgg

SEQ ID NO: 45888 - DNA, 28 bp, synthetic construct
  source 1..28: mol_type = other DNA
cttcatgacgcacctgtccaactatggg

SEQ ID NO: 45889 - DNA, 28 bp, synthetic construct
  source 1..28: mol_type = other DNA
caggcggtcattcccatagttggacagg

SEQ ID NO: 45890 - DNA, 28 bp, synthetic construct
  source 1..28: mol_type = other DNA
ctgtccaactatgggaatgaccgcctgg

SEQ ID NO: 45891 - DNA, 28 bp, synthetic construct
  source 1..28: mol_type = other DNA
tgtccaactatgggaatgaccgcctggg

SEQ ID NO: 45892 - DNA, 28 bp, synthetic construct
  source 1..28: mol_type = other DNA
aggcccaggcggtcattcccatagttgg

SEQ ID NO: 45893 - DNA, 28 bp, synthetic construct
  source 1..28: mol_type = other DNA
gtgcttgaaggtgtacaggcccaggcgg

SEQ ID NO: 45894 - DNA, 28 bp, synthetic construct
  source 1..28: mol_type = other DNA
caggtgcttgaaggtgtacaggcccagg

SEQ ID NO: 45895 - DNA, 28 bp, synthetic construct
  source 1..28: mol_type = other DNA
ctgggcctgtacaccttcaagcacctgg

SEQ ID NO: 45896 - DNA, 28 bp, synthetic construct
  source 1..28: mol_type = other DNA
gcgcaccaggtgcttgaaggtgtacagg

SEQ ID NO: 45897 - DNA, 28 bp, synthetic construct
  source 1..28: mol_type = other DNA
tgcaggaagcgcaccaggtgcttgaagg

SEQ ID NO: 45898 - DNA, 28 bp, synthetic construct
  source 1..28: mol_type = other DNA
gcacctggtgcgcttcctgcactcctgg

SEQ ID NO: 45899 - DNA, 28 bp, synthetic construct
  source 1..28: mol_type = other DNA
cgtccaggagtgcaggaagcgcaccagg

SEQ ID NO: 45900 - DNA, 28 bp, synthetic construct
  source 1..28: mol_type = other DNA
cttcctgcactcctggacgaacctccgg

SEQ ID NO: 45901 - DNA, 28 bp, synthetic construct
  source 1..28: mol_type = other DNA
cagccggaggttcgtccaggagtgcagg

SEQ ID NO: 45902 - DNA, 28 bp, synthetic construct
  source 1..28: mol_type = other DNA
agtgtctgcagccggaggttcgtccagg

SEQ ID NO: 45903 - DNA, 28 bp, synthetic construct
  source 1..28: mol_type = other DNA
cacagggggcagtgtctgcagccggagg

SEQ ID NO: 45904 - DNA, 28 bp, synthetic construct
  source 1..28: mol_type = other DNA
ctgcacagggggcagtgtctgcagccgg

SEQ ID NO: 45905 - DNA, 28 bp, synthetic construct
  source 1..28: mol_type = other DNA
ctgcagacactgccccctgtgcagttgg

SEQ ID NO: 45906 - DNA, 28 bp, synthetic construct
  source 1..28: mol_type = other DNA
agtacttctgcgccaactgcacaggggg

SEQ ID NO: 45907 - DNA, 28 bp, synthetic construct
  source 1..28: mol_type = other DNA
aagtacttctgcgccaactgcacagggg

SEQ ID NO: 45908 - DNA, 28 bp, synthetic construct
  source 1..28: mol_type = other DNA
gaagtacttctgcgccaactgcacaggg

SEQ ID NO: 45909 - DNA, 28 bp, synthetic construct
  source 1..28: mol_type = other DNA
ggaagtacttctgcgccaactgcacagg

SEQ ID NO: 45910 - DNA, 28 bp, synthetic construct
  source 1..28: mol_type = other DNA
cagaagtacttccagatcttctccgagg

SEQ ID NO: 45911 - DNA, 28 bp, synthetic construct
  source 1..28: mol_type = other DNA
tacttccagatcttctccgaggagaagg

SEQ ID NO: 45912 - DNA, 28 bp, synthetic construct
  source 1..28: mol_type = other DNA
cgggtccttctcctcggagaagatctgg

SEQ ID NO: 45913 - DNA, 28 bp, synthetic construct
  source 1..28: mol_type = other DNA
cttctccgaggagaaggacccgctctgg

SEQ ID NO: 45914 - DNA, 28 bp, synthetic construct
  source 1..28: mol_type = other DNA
tccgaggagaaggacccgctctggcagg

SEQ ID NO: 45915 - DNA, 28 bp, synthetic construct
  source 1..28: mol_type = other DNA
acctgccagagcgggtccttctcctcgg

SEQ ID NO: 45916 - DNA, 28 bp, synthetic construct
  source 1..28: mol_type = other DNA
gaggagaaggacccgctctggcaggtgg

SEQ ID NO: 45917 - DNA, 28 bp, synthetic construct
  source 1..28: mol_type = other DNA
aggagaaggacccgctctggcaggtggg

SEQ ID NO: 45918 - DNA, 28 bp, synthetic construct
  source 1..28: mol_type = other DNA
ggagaaggacccgctctggcaggtgggg

SEQ ID NO: 45919 - DNA, 28 bp, synthetic construct
  source 1..28: mol_type = other DNA
gagaaggacccgctctggcaggtggggg

SEQ ID NO: 45920 - DNA, 28 bp, synthetic construct
  source 1..28: mol_type = other DNA
agaaggacccgctctggcaggtgggggg

SEQ ID NO: 45921 - DNA, 28 bp, synthetic construct
  source 1..28: mol_type = other DNA
ggacccgctctggcaggtggggggctgg

SEQ ID NO: 45922 - DNA, 28 bp, synthetic construct
  source 1..28: mol_type = other DNA
gacccgctctggcaggtggggggctggg

SEQ ID NO: 45923 - DNA, 28 bp, synthetic construct
  source 1..28: mol_type = other DNA
tgcccagccccccacctgccagagcggg

SEQ ID NO: 45924 - DNA, 28 bp, synthetic construct
  source 1..28: mol_type = other DNA
ctgcccagccccccacctgccagagcgg

SEQ ID NO: 45925 - DNA, 28 bp, synthetic construct
  source 1..28: mol_type = other DNA
ctggcaggtggggggctgggcagcctgg

SEQ ID NO: 45926 - DNA, 28 bp, synthetic construct
  source 1..28: mol_type = other DNA
tggcaggtggggggctgggcagcctggg

SEQ ID NO: 45927 - DNA, 28 bp, synthetic construct
  source 1..28: mol_type = other DNA
aggtggggggctgggcagcctgggcagg

SEQ ID NO: 45928 - DNA, 28 bp, synthetic construct
  source 1..28: mol_type = other DNA
ctgggcagcctgggcaggttgctacagg

SEQ ID NO: 45929 - DNA, 28 bp, synthetic construct
  source 1..28: mol_type = other DNA
tgggcagcctgggcaggttgctacaggg

SEQ ID NO: 45930 - DNA, 28 bp, synthetic construct
  source 1..28: mol_type = other DNA
cagcctgggcaggttgctacagggatgg

SEQ ID NO: 45931 - DNA, 28 bp, synthetic construct
  source 1..28: mol_type = other DNA
gttccatccctgtagcaacctgcccagg

SEQ ID NO: 45932 - DNA, 28 bp, synthetic construct
  source 1..28: mol_type = other DNA
acagggatggaacgccaccactcacagg

SEQ ID NO: 45933 - DNA, 28 bp, synthetic construct
  source 1..28: mol_type = other DNA
atctggagtgtgtgcctgtgagtggtgg

SEQ ID NO: 45934 - DNA, 28 bp, synthetic construct
  source 1..28: mol_type = other DNA
catatctggagtgtgtgcctgtgagtgg

SEQ ID NO: 45935 - DNA, 28 bp, synthetic construct
  source 1..28: mol_type = other DNA
cactcacaggcacacactccagatatgg

SEQ ID NO: 45936 - DNA, 28 bp, synthetic construct
  source 1..28: mol_type = other DNA
ggcacacactccagatatggactcaagg

SEQ ID NO: 45937 - DNA, 28 bp, synthetic construct
  source 1..28: mol_type = other DNA
gatggctgagccttgagtccatatctgg

SEQ ID NO: 45938 - DNA, 28 bp, synthetic construct
  source 1..28: mol_type = other DNA
ttcgagcgagagtgtgaaggcatgatgg

SEQ ID NO: 45939 - DNA, 28 bp, synthetic construct
  source 1..28: mol_type = other DNA
agtttacattcgagcgagagtgtgaagg

SEQ ID NO: 45940 - DNA, 28 bp, synthetic construct
  source 1..28: mol_type = other DNA
tgtagcatgtaggtatcatgcccattgg

SEQ ID NO: 45941 - DNA, 28 bp, synthetic construct
  source 1..28: mol_type = other DNA
gtagcatgtaggtatcatgcccattggg

SEQ ID NO: 45942 - DNA, 28 bp, synthetic construct
  source 1..28: mol_type = other DNA
taggtatcatgcccattgggctgtaagg

SEQ ID NO: 45943 - DNA, 28 bp, synthetic construct
  source 1..28: mol_type = other DNA
aggtatcatgcccattgggctgtaaggg

SEQ ID NO: 45944 - DNA, 28 bp, synthetic construct
  source 1..28: mol_type = other DNA
ggatatgtggcccttacagcccaatggg

SEQ ID NO: 45945 - DNA, 28 bp, synthetic construct
  source 1..28: mol_type = other DNA
tggatatgtggcccttacagcccaatgg

SEQ ID NO: 45946 - DNA, 28 bp, synthetic construct
  source 1..28: mol_type = other DNA
gtaagggccacatatccatgtgcagtgg

SEQ ID NO: 45947 - DNA, 28 bp, synthetic construct
  source 1..28: mol_type = other DNA
taagggccacatatccatgtgcagtggg

SEQ ID NO: 45948 - DNA, 28 bp, synthetic construct
  source 1..28: mol_type = other DNA
tggactcccactgcacatggatatgtgg

SEQ ID NO: 45949 - DNA, 28 bp, synthetic construct
  source 1..28: mol_type = other DNA
ccatgtgcagtgggagtccactgactgg

SEQ ID NO: 45950 - DNA, 28 bp, synthetic construct
  source 1..28: mol_type = other DNA
catgtgcagtgggagtccactgactggg

SEQ ID NO: 45951 - DNA, 28 bp, synthetic construct
  source 1..28: mol_type = other DNA
cagtgggagtccactgactgggttctgg

SEQ ID NO: 45952 - DNA, 28 bp, synthetic construct
  source 1..28: mol_type = other DNA
agtgggagtccactgactgggttctggg

SEQ ID NO: 45953 - DNA, 28 bp, synthetic construct
  source 1..28: mol_type = other DNA
gtgggagtccactgactgggttctgggg

SEQ ID NO: 45954 - DNA, 28 bp, synthetic construct
  source 1..28: mol_type = other DNA
gtggggcgccccagaacccagtcagtgg

SEQ ID NO: 45955 - DNA, 28 bp, synthetic construct
  source 1..28: mol_type = other DNA
aaaacaacagtggaagggatgtgtgggg

SEQ ID NO: 45956 - DNA, 28 bp, synthetic construct
  source 1..28: mol_type = other DNA
taaaacaacagtggaagggatgtgtggg

SEQ ID NO: 45957 - DNA, 28 bp, synthetic construct
  source 1..28: mol_type = other DNA
ctaaaacaacagtggaagggatgtgtgg

SEQ ID NO: 45958 - DNA, 28 bp, synthetic construct
  source 1..28: mol_type = other DNA
cacacatcccttccactgttgttttagg

SEQ ID NO: 45959 - DNA, 28 bp, synthetic construct
  source 1..28: mol_type = other DNA
caggggtcctaaaacaacagtggaaggg

SEQ ID NO: 45960 - DNA, 28 bp, synthetic construct
  source 1..28: mol_type = other DNA
gcaggggtcctaaaacaacagtggaagg

SEQ ID NO: 45961 - DNA, 28 bp, synthetic construct
  source 1..28: mol_type = other DNA
ccactgttgttttaggacccctgcgagg

SEQ ID NO: 45962 - DNA, 28 bp, synthetic construct
  source 1..28: mol_type = other DNA
gtctttgtgacgtttgtcctcgcagggg

SEQ ID NO: 45963 - DNA, 28 bp, synthetic construct
  source 1..28: mol_type = other DNA
tgtctttgtgacgtttgtcctcgcaggg

SEQ ID NO: 45964 - DNA, 28 bp, synthetic construct
  source 1..28: mol_type = other DNA
atgtctttgtgacgtttgtcctcgcagg

SEQ ID NO: 45965 - DNA, 28 bp, synthetic construct
  source 1..28: mol_type = other DNA
cgaggacaaacgtcacaaagacatctgg

SEQ ID NO: 45966 - DNA, 28 bp, synthetic construct
  source 1..28: mol_type = other DNA
aaacgtcacaaagacatctggtccaagg

SEQ ID NO: 45967 - DNA, 28 bp, synthetic construct
  source 1..28: mol_type = other DNA
gggaagcggtcacacgtcttctccttgg

SEQ ID NO: 45968 - DNA, 28 bp, synthetic construct
  source 1..28: mol_type = other DNA
accgcttcccaaagctcctcatcatcgg

SEQ ID NO: 45969 - DNA, 28 bp, synthetic construct
  source 1..28: mol_type = other DNA
gccgatgatgaggagctttgggaagcgg

SEQ ID NO: 45970 - DNA, 28 bp, synthetic construct
  source 1..28: mol_type = other DNA
ctgggggccgatgatgaggagctttggg

SEQ ID NO: 45971 - DNA, 28 bp, synthetic construct
  source 1..28: mol_type = other DNA
tctgggggccgatgatgaggagctttgg

SEQ ID NO: 45972 - DNA, 28 bp, synthetic construct
  source 1..28: mol_type = other DNA
tcctcatcatcggcccccagaaaacagg

SEQ ID NO: 45973 - DNA, 28 bp, synthetic construct
  source 1..28: mol_type = other DNA
gcctgttttctgggggccgatgatgagg

SEQ ID NO: 45974 - DNA, 28 bp, synthetic construct
  source 1..28: mol_type = other DNA
catcatcggcccccagaaaacaggcagg

SEQ ID NO: 45975 - DNA, 28 bp, synthetic construct
  source 1..28: mol_type = other DNA
gcagagagacctgcctgttttctggggg

SEQ ID NO: 45976 - DNA, 28 bp, synthetic construct
  source 1..28: mol_type = other DNA
agcagagagacctgcctgttttctgggg

SEQ ID NO: 45977 - DNA, 28 bp, synthetic construct
  source 1..28: mol_type = other DNA
gagcagagagacctgcctgttttctggg

SEQ ID NO: 45978 - DNA, 28 bp, synthetic construct
  source 1..28: mol_type = other DNA
agagcagagagacctgcctgttttctgg

SEQ ID NO: 45979 - DNA, 28 bp, synthetic construct
  source 1..28: mol_type = other DNA
gagacagcaggcagttggggaagctcgg

SEQ ID NO: 45980 - DNA, 28 bp, synthetic construct
  source 1..28: mol_type = other DNA
ctgtggctgagacagcaggcagttgggg

SEQ ID NO: 45981 - DNA, 28 bp, synthetic construct
  source 1..28: mol_type = other DNA
tctgtggctgagacagcaggcagttggg

SEQ ID NO: 45982 - DNA, 28 bp, synthetic construct
  source 1..28: mol_type = other DNA
ttctgtggctgagacagcaggcagttgg

SEQ ID NO: 45983 - DNA, 28 bp, synthetic construct
  source 1..28: mol_type = other DNA
ctcagaattctgtggctgagacagcagg

SEQ ID NO: 45984 - DNA, 28 bp, synthetic construct
  source 1..28: mol_type = other DNA
ctgctgtctcagccacagaattctgagg

SEQ ID NO: 45985 - DNA, 28 bp, synthetic construct
  source 1..28: mol_type = other DNA
gggcaaggcagtcctcagaattctgtgg

SEQ ID NO: 45986 - DNA, 28 bp, synthetic construct
  source 1..28: mol_type = other DNA
cagaattctgaggactgccttgccctgg

SEQ ID NO: 45987 - DNA, 28 bp, synthetic construct
  source 1..28: mol_type = other DNA
gactgccttgccctggccccactcccgg

SEQ ID NO: 45988 - DNA, 28 bp, synthetic construct
  source 1..28: mol_type = other DNA
attatccgggagtggggccagggcaagg

SEQ ID NO: 45989 - DNA, 28 bp, synthetic construct
  source 1..28: mol_type = other DNA
agcaaattatccgggagtggggccaggg

SEQ ID NO: 45990 - DNA, 28 bp, synthetic construct
  source 1..28: mol_type = other DNA
gagcaaattatccgggagtggggccagg

SEQ ID NO: 45991 - DNA, 28 bp, synthetic construct
  source 1..28: mol_type = other DNA
agagggagcaaattatccgggagtgggg

SEQ ID NO: 45992 - DNA, 28 bp, synthetic construct
  source 1..28: mol_type = other DNA
aagagggagcaaattatccgggagtggg

SEQ ID NO: 45993 - DNA, 28 bp, synthetic construct
  source 1..28: mol_type = other DNA
aaagagggagcaaattatccgggagtgg

SEQ ID NO: 45994 - DNA, 28 bp, synthetic construct
  source 1..28: mol_type = other DNA
ctgggaaagagggagcaaattatccggg

SEQ ID NO: 45995 - DNA, 28 bp, synthetic construct
  source 1..28: mol_type = other DNA
cctgggaaagagggagcaaattatccgg

SEQ ID NO: 45996 - DNA, 28 bp, synthetic construct
  source 1..28: mol_type = other DNA
atttgctccctctttcccaggaagtagg

SEQ ID NO: 45997 - DNA, 28 bp, synthetic construct
  source 1..28: mol_type = other DNA
accagagaaaggcagagaccttcccagg

SEQ ID NO: 45998 - DNA, 28 bp, synthetic construct
  source 1..28: mol_type = other DNA
tcctgggaaggtctctgcctttctctgg

SEQ ID NO: 45999 - DNA, 28 bp, synthetic construct
  source 1..28: mol_type = other DNA
cagagaccttcccaggagcccccagtgg

SEQ ID NO: 46000 - DNA, 28 bp, synthetic construct
  source 1..28: mol_type = other DNA
agagaccttcccaggagcccccagtggg

SEQ ID NO: 46001 - DNA, 28 bp, synthetic construct
  source 1..28: mol_type = other DNA
cacgacccactgggggctcctgggaagg

SEQ ID NO: 46002 - DNA, 28 bp, synthetic construct
  source 1..28: mol_type = other DNA
cttcccaggagcccccagtgggtcgtgg

SEQ ID NO: 46003 - DNA, 28 bp, synthetic construct
  source 1..28: mol_type = other DNA
ttcccaggagcccccagtgggtcgtggg

SEQ ID NO: 46004 - DNA, 28 bp, synthetic construct
  source 1..28: mol_type = other DNA
tcccaggagcccccagtgggtcgtgggg

SEQ ID NO: 46005 - DNA, 28 bp, synthetic construct
  source 1..28: mol_type = other DNA
tccccacgacccactgggggctcctggg

SEQ ID NO: 46006 - DNA, 28 bp, synthetic construct
  source 1..28: mol_type = other DNA
ctccccacgacccactgggggctcctgg

SEQ ID NO: 46007 - DNA, 28 bp, synthetic construct
  source 1..28: mol_type = other DNA
agcccccagtgggtcgtggggagctagg

SEQ ID NO: 46008 - DNA, 28 bp, synthetic construct
  source 1..28: mol_type = other DNA
ggcctagctccccacgacccactggggg

SEQ ID NO: 46009 - DNA, 28 bp, synthetic construct
  source 1..28: mol_type = other DNA
gggcctagctccccacgacccactgggg

SEQ ID NO: 46010 - DNA, 28 bp, synthetic construct
  source 1..28: mol_type = other DNA
tgggcctagctccccacgacccactggg

SEQ ID NO: 46011 - DNA, 28 bp, synthetic construct
  source 1..28: mol_type = other DNA
ctgggcctagctccccacgacccactgg

SEQ ID NO: 46012 - DNA, 28 bp, synthetic construct
  source 1..28: mol_type = other DNA
ggcccagaacccagactctatcttttgg

SEQ ID NO: 46013 - DNA, 28 bp, synthetic construct
  source 1..28: mol_type = other DNA
agccaaaagatagagtctgggttctggg

SEQ ID NO: 46014 - DNA, 28 bp, synthetic construct
  source 1..28: mol_type = other DNA
cagccaaaagatagagtctgggttctgg

SEQ ID NO: 46015 - DNA, 28 bp, synthetic construct
  source 1..28: mol_type = other DNA
cagaacccagactctatcttttggctgg

SEQ ID NO: 46016 - DNA, 28 bp, synthetic construct
  source 1..28: mol_type = other DNA
agaacccagactctatcttttggctggg

SEQ ID NO: 46017 - DNA, 28 bp, synthetic construct
  source 1..28: mol_type = other DNA
gaacccagactctatcttttggctgggg

SEQ ID NO: 46018 - DNA, 28 bp, synthetic construct
  source 1..28: mol_type = other DNA
aacccagactctatcttttggctggggg

SEQ ID NO: 46019 - DNA, 28 bp, synthetic construct
  source 1..28: mol_type = other DNA
agcccccagccaaaagatagagtctggg

SEQ ID NO: 46020 - DNA, 28 bp, synthetic construct
  source 1..28: mol_type = other DNA
cagcccccagccaaaagatagagtctgg

SEQ ID NO: 46021 - DNA, 28 bp, synthetic construct
  source 1..28: mol_type = other DNA
cagactctatcttttggctgggggctgg

SEQ ID NO: 46022 - DNA, 28 bp, synthetic construct
  source 1..28: mol_type = other DNA
agactctatcttttggctgggggctggg

SEQ ID NO: 46023 - DNA, 28 bp, synthetic construct
  source 1..28: mol_type = other DNA
tatcttttggctgggggctgggccctgg

SEQ ID NO: 46024 - DNA, 28 bp, synthetic construct
  source 1..28: mol_type = other DNA
atcttttggctgggggctgggccctggg

SEQ ID NO: 46025 - DNA, 28 bp, synthetic construct
  source 1..28: mol_type = other DNA
ggctgggggctgggccctgggtctcagg

SEQ ID NO: 46026 - DNA, 28 bp, synthetic construct
  source 1..28: mol_type = other DNA
ggggagggtagacacctgagacccaggg

SEQ ID NO: 46027 - DNA, 28 bp, synthetic construct
  source 1..28: mol_type = other DNA
tggggagggtagacacctgagacccagg

SEQ ID NO: 46028 - DNA, 28 bp, synthetic construct
  source 1..28: mol_type = other DNA
ggtctcaggtgtctaccctccccacagg

SEQ ID NO: 46029 - DNA, 28 bp, synthetic construct
  source 1..28: mol_type = other DNA
tagagggcagtggtgcctgtggggaggg

SEQ ID NO: 46030 - DNA, 28 bp, synthetic construct
  source 1..28: mol_type = other DNA
gtagagggcagtggtgcctgtggggagg

SEQ ID NO: 46031 - DNA, 28 bp, synthetic construct
  source 1..28: mol_type = other DNA
caggtagagggcagtggtgcctgtgggg

SEQ ID NO: 46032 - DNA, 28 bp, synthetic construct
  source 1..28: mol_type = other DNA
acaggtagagggcagtggtgcctgtggg

SEQ ID NO: 46033 - DNA, 28 bp, synthetic construct
  source 1..28: mol_type = other DNA
aacaggtagagggcagtggtgcctgtgg

SEQ ID NO: 46034 - DNA, 28 bp, synthetic construct
  source 1..28: mol_type = other DNA
ggcaccactgccctctacctgttcctgg

SEQ ID NO: 46035 - DNA, 28 bp, synthetic construct
  source 1..28: mol_type = other DNA
gcaccactgccctctacctgttcctggg

SEQ ID NO: 46036 - DNA, 28 bp, synthetic construct
  source 1..28: mol_type = other DNA
atgcccaggaacaggtagagggcagtgg

SEQ ID NO: 46037 - DNA, 28 bp, synthetic construct
  source 1..28: mol_type = other DNA
gggtgcatgcccaggaacaggtagaggg

SEQ ID NO: 46038 - DNA, 28 bp, synthetic construct
  source 1..28: mol_type = other DNA
agggtgcatgcccaggaacaggtagagg

SEQ ID NO: 46039 - DNA, 28 bp, synthetic construct
  source 1..28: mol_type = other DNA
taggtcagggtgcatgcccaggaacagg

SEQ ID NO: 46040 - DNA, 28 bp, synthetic construct
  source 1..28: mol_type = other DNA
gctgcttaggtcagggtgcatgcccagg

SEQ ID NO: 46041 - DNA, 28 bp, synthetic construct
  source 1..28: mol_type = other DNA
gctggggtagttgctgcttaggtcaggg

SEQ ID NO: 46042 - DNA, 28 bp, synthetic construct
  source 1..28: mol_type = other DNA
agctggggtagttgctgcttaggtcagg

SEQ ID NO: 46043 - DNA, 28 bp, synthetic construct
  source 1..28: mol_type = other DNA
ctcagagctggggtagttgctgcttagg

SEQ ID NO: 46044 - DNA, 28 bp, synthetic construct
  source 1..28: mol_type = other DNA
aactaccccagctctgagacctttgagg

SEQ ID NO: 46045 - DNA, 28 bp, synthetic construct
  source 1..28: mol_type = other DNA
gatctcctcaaaggtctcagagctgggg

SEQ ID NO: 46046 - DNA, 28 bp, synthetic construct
  source 1..28: mol_type = other DNA
ggatctcctcaaaggtctcagagctggg

SEQ ID NO: 46047 - DNA, 28 bp, synthetic construct
  source 1..28: mol_type = other DNA
tggatctcctcaaaggtctcagagctgg

SEQ ID NO: 46048 - DNA, 28 bp, synthetic construct
  source 1..28: mol_type = other DNA
cctttgaggagatccagttttttaatgg

SEQ ID NO: 46049 - DNA, 28 bp, synthetic construct
  source 1..28: mol_type = other DNA
gtgatagttgtggccattaaaaaactgg

SEQ ID NO: 46050 - DNA, 28 bp, synthetic construct
  source 1..28: mol_type = other DNA
tttttaatggccacaactatcacaaagg

SEQ ID NO: 46051 - DNA, 28 bp, synthetic construct
  source 1..28: mol_type = other DNA
ccagtcgatgcctttgtgatagttgtgg

SEQ ID NO: 46052 - DNA, 28 bp, synthetic construct
  source 1..28: mol_type = other DNA
atcacaaaggcatcgactggtgagttgg

SEQ ID NO: 46053 - DNA, 28 bp, synthetic construct
  source 1..28: mol_type = other DNA
ggtgagttggcctttctgtccacagcgg

SEQ ID NO: 46054 - DNA, 28 bp, synthetic construct
  source 1..28: mol_type = other DNA
gtgagttggcctttctgtccacagcggg

SEQ ID NO: 46055 - DNA, 28 bp, synthetic construct
  source 1..28: mol_type = other DNA
gttggcctttctgtccacagcgggacgg

SEQ ID NO: 46056 - DNA, 28 bp, synthetic construct
  source 1..28: mol_type = other DNA
ttggcctttctgtccacagcgggacggg

SEQ ID NO: 46057 - DNA, 28 bp, synthetic construct
  source 1..28: mol_type = other DNA
ccttcccgtcccgctgtggacagaaagg

SEQ ID NO: 46058 - DNA, 28 bp, synthetic construct
  source 1..28: mol_type = other DNA
ccaggatggccttcccgtcccgctgtgg

SEQ ID NO: 46059 - DNA, 28 bp, synthetic construct
  source 1..28: mol_type = other DNA
cacagcgggacgggaaggccatcctggg

SEQ ID NO: 46060 - DNA, 28 bp, synthetic construct
  source 1..28: mol_type = other DNA
acagcgggacgggaaggccatcctgggg

SEQ ID NO: 46061 - DNA, 28 bp, synthetic construct
  source 1..28: mol_type = other DNA
cgggaaggccatcctggggcctcccagg

SEQ ID NO: 46062 - DNA, 28 bp, synthetic construct
  source 1..28: mol_type = other DNA
agcagactcctgggaggccccaggatgg

SEQ ID NO: 46063 - DNA, 28 bp, synthetic construct
  source 1..28: mol_type = other DNA
cctggggcctcccaggagtctgctgtgg

SEQ ID NO: 46064 - DNA, 28 bp, synthetic construct
  source 1..28: mol_type = other DNA
gctgtggccacagcagactcctgggagg

SEQ ID NO: 46065 - DNA, 28 bp, synthetic construct
  source 1..28: mol_type = other DNA
cctgctgtggccacagcagactcctggg

SEQ ID NO: 46066 - DNA, 28 bp, synthetic construct
  source 1..28: mol_type = other DNA
tcctgctgtggccacagcagactcctgg

SEQ ID NO: 46067 - DNA, 28 bp, synthetic construct
  source 1..28: mol_type = other DNA
tgctgtggccacagcaggaagcagctgg

SEQ ID NO: 46068 - DNA, 28 bp, synthetic construct
  source 1..28: mol_type = other DNA
agcaagctccagctgcttcctgctgtgg

SEQ ID NO: 46069 - DNA, 28 bp, synthetic construct
  source 1..28: mol_type = other DNA
acacacagctgtcattcctgtaaacagg

SEQ ID NO: 46070 - DNA, 28 bp, synthetic construct
  source 1..28: mol_type = other DNA
cacacagctgtcattcctgtaaacaggg

SEQ ID NO: 46071 - DNA, 28 bp, synthetic construct
  source 1..28: mol_type = other DNA
agcaaagcttcccacttgctctctgagg

SEQ ID NO: 46072 - DNA, 28 bp, synthetic construct
  source 1..28: mol_type = other DNA
ggtagaatgtcctcagagagcaagtggg

SEQ ID NO: 46073 - DNA, 28 bp, synthetic construct
  source 1..28: mol_type = other DNA
gggtagaatgtcctcagagagcaagtgg

SEQ ID NO: 46074 - DNA, 28 bp, synthetic construct
  source 1..28: mol_type = other DNA
aatgcagcacaagggcgaggcactgggg

SEQ ID NO: 46075 - DNA, 28 bp, synthetic construct
  source 1..28: mol_type = other DNA
gaatgcagcacaagggcgaggcactggg

SEQ ID NO: 46076 - DNA, 28 bp, synthetic construct
  source 1..28: mol_type = other DNA
ggaatgcagcacaagggcgaggcactgg

SEQ ID NO: 46077 - DNA, 28 bp, synthetic construct
  source 1..28: mol_type = other DNA
gctaagggaatgcagcacaagggcgagg

SEQ ID NO: 46078 - DNA, 28 bp, synthetic construct
  source 1..28: mol_type = other DNA
agggggctaagggaatgcagcacaaggg

SEQ ID NO: 46079 - DNA, 28 bp, synthetic construct
  source 1..28: mol_type = other DNA
gagggggctaagggaatgcagcacaagg

SEQ ID NO: 46080 - DNA, 28 bp, synthetic construct
  source 1..28: mol_type = other DNA
acaaaactcatgaggagggggctaaggg

SEQ ID NO: 46081 - DNA, 28 bp, synthetic construct
  source 1..28: mol_type = other DNA
gacaaaactcatgaggagggggctaagg

SEQ ID NO: 46082 - DNA, 28 bp, synthetic construct
  source 1..28: mol_type = other DNA
ctcacagacaaaactcatgaggaggggg

SEQ ID NO: 46083 - DNA, 28 bp, synthetic construct
  source 1..28: mol_type = other DNA
gctcacagacaaaactcatgaggagggg

SEQ ID NO: 46084 - DNA, 28 bp, synthetic construct
  source 1..28: mol_type = other DNA
ggctcacagacaaaactcatgaggaggg

SEQ ID NO: 46085 - DNA, 28 bp, synthetic construct
  source 1..28: mol_type = other DNA
cggctcacagacaaaactcatgaggagg

SEQ ID NO: 46086 - DNA, 28 bp, synthetic construct
  source 1..28: mol_type = other DNA
aggcggctcacagacaaaactcatgagg

SEQ ID NO: 46087 - DNA, 28 bp, synthetic construct
  source 1..28: mol_type = other DNA
gagttttgtctgtgagccgcctctctgg

SEQ ID NO: 46088 - DNA, 28 bp, synthetic construct
  source 1..28: mol_type = other DNA
agttttgtctgtgagccgcctctctggg

SEQ ID NO: 46089 - DNA, 28 bp, synthetic construct
  source 1..28: mol_type = other DNA
tgagccgcctctctgggcttcctgcagg

SEQ ID NO: 46090 - DNA, 28 bp, synthetic construct
  source 1..28: mol_type = other DNA
tgtacctgcaggaagcccagagaggcgg

SEQ ID NO: 46091 - DNA, 28 bp, synthetic construct
  source 1..28: mol_type = other DNA
ccatgtacctgcaggaagcccagagagg

SEQ ID NO: 46092 - DNA, 28 bp, synthetic construct
  source 1..28: mol_type = other DNA
atggggaagaactccatgtacctgcagg

SEQ ID NO: 46093 - DNA, 28 bp, synthetic construct
  source 1..28: mol_type = other DNA
gtcggaggtggtgttggaagggatgggg

SEQ ID NO: 46094 - DNA, 28 bp, synthetic construct
  source 1..28: mol_type = other DNA
agtcggaggtggtgttggaagggatggg

SEQ ID NO: 46095 - DNA, 28 bp, synthetic construct
  source 1..28: mol_type = other DNA
aagtcggaggtggtgttggaagggatgg

SEQ ID NO: 46096 - DNA, 28 bp, synthetic construct
  source 1..28: mol_type = other DNA
gtagaagtcggaggtggtgttggaaggg

SEQ ID NO: 46097 - DNA, 28 bp, synthetic construct
  source 1..28: mol_type = other DNA
agtagaagtcggaggtggtgttggaagg

SEQ ID NO: 46098 - DNA, 28 bp, synthetic construct
  source 1..28: mol_type = other DNA
tcaaagtagaagtcggaggtggtgttgg

SEQ ID NO: 46099 - DNA, 28 bp, synthetic construct
  source 1..28: mol_type = other DNA
cttttctcaaagtagaagtcggaggtgg

SEQ ID NO: 46100 - DNA, 28 bp, synthetic construct
  source 1..28: mol_type = other DNA
gcgcttttctcaaagtagaagtcggagg

SEQ ID NO: 46101 - DNA, 28 bp, synthetic construct
  source 1..28: mol_type = other DNA
ttggcgcttttctcaaagtagaagtcgg

SEQ ID NO: 46102 - DNA, 28 bp, synthetic construct
  source 1..28: mol_type = other DNA
agcgccaactactttgattcagaagtgg

SEQ ID NO: 46103 - DNA, 28 bp, synthetic construct
  source 1..28: mol_type = other DNA
ggcgccacttctgaatcaaagtagttgg

SEQ ID NO: 46104 - DNA, 28 bp, synthetic construct
  source 1..28: mol_type = other DNA
ctactttgattcagaagtggcgccccgg

SEQ ID NO: 46105 - DNA, 28 bp, synthetic construct
  source 1..28: mol_type = other DNA
ctttgattcagaagtggcgccccggcgg

SEQ ID NO: 46106 - DNA, 28 bp, synthetic construct
  source 1..28: mol_type = other DNA
tttgattcagaagtggcgccccggcggg

SEQ ID NO: 46107 - DNA, 28 bp, synthetic construct
  source 1..28: mol_type = other DNA
tgggcaagagggctgctgcccgccgggg

SEQ ID NO: 46108 - DNA, 28 bp, synthetic construct
  source 1..28: mol_type = other DNA
ttgggcaagagggctgctgcccgccggg

SEQ ID NO: 46109 - DNA, 28 bp, synthetic construct
  source 1..28: mol_type = other DNA
tttgggcaagagggctgctgcccgccgg

SEQ ID NO: 46110 - DNA, 28 bp, synthetic construct
  source 1..28: mol_type = other DNA
gcagcagccctcttgcccaaagccaagg

SEQ ID NO: 46111 - DNA, 28 bp, synthetic construct
  source 1..28: mol_type = other DNA
gtcaggaccttggctttgggcaagaggg

SEQ ID NO: 46112 - DNA, 28 bp, synthetic construct
  source 1..28: mol_type = other DNA
ggtcaggaccttggctttgggcaagagg

SEQ ID NO: 46113 - DNA, 28 bp, synthetic construct
  source 1..28: mol_type = other DNA
tgaggatggtcaggaccttggctttggg

SEQ ID NO: 46114 - DNA, 28 bp, synthetic construct
  source 1..28: mol_type = other DNA
atgaggatggtcaggaccttggctttgg

SEQ ID NO: 46115 - DNA, 28 bp, synthetic construct
  source 1..28: mol_type = other DNA
gggttgatgaggatggtcaggaccttgg

SEQ ID NO: 46116 - DNA, 28 bp, synthetic construct
  source 1..28: mol_type = other DNA
gtcctgaccatcctcatcaaccccgcgg

SEQ ID NO: 46117 - DNA, 28 bp, synthetic construct
  source 1..28: mol_type = other DNA
gtccgcggggttgatgaggatggtcagg

SEQ ID NO: 46118 - DNA, 28 bp, synthetic construct
  source 1..28: mol_type = other DNA
gaccatcctcatcaaccccgcggaccgg

SEQ ID NO: 46119 - DNA, 28 bp, synthetic construct
  source 1..28: mol_type = other DNA
accatcctcatcaaccccgcggaccggg

SEQ ID NO: 46120 - DNA, 28 bp, synthetic construct
  source 1..28: mol_type = other DNA
gcccggtccgcggggttgatgaggatgg

SEQ ID NO: 46121 - DNA, 28 bp, synthetic construct
  source 1..28: mol_type = other DNA
ataggcccggtccgcggggttgatgagg

SEQ ID NO: 46122 - DNA, 28 bp, synthetic construct
  source 1..28: mol_type = other DNA
caaccccgcggaccgggcctattcctgg

SEQ ID NO: 46123 - DNA, 28 bp, synthetic construct
  source 1..28: mol_type = other DNA
gtaccaggaataggcccggtccgcgggg

SEQ ID NO: 46124 - DNA, 28 bp, synthetic construct
  source 1..28: mol_type = other DNA
ggtaccaggaataggcccggtccgcggg

SEQ ID NO: 46125 - DNA, 28 bp, synthetic construct
  source 1..28: mol_type = other DNA
tggtaccaggaataggcccggtccgcgg

SEQ ID NO: 46126 - DNA, 28 bp, synthetic construct
  source 1..28: mol_type = other DNA
gcggaccgggcctattcctggtaccagg

SEQ ID NO: 46127 - DNA, 28 bp, synthetic construct
  source 1..28: mol_type = other DNA
actcacctggtaccaggaataggcccgg

SEQ ID NO: 46128 - DNA, 28 bp, synthetic construct
  source 1..28: mol_type = other DNA
gggcctattcctggtaccaggtgagtgg

SEQ ID NO: 46129 - DNA, 28 bp, synthetic construct
  source 1..28: mol_type = other DNA
ggcctattcctggtaccaggtgagtggg

SEQ ID NO: 46130 - DNA, 28 bp, synthetic construct
  source 1..28: mol_type = other DNA
gcctattcctggtaccaggtgagtgggg

SEQ ID NO: 46131 - DNA, 28 bp, synthetic construct
  source 1..28: mol_type = other DNA
gccccactcacctggtaccaggaatagg

SEQ ID NO: 46132 - DNA, 28 bp, synthetic construct
  source 1..28: mol_type = other DNA
attcctggtaccaggtgagtggggctgg

SEQ ID NO: 46133 - DNA, 28 bp, synthetic construct
  source 1..28: mol_type = other DNA
ttcctggtaccaggtgagtggggctggg

SEQ ID NO: 46134 - DNA, 28 bp, synthetic construct
  source 1..28: mol_type = other DNA
tcctggtaccaggtgagtggggctgggg

SEQ ID NO: 46135 - DNA, 28 bp, synthetic construct
  source 1..28: mol_type = other DNA
accccagccccactcacctggtaccagg

SEQ ID NO: 46136 - DNA, 28 bp, synthetic construct
  source 1..28: mol_type = other DNA
tggtaccaggtgagtggggctggggtgg

SEQ ID NO: 46137 - DNA, 28 bp, synthetic construct
  source 1..28: mol_type = other DNA
ggactccaccccagccccactcacctgg

SEQ ID NO: 46138 - DNA, 28 bp, synthetic construct
  source 1..28: mol_type = other DNA
tggggctggggtggagtccctgtgtcgg

SEQ ID NO: 46139 - DNA, 28 bp, synthetic construct
  source 1..28: mol_type = other DNA
ggggctggggtggagtccctgtgtcggg

SEQ ID NO: 46140 - DNA, 28 bp, synthetic construct
  source 1..28: mol_type = other DNA
ggtggagtccctgtgtcgggaacacagg

SEQ ID NO: 46141 - DNA, 28 bp, synthetic construct
  source 1..28: mol_type = other DNA
gtggagtccctgtgtcgggaacacaggg

SEQ ID NO: 46142 - DNA, 28 bp, synthetic construct
  source 1..28: mol_type = other DNA
gacggagccctgtgttcccgacacaggg

SEQ ID NO: 46143 - DNA, 28 bp, synthetic construct
  source 1..28: mol_type = other DNA
agacggagccctgtgttcccgacacagg

SEQ ID NO: 46144 - DNA, 28 bp, synthetic construct
  source 1..28: mol_type = other DNA
agtgagtgagtaactgagtgtcagacgg

SEQ ID NO: 46145 - DNA, 28 bp, synthetic construct
  source 1..28: mol_type = other DNA
acctactgtgtgccagccctgagccagg

SEQ ID NO: 46146 - DNA, 28 bp, synthetic construct
  source 1..28: mol_type = other DNA
gcctggctcagggctggcacacagtagg

SEQ ID NO: 46147 - DNA, 28 bp, synthetic construct
  source 1..28: mol_type = other DNA
gacccagagctcctgggtccagctgagg

SEQ ID NO: 46148 - DNA, 28 bp, synthetic construct
  source 1..28: mol_type = other DNA
atcctcagctggacccaggagctctggg

SEQ ID NO: 46149 - DNA, 28 bp, synthetic construct
  source 1..28: mol_type = other DNA
gatcctcagctggacccaggagctctgg

SEQ ID NO: 46150 - DNA, 28 bp, synthetic construct
  source 1..28: mol_type = other DNA
ctcctgggtccagctgaggatcttctgg

SEQ ID NO: 46151 - DNA, 28 bp, synthetic construct
  source 1..28: mol_type = other DNA
ggccagaagatcctcagctggacccagg

SEQ ID NO: 46152 - DNA, 28 bp, synthetic construct
  source 1..28: mol_type = other DNA
gcaaggtggccagaagatcctcagctgg

SEQ ID NO: 46153 - DNA, 28 bp, synthetic construct
  source 1..28: mol_type = other DNA
agctgaggatcttctggccaccttgcgg

SEQ ID NO: 46154 - DNA, 28 bp, synthetic construct
  source 1..28: mol_type = other DNA
gctgaggatcttctggccaccttgcggg

SEQ ID NO: 46155 - DNA, 28 bp, synthetic construct
  source 1..28: mol_type = other DNA
ctgagagggacagcagcccgcaaggtgg

SEQ ID NO: 46156 - DNA, 28 bp, synthetic construct
  source 1..28: mol_type = other DNA
caccttgcgggctgctgtccctctcagg

SEQ ID NO: 46157 - DNA, 28 bp, synthetic construct
  source 1..28: mol_type = other DNA
ggcctgagagggacagcagcccgcaagg

SEQ ID NO: 46158 - DNA, 28 bp, synthetic construct
  source 1..28: mol_type = other DNA
aggacacaaaggaagtggcctgagaggg

SEQ ID NO: 46159 - DNA, 28 bp, synthetic construct
  source 1..28: mol_type = other DNA
gaggacacaaaggaagtggcctgagagg

SEQ ID NO: 46160 - DNA, 28 bp, synthetic construct
  source 1..28: mol_type = other DNA
ggccacttcctttgtgtcctccaagtgg

SEQ ID NO: 46161 - DNA, 28 bp, synthetic construct
  source 1..28: mol_type = other DNA
tgccacttggaggacacaaaggaagtgg

SEQ ID NO: 46162 - DNA, 28 bp, synthetic construct
  source 1..28: mol_type = other DNA
tcagcatgccacttggaggacacaaagg

SEQ ID NO: 46163 - DNA, 28 bp, synthetic construct
  source 1..28: mol_type = other DNA
gaaagagggtcagcatgccacttggagg

SEQ ID NO: 46164 - DNA, 28 bp, synthetic construct
  source 1..28: mol_type = other DNA
aaggaaagagggtcagcatgccacttgg

SEQ ID NO: 46165 - DNA, 28 bp, synthetic construct
  source 1..28: mol_type = other DNA
cgctggtgctgcaggcaaggaaagaggg

SEQ ID NO: 46166 - DNA, 28 bp, synthetic construct
  source 1..28: mol_type = other DNA
tcgctggtgctgcaggcaaggaaagagg

SEQ ID NO: 46167 - DNA, 28 bp, synthetic construct
  source 1..28: mol_type = other DNA
catgggctcgctggtgctgcaggcaagg

SEQ ID NO: 46168 - DNA, 28 bp, synthetic construct
  source 1..28: mol_type = other DNA
gtcgtcatgggctcgctggtgctgcagg

SEQ ID NO: 46169 - DNA, 28 bp, synthetic construct
  source 1..28: mol_type = other DNA
caccagcgagcccatgacgacccagtgg

SEQ ID NO: 46170 - DNA, 28 bp, synthetic construct
  source 1..28: mol_type = other DNA
ggccactgggtcgtcatgggctcgctgg

SEQ ID NO: 46171 - DNA, 28 bp, synthetic construct
  source 1..28: mol_type = other DNA
tactttagggccactgggtcgtcatggg

SEQ ID NO: 46172 - DNA, 28 bp, synthetic construct
  source 1..28: mol_type = other DNA
gtactttagggccactgggtcgtcatgg

SEQ ID NO: 46173 - DNA, 28 bp, synthetic construct
  source 1..28: mol_type = other DNA
atggaaggtgtactttagggccactggg

SEQ ID NO: 46174 - DNA, 28 bp, synthetic construct
  source 1..28: mol_type = other DNA
catggaaggtgtactttagggccactgg

SEQ ID NO: 46175 - DNA, 28 bp, synthetic construct
  source 1..28: mol_type = other DNA
gtggccctaaagtacaccttccatgagg

SEQ ID NO: 46176 - DNA, 28 bp, synthetic construct
  source 1..28: mol_type = other DNA
atcacctcatggaaggtgtactttaggg

SEQ ID NO: 46177 - DNA, 28 bp, synthetic construct
  source 1..28: mol_type = other DNA
aatcacctcatggaaggtgtactttagg

SEQ ID NO: 46178 - DNA, 28 bp, synthetic construct
  source 1..28: mol_type = other DNA
acaccttccatgaggtgattaccgccgg

SEQ ID NO: 46179 - DNA, 28 bp, synthetic construct
  source 1..28: mol_type = other DNA
gagccggcggtaatcacctcatggaagg

SEQ ID NO: 46180 - DNA, 28 bp, synthetic construct
  source 1..28: mol_type = other DNA
gtcagagccggcggtaatcacctcatgg

SEQ ID NO: 46181 - DNA, 28 bp, synthetic construct
  source 1..28: mol_type = other DNA
agcttcgaggatgcgtcagagccggcgg

SEQ ID NO: 46182 - DNA, 28 bp, synthetic construct
  source 1..28: mol_type = other DNA
cgcagcttcgaggatgcgtcagagccgg

SEQ ID NO: 46183 - DNA, 28 bp, synthetic construct
  source 1..28: mol_type = other DNA
cggttctggagggcacgcagcttcgagg

SEQ ID NO: 46184 - DNA, 28 bp, synthetic construct
  source 1..28: mol_type = other DNA
ctgcgtgccctccagaaccgctgcctgg

SEQ ID NO: 46185 - DNA, 28 bp, synthetic construct
  source 1..28: mol_type = other DNA
ccagggaccaggcagcggttctggaggg

SEQ ID NO: 46186 - DNA, 28 bp, synthetic construct
  source 1..28: mol_type = other DNA
gccagggaccaggcagcggttctggagg

SEQ ID NO: 46187 - DNA, 28 bp, synthetic construct
  source 1..28: mol_type = other DNA
ccagaaccgctgcctggtccctggctgg

SEQ ID NO: 46188 - DNA, 28 bp, synthetic construct
  source 1..28: mol_type = other DNA
ggcgtaccagccagggaccaggcagcgg

SEQ ID NO: 46189 - DNA, 28 bp, synthetic construct
  source 1..28: mol_type = other DNA
gtgggtggcgtaccagccagggaccagg

SEQ ID NO: 46190 - DNA, 28 bp, synthetic construct
  source 1..28: mol_type = other DNA
ctcgatgtgggtggcgtaccagccaggg

SEQ ID NO: 46191 - DNA, 28 bp, synthetic construct
  source 1..28: mol_type = other DNA
gctcgatgtgggtggcgtaccagccagg

SEQ ID NO: 46192 - DNA, 28 bp, synthetic construct
  source 1..28: mol_type = other DNA
ctggtacgccacccacatcgagcgctgg

SEQ ID NO: 46193 - DNA, 28 bp, synthetic construct
  source 1..28: mol_type = other DNA
gcactgagccagcgctcgatgtgggtgg

SEQ ID NO: 46194 - DNA, 28 bp, synthetic construct
  source 1..28: mol_type = other DNA
taggcactgagccagcgctcgatgtggg

SEQ ID NO: 46195 - DNA, 28 bp, synthetic construct
  source 1..28: mol_type = other DNA
ataggcactgagccagcgctcgatgtgg

SEQ ID NO: 46196 - DNA, 28 bp, synthetic construct
  source 1..28: mol_type = other DNA
tggctcagtgcctatcacgccaaccagg

SEQ ID NO: 46197 - DNA, 28 bp, synthetic construct
  source 1..28: mol_type = other DNA
acagcagctacctggttggcgtgatagg

SEQ ID NO: 46198 - DNA, 28 bp, synthetic construct
  source 1..28: mol_type = other DNA
gggtcagggacagcagctacctggttgg

SEQ ID NO: 46199 - DNA, 28 bp, synthetic construct
  source 1..28: mol_type = other DNA
acaagggtcagggacagcagctacctgg

SEQ ID NO: 46200 - DNA, 28 bp, synthetic construct
  source 1..28: mol_type = other DNA
gtagctgctgtccctgacccttgtgagg

SEQ ID NO: 46201 - DNA, 28 bp, synthetic construct
  source 1..28: mol_type = other DNA
tagctgctgtccctgacccttgtgaggg

SEQ ID NO: 46202 - DNA, 28 bp, synthetic construct
  source 1..28: mol_type = other DNA
actgtgactgccctcacaagggtcaggg

SEQ ID NO: 46203 - DNA, 28 bp, synthetic construct
  source 1..28: mol_type = other DNA
tactgtgactgccctcacaagggtcagg

SEQ ID NO: 46204 - DNA, 28 bp, synthetic construct
  source 1..28: mol_type = other DNA
acccttgtgagggcagtcacagtactgg

SEQ ID NO: 46205 - DNA, 28 bp, synthetic construct
  source 1..28: mol_type = other DNA
gccagtactgtgactgccctcacaaggg

SEQ ID NO: 46206 - DNA, 28 bp, synthetic construct
  source 1..28: mol_type = other DNA
agccagtactgtgactgccctcacaagg

SEQ ID NO: 46207 - DNA, 28 bp, synthetic construct
  source 1..28: mol_type = other DNA
gggcagtcacagtactggcttgctgtgg

SEQ ID NO: 46208 - DNA, 28 bp, synthetic construct
  source 1..28: mol_type = other DNA
cacagtactggcttgctgtggttagcgg

SEQ ID NO: 46209 - DNA, 28 bp, synthetic construct
  source 1..28: mol_type = other DNA
gcctccaactctttctcaccagccgtgg

SEQ ID NO: 46210 - DNA, 28 bp, synthetic construct
  source 1..28: mol_type = other DNA
cccacggctggtgagaaagagttggagg

SEQ ID NO: 46211 - DNA, 28 bp, synthetic construct
  source 1..28: mol_type = other DNA
ctccaactctttctcaccagccgtgggg

SEQ ID NO: 46212 - DNA, 28 bp, synthetic construct
  source 1..28: mol_type = other DNA
gtccccacggctggtgagaaagagttgg

SEQ ID NO: 46213 - DNA, 28 bp, synthetic construct
  source 1..28: mol_type = other DNA
aggagggcatatctgtccccacggctgg

SEQ ID NO: 46214 - DNA, 28 bp, synthetic construct
  source 1..28: mol_type = other DNA
gccgtggggacagatatgccctccttgg

SEQ ID NO: 46215 - DNA, 28 bp, synthetic construct
  source 1..28: mol_type = other DNA
tccaaggagggcatatctgtccccacgg

SEQ ID NO: 46216 - DNA, 28 bp, synthetic construct
  source 1..28: mol_type = other DNA
ggaggagccagttctagagggtgcaggg

SEQ ID NO: 46217 - DNA, 28 bp, synthetic construct
  source 1..28: mol_type = other DNA
tatgggaccctgcaccctctagaactgg

SEQ ID NO: 46218 - DNA, 28 bp, synthetic construct
  source 1..28: mol_type = other DNA
ggtgcagggtcccatatttataagcagg

SEQ ID NO: 46219 - DNA, 28 bp, synthetic construct
  source 1..28: mol_type = other DNA
caggaatgggcctgcttataaatatggg

SEQ ID NO: 46220 - DNA, 28 bp, synthetic construct
  source 1..28: mol_type = other DNA
gcaggaatgggcctgcttataaatatgg

SEQ ID NO: 46221 - DNA, 28 bp, synthetic construct
  source 1..28: mol_type = other DNA
ataagcaggcccattcctgctgccgtgg

SEQ ID NO: 46222 - DNA, 28 bp, synthetic construct
  source 1..28: mol_type = other DNA
gggcaacagccacggcagcaggaatggg

SEQ ID NO: 46223 - DNA, 28 bp, synthetic construct
  source 1..28: mol_type = other DNA
agggcaacagccacggcagcaggaatgg

SEQ ID NO: 46224 - DNA, 28 bp, synthetic construct
  source 1..28: mol_type = other DNA
aaacaagggcaacagccacggcagcagg

SEQ ID NO: 46225 - DNA, 28 bp, synthetic construct
  source 1..28: mol_type = other DNA
cggtggcaaacaagggcaacagccacgg

SEQ ID NO: 46226 - DNA, 28 bp, synthetic construct
  source 1..28: mol_type = other DNA
ctgctttgacttcggtggcaaacaaggg

SEQ ID NO: 46227 - DNA, 28 bp, synthetic construct
  source 1..28: mol_type = other DNA
ccttgtttgccaccgaagtcaaagcagg

SEQ ID NO: 46228 - DNA, 28 bp, synthetic construct
  source 1..28: mol_type = other DNA
ggatcgggacctgctttgacttcggtgg

SEQ ID NO: 46229 - DNA, 28 bp, synthetic construct
  source 1..28: mol_type = other DNA
aggggatcgggacctgctttgacttcgg

SEQ ID NO: 46230 - DNA, 28 bp, synthetic construct
  source 1..28: mol_type = other DNA
aatctggaaagggagaaaggggatcggg

SEQ ID NO: 46231 - DNA, 28 bp, synthetic construct
  source 1..28: mol_type = other DNA
gaatctggaaagggagaaaggggatcgg

SEQ ID NO: 46232 - DNA, 28 bp, synthetic construct
  source 1..28: mol_type = other DNA
atcccctttctccctttccagattctgg

SEQ ID NO: 46233 - DNA, 28 bp, synthetic construct
  source 1..28: mol_type = other DNA
gaccagaatctggaaagggagaaagggg

SEQ ID NO: 46234 - DNA, 28 bp, synthetic construct
  source 1..28: mol_type = other DNA
agaccagaatctggaaagggagaaaggg

SEQ ID NO: 46235 - DNA, 28 bp, synthetic construct
  source 1..28: mol_type = other DNA
aagaccagaatctggaaagggagaaagg

SEQ ID NO: 46236 - DNA, 28 bp, synthetic construct
  source 1..28: mol_type = other DNA
tttctccctttccagattctggtcttgg

SEQ ID NO: 46237 - DNA, 28 bp, synthetic construct
  source 1..28: mol_type = other DNA
tccctttccagattctggtcttggatgg

SEQ ID NO: 46238 - DNA, 28 bp, synthetic construct
  source 1..28: mol_type = other DNA
gccatccaagaccagaatctggaaaggg

SEQ ID NO: 46239 - DNA, 28 bp, synthetic construct
  source 1..28: mol_type = other DNA
tgccatccaagaccagaatctggaaagg

SEQ ID NO: 46240 - DNA, 28 bp, synthetic construct
  source 1..28: mol_type = other DNA
cagtttgccatccaagaccagaatctgg

SEQ ID NO: 46241 - DNA, 28 bp, synthetic construct
  source 1..28: mol_type = other DNA
cttcgcacagaacctgccaaagtgatgg

SEQ ID NO: 46242 - DNA, 28 bp, synthetic construct
  source 1..28: mol_type = other DNA
acagaacctgccaaagtgatggacatgg

SEQ ID NO: 46243 - DNA, 28 bp, synthetic construct
  source 1..28: mol_type = other DNA
tctgcaccatgtccatcactttggcagg

SEQ ID NO: 46244 - DNA, 28 bp, synthetic construct
  source 1..28: mol_type = other DNA
aacttctgcaccatgtccatcactttgg

SEQ ID NO: 46245 - DNA, 28 bp, synthetic construct
  source 1..28: mol_type = other DNA
tgatggacatggtgcagaagttccttgg

SEQ ID NO: 46246 - DNA, 28 bp, synthetic construct
  source 1..28: mol_type = other DNA
gatggacatggtgcagaagttccttggg

SEQ ID NO: 46247 - DNA, 28 bp, synthetic construct
  source 1..28: mol_type = other DNA
atggacatggtgcagaagttccttgggg

SEQ ID NO: 46248 - DNA, 28 bp, synthetic construct
  source 1..28: mol_type = other DNA
gtagtcaatggtgttggtcaccccaagg

SEQ ID NO: 46249 - DNA, 28 bp, synthetic construct
  source 1..28: mol_type = other DNA
aaggttttgtggtagtcaatggtgttgg

SEQ ID NO: 46250 - DNA, 28 bp, synthetic construct
  source 1..28: mol_type = other DNA
aacaccattgactaccacaaaaccttgg

SEQ ID NO: 46251 - DNA, 28 bp, synthetic construct
  source 1..28: mol_type = other DNA
cacgccaaggttttgtggtagtcaatgg

SEQ ID NO: 46252 - DNA, 28 bp, synthetic construct
  source 1..28: mol_type = other DNA
aggcaacactcacgccaaggttttgtgg

SEQ ID NO: 46253 - DNA, 28 bp, synthetic construct
  source 1..28: mol_type = other DNA
aaaggaaaaggcaacactcacgccaagg

SEQ ID NO: 46254 - DNA, 28 bp, synthetic construct
  source 1..28: mol_type = other DNA
gtgagtgttgccttttcctttctgcagg

SEQ ID NO: 46255 - DNA, 28 bp, synthetic construct
  source 1..28: mol_type = other DNA
agggaaataacctgcagaaaggaaaagg

SEQ ID NO: 46256 - DNA, 28 bp, synthetic construct
  source 1..28: mol_type = other DNA
cttatcagggaaataacctgcagaaagg

SEQ ID NO: 46257 - DNA, 28 bp, synthetic construct
  source 1..28: mol_type = other DNA
ctttctgcaggttatttccctgataagg

SEQ ID NO: 46258 - DNA, 28 bp, synthetic construct
  source 1..28: mol_type = other DNA
caggttatttccctgataaggcacctgg

SEQ ID NO: 46259 - DNA, 28 bp, synthetic construct
  source 1..28: mol_type = other DNA
aggttatttccctgataaggcacctggg

SEQ ID NO: 46260 - DNA, 28 bp, synthetic construct
  source 1..28: mol_type = other DNA
ctttgttggcccaggtgccttatcaggg

SEQ ID NO: 46261 - DNA, 28 bp, synthetic construct
  source 1..28: mol_type = other DNA
gctttgttggcccaggtgccttatcagg

SEQ ID NO: 46262 - DNA, 28 bp, synthetic construct
  source 1..28: mol_type = other DNA
ttcaagactttggctttgttggcccagg

SEQ ID NO: 46263 - DNA, 28 bp, synthetic construct
  source 1..28: mol_type = other DNA
taattattcaagactttggctttgttgg

SEQ ID NO: 46264 - DNA, 28 bp, synthetic construct
  source 1..28: mol_type = other DNA
tctctctcataattattcaagactttgg

SEQ ID NO: 46265 - DNA, 28 bp, synthetic construct
  source 1..28: mol_type = other DNA
agaagttagttagagtcagaaagtatgg

SEQ ID NO: 46266 - DNA, 28 bp, synthetic construct
  source 1..28: mol_type = other DNA
ggaatctactgctcttgaacccacatgg

SEQ ID NO: 46267 - DNA, 28 bp, synthetic construct
  source 1..28: mol_type = other DNA
gtgggttcaagagcagtagattccctgg

SEQ ID NO: 46268 - DNA, 28 bp, synthetic construct
  source 1..28: mol_type = other DNA
tagattccctggtctctgccattcctgg

SEQ ID NO: 46269 - DNA, 28 bp, synthetic construct
  source 1..28: mol_type = other DNA
agattccctggtctctgccattcctggg

SEQ ID NO: 46270 - DNA, 28 bp, synthetic construct
  source 1..28: mol_type = other DNA
gattccctggtctctgccattcctgggg

SEQ ID NO: 46271 - DNA, 28 bp, synthetic construct
  source 1..28: mol_type = other DNA
tggaccccaggaatggcagagaccaggg

SEQ ID NO: 46272 - DNA, 28 bp, synthetic construct
  source 1..28: mol_type = other DNA
atggaccccaggaatggcagagaccagg

SEQ ID NO: 46273 - DNA, 28 bp, synthetic construct
  source 1..28: mol_type = other DNA
ctgccattcctggggtccatgaacatgg

SEQ ID NO: 46274 - DNA, 28 bp, synthetic construct
  source 1..28: mol_type = other DNA
aagccatgttcatggaccccaggaatgg

SEQ ID NO: 46275 - DNA, 28 bp, synthetic construct
  source 1..28: mol_type = other DNA
cctggggtccatgaacatggctttaagg

SEQ ID NO: 46276 - DNA, 28 bp, synthetic construct
  source 1..28: mol_type = other DNA
gggtccatgaacatggctttaaggtcgg

SEQ ID NO: 46277 - DNA, 28 bp, synthetic construct
  source 1..28: mol_type = other DNA
acttccgaccttaaagccatgttcatgg

SEQ ID NO: 46278 - DNA, 28 bp, synthetic construct
  source 1..28: mol_type = other DNA
atgaacatggctttaaggtcggaagtgg

SEQ ID NO: 46279 - DNA, 28 bp, synthetic construct
  source 1..28: mol_type = other DNA
tgaacatggctttaaggtcggaagtggg

SEQ ID NO: 46280 - DNA, 28 bp, synthetic construct
  source 1..28: mol_type = other DNA
acatggctttaaggtcggaagtgggtgg

SEQ ID NO: 46281 - DNA, 28 bp, synthetic construct
  source 1..28: mol_type = other DNA
ggtgggaaagtctttggatgggagctgg

SEQ ID NO: 46282 - DNA, 28 bp, synthetic construct
  source 1..28: mol_type = other DNA
tgtggaggtgggaaagtctttggatggg

SEQ ID NO: 46283 - DNA, 28 bp, synthetic construct
  source 1..28: mol_type = other DNA
ctgtggaggtgggaaagtctttggatgg

SEQ ID NO: 46284 - DNA, 28 bp, synthetic construct
  source 1..28: mol_type = other DNA
catccaaagactttcccacctccacagg

SEQ ID NO: 46285 - DNA, 28 bp, synthetic construct
  source 1..28: mol_type = other DNA
aaacctgtggaggtgggaaagtctttgg

SEQ ID NO: 46286 - DNA, 28 bp, synthetic construct
  source 1..28: mol_type = other DNA
ttctttggatcaaacctgtggaggtggg

SEQ ID NO: 46287 - DNA, 28 bp, synthetic construct
  source 1..28: mol_type = other DNA
tttctttggatcaaacctgtggaggtgg

SEQ ID NO: 46288 - DNA, 28 bp, synthetic construct
  source 1..28: mol_type = other DNA
acctccacaggtttgatccaaagaaagg

SEQ ID NO: 46289 - DNA, 28 bp, synthetic construct
  source 1..28: mol_type = other DNA
tcctttctttggatcaaacctgtggagg

SEQ ID NO: 46290 - DNA, 28 bp, synthetic construct
  source 1..28: mol_type = other DNA
aaatcctttctttggatcaaacctgtgg

SEQ ID NO: 46291 - DNA, 28 bp, synthetic construct
  source 1..28: mol_type = other DNA
caggtttgatccaaagaaaggattttgg

SEQ ID NO: 46292 - DNA, 28 bp, synthetic construct
  source 1..28: mol_type = other DNA
gcagttggcaccaaaatcctttctttgg

SEQ ID NO: 46293 - DNA, 28 bp, synthetic construct
  source 1..28: mol_type = other DNA
aaggattttggtgccaactgcttgaagg

SEQ ID NO: 46294 - DNA, 28 bp, synthetic construct
  source 1..28: mol_type = other DNA
gattttggtgccaactgcttgaaggagg

SEQ ID NO: 46295 - DNA, 28 bp, synthetic construct
  source 1..28: mol_type = other DNA
cttggtttttcctccttcaagcagttgg

SEQ ID NO: 46296 - DNA, 28 bp, synthetic construct
  source 1..28: mol_type = other DNA
cttgaaggaggaaaaaccaagtgtctgg

SEQ ID NO: 46297 - DNA, 28 bp, synthetic construct
  source 1..28: mol_type = other DNA
ttgaaggaggaaaaaccaagtgtctggg

SEQ ID NO: 46298 - DNA, 28 bp, synthetic construct
  source 1..28: mol_type = other DNA
aaaaccaagtgtctgggcaaaagcaagg

SEQ ID NO: 46299 - DNA, 28 bp, synthetic construct
  source 1..28: mol_type = other DNA
aaaccaagtgtctgggcaaaagcaaggg

SEQ ID NO: 46300 - DNA, 28 bp, synthetic construct
  source 1..28: mol_type = other DNA
cggcccttgcttttgcccagacacttgg

SEQ ID NO: 46301 - DNA, 28 bp, synthetic construct
  source 1..28: mol_type = other DNA
caagtgtctgggcaaaagcaagggccgg

SEQ ID NO: 46302 - DNA, 28 bp, synthetic construct
  source 1..28: mol_type = other DNA
agcaagggccggaaatatcccgagatgg

SEQ ID NO: 46303 - DNA, 28 bp, synthetic construct
  source 1..28: mol_type = other DNA
ggccggaaatatcccgagatggacttgg

SEQ ID NO: 46304 - DNA, 28 bp, synthetic construct
  source 1..28: mol_type = other DNA
atccaagtccatctcgggatatttccgg

SEQ ID NO: 46305 - DNA, 28 bp, synthetic construct
  source 1..28: mol_type = other DNA
atcccgagatggacttggatgtaagtgg

SEQ ID NO: 46306 - DNA, 28 bp, synthetic construct
  source 1..28: mol_type = other DNA
caccacttacatccaagtccatctcggg

SEQ ID NO: 46307 - DNA, 28 bp, synthetic construct
  source 1..28: mol_type = other DNA
ccaccacttacatccaagtccatctcgg

SEQ ID NO: 46308 - DNA, 28 bp, synthetic construct
  source 1..28: mol_type = other DNA
acacactacctgtagcacctgcataagg

SEQ ID NO: 46309 - DNA, 28 bp, synthetic construct
  source 1..28: mol_type = other DNA
cacactacctgtagcacctgcataaggg

SEQ ID NO: 46310 - DNA, 28 bp, synthetic construct
  source 1..28: mol_type = other DNA
tacctgtagcacctgcataagggtaagg

SEQ ID NO: 46311 - DNA, 28 bp, synthetic construct
  source 1..28: mol_type = other DNA
acctgtagcacctgcataagggtaaggg

SEQ ID NO: 46312 - DNA, 28 bp, synthetic construct
  source 1..28: mol_type = other DNA
ccccttacccttatgcaggtgctacagg

SEQ ID NO: 46313 - DNA, 28 bp, synthetic construct
  source 1..28: mol_type = other DNA
atacagggaccccttacccttatgcagg

SEQ ID NO: 46314 - DNA, 28 bp, synthetic construct
  source 1..28: mol_type = other DNA
tgcataagggtaaggggtccctgtatgg

SEQ ID NO: 46315 - DNA, 28 bp, synthetic construct
  source 1..28: mol_type = other DNA
ggtaaggggtccctgtatggagttgagg

SEQ ID NO: 46316 - DNA, 28 bp, synthetic construct
  source 1..28: mol_type = other DNA
gtaaggggtccctgtatggagttgaggg

SEQ ID NO: 46317 - DNA, 28 bp, synthetic construct
  source 1..28: mol_type = other DNA
taaggggtccctgtatggagttgagggg

SEQ ID NO: 46318 - DNA, 28 bp, synthetic construct
  source 1..28: mol_type = other DNA
aaggggtccctgtatggagttgaggggg

SEQ ID NO: 46319 - DNA, 28 bp, synthetic construct
  source 1..28: mol_type = other DNA
agagaatccccctcaactccatacaggg

SEQ ID NO: 46320 - DNA, 28 bp, synthetic construct
  source 1..28: mol_type = other DNA
aagagaatccccctcaactccatacagg

SEQ ID NO: 46321 - DNA, 28 bp, synthetic construct
  source 1..28: mol_type = other DNA
catgaacatgctgagtgcatggtaaagg

SEQ ID NO: 46322 - DNA, 28 bp, synthetic construct
  source 1..28: mol_type = other DNA
ctttaccatgcactcagcatgttcatgg

SEQ ID NO: 46323 - DNA, 28 bp, synthetic construct
  source 1..28: mol_type = other DNA
taaggccatgaacatgctgagtgcatgg

SEQ ID NO: 46324 - DNA, 28 bp, synthetic construct
  source 1..28: mol_type = other DNA
gcatgttcatggccttagcatttcttgg

SEQ ID NO: 46325 - DNA, 28 bp, synthetic construct
  source 1..28: mol_type = other DNA
gtaatcccagcactttgggaggccgagg

SEQ ID NO: 46326 - DNA, 28 bp, synthetic construct
  source 1..28: mol_type = other DNA
cggcctcccaaagtgctgggattacagg

SEQ ID NO: 46327 - DNA, 28 bp, synthetic construct
  source 1..28: mol_type = other DNA
atgcctgtaatcccagcactttgggagg

SEQ ID NO: 46328 - DNA, 28 bp, synthetic construct
  source 1..28: mol_type = other DNA
ctcatgcctgtaatcccagcactttggg

SEQ ID NO: 46329 - DNA, 28 bp, synthetic construct
  source 1..28: mol_type = other DNA
gctcatgcctgtaatcccagcactttgg

SEQ ID NO: 46330 - DNA, 28 bp, synthetic construct
  source 1..28: mol_type = other DNA
gattacaggcatgagccaccgtgcccgg

SEQ ID NO: 46331 - DNA, 28 bp, synthetic construct
  source 1..28: mol_type = other DNA
atgagccaccgtgcccggccgagcatgg

SEQ ID NO: 46332 - DNA, 28 bp, synthetic construct
  source 1..28: mol_type = other DNA
aatcgccatgctcggccgggcacggtgg

SEQ ID NO: 46333 - DNA, 28 bp, synthetic construct
  source 1..28: mol_type = other DNA
aaaaatcgccatgctcggccgggcacgg

SEQ ID NO: 46334 - DNA, 28 bp, synthetic construct
  source 1..28: mol_type = other DNA
cctctaaaaatcgccatgctcggccggg

SEQ ID NO: 46335 - DNA, 28 bp, synthetic construct
  source 1..28: mol_type = other DNA
tcctctaaaaatcgccatgctcggccgg

SEQ ID NO: 46336 - DNA, 28 bp, synthetic construct
  source 1..28: mol_type = other DNA
ggccgagcatggcgatttttagaggagg

SEQ ID NO: 46337 - DNA, 28 bp, synthetic construct
  source 1..28: mol_type = other DNA
gacctcctctaaaaatcgccatgctcgg

SEQ ID NO: 46338 - DNA, 28 bp, synthetic construct
  source 1..28: mol_type = other DNA
gaggtcactcttaagtcagtacacaagg

SEQ ID NO: 46339 - DNA, 28 bp, synthetic construct
  source 1..28: mol_type = other DNA
aggaaggctcgggactgtaacgggaagg

SEQ ID NO: 46340 - DNA, 28 bp, synthetic construct
  source 1..28: mol_type = other DNA
cttcaggaaggctcgggactgtaacggg

SEQ ID NO: 46341 - DNA, 28 bp, synthetic construct
  source 1..28: mol_type = other DNA
ccttcaggaaggctcgggactgtaacgg

SEQ ID NO: 46342 - DNA, 28 bp, synthetic construct
  source 1..28: mol_type = other DNA
cggtaatagtccttcaggaaggctcggg

SEQ ID NO: 46343 - DNA, 28 bp, synthetic construct
  source 1..28: mol_type = other DNA
ccggtaatagtccttcaggaaggctcgg

SEQ ID NO: 46344 - DNA, 28 bp, synthetic construct
  source 1..28: mol_type = other DNA
cgagccttcctgaaggactattaccggg

SEQ ID NO: 46345 - DNA, 28 bp, synthetic construct
  source 1..28: mol_type = other DNA
tggtcccggtaatagtccttcaggaagg

SEQ ID NO: 46346 - DNA, 28 bp, synthetic construct
  source 1..28: mol_type = other DNA
gttgtggtcccggtaatagtccttcagg

SEQ ID NO: 46347 - DNA, 28 bp, synthetic construct
  source 1..28: mol_type = other DNA
cttggagagctcgatgttgtggtcccgg

SEQ ID NO: 46348 - DNA, 28 bp, synthetic construct
  source 1..28: mol_type = other DNA
cagcagcttggagagctcgatgttgtgg

SEQ ID NO: 46349 - DNA, 28 bp, synthetic construct
  source 1..28: mol_type = other DNA
gagctctccaagctgctgtataagatgg

SEQ ID NO: 46350 - DNA, 28 bp, synthetic construct
  source 1..28: mol_type = other DNA
agctctccaagctgctgtataagatggg

SEQ ID NO: 46351 - DNA, 28 bp, synthetic construct
  source 1..28: mol_type = other DNA
gtctggcccatcttatacagcagcttgg

SEQ ID NO: 46352 - DNA, 28 bp, synthetic construct
  source 1..28: mol_type = other DNA
taagatgggccagacacttcccacttgg

SEQ ID NO: 46353 - DNA, 28 bp, synthetic construct
  source 1..28: mol_type = other DNA
ctctcgtagccaagtgggaagtgtctgg

SEQ ID NO: 46354 - DNA, 28 bp, synthetic construct
  source 1..28: mol_type = other DNA
cagacacttcccacttggctacgagagg

SEQ ID NO: 46355 - DNA, 28 bp, synthetic construct
  source 1..28: mol_type = other DNA
tctggaggtcctctcgtagccaagtggg

SEQ ID NO: 46356 - DNA, 28 bp, synthetic construct
  source 1..28: mol_type = other DNA
ttctggaggtcctctcgtagccaagtgg

SEQ ID NO: 46357 - DNA, 28 bp, synthetic construct
  source 1..28: mol_type = other DNA
gctacgagaggacctccagaacaccagg

SEQ ID NO: 46358 - DNA, 28 bp, synthetic construct
  source 1..28: mol_type = other DNA
ggacctccagaacaccaggtagccgtgg

SEQ ID NO: 46359 - DNA, 28 bp, synthetic construct
  source 1..28: mol_type = other DNA
tggccacggctacctggtgttctggagg

SEQ ID NO: 46360 - DNA, 28 bp, synthetic construct
  source 1..28: mol_type = other DNA
tggtggccacggctacctggtgttctgg

SEQ ID NO: 46361 - DNA, 28 bp, synthetic construct
  source 1..28: mol_type = other DNA
tctggctgtggtggccacggctacctgg

SEQ ID NO: 46362 - DNA, 28 bp, synthetic construct
  source 1..28: mol_type = other DNA
acgttcagtctggctgtggtggccacgg

SEQ ID NO: 46363 - DNA, 28 bp, synthetic construct
  source 1..28: mol_type = other DNA
tcacaaacgttcagtctggctgtggtgg

SEQ ID NO: 46364 - DNA, 28 bp, synthetic construct
  source 1..28: mol_type = other DNA
ctttcacaaacgttcagtctggctgtgg

SEQ ID NO: 46365 - DNA, 28 bp, synthetic construct
  source 1..28: mol_type = other DNA
agccagactgaacgtttgtgaaagctgg

SEQ ID NO: 46366 - DNA, 28 bp, synthetic construct
  source 1..28: mol_type = other DNA
gccagactgaacgtttgtgaaagctggg

SEQ ID NO: 46367 - DNA, 28 bp, synthetic construct
  source 1..28: mol_type = other DNA
tcccagctttcacaaacgttcagtctgg

SEQ ID NO: 46368 - DNA, 28 bp, synthetic construct
  source 1..28: mol_type = other DNA
ctgcaggtctggctcagcgtgtggtggg

SEQ ID NO: 46369 - DNA, 28 bp, synthetic construct
  source 1..28: mol_type = other DNA
tctgcaggtctggctcagcgtgtggtgg

SEQ ID NO: 46370 - DNA, 28 bp, synthetic construct
  source 1..28: mol_type = other DNA
cactctgcaggtctggctcagcgtgtgg

SEQ ID NO: 46371 - DNA, 28 bp, synthetic construct
  source 1..28: mol_type = other DNA
cacacgctgagccagacctgcagagtgg

SEQ ID NO: 46372 - DNA, 28 bp, synthetic construct
  source 1..28: mol_type = other DNA
acacgctgagccagacctgcagagtggg

SEQ ID NO: 46373 - DNA, 28 bp, synthetic construct
  source 1..28: mol_type = other DNA
gagccagacctgcagagtgggaagctgg

SEQ ID NO: 46374 - DNA, 28 bp, synthetic construct
  source 1..28: mol_type = other DNA
ggtccagcttcccactctgcaggtctgg

SEQ ID NO: 46375 - DNA, 28 bp, synthetic construct
  source 1..28: mol_type = other DNA
gacctgcagagtgggaagctggaccagg

SEQ ID NO: 46376 - DNA, 28 bp, synthetic construct
  source 1..28: mol_type = other DNA
acctgcagagtgggaagctggaccaggg

SEQ ID NO: 46377 - DNA, 28 bp, synthetic construct
  source 1..28: mol_type = other DNA
gccctggtccagcttcccactctgcagg

SEQ ID NO: 46378 - DNA, 28 bp, synthetic construct
  source 1..28: mol_type = other DNA
attgctcataagtgcgcagctgccctgg

SEQ ID NO: 46379 - DNA, 28 bp, synthetic construct
  source 1..28: mol_type = other DNA
ctgcgcacttatgagcaatactctgtgg

SEQ ID NO: 46380 - DNA, 28 bp, synthetic construct
  source 1..28: mol_type = other DNA
cgcacttatgagcaatactctgtggagg

SEQ ID NO: 46381 - DNA, 28 bp, synthetic construct
  source 1..28: mol_type = other DNA
ttatgagcaatactctgtggaggtctgg

SEQ ID NO: 46382 - DNA, 28 bp, synthetic construct
  source 1..28: mol_type = other DNA
tgagcaatactctgtggaggtctggtgg

SEQ ID NO: 46383 - DNA, 28 bp, synthetic construct
  source 1..28: mol_type = other DNA
gagcaatactctgtggaggtctggtggg

SEQ ID NO: 46384 - DNA, 28 bp, synthetic construct
  source 1..28: mol_type = other DNA
agcaatactctgtggaggtctggtgggg

SEQ ID NO: 46385 - DNA, 28 bp, synthetic construct
  source 1..28: mol_type = other DNA
atactctgtggaggtctggtggggctgg

SEQ ID NO: 46386 - DNA, 28 bp, synthetic construct
  source 1..28: mol_type = other DNA
tactctgtggaggtctggtggggctggg

SEQ ID NO: 46387 - DNA, 28 bp, synthetic construct
  source 1..28: mol_type = other DNA
actctgtggaggtctggtggggctgggg

SEQ ID NO: 46388 - DNA, 28 bp, synthetic construct
  source 1..28: mol_type = other DNA
ctctgtggaggtctggtggggctggggg

SEQ ID NO: 46389 - DNA, 28 bp, synthetic construct
  source 1..28: mol_type = other DNA
gtctggtggggctgggggagcacccagg

SEQ ID NO: 46390 - DNA, 28 bp, synthetic construct
  source 1..28: mol_type = other DNA
tggtggggctgggggagcacccaggcgg

SEQ ID NO: 46391 - DNA, 28 bp, synthetic construct
  source 1..28: mol_type = other DNA
cacccaggcggatctgcaagcacctcgg

SEQ ID NO: 46392 - DNA, 28 bp, synthetic construct
  source 1..28: mol_type = other DNA
ctccgaggtgcttgcagatccgcctggg

SEQ ID NO: 46393 - DNA, 28 bp, synthetic construct
  source 1..28: mol_type = other DNA
gctccgaggtgcttgcagatccgcctgg

SEQ ID NO: 46394 - DNA, 28 bp, synthetic construct
  source 1..28: mol_type = other DNA
gcaagcacctcggagcacccaccgctgg

SEQ ID NO: 46395 - DNA, 28 bp, synthetic construct
  source 1..28: mol_type = other DNA
caagcacctcggagcacccaccgctggg

SEQ ID NO: 46396 - DNA, 28 bp, synthetic construct
  source 1..28: mol_type = other DNA
cgcagacccagcggtgggtgctccgagg

SEQ ID NO: 46397 - DNA, 28 bp, synthetic construct
  source 1..28: mol_type = other DNA
ctcggagcacccaccgctgggtctgcgg

SEQ ID NO: 46398 - DNA, 28 bp, synthetic construct
  source 1..28: mol_type = other DNA
cacccaccgctgggtctgcggcctaagg

SEQ ID NO: 46399 - DNA, 28 bp, synthetic construct
  source 1..28: mol_type = other DNA
acccaccgctgggtctgcggcctaaggg

SEQ ID NO: 46400 - DNA, 28 bp, synthetic construct
  source 1..28: mol_type = other DNA
tcccttaggccgcagacccagcggtggg

SEQ ID NO: 46401 - DNA, 28 bp, synthetic construct
  source 1..28: mol_type = other DNA
gtcccttaggccgcagacccagcggtgg

SEQ ID NO: 46402 - DNA, 28 bp, synthetic construct
  source 1..28: mol_type = other DNA
gaggtcccttaggccgcagacccagcgg

SEQ ID NO: 46403 - DNA, 28 bp, synthetic construct
  source 1..28: mol_type = other DNA
cctctgctggcgagggaggtcccttagg

SEQ ID NO: 46404 - DNA, 28 bp, synthetic construct
  source 1..28: mol_type = other DNA
cggaatggacctctgctggcgagggagg

SEQ ID NO: 46405 - DNA, 28 bp, synthetic construct
  source 1..28: mol_type = other DNA
gaacggaatggacctctgctggcgaggg

SEQ ID NO: 46406 - DNA, 28 bp, synthetic construct
  source 1..28: mol_type = other DNA
ggaacggaatggacctctgctggcgagg

SEQ ID NO: 46407 - DNA, 28 bp, synthetic construct
  source 1..28: mol_type = other DNA
agctgggaacggaatggacctctgctgg

SEQ ID NO: 46408 - DNA, 28 bp, synthetic construct
  source 1..28: mol_type = other DNA
ggtccattccgttcccagctgctcctgg

SEQ ID NO: 46409 - DNA, 28 bp, synthetic construct
  source 1..28: mol_type = other DNA
gtccattccgttcccagctgctcctggg

SEQ ID NO: 46410 - DNA, 28 bp, synthetic construct
  source 1..28: mol_type = other DNA
tccattccgttcccagctgctcctgggg

SEQ ID NO: 46411 - DNA, 28 bp, synthetic construct
  source 1..28: mol_type = other DNA
tccccaggagcagctgggaacggaatgg

SEQ ID NO: 46412 - DNA, 28 bp, synthetic construct
  source 1..28: mol_type = other DNA
attccgttcccagctgctcctggggagg

SEQ ID NO: 46413 - DNA, 28 bp, synthetic construct
  source 1..28: mol_type = other DNA
cggcctccccaggagcagctgggaacgg

SEQ ID NO: 46414 - DNA, 28 bp, synthetic construct
  source 1..28: mol_type = other DNA
ggaagcggcctccccaggagcagctggg

SEQ ID NO: 46415 - DNA, 28 bp, synthetic construct
  source 1..28: mol_type = other DNA
aggaagcggcctccccaggagcagctgg

SEQ ID NO: 46416 - DNA, 28 bp, synthetic construct
  source 1..28: mol_type = other DNA
agctgctcctggggaggccgcttcctgg

SEQ ID NO: 46417 - DNA, 28 bp, synthetic construct
  source 1..28: mol_type = other DNA
gctcctggggaggccgcttcctggtagg

SEQ ID NO: 46418 - DNA, 28 bp, synthetic construct
  source 1..28: mol_type = other DNA
cctcctaccaggaagcggcctccccagg

SEQ ID NO: 46419 - DNA, 28 bp, synthetic construct
  source 1..28: mol_type = other DNA
ctggggaggccgcttcctggtaggaggg

SEQ ID NO: 46420 - DNA, 28 bp, synthetic construct
  source 1..28: mol_type = other DNA
tcgtggactccctcctaccaggaagcgg

SEQ ID NO: 46421 - DNA, 28 bp, synthetic construct
  source 1..28: mol_type = other DNA
agagtctcgtggactccctcctaccagg

SEQ ID NO: 46422 - DNA, 28 bp, synthetic construct
  source 1..28: mol_type = other DNA
cagtgagggacagaaaagagtctcgtgg

SEQ ID NO: 46423 - DNA, 28 bp, synthetic construct
  source 1..28: mol_type = other DNA
ggggacagtcggcggaacacagtgaggg

SEQ ID NO: 46424 - DNA, 28 bp, synthetic construct
  source 1..28: mol_type = other DNA
aggggacagtcggcggaacacagtgagg

SEQ ID NO: 46425 - DNA, 28 bp, synthetic construct
  source 1..28: mol_type = other DNA
atgggtgacgagaggggacagtcggcgg

SEQ ID NO: 46426 - DNA, 28 bp, synthetic construct
  source 1..28: mol_type = other DNA
gtgatgggtgacgagaggggacagtcgg

SEQ ID NO: 46427 - DNA, 28 bp, synthetic construct
  source 1..28: mol_type = other DNA
agcagggagtgatgggtgacgagagggg

SEQ ID NO: 46428 - DNA, 28 bp, synthetic construct
  source 1..28: mol_type = other DNA
aagcagggagtgatgggtgacgagaggg

SEQ ID NO: 46429 - DNA, 28 bp, synthetic construct
  source 1..28: mol_type = other DNA
gaagcagggagtgatgggtgacgagagg

SEQ ID NO: 46430 - DNA, 28 bp, synthetic construct
  source 1..28: mol_type = other DNA
gtcacccatcactccctgcttccgcagg

SEQ ID NO: 46431 - DNA, 28 bp, synthetic construct
  source 1..28: mol_type = other DNA
tcacccatcactccctgcttccgcaggg

SEQ ID NO: 46432 - DNA, 28 bp, synthetic construct
  source 1..28: mol_type = other DNA
gcgccctgcggaagcagggagtgatggg

SEQ ID NO: 46433 - DNA, 28 bp, synthetic construct
  source 1..28: mol_type = other DNA
ggcgccctgcggaagcagggagtgatgg

SEQ ID NO: 46434 - DNA, 28 bp, synthetic construct
  source 1..28: mol_type = other DNA
tactgaggggcgccctgcggaagcaggg

SEQ ID NO: 46435 - DNA, 28 bp, synthetic construct
  source 1..28: mol_type = other DNA
atactgaggggcgccctgcggaagcagg

SEQ ID NO: 46436 - DNA, 28 bp, synthetic construct
  source 1..28: mol_type = other DNA
gcagcgaatactgaggggcgccctgcgg

SEQ ID NO: 46437 - DNA, 28 bp, synthetic construct
  source 1..28: mol_type = other DNA
gggacatatggcagcgaatactgagggg

SEQ ID NO: 46438 - DNA, 28 bp, synthetic construct
  source 1..28: mol_type = other DNA
agggacatatggcagcgaatactgaggg

SEQ ID NO: 46439 - DNA, 28 bp, synthetic construct
  source 1..28: mol_type = other DNA
cagggacatatggcagcgaatactgagg

SEQ ID NO: 46440 - DNA, 28 bp, synthetic construct
  source 1..28: mol_type = other DNA
tcgctgccatatgtccctgtcctccagg

SEQ ID NO: 46441 - DNA, 28 bp, synthetic construct
  source 1..28: mol_type = other DNA
ctacagcctggaggacagggacatatgg

SEQ ID NO: 46442 - DNA, 28 bp, synthetic construct
  source 1..28: mol_type = other DNA
catatgtccctgtcctccaggctgtagg

SEQ ID NO: 46443 - DNA, 28 bp, synthetic construct
  source 1..28: mol_type = other DNA
atatgtccctgtcctccaggctgtaggg

SEQ ID NO: 46444 - DNA, 28 bp, synthetic construct
  source 1..28: mol_type = other DNA
tatgtccctgtcctccaggctgtagggg

SEQ ID NO: 46445 - DNA, 28 bp, synthetic construct
  source 1..28: mol_type = other DNA
gtccctgtcctccaggctgtaggggagg

SEQ ID NO: 46446 - DNA, 28 bp, synthetic construct
  source 1..28: mol_type = other DNA
ctcctcccctacagcctggaggacaggg

SEQ ID NO: 46447 - DNA, 28 bp, synthetic construct
  source 1..28: mol_type = other DNA
tctcctcccctacagcctggaggacagg

SEQ ID NO: 46448 - DNA, 28 bp, synthetic construct
  source 1..28: mol_type = other DNA
caggctctcctcccctacagcctggagg

SEQ ID NO: 46449 - DNA, 28 bp, synthetic construct
  source 1..28: mol_type = other DNA
ctccaggctgtaggggaggagagcctgg

SEQ ID NO: 46450 - DNA, 28 bp, synthetic construct
  source 1..28: mol_type = other DNA
ggccaggctctcctcccctacagcctgg

SEQ ID NO: 46451 - DNA, 28 bp, synthetic construct
  source 1..28: mol_type = other DNA
aggctgtaggggaggagagcctggccgg

SEQ ID NO: 46452 - DNA, 28 bp, synthetic construct
  source 1..28: mol_type = other DNA
ggctgtaggggaggagagcctggccggg

SEQ ID NO: 46453 - DNA, 28 bp, synthetic construct
  source 1..28: mol_type = other DNA
gctgtaggggaggagagcctggccgggg

SEQ ID NO: 46454 - DNA, 28 bp, synthetic construct
  source 1..28: mol_type = other DNA
ctgtaggggaggagagcctggccggggg

SEQ ID NO: 46455 - DNA, 28 bp, synthetic construct
  source 1..28: mol_type = other DNA
gagagcctggccgggggagacagactgg

SEQ ID NO: 46456 - DNA, 28 bp, synthetic construct
  source 1..28: mol_type = other DNA
aatgtccagtctgtctcccccggccagg

SEQ ID NO: 46457 - DNA, 28 bp, synthetic construct
  source 1..28: mol_type = other DNA
agggaaatgtccagtctgtctcccccgg

SEQ ID NO: 46458 - DNA, 28 bp, synthetic construct
  source 1..28: mol_type = other DNA
actggacatttccctgtttcgagccagg

SEQ ID NO: 46459 - DNA, 28 bp, synthetic construct
  source 1..28: mol_type = other DNA
ccttggaagagcctggctcgaaacaggg

SEQ ID NO: 46460 - DNA, 28 bp, synthetic construct
  source 1..28: mol_type = other DNA
cctgtttcgagccaggctcttccaaggg

SEQ ID NO: 46461 - DNA, 28 bp, synthetic construct
  source 1..28: mol_type = other DNA
ctgtttcgagccaggctcttccaagggg

SEQ ID NO: 46462 - DNA, 28 bp, synthetic construct
  source 1..28: mol_type = other DNA
agccaggctcttccaaggggccagctgg

SEQ ID NO: 46463 - DNA, 28 bp, synthetic construct
  source 1..28: mol_type = other DNA
gccaggctcttccaaggggccagctggg

SEQ ID NO: 46464 - DNA, 28 bp, synthetic construct
  source 1..28: mol_type = other DNA
acccagctggccccttggaagagcctgg

SEQ ID NO: 46465 - DNA, 28 bp, synthetic construct
  source 1..28: mol_type = other DNA
tcttccaaggggccagctgggtccccgg

SEQ ID NO: 46466 - DNA, 28 bp, synthetic construct
  source 1..28: mol_type = other DNA
gactccggggacccagctggccccttgg

SEQ ID NO: 46467 - DNA, 28 bp, synthetic construct
  source 1..28: mol_type = other DNA
ctaggactgactccggggacccagctgg

SEQ ID NO: 46468 - DNA, 28 bp, synthetic construct
  source 1..28: mol_type = other DNA
cagctgggtccccggagtcagtcctagg

SEQ ID NO: 46469 - DNA, 28 bp, synthetic construct
  source 1..28: mol_type = other DNA
tgggtccccggagtcagtcctaggctgg

SEQ ID NO: 46470 - DNA, 28 bp, synthetic construct
  source 1..28: mol_type = other DNA
tccccggagtcagtcctaggctggatgg

SEQ ID NO: 46471 - DNA, 28 bp, synthetic construct
  source 1..28: mol_type = other DNA
cccatccagcctaggactgactccgggg

SEQ ID NO: 46472 - DNA, 28 bp, synthetic construct
  source 1..28: mol_type = other DNA
tcccatccagcctaggactgactccggg

SEQ ID NO: 46473 - DNA, 28 bp, synthetic construct
  source 1..28: mol_type = other DNA
ctcccatccagcctaggactgactccgg

SEQ ID NO: 46474 - DNA, 28 bp, synthetic construct
  source 1..28: mol_type = other DNA
cggagtcagtcctaggctggatgggagg

SEQ ID NO: 46475 - DNA, 28 bp, synthetic construct
  source 1..28: mol_type = other DNA
ggagtcagtcctaggctggatgggaggg

SEQ ID NO: 46476 - DNA, 28 bp, synthetic construct
  source 1..28: mol_type = other DNA
gtcagtcctaggctggatgggagggtgg

SEQ ID NO: 46477 - DNA, 28 bp, synthetic construct
  source 1..28: mol_type = other DNA
agggggccaccctcccatccagcctagg

SEQ ID NO: 46478 - DNA, 28 bp, synthetic construct
  source 1..28: mol_type = other DNA
tggatgggagggtggccccctcaagagg

SEQ ID NO: 46479 - DNA, 28 bp, synthetic construct
  source 1..28: mol_type = other DNA
gtggaggctgggagtcctcttgaggggg

SEQ ID NO: 46480 - DNA, 28 bp, synthetic construct
  source 1..28: mol_type = other DNA
tgtggaggctgggagtcctcttgagggg

SEQ ID NO: 46481 - DNA, 28 bp, synthetic construct
  source 1..28: mol_type = other DNA
atgtggaggctgggagtcctcttgaggg

SEQ ID NO: 46482 - DNA, 28 bp, synthetic construct
  source 1..28: mol_type = other DNA
gatgtggaggctgggagtcctcttgagg

SEQ ID NO: 46483 - DNA, 28 bp, synthetic construct
  source 1..28: mol_type = other DNA
caagaggactcccagcctccacatctgg

SEQ ID NO: 46484 - DNA, 28 bp, synthetic construct
  source 1..28: mol_type = other DNA
aaggtaggaaccagatgtggaggctggg

SEQ ID NO: 46485 - DNA, 28 bp, synthetic construct
  source 1..28: mol_type = other DNA
gaaggtaggaaccagatgtggaggctgg

SEQ ID NO: 46486 - DNA, 28 bp, synthetic construct
  source 1..28: mol_type = other DNA
atgtgaaggtaggaaccagatgtggagg

SEQ ID NO: 46487 - DNA, 28 bp, synthetic construct
  source 1..28: mol_type = other DNA
gagatgtgaaggtaggaaccagatgtgg

SEQ ID NO: 46488 - DNA, 28 bp, synthetic construct
  source 1..28: mol_type = other DNA
gaacgggagggtgagatgtgaaggtagg

SEQ ID NO: 46489 - DNA, 28 bp, synthetic construct
  source 1..28: mol_type = other DNA
accttcacatctcaccctcccgttctgg

SEQ ID NO: 46490 - DNA, 28 bp, synthetic construct
  source 1..28: mol_type = other DNA
ccttcacatctcaccctcccgttctggg

SEQ ID NO: 46491 - DNA, 28 bp, synthetic construct
  source 1..28: mol_type = other DNA
cttcacatctcaccctcccgttctgggg

SEQ ID NO: 46492 - DNA, 28 bp, synthetic construct
  source 1..28: mol_type = other DNA
ccagaaattcttccccagaacgggaggg

SEQ ID NO: 46493 - DNA, 28 bp, synthetic construct
  source 1..28: mol_type = other DNA
accagaaattcttccccagaacgggagg

SEQ ID NO: 46494 - DNA, 28 bp, synthetic construct
  source 1..28: mol_type = other DNA
ggaaccagaaattcttccccagaacggg

SEQ ID NO: 46495 - DNA, 28 bp, synthetic construct
  source 1..28: mol_type = other DNA
aggaaccagaaattcttccccagaacgg

SEQ ID NO: 46496 - DNA, 28 bp, synthetic construct
  source 1..28: mol_type = other DNA
tcctacagtatccactccatcctcaagg

SEQ ID NO: 46497 - DNA, 28 bp, synthetic construct
  source 1..28: mol_type = other DNA
gccttgaggatggagtggatactgtagg

SEQ ID NO: 46498 - DNA, 28 bp, synthetic construct
  source 1..28: mol_type = other DNA
ccactccatcctcaaggcttcccgcagg

SEQ ID NO: 46499 - DNA, 28 bp, synthetic construct
  source 1..28: mol_type = other DNA
cactccatcctcaaggcttcccgcaggg

SEQ ID NO: 46500 - DNA, 28 bp, synthetic construct
  source 1..28: mol_type = other DNA
aaggccctgcgggaagccttgaggatgg

SEQ ID NO: 46501 - DNA, 28 bp, synthetic construct
  source 1..28: mol_type = other DNA
atcctcaaggcttcccgcagggccttgg

SEQ ID NO: 46502 - DNA, 28 bp, synthetic construct
  source 1..28: mol_type = other DNA
tcctcaaggcttcccgcagggccttggg

SEQ ID NO: 46503 - DNA, 28 bp, synthetic construct
  source 1..28: mol_type = other DNA
cctcaaggcttcccgcagggccttgggg

SEQ ID NO: 46504 - DNA, 28 bp, synthetic construct
  source 1..28: mol_type = other DNA
gcaaggcagtgccccaaggccctgcggg

SEQ ID NO: 46505 - DNA, 28 bp, synthetic construct
  source 1..28: mol_type = other DNA
ggcaaggcagtgccccaaggccctgcgg

SEQ ID NO: 46506 - DNA, 28 bp, synthetic construct
  source 1..28: mol_type = other DNA
gggccttggggcactgccttgccatcgg

SEQ ID NO: 46507 - DNA, 28 bp, synthetic construct
  source 1..28: mol_type = other DNA
ggccttggggcactgccttgccatcggg

SEQ ID NO: 46508 - DNA, 28 bp, synthetic construct
  source 1..28: mol_type = other DNA
ggcccgatggcaaggcagtgccccaagg

SEQ ID NO: 46509 - DNA, 28 bp, synthetic construct
  source 1..28: mol_type = other DNA
tgccttgccatcgggcccagttctccgg

SEQ ID NO: 46510 - DNA, 28 bp, synthetic construct
  source 1..28: mol_type = other DNA
gccttgccatcgggcccagttctccggg

SEQ ID NO: 46511 - DNA, 28 bp, synthetic construct
  source 1..28: mol_type = other DNA
gcccggagaactgggcccgatggcaagg

SEQ ID NO: 46512 - DNA, 28 bp, synthetic construct
  source 1..28: mol_type = other DNA
gtggggcccggagaactgggcccgatgg

SEQ ID NO: 46513 - DNA, 28 bp, synthetic construct
  source 1..28: mol_type = other DNA
gggtgcaggtggggcccggagaactggg

SEQ ID NO: 46514 - DNA, 28 bp, synthetic construct
  source 1..28: mol_type = other DNA
ggggtgcaggtggggcccggagaactgg

SEQ ID NO: 46515 - DNA, 28 bp, synthetic construct
  source 1..28: mol_type = other DNA
ggaagaaaggggtgcaggtggggcccgg

SEQ ID NO: 46516 - DNA, 28 bp, synthetic construct
  source 1..28: mol_type = other DNA
cagggggaagaaaggggtgcaggtgggg

SEQ ID NO: 46517 - DNA, 28 bp, synthetic construct
  source 1..28: mol_type = other DNA
ccagggggaagaaaggggtgcaggtggg

SEQ ID NO: 46518 - DNA, 28 bp, synthetic construct
  source 1..28: mol_type = other DNA
ccacctgcacccctttcttccccctggg

SEQ ID NO: 46519 - DNA, 28 bp, synthetic construct
  source 1..28: mol_type = other DNA
tatcccagggggaagaaaggggtgcagg

SEQ ID NO: 46520 - DNA, 28 bp, synthetic construct
  source 1..28: mol_type = other DNA
acatcatatcccagggggaagaaagggg

SEQ ID NO: 46521 - DNA, 28 bp, synthetic construct
  source 1..28: mol_type = other DNA
cacatcatatcccagggggaagaaaggg

SEQ ID NO: 46522 - DNA, 28 bp, synthetic construct
  source 1..28: mol_type = other DNA
acacatcatatcccagggggaagaaagg

SEQ ID NO: 46523 - DNA, 28 bp, synthetic construct
  source 1..28: mol_type = other DNA
tttcttccccctgggatatgatgtgtgg

SEQ ID NO: 46524 - DNA, 28 bp, synthetic construct
  source 1..28: mol_type = other DNA
gaaacaccacacatcatatcccaggggg

SEQ ID NO: 46525 - DNA, 28 bp, synthetic construct
  source 1..28: mol_type = other DNA
ggaaacaccacacatcatatcccagggg

SEQ ID NO: 46526 - DNA, 28 bp, synthetic construct
  source 1..28: mol_type = other DNA
aggaaacaccacacatcatatcccaggg

SEQ ID NO: 46527 - DNA, 28 bp, synthetic construct
  source 1..28: mol_type = other DNA
caggaaacaccacacatcatatcccagg

SEQ ID NO: 46528 - DNA, 28 bp, synthetic construct
  source 1..28: mol_type = other DNA
gggatatgatgtgtggtgtttcctgtgg

SEQ ID NO: 46529 - DNA, 28 bp, synthetic construct
  source 1..28: mol_type = other DNA
tggtgtttcctgtggtaaaagactgagg

SEQ ID NO: 46530 - DNA, 28 bp, synthetic construct
  source 1..28: mol_type = other DNA
gtttcctgtggtaaaagactgaggcagg

SEQ ID NO: 46531 - DNA, 28 bp, synthetic construct
  source 1..28: mol_type = other DNA
ctggcctgcctcagtcttttaccacagg

SEQ ID NO: 46532 - DNA, 28 bp, synthetic construct
  source 1..28: mol_type = other DNA
ctgtggtaaaagactgaggcaggccagg

SEQ ID NO: 46533 - DNA, 28 bp, synthetic construct
  source 1..28: mol_type = other DNA
tgtggtaaaagactgaggcaggccaggg

SEQ ID NO: 46534 - DNA, 28 bp, synthetic construct
  source 1..28: mol_type = other DNA
gtggtaaaagactgaggcaggccagggg

SEQ ID NO: 46535 - DNA, 28 bp, synthetic construct
  source 1..28: mol_type = other DNA
tgggaacatgttactggcagacccctgg

SEQ ID NO: 46536 - DNA, 28 bp, synthetic construct
  source 1..28: mol_type = other DNA
gtgtctgtacatgggaacatgttactgg

SEQ ID NO: 46537 - DNA, 28 bp, synthetic construct
  source 1..28: mol_type = other DNA
agtaacatgttcccatgtacagacacgg

SEQ ID NO: 46538 - DNA, 28 bp, synthetic construct
  source 1..28: mol_type = other DNA
gggtgtggggaccgtgtctgtacatggg

SEQ ID NO: 46539 - DNA, 28 bp, synthetic construct
  source 1..28: mol_type = other DNA
agggtgtggggaccgtgtctgtacatgg

SEQ ID NO: 46540 - DNA, 28 bp, synthetic construct
  source 1..28: mol_type = other DNA
acggtccccacaccctcccagcctcagg

SEQ ID NO: 46541 - DNA, 28 bp, synthetic construct
  source 1..28: mol_type = other DNA
ctgggcctgaggctgggagggtgtgggg

SEQ ID NO: 46542 - DNA, 28 bp, synthetic construct
  source 1..28: mol_type = other DNA
cccacaccctcccagcctcaggcccagg

SEQ ID NO: 46543 - DNA, 28 bp, synthetic construct
  source 1..28: mol_type = other DNA
gcctgggcctgaggctgggagggtgtgg

SEQ ID NO: 46544 - DNA, 28 bp, synthetic construct
  source 1..28: mol_type = other DNA
tgtctgcctgggcctgaggctgggaggg

SEQ ID NO: 46545 - DNA, 28 bp, synthetic construct
  source 1..28: mol_type = other DNA
atgtctgcctgggcctgaggctgggagg

SEQ ID NO: 46546 - DNA, 28 bp, synthetic construct
  source 1..28: mol_type = other DNA
tcccagcctcaggcccaggcagacatgg

SEQ ID NO: 46547 - DNA, 28 bp, synthetic construct
  source 1..28: mol_type = other DNA
cccatgtctgcctgggcctgaggctggg

SEQ ID NO: 46548 - DNA, 28 bp, synthetic construct
  source 1..28: mol_type = other DNA
gcccatgtctgcctgggcctgaggctgg

SEQ ID NO: 46549 - DNA, 28 bp, synthetic construct
  source 1..28: mol_type = other DNA
gctcgcccatgtctgcctgggcctgagg

SEQ ID NO: 46550 - DNA, 28 bp, synthetic construct
  source 1..28: mol_type = other DNA
caggcccaggcagacatgggcgagctgg

SEQ ID NO: 46551 - DNA, 28 bp, synthetic construct
  source 1..28: mol_type = other DNA
ctcaccagctcgcccatgtctgcctggg

SEQ ID NO: 46552 - DNA, 28 bp, synthetic construct
  source 1..28: mol_type = other DNA
tctcaccagctcgcccatgtctgcctgg

SEQ ID NO: 46553 - DNA, 28 bp, synthetic construct
  source 1..28: mol_type = other DNA
ggcgagctggtgagactgccagccacgg

SEQ ID NO: 46554 - DNA, 28 bp, synthetic construct
  source 1..28: mol_type = other DNA
acaggtggctaagcaaagccgtggctgg

SEQ ID NO: 46555 - DNA, 28 bp, synthetic construct
  source 1..28: mol_type = other DNA
agccacggctttgcttagccacctgtgg

SEQ ID NO: 46556 - DNA, 28 bp, synthetic construct
  source 1..28: mol_type = other DNA
ggccacaggtggctaagcaaagccgtgg

SEQ ID NO: 46557 - DNA, 28 bp, synthetic construct
  source 1..28: mol_type = other DNA
ggctttgcttagccacctgtggccgagg

SEQ ID NO: 46558 - DNA, 28 bp, synthetic construct
  source 1..28: mol_type = other DNA
gctttgcttagccacctgtggccgaggg

SEQ ID NO: 46559 - DNA, 28 bp, synthetic construct
  source 1..28: mol_type = other DNA
gtctctgagagccctcggccacaggtgg

SEQ ID NO: 46560 - DNA, 28 bp, synthetic construct
  source 1..28: mol_type = other DNA
ggggtctctgagagccctcggccacagg

SEQ ID NO: 46561 - DNA, 28 bp, synthetic construct
  source 1..28: mol_type = other DNA
ggttaagggggtctctgagagccctcgg

SEQ ID NO: 46562 - DNA, 28 bp, synthetic construct
  source 1..28: mol_type = other DNA
cttcttagtatttgggaggttaaggggg

SEQ ID NO: 46563 - DNA, 28 bp, synthetic construct
  source 1..28: mol_type = other DNA
gcttcttagtatttgggaggttaagggg

SEQ ID NO: 46564 - DNA, 28 bp, synthetic construct
  source 1..28: mol_type = other DNA
agcttcttagtatttgggaggttaaggg

SEQ ID NO: 46565 - DNA, 28 bp, synthetic construct
  source 1..28: mol_type = other DNA
tagcttcttagtatttgggaggttaagg

SEQ ID NO: 46566 - DNA, 28 bp, synthetic construct
  source 1..28: mol_type = other DNA
atattttagcttcttagtatttgggagg

SEQ ID NO: 46567 - DNA, 28 bp, synthetic construct
  source 1..28: mol_type = other DNA
aaaatattttagcttcttagtatttggg

SEQ ID NO: 46568 - DNA, 28 bp, synthetic construct
  source 1..28: mol_type = other DNA
taaaatattttagcttcttagtatttgg

SEQ ID NO: 46569 - DNA, 28 bp, synthetic construct
  source 1..28: mol_type = other DNA
tttaatattttgtttttttttttcttgg

SEQ ID NO: 46570 - DNA, 28 bp, synthetic construct
  source 1..28: mol_type = other DNA
tttcttggtgccagagtttataccctgg

SEQ ID NO: 46571 - DNA, 28 bp, synthetic construct
  source 1..28: mol_type = other DNA
ttcttggtgccagagtttataccctggg

SEQ ID NO: 46572 - DNA, 28 bp, synthetic construct
  source 1..28: mol_type = other DNA
gtgccagagtttataccctgggtgctgg

SEQ ID NO: 46573 - DNA, 28 bp, synthetic construct
  source 1..28: mol_type = other DNA
tgccagagtttataccctgggtgctggg

SEQ ID NO: 46574 - DNA, 28 bp, synthetic construct
  source 1..28: mol_type = other DNA
gccagagtttataccctgggtgctgggg

SEQ ID NO: 46575 - DNA, 28 bp, synthetic construct
  source 1..28: mol_type = other DNA
accccagcacccagggtataaactctgg

SEQ ID NO: 46576 - DNA, 28 bp, synthetic construct
  source 1..28: mol_type = other DNA
taacacagtgcgaccccagcacccaggg

SEQ ID NO: 46577 - DNA, 28 bp, synthetic construct
  source 1..28: mol_type = other DNA
ataacacagtgcgaccccagcacccagg

SEQ ID NO: 46578 - DNA, 28 bp, synthetic construct
  source 1..28: mol_type = other DNA
gtatatatatatattctattttttttgg

SEQ ID NO: 46579 - DNA, 28 bp, synthetic construct
  source 1..28: mol_type = other DNA
atatatatattctattttttttggttgg

SEQ ID NO: 46580 - DNA, 28 bp, synthetic construct
  source 1..28: mol_type = other DNA
tatatatattctattttttttggttggg

SEQ ID NO: 46581 - DNA, 28 bp, synthetic construct
  source 1..28: mol_type = other DNA
tcgtttttaattcagtcctacaaaatgg

SEQ ID NO: 46582 - DNA, 28 bp, synthetic construct
  source 1..28: mol_type = other DNA
tttttaattcagtcctacaaaatggtgg

SEQ ID NO: 46583 - DNA, 28 bp, synthetic construct
  source 1..28: mol_type = other DNA
agactggggcttaccaccattttgtagg

SEQ ID NO: 46584 - DNA, 28 bp, synthetic construct
  source 1..28: mol_type = other DNA
caaaatggtggtaagccccagtctcagg

SEQ ID NO: 46585 - DNA, 28 bp, synthetic construct
  source 1..28: mol_type = other DNA
aaaatggtggtaagccccagtctcaggg

SEQ ID NO: 46586 - DNA, 28 bp, synthetic construct
  source 1..28: mol_type = other DNA
aaatggtggtaagccccagtctcagggg

SEQ ID NO: 46587 - DNA, 28 bp, synthetic construct
  source 1..28: mol_type = other DNA
taagacagggtgacccctgagactgggg

SEQ ID NO: 46588 - DNA, 28 bp, synthetic construct
  source 1..28: mol_type = other DNA
ctaagacagggtgacccctgagactggg

SEQ ID NO: 46589 - DNA, 28 bp, synthetic construct
  source 1..28: mol_type = other DNA
tctaagacagggtgacccctgagactgg

SEQ ID NO: 46590 - DNA, 28 bp, synthetic construct
  source 1..28: mol_type = other DNA
tcaccctgtcttagagctagagatgagg

SEQ ID NO: 46591 - DNA, 28 bp, synthetic construct
  source 1..28: mol_type = other DNA
ccctgtcttagagctagagatgaggtgg

SEQ ID NO: 46592 - DNA, 28 bp, synthetic construct
  source 1..28: mol_type = other DNA
gccacctcatctctagctctaagacagg

SEQ ID NO: 46593 - DNA, 28 bp, synthetic construct
  source 1..28: mol_type = other DNA
gtcttagagctagagatgaggtggcagg

SEQ ID NO: 46594 - DNA, 28 bp, synthetic construct
  source 1..28: mol_type = other DNA
tcttagagctagagatgaggtggcaggg

SEQ ID NO: 46595 - DNA, 28 bp, synthetic construct
  source 1..28: mol_type = other DNA
tagagctagagatgaggtggcagggagg

SEQ ID NO: 46596 - DNA, 28 bp, synthetic construct
  source 1..28: mol_type = other DNA
agagctagagatgaggtggcagggaggg

SEQ ID NO: 46597 - DNA, 28 bp, synthetic construct
  source 1..28: mol_type = other DNA
gctagagatgaggtggcagggagggagg

SEQ ID NO: 46598 - DNA, 28 bp, synthetic construct
  source 1..28: mol_type = other DNA
gcagggagggaggctgtgtcctcagtgg

SEQ ID NO: 46599 - DNA, 28 bp, synthetic construct
  source 1..28: mol_type = other DNA
gagggaggctgtgtcctcagtggcctgg

SEQ ID NO: 46600 - DNA, 28 bp, synthetic construct
  source 1..28: mol_type = other DNA
agggaggctgtgtcctcagtggcctggg

SEQ ID NO: 46601 - DNA, 28 bp, synthetic construct
  source 1..28: mol_type = other DNA
gggaggctgtgtcctcagtggcctgggg

SEQ ID NO: 46602 - DNA, 28 bp, synthetic construct
  source 1..28: mol_type = other DNA
aggtctgctcagccccaggccactgagg

SEQ ID NO: 46603 - DNA, 28 bp, synthetic construct
  source 1..28: mol_type = other DNA
agtggcctggggctgagcagaccttagg

SEQ ID NO: 46604 - DNA, 28 bp, synthetic construct
  source 1..28: mol_type = other DNA
gcctggggctgagcagaccttaggaagg

SEQ ID NO: 46605 - DNA, 28 bp, synthetic construct
  source 1..28: mol_type = other DNA
cctggggctgagcagaccttaggaaggg

SEQ ID NO: 46606 - DNA, 28 bp, synthetic construct
  source 1..28: mol_type = other DNA
ctggggctgagcagaccttaggaagggg

SEQ ID NO: 46607 - DNA, 28 bp, synthetic construct
  source 1..28: mol_type = other DNA
cggcactggggagggccccttcctaagg

SEQ ID NO: 46608 - DNA, 28 bp, synthetic construct
  source 1..28: mol_type = other DNA
taggaaggggccctccccagtgccgtgg

SEQ ID NO: 46609 - DNA, 28 bp, synthetic construct
  source 1..28: mol_type = other DNA
gccctccccagtgccgtggctgctctgg

SEQ ID NO: 46610 - DNA, 28 bp, synthetic construct
  source 1..28: mol_type = other DNA
cccagagcagccacggcactggggaggg

SEQ ID NO: 46611 - DNA, 28 bp, synthetic construct
  source 1..28: mol_type = other DNA
ccccagagcagccacggcactggggagg

SEQ ID NO: 46612 - DNA, 28 bp, synthetic construct
  source 1..28: mol_type = other DNA
tagccccagagcagccacggcactgggg

SEQ ID NO: 46613 - DNA, 28 bp, synthetic construct
  source 1..28: mol_type = other DNA
gtagccccagagcagccacggcactggg

SEQ ID NO: 46614 - DNA, 28 bp, synthetic construct
  source 1..28: mol_type = other DNA
ggtagccccagagcagccacggcactgg

SEQ ID NO: 46615 - DNA, 28 bp, synthetic construct
  source 1..28: mol_type = other DNA
gccgtggctgctctggggctaccccagg

SEQ ID NO: 46616 - DNA, 28 bp, synthetic construct
  source 1..28: mol_type = other DNA
acctggggtagccccagagcagccacgg

SEQ ID NO: 46617 - DNA, 28 bp, synthetic construct
  source 1..28: mol_type = other DNA
ctctggggctaccccaggtgaacagagg

SEQ ID NO: 46618 - DNA, 28 bp, synthetic construct
  source 1..28: mol_type = other DNA
tggggctaccccaggtgaacagaggtgg

SEQ ID NO: 46619 - DNA, 28 bp, synthetic construct
  source 1..28: mol_type = other DNA
gcatctcaccacctctgttcacctgggg

SEQ ID NO: 46620 - DNA, 28 bp, synthetic construct
  source 1..28: mol_type = other DNA
cgcatctcaccacctctgttcacctggg

SEQ ID NO: 46621 - DNA, 28 bp, synthetic construct
  source 1..28: mol_type = other DNA
gcgcatctcaccacctctgttcacctgg

SEQ ID NO: 46622 - DNA, 28 bp, synthetic construct
  source 1..28: mol_type = other DNA
ggtgaacagaggtggtgagatgcgcagg

SEQ ID NO: 46623 - DNA, 28 bp, synthetic construct
  source 1..28: mol_type = other DNA
gtgaacagaggtggtgagatgcgcaggg

SEQ ID NO: 46624 - DNA, 28 bp, synthetic construct
  source 1..28: mol_type = other DNA
tgcgcagggaagaccagctctctccagg

SEQ ID NO: 46625 - DNA, 28 bp, synthetic construct
  source 1..28: mol_type = other DNA
ggaagaccagctctctccaggacatcgg

SEQ ID NO: 46626 - DNA, 28 bp, synthetic construct
  source 1..28: mol_type = other DNA
gaagaccagctctctccaggacatcggg

SEQ ID NO: 46627 - DNA, 28 bp, synthetic construct
  source 1..28: mol_type = other DNA
cgcagcccgatgtcctggagagagctgg

SEQ ID NO: 46628 - DNA, 28 bp, synthetic construct
  source 1..28: mol_type = other DNA
ctggacttcacgcagcccgatgtcctgg

SEQ ID NO: 46629 - DNA, 28 bp, synthetic construct
  source 1..28: mol_type = other DNA
ggctgcgtgaagtccagtgaccctgagg

SEQ ID NO: 46630 - DNA, 28 bp, synthetic construct
  source 1..28: mol_type = other DNA
gctgcgtgaagtccagtgaccctgaggg

SEQ ID NO: 46631 - DNA, 28 bp, synthetic construct
  source 1..28: mol_type = other DNA
ctgcgtgaagtccagtgaccctgagggg

SEQ ID NO: 46632 - DNA, 28 bp, synthetic construct
  source 1..28: mol_type = other DNA
aagtccagtgaccctgaggggattttgg

SEQ ID NO: 46633 - DNA, 28 bp, synthetic construct
  source 1..28: mol_type = other DNA
ttggccaaaatcccctcagggtcactgg

SEQ ID NO: 46634 - DNA, 28 bp, synthetic construct
  source 1..28: mol_type = other DNA
gtgaccctgaggggattttggccaaagg

SEQ ID NO: 46635 - DNA, 28 bp, synthetic construct
  source 1..28: mol_type = other DNA
gtttcctttggccaaaatcccctcaggg

SEQ ID NO: 46636 - DNA, 28 bp, synthetic construct
  source 1..28: mol_type = other DNA
tgtttcctttggccaaaatcccctcagg

SEQ ID NO: 46637 - DNA, 28 bp, synthetic construct
  source 1..28: mol_type = other DNA
gggattttggccaaaggaaacagccagg

SEQ ID NO: 46638 - DNA, 28 bp, synthetic construct
  source 1..28: mol_type = other DNA
ggattttggccaaaggaaacagccaggg

SEQ ID NO: 46639 - DNA, 28 bp, synthetic construct
  source 1..28: mol_type = other DNA
tttggccaaaggaaacagccagggctgg

SEQ ID NO: 46640 - DNA, 28 bp, synthetic construct
  source 1..28: mol_type = other DNA
ttggccaaaggaaacagccagggctggg

SEQ ID NO: 46641 - DNA, 28 bp, synthetic construct
  source 1..28: mol_type = other DNA
ctagcccagccctggctgtttcctttgg

SEQ ID NO: 46642 - DNA, 28 bp, synthetic construct
  source 1..28: mol_type = other DNA
caaaggaaacagccagggctgggctagg

SEQ ID NO: 46643 - DNA, 28 bp, synthetic construct
  source 1..28: mol_type = other DNA
acagccagggctgggctaggagagctgg

SEQ ID NO: 46644 - DNA, 28 bp, synthetic construct
  source 1..28: mol_type = other DNA
cagccagggctgggctaggagagctggg

SEQ ID NO: 46645 - DNA, 28 bp, synthetic construct
  source 1..28: mol_type = other DNA
agccagggctgggctaggagagctgggg

SEQ ID NO: 46646 - DNA, 28 bp, synthetic construct
  source 1..28: mol_type = other DNA
gaccccagctctcctagcccagccctgg

SEQ ID NO: 46647 - DNA, 28 bp, synthetic construct
  source 1..28: mol_type = other DNA
gctgccccacccactctccctcacatgg

SEQ ID NO: 46648 - DNA, 28 bp, synthetic construct
  source 1..28: mol_type = other DNA
agcaccatgtgagggagagtgggtgggg

SEQ ID NO: 46649 - DNA, 28 bp, synthetic construct
  source 1..28: mol_type = other DNA
tagcaccatgtgagggagagtgggtggg

SEQ ID NO: 46650 - DNA, 28 bp, synthetic construct
  source 1..28: mol_type = other DNA
ctagcaccatgtgagggagagtgggtgg

SEQ ID NO: 46651 - DNA, 28 bp, synthetic construct
  source 1..28: mol_type = other DNA
cacccactctccctcacatggtgctagg

SEQ ID NO: 46652 - DNA, 28 bp, synthetic construct
  source 1..28: mol_type = other DNA
agcctagcaccatgtgagggagagtggg

SEQ ID NO: 46653 - DNA, 28 bp, synthetic construct
  source 1..28: mol_type = other DNA
cagcctagcaccatgtgagggagagtgg

SEQ ID NO: 46654 - DNA, 28 bp, synthetic construct
  source 1..28: mol_type = other DNA
cactctccctcacatggtgctaggctgg

SEQ ID NO: 46655 - DNA, 28 bp, synthetic construct
  source 1..28: mol_type = other DNA
actctccctcacatggtgctaggctggg

SEQ ID NO: 46656 - DNA, 28 bp, synthetic construct
  source 1..28: mol_type = other DNA
cagctcccagcctagcaccatgtgaggg

SEQ ID NO: 46657 - DNA, 28 bp, synthetic construct
  source 1..28: mol_type = other DNA
gcagctcccagcctagcaccatgtgagg

SEQ ID NO: 46658 - DNA, 28 bp, synthetic construct
  source 1..28: mol_type = other DNA
ctaggctgggagctgccctgagagctgg

SEQ ID NO: 46659 - DNA, 28 bp, synthetic construct
  source 1..28: mol_type = other DNA
taggctgggagctgccctgagagctggg

SEQ ID NO: 46660 - DNA, 28 bp, synthetic construct
  source 1..28: mol_type = other DNA
gccctgagagctgggatgcccaccaagg

SEQ ID NO: 46661 - DNA, 28 bp, synthetic construct
  source 1..28: mol_type = other DNA
gccttggtgggcatcccagctctcaggg

SEQ ID NO: 46662 - DNA, 28 bp, synthetic construct
  source 1..28: mol_type = other DNA
ggccttggtgggcatcccagctctcagg

SEQ ID NO: 46663 - DNA, 28 bp, synthetic construct
  source 1..28: mol_type = other DNA
tggagacagttctgtgggccttggtggg

SEQ ID NO: 46664 - DNA, 28 bp, synthetic construct
  source 1..28: mol_type = other DNA
ctggagacagttctgtgggccttggtgg

SEQ ID NO: 46665 - DNA, 28 bp, synthetic construct
  source 1..28: mol_type = other DNA
caccaaggcccacagaactgtctccagg

SEQ ID NO: 46666 - DNA, 28 bp, synthetic construct
  source 1..28: mol_type = other DNA
ggcctggagacagttctgtgggccttgg

SEQ ID NO: 46667 - DNA, 28 bp, synthetic construct
  source 1..28: mol_type = other DNA
tacaagggcctggagacagttctgtggg

SEQ ID NO: 46668 - DNA, 28 bp, synthetic construct
  source 1..28: mol_type = other DNA
ctacaagggcctggagacagttctgtgg

SEQ ID NO: 46669 - DNA, 28 bp, synthetic construct
  source 1..28: mol_type = other DNA
actgtctccaggcccttgtagacagtgg

SEQ ID NO: 46670 - DNA, 28 bp, synthetic construct
  source 1..28: mol_type = other DNA
ctgtctccaggcccttgtagacagtggg

SEQ ID NO: 46671 - DNA, 28 bp, synthetic construct
  source 1..28: mol_type = other DNA
agagatcccactgtctacaagggcctgg

SEQ ID NO: 46672 - DNA, 28 bp, synthetic construct
  source 1..28: mol_type = other DNA
aggcccttgtagacagtgggatctctgg

SEQ ID NO: 46673 - DNA, 28 bp, synthetic construct
  source 1..28: mol_type = other DNA
ggcccttgtagacagtgggatctctggg

SEQ ID NO: 46674 - DNA, 28 bp, synthetic construct
  source 1..28: mol_type = other DNA
agcccagagatcccactgtctacaaggg

SEQ ID NO: 46675 - DNA, 28 bp, synthetic construct
  source 1..28: mol_type = other DNA
cagcccagagatcccactgtctacaagg

SEQ ID NO: 46676 - DNA, 28 bp, synthetic construct
  source 1..28: mol_type = other DNA
acagtgggatctctgggctgatttctgg

SEQ ID NO: 46677 - DNA, 28 bp, synthetic construct
  source 1..28: mol_type = other DNA
tgggatctctgggctgatttctggttgg

SEQ ID NO: 46678 - DNA, 28 bp, synthetic construct
  source 1..28: mol_type = other DNA
gggatctctgggctgatttctggttggg

SEQ ID NO: 46679 - DNA, 28 bp, synthetic construct
  source 1..28: mol_type = other DNA
ggatctctgggctgatttctggttgggg

SEQ ID NO: 46680 - DNA, 28 bp, synthetic construct
  source 1..28: mol_type = other DNA
ttcacattgttaaatggggtggggtagg

SEQ ID NO: 46681 - DNA, 28 bp, synthetic construct
  source 1..28: mol_type = other DNA
tcacttcacattgttaaatggggtgggg

SEQ ID NO: 46682 - DNA, 28 bp, synthetic construct
  source 1..28: mol_type = other DNA
gtcacttcacattgttaaatggggtggg

SEQ ID NO: 46683 - DNA, 28 bp, synthetic construct
  source 1..28: mol_type = other DNA
agtcacttcacattgttaaatggggtgg

SEQ ID NO: 46684 - DNA, 28 bp, synthetic construct
  source 1..28: mol_type = other DNA
ctcagtcacttcacattgttaaatgggg

SEQ ID NO: 46685 - DNA, 28 bp, synthetic construct
  source 1..28: mol_type = other DNA
cctcagtcacttcacattgttaaatggg

SEQ ID NO: 46686 - DNA, 28 bp, synthetic construct
  source 1..28: mol_type = other DNA
gcctcagtcacttcacattgttaaatgg

SEQ ID NO: 46687 - DNA, 28 bp, synthetic construct
  source 1..28: mol_type = other DNA
tttaacaatgtgaagtgactgaggctgg

SEQ ID NO: 46688 - DNA, 28 bp, synthetic construct
  source 1..28: mol_type = other DNA
ttaacaatgtgaagtgactgaggctggg

SEQ ID NO: 46689 - DNA, 28 bp, synthetic construct
  source 1..28: mol_type = other DNA
taacaatgtgaagtgactgaggctgggg

SEQ ID NO: 46690 - DNA, 28 bp, synthetic construct
  source 1..28: mol_type = other DNA
tgactgaggctggggtgcctctccctgg

SEQ ID NO: 46691 - DNA, 28 bp, synthetic construct
  source 1..28: mol_type = other DNA
ttggcagttggagggggccagggagagg

SEQ ID NO: 46692 - DNA, 28 bp, synthetic construct
  source 1..28: mol_type = other DNA
agaatttggcagttggagggggccaggg

SEQ ID NO: 46693 - DNA, 28 bp, synthetic construct
  source 1..28: mol_type = other DNA
cagaatttggcagttggagggggccagg

SEQ ID NO: 46694 - DNA, 28 bp, synthetic construct
  source 1..28: mol_type = other DNA
ggaagcagaatttggcagttggaggggg

SEQ ID NO: 46695 - DNA, 28 bp, synthetic construct
  source 1..28: mol_type = other DNA
gggaagcagaatttggcagttggagggg

SEQ ID NO: 46696 - DNA, 28 bp, synthetic construct
  source 1..28: mol_type = other DNA
agggaagcagaatttggcagttggaggg

SEQ ID NO: 46697 - DNA, 28 bp, synthetic construct
  source 1..28: mol_type = other DNA
gagggaagcagaatttggcagttggagg

SEQ ID NO: 46698 - DNA, 28 bp, synthetic construct
  source 1..28: mol_type = other DNA
tcagagggaagcagaatttggcagttgg

SEQ ID NO: 46699 - DNA, 28 bp, synthetic construct
  source 1..28: mol_type = other DNA
ctggggttcagagggaagcagaatttgg

SEQ ID NO: 46700 - DNA, 28 bp, synthetic construct
  source 1..28: mol_type = other DNA
caaattctgcttccctctgaaccccagg

SEQ ID NO: 46701 - DNA, 28 bp, synthetic construct
  source 1..28: mol_type = other DNA
cagaaagtatttcctggggttcagaggg

SEQ ID NO: 46702 - DNA, 28 bp, synthetic construct
  source 1..28: mol_type = other DNA
cctctgaaccccaggaaatactttctgg

SEQ ID NO: 46703 - DNA, 28 bp, synthetic construct
  source 1..28: mol_type = other DNA
gaaccccaggaaatactttctggagagg

SEQ ID NO: 46704 - DNA, 28 bp, synthetic construct
  source 1..28: mol_type = other DNA
aagcctctccagaaagtatttcctgggg

SEQ ID NO: 46705 - DNA, 28 bp, synthetic construct
  source 1..28: mol_type = other DNA
caagcctctccagaaagtatttcctggg

SEQ ID NO: 46706 - DNA, 28 bp, synthetic construct
  source 1..28: mol_type = other DNA
acaagcctctccagaaagtatttcctgg

SEQ ID NO: 46707 - DNA, 28 bp, synthetic construct
  source 1..28: mol_type = other DNA
tcttgttcagaagactctagcatcttgg

SEQ ID NO: 46708 - DNA, 28 bp, synthetic construct
  source 1..28: mol_type = other DNA
cttgttcagaagactctagcatcttggg

SEQ ID NO: 46709 - DNA, 28 bp, synthetic construct
  source 1..28: mol_type = other DNA
ttgttcagaagactctagcatcttgggg

SEQ ID NO: 46710 - DNA, 28 bp, synthetic construct
  source 1..28: mol_type = other DNA
tcagaagactctagcatcttggggctgg

SEQ ID NO: 46711 - DNA, 28 bp, synthetic construct
  source 1..28: mol_type = other DNA
aagactctagcatcttggggctggaagg

SEQ ID NO: 46712 - DNA, 28 bp, synthetic construct
  source 1..28: mol_type = other DNA
atcttggggctggaaggtcctttgacgg

SEQ ID NO: 46713 - DNA, 28 bp, synthetic construct
  source 1..28: mol_type = other DNA
tcttggggctggaaggtcctttgacggg

SEQ ID NO: 46714 - DNA, 28 bp, synthetic construct
  source 1..28: mol_type = other DNA
gaaggtcctttgacgggtatgaaacagg

SEQ ID NO: 46715 - DNA, 28 bp, synthetic construct
  source 1..28: mol_type = other DNA
tctggacctgtttcatacccgtcaaagg

SEQ ID NO: 46716 - DNA, 28 bp, synthetic construct
  source 1..28: mol_type = other DNA
tgacgggtatgaaacaggtccagaaagg

SEQ ID NO: 46717 - DNA, 28 bp, synthetic construct
  source 1..28: mol_type = other DNA
gacgggtatgaaacaggtccagaaaggg

SEQ ID NO: 46718 - DNA, 28 bp, synthetic construct
  source 1..28: mol_type = other DNA
acgggtatgaaacaggtccagaaagggg

SEQ ID NO: 46719 - DNA, 28 bp, synthetic construct
  source 1..28: mol_type = other DNA
ggtatgaaacaggtccagaaaggggagg

SEQ ID NO: 46720 - DNA, 28 bp, synthetic construct
  source 1..28: mol_type = other DNA
atgaaacaggtccagaaaggggaggtgg

SEQ ID NO: 46721 - DNA, 28 bp, synthetic construct
  source 1..28: mol_type = other DNA
gtccagaaaggggaggtggcctgcttgg

SEQ ID NO: 46722 - DNA, 28 bp, synthetic construct
  source 1..28: mol_type = other DNA
ggccaagcaggccacctcccctttctgg

SEQ ID NO: 46723 - DNA, 28 bp, synthetic construct
  source 1..28: mol_type = other DNA
gaggtggcctgcttggccgacgtcatgg

SEQ ID NO: 46724 - DNA, 28 bp, synthetic construct
  source 1..28: mol_type = other DNA
gctggctccatgacgtcggccaagcagg

SEQ ID NO: 46725 - DNA, 28 bp, synthetic construct
  source 1..28: mol_type = other DNA
gcttggccgacgtcatggagccagctgg

SEQ ID NO: 46726 - DNA, 28 bp, synthetic construct
  source 1..28: mol_type = other DNA
cttggccgacgtcatggagccagctggg

SEQ ID NO: 46727 - DNA, 28 bp, synthetic construct
  source 1..28: mol_type = other DNA
ctgctcccagctggctccatgacgtcgg

SEQ ID NO: 46728 - DNA, 28 bp, synthetic construct
  source 1..28: mol_type = other DNA
cgacgtcatggagccagctgggagcagg

SEQ ID NO: 46729 - DNA, 28 bp, synthetic construct
  source 1..28: mol_type = other DNA
gacgtcatggagccagctgggagcaggg

SEQ ID NO: 46730 - DNA, 28 bp, synthetic construct
  source 1..28: mol_type = other DNA
ttcaacgctcagccctgctcccagctgg

SEQ ID NO: 46731 - DNA, 28 bp, synthetic construct
  source 1..28: mol_type = other DNA
ggagcagggctgagcgttgaacccgagg

SEQ ID NO: 46732 - DNA, 28 bp, synthetic construct
  source 1..28: mol_type = other DNA
ggctgagcgttgaacccgaggctcccgg

SEQ ID NO: 46733 - DNA, 28 bp, synthetic construct
  source 1..28: mol_type = other DNA
gatgggacttggaaccgggagcctcggg

SEQ ID NO: 46734 - DNA, 28 bp, synthetic construct
  source 1..28: mol_type = other DNA
cgatgggacttggaaccgggagcctcgg

SEQ ID NO: 46735 - DNA, 28 bp, synthetic construct
  source 1..28: mol_type = other DNA
gaggagcacgatgggacttggaaccggg

SEQ ID NO: 46736 - DNA, 28 bp, synthetic construct
  source 1..28: mol_type = other DNA
agaggagcacgatgggacttggaaccgg

SEQ ID NO: 46737 - DNA, 28 bp, synthetic construct
  source 1..28: mol_type = other DNA
attggaagaggagcacgatgggacttgg

SEQ ID NO: 46738 - DNA, 28 bp, synthetic construct
  source 1..28: mol_type = other DNA
tgtggcattggaagaggagcacgatggg

SEQ ID NO: 46739 - DNA, 28 bp, synthetic construct
  source 1..28: mol_type = other DNA
gtgtggcattggaagaggagcacgatgg

SEQ ID NO: 46740 - DNA, 28 bp, synthetic construct
  source 1..28: mol_type = other DNA
ctcagaggcagtgtggcattggaagagg

SEQ ID NO: 46741 - DNA, 28 bp, synthetic construct
  source 1..28: mol_type = other DNA
gatgggctcagaggcagtgtggcattgg

SEQ ID NO: 46742 - DNA, 28 bp, synthetic construct
  source 1..28: mol_type = other DNA
gccacactgcctctgagcccatccttgg

SEQ ID NO: 46743 - DNA, 28 bp, synthetic construct
  source 1..28: mol_type = other DNA
cccaaggatgggctcagaggcagtgtgg

SEQ ID NO: 46744 - DNA, 28 bp, synthetic construct
  source 1..28: mol_type = other DNA
agtagggtcccaaggatgggctcagagg

SEQ ID NO: 46745 - DNA, 28 bp, synthetic construct
  source 1..28: mol_type = other DNA
tggcacagagtagggtcccaaggatggg

SEQ ID NO: 46746 - DNA, 28 bp, synthetic construct
  source 1..28: mol_type = other DNA
ctggcacagagtagggtcccaaggatgg

SEQ ID NO: 46747 - DNA, 28 bp, synthetic construct
  source 1..28: mol_type = other DNA
catccttgggaccctactctgtgccagg

SEQ ID NO: 46748 - DNA, 28 bp, synthetic construct
  source 1..28: mol_type = other DNA
gaacctggcacagagtagggtcccaagg

SEQ ID NO: 46749 - DNA, 28 bp, synthetic construct
  source 1..28: mol_type = other DNA
agggacaggaacctggcacagagtaggg

SEQ ID NO: 46750 - DNA, 28 bp, synthetic construct
  source 1..28: mol_type = other DNA
aagggacaggaacctggcacagagtagg

SEQ ID NO: 46751 - DNA, 28 bp, synthetic construct
  source 1..28: mol_type = other DNA
tgtgacggaggaagggacaggaacctgg

SEQ ID NO: 46752 - DNA, 28 bp, synthetic construct
  source 1..28: mol_type = other DNA
tcctgtcccttcctccgtcacagcatgg

SEQ ID NO: 46753 - DNA, 28 bp, synthetic construct
  source 1..28: mol_type = other DNA
accatgctgtgacggaggaagggacagg

SEQ ID NO: 46754 - DNA, 28 bp, synthetic construct
  source 1..28: mol_type = other DNA
gaatgaccatgctgtgacggaggaaggg

SEQ ID NO: 46755 - DNA, 28 bp, synthetic construct
  source 1..28: mol_type = other DNA
ggaatgaccatgctgtgacggaggaagg

SEQ ID NO: 46756 - DNA, 28 bp, synthetic construct
  source 1..28: mol_type = other DNA
tcctccgtcacagcatggtcattccagg

SEQ ID NO: 46757 - DNA, 28 bp, synthetic construct
  source 1..28: mol_type = other DNA
tcctggaatgaccatgctgtgacggagg

SEQ ID NO: 46758 - DNA, 28 bp, synthetic construct
  source 1..28: mol_type = other DNA
atatcctggaatgaccatgctgtgacgg

SEQ ID NO: 46759 - DNA, 28 bp, synthetic construct
  source 1..28: mol_type = other DNA
gtcacagcatggtcattccaggatatgg

SEQ ID NO: 46760 - DNA, 28 bp, synthetic construct
  source 1..28: mol_type = other DNA
tcacagcatggtcattccaggatatggg

SEQ ID NO: 46761 - DNA, 28 bp, synthetic construct
  source 1..28: mol_type = other DNA
cacagcatggtcattccaggatatgggg

SEQ ID NO: 46762 - DNA, 28 bp, synthetic construct
  source 1..28: mol_type = other DNA
gaaggagtggtttgtccccatatcctgg

SEQ ID NO: 46763 - DNA, 28 bp, synthetic construct
  source 1..28: mol_type = other DNA
ggggacaaaccactccttcccagccagg

SEQ ID NO: 46764 - DNA, 28 bp, synthetic construct
  source 1..28: mol_type = other DNA
gggacaaaccactccttcccagccaggg

SEQ ID NO: 46765 - DNA, 28 bp, synthetic construct
  source 1..28: mol_type = other DNA
caaaggcaccctggctgggaaggagtgg

SEQ ID NO: 46766 - DNA, 28 bp, synthetic construct
  source 1..28: mol_type = other DNA
aggctcaaaggcaccctggctgggaagg

SEQ ID NO: 46767 - DNA, 28 bp, synthetic construct
  source 1..28: mol_type = other DNA
gagaaggctcaaaggcaccctggctggg

SEQ ID NO: 46768 - DNA, 28 bp, synthetic construct
  source 1..28: mol_type = other DNA
tgagaaggctcaaaggcaccctggctgg

SEQ ID NO: 46769 - DNA, 28 bp, synthetic construct
  source 1..28: mol_type = other DNA
ggaatgagaaggctcaaaggcaccctgg

SEQ ID NO: 46770 - DNA, 28 bp, synthetic construct
  source 1..28: mol_type = other DNA
ggtgcctttgagccttctcattccgagg

SEQ ID NO: 46771 - DNA, 28 bp, synthetic construct
  source 1..28: mol_type = other DNA
cagacctcggaatgagaaggctcaaagg

SEQ ID NO: 46772 - DNA, 28 bp, synthetic construct
  source 1..28: mol_type = other DNA
tgcaaacgcagacctcggaatgagaagg

SEQ ID NO: 46773 - DNA, 28 bp, synthetic construct
  source 1..28: mol_type = other DNA
acgacagggatgcaaacgcagacctcgg

SEQ ID NO: 46774 - DNA, 28 bp, synthetic construct
  source 1..28: mol_type = other DNA
tgcatccctgtcgtgttctccctcgagg

SEQ ID NO: 46775 - DNA, 28 bp, synthetic construct
  source 1..28: mol_type = other DNA
gcatccctgtcgtgttctccctcgaggg

SEQ ID NO: 46776 - DNA, 28 bp, synthetic construct
  source 1..28: mol_type = other DNA
catccctgtcgtgttctccctcgagggg

SEQ ID NO: 46777 - DNA, 28 bp, synthetic construct
  source 1..28: mol_type = other DNA
ggacccctcgagggagaacacgacaggg

SEQ ID NO: 46778 - DNA, 28 bp, synthetic construct
  source 1..28: mol_type = other DNA
aggacccctcgagggagaacacgacagg

SEQ ID NO: 46779 - DNA, 28 bp, synthetic construct
  source 1..28: mol_type = other DNA
cacaggctggggaaggacccctcgaggg

SEQ ID NO: 46780 - DNA, 28 bp, synthetic construct
  source 1..28: mol_type = other DNA
cctcgaggggtccttccccagcctgtgg

SEQ ID NO: 46781 - DNA, 28 bp, synthetic construct
  source 1..28: mol_type = other DNA
ctcgaggggtccttccccagcctgtggg

SEQ ID NO: 46782 - DNA, 28 bp, synthetic construct
  source 1..28: mol_type = other DNA
tcgaggggtccttccccagcctgtgggg

SEQ ID NO: 46783 - DNA, 28 bp, synthetic construct
  source 1..28: mol_type = other DNA
cgaggggtccttccccagcctgtggggg

SEQ ID NO: 46784 - DNA, 28 bp, synthetic construct
  source 1..28: mol_type = other DNA
ggtccttccccagcctgtgggggcctgg

SEQ ID NO: 46785 - DNA, 28 bp, synthetic construct
  source 1..28: mol_type = other DNA
gtccttccccagcctgtgggggcctggg

SEQ ID NO: 46786 - DNA, 28 bp, synthetic construct
  source 1..28: mol_type = other DNA
gacccaggcccccacaggctggggaagg

SEQ ID NO: 46787 - DNA, 28 bp, synthetic construct
  source 1..28: mol_type = other DNA
aacagacccaggcccccacaggctgggg

SEQ ID NO: 46788 - DNA, 28 bp, synthetic construct
  source 1..28: mol_type = other DNA
gaacagacccaggcccccacaggctggg

SEQ ID NO: 46789 - DNA, 28 bp, synthetic construct
  source 1..28: mol_type = other DNA
agaacagacccaggcccccacaggctgg

SEQ ID NO: 46790 - DNA, 28 bp, synthetic construct
  source 1..28: mol_type = other DNA
gctcagaacagacccaggcccccacagg

SEQ ID NO: 46791 - DNA, 28 bp, synthetic construct
  source 1..28: mol_type = other DNA
aagggaatcagctcagaacagacccagg

SEQ ID NO: 46792 - DNA, 28 bp, synthetic construct
  source 1..28: mol_type = other DNA
gattcccttttctccagttctctgctgg

SEQ ID NO: 46793 - DNA, 28 bp, synthetic construct
  source 1..28: mol_type = other DNA
attcccttttctccagttctctgctggg

SEQ ID NO: 46794 - DNA, 28 bp, synthetic construct
  source 1..28: mol_type = other DNA
catcccagcagagaactggagaaaaggg

SEQ ID NO: 46795 - DNA, 28 bp, synthetic construct
  source 1..28: mol_type = other DNA
tcatcccagcagagaactggagaaaagg

SEQ ID NO: 46796 - DNA, 28 bp, synthetic construct
  source 1..28: mol_type = other DNA
aactttcttcatcccagcagagaactgg

SEQ ID NO: 46797 - DNA, 28 bp, synthetic construct
  source 1..28: mol_type = other DNA
agttctctgctgggatgaagaaagttgg

SEQ ID NO: 46798 - DNA, 28 bp, synthetic construct
  source 1..28: mol_type = other DNA
gggatgaagaaagttggacactcagtgg

SEQ ID NO: 46799 - DNA, 28 bp, synthetic construct
  source 1..28: mol_type = other DNA
ggatgaagaaagttggacactcagtggg

SEQ ID NO: 46800 - DNA, 28 bp, synthetic construct
  source 1..28: mol_type = other DNA
ttggacactcagtgggaccagctgcagg

SEQ ID NO: 46801 - DNA, 28 bp, synthetic construct
  source 1..28: mol_type = other DNA
gacactcagtgggaccagctgcaggtgg

SEQ ID NO: 46802 - DNA, 28 bp, synthetic construct
  source 1..28: mol_type = other DNA
tgtacacagtgaaaccacctgcagctgg

SEQ ID NO: 46803 - DNA, 28 bp, synthetic construct
  source 1..28: mol_type = other DNA
gcagtgtccccatcatgcctctcaatgg

SEQ ID NO: 46804 - DNA, 28 bp, synthetic construct
  source 1..28: mol_type = other DNA
cagtgtccccatcatgcctctcaatggg

SEQ ID NO: 46805 - DNA, 28 bp, synthetic construct
  source 1..28: mol_type = other DNA
agtgtccccatcatgcctctcaatgggg

SEQ ID NO: 46806 - DNA, 28 bp, synthetic construct
  source 1..28: mol_type = other DNA
gcaggccccattgagaggcatgatgggg

SEQ ID NO: 46807 - DNA, 28 bp, synthetic construct
  source 1..28: mol_type = other DNA
tgcaggccccattgagaggcatgatggg

SEQ ID NO: 46808 - DNA, 28 bp, synthetic construct
  source 1..28: mol_type = other DNA
ttgcaggccccattgagaggcatgatgg

SEQ ID NO: 46809 - DNA, 28 bp, synthetic construct
  source 1..28: mol_type = other DNA
tgcctctcaatggggcctgcaagcctgg

SEQ ID NO: 46810 - DNA, 28 bp, synthetic construct
  source 1..28: mol_type = other DNA
gcctctcaatggggcctgcaagcctggg

SEQ ID NO: 46811 - DNA, 28 bp, synthetic construct
  source 1..28: mol_type = other DNA
tcccaggcttgcaggccccattgagagg

SEQ ID NO: 46812 - DNA, 28 bp, synthetic construct
  source 1..28: mol_type = other DNA
aatggggcctgcaagcctgggaacttgg

SEQ ID NO: 46813 - DNA, 28 bp, synthetic construct
  source 1..28: mol_type = other DNA
atggggcctgcaagcctgggaacttggg

SEQ ID NO: 46814 - DNA, 28 bp, synthetic construct
  source 1..28: mol_type = other DNA
acgatgcccaagttcccaggcttgcagg

SEQ ID NO: 46815 - DNA, 28 bp, synthetic construct
  source 1..28: mol_type = other DNA
gcaagcctgggaacttgggcatcgttgg

SEQ ID NO: 46816 - DNA, 28 bp, synthetic construct
  source 1..28: mol_type = other DNA
caagcctgggaacttgggcatcgttggg

SEQ ID NO: 46817 - DNA, 28 bp, synthetic construct
  source 1..28: mol_type = other DNA
ctggcccaacgatgcccaagttcccagg

SEQ ID NO: 46818 - DNA, 28 bp, synthetic construct
  source 1..28: mol_type = other DNA
ggaacttgggcatcgttgggccagcagg

SEQ ID NO: 46819 - DNA, 28 bp, synthetic construct
  source 1..28: mol_type = other DNA
gttgggccagcaggatgagcagcaaagg

SEQ ID NO: 46820 - DNA, 28 bp, synthetic construct
  source 1..28: mol_type = other DNA
ttgggccagcaggatgagcagcaaaggg

SEQ ID NO: 46821 - DNA, 28 bp, synthetic construct
  source 1..28: mol_type = other DNA
tcagaccctttgctgctcatcctgctgg

SEQ ID NO: 46822 - DNA, 28 bp, synthetic construct
  source 1..28: mol_type = other DNA
agcaggatgagcagcaaagggtctgagg

SEQ ID NO: 46823 - DNA, 28 bp, synthetic construct
  source 1..28: mol_type = other DNA
gatgagcagcaaagggtctgaggacagg

SEQ ID NO: 46824 - DNA, 28 bp, synthetic construct
  source 1..28: mol_type = other DNA
atgagcagcaaagggtctgaggacaggg

SEQ ID NO: 46825 - DNA, 28 bp, synthetic construct
  source 1..28: mol_type = other DNA
agcagcaaagggtctgaggacagggtgg

SEQ ID NO: 46826 - DNA, 28 bp, synthetic construct
  source 1..28: mol_type = other DNA
tgctcatgaagacatgcccacgccatgg

SEQ ID NO: 46827 - DNA, 28 bp, synthetic construct
  source 1..28: mol_type = other DNA
gaagacatgcccacgccatggagccagg

SEQ ID NO: 46828 - DNA, 28 bp, synthetic construct
  source 1..28: mol_type = other DNA
aagacatgcccacgccatggagccaggg

SEQ ID NO: 46829 - DNA, 28 bp, synthetic construct
  source 1..28: mol_type = other DNA
agacatgcccacgccatggagccagggg

SEQ ID NO: 46830 - DNA, 28 bp, synthetic construct
  source 1..28: mol_type = other DNA
ctataagcccctggctccatggcgtggg

SEQ ID NO: 46831 - DNA, 28 bp, synthetic construct
  source 1..28: mol_type = other DNA
tctataagcccctggctccatggcgtgg

SEQ ID NO: 46832 - DNA, 28 bp, synthetic construct
  source 1..28: mol_type = other DNA
gccatggagccaggggcttatagagagg

SEQ ID NO: 46833 - DNA, 28 bp, synthetic construct
  source 1..28: mol_type = other DNA
ccctctctataagcccctggctccatgg

SEQ ID NO: 46834 - DNA, 28 bp, synthetic construct
  source 1..28: mol_type = other DNA
catggagccaggggcttatagagagggg

SEQ ID NO: 46835 - DNA, 28 bp, synthetic construct
  source 1..28: mol_type = other DNA
gtcactgcccctctctataagcccctgg

SEQ ID NO: 46836 - DNA, 28 bp, synthetic construct
  source 1..28: mol_type = other DNA
acttccagagtcccatccgtcagtgagg

SEQ ID NO: 46837 - DNA, 28 bp, synthetic construct
  source 1..28: mol_type = other DNA
cttccagagtcccatccgtcagtgaggg

SEQ ID NO: 46838 - DNA, 28 bp, synthetic construct
  source 1..28: mol_type = other DNA
ttccagagtcccatccgtcagtgagggg

SEQ ID NO: 46839 - DNA, 28 bp, synthetic construct
  source 1..28: mol_type = other DNA
gtcccctcactgacggatgggactctgg

SEQ ID NO: 46840 - DNA, 28 bp, synthetic construct
  source 1..28: mol_type = other DNA
gagtcccatccgtcagtgaggggactgg

SEQ ID NO: 46841 - DNA, 28 bp, synthetic construct
  source 1..28: mol_type = other DNA
agtcccatccgtcagtgaggggactggg

SEQ ID NO: 46842 - DNA, 28 bp, synthetic construct
  source 1..28: mol_type = other DNA
cagcccagtcccctcactgacggatggg

SEQ ID NO: 46843 - DNA, 28 bp, synthetic construct
  source 1..28: mol_type = other DNA
gcagcccagtcccctcactgacggatgg

SEQ ID NO: 46844 - DNA, 28 bp, synthetic construct
  source 1..28: mol_type = other DNA
atccgtcagtgaggggactgggctgcgg

SEQ ID NO: 46845 - DNA, 28 bp, synthetic construct
  source 1..28: mol_type = other DNA
tccgtcagtgaggggactgggctgcggg

SEQ ID NO: 46846 - DNA, 28 bp, synthetic construct
  source 1..28: mol_type = other DNA
tcccgcagcccagtcccctcactgacgg

SEQ ID NO: 46847 - DNA, 28 bp, synthetic construct
  source 1..28: mol_type = other DNA
tcagtgaggggactgggctgcgggatgg

SEQ ID NO: 46848 - DNA, 28 bp, synthetic construct
  source 1..28: mol_type = other DNA
cagtgaggggactgggctgcgggatggg

SEQ ID NO: 46849 - DNA, 28 bp, synthetic construct
  source 1..28: mol_type = other DNA
aggggactgggctgcgggatgggtgagg

SEQ ID NO: 46850 - DNA, 28 bp, synthetic construct
  source 1..28: mol_type = other DNA
gatgggtgaggatcttacagctcccagg

SEQ ID NO: 46851 - DNA, 28 bp, synthetic construct
  source 1..28: mol_type = other DNA
gtgaggatcttacagctcccaggttcgg

SEQ ID NO: 46852 - DNA, 28 bp, synthetic construct
  source 1..28: mol_type = other DNA
tcccaggttcggaaatctaccctctagg

SEQ ID NO: 46853 - DNA, 28 bp, synthetic construct
  source 1..28: mol_type = other DNA
gcctagagggtagatttccgaacctggg

SEQ ID NO: 46854 - DNA, 28 bp, synthetic construct
  source 1..28: mol_type = other DNA
ggcctagagggtagatttccgaacctgg

SEQ ID NO: 46855 - DNA, 28 bp, synthetic construct
  source 1..28: mol_type = other DNA
ggttcggaaatctaccctctaggcctgg

SEQ ID NO: 46856 - DNA, 28 bp, synthetic construct
  source 1..28: mol_type = other DNA
tcggaaatctaccctctaggcctggagg

SEQ ID NO: 46857 - DNA, 28 bp, synthetic construct
  source 1..28: mol_type = other DNA
tgcgagagaggcctccaggcctagaggg

SEQ ID NO: 46858 - DNA, 28 bp, synthetic construct
  source 1..28: mol_type = other DNA
ctgcgagagaggcctccaggcctagagg

SEQ ID NO: 46859 - DNA, 28 bp, synthetic construct
  source 1..28: mol_type = other DNA
gcctggaggcctctctcgcagagcatgg

SEQ ID NO: 46860 - DNA, 28 bp, synthetic construct
  source 1..28: mol_type = other DNA
tccatgctctgcgagagaggcctccagg

SEQ ID NO: 46861 - DNA, 28 bp, synthetic construct
  source 1..28: mol_type = other DNA
ggaggcctctctcgcagagcatggaagg

SEQ ID NO: 46862 - DNA, 28 bp, synthetic construct
  source 1..28: mol_type = other DNA
gcctctctcgcagagcatggaaggcagg

SEQ ID NO: 46863 - DNA, 28 bp, synthetic construct
  source 1..28: mol_type = other DNA
tcctgccttccatgctctgcgagagagg

SEQ ID NO: 46864 - DNA, 28 bp, synthetic construct
  source 1..28: mol_type = other DNA
tctcgcagagcatggaaggcaggagagg

SEQ ID NO: 46865 - DNA, 28 bp, synthetic construct
  source 1..28: mol_type = other DNA
cgcagagcatggaaggcaggagaggtgg

SEQ ID NO: 46866 - DNA, 28 bp, synthetic construct
  source 1..28: mol_type = other DNA
gcagagcatggaaggcaggagaggtggg

SEQ ID NO: 46867 - DNA, 28 bp, synthetic construct
  source 1..28: mol_type = other DNA
agcatggaaggcaggagaggtgggctgg

SEQ ID NO: 46868 - DNA, 28 bp, synthetic construct
  source 1..28: mol_type = other DNA
gaaggcaggagaggtgggctggcctagg

SEQ ID NO: 46869 - DNA, 28 bp, synthetic construct
  source 1..28: mol_type = other DNA
aaggcaggagaggtgggctggcctaggg

SEQ ID NO: 46870 - DNA, 28 bp, synthetic construct
  source 1..28: mol_type = other DNA
caggagaggtgggctggcctagggcagg

SEQ ID NO: 46871 - DNA, 28 bp, synthetic construct
  source 1..28: mol_type = other DNA
cagagagaagtggagctcctgccctagg

SEQ ID NO: 46872 - DNA, 28 bp, synthetic construct
  source 1..28: mol_type = other DNA
caggagctccacttctctctgcctctgg

SEQ ID NO: 46873 - DNA, 28 bp, synthetic construct
  source 1..28: mol_type = other DNA
ctccacttctctctgcctctggctatgg

SEQ ID NO: 46874 - DNA, 28 bp, synthetic construct
  source 1..28: mol_type = other DNA
tccacttctctctgcctctggctatggg

SEQ ID NO: 46875 - DNA, 28 bp, synthetic construct
  source 1..28: mol_type = other DNA
tcccatagccagaggcagagagaagtgg

SEQ ID NO: 46876 - DNA, 28 bp, synthetic construct
  source 1..28: mol_type = other DNA
cttctctctgcctctggctatgggaagg

SEQ ID NO: 46877 - DNA, 28 bp, synthetic construct
  source 1..28: mol_type = other DNA
tctgcctctggctatgggaaggagcagg

SEQ ID NO: 46878 - DNA, 28 bp, synthetic construct
  source 1..28: mol_type = other DNA
gcctctggctatgggaaggagcaggcgg

SEQ ID NO: 46879 - DNA, 28 bp, synthetic construct
  source 1..28: mol_type = other DNA
accgcctgctccttcccatagccagagg

SEQ ID NO: 46880 - DNA, 28 bp, synthetic construct
  source 1..28: mol_type = other DNA
ctggctatgggaaggagcaggcggttgg

SEQ ID NO: 46881 - DNA, 28 bp, synthetic construct
  source 1..28: mol_type = other DNA
aaatcctgtgacagcagagatcttctgg

SEQ ID NO: 46882 - DNA, 28 bp, synthetic construct
  source 1..28: mol_type = other DNA
aaatccagaagatctctgctgtcacagg

SEQ ID NO: 46883 - DNA, 28 bp, synthetic construct
  source 1..28: mol_type = other DNA
agcagagatcttctggatttttgcctgg

SEQ ID NO: 46884 - DNA, 28 bp, synthetic construct
  source 1..28: mol_type = other DNA
ttttgcctggacccttctgcaagcctgg

SEQ ID NO: 46885 - DNA, 28 bp, synthetic construct
  source 1..28: mol_type = other DNA
agtctccaggcttgcagaagggtccagg

SEQ ID NO: 46886 - DNA, 28 bp, synthetic construct
  source 1..28: mol_type = other DNA
tggacccttctgcaagcctggagactgg

SEQ ID NO: 46887 - DNA, 28 bp, synthetic construct
  source 1..28: mol_type = other DNA
aggtccagtctccaggcttgcagaaggg

SEQ ID NO: 46888 - DNA, 28 bp, synthetic construct
  source 1..28: mol_type = other DNA
caggtccagtctccaggcttgcagaagg

SEQ ID NO: 46889 - DNA, 28 bp, synthetic construct
  source 1..28: mol_type = other DNA
ggaacatgtggcaggtccagtctccagg

SEQ ID NO: 46890 - DNA, 28 bp, synthetic construct
  source 1..28: mol_type = other DNA
ggcagacagacttggaacatgtggcagg

SEQ ID NO: 46891 - DNA, 28 bp, synthetic construct
  source 1..28: mol_type = other DNA
cctaggcagacagacttggaacatgtgg

SEQ ID NO: 46892 - DNA, 28 bp, synthetic construct
  source 1..28: mol_type = other DNA
cagcagtgacctaggcagacagacttgg

SEQ ID NO: 46893 - DNA, 28 bp, synthetic construct
  source 1..28: mol_type = other DNA
ggaggagaagtggcagcagtgacctagg

SEQ ID NO: 46894 - DNA, 28 bp, synthetic construct
  source 1..28: mol_type = other DNA
aaaggtctgttagtgggaggagaagtgg

SEQ ID NO: 46895 - DNA, 28 bp, synthetic construct
  source 1..28: mol_type = other DNA
tcttcaagaaaggtctgttagtgggagg

SEQ ID NO: 46896 - DNA, 28 bp, synthetic construct
  source 1..28: mol_type = other DNA
gggtcttcaagaaaggtctgttagtggg

SEQ ID NO: 46897 - DNA, 28 bp, synthetic construct
  source 1..28: mol_type = other DNA
tgggtcttcaagaaaggtctgttagtgg

SEQ ID NO: 46898 - DNA, 28 bp, synthetic construct
  source 1..28: mol_type = other DNA
aacagacctttcttgaagacccactagg

SEQ ID NO: 46899 - DNA, 28 bp, synthetic construct
  source 1..28: mol_type = other DNA
tctggacctagtgggtcttcaagaaagg

SEQ ID NO: 46900 - DNA, 28 bp, synthetic construct
  source 1..28: mol_type = other DNA
aagacccactaggtccagacactgccgg

SEQ ID NO: 46901 - DNA, 28 bp, synthetic construct
  source 1..28: mol_type = other DNA
agacccactaggtccagacactgccggg

SEQ ID NO: 46902 - DNA, 28 bp, synthetic construct
  source 1..28: mol_type = other DNA
agtcccggcagtgtctggacctagtggg

SEQ ID NO: 46903 - DNA, 28 bp, synthetic construct
  source 1..28: mol_type = other DNA
aagtcccggcagtgtctggacctagtgg

SEQ ID NO: 46904 - DNA, 28 bp, synthetic construct
  source 1..28: mol_type = other DNA
aggtccagacactgccgggacttgcagg

SEQ ID NO: 46905 - DNA, 28 bp, synthetic construct
  source 1..28: mol_type = other DNA
catacctgcaagtcccggcagtgtctgg

SEQ ID NO: 46906 - DNA, 28 bp, synthetic construct
  source 1..28: mol_type = other DNA
cagacactgccgggacttgcaggtatgg

SEQ ID NO: 46907 - DNA, 28 bp, synthetic construct
  source 1..28: mol_type = other DNA
agacactgccgggacttgcaggtatggg

SEQ ID NO: 46908 - DNA, 28 bp, synthetic construct
  source 1..28: mol_type = other DNA
gacactgccgggacttgcaggtatgggg

SEQ ID NO: 46909 - DNA, 28 bp, synthetic construct
  source 1..28: mol_type = other DNA
acactgccgggacttgcaggtatggggg

SEQ ID NO: 46910 - DNA, 28 bp, synthetic construct
  source 1..28: mol_type = other DNA
cactgccgggacttgcaggtatgggggg

SEQ ID NO: 46911 - DNA, 28 bp, synthetic construct
  source 1..28: mol_type = other DNA
ttctaccccccatacctgcaagtcccgg

SEQ ID NO: 46912 - DNA, 28 bp, synthetic construct
  source 1..28: mol_type = other DNA
gggacttgcaggtatggggggtagaagg

SEQ ID NO: 46913 - DNA, 28 bp, synthetic construct
  source 1..28: mol_type = other DNA
ttgcaggtatggggggtagaaggagagg

SEQ ID NO: 46914 - DNA, 28 bp, synthetic construct
  source 1..28: mol_type = other DNA
tagaaggagaggcagataagctgcctgg

SEQ ID NO: 46915 - DNA, 28 bp, synthetic construct
  source 1..28: mol_type = other DNA
agaaggagaggcagataagctgcctggg

SEQ ID NO: 46916 - DNA, 28 bp, synthetic construct
  source 1..28: mol_type = other DNA
gaaggagaggcagataagctgcctgggg

SEQ ID NO: 46917 - DNA, 28 bp, synthetic construct
  source 1..28: mol_type = other DNA
aaggagaggcagataagctgcctggggg

SEQ ID NO: 46918 - DNA, 28 bp, synthetic construct
  source 1..28: mol_type = other DNA
aggagaggcagataagctgcctgggggg

SEQ ID NO: 46919 - DNA, 28 bp, synthetic construct
  source 1..28: mol_type = other DNA
agctgcctggggggctgttagctaatgg

SEQ ID NO: 46920 - DNA, 28 bp, synthetic construct
  source 1..28: mol_type = other DNA
gctgcctggggggctgttagctaatggg

SEQ ID NO: 46921 - DNA, 28 bp, synthetic construct
  source 1..28: mol_type = other DNA
tgtacccattagctaacagccccccagg

SEQ ID NO: 46922 - DNA, 28 bp, synthetic construct
  source 1..28: mol_type = other DNA
ggggggctgttagctaatgggtacaagg

SEQ ID NO: 46923 - DNA, 28 bp, synthetic construct
  source 1..28: mol_type = other DNA
atctgtggcttctcttctcgggaggggg

SEQ ID NO: 46924 - DNA, 28 bp, synthetic construct
  source 1..28: mol_type = other DNA
catctgtggcttctcttctcgggagggg

SEQ ID NO: 46925 - DNA, 28 bp, synthetic construct
  source 1..28: mol_type = other DNA
tcatctgtggcttctcttctcgggaggg

SEQ ID NO: 46926 - DNA, 28 bp, synthetic construct
  source 1..28: mol_type = other DNA
ctcatctgtggcttctcttctcgggagg

SEQ ID NO: 46927 - DNA, 28 bp, synthetic construct
  source 1..28: mol_type = other DNA
cccgagaagagaagccacagatgagtgg

SEQ ID NO: 46928 - DNA, 28 bp, synthetic construct
  source 1..28: mol_type = other DNA
ccgagaagagaagccacagatgagtggg

SEQ ID NO: 46929 - DNA, 28 bp, synthetic construct
  source 1..28: mol_type = other DNA
gaagccacagatgagtgggccagcgagg

SEQ ID NO: 46930 - DNA, 28 bp, synthetic construct
  source 1..28: mol_type = other DNA
ctggcctcgctggcccactcatctgtgg

SEQ ID NO: 46931 - DNA, 28 bp, synthetic construct
  source 1..28: mol_type = other DNA
agtggacattgaagactggcctcgctgg

SEQ ID NO: 46932 - DNA, 28 bp, synthetic construct
  source 1..28: mol_type = other DNA
gagtgaattagtggacattgaagactgg

SEQ ID NO: 46933 - DNA, 28 bp, synthetic construct
  source 1..28: mol_type = other DNA
tgtccactaattcactctaagcatttgg

SEQ ID NO: 46934 - DNA, 28 bp, synthetic construct
  source 1..28: mol_type = other DNA
tggccaaatgcttagagtgaattagtgg

SEQ ID NO: 46935 - DNA, 28 bp, synthetic construct
  source 1..28: mol_type = other DNA
tcactctaagcatttggccaaaaaaagg

SEQ ID NO: 46936 - DNA, 28 bp, synthetic construct
  source 1..28: mol_type = other DNA
ttcagttatttctctctcctttttttgg

SEQ ID NO: 46937 - DNA, 28 bp, synthetic construct
  source 1..28: mol_type = other DNA
gagagagaaataactgaaattgttcagg

SEQ ID NO: 46938 - DNA, 28 bp, synthetic construct
  source 1..28: mol_type = other DNA
agagaaataactgaaattgttcaggtgg

SEQ ID NO: 46939 - DNA, 28 bp, synthetic construct
  source 1..28: mol_type = other DNA
tcaggtggctccatcgtctattctgtgg

SEQ ID NO: 46940 - DNA, 28 bp, synthetic construct
  source 1..28: mol_type = other DNA
atggaggggaccacagaatagacgatgg

SEQ ID NO: 46941 - DNA, 28 bp, synthetic construct
  source 1..28: mol_type = other DNA
ggtcccctccatgagcctttgccccagg

SEQ ID NO: 46942 - DNA, 28 bp, synthetic construct
  source 1..28: mol_type = other DNA
gtcccctccatgagcctttgccccaggg

SEQ ID NO: 46943 - DNA, 28 bp, synthetic construct
  source 1..28: mol_type = other DNA
caccctggggcaaaggctcatggagggg

SEQ ID NO: 46944 - DNA, 28 bp, synthetic construct
  source 1..28: mol_type = other DNA
ccctccatgagcctttgccccagggtgg

SEQ ID NO: 46945 - DNA, 28 bp, synthetic construct
  source 1..28: mol_type = other DNA
cccaccctggggcaaaggctcatggagg

SEQ ID NO: 46946 - DNA, 28 bp, synthetic construct
  source 1..28: mol_type = other DNA
gcacccaccctggggcaaaggctcatgg

SEQ ID NO: 46947 - DNA, 28 bp, synthetic construct
  source 1..28: mol_type = other DNA
tgagcctttgccccagggtgggtgcagg

SEQ ID NO: 46948 - DNA, 28 bp, synthetic construct
  source 1..28: mol_type = other DNA
cgcacctgcacccaccctggggcaaagg

SEQ ID NO: 46949 - DNA, 28 bp, synthetic construct
  source 1..28: mol_type = other DNA
gacactcgcacctgcacccaccctgggg

SEQ ID NO: 46950 - DNA, 28 bp, synthetic construct
  source 1..28: mol_type = other DNA
tgacactcgcacctgcacccaccctggg

SEQ ID NO: 46951 - DNA, 28 bp, synthetic construct
  source 1..28: mol_type = other DNA
gtgacactcgcacctgcacccaccctgg

SEQ ID NO: 46952 - DNA, 28 bp, synthetic construct
  source 1..28: mol_type = other DNA
aactctgaatgactgaggcagctgcagg

SEQ ID NO: 46953 - DNA, 28 bp, synthetic construct
  source 1..28: mol_type = other DNA
aaggctctggaactctgaatgactgagg

SEQ ID NO: 46954 - DNA, 28 bp, synthetic construct
  source 1..28: mol_type = other DNA
tcattcagagttccagagccttctgtgg

SEQ ID NO: 46955 - DNA, 28 bp, synthetic construct
  source 1..28: mol_type = other DNA
ttcagagttccagagccttctgtggtgg

SEQ ID NO: 46956 - DNA, 28 bp, synthetic construct
  source 1..28: mol_type = other DNA
caggatgctccaccacagaaggctctgg

SEQ ID NO: 46957 - DNA, 28 bp, synthetic construct
  source 1..28: mol_type = other DNA
aagcagcaggatgctccaccacagaagg

SEQ ID NO: 46958 - DNA, 28 bp, synthetic construct
  source 1..28: mol_type = other DNA
ttctgtggtggagcatcctgctgcttgg

SEQ ID NO: 46959 - DNA, 28 bp, synthetic construct
  source 1..28: mol_type = other DNA
tgtggtggagcatcctgctgcttggagg

SEQ ID NO: 46960 - DNA, 28 bp, synthetic construct
  source 1..28: mol_type = other DNA
acttcagactcatcctccaagcagcagg

SEQ ID NO: 46961 - DNA, 28 bp, synthetic construct
  source 1..28: mol_type = other DNA
ggaggatgagtctgaagtttaaaaatgg

SEQ ID NO: 46962 - DNA, 28 bp, synthetic construct
  source 1..28: mol_type = other DNA
gaggatgagtctgaagtttaaaaatggg

SEQ ID NO: 46963 - DNA, 28 bp, synthetic construct
  source 1..28: mol_type = other DNA
actgctcatcaggggggctcagaaaagg

SEQ ID NO: 46964 - DNA, 28 bp, synthetic construct
  source 1..28: mol_type = other DNA
cagaagcactgactgctcatcagggggg

SEQ ID NO: 46965 - DNA, 28 bp, synthetic construct
  source 1..28: mol_type = other DNA
ccagaagcactgactgctcatcaggggg

SEQ ID NO: 46966 - DNA, 28 bp, synthetic construct
  source 1..28: mol_type = other DNA
cccagaagcactgactgctcatcagggg

SEQ ID NO: 46967 - DNA, 28 bp, synthetic construct
  source 1..28: mol_type = other DNA
gcccagaagcactgactgctcatcaggg

SEQ ID NO: 46968 - DNA, 28 bp, synthetic construct
  source 1..28: mol_type = other DNA
ggcccagaagcactgactgctcatcagg

SEQ ID NO: 46969 - DNA, 28 bp, synthetic construct
  source 1..28: mol_type = other DNA
cagtcagtgcttctgggcccagctaagg

SEQ ID NO: 46970 - DNA, 28 bp, synthetic construct
  source 1..28: mol_type = other DNA
ctgggaacagatggcttccttagctggg

SEQ ID NO: 46971 - DNA, 28 bp, synthetic construct
  source 1..28: mol_type = other DNA
gctgggaacagatggcttccttagctgg

SEQ ID NO: 46972 - DNA, 28 bp, synthetic construct
  source 1..28: mol_type = other DNA
taaggaagccatctgttcccagcagagg

SEQ ID NO: 46973 - DNA, 28 bp, synthetic construct
  source 1..28: mol_type = other DNA
gcagctctcctctgctgggaacagatgg

SEQ ID NO: 46974 - DNA, 28 bp, synthetic construct
  source 1..28: mol_type = other DNA
gtcagcgcagcagctctcctctgctggg

SEQ ID NO: 46975 - DNA, 28 bp, synthetic construct
  source 1..28: mol_type = other DNA
ggtcagcgcagcagctctcctctgctgg

SEQ ID NO: 46976 - DNA, 28 bp, synthetic construct
  source 1..28: mol_type = other DNA
ggagagctgctgcgctgacctgcagagg

SEQ ID NO: 46977 - DNA, 28 bp, synthetic construct
  source 1..28: mol_type = other DNA
agctgctgcgctgacctgcagaggttgg

SEQ ID NO: 46978 - DNA, 28 bp, synthetic construct
  source 1..28: mol_type = other DNA
tgctgcgctgacctgcagaggttggtgg

SEQ ID NO: 46979 - DNA, 28 bp, synthetic construct
  source 1..28: mol_type = other DNA
ctgtgctgggaccaccaacctctgcagg

SEQ ID NO: 46980 - DNA, 28 bp, synthetic construct
  source 1..28: mol_type = other DNA
tggtcccagcacagagctgtgcccatgg

SEQ ID NO: 46981 - DNA, 28 bp, synthetic construct
  source 1..28: mol_type = other DNA
ggtcccagcacagagctgtgcccatggg

SEQ ID NO: 46982 - DNA, 28 bp, synthetic construct
  source 1..28: mol_type = other DNA
aagcccatgggcacagctctgtgctggg

SEQ ID NO: 46983 - DNA, 28 bp, synthetic construct
  source 1..28: mol_type = other DNA
caagcccatgggcacagctctgtgctgg

SEQ ID NO: 46984 - DNA, 28 bp, synthetic construct
  source 1..28: mol_type = other DNA
agagctgtgcccatgggcttgttagtgg

SEQ ID NO: 46985 - DNA, 28 bp, synthetic construct
  source 1..28: mol_type = other DNA
gagctgtgcccatgggcttgttagtggg

SEQ ID NO: 46986 - DNA, 28 bp, synthetic construct
  source 1..28: mol_type = other DNA
ttgcttttcccactaacaagcccatggg

SEQ ID NO: 46987 - DNA, 28 bp, synthetic construct
  source 1..28: mol_type = other DNA
tttgcttttcccactaacaagcccatgg

SEQ ID NO: 46988 - DNA, 28 bp, synthetic construct
  source 1..28: mol_type = other DNA
gagtgggcattcataattaaatgtttgg

SEQ ID NO: 46989 - DNA, 28 bp, synthetic construct
  source 1..28: mol_type = other DNA
attttagatctagatgctggggagtggg

SEQ ID NO: 46990 - DNA, 28 bp, synthetic construct
  source 1..28: mol_type = other DNA
aattttagatctagatgctggggagtgg

SEQ ID NO: 46991 - DNA, 28 bp, synthetic construct
  source 1..28: mol_type = other DNA
ttaataattttagatctagatgctgggg

SEQ ID NO: 46992 - DNA, 28 bp, synthetic construct
  source 1..28: mol_type = other DNA
gttaataattttagatctagatgctggg

SEQ ID NO: 46993 - DNA, 28 bp, synthetic construct
  source 1..28: mol_type = other DNA
tgttaataattttagatctagatgctgg

SEQ ID NO: 46994 - DNA, 28 bp, synthetic construct
  source 1..28: mol_type = other DNA
catacacagagagagaaaaagaatgtgg

SEQ ID NO: 46995 - DNA, 28 bp, synthetic construct
  source 1..28: mol_type = other DNA
gatgtttgcaatgtacttttaaattagg

SEQ ID NO: 46996 - DNA, 28 bp, synthetic construct
  source 1..28: mol_type = other DNA
taggagatgcaggctgaagctttcaggg

SEQ ID NO: 46997 - DNA, 28 bp, synthetic construct
  source 1..28: mol_type = other DNA
ttaggagatgcaggctgaagctttcagg

SEQ ID NO: 46998 - DNA, 28 bp, synthetic construct
  source 1..28: mol_type = other DNA
cttcagcctgcatctcctaagagttagg

SEQ ID NO: 46999 - DNA, 28 bp, synthetic construct
  source 1..28: mol_type = other DNA
ttcagcctgcatctcctaagagttaggg

SEQ ID NO: 47000 - DNA, 28 bp, synthetic construct
  source 1..28: mol_type = other DNA
caatgccctaactcttaggagatgcagg

SEQ ID NO: 47001 - DNA, 28 bp, synthetic construct
  source 1..28: mol_type = other DNA
tgtgtaggacaatgccctaactcttagg

SEQ ID NO: 47002 - DNA, 28 bp, synthetic construct
  source 1..28: mol_type = other DNA
agagttagggcattgtcctacacattgg

SEQ ID NO: 47003 - DNA, 28 bp, synthetic construct
  source 1..28: mol_type = other DNA
tggctgtgatactgggccaatgtgtagg

SEQ ID NO: 47004 - DNA, 28 bp, synthetic construct
  source 1..28: mol_type = other DNA
gacttctcgtcttggctgtgatactggg

SEQ ID NO: 47005 - DNA, 28 bp, synthetic construct
  source 1..28: mol_type = other DNA
tgacttctcgtcttggctgtgatactgg

SEQ ID NO: 47006 - DNA, 28 bp, synthetic construct
  source 1..28: mol_type = other DNA
atcgctgggaaatgacttctcgtcttgg

SEQ ID NO: 47007 - DNA, 28 bp, synthetic construct
  source 1..28: mol_type = other DNA
tacagattagatagcagacatcgctggg

SEQ ID NO: 47008 - DNA, 28 bp, synthetic construct
  source 1..28: mol_type = other DNA
atacagattagatagcagacatcgctgg

SEQ ID NO: 47009 - DNA, 28 bp, synthetic construct
  source 1..28: mol_type = other DNA
attcaaatccccccaattgtctcccagg

SEQ ID NO: 47010 - DNA, 28 bp, synthetic construct
  source 1..28: mol_type = other DNA
ataagttacctgggagacaattgggggg

SEQ ID NO: 47011 - DNA, 28 bp, synthetic construct
  source 1..28: mol_type = other DNA
cataagttacctgggagacaattggggg

SEQ ID NO: 47012 - DNA, 28 bp, synthetic construct
  source 1..28: mol_type = other DNA
acataagttacctgggagacaattgggg

SEQ ID NO: 47013 - DNA, 28 bp, synthetic construct
  source 1..28: mol_type = other DNA
cacataagttacctgggagacaattggg

SEQ ID NO: 47014 - DNA, 28 bp, synthetic construct
  source 1..28: mol_type = other DNA
acacataagttacctgggagacaattgg

SEQ ID NO: 47015 - DNA, 28 bp, synthetic construct
  source 1..28: mol_type = other DNA
ttgtctcccaggtaacttatgtgtctgg

SEQ ID NO: 47016 - DNA, 28 bp, synthetic construct
  source 1..28: mol_type = other DNA
ccaaaaccagacacataagttacctggg

SEQ ID NO: 47017 - DNA, 28 bp, synthetic construct
  source 1..28: mol_type = other DNA
tccaaaaccagacacataagttacctgg

SEQ ID NO: 47018 - DNA, 28 bp, synthetic construct
  source 1..28: mol_type = other DNA
tggttttggaatcagcatccagtcacgg

SEQ ID NO: 47019 - DNA, 28 bp, synthetic construct
  source 1..28: mol_type = other DNA
gaaaatgcaatgtgtgcaccgtgactgg

SEQ ID NO: 47020 - DNA, 28 bp, synthetic construct
  source 1..28: mol_type = other DNA
ttttaaaacctctttgaatgctgaaagg

SEQ ID NO: 47021 - DNA, 28 bp, synthetic construct
  source 1..28: mol_type = other DNA
agggaagacctttcagcattcaaagagg

SEQ ID NO: 47022 - DNA, 28 bp, synthetic construct
  source 1..28: mol_type = other DNA
catttaaaaactcaaagtgagctgaggg

SEQ ID NO: 47023 - DNA, 28 bp, synthetic construct
  source 1..28: mol_type = other DNA
tcatttaaaaactcaaagtgagctgagg

SEQ ID NO: 47024 - DNA, 28 bp, synthetic construct
  source 1..28: mol_type = other DNA
gagtttttaaatgacattgtttttgagg

SEQ ID NO: 47025 - DNA, 28 bp, synthetic construct
  source 1..28: mol_type = other DNA
taaatgacattgtttttgaggccctagg

SEQ ID NO: 47026 - DNA, 28 bp, synthetic construct
  source 1..28: mol_type = other DNA
gggcttcaaaaagacagcaggcctaggg

SEQ ID NO: 47027 - DNA, 28 bp, synthetic construct
  source 1..28: mol_type = other DNA
ggggcttcaaaaagacagcaggcctagg

SEQ ID NO: 47028 - DNA, 28 bp, synthetic construct
  source 1..28: mol_type = other DNA
gaatgtggggcttcaaaaagacagcagg

SEQ ID NO: 47029 - DNA, 28 bp, synthetic construct
  source 1..28: mol_type = other DNA
aacaatctgacaaattcagaatgtgggg

SEQ ID NO: 47030 - DNA, 28 bp, synthetic construct
  source 1..28: mol_type = other DNA
aaacaatctgacaaattcagaatgtggg

SEQ ID NO: 47031 - DNA, 28 bp, synthetic construct
  source 1..28: mol_type = other DNA
caaacaatctgacaaattcagaatgtgg

SEQ ID NO: 47032 - DNA, 28 bp, synthetic construct
  source 1..28: mol_type = other DNA
ctgaatttgtcagattgtttgctcatgg

SEQ ID NO: 47033 - DNA, 28 bp, synthetic construct
  source 1..28: mol_type = other DNA
ttgaaagtacaggggatagaagaagtgg

SEQ ID NO: 47034 - DNA, 28 bp, synthetic construct
  source 1..28: mol_type = other DNA
acttcttctatcccctgtactttcaagg

SEQ ID NO: 47035 - DNA, 28 bp, synthetic construct
  source 1..28: mol_type = other DNA
tcccctgtactttcaaggataatttagg

SEQ ID NO: 47036 - DNA, 28 bp, synthetic construct
  source 1..28: mol_type = other DNA
gcctaaattatccttgaaagtacagggg

SEQ ID NO: 47037 - DNA, 28 bp, synthetic construct
  source 1..28: mol_type = other DNA
agcctaaattatccttgaaagtacaggg

SEQ ID NO: 47038 - DNA, 28 bp, synthetic construct
  source 1..28: mol_type = other DNA
tagcctaaattatccttgaaagtacagg

SEQ ID NO: 47039 - DNA, 28 bp, synthetic construct
  source 1..28: mol_type = other DNA
agtgaagctgtcaagtcagcacaaaagg

SEQ ID NO: 47040 - DNA, 28 bp, synthetic construct
  source 1..28: mol_type = other DNA
acaggtgacagtggaggcgcatcttagg

SEQ ID NO: 47041 - DNA, 28 bp, synthetic construct
  source 1..28: mol_type = other DNA
tggcacttggtacaggtgacagtggagg

SEQ ID NO: 47042 - DNA, 28 bp, synthetic construct
  source 1..28: mol_type = other DNA
ttttggcacttggtacaggtgacagtgg

SEQ ID NO: 47043 - DNA, 28 bp, synthetic construct
  source 1..28: mol_type = other DNA
cctgtaccaagtgccaaaacagcagagg

SEQ ID NO: 47044 - DNA, 28 bp, synthetic construct
  source 1..28: mol_type = other DNA
ctgtaccaagtgccaaaacagcagaggg

SEQ ID NO: 47045 - DNA, 28 bp, synthetic construct
  source 1..28: mol_type = other DNA
tgtaccaagtgccaaaacagcagagggg

SEQ ID NO: 47046 - DNA, 28 bp, synthetic construct
  source 1..28: mol_type = other DNA
ctggcccctctgctgttttggcacttgg

SEQ ID NO: 47047 - DNA, 28 bp, synthetic construct
  source 1..28: mol_type = other DNA
gctctaactggcccctctgctgttttgg

SEQ ID NO: 47048 - DNA, 28 bp, synthetic construct
  source 1..28: mol_type = other DNA
gaggggccagttagagcaagagctctgg

SEQ ID NO: 47049 - DNA, 28 bp, synthetic construct
  source 1..28: mol_type = other DNA
aggggccagttagagcaagagctctggg

SEQ ID NO: 47050 - DNA, 28 bp, synthetic construct
  source 1..28: mol_type = other DNA
ggggccagttagagcaagagctctgggg

SEQ ID NO: 47051 - DNA, 28 bp, synthetic construct
  source 1..28: mol_type = other DNA
gggccagttagagcaagagctctggggg

SEQ ID NO: 47052 - DNA, 28 bp, synthetic construct
  source 1..28: mol_type = other DNA
ggccagttagagcaagagctctgggggg

SEQ ID NO: 47053 - DNA, 28 bp, synthetic construct
  source 1..28: mol_type = other DNA
gccagttagagcaagagctctggggggg

SEQ ID NO: 47054 - DNA, 28 bp, synthetic construct
  source 1..28: mol_type = other DNA
gcccccccagagctcttgctctaactgg

SEQ ID NO: 47055 - DNA, 28 bp, synthetic construct
  source 1..28: mol_type = other DNA
gttagagcaagagctctgggggggccgg

SEQ ID NO: 47056 - DNA, 28 bp, synthetic construct
  source 1..28: mol_type = other DNA
ctctgggggggccggaaagtctccctgg

SEQ ID NO: 47057 - DNA, 28 bp, synthetic construct
  source 1..28: mol_type = other DNA
gggggccggaaagtctccctggagaagg

SEQ ID NO: 47058 - DNA, 28 bp, synthetic construct
  source 1..28: mol_type = other DNA
tacggccttctccagggagactttccgg

SEQ ID NO: 47059 - DNA, 28 bp, synthetic construct
  source 1..28: mol_type = other DNA
tctccctggagaaggccgtaatatctgg

SEQ ID NO: 47060 - DNA, 28 bp, synthetic construct
  source 1..28: mol_type = other DNA
ctccctggagaaggccgtaatatctggg

SEQ ID NO: 47061 - DNA, 28 bp, synthetic construct
  source 1..28: mol_type = other DNA
ggcccagatattacggccttctccaggg

SEQ ID NO: 47062 - DNA, 28 bp, synthetic construct
  source 1..28: mol_type = other DNA
aggcccagatattacggccttctccagg

SEQ ID NO: 47063 - DNA, 28 bp, synthetic construct
  source 1..28: mol_type = other DNA
ggagaaggccgtaatatctgggccttgg

SEQ ID NO: 47064 - DNA, 28 bp, synthetic construct
  source 1..28: mol_type = other DNA
aaggccgtaatatctgggccttggaagg

SEQ ID NO: 47065 - DNA, 28 bp, synthetic construct
  source 1..28: mol_type = other DNA
ccgtaatatctgggccttggaaggaagg

SEQ ID NO: 47066 - DNA, 28 bp, synthetic construct
  source 1..28: mol_type = other DNA
atctgggccttggaaggaaggacacagg

SEQ ID NO: 47067 - DNA, 28 bp, synthetic construct
  source 1..28: mol_type = other DNA
tctgggccttggaaggaaggacacaggg

SEQ ID NO: 47068 - DNA, 28 bp, synthetic construct
  source 1..28: mol_type = other DNA
ccagagccctgtgtccttccttccaagg

SEQ ID NO: 47069 - DNA, 28 bp, synthetic construct
  source 1..28: mol_type = other DNA
ggaaggaaggacacagggctctggaagg

SEQ ID NO: 47070 - DNA, 28 bp, synthetic construct
  source 1..28: mol_type = other DNA
aggaaggacacagggctctggaaggagg

SEQ ID NO: 47071 - DNA, 28 bp, synthetic construct
  source 1..28: mol_type = other DNA
aaggacacagggctctggaaggaggagg

SEQ ID NO: 47072 - DNA, 28 bp, synthetic construct
  source 1..28: mol_type = other DNA
tggaaggaggaggctgcatgcctgaagg

SEQ ID NO: 47073 - DNA, 28 bp, synthetic construct
  source 1..28: mol_type = other DNA
aggaggaggctgcatgcctgaaggctgg

SEQ ID NO: 47074 - DNA, 28 bp, synthetic construct
  source 1..28: mol_type = other DNA
ggaggaggctgcatgcctgaaggctggg

SEQ ID NO: 47075 - DNA, 28 bp, synthetic construct
  source 1..28: mol_type = other DNA
tgcctgaaggctgggccttcgaccctgg

SEQ ID NO: 47076 - DNA, 28 bp, synthetic construct
  source 1..28: mol_type = other DNA
gcctgaaggctgggccttcgaccctggg

SEQ ID NO: 47077 - DNA, 28 bp, synthetic construct
  source 1..28: mol_type = other DNA
cctgaaggctgggccttcgaccctgggg

SEQ ID NO: 47078 - DNA, 28 bp, synthetic construct
  source 1..28: mol_type = other DNA
aaggctgggccttcgaccctggggatgg

SEQ ID NO: 47079 - DNA, 28 bp, synthetic construct
  source 1..28: mol_type = other DNA
aggctgggccttcgaccctggggatggg

SEQ ID NO: 47080 - DNA, 28 bp, synthetic construct
  source 1..28: mol_type = other DNA
gccttcgaccctggggatgggccacagg

SEQ ID NO: 47081 - DNA, 28 bp, synthetic construct
  source 1..28: mol_type = other DNA
ccttcgaccctggggatgggccacaggg

SEQ ID NO: 47082 - DNA, 28 bp, synthetic construct
  source 1..28: mol_type = other DNA
tttggtgccctgtggcccatccccaggg

SEQ ID NO: 47083 - DNA, 28 bp, synthetic construct
  source 1..28: mol_type = other DNA
gtttggtgccctgtggcccatccccagg

SEQ ID NO: 47084 - DNA, 28 bp, synthetic construct
  source 1..28: mol_type = other DNA
gacatatgatgtgtttggtgccctgtgg

SEQ ID NO: 47085 - DNA, 28 bp, synthetic construct
  source 1..28: mol_type = other DNA
gaaagagagagacatatgatgtgtttgg

SEQ ID NO: 47086 - DNA, 28 bp, synthetic construct
  source 1..28: mol_type = other DNA
atcatatgtctctctctttctattttgg

SEQ ID NO: 47087 - DNA, 28 bp, synthetic construct
  source 1..28: mol_type = other DNA
tcatatgtctctctctttctattttggg

SEQ ID NO: 47088 - DNA, 28 bp, synthetic construct
  source 1..28: mol_type = other DNA
catatgtctctctctttctattttgggg

SEQ ID NO: 47089 - DNA, 28 bp, synthetic construct
  source 1..28: mol_type = other DNA
ctctctctttctattttggggtcccagg

SEQ ID NO: 47090 - DNA, 28 bp, synthetic construct
  source 1..28: mol_type = other DNA
tctctctttctattttggggtcccaggg

SEQ ID NO: 47091 - DNA, 28 bp, synthetic construct
  source 1..28: mol_type = other DNA
ttggggtcccagggttttcatttcctgg

SEQ ID NO: 47092 - DNA, 28 bp, synthetic construct
  source 1..28: mol_type = other DNA
cgggtctccaggaaatgaaaaccctggg

SEQ ID NO: 47093 - DNA, 28 bp, synthetic construct
  source 1..28: mol_type = other DNA
acgggtctccaggaaatgaaaaccctgg

SEQ ID NO: 47094 - DNA, 28 bp, synthetic construct
  source 1..28: mol_type = other DNA
agggttttcatttcctggagacccgtgg

SEQ ID NO: 47095 - DNA, 28 bp, synthetic construct
  source 1..28: mol_type = other DNA
cagtgcacacagaccacgggtctccagg

SEQ ID NO: 47096 - DNA, 28 bp, synthetic construct
  source 1..28: mol_type = other DNA
ctggagacccgtggtctgtgtgcactgg

SEQ ID NO: 47097 - DNA, 28 bp, synthetic construct
  source 1..28: mol_type = other DNA
ctctgctccagtgcacacagaccacggg

SEQ ID NO: 47098 - DNA, 28 bp, synthetic construct
  source 1..28: mol_type = other DNA
gctctgctccagtgcacacagaccacgg

SEQ ID NO: 47099 - DNA, 28 bp, synthetic construct
  source 1..28: mol_type = other DNA
ggtctgtgtgcactggagcagagccagg

SEQ ID NO: 47100 - DNA, 28 bp, synthetic construct
  source 1..28: mol_type = other DNA
gcagagccaggctctcagttgcagcagg

SEQ ID NO: 47101 - DNA, 28 bp, synthetic construct
  source 1..28: mol_type = other DNA
cagagccaggctctcagttgcagcaggg

SEQ ID NO: 47102 - DNA, 28 bp, synthetic construct
  source 1..28: mol_type = other DNA
cttttccctgctgcaactgagagcctgg

SEQ ID NO: 47103 - DNA, 28 bp, synthetic construct
  source 1..28: mol_type = other DNA
cagttgcagcagggaaaagcctacatgg

SEQ ID NO: 47104 - DNA, 28 bp, synthetic construct
  source 1..28: mol_type = other DNA
agttgcagcagggaaaagcctacatggg

SEQ ID NO: 47105 - DNA, 28 bp, synthetic construct
  source 1..28: mol_type = other DNA
gttgcagcagggaaaagcctacatgggg

SEQ ID NO: 47106 - DNA, 28 bp, synthetic construct
  source 1..28: mol_type = other DNA
gcttgcgggaggcagttccccatgtagg

SEQ ID NO: 47107 - DNA, 28 bp, synthetic construct
  source 1..28: mol_type = other DNA
atggggaactgcctcccgcaagctgtgg

SEQ ID NO: 47108 - DNA, 28 bp, synthetic construct
  source 1..28: mol_type = other DNA
ctcttctcacaccacagcttgcgggagg

SEQ ID NO: 47109 - DNA, 28 bp, synthetic construct
  source 1..28: mol_type = other DNA
gggctcttctcacaccacagcttgcggg

SEQ ID NO: 47110 - DNA, 28 bp, synthetic construct
  source 1..28: mol_type = other DNA
agggctcttctcacaccacagcttgcgg

SEQ ID NO: 47111 - DNA, 28 bp, synthetic construct
  source 1..28: mol_type = other DNA
gcaagctgtggtgtgagaagagccctgg

SEQ ID NO: 47112 - DNA, 28 bp, synthetic construct
  source 1..28: mol_type = other DNA
gctgtggtgtgagaagagccctggctgg

SEQ ID NO: 47113 - DNA, 28 bp, synthetic construct
  source 1..28: mol_type = other DNA
tgtgagaagagccctggctggcagcagg

SEQ ID NO: 47114 - DNA, 28 bp, synthetic construct
  source 1..28: mol_type = other DNA
acttcacagctcctgctgccagccaggg

SEQ ID NO: 47115 - DNA, 28 bp, synthetic construct
  source 1..28: mol_type = other DNA
aacttcacagctcctgctgccagccagg

SEQ ID NO: 47116 - DNA, 28 bp, synthetic construct
  source 1..28: mol_type = other DNA
aggagctgtgaagtttcatcccagccgg

SEQ ID NO: 47117 - DNA, 28 bp, synthetic construct
  source 1..28: mol_type = other DNA
ggagctgtgaagtttcatcccagccggg

SEQ ID NO: 47118 - DNA, 28 bp, synthetic construct
  source 1..28: mol_type = other DNA
aggcagctactaaatgcacccggctggg

SEQ ID NO: 47119 - DNA, 28 bp, synthetic construct
  source 1..28: mol_type = other DNA
caggcagctactaaatgcacccggctgg

SEQ ID NO: 47120 - DNA, 28 bp, synthetic construct
  source 1..28: mol_type = other DNA
tggtcaggcagctactaaatgcacccgg

SEQ ID NO: 47121 - DNA, 28 bp, synthetic construct
  source 1..28: mol_type = other DNA
gtagctgcctgaccatcttcctcccagg

SEQ ID NO: 47122 - DNA, 28 bp, synthetic construct
  source 1..28: mol_type = other DNA
ctgagggcctgggaggaagatggtcagg

SEQ ID NO: 47123 - DNA, 28 bp, synthetic construct
  source 1..28: mol_type = other DNA
agaaactgagggcctgggaggaagatgg

SEQ ID NO: 47124 - DNA, 28 bp, synthetic construct
  source 1..28: mol_type = other DNA
cagatgaagaaactgagggcctgggagg

SEQ ID NO: 47125 - DNA, 28 bp, synthetic construct
  source 1..28: mol_type = other DNA
ctacagatgaagaaactgagggcctggg

SEQ ID NO: 47126 - DNA, 28 bp, synthetic construct
  source 1..28: mol_type = other DNA
tctacagatgaagaaactgagggcctgg

SEQ ID NO: 47127 - DNA, 28 bp, synthetic construct
  source 1..28: mol_type = other DNA
ctcattctacagatgaagaaactgaggg

SEQ ID NO: 47128 - DNA, 28 bp, synthetic construct
  source 1..28: mol_type = other DNA
gctcattctacagatgaagaaactgagg

SEQ ID NO: 47129 - DNA, 28 bp, synthetic construct
  source 1..28: mol_type = other DNA
ttcttcatctgtagaatgagcagatagg

SEQ ID NO: 47130 - DNA, 28 bp, synthetic construct
  source 1..28: mol_type = other DNA
tcttcatctgtagaatgagcagataggg

SEQ ID NO: 47131 - DNA, 28 bp, synthetic construct
  source 1..28: mol_type = other DNA
cttcatctgtagaatgagcagatagggg

SEQ ID NO: 47132 - DNA, 28 bp, synthetic construct
  source 1..28: mol_type = other DNA
agaatgagcagataggggccacagcagg

SEQ ID NO: 47133 - DNA, 28 bp, synthetic construct
  source 1..28: mol_type = other DNA
gaatgagcagataggggccacagcaggg

SEQ ID NO: 47134 - DNA, 28 bp, synthetic construct
  source 1..28: mol_type = other DNA
ctttgatgtgtgaaaatccctgctgtgg

SEQ ID NO: 47135 - DNA, 28 bp, synthetic construct
  source 1..28: mol_type = other DNA
cacagcagggattttcacacatcaaagg

SEQ ID NO: 47136 - DNA, 28 bp, synthetic construct
  source 1..28: mol_type = other DNA
agcagggattttcacacatcaaaggagg

SEQ ID NO: 47137 - DNA, 28 bp, synthetic construct
  source 1..28: mol_type = other DNA
ggcagcctctgctctagttgatgtgagg

SEQ ID NO: 47138 - DNA, 28 bp, synthetic construct
  source 1..28: mol_type = other DNA
ctcatcctcacatcaactagagcagagg

SEQ ID NO: 47139 - DNA, 28 bp, synthetic construct
  source 1..28: mol_type = other DNA
ctctgctctagttgatgtgaggatgagg

SEQ ID NO: 47140 - DNA, 28 bp, synthetic construct
  source 1..28: mol_type = other DNA
tctgctctagttgatgtgaggatgaggg

SEQ ID NO: 47141 - DNA, 28 bp, synthetic construct
  source 1..28: mol_type = other DNA
ctgctctagttgatgtgaggatgagggg

SEQ ID NO: 47142 - DNA, 28 bp, synthetic construct
  source 1..28: mol_type = other DNA
tgctctagttgatgtgaggatgaggggg

SEQ ID NO: 47143 - DNA, 28 bp, synthetic construct
  source 1..28: mol_type = other DNA
tctagttgatgtgaggatgagggggcgg

SEQ ID NO: 47144 - DNA, 28 bp, synthetic construct
  source 1..28: mol_type = other DNA
gggcggcctagaccccctgctgcccagg

SEQ ID NO: 47145 - DNA, 28 bp, synthetic construct
  source 1..28: mol_type = other DNA
caacggcctgggcagcagggggtctagg

SEQ ID NO: 47146 - DNA, 28 bp, synthetic construct
  source 1..28: mol_type = other DNA
agaccccctgctgcccaggccgttgagg

SEQ ID NO: 47147 - DNA, 28 bp, synthetic construct
  source 1..28: mol_type = other DNA
ttgcctcaacggcctgggcagcaggggg

SEQ ID NO: 47148 - DNA, 28 bp, synthetic construct
  source 1..28: mol_type = other DNA
gttgcctcaacggcctgggcagcagggg

SEQ ID NO: 47149 - DNA, 28 bp, synthetic construct
  source 1..28: mol_type = other DNA
tgttgcctcaacggcctgggcagcaggg

SEQ ID NO: 47150 - DNA, 28 bp, synthetic construct
  source 1..28: mol_type = other DNA
gtgttgcctcaacggcctgggcagcagg

SEQ ID NO: 47151 - DNA, 28 bp, synthetic construct
  source 1..28: mol_type = other DNA
gctgcccaggccgttgaggcaacactgg

SEQ ID NO: 47152 - DNA, 28 bp, synthetic construct
  source 1..28: mol_type = other DNA
ctgcccaggccgttgaggcaacactggg

SEQ ID NO: 47153 - DNA, 28 bp, synthetic construct
  source 1..28: mol_type = other DNA
gaacccagtgttgcctcaacggcctggg

SEQ ID NO: 47154 - DNA, 28 bp, synthetic construct
  source 1..28: mol_type = other DNA
ggaacccagtgttgcctcaacggcctgg

SEQ ID NO: 47155 - DNA, 28 bp, synthetic construct
  source 1..28: mol_type = other DNA
ggccgttgaggcaacactgggttcctgg

SEQ ID NO: 47156 - DNA, 28 bp, synthetic construct
  source 1..28: mol_type = other DNA
agccaggaacccagtgttgcctcaacgg

SEQ ID NO: 47157 - DNA, 28 bp, synthetic construct
  source 1..28: mol_type = other DNA
cactgggttcctggcttgacagctgtgg

SEQ ID NO: 47158 - DNA, 28 bp, synthetic construct
  source 1..28: mol_type = other DNA
actgggttcctggcttgacagctgtggg

SEQ ID NO: 47159 - DNA, 28 bp, synthetic construct
  source 1..28: mol_type = other DNA
ggttcctggcttgacagctgtgggctgg

SEQ ID NO: 47160 - DNA, 28 bp, synthetic construct
  source 1..28: mol_type = other DNA
gcagccagcccacagctgtcaagccagg

SEQ ID NO: 47161 - DNA, 28 bp, synthetic construct
  source 1..28: mol_type = other DNA
ggctggctgcccttgccagctcagacgg

SEQ ID NO: 47162 - DNA, 28 bp, synthetic construct
  source 1..28: mol_type = other DNA
ggctgcccttgccagctcagacggctgg

SEQ ID NO: 47163 - DNA, 28 bp, synthetic construct
  source 1..28: mol_type = other DNA
actcgccagccgtctgagctggcaaggg

SEQ ID NO: 47164 - DNA, 28 bp, synthetic construct
  source 1..28: mol_type = other DNA
aactcgccagccgtctgagctggcaagg

SEQ ID NO: 47165 - DNA, 28 bp, synthetic construct
  source 1..28: mol_type = other DNA
ctgaaaactcgccagccgtctgagctgg

SEQ ID NO: 47166 - DNA, 28 bp, synthetic construct
  source 1..28: mol_type = other DNA
ggctggcgagttttcagcttccctaagg

SEQ ID NO: 47167 - DNA, 28 bp, synthetic construct
  source 1..28: mol_type = other DNA
gctggcgagttttcagcttccctaaggg

SEQ ID NO: 47168 - DNA, 28 bp, synthetic construct
  source 1..28: mol_type = other DNA
cgagttttcagcttccctaagggactgg

SEQ ID NO: 47169 - DNA, 28 bp, synthetic construct
  source 1..28: mol_type = other DNA
ttcagcttccctaagggactggcatagg

SEQ ID NO: 47170 - DNA, 28 bp, synthetic construct
  source 1..28: mol_type = other DNA
tcagcttccctaagggactggcataggg

SEQ ID NO: 47171 - DNA, 28 bp, synthetic construct
  source 1..28: mol_type = other DNA
cacaaaaccctatgccagtcccttaggg

SEQ ID NO: 47172 - DNA, 28 bp, synthetic construct
  source 1..28: mol_type = other DNA
ccacaaaaccctatgccagtcccttagg

SEQ ID NO: 47173 - DNA, 28 bp, synthetic construct
  source 1..28: mol_type = other DNA
ctaagggactggcatagggttttgtggg

SEQ ID NO: 47174 - DNA, 28 bp, synthetic construct
  source 1..28: mol_type = other DNA
taagggactggcatagggttttgtgggg

SEQ ID NO: 47175 - DNA, 28 bp, synthetic construct
  source 1..28: mol_type = other DNA
catagggttttgtggggtcaatgccagg

SEQ ID NO: 47176 - DNA, 28 bp, synthetic construct
  source 1..28: mol_type = other DNA
ttttgtggggtcaatgccaggaacctgg

SEQ ID NO: 47177 - DNA, 28 bp, synthetic construct
  source 1..28: mol_type = other DNA
tttgtggggtcaatgccaggaacctggg

SEQ ID NO: 47178 - DNA, 28 bp, synthetic construct
  source 1..28: mol_type = other DNA
ttgtggggtcaatgccaggaacctgggg

SEQ ID NO: 47179 - DNA, 28 bp, synthetic construct
  source 1..28: mol_type = other DNA
tgtggggtcaatgccaggaacctggggg

SEQ ID NO: 47180 - DNA, 28 bp, synthetic construct
  source 1..28: mol_type = other DNA
tcaatgccaggaacctgggggaaactgg

SEQ ID NO: 47181 - DNA, 28 bp, synthetic construct
  source 1..28: mol_type = other DNA
acgcatccagtttcccccaggttcctgg

SEQ ID NO: 47182 - DNA, 28 bp, synthetic construct
  source 1..28: mol_type = other DNA
ggataaaacgcatccagtttcccccagg

SEQ ID NO: 47183 - DNA, 28 bp, synthetic construct
  source 1..28: mol_type = other DNA
taagagcaggagggatgaacttcttagg

SEQ ID NO: 47184 - DNA, 28 bp, synthetic construct
  source 1..28: mol_type = other DNA
tcatccctcctgctcttactgtttccgg

SEQ ID NO: 47185 - DNA, 28 bp, synthetic construct
  source 1..28: mol_type = other DNA
agggccggaaacagtaagagcaggaggg

SEQ ID NO: 47186 - DNA, 28 bp, synthetic construct
  source 1..28: mol_type = other DNA
cagggccggaaacagtaagagcaggagg

SEQ ID NO: 47187 - DNA, 28 bp, synthetic construct
  source 1..28: mol_type = other DNA
ctcctgctcttactgtttccggccctgg

SEQ ID NO: 47188 - DNA, 28 bp, synthetic construct
  source 1..28: mol_type = other DNA
ctccagggccggaaacagtaagagcagg

SEQ ID NO: 47189 - DNA, 28 bp, synthetic construct
  source 1..28: mol_type = other DNA
ctgctcttactgtttccggccctggagg

SEQ ID NO: 47190 - DNA, 28 bp, synthetic construct
  source 1..28: mol_type = other DNA
ctgtttccggccctggaggagaatgagg

SEQ ID NO: 47191 - DNA, 28 bp, synthetic construct
  source 1..28: mol_type = other DNA
tgtttccggccctggaggagaatgaggg

SEQ ID NO: 47192 - DNA, 28 bp, synthetic construct
  source 1..28: mol_type = other DNA
ttccggccctggaggagaatgagggagg

SEQ ID NO: 47193 - DNA, 28 bp, synthetic construct
  source 1..28: mol_type = other DNA
ctcctccctcattctcctccagggccgg

SEQ ID NO: 47194 - DNA, 28 bp, synthetic construct
  source 1..28: mol_type = other DNA
gccctggaggagaatgagggaggagagg

SEQ ID NO: 47195 - DNA, 28 bp, synthetic construct
  source 1..28: mol_type = other DNA
ccctctcctccctcattctcctccaggg

SEQ ID NO: 47196 - DNA, 28 bp, synthetic construct
  source 1..28: mol_type = other DNA
accctctcctccctcattctcctccagg

SEQ ID NO: 47197 - DNA, 28 bp, synthetic construct
  source 1..28: mol_type = other DNA
tgtgttagcttttattattagcaagagg

SEQ ID NO: 47198 - DNA, 28 bp, synthetic construct
  source 1..28: mol_type = other DNA
gtgttagcttttattattagcaagaggg

SEQ ID NO: 47199 - DNA, 28 bp, synthetic construct
  source 1..28: mol_type = other DNA
atgaatttcatgcacaaattacaaaagg

SEQ ID NO: 47200 - DNA, 28 bp, synthetic construct
  source 1..28: mol_type = other DNA
tgtgcatgaaattcatgtcatttcctgg

SEQ ID NO: 47201 - DNA, 28 bp, synthetic construct
  source 1..28: mol_type = other DNA
gtgcatgaaattcatgtcatttcctggg

SEQ ID NO: 47202 - DNA, 28 bp, synthetic construct
  source 1..28: mol_type = other DNA
tgaaattcatgtcatttcctgggagagg

SEQ ID NO: 47203 - DNA, 28 bp, synthetic construct
  source 1..28: mol_type = other DNA
ttcatgtcatttcctgggagaggagagg

SEQ ID NO: 47204 - DNA, 28 bp, synthetic construct
  source 1..28: mol_type = other DNA
tcatgtcatttcctgggagaggagaggg

SEQ ID NO: 47205 - DNA, 28 bp, synthetic construct
  source 1..28: mol_type = other DNA
tttcctgggagaggagagggccgactgg

SEQ ID NO: 47206 - DNA, 28 bp, synthetic construct
  source 1..28: mol_type = other DNA
tctccagtcggccctctcctctcccagg

SEQ ID NO: 47207 - DNA, 28 bp, synthetic construct
  source 1..28: mol_type = other DNA
tgggagaggagagggccgactggagagg

SEQ ID NO: 47208 - DNA, 28 bp, synthetic construct
  source 1..28: mol_type = other DNA
gggagaggagagggccgactggagaggg

SEQ ID NO: 47209 - DNA, 28 bp, synthetic construct
  source 1..28: mol_type = other DNA
agaggagagggccgactggagagggtgg

SEQ ID NO: 47210 - DNA, 28 bp, synthetic construct
  source 1..28: mol_type = other DNA
gaggagagggccgactggagagggtggg

SEQ ID NO: 47211 - DNA, 28 bp, synthetic construct
  source 1..28: mol_type = other DNA
aggagagggccgactggagagggtgggg

SEQ ID NO: 47212 - DNA, 28 bp, synthetic construct
  source 1..28: mol_type = other DNA
ggagagggccgactggagagggtggggg

SEQ ID NO: 47213 - DNA, 28 bp, synthetic construct
  source 1..28: mol_type = other DNA
gagagggccgactggagagggtgggggg

SEQ ID NO: 47214 - DNA, 28 bp, synthetic construct
  source 1..28: mol_type = other DNA
cagtgtgccccccaccctctccagtcgg

SEQ ID NO: 47215 - DNA, 28 bp, synthetic construct
  source 1..28: mol_type = other DNA
cgactggagagggtggggggcacactgg

SEQ ID NO: 47216 - DNA, 28 bp, synthetic construct
  source 1..28: mol_type = other DNA
gactggagagggtggggggcacactggg

SEQ ID NO: 47217 - DNA, 28 bp, synthetic construct
  source 1..28: mol_type = other DNA
actggagagggtggggggcacactgggg

SEQ ID NO: 47218 - DNA, 28 bp, synthetic construct
  source 1..28: mol_type = other DNA
agggtggggggcacactggggaagcagg

SEQ ID NO: 47219 - DNA, 28 bp, synthetic construct
  source 1..28: mol_type = other DNA
gggggcacactggggaagcaggcagagg

SEQ ID NO: 47220 - DNA, 28 bp, synthetic construct
  source 1..28: mol_type = other DNA
gcaggcagaggtttccttcccttgtagg

SEQ ID NO: 47221 - DNA, 28 bp, synthetic construct
  source 1..28: mol_type = other DNA
caggcagaggtttccttcccttgtaggg

SEQ ID NO: 47222 - DNA, 28 bp, synthetic construct
  source 1..28: mol_type = other DNA
aggcagaggtttccttcccttgtagggg

SEQ ID NO: 47223 - DNA, 28 bp, synthetic construct
  source 1..28: mol_type = other DNA
ggcagaggtttccttcccttgtaggggg

SEQ ID NO: 47224 - DNA, 28 bp, synthetic construct
  source 1..28: mol_type = other DNA
gcagaggtttccttcccttgtagggggg

SEQ ID NO: 47225 - DNA, 28 bp, synthetic construct
  source 1..28: mol_type = other DNA
gaggtttccttcccttgtaggggggtgg

SEQ ID NO: 47226 - DNA, 28 bp, synthetic construct
  source 1..28: mol_type = other DNA
aggtttccttcccttgtaggggggtggg

SEQ ID NO: 47227 - DNA, 28 bp, synthetic construct
  source 1..28: mol_type = other DNA
ggtttccttcccttgtaggggggtgggg

SEQ ID NO: 47228 - DNA, 28 bp, synthetic construct
  source 1..28: mol_type = other DNA
actctccccacccccctacaagggaagg

SEQ ID NO: 47229 - DNA, 28 bp, synthetic construct
  source 1..28: mol_type = other DNA
ttcccttgtaggggggtggggagagtgg

SEQ ID NO: 47230 - DNA, 28 bp, synthetic construct
  source 1..28: mol_type = other DNA
tcccttgtaggggggtggggagagtggg

SEQ ID NO: 47231 - DNA, 28 bp, synthetic construct
  source 1..28: mol_type = other DNA
ccccactctccccacccccctacaaggg

SEQ ID NO: 47232 - DNA, 28 bp, synthetic construct
  source 1..28: mol_type = other DNA
tccccactctccccacccccctacaagg

SEQ ID NO: 47233 - DNA, 28 bp, synthetic construct
  source 1..28: mol_type = other DNA
gtaggggggtggggagagtggggagagg

SEQ ID NO: 47234 - DNA, 28 bp, synthetic construct
  source 1..28: mol_type = other DNA
taggggggtggggagagtggggagaggg

SEQ ID NO: 47235 - DNA, 28 bp, synthetic construct
  source 1..28: mol_type = other DNA
aggggggtggggagagtggggagagggg

SEQ ID NO: 47236 - DNA, 28 bp, synthetic construct
  source 1..28: mol_type = other DNA
ggggggtggggagagtggggagaggggg

SEQ ID NO: 47237 - DNA, 28 bp, synthetic construct
  source 1..28: mol_type = other DNA
ggggtgctatccagttcgcctgatgagg

SEQ ID NO: 47238 - DNA, 28 bp, synthetic construct
  source 1..28: mol_type = other DNA
gggtgctatccagttcgcctgatgaggg

SEQ ID NO: 47239 - DNA, 28 bp, synthetic construct
  source 1..28: mol_type = other DNA
gttcgagagccctcatcaggcgaactgg

SEQ ID NO: 47240 - DNA, 28 bp, synthetic construct
  source 1..28: mol_type = other DNA
aacggctggttcgagagccctcatcagg

SEQ ID NO: 47241 - DNA, 28 bp, synthetic construct
  source 1..28: mol_type = other DNA
atgagggctctcgaaccagccgttttgg

SEQ ID NO: 47242 - DNA, 28 bp, synthetic construct
  source 1..28: mol_type = other DNA
tgagggctctcgaaccagccgttttggg

SEQ ID NO: 47243 - DNA, 28 bp, synthetic construct
  source 1..28: mol_type = other DNA
aaccagccgttttgggttgtgttaaagg

SEQ ID NO: 47244 - DNA, 28 bp, synthetic construct
  source 1..28: mol_type = other DNA
cacctttaacacaacccaaaacggctgg

SEQ ID NO: 47245 - DNA, 28 bp, synthetic construct
  source 1..28: mol_type = other DNA
gtctcacctttaacacaacccaaaacgg

SEQ ID NO: 47246 - DNA, 28 bp, synthetic construct
  source 1..28: mol_type = other DNA
ttcgagattgtacattaatggaggaagg

SEQ ID NO: 47247 - DNA, 28 bp, synthetic construct
  source 1..28: mol_type = other DNA
ttagttcgagattgtacattaatggagg

SEQ ID NO: 47248 - DNA, 28 bp, synthetic construct
  source 1..28: mol_type = other DNA
cagttagttcgagattgtacattaatgg

SEQ ID NO: 47249 - DNA, 28 bp, synthetic construct
  source 1..28: mol_type = other DNA
aatctcgaactaactgctaataaagtgg

SEQ ID NO: 47250 - DNA, 28 bp, synthetic construct
  source 1..28: mol_type = other DNA
atctcgaactaactgctaataaagtggg

SEQ ID NO: 47251 - DNA, 28 bp, synthetic construct
  source 1..28: mol_type = other DNA
tctcgaactaactgctaataaagtgggg

SEQ ID NO: 47252 - DNA, 28 bp, synthetic construct
  source 1..28: mol_type = other DNA
ccttttaaaagaaatatttattgtgtgg

SEQ ID NO: 47253 - DNA, 28 bp, synthetic construct
  source 1..28: mol_type = other DNA
aaactagaaattgagaaaacagtgtagg

SEQ ID NO: 47254 - DNA, 28 bp, synthetic construct
  source 1..28: mol_type = other DNA
taaaataaagcctcccacaatcccaagg

SEQ ID NO: 47255 - DNA, 28 bp, synthetic construct
  source 1..28: mol_type = other DNA
tatctctggaccttgggattgtgggagg

SEQ ID NO: 47256 - DNA, 28 bp, synthetic construct
  source 1..28: mol_type = other DNA
tattatctctggaccttgggattgtggg

SEQ ID NO: 47257 - DNA, 28 bp, synthetic construct
  source 1..28: mol_type = other DNA
gtattatctctggaccttgggattgtgg

SEQ ID NO: 47258 - DNA, 28 bp, synthetic construct
  source 1..28: mol_type = other DNA
ttgagctgtattatctctggaccttggg

SEQ ID NO: 47259 - DNA, 28 bp, synthetic construct
  source 1..28: mol_type = other DNA
cttgagctgtattatctctggaccttgg

SEQ ID NO: 47260 - DNA, 28 bp, synthetic construct
  source 1..28: mol_type = other DNA
tccagagataatacagctcaagaattgg

SEQ ID NO: 47261 - DNA, 28 bp, synthetic construct
  source 1..28: mol_type = other DNA
accaattcttgagctgtattatctctgg

SEQ ID NO: 47262 - DNA, 28 bp, synthetic construct
  source 1..28: mol_type = other DNA
gagagacagagaaaaaaaaggaagaagg

SEQ ID NO: 47263 - DNA, 28 bp, synthetic construct
  source 1..28: mol_type = other DNA
gcagatggagagacagagaaaaaaaagg

SEQ ID NO: 47264 - DNA, 28 bp, synthetic construct
  source 1..28: mol_type = other DNA
caggttgtacacatacagatgcagatgg

SEQ ID NO: 47265 - DNA, 28 bp, synthetic construct
  source 1..28: mol_type = other DNA
tgggtgaagagcaagaagagaaaacagg

SEQ ID NO: 47266 - DNA, 28 bp, synthetic construct
  source 1..28: mol_type = other DNA
cttcttgctcttcacccacaaaagcagg

SEQ ID NO: 47267 - DNA, 28 bp, synthetic construct
  source 1..28: mol_type = other DNA
caaaaggctggatgcctgcttttgtggg

SEQ ID NO: 47268 - DNA, 28 bp, synthetic construct
  source 1..28: mol_type = other DNA
tcaaaaggctggatgcctgcttttgtgg

SEQ ID NO: 47269 - DNA, 28 bp, synthetic construct
  source 1..28: mol_type = other DNA
atcatatgcgagatgctcaaaaggctgg

SEQ ID NO: 47270 - DNA, 28 bp, synthetic construct
  source 1..28: mol_type = other DNA
cttaatcatatgcgagatgctcaaaagg

SEQ ID NO: 47271 - DNA, 28 bp, synthetic construct
  source 1..28: mol_type = other DNA
gggcttaggtgaggcaggtctttgaagg

SEQ ID NO: 47272 - DNA, 28 bp, synthetic construct
  source 1..28: mol_type = other DNA
tctgagaaatgggcttaggtgaggcagg

SEQ ID NO: 47273 - DNA, 28 bp, synthetic construct
  source 1..28: mol_type = other DNA
tgggtctgagaaatgggcttaggtgagg

SEQ ID NO: 47274 - DNA, 28 bp, synthetic construct
  source 1..28: mol_type = other DNA
gcaggtgggtctgagaaatgggcttagg

SEQ ID NO: 47275 - DNA, 28 bp, synthetic construct
  source 1..28: mol_type = other DNA
taagcccatttctcagacccacctgcgg

SEQ ID NO: 47276 - DNA, 28 bp, synthetic construct
  source 1..28: mol_type = other DNA
tagaccgcaggtgggtctgagaaatggg

SEQ ID NO: 47277 - DNA, 28 bp, synthetic construct
  source 1..28: mol_type = other DNA
gtagaccgcaggtgggtctgagaaatgg

SEQ ID NO: 47278 - DNA, 28 bp, synthetic construct
  source 1..28: mol_type = other DNA
tctcagacccacctgcggtctactcagg

SEQ ID NO: 47279 - DNA, 28 bp, synthetic construct
  source 1..28: mol_type = other DNA
aaggaggcctgagtagaccgcaggtggg

SEQ ID NO: 47280 - DNA, 28 bp, synthetic construct
  source 1..28: mol_type = other DNA
caaggaggcctgagtagaccgcaggtgg

SEQ ID NO: 47281 - DNA, 28 bp, synthetic construct
  source 1..28: mol_type = other DNA
tgacaaggaggcctgagtagaccgcagg

SEQ ID NO: 47282 - DNA, 28 bp, synthetic construct
  source 1..28: mol_type = other DNA
agagagggcttggtggatgacaaggagg

SEQ ID NO: 47283 - DNA, 28 bp, synthetic construct
  source 1..28: mol_type = other DNA
tccttgtcatccaccaagccctctctgg

SEQ ID NO: 47284 - DNA, 28 bp, synthetic construct
  source 1..28: mol_type = other DNA
gccagagagggcttggtggatgacaagg

SEQ ID NO: 47285 - DNA, 28 bp, synthetic construct
  source 1..28: mol_type = other DNA
tccaccaagccctctctggcttcattgg

SEQ ID NO: 47286 - DNA, 28 bp, synthetic construct
  source 1..28: mol_type = other DNA
accaatgaagccagagagggcttggtgg

SEQ ID NO: 47287 - DNA, 28 bp, synthetic construct
  source 1..28: mol_type = other DNA
agtaccaatgaagccagagagggcttgg

SEQ ID NO: 47288 - DNA, 28 bp, synthetic construct
  source 1..28: mol_type = other DNA
gcggcagtaccaatgaagccagagaggg

SEQ ID NO: 47289 - DNA, 28 bp, synthetic construct
  source 1..28: mol_type = other DNA
tgcggcagtaccaatgaagccagagagg

SEQ ID NO: 47290 - DNA, 28 bp, synthetic construct
  source 1..28: mol_type = other DNA
tctctggcttcattggtactgccgcagg

SEQ ID NO: 47291 - DNA, 28 bp, synthetic construct
  source 1..28: mol_type = other DNA
cttcattggtactgccgcaggctgctgg

SEQ ID NO: 47292 - DNA, 28 bp, synthetic construct
  source 1..28: mol_type = other DNA
ttcattggtactgccgcaggctgctggg

SEQ ID NO: 47293 - DNA, 28 bp, synthetic construct
  source 1..28: mol_type = other DNA
ggagatactagtgcccagcagcctgcgg

SEQ ID NO: 47294 - DNA, 28 bp, synthetic construct
  source 1..28: mol_type = other DNA
caggctgctgggcactagtatctcctgg

SEQ ID NO: 47295 - DNA, 28 bp, synthetic construct
  source 1..28: mol_type = other DNA
tctcctggcgtctctgttgcacctgagg

SEQ ID NO: 47296 - DNA, 28 bp, synthetic construct
  source 1..28: mol_type = other DNA
gaacctcaggtgcaacagagacgccagg

SEQ ID NO: 47297 - DNA, 28 bp, synthetic construct
  source 1..28: mol_type = other DNA
cgtctctgttgcacctgaggttccacgg

SEQ ID NO: 47298 - DNA, 28 bp, synthetic construct
  source 1..28: mol_type = other DNA
tctgttgcacctgaggttccacggctgg

SEQ ID NO: 47299 - DNA, 28 bp, synthetic construct
  source 1..28: mol_type = other DNA
ttgcacctgaggttccacggctggctgg

SEQ ID NO: 47300 - DNA, 28 bp, synthetic construct
  source 1..28: mol_type = other DNA
gaacaccagccagccgtggaacctcagg

SEQ ID NO: 47301 - DNA, 28 bp, synthetic construct
  source 1..28: mol_type = other DNA
tccacggctggctggtgttccttcctgg

SEQ ID NO: 47302 - DNA, 28 bp, synthetic construct
  source 1..28: mol_type = other DNA
tccaggaaggaacaccagccagccgtgg

SEQ ID NO: 47303 - DNA, 28 bp, synthetic construct
  source 1..28: mol_type = other DNA
ggctggctggtgttccttcctggaatgg

SEQ ID NO: 47304 - DNA, 28 bp, synthetic construct
  source 1..28: mol_type = other DNA
tggctggtgttccttcctggaatggagg

SEQ ID NO: 47305 - DNA, 28 bp, synthetic construct
  source 1..28: mol_type = other DNA
ggctggtgttccttcctggaatggaggg

SEQ ID NO: 47306 - DNA, 28 bp, synthetic construct
  source 1..28: mol_type = other DNA
tgattgttctccctccattccaggaagg

SEQ ID NO: 47307 - DNA, 28 bp, synthetic construct
  source 1..28: mol_type = other DNA
caagtgattgttctccctccattccagg

SEQ ID NO: 47308 - DNA, 28 bp, synthetic construct
  source 1..28: mol_type = other DNA
ctggaatggagggagaacaatcacttgg

SEQ ID NO: 47309 - DNA, 28 bp, synthetic construct
  source 1..28: mol_type = other DNA
tggatttatttgagtcccagtagattgg

SEQ ID NO: 47310 - DNA, 28 bp, synthetic construct
  source 1..28: mol_type = other DNA
ttatttgagtcccagtagattggagagg

SEQ ID NO: 47311 - DNA, 28 bp, synthetic construct
  source 1..28: mol_type = other DNA
gtcccagtagattggagaggtccactgg

SEQ ID NO: 47312 - DNA, 28 bp, synthetic construct
  source 1..28: mol_type = other DNA
ggccagtggacctctccaatctactggg

SEQ ID NO: 47313 - DNA, 28 bp, synthetic construct
  source 1..28: mol_type = other DNA
cggccagtggacctctccaatctactgg

SEQ ID NO: 47314 - DNA, 28 bp, synthetic construct
  source 1..28: mol_type = other DNA
cagtagattggagaggtccactggccgg

SEQ ID NO: 47315 - DNA, 28 bp, synthetic construct
  source 1..28: mol_type = other DNA
tgctgcaactaacaaagccggccagtgg

SEQ ID NO: 47316 - DNA, 28 bp, synthetic construct
  source 1..28: mol_type = other DNA
ttggatttgctgcaactaacaaagccgg

SEQ ID NO: 47317 - DNA, 28 bp, synthetic construct
  source 1..28: mol_type = other DNA
ggagttctctgatggcagtttgagttgg

SEQ ID NO: 47318 - DNA, 28 bp, synthetic construct
  source 1..28: mol_type = other DNA
cagccagtcgggactgctgtgcctatgg

SEQ ID NO: 47319 - DNA, 28 bp, synthetic construct
  source 1..28: mol_type = other DNA
actccataggcacagcagtcccgactgg

SEQ ID NO: 47320 - DNA, 28 bp, synthetic construct
  source 1..28: mol_type = other DNA
gtcgggactgctgtgcctatggagtagg

SEQ ID NO: 47321 - DNA, 28 bp, synthetic construct
  source 1..28: mol_type = other DNA
aggaataagaagttacctactccatagg

SEQ ID NO: 47322 - DNA, 28 bp, synthetic construct
  source 1..28: mol_type = other DNA
tacaaaaaagaaaaaatgaaaataaagg

SEQ ID NO: 47323 - DNA, 28 bp, synthetic construct
  source 1..28: mol_type = other DNA
tttaagtaaaaaatttttaatttatagg

SEQ ID NO: 47324 - DNA, 28 bp, synthetic construct
  source 1..28: mol_type = other DNA
ttaagtaaaaaatttttaatttataggg

SEQ ID NO: 47325 - DNA, 28 bp, synthetic construct
  source 1..28: mol_type = other DNA
taagtaaaaaatttttaatttatagggg

SEQ ID NO: 47326 - DNA, 28 bp, synthetic construct
  source 1..28: mol_type = other DNA
aaatttttaatttataggggttttctgg

SEQ ID NO: 47327 - DNA, 28 bp, synthetic construct
  source 1..28: mol_type = other DNA
tttataggggttttctggtaaaaactgg

SEQ ID NO: 47328 - DNA, 28 bp, synthetic construct
  source 1..28: mol_type = other DNA
acagctcttttagaatttgtctagcagg

SEQ ID NO: 47329 - DNA, 28 bp, synthetic construct
  source 1..28: mol_type = other DNA
ggaaggaagtttattcagaaaataaagg

SEQ ID NO: 47330 - DNA, 28 bp, synthetic construct
  source 1..28: mol_type = other DNA
taaacttccttccactttactctgttgg

SEQ ID NO: 47331 - DNA, 28 bp, synthetic construct
  source 1..28: mol_type = other DNA
gagcaagccaacagagtaaagtggaagg

SEQ ID NO: 47332 - DNA, 28 bp, synthetic construct
  source 1..28: mol_type = other DNA
acaagagcaagccaacagagtaaagtgg

SEQ ID NO: 47333 - DNA, 28 bp, synthetic construct
  source 1..28: mol_type = other DNA
tcctgtacaaagccaagaatccacgtgg

SEQ ID NO: 47334 - DNA, 28 bp, synthetic construct
  source 1..28: mol_type = other DNA
gccacgtggattcttggctttgtacagg

SEQ ID NO: 47335 - DNA, 28 bp, synthetic construct
  source 1..28: mol_type = other DNA
cagcgtgggaggccacgtggattcttgg

SEQ ID NO: 47336 - DNA, 28 bp, synthetic construct
  source 1..28: mol_type = other DNA
ttggggttcagcgtgggaggccacgtgg

SEQ ID NO: 47337 - DNA, 28 bp, synthetic construct
  source 1..28: mol_type = other DNA
ggcctcccacgctgaaccccaattttgg

SEQ ID NO: 47338 - DNA, 28 bp, synthetic construct
  source 1..28: mol_type = other DNA
gcctcccacgctgaaccccaattttggg

SEQ ID NO: 47339 - DNA, 28 bp, synthetic construct
  source 1..28: mol_type = other DNA
ccccaaaattggggttcagcgtgggagg

SEQ ID NO: 47340 - DNA, 28 bp, synthetic construct
  source 1..28: mol_type = other DNA
gagccccaaaattggggttcagcgtggg

SEQ ID NO: 47341 - DNA, 28 bp, synthetic construct
  source 1..28: mol_type = other DNA
tgagccccaaaattggggttcagcgtgg

SEQ ID NO: 47342 - DNA, 28 bp, synthetic construct
  source 1..28: mol_type = other DNA
tgtcacagggtgagccccaaaattgggg

SEQ ID NO: 47343 - DNA, 28 bp, synthetic construct
  source 1..28: mol_type = other DNA
gtgtcacagggtgagccccaaaattggg

SEQ ID NO: 47344 - DNA, 28 bp, synthetic construct
  source 1..28: mol_type = other DNA
tgtgtcacagggtgagccccaaaattgg

SEQ ID NO: 47345 - DNA, 28 bp, synthetic construct
  source 1..28: mol_type = other DNA
ggggctcaccctgtgacacagccagagg

SEQ ID NO: 47346 - DNA, 28 bp, synthetic construct
  source 1..28: mol_type = other DNA
accctgtgacacagccagaggcaaatgg

SEQ ID NO: 47347 - DNA, 28 bp, synthetic construct
  source 1..28: mol_type = other DNA
accatttgcctctggctgtgtcacaggg

SEQ ID NO: 47348 - DNA, 28 bp, synthetic construct
  source 1..28: mol_type = other DNA
aaccatttgcctctggctgtgtcacagg

SEQ ID NO: 47349 - DNA, 28 bp, synthetic construct
  source 1..28: mol_type = other DNA
ggagggacatggaaccatttgcctctgg

SEQ ID NO: 47350 - DNA, 28 bp, synthetic construct
  source 1..28: mol_type = other DNA
ggcgcaaagaggaataggagggacatgg

SEQ ID NO: 47351 - DNA, 28 bp, synthetic construct
  source 1..28: mol_type = other DNA
tgtccctcctattcctctttgcgcctgg

SEQ ID NO: 47352 - DNA, 28 bp, synthetic construct
  source 1..28: mol_type = other DNA
catccaggcgcaaagaggaataggaggg

SEQ ID NO: 47353 - DNA, 28 bp, synthetic construct
  source 1..28: mol_type = other DNA
cctcctattcctctttgcgcctggatgg

SEQ ID NO: 47354 - DNA, 28 bp, synthetic construct
  source 1..28: mol_type = other DNA
ctcctattcctctttgcgcctggatggg

SEQ ID NO: 47355 - DNA, 28 bp, synthetic construct
  source 1..28: mol_type = other DNA
atcccatccaggcgcaaagaggaatagg

SEQ ID NO: 47356 - DNA, 28 bp, synthetic construct
  source 1..28: mol_type = other DNA
ttcctctttgcgcctggatgggatccgg

SEQ ID NO: 47357 - DNA, 28 bp, synthetic construct
  source 1..28: mol_type = other DNA
ctccggatcccatccaggcgcaaagagg

SEQ ID NO: 47358 - DNA, 28 bp, synthetic construct
  source 1..28: mol_type = other DNA
ctctttgcgcctggatgggatccggagg

SEQ ID NO: 47359 - DNA, 28 bp, synthetic construct
  source 1..28: mol_type = other DNA
tctttgcgcctggatgggatccggaggg

SEQ ID NO: 47360 - DNA, 28 bp, synthetic construct
  source 1..28: mol_type = other DNA
gcctggatgggatccggagggctctagg

SEQ ID NO: 47361 - DNA, 28 bp, synthetic construct
  source 1..28: mol_type = other DNA
gcctagagccctccggatcccatccagg

SEQ ID NO: 47362 - DNA, 28 bp, synthetic construct
  source 1..28: mol_type = other DNA
gatgggatccggagggctctaggcttgg

SEQ ID NO: 47363 - DNA, 28 bp, synthetic construct
  source 1..28: mol_type = other DNA
cacagcagccaagcctagagccctccgg

SEQ ID NO: 47364 - DNA, 28 bp, synthetic construct
  source 1..28: mol_type = other DNA
cggagggctctaggcttggctgctgtgg

SEQ ID NO: 47365 - DNA, 28 bp, synthetic construct
  source 1..28: mol_type = other DNA
gcttggctgctgtggccaccagatgagg

SEQ ID NO: 47366 - DNA, 28 bp, synthetic construct
  source 1..28: mol_type = other DNA
tgtggccaccagatgaggctctatgagg

SEQ ID NO: 47367 - DNA, 28 bp, synthetic construct
  source 1..28: mol_type = other DNA
gcagacctcatagagcctcatctggtgg

SEQ ID NO: 47368 - DNA, 28 bp, synthetic construct
  source 1..28: mol_type = other DNA
ccagatgaggctctatgaggtctgcagg

SEQ ID NO: 47369 - DNA, 28 bp, synthetic construct
  source 1..28: mol_type = other DNA
cagatgaggctctatgaggtctgcaggg

SEQ ID NO: 47370 - DNA, 28 bp, synthetic construct
  source 1..28: mol_type = other DNA
agatgaggctctatgaggtctgcagggg

SEQ ID NO: 47371 - DNA, 28 bp, synthetic construct
  source 1..28: mol_type = other DNA
ctgcaggggtcttgccagctccagatgg

SEQ ID NO: 47372 - DNA, 28 bp, synthetic construct
  source 1..28: mol_type = other DNA
atctcagggaatgtccatctggagctgg

SEQ ID NO: 47373 - DNA, 28 bp, synthetic construct
  source 1..28: mol_type = other DNA
aacagcatctcagggaatgtccatctgg

SEQ ID NO: 47374 - DNA, 28 bp, synthetic construct
  source 1..28: mol_type = other DNA
gatggacattccctgagatgctgttagg

SEQ ID NO: 47375 - DNA, 28 bp, synthetic construct
  source 1..28: mol_type = other DNA
ttccctgagatgctgttaggccacctgg

SEQ ID NO: 47376 - DNA, 28 bp, synthetic construct
  source 1..28: mol_type = other DNA
gtccaggtggcctaacagcatctcaggg

SEQ ID NO: 47377 - DNA, 28 bp, synthetic construct
  source 1..28: mol_type = other DNA
agtccaggtggcctaacagcatctcagg

SEQ ID NO: 47378 - DNA, 28 bp, synthetic construct
  source 1..28: mol_type = other DNA
tgagatgctgttaggccacctggactgg

SEQ ID NO: 47379 - DNA, 28 bp, synthetic construct
  source 1..28: mol_type = other DNA
gagatgctgttaggccacctggactggg

SEQ ID NO: 47380 - DNA, 28 bp, synthetic construct
  source 1..28: mol_type = other DNA
agatgctgttaggccacctggactgggg

SEQ ID NO: 47381 - DNA, 28 bp, synthetic construct
  source 1..28: mol_type = other DNA
aggccacctggactggggccccctgtgg

SEQ ID NO: 47382 - DNA, 28 bp, synthetic construct
  source 1..28: mol_type = other DNA
atgccacagggggccccagtccaggtgg

SEQ ID NO: 47383 - DNA, 28 bp, synthetic construct
  source 1..28: mol_type = other DNA
gggatgccacagggggccccagtccagg

SEQ ID NO: 47384 - DNA, 28 bp, synthetic construct
  source 1..28: mol_type = other DNA
ggactggggccccctgtggcatccctgg

SEQ ID NO: 47385 - DNA, 28 bp, synthetic construct
  source 1..28: mol_type = other DNA
ggggccccctgtggcatccctggcatgg

SEQ ID NO: 47386 - DNA, 28 bp, synthetic construct
  source 1..28: mol_type = other DNA
gtgtccatgccagggatgccacaggggg

SEQ ID NO: 47387 - DNA, 28 bp, synthetic construct
  source 1..28: mol_type = other DNA
tgtgtccatgccagggatgccacagggg

SEQ ID NO: 47388 - DNA, 28 bp, synthetic construct
  source 1..28: mol_type = other DNA
atgtgtccatgccagggatgccacaggg

SEQ ID NO: 47389 - DNA, 28 bp, synthetic construct
  source 1..28: mol_type = other DNA
tatgtgtccatgccagggatgccacagg

SEQ ID NO: 47390 - DNA, 28 bp, synthetic construct
  source 1..28: mol_type = other DNA
tgctgggcattatgtgtccatgccaggg

SEQ ID NO: 47391 - DNA, 28 bp, synthetic construct
  source 1..28: mol_type = other DNA
ttgctgggcattatgtgtccatgccagg

SEQ ID NO: 47392 - DNA, 28 bp, synthetic construct
  source 1..28: mol_type = other DNA
ggcatggacacataatgcccagcaaagg

SEQ ID NO: 47393 - DNA, 28 bp, synthetic construct
  source 1..28: mol_type = other DNA
atggaactttgatgatgcctttgctggg

SEQ ID NO: 47394 - DNA, 28 bp, synthetic construct
  source 1..28: mol_type = other DNA
aatggaactttgatgatgcctttgctgg

SEQ ID NO: 47395 - DNA, 28 bp, synthetic construct
  source 1..28: mol_type = other DNA
catcaaagttccattactttagtgctgg

SEQ ID NO: 47396 - DNA, 28 bp, synthetic construct
  source 1..28: mol_type = other DNA
aaagttccattactttagtgctggaagg

SEQ ID NO: 47397 - DNA, 28 bp, synthetic construct
  source 1..28: mol_type = other DNA
ggtttgccttccagcactaaagtaatgg

SEQ ID NO: 47398 - DNA, 28 bp, synthetic construct
  source 1..28: mol_type = other DNA
ctttagtgctggaaggcaaaccagatgg

SEQ ID NO: 47399 - DNA, 28 bp, synthetic construct
  source 1..28: mol_type = other DNA
ctttctctgcaaacaagttgccatctgg

SEQ ID NO: 47400 - DNA, 28 bp, synthetic construct
  source 1..28: mol_type = other DNA
agagaaagaaactgagacccaaagaagg

SEQ ID NO: 47401 - DNA, 28 bp, synthetic construct
  source 1..28: mol_type = other DNA
gagaaagaaactgagacccaaagaaggg

SEQ ID NO: 47402 - DNA, 28 bp, synthetic construct
  source 1..28: mol_type = other DNA
acccaaagaagggtcagccaaagccagg

SEQ ID NO: 47403 - DNA, 28 bp, synthetic construct
  source 1..28: mol_type = other DNA
tcctggctttggctgacccttctttggg

SEQ ID NO: 47404 - DNA, 28 bp, synthetic construct
  source 1..28: mol_type = other DNA
gtcctggctttggctgacccttctttgg

SEQ ID NO: 47405 - DNA, 28 bp, synthetic construct
  source 1..28: mol_type = other DNA
aagggtcagccaaagccaggactcaagg

SEQ ID NO: 47406 - DNA, 28 bp, synthetic construct
  source 1..28: mol_type = other DNA
agggtcagccaaagccaggactcaaggg

SEQ ID NO: 47407 - DNA, 28 bp, synthetic construct
  source 1..28: mol_type = other DNA
agccaaagccaggactcaagggtcaagg

SEQ ID NO: 47408 - DNA, 28 bp, synthetic construct
  source 1..28: mol_type = other DNA
gccaaagccaggactcaagggtcaaggg

SEQ ID NO: 47409 - DNA, 28 bp, synthetic construct
  source 1..28: mol_type = other DNA
gcccttgacccttgagtcctggctttgg

SEQ ID NO: 47410 - DNA, 28 bp, synthetic construct
  source 1..28: mol_type = other DNA
aagccaggactcaagggtcaagggctgg

SEQ ID NO: 47411 - DNA, 28 bp, synthetic construct
  source 1..28: mol_type = other DNA
acaccagcccttgacccttgagtcctgg

SEQ ID NO: 47412 - DNA, 28 bp, synthetic construct
  source 1..28: mol_type = other DNA
tggtgttgatacttcagctgctgagtgg

SEQ ID NO: 47413 - DNA, 28 bp, synthetic construct
  source 1..28: mol_type = other DNA
gttgatacttcagctgctgagtggcagg

SEQ ID NO: 47414 - DNA, 28 bp, synthetic construct
  source 1..28: mol_type = other DNA
aactctgggagaagggcagcaaaaaggg

SEQ ID NO: 47415 - DNA, 28 bp, synthetic construct
  source 1..28: mol_type = other DNA
gaactctgggagaagggcagcaaaaagg

SEQ ID NO: 47416 - DNA, 28 bp, synthetic construct
  source 1..28: mol_type = other DNA
gcccttctcccagagttccataatgagg

SEQ ID NO: 47417 - DNA, 28 bp, synthetic construct
  source 1..28: mol_type = other DNA
acctcattatggaactctgggagaaggg

SEQ ID NO: 47418 - DNA, 28 bp, synthetic construct
  source 1..28: mol_type = other DNA
cacctcattatggaactctgggagaagg

SEQ ID NO: 47419 - DNA, 28 bp, synthetic construct
  source 1..28: mol_type = other DNA
tctcccagagttccataatgaggtgagg

SEQ ID NO: 47420 - DNA, 28 bp, synthetic construct
  source 1..28: mol_type = other DNA
catcctcacctcattatggaactctggg

SEQ ID NO: 47421 - DNA, 28 bp, synthetic construct
  source 1..28: mol_type = other DNA
ccagagttccataatgaggtgaggatgg

SEQ ID NO: 47422 - DNA, 28 bp, synthetic construct
  source 1..28: mol_type = other DNA
cagagttccataatgaggtgaggatggg

SEQ ID NO: 47423 - DNA, 28 bp, synthetic construct
  source 1..28: mol_type = other DNA
aaggagacccatcctcacctcattatgg

SEQ ID NO: 47424 - DNA, 28 bp, synthetic construct
  source 1..28: mol_type = other DNA
aatgaggtgaggatgggtctccttcagg

SEQ ID NO: 47425 - DNA, 28 bp, synthetic construct
  source 1..28: mol_type = other DNA
atgaggtgaggatgggtctccttcaggg

SEQ ID NO: 47426 - DNA, 28 bp, synthetic construct
  source 1..28: mol_type = other DNA
gtgaggatgggtctccttcagggcttgg

SEQ ID NO: 47427 - DNA, 28 bp, synthetic construct
  source 1..28: mol_type = other DNA
aaagatggactctaccaagccctgaagg

SEQ ID NO: 47428 - DNA, 28 bp, synthetic construct
  source 1..28: mol_type = other DNA
ttggtagagtccatctttgcacttccgg

SEQ ID NO: 47429 - DNA, 28 bp, synthetic construct
  source 1..28: mol_type = other DNA
agtccatctttgcacttccggtcccagg

SEQ ID NO: 47430 - DNA, 28 bp, synthetic construct
  source 1..28: mol_type = other DNA
agtcctgggaccggaagtgcaaagatgg

SEQ ID NO: 47431 - DNA, 28 bp, synthetic construct
  source 1..28: mol_type = other DNA
atctttgcacttccggtcccaggactgg

SEQ ID NO: 47432 - DNA, 28 bp, synthetic construct
  source 1..28: mol_type = other DNA
gttcagcttgagccagtcctgggaccgg

SEQ ID NO: 47433 - DNA, 28 bp, synthetic construct
  source 1..28: mol_type = other DNA
aagctgttcagcttgagccagtcctggg

SEQ ID NO: 47434 - DNA, 28 bp, synthetic construct
  source 1..28: mol_type = other DNA
gaagctgttcagcttgagccagtcctgg

SEQ ID NO: 47435 - DNA, 28 bp, synthetic construct
  source 1..28: mol_type = other DNA
gctcaagctgaacagcttccgcatctgg

SEQ ID NO: 47436 - DNA, 28 bp, synthetic construct
  source 1..28: mol_type = other DNA
aagctgaacagcttccgcatctggctgg

SEQ ID NO: 47437 - DNA, 28 bp, synthetic construct
  source 1..28: mol_type = other DNA
agctgaacagcttccgcatctggctggg

SEQ ID NO: 47438 - DNA, 28 bp, synthetic construct
  source 1..28: mol_type = other DNA
tgagaacacgaggcccagccagatgcgg

SEQ ID NO: 47439 - DNA, 28 bp, synthetic construct
  source 1..28: mol_type = other DNA
cgagagggtgctggctgagaacacgagg

SEQ ID NO: 47440 - DNA, 28 bp, synthetic construct
  source 1..28: mol_type = other DNA
agccagcaccctctcgtactgctcctgg

SEQ ID NO: 47441 - DNA, 28 bp, synthetic construct
  source 1..28: mol_type = other DNA
agccaggagcagtacgagagggtgctgg

SEQ ID NO: 47442 - DNA, 28 bp, synthetic construct
  source 1..28: mol_type = other DNA
gtgctgagccaggagcagtacgagaggg

SEQ ID NO: 47443 - DNA, 28 bp, synthetic construct
  source 1..28: mol_type = other DNA
ggtgctgagccaggagcagtacgagagg

SEQ ID NO: 47444 - DNA, 28 bp, synthetic construct
  source 1..28: mol_type = other DNA
aaactgcatggacaggtgctgagccagg

SEQ ID NO: 47445 - DNA, 28 bp, synthetic construct
  source 1..28: mol_type = other DNA
gttgtcttggacaaactgcatggacagg

SEQ ID NO: 47446 - DNA, 28 bp, synthetic construct
  source 1..28: mol_type = other DNA
tggaggttgtcttggacaaactgcatgg

SEQ ID NO: 47447 - DNA, 28 bp, synthetic construct
  source 1..28: mol_type = other DNA
cgagtgacatcggtggaggttgtcttgg

SEQ ID NO: 47448 - DNA, 28 bp, synthetic construct
  source 1..28: mol_type = other DNA
caagacaacctccaccgatgtcactcgg

SEQ ID NO: 47449 - DNA, 28 bp, synthetic construct
  source 1..28: mol_type = other DNA
aagacaacctccaccgatgtcactcggg

SEQ ID NO: 47450 - DNA, 28 bp, synthetic construct
  source 1..28: mol_type = other DNA
ctgatagcccgagtgacatcggtggagg

SEQ ID NO: 47451 - DNA, 28 bp, synthetic construct
  source 1..28: mol_type = other DNA
cagctgatagcccgagtgacatcggtgg

SEQ ID NO: 47452 - DNA, 28 bp, synthetic construct
  source 1..28: mol_type = other DNA
gagcagctgatagcccgagtgacatcgg

SEQ ID NO: 47453 - DNA, 28 bp, synthetic construct
  source 1..28: mol_type = other DNA
tcgggctatcagctgctctcgatactgg

SEQ ID NO: 47454 - DNA, 28 bp, synthetic construct
  source 1..28: mol_type = other DNA
actggtccacaaagtgcagcaactgcgg

SEQ ID NO: 47455 - DNA, 28 bp, synthetic construct
  source 1..28: mol_type = other DNA
ctggtccacaaagtgcagcaactgcggg

SEQ ID NO: 47456 - DNA, 28 bp, synthetic construct
  source 1..28: mol_type = other DNA
tggtccacaaagtgcagcaactgcgggg

SEQ ID NO: 47457 - DNA, 28 bp, synthetic construct
  source 1..28: mol_type = other DNA
gatgccccgcagttgctgcactttgtgg

SEQ ID NO: 47458 - DNA, 28 bp, synthetic construct
  source 1..28: mol_type = other DNA
agtgcagcaactgcggggcatccagagg

SEQ ID NO: 47459 - DNA, 28 bp, synthetic construct
  source 1..28: mol_type = other DNA
gcaactgcggggcatccagaggtgaagg

SEQ ID NO: 47460 - DNA, 28 bp, synthetic construct
  source 1..28: mol_type = other DNA
tgcggggcatccagaggtgaaggtacgg

SEQ ID NO: 47461 - DNA, 28 bp, synthetic construct
  source 1..28: mol_type = other DNA
gggcatccagaggtgaaggtacggctgg

SEQ ID NO: 47462 - DNA, 28 bp, synthetic construct
  source 1..28: mol_type = other DNA
tcgttgccagccgtaccttcacctctgg

SEQ ID NO: 47463 - DNA, 28 bp, synthetic construct
  source 1..28: mol_type = other DNA
aggtacggctggcaacgaacaaagaagg

SEQ ID NO: 47464 - DNA, 28 bp, synthetic construct
  source 1..28: mol_type = other DNA
ggtacggctggcaacgaacaaagaaggg

SEQ ID NO: 47465 - DNA, 28 bp, synthetic construct
  source 1..28: mol_type = other DNA
ggggattggaggtggaggctgtggttgg

SEQ ID NO: 47466 - DNA, 28 bp, synthetic construct
  source 1..28: mol_type = other DNA
aggtggggattggaggtggaggctgtgg

SEQ ID NO: 47467 - DNA, 28 bp, synthetic construct
  source 1..28: mol_type = other DNA
cactgaaggtggggattggaggtggagg

SEQ ID NO: 47468 - DNA, 28 bp, synthetic construct
  source 1..28: mol_type = other DNA
aagcactgaaggtggggattggaggtgg

SEQ ID NO: 47469 - DNA, 28 bp, synthetic construct
  source 1..28: mol_type = other DNA
ggaaagcactgaaggtggggattggagg

SEQ ID NO: 47470 - DNA, 28 bp, synthetic construct
  source 1..28: mol_type = other DNA
agaggaaagcactgaaggtggggattgg

SEQ ID NO: 47471 - DNA, 28 bp, synthetic construct
  source 1..28: mol_type = other DNA
atgagagaggaaagcactgaaggtgggg

SEQ ID NO: 47472 - DNA, 28 bp, synthetic construct
  source 1..28: mol_type = other DNA
gatgagagaggaaagcactgaaggtggg

SEQ ID NO: 47473 - DNA, 28 bp, synthetic construct
  source 1..28: mol_type = other DNA
agatgagagaggaaagcactgaaggtgg

SEQ ID NO: 47474 - DNA, 28 bp, synthetic construct
  source 1..28: mol_type = other DNA
cagagatgagagaggaaagcactgaagg

SEQ ID NO: 47475 - DNA, 28 bp, synthetic construct
  source 1..28: mol_type = other DNA
gaagcgagggatgcagagatgagagagg

SEQ ID NO: 47476 - DNA, 28 bp, synthetic construct
  source 1..28: mol_type = other DNA
catttctggaggcagaaggaagcgaggg

SEQ ID NO: 47477 - DNA, 28 bp, synthetic construct
  source 1..28: mol_type = other DNA
gcatttctggaggcagaaggaagcgagg

SEQ ID NO: 47478 - DNA, 28 bp, synthetic construct
  source 1..28: mol_type = other DNA
acacaggtgcatttctggaggcagaagg

SEQ ID NO: 47479 - DNA, 28 bp, synthetic construct
  source 1..28: mol_type = other DNA
agggaggacacaggtgcatttctggagg

SEQ ID NO: 47480 - DNA, 28 bp, synthetic construct
  source 1..28: mol_type = other DNA
gcaaacctcacaaagagtcaggccctgg

SEQ ID NO: 47481 - DNA, 28 bp, synthetic construct
  source 1..28: mol_type = other DNA
atcactgcaaacctcacaaagagtcagg

SEQ ID NO: 47482 - DNA, 28 bp, synthetic construct
  source 1..28: mol_type = other DNA
tgggggaagggaagagagaaaggaaggg

SEQ ID NO: 47483 - DNA, 28 bp, synthetic construct
  source 1..28: mol_type = other DNA
ctgggggaagggaagagagaaaggaagg

SEQ ID NO: 47484 - DNA, 28 bp, synthetic construct
  source 1..28: mol_type = other DNA
ggttctgggggaagggaagagagaaagg

SEQ ID NO: 47485 - DNA, 28 bp, synthetic construct
  source 1..28: mol_type = other DNA
ggggtactgtctggttctgggggaaggg

SEQ ID NO: 47486 - DNA, 28 bp, synthetic construct
  source 1..28: mol_type = other DNA
tggggtactgtctggttctgggggaagg

SEQ ID NO: 47487 - DNA, 28 bp, synthetic construct
  source 1..28: mol_type = other DNA
gttctggggtactgtctggttctggggg

SEQ ID NO: 47488 - DNA, 28 bp, synthetic construct
  source 1..28: mol_type = other DNA
agttctggggtactgtctggttctgggg

SEQ ID NO: 47489 - DNA, 28 bp, synthetic construct
  source 1..28: mol_type = other DNA
cagttctggggtactgtctggttctggg

SEQ ID NO: 47490 - DNA, 28 bp, synthetic construct
  source 1..28: mol_type = other DNA
gcagttctggggtactgtctggttctgg

SEQ ID NO: 47491 - DNA, 28 bp, synthetic construct
  source 1..28: mol_type = other DNA
gcggtggcagttctggggtactgtctgg

SEQ ID NO: 47492 - DNA, 28 bp, synthetic construct
  source 1..28: mol_type = other DNA
accccagaactgccaccgcctcctgtgg

SEQ ID NO: 47493 - DNA, 28 bp, synthetic construct
  source 1..28: mol_type = other DNA
accacaggaggcggtggcagttctgggg

SEQ ID NO: 47494 - DNA, 28 bp, synthetic construct
  source 1..28: mol_type = other DNA
gaccacaggaggcggtggcagttctggg

SEQ ID NO: 47495 - DNA, 28 bp, synthetic construct
  source 1..28: mol_type = other DNA
agaccacaggaggcggtggcagttctgg

SEQ ID NO: 47496 - DNA, 28 bp, synthetic construct
  source 1..28: mol_type = other DNA
agctctcagagaccacaggaggcggtgg

SEQ ID NO: 47497 - DNA, 28 bp, synthetic construct
  source 1..28: mol_type = other DNA
aacagctctcagagaccacaggaggcgg

SEQ ID NO: 47498 - DNA, 28 bp, synthetic construct
  source 1..28: mol_type = other DNA
agtaacagctctcagagaccacaggagg

SEQ ID NO: 47499 - DNA, 28 bp, synthetic construct
  source 1..28: mol_type = other DNA
gtcagtaacagctctcagagaccacagg

SEQ ID NO: 47500 - DNA, 28 bp, synthetic construct
  source 1..28: mol_type = other DNA
ctctgagagctgttactgacctatgcgg

SEQ ID NO: 47501 - DNA, 28 bp, synthetic construct
  source 1..28: mol_type = other DNA
tctgagagctgttactgacctatgcggg

SEQ ID NO: 47502 - DNA, 28 bp, synthetic construct
  source 1..28: mol_type = other DNA
agagctgttactgacctatgcgggctgg

SEQ ID NO: 47503 - DNA, 28 bp, synthetic construct
  source 1..28: mol_type = other DNA
gctgttactgacctatgcgggctggagg

SEQ ID NO: 47504 - DNA, 28 bp, synthetic construct
  source 1..28: mol_type = other DNA
ctgttactgacctatgcgggctggaggg

SEQ ID NO: 47505 - DNA, 28 bp, synthetic construct
  source 1..28: mol_type = other DNA
ctactctgatccctccagcccgcatagg

SEQ ID NO: 47506 - DNA, 28 bp, synthetic construct
  source 1..28: mol_type = other DNA
gggctggagggatcagagtagttgcagg

SEQ ID NO: 47507 - DNA, 28 bp, synthetic construct
  source 1..28: mol_type = other DNA
gagtagttgcaggcatgagatctcctgg

SEQ ID NO: 47508 - DNA, 28 bp, synthetic construct
  source 1..28: mol_type = other DNA
tagttgcaggcatgagatctcctggagg

SEQ ID NO: 47509 - DNA, 28 bp, synthetic construct
  source 1..28: mol_type = other DNA
tgcatcttcatctctgttttcctccagg

SEQ ID NO: 47510 - DNA, 28 bp, synthetic construct
  source 1..28: mol_type = other DNA
aacagtgctaagttattaacacacatgg

SEQ ID NO: 47511 - DNA, 28 bp, synthetic construct
  source 1..28: mol_type = other DNA
atctcagaagtgagtgggagcttggagg

SEQ ID NO: 47512 - DNA, 28 bp, synthetic construct
  source 1..28: mol_type = other DNA
agaatctcagaagtgagtgggagcttgg

SEQ ID NO: 47513 - DNA, 28 bp, synthetic construct
  source 1..28: mol_type = other DNA
aaatcaaagaatctcagaagtgagtggg

SEQ ID NO: 47514 - DNA, 28 bp, synthetic construct
  source 1..28: mol_type = other DNA
taaatcaaagaatctcagaagtgagtgg

SEQ ID NO: 47515 - DNA, 28 bp, synthetic construct
  source 1..28: mol_type = other DNA
tgcctgcctcggcctcccaaagttctgg

SEQ ID NO: 47516 - DNA, 28 bp, synthetic construct
  source 1..28: mol_type = other DNA
gcctgcctcggcctcccaaagttctggg

SEQ ID NO: 47517 - DNA, 28 bp, synthetic construct
  source 1..28: mol_type = other DNA
tcccagaactttgggaggccgaggcagg

SEQ ID NO: 47518 - DNA, 28 bp, synthetic construct
  source 1..28: mol_type = other DNA
gtaatcccagaactttgggaggccgagg

SEQ ID NO: 47519 - DNA, 28 bp, synthetic construct
  source 1..28: mol_type = other DNA
cggcctcccaaagttctgggattacagg

SEQ ID NO: 47520 - DNA, 28 bp, synthetic construct
  source 1..28: mol_type = other DNA
acgcctgtaatcccagaactttgggagg

SEQ ID NO: 47521 - DNA, 28 bp, synthetic construct
  source 1..28: mol_type = other DNA
ctcacgcctgtaatcccagaactttggg

SEQ ID NO: 47522 - DNA, 28 bp, synthetic construct
  source 1..28: mol_type = other DNA
gctcacgcctgtaatcccagaactttgg

SEQ ID NO: 47523 - DNA, 28 bp, synthetic construct
  source 1..28: mol_type = other DNA
aaatcaatgaaggagctgggcacagtgg

SEQ ID NO: 47524 - DNA, 28 bp, synthetic construct
  source 1..28: mol_type = other DNA
gagaaagaaaatcaatgaaggagctggg

SEQ ID NO: 47525 - DNA, 28 bp, synthetic construct
  source 1..28: mol_type = other DNA
ggagaaagaaaatcaatgaaggagctgg

SEQ ID NO: 47526 - DNA, 28 bp, synthetic construct
  source 1..28: mol_type = other DNA
gtgggaggagaaagaaaatcaatgaagg

SEQ ID NO: 47527 - DNA, 28 bp, synthetic construct
  source 1..28: mol_type = other DNA
tttctcctcccacctctgagttctctgg

SEQ ID NO: 47528 - DNA, 28 bp, synthetic construct
  source 1..28: mol_type = other DNA
caattccagagaactcagaggtgggagg

SEQ ID NO: 47529 - DNA, 28 bp, synthetic construct
  source 1..28: mol_type = other DNA
ggacaattccagagaactcagaggtggg

SEQ ID NO: 47530 - DNA, 28 bp, synthetic construct
  source 1..28: mol_type = other DNA
aggacaattccagagaactcagaggtgg

SEQ ID NO: 47531 - DNA, 28 bp, synthetic construct
  source 1..28: mol_type = other DNA
acctctgagttctctggaattgtcctgg

SEQ ID NO: 47532 - DNA, 28 bp, synthetic construct
  source 1..28: mol_type = other DNA
tccaggacaattccagagaactcagagg

SEQ ID NO: 47533 - DNA, 28 bp, synthetic construct
  source 1..28: mol_type = other DNA
tctctggaattgtcctggatttacctgg

SEQ ID NO: 47534 - DNA, 28 bp, synthetic construct
  source 1..28: mol_type = other DNA
gtcctggatttacctggtttcaccaagg

SEQ ID NO: 47535 - DNA, 28 bp, synthetic construct
  source 1..28: mol_type = other DNA
ggccttggtgaaaccaggtaaatccagg

SEQ ID NO: 47536 - DNA, 28 bp, synthetic construct
  source 1..28: mol_type = other DNA
tggtgtgggaggccttggtgaaaccagg

SEQ ID NO: 47537 - DNA, 28 bp, synthetic construct
  source 1..28: mol_type = other DNA
gatgagactctggtgtgggaggccttgg

SEQ ID NO: 47538 - DNA, 28 bp, synthetic construct
  source 1..28: mol_type = other DNA
aagaaagatgagactctggtgtgggagg

SEQ ID NO: 47539 - DNA, 28 bp, synthetic construct
  source 1..28: mol_type = other DNA
gacaagaaagatgagactctggtgtggg

SEQ ID NO: 47540 - DNA, 28 bp, synthetic construct
  source 1..28: mol_type = other DNA
agacaagaaagatgagactctggtgtgg

SEQ ID NO: 47541 - DNA, 28 bp, synthetic construct
  source 1..28: mol_type = other DNA
gtgaaagacaagaaagatgagactctgg

SEQ ID NO: 47542 - DNA, 28 bp, synthetic construct
  source 1..28: mol_type = other DNA
ttgcagcctgatccctgatcccaagtgg

SEQ ID NO: 47543 - DNA, 28 bp, synthetic construct
  source 1..28: mol_type = other DNA
cgttggccacttgggatcagggatcagg

SEQ ID NO: 47544 - DNA, 28 bp, synthetic construct
  source 1..28: mol_type = other DNA
gttctacgttggccacttgggatcaggg

SEQ ID NO: 47545 - DNA, 28 bp, synthetic construct
  source 1..28: mol_type = other DNA
agttctacgttggccacttgggatcagg

SEQ ID NO: 47546 - DNA, 28 bp, synthetic construct
  source 1..28: mol_type = other DNA
tctcggagttctacgttggccacttggg

SEQ ID NO: 47547 - DNA, 28 bp, synthetic construct
  source 1..28: mol_type = other DNA
ttctcggagttctacgttggccacttgg

SEQ ID NO: 47548 - DNA, 28 bp, synthetic construct
  source 1..28: mol_type = other DNA
gccaacgtagaactccgagaacagctgg

SEQ ID NO: 47549 - DNA, 28 bp, synthetic construct
  source 1..28: mol_type = other DNA
accagctgttctcggagttctacgttgg

SEQ ID NO: 47550 - DNA, 28 bp, synthetic construct
  source 1..28: mol_type = other DNA
actccgagaacagctggtcttctccagg

SEQ ID NO: 47551 - DNA, 28 bp, synthetic construct
  source 1..28: mol_type = other DNA
ctccgagaacagctggtcttctccaggg

SEQ ID NO: 47552 - DNA, 28 bp, synthetic construct
  source 1..28: mol_type = other DNA
agccctggagaagaccagctgttctcgg

SEQ ID NO: 47553 - DNA, 28 bp, synthetic construct
  source 1..28: mol_type = other DNA
aactggagctctgctatcgaagccctgg

SEQ ID NO: 47554 - DNA, 28 bp, synthetic construct
  source 1..28: mol_type = other DNA
gatagcagagctccagttcctgaagagg

SEQ ID NO: 47555 - DNA, 28 bp, synthetic construct
  source 1..28: mol_type = other DNA
ctcaactctttgcctcttcaggaactgg

SEQ ID NO: 47556 - DNA, 28 bp, synthetic construct
  source 1..28: mol_type = other DNA
tggcaactcaactctttgcctcttcagg

SEQ ID NO: 47557 - DNA, 28 bp, synthetic construct
  source 1..28: mol_type = other DNA
gagttgccaccctgttcatcttgcatgg

SEQ ID NO: 47558 - DNA, 28 bp, synthetic construct
  source 1..28: mol_type = other DNA
tgccaccctgttcatcttgcatggaagg

SEQ ID NO: 47559 - DNA, 28 bp, synthetic construct
  source 1..28: mol_type = other DNA
gaccttccatgcaagatgaacagggtgg

SEQ ID NO: 47560 - DNA, 28 bp, synthetic construct
  source 1..28: mol_type = other DNA
aaagaccttccatgcaagatgaacaggg

SEQ ID NO: 47561 - DNA, 28 bp, synthetic construct
  source 1..28: mol_type = other DNA
gaaagaccttccatgcaagatgaacagg

SEQ ID NO: 47562 - DNA, 28 bp, synthetic construct
  source 1..28: mol_type = other DNA
ggtctttccccacctgacaccttcttgg

SEQ ID NO: 47563 - DNA, 28 bp, synthetic construct
  source 1..28: mol_type = other DNA
agcagggccaagaaggtgtcaggtgggg

SEQ ID NO: 47564 - DNA, 28 bp, synthetic construct
  source 1..28: mol_type = other DNA
aagcagggccaagaaggtgtcaggtggg

SEQ ID NO: 47565 - DNA, 28 bp, synthetic construct
  source 1..28: mol_type = other DNA
caagcagggccaagaaggtgtcaggtgg

SEQ ID NO: 47566 - DNA, 28 bp, synthetic construct
  source 1..28: mol_type = other DNA
cacctgacaccttcttggccctgcttgg

SEQ ID NO: 47567 - DNA, 28 bp, synthetic construct
  source 1..28: mol_type = other DNA
agccaagcagggccaagaaggtgtcagg

SEQ ID NO: 47568 - DNA, 28 bp, synthetic construct
  source 1..28: mol_type = other DNA
cttatggagccaagcagggccaagaagg

SEQ ID NO: 47569 - DNA, 28 bp, synthetic construct
  source 1..28: mol_type = other DNA
cttcttggccctgcttggctccataagg

SEQ ID NO: 47570 - DNA, 28 bp, synthetic construct
  source 1..28: mol_type = other DNA
cagagtgtccttatggagccaagcaggg

SEQ ID NO: 47571 - DNA, 28 bp, synthetic construct
  source 1..28: mol_type = other DNA
tcagagtgtccttatggagccaagcagg

SEQ ID NO: 47572 - DNA, 28 bp, synthetic construct
  source 1..28: mol_type = other DNA
tacagggatcatcagagtgtccttatgg

SEQ ID NO: 47573 - DNA, 28 bp, synthetic construct
  source 1..28: mol_type = other DNA
aatcgaggttgaacagaaagtgagtggg

SEQ ID NO: 47574 - DNA, 28 bp, synthetic construct
  source 1..28: mol_type = other DNA
aaatcgaggttgaacagaaagtgagtgg

SEQ ID NO: 47575 - DNA, 28 bp, synthetic construct
  source 1..28: mol_type = other DNA
gctttctcagggacaggataaatcgagg

SEQ ID NO: 47576 - DNA, 28 bp, synthetic construct
  source 1..28: mol_type = other DNA
caggtctcagggctttctcagggacagg

SEQ ID NO: 47577 - DNA, 28 bp, synthetic construct
  source 1..28: mol_type = other DNA
tggggcaggtctcagggctttctcaggg

SEQ ID NO: 47578 - DNA, 28 bp, synthetic construct
  source 1..28: mol_type = other DNA
gtggggcaggtctcagggctttctcagg

SEQ ID NO: 47579 - DNA, 28 bp, synthetic construct
  source 1..28: mol_type = other DNA
gagaaagccctgagacctgccccacagg

SEQ ID NO: 47580 - DNA, 28 bp, synthetic construct
  source 1..28: mol_type = other DNA
atgaatgcctgtggggcaggtctcaggg

SEQ ID NO: 47581 - DNA, 28 bp, synthetic construct
  source 1..28: mol_type = other DNA
aatgaatgcctgtggggcaggtctcagg

SEQ ID NO: 47582 - DNA, 28 bp, synthetic construct
  source 1..28: mol_type = other DNA
acctgccccacaggcattcattcccagg

SEQ ID NO: 47583 - DNA, 28 bp, synthetic construct
  source 1..28: mol_type = other DNA
acctgggaatgaatgcctgtggggcagg

SEQ ID NO: 47584 - DNA, 28 bp, synthetic construct
  source 1..28: mol_type = other DNA
gccccacaggcattcattcccaggtagg

SEQ ID NO: 47585 - DNA, 28 bp, synthetic construct
  source 1..28: mol_type = other DNA
tcctacctgggaatgaatgcctgtgggg

SEQ ID NO: 47586 - DNA, 28 bp, synthetic construct
  source 1..28: mol_type = other DNA
gtcctacctgggaatgaatgcctgtggg

SEQ ID NO: 47587 - DNA, 28 bp, synthetic construct
  source 1..28: mol_type = other DNA
agtcctacctgggaatgaatgcctgtgg

SEQ ID NO: 47588 - DNA, 28 bp, synthetic construct
  source 1..28: mol_type = other DNA
ttcactgcgaacagaagtcctacctggg

SEQ ID NO: 47589 - DNA, 28 bp, synthetic construct
  source 1..28: mol_type = other DNA
cttcactgcgaacagaagtcctacctgg

SEQ ID NO: 47590 - DNA, 28 bp, synthetic construct
  source 1..28: mol_type = other DNA
ggtaggacttctgttcgcagtgaagagg

SEQ ID NO: 47591 - DNA, 28 bp, synthetic construct
  source 1..28: mol_type = other DNA
ctgttcgcagtgaagaggcagacactgg

SEQ ID NO: 47592 - DNA, 28 bp, synthetic construct
  source 1..28: mol_type = other DNA
tgttcgcagtgaagaggcagacactggg

SEQ ID NO: 47593 - DNA, 28 bp, synthetic construct
  source 1..28: mol_type = other DNA
gaggcagacactgggctgctcaccttgg

SEQ ID NO: 47594 - DNA, 28 bp, synthetic construct
  source 1..28: mol_type = other DNA
aggcagacactgggctgctcaccttggg

SEQ ID NO: 47595 - DNA, 28 bp, synthetic construct
  source 1..28: mol_type = other DNA
ggcagacactgggctgctcaccttgggg

SEQ ID NO: 47596 - DNA, 28 bp, synthetic construct
  source 1..28: mol_type = other DNA
tcagggatgctggaaatactccccaagg

SEQ ID NO: 47597 - DNA, 28 bp, synthetic construct
  source 1..28: mol_type = other DNA
gtgtctgggtctggttcagggatgctgg

SEQ ID NO: 47598 - DNA, 28 bp, synthetic construct
  source 1..28: mol_type = other DNA
ttacactgtgtctgggtctggttcaggg

SEQ ID NO: 47599 - DNA, 28 bp, synthetic construct
  source 1..28: mol_type = other DNA
gttacactgtgtctgggtctggttcagg

SEQ ID NO: 47600 - DNA, 28 bp, synthetic construct
  source 1..28: mol_type = other DNA
gctgtcgttacactgtgtctgggtctgg

SEQ ID NO: 47601 - DNA, 28 bp, synthetic construct
  source 1..28: mol_type = other DNA
tatgggctgtcgttacactgtgtctggg

SEQ ID NO: 47602 - DNA, 28 bp, synthetic construct
  source 1..28: mol_type = other DNA
atatgggctgtcgttacactgtgtctgg

SEQ ID NO: 47603 - DNA, 28 bp, synthetic construct
  source 1..28: mol_type = other DNA
cagtgtaacgacagcccatataaagtgg

SEQ ID NO: 47604 - DNA, 28 bp, synthetic construct
  source 1..28: mol_type = other DNA
agtgtaacgacagcccatataaagtggg

SEQ ID NO: 47605 - DNA, 28 bp, synthetic construct
  source 1..28: mol_type = other DNA
gtgtaacgacagcccatataaagtgggg

SEQ ID NO: 47606 - DNA, 28 bp, synthetic construct
  source 1..28: mol_type = other DNA
gacagcccatataaagtggggtcagcgg

SEQ ID NO: 47607 - DNA, 28 bp, synthetic construct
  source 1..28: mol_type = other DNA
acagcccatataaagtggggtcagcggg

SEQ ID NO: 47608 - DNA, 28 bp, synthetic construct
  source 1..28: mol_type = other DNA
cagcccatataaagtggggtcagcgggg

SEQ ID NO: 47609 - DNA, 28 bp, synthetic construct
  source 1..28: mol_type = other DNA
agcccatataaagtggggtcagcggggg

SEQ ID NO: 47610 - DNA, 28 bp, synthetic construct
  source 1..28: mol_type = other DNA
cacccccgctgaccccactttatatggg

SEQ ID NO: 47611 - DNA, 28 bp, synthetic construct
  source 1..28: mol_type = other DNA
ccatataaagtggggtcagcgggggtgg

SEQ ID NO: 47612 - DNA, 28 bp, synthetic construct
  source 1..28: mol_type = other DNA
aagtggggtcagcgggggtggcttgtgg

SEQ ID NO: 47613 - DNA, 28 bp, synthetic construct
  source 1..28: mol_type = other DNA
gggtggcttgtggattcgcacaaactgg

SEQ ID NO: 47614 - DNA, 28 bp, synthetic construct
  source 1..28: mol_type = other DNA
tggaatttcatttctagatcatctatgg

SEQ ID NO: 47615 - DNA, 28 bp, synthetic construct
  source 1..28: mol_type = other DNA
agatcatctatggcctacagaacatagg

SEQ ID NO: 47616 - DNA, 28 bp, synthetic construct
  source 1..28: mol_type = other DNA
gatcatctatggcctacagaacataggg

SEQ ID NO: 47617 - DNA, 28 bp, synthetic construct
  source 1..28: mol_type = other DNA
ttaatcattgttccctatgttctgtagg

SEQ ID NO: 47618 - DNA, 28 bp, synthetic construct
  source 1..28: mol_type = other DNA
tacagaacatagggaacaatgattaagg

SEQ ID NO: 47619 - DNA, 28 bp, synthetic construct
  source 1..28: mol_type = other DNA
acagaacatagggaacaatgattaaggg

SEQ ID NO: 47620 - DNA, 28 bp, synthetic construct
  source 1..28: mol_type = other DNA
gaacatagggaacaatgattaagggagg

SEQ ID NO: 47621 - DNA, 28 bp, synthetic construct
  source 1..28: mol_type = other DNA
atgattaagggaggcttctgccccgtgg

SEQ ID NO: 47622 - DNA, 28 bp, synthetic construct
  source 1..28: mol_type = other DNA
agggaggcttctgccccgtggaatgtgg

SEQ ID NO: 47623 - DNA, 28 bp, synthetic construct
  source 1..28: mol_type = other DNA
ctgccccgtggaatgtggtttgaatagg

SEQ ID NO: 47624 - DNA, 28 bp, synthetic construct
  source 1..28: mol_type = other DNA
tgccccgtggaatgtggtttgaataggg

SEQ ID NO: 47625 - DNA, 28 bp, synthetic construct
  source 1..28: mol_type = other DNA
gccccgtggaatgtggtttgaatagggg

SEQ ID NO: 47626 - DNA, 28 bp, synthetic construct
  source 1..28: mol_type = other DNA
ccccgtggaatgtggtttgaataggggg

SEQ ID NO: 47627 - DNA, 28 bp, synthetic construct
  source 1..28: mol_type = other DNA
cccgtggaatgtggtttgaatagggggg

SEQ ID NO: 47628 - DNA, 28 bp, synthetic construct
  source 1..28: mol_type = other DNA
tcccccctattcaaaccacattccacgg

SEQ ID NO: 47629 - DNA, 28 bp, synthetic construct
  source 1..28: mol_type = other DNA
tggaatgtggtttgaataggggggatgg

SEQ ID NO: 47630 - DNA, 28 bp, synthetic construct
  source 1..28: mol_type = other DNA
gggatggtgcatctgtgtgtttgtgtgg

SEQ ID NO: 47631 - DNA, 28 bp, synthetic construct
  source 1..28: mol_type = other DNA
catctgtgtgtttgtgtggacagagtgg

SEQ ID NO: 47632 - DNA, 28 bp, synthetic construct
  source 1..28: mol_type = other DNA
atctgtgtgtttgtgtggacagagtggg

SEQ ID NO: 47633 - DNA, 28 bp, synthetic construct
  source 1..28: mol_type = other DNA
tctgtgtgtttgtgtggacagagtgggg

SEQ ID NO: 47634 - DNA, 28 bp, synthetic construct
  source 1..28: mol_type = other DNA
ttctcctgtacaagaggcccatccttgg

SEQ ID NO: 47635 - DNA, 28 bp, synthetic construct
  source 1..28: mol_type = other DNA
gggaccaaggatgggcctcttgtacagg

SEQ ID NO: 47636 - DNA, 28 bp, synthetic construct
  source 1..28: mol_type = other DNA
agggtcttcaactgggaccaaggatggg

SEQ ID NO: 47637 - DNA, 28 bp, synthetic construct
  source 1..28: mol_type = other DNA
gagggtcttcaactgggaccaaggatgg

SEQ ID NO: 47638 - DNA, 28 bp, synthetic construct
  source 1..28: mol_type = other DNA
ccttggtcccagttgaagaccctctagg

SEQ ID NO: 47639 - DNA, 28 bp, synthetic construct
  source 1..28: mol_type = other DNA
cttggtcccagttgaagaccctctaggg

SEQ ID NO: 47640 - DNA, 28 bp, synthetic construct
  source 1..28: mol_type = other DNA
ttggtcccagttgaagaccctctagggg

SEQ ID NO: 47641 - DNA, 28 bp, synthetic construct
  source 1..28: mol_type = other DNA
tggtcccagttgaagaccctctaggggg

SEQ ID NO: 47642 - DNA, 28 bp, synthetic construct
  source 1..28: mol_type = other DNA
agagccccctagagggtcttcaactggg

SEQ ID NO: 47643 - DNA, 28 bp, synthetic construct
  source 1..28: mol_type = other DNA
gagagccccctagagggtcttcaactgg

SEQ ID NO: 47644 - DNA, 28 bp, synthetic construct
  source 1..28: mol_type = other DNA
gttgaagaccctctagggggctctctgg

SEQ ID NO: 47645 - DNA, 28 bp, synthetic construct
  source 1..28: mol_type = other DNA
aaatgcagccagagagccccctagaggg

SEQ ID NO: 47646 - DNA, 28 bp, synthetic construct
  source 1..28: mol_type = other DNA
aaaatgcagccagagagccccctagagg

SEQ ID NO: 47647 - DNA, 28 bp, synthetic construct
  source 1..28: mol_type = other DNA
ttttgtgtttaccgtcaacccaccgtgg

SEQ ID NO: 47648 - DNA, 28 bp, synthetic construct
  source 1..28: mol_type = other DNA
gaaaggctgggccacggtgggttgacgg

SEQ ID NO: 47649 - DNA, 28 bp, synthetic construct
  source 1..28: mol_type = other DNA
tcaacccaccgtggcccagcctttctgg

SEQ ID NO: 47650 - DNA, 28 bp, synthetic construct
  source 1..28: mol_type = other DNA
agagccagaaaggctgggccacggtggg

SEQ ID NO: 47651 - DNA, 28 bp, synthetic construct
  source 1..28: mol_type = other DNA
aagagccagaaaggctgggccacggtgg

SEQ ID NO: 47652 - DNA, 28 bp, synthetic construct
  source 1..28: mol_type = other DNA
actaagagccagaaaggctgggccacgg

SEQ ID NO: 47653 - DNA, 28 bp, synthetic construct
  source 1..28: mol_type = other DNA
ggtgacactaagagccagaaaggctggg

SEQ ID NO: 47654 - DNA, 28 bp, synthetic construct
  source 1..28: mol_type = other DNA
aggtgacactaagagccagaaaggctgg

SEQ ID NO: 47655 - DNA, 28 bp, synthetic construct
  source 1..28: mol_type = other DNA
cggaaggtgacactaagagccagaaagg

SEQ ID NO: 47656 - DNA, 28 bp, synthetic construct
  source 1..28: mol_type = other DNA
ctggctcttagtgtcaccttccgaatgg

SEQ ID NO: 47657 - DNA, 28 bp, synthetic construct
  source 1..28: mol_type = other DNA
tcaccttccgaatggagcagtcacttgg

SEQ ID NO: 47658 - DNA, 28 bp, synthetic construct
  source 1..28: mol_type = other DNA
caccttccgaatggagcagtcacttggg

SEQ ID NO: 47659 - DNA, 28 bp, synthetic construct
  source 1..28: mol_type = other DNA
atcccaagtgactgctccattcggaagg

SEQ ID NO: 47660 - DNA, 28 bp, synthetic construct
  source 1..28: mol_type = other DNA
ccgaatggagcagtcacttgggatcagg

SEQ ID NO: 47661 - DNA, 28 bp, synthetic construct
  source 1..28: mol_type = other DNA
ggagcagtcacttgggatcaggtagagg

SEQ ID NO: 47662 - DNA, 28 bp, synthetic construct
  source 1..28: mol_type = other DNA
gcagtcacttgggatcaggtagaggtgg

SEQ ID NO: 47663 - DNA, 28 bp, synthetic construct
  source 1..28: mol_type = other DNA
tcacttgggatcaggtagaggtggaagg

SEQ ID NO: 47664 - DNA, 28 bp, synthetic construct
  source 1..28: mol_type = other DNA
ggtagaggtggaaggtgacttcctcagg

SEQ ID NO: 47665 - DNA, 28 bp, synthetic construct
  source 1..28: mol_type = other DNA
gaggtggaaggtgacttcctcaggatgg

SEQ ID NO: 47666 - DNA, 28 bp, synthetic construct
  source 1..28: mol_type = other DNA
gaaggtgacttcctcaggatggacgcgg

SEQ ID NO: 47667 - DNA, 28 bp, synthetic construct
  source 1..28: mol_type = other DNA
ggtgacttcctcaggatggacgcggtgg

SEQ ID NO: 47668 - DNA, 28 bp, synthetic construct
  source 1..28: mol_type = other DNA
ttgctttaccaccgcgtccatcctgagg

SEQ ID NO: 47669 - DNA, 28 bp, synthetic construct
  source 1..28: mol_type = other DNA
acgcggtggtaaagcaacaccacagagg

SEQ ID NO: 47670 - DNA, 28 bp, synthetic construct
  source 1..28: mol_type = other DNA
tggtaaagcaacaccacagaggtgacgg

SEQ ID NO: 47671 - DNA, 28 bp, synthetic construct
  source 1..28: mol_type = other DNA
ggtaaagcaacaccacagaggtgacggg

SEQ ID NO: 47672 - DNA, 28 bp, synthetic construct
  source 1..28: mol_type = other DNA
ctgcgcttcattcccgtcacctctgtgg

SEQ ID NO: 47673 - DNA, 28 bp, synthetic construct
  source 1..28: mol_type = other DNA
cacagaggtgacgggaatgaagcgcagg

SEQ ID NO: 47674 - DNA, 28 bp, synthetic construct
  source 1..28: mol_type = other DNA
acagaggtgacgggaatgaagcgcaggg

SEQ ID NO: 47675 - DNA, 28 bp, synthetic construct
  source 1..28: mol_type = other DNA
gacgggaatgaagcgcagggcattatgg

SEQ ID NO: 47676 - DNA, 28 bp, synthetic construct
  source 1..28: mol_type = other DNA
gcgcagggcattatggatcattttcagg

SEQ ID NO: 47677 - DNA, 28 bp, synthetic construct
  source 1..28: mol_type = other DNA
cagggcattatggatcattttcaggagg

SEQ ID NO: 47678 - DNA, 28 bp, synthetic construct
  source 1..28: mol_type = other DNA
tggatcattttcaggaggactcccaagg

SEQ ID NO: 47679 - DNA, 28 bp, synthetic construct
  source 1..28: mol_type = other DNA
ggatcattttcaggaggactcccaaggg

SEQ ID NO: 47680 - DNA, 28 bp, synthetic construct
  source 1..28: mol_type = other DNA
gatcattttcaggaggactcccaagggg

SEQ ID NO: 47681 - DNA, 28 bp, synthetic construct
  source 1..28: mol_type = other DNA
atcattttcaggaggactcccaaggggg

SEQ ID NO: 47682 - DNA, 28 bp, synthetic construct
  source 1..28: mol_type = other DNA
aggaggactcccaagggggagaagctgg

SEQ ID NO: 47683 - DNA, 28 bp, synthetic construct
  source 1..28: mol_type = other DNA
ggaggactcccaagggggagaagctggg

SEQ ID NO: 47684 - DNA, 28 bp, synthetic construct
  source 1..28: mol_type = other DNA
gaggactcccaagggggagaagctgggg

SEQ ID NO: 47685 - DNA, 28 bp, synthetic construct
  source 1..28: mol_type = other DNA
tggaaaaccccagcttctcccccttggg

SEQ ID NO: 47686 - DNA, 28 bp, synthetic construct
  source 1..28: mol_type = other DNA
ctggaaaaccccagcttctcccccttgg

SEQ ID NO: 47687 - DNA, 28 bp, synthetic construct
  source 1..28: mol_type = other DNA
agggtggagctgcatcacatagttctgg

SEQ ID NO: 47688 - DNA, 28 bp, synthetic construct
  source 1..28: mol_type = other DNA
agaactatgtgatgcagctccaccctgg

SEQ ID NO: 47689 - DNA, 28 bp, synthetic construct
  source 1..28: mol_type = other DNA
ctatgtgatgcagctccaccctggctgg

SEQ ID NO: 47690 - DNA, 28 bp, synthetic construct
  source 1..28: mol_type = other DNA
cagctccaccctggctggcttctccagg

SEQ ID NO: 47691 - DNA, 28 bp, synthetic construct
  source 1..28: mol_type = other DNA
atgctcctggagaagccagccagggtgg

SEQ ID NO: 47692 - DNA, 28 bp, synthetic construct
  source 1..28: mol_type = other DNA
gggatgctcctggagaagccagccaggg

SEQ ID NO: 47693 - DNA, 28 bp, synthetic construct
  source 1..28: mol_type = other DNA
ggggatgctcctggagaagccagccagg

SEQ ID NO: 47694 - DNA, 28 bp, synthetic construct
  source 1..28: mol_type = other DNA
cactttaaagaggaggggatgctcctgg

SEQ ID NO: 47695 - DNA, 28 bp, synthetic construct
  source 1..28: mol_type = other DNA
caggagcatcccctcctctttaaagtgg

SEQ ID NO: 47696 - DNA, 28 bp, synthetic construct
  source 1..28: mol_type = other DNA
aggagcatcccctcctctttaaagtggg

SEQ ID NO: 47697 - DNA, 28 bp, synthetic construct
  source 1..28: mol_type = other DNA
cccctcctctttaaagtgggccatttgg

SEQ ID NO: 47698 - DNA, 28 bp, synthetic construct
  source 1..28: mol_type = other DNA
tccaaatggcccactttaaagaggaggg

SEQ ID NO: 47699 - DNA, 28 bp, synthetic construct
  source 1..28: mol_type = other DNA
ttccaaatggcccactttaaagaggagg

SEQ ID NO: 47700 - DNA, 28 bp, synthetic construct
  source 1..28: mol_type = other DNA
ctgttccaaatggcccactttaaagagg

SEQ ID NO: 47701 - DNA, 28 bp, synthetic construct
  source 1..28: mol_type = other DNA
ctctttaaagtgggccatttggaacagg

SEQ ID NO: 47702 - DNA, 28 bp, synthetic construct
  source 1..28: mol_type = other DNA
tctttaaagtgggccatttggaacaggg

SEQ ID NO: 47703 - DNA, 28 bp, synthetic construct
  source 1..28: mol_type = other DNA
catgtggacacatccctgttccaaatgg

SEQ ID NO: 47704 - DNA, 28 bp, synthetic construct
  source 1..28: mol_type = other DNA
catttggaacagggatgtgtccacatgg

SEQ ID NO: 47705 - DNA, 28 bp, synthetic construct
  source 1..28: mol_type = other DNA
gtccacatggccccctgtaaaagaatgg

SEQ ID NO: 47706 - DNA, 28 bp, synthetic construct
  source 1..28: mol_type = other DNA
atccattcttttacagggggccatgtgg

SEQ ID NO: 47707 - DNA, 28 bp, synthetic construct
  source 1..28: mol_type = other DNA
cctcttcaatccattcttttacaggggg

SEQ ID NO: 47708 - DNA, 28 bp, synthetic construct
  source 1..28: mol_type = other DNA
gcctcttcaatccattcttttacagggg

SEQ ID NO: 47709 - DNA, 28 bp, synthetic construct
  source 1..28: mol_type = other DNA
tgcctcttcaatccattcttttacaggg

SEQ ID NO: 47710 - DNA, 28 bp, synthetic construct
  source 1..28: mol_type = other DNA
gtgcctcttcaatccattcttttacagg

SEQ ID NO: 47711 - DNA, 28 bp, synthetic construct
  source 1..28: mol_type = other DNA
gtaaaagaatggattgaagaggcacagg

SEQ ID NO: 47712 - DNA, 28 bp, synthetic construct
  source 1..28: mol_type = other DNA
agacagagtttcgctcttgtcgcccagg

SEQ ID NO: 47713 - DNA, 28 bp, synthetic construct
  source 1..28: mol_type = other DNA
agagtttcgctcttgtcgcccaggctgg

SEQ ID NO: 47714 - DNA, 28 bp, synthetic construct
  source 1..28: mol_type = other DNA
tcttgtcgcccaggctggagtgcaatgg

SEQ ID NO: 47715 - DNA, 28 bp, synthetic construct
  source 1..28: mol_type = other DNA
agattgtaccattgcactccagcctggg

SEQ ID NO: 47716 - DNA, 28 bp, synthetic construct
  source 1..28: mol_type = other DNA
gagattgtaccattgcactccagcctgg

SEQ ID NO: 47717 - DNA, 28 bp, synthetic construct
  source 1..28: mol_type = other DNA
aggctggagtgcaatggtacaatctcgg

SEQ ID NO: 47718 - DNA, 28 bp, synthetic construct
  source 1..28: mol_type = other DNA
ccttagaggggccgagggggggttatgg

SEQ ID NO: 47719 - DNA, 28 bp, synthetic construct
  source 1..28: mol_type = other DNA
tggcttccttagaggggccgaggggggg

SEQ ID NO: 47720 - DNA, 28 bp, synthetic construct
  source 1..28: mol_type = other DNA
gtggcttccttagaggggccgagggggg

SEQ ID NO: 47721 - DNA, 28 bp, synthetic construct
  source 1..28: mol_type = other DNA
tgtggcttccttagaggggccgaggggg

SEQ ID NO: 47722 - DNA, 28 bp, synthetic construct
  source 1..28: mol_type = other DNA
ttgtggcttccttagaggggccgagggg

SEQ ID NO: 47723 - DNA, 28 bp, synthetic construct
  source 1..28: mol_type = other DNA
gttgtggcttccttagaggggccgaggg

SEQ ID NO: 47724 - DNA, 28 bp, synthetic construct
  source 1..28: mol_type = other DNA
tgttgtggcttccttagaggggccgagg

SEQ ID NO: 47725 - DNA, 28 bp, synthetic construct
  source 1..28: mol_type = other DNA
agagggtgttgtggcttccttagagggg

SEQ ID NO: 47726 - DNA, 28 bp, synthetic construct
  source 1..28: mol_type = other DNA
gagagggtgttgtggcttccttagaggg

SEQ ID NO: 47727 - DNA, 28 bp, synthetic construct
  source 1..28: mol_type = other DNA
ggagagggtgttgtggcttccttagagg

SEQ ID NO: 47728 - DNA, 28 bp, synthetic construct
  source 1..28: mol_type = other DNA
taaggaagccacaacaccctctcccagg

SEQ ID NO: 47729 - DNA, 28 bp, synthetic construct
  source 1..28: mol_type = other DNA
gataatctcctgggagagggtgttgtgg

SEQ ID NO: 47730 - DNA, 28 bp, synthetic construct
  source 1..28: mol_type = other DNA
tgtagaatgataatctcctgggagaggg

SEQ ID NO: 47731 - DNA, 28 bp, synthetic construct
  source 1..28: mol_type = other DNA
gtgtagaatgataatctcctgggagagg

SEQ ID NO: 47732 - DNA, 28 bp, synthetic construct
  source 1..28: mol_type = other DNA
agggagtgtagaatgataatctcctggg

SEQ ID NO: 47733 - DNA, 28 bp, synthetic construct
  source 1..28: mol_type = other DNA
aagggagtgtagaatgataatctcctgg

SEQ ID NO: 47734 - DNA, 28 bp, synthetic construct
  source 1..28: mol_type = other DNA
agattatcattctacactccctttcagg

SEQ ID NO: 47735 - DNA, 28 bp, synthetic construct
  source 1..28: mol_type = other DNA
ggtggtggtaattatgggcctgaaaggg

SEQ ID NO: 47736 - DNA, 28 bp, synthetic construct
  source 1..28: mol_type = other DNA
aggtggtggtaattatgggcctgaaagg

SEQ ID NO: 47737 - DNA, 28 bp, synthetic construct
  source 1..28: mol_type = other DNA
tagggaggaaggtggtggtaattatggg

SEQ ID NO: 47738 - DNA, 28 bp, synthetic construct
  source 1..28: mol_type = other DNA
atagggaggaaggtggtggtaattatgg

SEQ ID NO: 47739 - DNA, 28 bp, synthetic construct
  source 1..28: mol_type = other DNA
cagggaaggatagggaggaaggtggtgg

SEQ ID NO: 47740 - DNA, 28 bp, synthetic construct
  source 1..28: mol_type = other DNA
caacagggaaggatagggaggaaggtgg

SEQ ID NO: 47741 - DNA, 28 bp, synthetic construct
  source 1..28: mol_type = other DNA
aaacaacagggaaggatagggaggaagg

SEQ ID NO: 47742 - DNA, 28 bp, synthetic construct
  source 1..28: mol_type = other DNA
aggtaaacaacagggaaggatagggagg

SEQ ID NO: 47743 - DNA, 28 bp, synthetic construct
  source 1..28: mol_type = other DNA
ccaaggtaaacaacagggaaggataggg

SEQ ID NO: 47744 - DNA, 28 bp, synthetic construct
  source 1..28: mol_type = other DNA
tccaaggtaaacaacagggaaggatagg

SEQ ID NO: 47745 - DNA, 28 bp, synthetic construct
  source 1..28: mol_type = other DNA
ggctctccaaggtaaacaacagggaagg

SEQ ID NO: 47746 - DNA, 28 bp, synthetic construct
  source 1..28: mol_type = other DNA
ttgtggctctccaaggtaaacaacaggg

SEQ ID NO: 47747 - DNA, 28 bp, synthetic construct
  source 1..28: mol_type = other DNA
tttgtggctctccaaggtaaacaacagg

SEQ ID NO: 47748 - DNA, 28 bp, synthetic construct
  source 1..28: mol_type = other DNA
gtttaccttggagagccacaaagtgagg

SEQ ID NO: 47749 - DNA, 28 bp, synthetic construct
  source 1..28: mol_type = other DNA
tttaccttggagagccacaaagtgaggg

SEQ ID NO: 47750 - DNA, 28 bp, synthetic construct
  source 1..28: mol_type = other DNA
accttggagagccacaaagtgagggagg

SEQ ID NO: 47751 - DNA, 28 bp, synthetic construct
  source 1..28: mol_type = other DNA
acctccctcactttgtggctctccaagg

SEQ ID NO: 47752 - DNA, 28 bp, synthetic construct
  source 1..28: mol_type = other DNA
gaagctgtgcacctccctcactttgtgg

SEQ ID NO: 47753 - DNA, 28 bp, synthetic construct
  source 1..28: mol_type = other DNA
ggaggtgcacagcttccacagctccagg

SEQ ID NO: 47754 - DNA, 28 bp, synthetic construct
  source 1..28: mol_type = other DNA
gacatcaaggctgagcctggagctgtgg

SEQ ID NO: 47755 - DNA, 28 bp, synthetic construct
  source 1..28: mol_type = other DNA
ctctgctggacatcaaggctgagcctgg

SEQ ID NO: 47756 - DNA, 28 bp, synthetic construct
  source 1..28: mol_type = other DNA
caggctcagccttgatgtccagcagagg

SEQ ID NO: 47757 - DNA, 28 bp, synthetic construct
  source 1..28: mol_type = other DNA
gtggcagggcctctgctggacatcaagg

SEQ ID NO: 47758 - DNA, 28 bp, synthetic construct
  source 1..28: mol_type = other DNA
agctggatggtggcagggcctctgctgg

SEQ ID NO: 47759 - DNA, 28 bp, synthetic construct
  source 1..28: mol_type = other DNA
gccctgccaccatccagctgtgctgtgg

SEQ ID NO: 47760 - DNA, 28 bp, synthetic construct
  source 1..28: mol_type = other DNA
cccacagcacagctggatggtggcaggg

SEQ ID NO: 47761 - DNA, 28 bp, synthetic construct
  source 1..28: mol_type = other DNA
acccacagcacagctggatggtggcagg

SEQ ID NO: 47762 - DNA, 28 bp, synthetic construct
  source 1..28: mol_type = other DNA
atcaacccacagcacagctggatggtgg

SEQ ID NO: 47763 - DNA, 28 bp, synthetic construct
  source 1..28: mol_type = other DNA
gagatcaacccacagcacagctggatgg

SEQ ID NO: 47764 - DNA, 28 bp, synthetic construct
  source 1..28: mol_type = other DNA
gggtgagatcaacccacagcacagctgg

SEQ ID NO: 47765 - DNA, 28 bp, synthetic construct
  source 1..28: mol_type = other DNA
gctgtgctgtgggttgatctcacccagg

SEQ ID NO: 47766 - DNA, 28 bp, synthetic construct
  source 1..28: mol_type = other DNA
ctgtgggttgatctcacccaggaactgg

SEQ ID NO: 47767 - DNA, 28 bp, synthetic construct
  source 1..28: mol_type = other DNA
aattctgtgtgtgggaccagttcctggg

SEQ ID NO: 47768 - DNA, 28 bp, synthetic construct
  source 1..28: mol_type = other DNA
gaattctgtgtgtgggaccagttcctgg

SEQ ID NO: 47769 - DNA, 28 bp, synthetic construct
  source 1..28: mol_type = other DNA
tcccacacacagaattcaatctcaacgg

SEQ ID NO: 47770 - DNA, 28 bp, synthetic construct
  source 1..28: mol_type = other DNA
accgttgagattgaattctgtgtgtggg

SEQ ID NO: 47771 - DNA, 28 bp, synthetic construct
  source 1..28: mol_type = other DNA
gaccgttgagattgaattctgtgtgtgg

SEQ ID NO: 47772 - DNA, 28 bp, synthetic construct
  source 1..28: mol_type = other DNA
ggtctctgctttgtgatgagagaagcgg

SEQ ID NO: 47773 - DNA, 28 bp, synthetic construct
  source 1..28: mol_type = other DNA
ctcatcacaaagcagagacccgtgttgg

SEQ ID NO: 47774 - DNA, 28 bp, synthetic construct
  source 1..28: mol_type = other DNA
tcatcacaaagcagagacccgtgttggg

SEQ ID NO: 47775 - DNA, 28 bp, synthetic construct
  source 1..28: mol_type = other DNA
aaagcagagacccgtgttgggccagcgg

SEQ ID NO: 47776 - DNA, 28 bp, synthetic construct
  source 1..28: mol_type = other DNA
cagagacccgtgttgggccagcggtagg

SEQ ID NO: 47777 - DNA, 28 bp, synthetic construct
  source 1..28: mol_type = other DNA
ctggctcctaccgctggcccaacacggg

SEQ ID NO: 47778 - DNA, 28 bp, synthetic construct
  source 1..28: mol_type = other DNA
gctggctcctaccgctggcccaacacgg

SEQ ID NO: 47779 - DNA, 28 bp, synthetic construct
  source 1..28: mol_type = other DNA
tgggccagcggtaggagccagctacagg

SEQ ID NO: 47780 - DNA, 28 bp, synthetic construct
  source 1..28: mol_type = other DNA
gggccagcggtaggagccagctacaggg

SEQ ID NO: 47781 - DNA, 28 bp, synthetic construct
  source 1..28: mol_type = other DNA
cttccctgtagctggctcctaccgctgg

SEQ ID NO: 47782 - DNA, 28 bp, synthetic construct
  source 1..28: mol_type = other DNA
gagccagctacagggaagtgaactctgg

SEQ ID NO: 47783 - DNA, 28 bp, synthetic construct
  source 1..28: mol_type = other DNA
agccagctacagggaagtgaactctggg

SEQ ID NO: 47784 - DNA, 28 bp, synthetic construct
  source 1..28: mol_type = other DNA
ttcccagagttcacttccctgtagctgg

SEQ ID NO: 47785 - DNA, 28 bp, synthetic construct
  source 1..28: mol_type = other DNA
cagggaagtgaactctgggaagaagagg

SEQ ID NO: 47786 - DNA, 28 bp, synthetic construct
  source 1..28: mol_type = other DNA
agggaagtgaactctgggaagaagaggg

SEQ ID NO: 47787 - DNA, 28 bp, synthetic construct
  source 1..28: mol_type = other DNA
agtgaactctgggaagaagagggagagg

SEQ ID NO: 47788 - DNA, 28 bp, synthetic construct
  source 1..28: mol_type = other DNA
ctgcacgaactcactgagcacctgctgg

SEQ ID NO: 47789 - DNA, 28 bp, synthetic construct
  source 1..28: mol_type = other DNA
acctgctggatgccagaccccatgcagg

SEQ ID NO: 47790 - DNA, 28 bp, synthetic construct
  source 1..28: mol_type = other DNA
cctgctggatgccagaccccatgcaggg

SEQ ID NO: 47791 - DNA, 28 bp, synthetic construct
  source 1..28: mol_type = other DNA
ctgctggatgccagaccccatgcagggg

SEQ ID NO: 47792 - DNA, 28 bp, synthetic construct
  source 1..28: mol_type = other DNA
atgccagaccccatgcaggggcttgcgg

SEQ ID NO: 47793 - DNA, 28 bp, synthetic construct
  source 1..28: mol_type = other DNA
tatccgcaagcccctgcatggggtctgg

SEQ ID NO: 47794 - DNA, 28 bp, synthetic construct
  source 1..28: mol_type = other DNA
gaccccatgcaggggcttgcggatacgg

SEQ ID NO: 47795 - DNA, 28 bp, synthetic construct
  source 1..28: mol_type = other DNA
taccgtatccgcaagcccctgcatgggg

SEQ ID NO: 47796 - DNA, 28 bp, synthetic construct
  source 1..28: mol_type = other DNA
gtaccgtatccgcaagcccctgcatggg

SEQ ID NO: 47797 - DNA, 28 bp, synthetic construct
  source 1..28: mol_type = other DNA
tgtaccgtatccgcaagcccctgcatgg

SEQ ID NO: 47798 - DNA, 28 bp, synthetic construct
  source 1..28: mol_type = other DNA
gcaggggcttgcggatacggtacagtgg

SEQ ID NO: 47799 - DNA, 28 bp, synthetic construct
  source 1..28: mol_type = other DNA
gtacagtggcttcaagcccagacttcgg

SEQ ID NO: 47800 - DNA, 28 bp, synthetic construct
  source 1..28: mol_type = other DNA
aggggacccagtggtgagtgtgagttgg

SEQ ID NO: 47801 - DNA, 28 bp, synthetic construct
  source 1..28: mol_type = other DNA
ggggacccagtggtgagtgtgagttggg

SEQ ID NO: 47802 - DNA, 28 bp, synthetic construct
  source 1..28: mol_type = other DNA
gggacccagtggtgagtgtgagttgggg

SEQ ID NO: 47803 - DNA, 28 bp, synthetic construct
  source 1..28: mol_type = other DNA
ggacccagtggtgagtgtgagttggggg

SEQ ID NO: 47804 - DNA, 28 bp, synthetic construct
  source 1..28: mol_type = other DNA
ctacccccaactcacactcaccactggg

SEQ ID NO: 47805 - DNA, 28 bp, synthetic construct
  source 1..28: mol_type = other DNA
ccagtggtgagtgtgagttgggggtagg

SEQ ID NO: 47806 - DNA, 28 bp, synthetic construct
  source 1..28: mol_type = other DNA
cagtggtgagtgtgagttgggggtaggg

SEQ ID NO: 47807 - DNA, 28 bp, synthetic construct
  source 1..28: mol_type = other DNA
agtggtgagtgtgagttgggggtagggg

SEQ ID NO: 47808 - DNA, 28 bp, synthetic construct
  source 1..28: mol_type = other DNA
gtggtgagtgtgagttgggggtaggggg

SEQ ID NO: 47809 - DNA, 28 bp, synthetic construct
  source 1..28: mol_type = other DNA
gtgagtgtgagttgggggtagggggtgg

SEQ ID NO: 47810 - DNA, 28 bp, synthetic construct
  source 1..28: mol_type = other DNA
ggtagggggtggcgctgactgtctgtgg

SEQ ID NO: 47811 - DNA, 28 bp, synthetic construct
  source 1..28: mol_type = other DNA
gtagggggtggcgctgactgtctgtggg

SEQ ID NO: 47812 - DNA, 28 bp, synthetic construct
  source 1..28: mol_type = other DNA
tagggggtggcgctgactgtctgtgggg

SEQ ID NO: 47813 - DNA, 28 bp, synthetic construct
  source 1..28: mol_type = other DNA
tggcgctgactgtctgtggggacccagg

SEQ ID NO: 47814 - DNA, 28 bp, synthetic construct
  source 1..28: mol_type = other DNA
gctgactgtctgtggggacccaggatgg

SEQ ID NO: 47815 - DNA, 28 bp, synthetic construct
  source 1..28: mol_type = other DNA
ctgactgtctgtggggacccaggatggg

SEQ ID NO: 47816 - DNA, 28 bp, synthetic construct
  source 1..28: mol_type = other DNA
gtctgtggggacccaggatgggcagtgg

SEQ ID NO: 47817 - DNA, 28 bp, synthetic construct
  source 1..28: mol_type = other DNA
tctgtggggacccaggatgggcagtggg

SEQ ID NO: 47818 - DNA, 28 bp, synthetic construct
  source 1..28: mol_type = other DNA
ctgtggggacccaggatgggcagtgggg

SEQ ID NO: 47819 - DNA, 28 bp, synthetic construct
  source 1..28: mol_type = other DNA
gggacccaggatgggcagtggggtgcgg

SEQ ID NO: 47820 - DNA, 28 bp, synthetic construct
  source 1..28: mol_type = other DNA
ggacccaggatgggcagtggggtgcggg

SEQ ID NO: 47821 - DNA, 28 bp, synthetic construct
  source 1..28: mol_type = other DNA
cccaggatgggcagtggggtgcgggagg

SEQ ID NO: 47822 - DNA, 28 bp, synthetic construct
  source 1..28: mol_type = other DNA
gcctcccgcaccccactgcccatcctgg

SEQ ID NO: 47823 - DNA, 28 bp, synthetic construct
  source 1..28: mol_type = other DNA
ggcagtggggtgcgggaggccagcctgg

SEQ ID NO: 47824 - DNA, 28 bp, synthetic construct
  source 1..28: mol_type = other DNA
gcagtggggtgcgggaggccagcctggg

SEQ ID NO: 47825 - DNA, 28 bp, synthetic construct
  source 1..28: mol_type = other DNA
tgagggggctctgctggtcccaggctgg

SEQ ID NO: 47826 - DNA, 28 bp, synthetic construct
  source 1..28: mol_type = other DNA
tgagtgagggggctctgctggtcccagg

SEQ ID NO: 47827 - DNA, 28 bp, synthetic construct
  source 1..28: mol_type = other DNA
ggaccagcagagccccctcactcaccgg

SEQ ID NO: 47828 - DNA, 28 bp, synthetic construct
  source 1..28: mol_type = other DNA
gtaccggtgagtgagggggctctgctgg

SEQ ID NO: 47829 - DNA, 28 bp, synthetic construct
  source 1..28: mol_type = other DNA
aaagaacttgtaccggtgagtgaggggg

SEQ ID NO: 47830 - DNA, 28 bp, synthetic construct
  source 1..28: mol_type = other DNA
aaaagaacttgtaccggtgagtgagggg

SEQ ID NO: 47831 - DNA, 28 bp, synthetic construct
  source 1..28: mol_type = other DNA
gaaaagaacttgtaccggtgagtgaggg

SEQ ID NO: 47832 - DNA, 28 bp, synthetic construct
  source 1..28: mol_type = other DNA
agaaaagaacttgtaccggtgagtgagg

SEQ ID NO: 47833 - DNA, 28 bp, synthetic construct
  source 1..28: mol_type = other DNA
agttgacaaagaaaagaacttgtaccgg

SEQ ID NO: 47834 - DNA, 28 bp, synthetic construct
  source 1..28: mol_type = other DNA
ctttgtcaactacctcagtagccacagg

SEQ ID NO: 47835 - DNA, 28 bp, synthetic construct
  source 1..28: mol_type = other DNA
actacctcagtagccacaggccccgtgg

SEQ ID NO: 47836 - DNA, 28 bp, synthetic construct
  source 1..28: mol_type = other DNA
ctacctcagtagccacaggccccgtggg

SEQ ID NO: 47837 - DNA, 28 bp, synthetic construct
  source 1..28: mol_type = other DNA
tacctcagtagccacaggccccgtgggg

SEQ ID NO: 47838 - DNA, 28 bp, synthetic construct
  source 1..28: mol_type = other DNA
ggccccacggggcctgtggctactgagg

SEQ ID NO: 47839 - DNA, 28 bp, synthetic construct
  source 1..28: mol_type = other DNA
gacttctggggccccacggggcctgtgg

SEQ ID NO: 47840 - DNA, 28 bp, synthetic construct
  source 1..28: mol_type = other DNA
tgacgatgacttctggggccccacgggg

SEQ ID NO: 47841 - DNA, 28 bp, synthetic construct
  source 1..28: mol_type = other DNA
ctgacgatgacttctggggccccacggg

SEQ ID NO: 47842 - DNA, 28 bp, synthetic construct
  source 1..28: mol_type = other DNA
actgacgatgacttctggggccccacgg

SEQ ID NO: 47843 - DNA, 28 bp, synthetic construct
  source 1..28: mol_type = other DNA
ctttggggactgacgatgacttctgggg

SEQ ID NO: 47844 - DNA, 28 bp, synthetic construct
  source 1..28: mol_type = other DNA
cccagaagtcatcgtcagtccccaaagg

SEQ ID NO: 47845 - DNA, 28 bp, synthetic construct
  source 1..28: mol_type = other DNA
gcctttggggactgacgatgacttctgg

SEQ ID NO: 47846 - DNA, 28 bp, synthetic construct
  source 1..28: mol_type = other DNA
gtcagtccccaaaggcttcgtatgcagg

SEQ ID NO: 47847 - DNA, 28 bp, synthetic construct
  source 1..28: mol_type = other DNA
aggggacctgcatacgaagcctttgggg

SEQ ID NO: 47848 - DNA, 28 bp, synthetic construct
  source 1..28: mol_type = other DNA
aaggggacctgcatacgaagcctttggg

SEQ ID NO: 47849 - DNA, 28 bp, synthetic construct
  source 1..28: mol_type = other DNA
caaggggacctgcatacgaagcctttgg

SEQ ID NO: 47850 - DNA, 28 bp, synthetic construct
  source 1..28: mol_type = other DNA
ggcttcgtatgcaggtccccttgagagg

SEQ ID NO: 47851 - DNA, 28 bp, synthetic construct
  source 1..28: mol_type = other DNA
tcgtatgcaggtccccttgagaggcagg

SEQ ID NO: 47852 - DNA, 28 bp, synthetic construct
  source 1..28: mol_type = other DNA
gcaggtccccttgagaggcaggagaagg

SEQ ID NO: 47853 - DNA, 28 bp, synthetic construct
  source 1..28: mol_type = other DNA
tgcgtgccttctcctgcctctcaagggg

SEQ ID NO: 47854 - DNA, 28 bp, synthetic construct
  source 1..28: mol_type = other DNA
gtgcgtgccttctcctgcctctcaaggg

SEQ ID NO: 47855 - DNA, 28 bp, synthetic construct
  source 1..28: mol_type = other DNA
tgtgcgtgccttctcctgcctctcaagg

SEQ ID NO: 47856 - DNA, 28 bp, synthetic construct
  source 1..28: mol_type = other DNA
gagaaggcacgcacaagagttccaccgg

SEQ ID NO: 47857 - DNA, 28 bp, synthetic construct
  source 1..28: mol_type = other DNA
acaagagttccaccggtactacctctgg

SEQ ID NO: 47858 - DNA, 28 bp, synthetic construct
  source 1..28: mol_type = other DNA
caagagttccaccggtactacctctggg

SEQ ID NO: 47859 - DNA, 28 bp, synthetic construct
  source 1..28: mol_type = other DNA
aagagttccaccggtactacctctgggg

SEQ ID NO: 47860 - DNA, 28 bp, synthetic construct
  source 1..28: mol_type = other DNA
gaaagctccccagaggtagtaccggtgg

SEQ ID NO: 47861 - DNA, 28 bp, synthetic construct
  source 1..28: mol_type = other DNA
gaggaaagctccccagaggtagtaccgg

SEQ ID NO: 47862 - DNA, 28 bp, synthetic construct
  source 1..28: mol_type = other DNA
gctgtttcagaggaaagctccccagagg

SEQ ID NO: 47863 - DNA, 28 bp, synthetic construct
  source 1..28: mol_type = other DNA
tggggagctttcctctgaaacagcaagg

SEQ ID NO: 47864 - DNA, 28 bp, synthetic construct
  source 1..28: mol_type = other DNA
gctttcctctgaaacagcaaggcagcgg

SEQ ID NO: 47865 - DNA, 28 bp, synthetic construct
  source 1..28: mol_type = other DNA
gctgaccgctgccttgctgtttcagagg

SEQ ID NO: 47866 - DNA, 28 bp, synthetic construct
  source 1..28: mol_type = other DNA
gcggtcagctccagattctcccgcctgg

SEQ ID NO: 47867 - DNA, 28 bp, synthetic construct
  source 1..28: mol_type = other DNA
ctaggggaggccaggcgggagaatctgg

SEQ ID NO: 47868 - DNA, 28 bp, synthetic construct
  source 1..28: mol_type = other DNA
ccataggggctaggggaggccaggcggg

SEQ ID NO: 47869 - DNA, 28 bp, synthetic construct
  source 1..28: mol_type = other DNA
gccataggggctaggggaggccaggcgg

SEQ ID NO: 47870 - DNA, 28 bp, synthetic construct
  source 1..28: mol_type = other DNA
gcagccataggggctaggggaggccagg

SEQ ID NO: 47871 - DNA, 28 bp, synthetic construct
  source 1..28: mol_type = other DNA
acagtgcagccataggggctaggggagg

SEQ ID NO: 47872 - DNA, 28 bp, synthetic construct
  source 1..28: mol_type = other DNA
cttacagtgcagccataggggctagggg

SEQ ID NO: 47873 - DNA, 28 bp, synthetic construct
  source 1..28: mol_type = other DNA
ccctagcccctatggctgcactgtaagg

SEQ ID NO: 47874 - DNA, 28 bp, synthetic construct
  source 1..28: mol_type = other DNA
cccttacagtgcagccataggggctagg

SEQ ID NO: 47875 - DNA, 28 bp, synthetic construct
  source 1..28: mol_type = other DNA
ctagcccctatggctgcactgtaagggg

SEQ ID NO: 47876 - DNA, 28 bp, synthetic construct
  source 1..28: mol_type = other DNA
agggccccttacagtgcagccatagggg

SEQ ID NO: 47877 - DNA, 28 bp, synthetic construct
  source 1..28: mol_type = other DNA
aagggccccttacagtgcagccataggg

SEQ ID NO: 47878 - DNA, 28 bp, synthetic construct
  source 1..28: mol_type = other DNA
gaagggccccttacagtgcagccatagg

SEQ ID NO: 47879 - DNA, 28 bp, synthetic construct
  source 1..28: mol_type = other DNA
gctgcactgtaaggggcccttcccaagg

SEQ ID NO: 47880 - DNA, 28 bp, synthetic construct
  source 1..28: mol_type = other DNA
cactgtaaggggcccttcccaaggctgg

SEQ ID NO: 47881 - DNA, 28 bp, synthetic construct
  source 1..28: mol_type = other DNA
gggcccttcccaaggctggcctgcctgg

SEQ ID NO: 47882 - DNA, 28 bp, synthetic construct
  source 1..28: mol_type = other DNA
ggtccaggcaggccagccttgggaaggg

SEQ ID NO: 47883 - DNA, 28 bp, synthetic construct
  source 1..28: mol_type = other DNA
tggtccaggcaggccagccttgggaagg

SEQ ID NO: 47884 - DNA, 28 bp, synthetic construct
  source 1..28: mol_type = other DNA
tcccaaggctggcctgcctggaccatgg

SEQ ID NO: 47885 - DNA, 28 bp, synthetic construct
  source 1..28: mol_type = other DNA
gccatggtccaggcaggccagccttggg

SEQ ID NO: 47886 - DNA, 28 bp, synthetic construct
  source 1..28: mol_type = other DNA
tgccatggtccaggcaggccagccttgg

SEQ ID NO: 47887 - DNA, 28 bp, synthetic construct
  source 1..28: mol_type = other DNA
aaggctggcctgcctggaccatggcagg

SEQ ID NO: 47888 - DNA, 28 bp, synthetic construct
  source 1..28: mol_type = other DNA
aggctggcctgcctggaccatggcaggg

SEQ ID NO: 47889 - DNA, 28 bp, synthetic construct
  source 1..28: mol_type = other DNA
acacactccctgccatggtccaggcagg

SEQ ID NO: 47890 - DNA, 28 bp, synthetic construct
  source 1..28: mol_type = other DNA
gcagacacactccctgccatggtccagg

SEQ ID NO: 47891 - DNA, 28 bp, synthetic construct
  source 1..28: mol_type = other DNA
gggagatgggcggaggctgggctggagg

SEQ ID NO: 47892 - DNA, 28 bp, synthetic construct
  source 1..28: mol_type = other DNA
aaggggagatgggcggaggctgggctgg

SEQ ID NO: 47893 - DNA, 28 bp, synthetic construct
  source 1..28: mol_type = other DNA
ggggaaggggagatgggcggaggctggg

SEQ ID NO: 47894 - DNA, 28 bp, synthetic construct
  source 1..28: mol_type = other DNA
tggggaaggggagatgggcggaggctgg

SEQ ID NO: 47895 - DNA, 28 bp, synthetic construct
  source 1..28: mol_type = other DNA
ccagtggggaaggggagatgggcggagg

SEQ ID NO: 47896 - DNA, 28 bp, synthetic construct
  source 1..28: mol_type = other DNA
attccagtggggaaggggagatgggcgg

SEQ ID NO: 47897 - DNA, 28 bp, synthetic construct
  source 1..28: mol_type = other DNA
tctattccagtggggaaggggagatggg

SEQ ID NO: 47898 - DNA, 28 bp, synthetic construct
  source 1..28: mol_type = other DNA
ttctattccagtggggaaggggagatgg

SEQ ID NO: 47899 - DNA, 28 bp, synthetic construct
  source 1..28: mol_type = other DNA
tggcacttctattccagtggggaagggg

SEQ ID NO: 47900 - DNA, 28 bp, synthetic construct
  source 1..28: mol_type = other DNA
gtggcacttctattccagtggggaaggg

SEQ ID NO: 47901 - DNA, 28 bp, synthetic construct
  source 1..28: mol_type = other DNA
agtggcacttctattccagtggggaagg

SEQ ID NO: 47902 - DNA, 28 bp, synthetic construct
  source 1..28: mol_type = other DNA
ggagagtggcacttctattccagtgggg

SEQ ID NO: 47903 - DNA, 28 bp, synthetic construct
  source 1..28: mol_type = other DNA
gggagagtggcacttctattccagtggg

SEQ ID NO: 47904 - DNA, 28 bp, synthetic construct
  source 1..28: mol_type = other DNA
ggggagagtggcacttctattccagtgg

SEQ ID NO: 47905 - DNA, 28 bp, synthetic construct
  source 1..28: mol_type = other DNA
aagtgccactctccccagcatgcccagg

SEQ ID NO: 47906 - DNA, 28 bp, synthetic construct
  source 1..28: mol_type = other DNA
tgccactctccccagcatgcccaggtgg

SEQ ID NO: 47907 - DNA, 28 bp, synthetic construct
  source 1..28: mol_type = other DNA
gccactctccccagcatgcccaggtggg

SEQ ID NO: 47908 - DNA, 28 bp, synthetic construct
  source 1..28: mol_type = other DNA
gcccacctgggcatgctggggagagtgg

SEQ ID NO: 47909 - DNA, 28 bp, synthetic construct
  source 1..28: mol_type = other DNA
ctctccccagcatgcccaggtgggcagg

SEQ ID NO: 47910 - DNA, 28 bp, synthetic construct
  source 1..28: mol_type = other DNA
tcaacctgcccacctgggcatgctgggg

SEQ ID NO: 47911 - DNA, 28 bp, synthetic construct
  source 1..28: mol_type = other DNA
ctcaacctgcccacctgggcatgctggg

SEQ ID NO: 47912 - DNA, 28 bp, synthetic construct
  source 1..28: mol_type = other DNA
tctcaacctgcccacctgggcatgctgg

SEQ ID NO: 47913 - DNA, 28 bp, synthetic construct
  source 1..28: mol_type = other DNA
atgttctctctcaacctgcccacctggg

SEQ ID NO: 47914 - DNA, 28 bp, synthetic construct
  source 1..28: mol_type = other DNA
catgttctctctcaacctgcccacctgg

SEQ ID NO: 47915 - DNA, 28 bp, synthetic construct
  source 1..28: mol_type = other DNA
caggtgggcaggttgagagagaacatgg

SEQ ID NO: 47916 - DNA, 28 bp, synthetic construct
  source 1..28: mol_type = other DNA
gagagaacatggttcaaaagatgaaagg

SEQ ID NO: 47917 - DNA, 28 bp, synthetic construct
  source 1..28: mol_type = other DNA
agagaacatggttcaaaagatgaaaggg

SEQ ID NO: 47918 - DNA, 28 bp, synthetic construct
  source 1..28: mol_type = other DNA
gagaacatggttcaaaagatgaaagggg

SEQ ID NO: 47919 - DNA, 28 bp, synthetic construct
  source 1..28: mol_type = other DNA
catggttcaaaagatgaaaggggccagg

SEQ ID NO: 47920 - DNA, 28 bp, synthetic construct
  source 1..28: mol_type = other DNA
aaaagatgaaaggggccaggcaccgtgg

SEQ ID NO: 47921 - DNA, 28 bp, synthetic construct
  source 1..28: mol_type = other DNA
gattgcaggcaagagccacggtgcctgg

SEQ ID NO: 47922 - DNA, 28 bp, synthetic construct
  source 1..28: mol_type = other DNA
ttgctgagattgcaggcaagagccacgg

SEQ ID NO: 47923 - DNA, 28 bp, synthetic construct
  source 1..28: mol_type = other DNA
ggctcttgcctgcaatctcagcaattgg

SEQ ID NO: 47924 - DNA, 28 bp, synthetic construct
  source 1..28: mol_type = other DNA
gctcttgcctgcaatctcagcaattggg

SEQ ID NO: 47925 - DNA, 28 bp, synthetic construct
  source 1..28: mol_type = other DNA
agatcttcccaattgctgagattgcagg

SEQ ID NO: 47926 - DNA, 28 bp, synthetic construct
  source 1..28: mol_type = other DNA
aattgggaagatcttgctcacgtccagg

SEQ ID NO: 47927 - DNA, 28 bp, synthetic construct
  source 1..28: mol_type = other DNA
gttgctcaggctaatctcaaactcctgg

SEQ ID NO: 47928 - DNA, 28 bp, synthetic construct
  source 1..28: mol_type = other DNA
gagtttgagattagcctgagcaacatgg

SEQ ID NO: 47929 - DNA, 28 bp, synthetic construct
  source 1..28: mol_type = other DNA
agtttgagattagcctgagcaacatggg

SEQ ID NO: 47930 - DNA, 28 bp, synthetic construct
  source 1..28: mol_type = other DNA
gagagggcggcttcccatgttgctcagg

SEQ ID NO: 47931 - DNA, 28 bp, synthetic construct
  source 1..28: mol_type = other DNA
atttttcttttttctgtagagagggcgg

SEQ ID NO: 47932 - DNA, 28 bp, synthetic construct
  source 1..28: mol_type = other DNA
gatatttttcttttttctgtagagaggg

SEQ ID NO: 47933 - DNA, 28 bp, synthetic construct
  source 1..28: mol_type = other DNA
tgatatttttcttttttctgtagagagg

SEQ ID NO: 47934 - DNA, 28 bp, synthetic construct
  source 1..28: mol_type = other DNA
tacagaaaaaagaaaaatatcagccagg

SEQ ID NO: 47935 - DNA, 28 bp, synthetic construct
  source 1..28: mol_type = other DNA
aaaaaagaaaaatatcagccaggcatgg

SEQ ID NO: 47936 - DNA, 28 bp, synthetic construct
  source 1..28: mol_type = other DNA
aaagaaaaatatcagccaggcatggtgg

SEQ ID NO: 47937 - DNA, 28 bp, synthetic construct
  source 1..28: mol_type = other DNA
gactgcagatgctcaccaccatgcctgg

SEQ ID NO: 47938 - DNA, 28 bp, synthetic construct
  source 1..28: mol_type = other DNA
agcatctgcagtcccagttctactcagg

SEQ ID NO: 47939 - DNA, 28 bp, synthetic construct
  source 1..28: mol_type = other DNA
atctgcagtcccagttctactcaggagg

SEQ ID NO: 47940 - DNA, 28 bp, synthetic construct
  source 1..28: mol_type = other DNA
tgcagtcccagttctactcaggaggcgg

SEQ ID NO: 47941 - DNA, 28 bp, synthetic construct
  source 1..28: mol_type = other DNA
agtcccagttctactcaggaggcggagg

SEQ ID NO: 47942 - DNA, 28 bp, synthetic construct
  source 1..28: mol_type = other DNA
ccacctccgcctcctgagtagaactggg

SEQ ID NO: 47943 - DNA, 28 bp, synthetic construct
  source 1..28: mol_type = other DNA
cccacctccgcctcctgagtagaactgg

SEQ ID NO: 47944 - DNA, 28 bp, synthetic construct
  source 1..28: mol_type = other DNA
gttctactcaggaggcggaggtgggagg

SEQ ID NO: 47945 - DNA, 28 bp, synthetic construct
  source 1..28: mol_type = other DNA
ggtgggaggattgtttgagctcagaagg

SEQ ID NO: 47946 - DNA, 28 bp, synthetic construct
  source 1..28: mol_type = other DNA
aggattgtttgagctcagaaggtttagg

SEQ ID NO: 47947 - DNA, 28 bp, synthetic construct
  source 1..28: mol_type = other DNA
gacggggcaggtttcctacccaagaggg

SEQ ID NO: 47948 - DNA, 28 bp, synthetic construct
  source 1..28: mol_type = other DNA
ggacggggcaggtttcctacccaagagg

SEQ ID NO: 47949 - DNA, 28 bp, synthetic construct
  source 1..28: mol_type = other DNA
taggaaacctgccccgtcccacatcagg

SEQ ID NO: 47950 - DNA, 28 bp, synthetic construct
  source 1..28: mol_type = other DNA
aggaaacctgccccgtcccacatcaggg

SEQ ID NO: 47951 - DNA, 28 bp, synthetic construct
  source 1..28: mol_type = other DNA
ggaaacctgccccgtcccacatcagggg

SEQ ID NO: 47952 - DNA, 28 bp, synthetic construct
  source 1..28: mol_type = other DNA
ctctgcccctgatgtgggacggggcagg

SEQ ID NO: 47953 - DNA, 28 bp, synthetic construct
  source 1..28: mol_type = other DNA
ctgccccgtcccacatcaggggcagagg

SEQ ID NO: 47954 - DNA, 28 bp, synthetic construct
  source 1..28: mol_type = other DNA
tgccccgtcccacatcaggggcagaggg

SEQ ID NO: 47955 - DNA, 28 bp, synthetic construct
  source 1..28: mol_type = other DNA
atccctctgcccctgatgtgggacgggg

SEQ ID NO: 47956 - DNA, 28 bp, synthetic construct
  source 1..28: mol_type = other DNA
catccctctgcccctgatgtgggacggg

SEQ ID NO: 47957 - DNA, 28 bp, synthetic construct
  source 1..28: mol_type = other DNA
ccatccctctgcccctgatgtgggacgg

SEQ ID NO: 47958 - DNA, 28 bp, synthetic construct
  source 1..28: mol_type = other DNA
tcccacatcaggggcagagggatggagg

SEQ ID NO: 47959 - DNA, 28 bp, synthetic construct
  source 1..28: mol_type = other DNA
ccctccatccctctgcccctgatgtggg

SEQ ID NO: 47960 - DNA, 28 bp, synthetic construct
  source 1..28: mol_type = other DNA
tccctccatccctctgcccctgatgtgg

SEQ ID NO: 47961 - DNA, 28 bp, synthetic construct
  source 1..28: mol_type = other DNA
ggggttgggggaggtcagctgtgggagg

SEQ ID NO: 47962 - DNA, 28 bp, synthetic construct
  source 1..28: mol_type = other DNA
acaggggttgggggaggtcagctgtggg

SEQ ID NO: 47963 - DNA, 28 bp, synthetic construct
  source 1..28: mol_type = other DNA
gacaggggttgggggaggtcagctgtgg

SEQ ID NO: 47964 - DNA, 28 bp, synthetic construct
  source 1..28: mol_type = other DNA
ggagcatcgtgacaggggttgggggagg

SEQ ID NO: 47965 - DNA, 28 bp, synthetic construct
  source 1..28: mol_type = other DNA
ctgggagcatcgtgacaggggttggggg

SEQ ID NO: 47966 - DNA, 28 bp, synthetic construct
  source 1..28: mol_type = other DNA
gctgggagcatcgtgacaggggttgggg

SEQ ID NO: 47967 - DNA, 28 bp, synthetic construct
  source 1..28: mol_type = other DNA
ggctgggagcatcgtgacaggggttggg

SEQ ID NO: 47968 - DNA, 28 bp, synthetic construct
  source 1..28: mol_type = other DNA
aggctgggagcatcgtgacaggggttgg

SEQ ID NO: 47969 - DNA, 28 bp, synthetic construct
  source 1..28: mol_type = other DNA
ggcaaggctgggagcatcgtgacagggg

SEQ ID NO: 47970 - DNA, 28 bp, synthetic construct
  source 1..28: mol_type = other DNA
gggcaaggctgggagcatcgtgacaggg

SEQ ID NO: 47971 - DNA, 28 bp, synthetic construct
  source 1..28: mol_type = other DNA
ggggcaaggctgggagcatcgtgacagg

SEQ ID NO: 47972 - DNA, 28 bp, synthetic construct
  source 1..28: mol_type = other DNA
tcaggtagtttgaaggggcaaggctggg

SEQ ID NO: 47973 - DNA, 28 bp, synthetic construct
  source 1..28: mol_type = other DNA
atcaggtagtttgaaggggcaaggctgg

SEQ ID NO: 47974 - DNA, 28 bp, synthetic construct
  source 1..28: mol_type = other DNA
tcggatcaggtagtttgaaggggcaagg

SEQ ID NO: 47975 - DNA, 28 bp, synthetic construct
  source 1..28: mol_type = other DNA
gagactcggatcaggtagtttgaagggg

SEQ ID NO: 47976 - DNA, 28 bp, synthetic construct
  source 1..28: mol_type = other DNA
agagactcggatcaggtagtttgaaggg

SEQ ID NO: 47977 - DNA, 28 bp, synthetic construct
  source 1..28: mol_type = other DNA
cagagactcggatcaggtagtttgaagg

SEQ ID NO: 47978 - DNA, 28 bp, synthetic construct
  source 1..28: mol_type = other DNA
cactcaagcggcagagactcggatcagg

SEQ ID NO: 47979 - DNA, 28 bp, synthetic construct
  source 1..28: mol_type = other DNA
gatccgagtctctgccgcttgagtgagg

SEQ ID NO: 47980 - DNA, 28 bp, synthetic construct
  source 1..28: mol_type = other DNA
catcctcactcaagcggcagagactcgg

SEQ ID NO: 47981 - DNA, 28 bp, synthetic construct
  source 1..28: mol_type = other DNA
gagtaatagcacatcctcactcaagcgg

SEQ ID NO: 47982 - DNA, 28 bp, synthetic construct
  source 1..28: mol_type = other DNA
gctattactcatctctcccgtatccagg

SEQ ID NO: 47983 - DNA, 28 bp, synthetic construct
  source 1..28: mol_type = other DNA
tctctcccgtatccaggccctcagtagg

SEQ ID NO: 47984 - DNA, 28 bp, synthetic construct
  source 1..28: mol_type = other DNA
ctctcccgtatccaggccctcagtaggg

SEQ ID NO: 47985 - DNA, 28 bp, synthetic construct
  source 1..28: mol_type = other DNA
tctcccgtatccaggccctcagtagggg

SEQ ID NO: 47986 - DNA, 28 bp, synthetic construct
  source 1..28: mol_type = other DNA
tgacccctactgagggcctggatacggg

SEQ ID NO: 47987 - DNA, 28 bp, synthetic construct
  source 1..28: mol_type = other DNA
atgacccctactgagggcctggatacgg

SEQ ID NO: 47988 - DNA, 28 bp, synthetic construct
  source 1..28: mol_type = other DNA
agtgtgatgacccctactgagggcctgg

SEQ ID NO: 47989 - DNA, 28 bp, synthetic construct
  source 1..28: mol_type = other DNA
ggccctcagtaggggtcatcacacttgg

SEQ ID NO: 47990 - DNA, 28 bp, synthetic construct
  source 1..28: mol_type = other DNA
aaccaagtgtgatgacccctactgaggg

SEQ ID NO: 47991 - DNA, 28 bp, synthetic construct
  source 1..28: mol_type = other DNA
aaaccaagtgtgatgacccctactgagg

SEQ ID NO: 47992 - DNA, 28 bp, synthetic construct
  source 1..28: mol_type = other DNA
gtaggggtcatcacacttggtttcctgg

SEQ ID NO: 47993 - DNA, 28 bp, synthetic construct
  source 1..28: mol_type = other DNA
aggcagaatgaacaattctttgtccagg

SEQ ID NO: 47994 - DNA, 28 bp, synthetic construct
  source 1..28: mol_type = other DNA
gaattgttcattctgcctaagatcttgg

SEQ ID NO: 47995 - DNA, 28 bp, synthetic construct
  source 1..28: mol_type = other DNA
ttgttcattctgcctaagatcttggagg

SEQ ID NO: 47996 - DNA, 28 bp, synthetic construct
  source 1..28: mol_type = other DNA
tctgcctaagatcttggaggaagcgagg

SEQ ID NO: 47997 - DNA, 28 bp, synthetic construct
  source 1..28: mol_type = other DNA
ctgcctaagatcttggaggaagcgaggg

SEQ ID NO: 47998 - DNA, 28 bp, synthetic construct
  source 1..28: mol_type = other DNA
cagccctcgcttcctccaagatcttagg

SEQ ID NO: 47999 - DNA, 28 bp, synthetic construct
  source 1..28: mol_type = other DNA
ttgaatttttagtgggaatgtcatgtgg

SEQ ID NO: 48000 - DNA, 28 bp, synthetic construct
  source 1..28: mol_type = other DNA
tcccactaaaaattcaactcctcctcgg

SEQ ID NO: 48001 - DNA, 28 bp, synthetic construct
  source 1..28: mol_type = other DNA
cccgaggaggagttgaatttttagtggg

SEQ ID NO: 48002 - DNA, 28 bp, synthetic construct
  source 1..28: mol_type = other DNA
acccgaggaggagttgaatttttagtgg

SEQ ID NO: 48003 - DNA, 28 bp, synthetic construct
  source 1..28: mol_type = other DNA
ctaaaaattcaactcctcctcgggtcgg

SEQ ID NO: 48004 - DNA, 28 bp, synthetic construct
  source 1..28: mol_type = other DNA
taaaaattcaactcctcctcgggtcggg

SEQ ID NO: 48005 - DNA, 28 bp, synthetic construct
  source 1..28: mol_type = other DNA
caactcctcctcgggtcgggtgcagtgg

SEQ ID NO: 48006 - DNA, 28 bp, synthetic construct
  source 1..28: mol_type = other DNA
atgagccactgcacccgacccgaggagg

SEQ ID NO: 48007 - DNA, 28 bp, synthetic construct
  source 1..28: mol_type = other DNA
gacatgagccactgcacccgacccgagg

SEQ ID NO: 48008 - DNA, 28 bp, synthetic construct
  source 1..28: mol_type = other DNA
ctgctgtggtgtctgggtttctccctgg

SEQ ID NO: 48009 - DNA, 28 bp, synthetic construct
  source 1..28: mol_type = other DNA
atggggtgagagacaaacacagccaggg

SEQ ID NO: 48010 - DNA, 28 bp, synthetic construct
  source 1..28: mol_type = other DNA
catggggtgagagacaaacacagccagg

SEQ ID NO: 48011 - DNA, 28 bp, synthetic construct
  source 1..28: mol_type = other DNA
ctggctgtgtttgtctctcaccccatgg

SEQ ID NO: 48012 - DNA, 28 bp, synthetic construct
  source 1..28: mol_type = other DNA
agcaggagacagggaaagagccatgggg

SEQ ID NO: 48013 - DNA, 28 bp, synthetic construct
  source 1..28: mol_type = other DNA
gagcaggagacagggaaagagccatggg

SEQ ID NO: 48014 - DNA, 28 bp, synthetic construct
  source 1..28: mol_type = other DNA
tgagcaggagacagggaaagagccatgg

SEQ ID NO: 48015 - DNA, 28 bp, synthetic construct
  source 1..28: mol_type = other DNA
tctttccctgtctcctgctcagccctgg

SEQ ID NO: 48016 - DNA, 28 bp, synthetic construct
  source 1..28: mol_type = other DNA
ctttccctgtctcctgctcagccctggg

SEQ ID NO: 48017 - DNA, 28 bp, synthetic construct
  source 1..28: mol_type = other DNA
caggcccagggctgagcaggagacaggg

SEQ ID NO: 48018 - DNA, 28 bp, synthetic construct
  source 1..28: mol_type = other DNA
ccaggcccagggctgagcaggagacagg

SEQ ID NO: 48019 - DNA, 28 bp, synthetic construct
  source 1..28: mol_type = other DNA
ctgtctcctgctcagccctgggcctggg

SEQ ID NO: 48020 - DNA, 28 bp, synthetic construct
  source 1..28: mol_type = other DNA
ggctgacccaggcccagggctgagcagg

SEQ ID NO: 48021 - DNA, 28 bp, synthetic construct
  source 1..28: mol_type = other DNA
tcagccctgggcctgggtcagccagagg

SEQ ID NO: 48022 - DNA, 28 bp, synthetic construct
  source 1..28: mol_type = other DNA
cagccctgggcctgggtcagccagaggg

SEQ ID NO: 48023 - DNA, 28 bp, synthetic construct
  source 1..28: mol_type = other DNA
actccctctggctgacccaggcccaggg

SEQ ID NO: 48024 - DNA, 28 bp, synthetic construct
  source 1..28: mol_type = other DNA
aactccctctggctgacccaggcccagg

SEQ ID NO: 48025 - DNA, 28 bp, synthetic construct
  source 1..28: mol_type = other DNA
ggcctgggtcagccagagggagttctgg

SEQ ID NO: 48026 - DNA, 28 bp, synthetic construct
  source 1..28: mol_type = other DNA
gcctgggtcagccagagggagttctggg

SEQ ID NO: 48027 - DNA, 28 bp, synthetic construct
  source 1..28: mol_type = other DNA
acccagaactccctctggctgacccagg

SEQ ID NO: 48028 - DNA, 28 bp, synthetic construct
  source 1..28: mol_type = other DNA
gtaaggggggacccagaactccctctgg

SEQ ID NO: 48029 - DNA, 28 bp, synthetic construct
  source 1..28: mol_type = other DNA
gctcatcttcagcagacggtaagggggg

SEQ ID NO: 48030 - DNA, 28 bp, synthetic construct
  source 1..28: mol_type = other DNA
tgctcatcttcagcagacggtaaggggg

SEQ ID NO: 48031 - DNA, 28 bp, synthetic construct
  source 1..28: mol_type = other DNA
ctgctcatcttcagcagacggtaagggg

SEQ ID NO: 48032 - DNA, 28 bp, synthetic construct
  source 1..28: mol_type = other DNA
gctgctcatcttcagcagacggtaaggg

SEQ ID NO: 48033 - DNA, 28 bp, synthetic construct
  source 1..28: mol_type = other DNA
agctgctcatcttcagcagacggtaagg

SEQ ID NO: 48034 - DNA, 28 bp, synthetic construct
  source 1..28: mol_type = other DNA
accgtctgctgaagatgagcagctgagg

SEQ ID NO: 48035 - DNA, 28 bp, synthetic construct
  source 1..28: mol_type = other DNA
acctcagctgctcatcttcagcagacgg

SEQ ID NO: 48036 - DNA, 28 bp, synthetic construct
  source 1..28: mol_type = other DNA
gagcagctgaggtttctcctgctccagg

SEQ ID NO: 48037 - DNA, 28 bp, synthetic construct
  source 1..28: mol_type = other DNA
agcagctgaggtttctcctgctccaggg

SEQ ID NO: 48038 - DNA, 28 bp, synthetic construct
  source 1..28: mol_type = other DNA
aggcaggaactgagggccctggagcagg

SEQ ID NO: 48039 - DNA, 28 bp, synthetic construct
  source 1..28: mol_type = other DNA
gagatgaggcaggaactgagggccctgg

SEQ ID NO: 48040 - DNA, 28 bp, synthetic construct
  source 1..28: mol_type = other DNA
agtgatgagatgaggcaggaactgaggg

SEQ ID NO: 48041 - DNA, 28 bp, synthetic construct
  source 1..28: mol_type = other DNA
gagtgatgagatgaggcaggaactgagg

SEQ ID NO: 48042 - DNA, 28 bp, synthetic construct
  source 1..28: mol_type = other DNA
acaactctgagtgatgagatgaggcagg

SEQ ID NO: 48043 - DNA, 28 bp, synthetic construct
  source 1..28: mol_type = other DNA
ccagacaactctgagtgatgagatgagg

SEQ ID NO: 48044 - DNA, 28 bp, synthetic construct
  source 1..28: mol_type = other DNA
tgtctggtccagcctgaaagcacaaagg

SEQ ID NO: 48045 - DNA, 28 bp, synthetic construct
  source 1..28: mol_type = other DNA
gtctggtccagcctgaaagcacaaaggg

SEQ ID NO: 48046 - DNA, 28 bp, synthetic construct
  source 1..28: mol_type = other DNA
tccagcctgaaagcacaaagggagccgg

SEQ ID NO: 48047 - DNA, 28 bp, synthetic construct
  source 1..28: mol_type = other DNA
cccggctccctttgtgctttcaggctgg

SEQ ID NO: 48048 - DNA, 28 bp, synthetic construct
  source 1..28: mol_type = other DNA
aggacccggctccctttgtgctttcagg

SEQ ID NO: 48049 - DNA, 28 bp, synthetic construct
  source 1..28: mol_type = other DNA
aagcacaaagggagccgggtcctcctgg

SEQ ID NO: 48050 - DNA, 28 bp, synthetic construct
  source 1..28: mol_type = other DNA
agcacaaagggagccgggtcctcctggg

SEQ ID NO: 48051 - DNA, 28 bp, synthetic construct
  source 1..28: mol_type = other DNA
ccgggtcctcctgggatcccccatgtgg

SEQ ID NO: 48052 - DNA, 28 bp, synthetic construct
  source 1..28: mol_type = other DNA
tggggaccacatgggggatcccaggagg

SEQ ID NO: 48053 - DNA, 28 bp, synthetic construct
  source 1..28: mol_type = other DNA
tcctgggatcccccatgtggtccccagg

SEQ ID NO: 48054 - DNA, 28 bp, synthetic construct
  source 1..28: mol_type = other DNA
acctggggaccacatgggggatcccagg

SEQ ID NO: 48055 - DNA, 28 bp, synthetic construct
  source 1..28: mol_type = other DNA
tcccccatgtggtccccaggtccccagg

SEQ ID NO: 48056 - DNA, 28 bp, synthetic construct
  source 1..28: mol_type = other DNA
ccctggggacctggggaccacatggggg

SEQ ID NO: 48057 - DNA, 28 bp, synthetic construct
  source 1..28: mol_type = other DNA
gccctggggacctggggaccacatgggg

SEQ ID NO: 48058 - DNA, 28 bp, synthetic construct
  source 1..28: mol_type = other DNA
ggccctggggacctggggaccacatggg

SEQ ID NO: 48059 - DNA, 28 bp, synthetic construct
  source 1..28: mol_type = other DNA
gggccctggggacctggggaccacatgg

SEQ ID NO: 48060 - DNA, 28 bp, synthetic construct
  source 1..28: mol_type = other DNA
caggattctgggccctggggacctgggg

SEQ ID NO: 48061 - DNA, 28 bp, synthetic construct
  source 1..28: mol_type = other DNA
cccaggtccccagggcccagaatcctgg

SEQ ID NO: 48062 - DNA, 28 bp, synthetic construct
  source 1..28: mol_type = other DNA
ccaggtccccagggcccagaatcctggg

SEQ ID NO: 48063 - DNA, 28 bp, synthetic construct
  source 1..28: mol_type = other DNA
acaggtcccaggattctgggccctgggg

SEQ ID NO: 48064 - DNA, 28 bp, synthetic construct
  source 1..28: mol_type = other DNA
gacaggtcccaggattctgggccctggg

SEQ ID NO: 48065 - DNA, 28 bp, synthetic construct
  source 1..28: mol_type = other DNA
tgacaggtcccaggattctgggccctgg

SEQ ID NO: 48066 - DNA, 28 bp, synthetic construct
  source 1..28: mol_type = other DNA
agaaggtgacaggtcccaggattctggg

SEQ ID NO: 48067 - DNA, 28 bp, synthetic construct
  source 1..28: mol_type = other DNA
cagaaggtgacaggtcccaggattctgg

SEQ ID NO: 48068 - DNA, 28 bp, synthetic construct
  source 1..28: mol_type = other DNA
gaatcctgggacctgtcaccttctgagg

SEQ ID NO: 48069 - DNA, 28 bp, synthetic construct
  source 1..28: mol_type = other DNA
gctgcctcagaaggtgacaggtcccagg

SEQ ID NO: 48070 - DNA, 28 bp, synthetic construct
  source 1..28: mol_type = other DNA
tgggacctgtcaccttctgaggcagcgg

SEQ ID NO: 48071 - DNA, 28 bp, synthetic construct
  source 1..28: mol_type = other DNA
tgcggccgctgcctcagaaggtgacagg

SEQ ID NO: 48072 - DNA, 28 bp, synthetic construct
  source 1..28: mol_type = other DNA
tgtcaccttctgaggcagcggccgcagg

SEQ ID NO: 48073 - DNA, 28 bp, synthetic construct
  source 1..28: mol_type = other DNA
gtcaccttctgaggcagcggccgcaggg

SEQ ID NO: 48074 - DNA, 28 bp, synthetic construct
  source 1..28: mol_type = other DNA
accttctgaggcagcggccgcagggtgg

SEQ ID NO: 48075 - DNA, 28 bp, synthetic construct
  source 1..28: mol_type = other DNA
ccttctgaggcagcggccgcagggtggg

SEQ ID NO: 48076 - DNA, 28 bp, synthetic construct
  source 1..28: mol_type = other DNA
ggcagcggccgcagggtgggttccctgg

SEQ ID NO: 48077 - DNA, 28 bp, synthetic construct
  source 1..28: mol_type = other DNA
taagtggtagagctggtaagaaacttgg

SEQ ID NO: 48078 - DNA, 28 bp, synthetic construct
  source 1..28: mol_type = other DNA
aagtggtagagctggtaagaaacttggg

SEQ ID NO: 48079 - DNA, 28 bp, synthetic construct
  source 1..28: mol_type = other DNA
ggtagagctggtaagaaacttgggttgg

SEQ ID NO: 48080 - DNA, 28 bp, synthetic construct
  source 1..28: mol_type = other DNA
ggggtatcggacaggggatggaaaaagg

SEQ ID NO: 48081 - DNA, 28 bp, synthetic construct
  source 1..28: mol_type = other DNA
ggttgggggggtatcggacaggggatgg

SEQ ID NO: 48082 - DNA, 28 bp, synthetic construct
  source 1..28: mol_type = other DNA
agagggttgggggggtatcggacagggg

SEQ ID NO: 48083 - DNA, 28 bp, synthetic construct
  source 1..28: mol_type = other DNA
aagagggttgggggggtatcggacaggg

SEQ ID NO: 48084 - DNA, 28 bp, synthetic construct
  source 1..28: mol_type = other DNA
gaagagggttgggggggtatcggacagg

SEQ ID NO: 48085 - DNA, 28 bp, synthetic construct
  source 1..28: mol_type = other DNA
agagggaagagggttgggggggtatcgg

SEQ ID NO: 48086 - DNA, 28 bp, synthetic construct
  source 1..28: mol_type = other DNA
ctgggcagagggaagagggttggggggg

SEQ ID NO: 48087 - DNA, 28 bp, synthetic construct
  source 1..28: mol_type = other DNA
tctgggcagagggaagagggttgggggg

SEQ ID NO: 48088 - DNA, 28 bp, synthetic construct
  source 1..28: mol_type = other DNA
ttctgggcagagggaagagggttggggg

SEQ ID NO: 48089 - DNA, 28 bp, synthetic construct
  source 1..28: mol_type = other DNA
cttctgggcagagggaagagggttgggg

SEQ ID NO: 48090 - DNA, 28 bp, synthetic construct
  source 1..28: mol_type = other DNA
cccaaccctcttccctctgcccagaagg

SEQ ID NO: 48091 - DNA, 28 bp, synthetic construct
  source 1..28: mol_type = other DNA
cccttctgggcagagggaagagggttgg

SEQ ID NO: 48092 - DNA, 28 bp, synthetic construct
  source 1..28: mol_type = other DNA
gggtcccttctgggcagagggaagaggg

SEQ ID NO: 48093 - DNA, 28 bp, synthetic construct
  source 1..28: mol_type = other DNA
tgggtcccttctgggcagagggaagagg

SEQ ID NO: 48094 - DNA, 28 bp, synthetic construct
  source 1..28: mol_type = other DNA
ttccctctgcccagaagggacccacagg

SEQ ID NO: 48095 - DNA, 28 bp, synthetic construct
  source 1..28: mol_type = other DNA
tccctctgcccagaagggacccacaggg

SEQ ID NO: 48096 - DNA, 28 bp, synthetic construct
  source 1..28: mol_type = other DNA
gccctgtgggtcccttctgggcagaggg

SEQ ID NO: 48097 - DNA, 28 bp, synthetic construct
  source 1..28: mol_type = other DNA
ggccctgtgggtcccttctgggcagagg

SEQ ID NO: 48098 - DNA, 28 bp, synthetic construct
  source 1..28: mol_type = other DNA
gggtaaggccctgtgggtcccttctggg

SEQ ID NO: 48099 - DNA, 28 bp, synthetic construct
  source 1..28: mol_type = other DNA
ggggtaaggccctgtgggtcccttctgg

SEQ ID NO: 48100 - DNA, 28 bp, synthetic construct
  source 1..28: mol_type = other DNA
gaagggacccacagggccttaccccagg

SEQ ID NO: 48101 - DNA, 28 bp, synthetic construct
  source 1..28: mol_type = other DNA
tcatacgcctggggtaaggccctgtggg

SEQ ID NO: 48102 - DNA, 28 bp, synthetic construct
  source 1..28: mol_type = other DNA
ctcatacgcctggggtaaggccctgtgg

SEQ ID NO: 48103 - DNA, 28 bp, synthetic construct
  source 1..28: mol_type = other DNA
cctgcaaactcatacgcctggggtaagg

SEQ ID NO: 48104 - DNA, 28 bp, synthetic construct
  source 1..28: mol_type = other DNA
accccaggcgtatgagtttgcaggcagg

SEQ ID NO: 48105 - DNA, 28 bp, synthetic construct
  source 1..28: mol_type = other DNA
tcctgcctgcaaactcatacgcctgggg

SEQ ID NO: 48106 - DNA, 28 bp, synthetic construct
  source 1..28: mol_type = other DNA
atcctgcctgcaaactcatacgcctggg

SEQ ID NO: 48107 - DNA, 28 bp, synthetic construct
  source 1..28: mol_type = other DNA
catcctgcctgcaaactcatacgcctgg

SEQ ID NO: 48108 - DNA, 28 bp, synthetic construct
  source 1..28: mol_type = other DNA
cgtgcgactgctctgtgaggggctcagg

SEQ ID NO: 48109 - DNA, 28 bp, synthetic construct
  source 1..28: mol_type = other DNA
cgttggcgtgcgactgctctgtgagggg

SEQ ID NO: 48110 - DNA, 28 bp, synthetic construct
  source 1..28: mol_type = other DNA
acgttggcgtgcgactgctctgtgaggg

SEQ ID NO: 48111 - DNA, 28 bp, synthetic construct
  source 1..28: mol_type = other DNA
gacgttggcgtgcgactgctctgtgagg

SEQ ID NO: 48112 - DNA, 28 bp, synthetic construct
  source 1..28: mol_type = other DNA
gagcagtcgcacgccaacgtcatccagg

SEQ ID NO: 48113 - DNA, 28 bp, synthetic construct
  source 1..28: mol_type = other DNA
tgcagcagaacaacctggatgacgttgg

SEQ ID NO: 48114 - DNA, 28 bp, synthetic construct
  source 1..28: mol_type = other DNA
aacgtcatccaggttgttctgctgcagg

SEQ ID NO: 48115 - DNA, 28 bp, synthetic construct
  source 1..28: mol_type = other DNA
gagctagacctgcagcagaacaacctgg

SEQ ID NO: 48116 - DNA, 28 bp, synthetic construct
  source 1..28: mol_type = other DNA
gttctgctgcaggtctagctccttcagg

SEQ ID NO: 48117 - DNA, 28 bp, synthetic construct
  source 1..28: mol_type = other DNA
tgctgcaggtctagctccttcaggctgg

SEQ ID NO: 48118 - DNA, 28 bp, synthetic construct
  source 1..28: mol_type = other DNA
gctgcaggtctagctccttcaggctggg

SEQ ID NO: 48119 - DNA, 28 bp, synthetic construct
  source 1..28: mol_type = other DNA
ctgcaggtctagctccttcaggctgggg

SEQ ID NO: 48120 - DNA, 28 bp, synthetic construct
  source 1..28: mol_type = other DNA
aggtctagctccttcaggctggggctgg

SEQ ID NO: 48121 - DNA, 28 bp, synthetic construct
  source 1..28: mol_type = other DNA
gtgcttagtgccagccccagcctgaagg

SEQ ID NO: 48122 - DNA, 28 bp, synthetic construct
  source 1..28: mol_type = other DNA
aggctggggctggcactaagcacagagg

SEQ ID NO: 48123 - DNA, 28 bp, synthetic construct
  source 1..28: mol_type = other DNA
ggggctggcactaagcacagaggccagg

SEQ ID NO: 48124 - DNA, 28 bp, synthetic construct
  source 1..28: mol_type = other DNA
ggcactaagcacagaggccaggtcctgg

SEQ ID NO: 48125 - DNA, 28 bp, synthetic construct
  source 1..28: mol_type = other DNA
ctcacgtctgactgctgccaggacctgg

SEQ ID NO: 48126 - DNA, 28 bp, synthetic construct
  source 1..28: mol_type = other DNA
caggtcctggcagcagtcagacgtgagg

SEQ ID NO: 48127 - DNA, 28 bp, synthetic construct
  source 1..28: mol_type = other DNA
tgtggcctcacgtctgactgctgccagg

SEQ ID NO: 48128 - DNA, 28 bp, synthetic construct
  source 1..28: mol_type = other DNA
gtgaggccacagctgaccagcctgcagg

SEQ ID NO: 48129 - DNA, 28 bp, synthetic construct
  source 1..28: mol_type = other DNA
atctttcctgcaggctggtcagctgtgg

SEQ ID NO: 48130 - DNA, 28 bp, synthetic construct
  source 1..28: mol_type = other DNA
gctggcgtgtatctttcctgcaggctgg

SEQ ID NO: 48131 - DNA, 28 bp, synthetic construct
  source 1..28: mol_type = other DNA
ctgggctggcgtgtatctttcctgcagg

SEQ ID NO: 48132 - DNA, 28 bp, synthetic construct
  source 1..28: mol_type = other DNA
ctgcaggaaagatacacgccagcccagg

SEQ ID NO: 48133 - DNA, 28 bp, synthetic construct
  source 1..28: mol_type = other DNA
cacgccagcccaggtcattgtcctaagg

SEQ ID NO: 48134 - DNA, 28 bp, synthetic construct
  source 1..28: mol_type = other DNA
acgccagcccaggtcattgtcctaaggg

SEQ ID NO: 48135 - DNA, 28 bp, synthetic construct
  source 1..28: mol_type = other DNA
gagcccttaggacaatgacctgggctgg

SEQ ID NO: 48136 - DNA, 28 bp, synthetic construct
  source 1..28: mol_type = other DNA
gagcgagcccttaggacaatgacctggg

SEQ ID NO: 48137 - DNA, 28 bp, synthetic construct
  source 1..28: mol_type = other DNA
agagcgagcccttaggacaatgacctgg

SEQ ID NO: 48138 - DNA, 28 bp, synthetic construct
  source 1..28: mol_type = other DNA
tcattgtcctaagggctcgctcttcagg

SEQ ID NO: 48139 - DNA, 28 bp, synthetic construct
  source 1..28: mol_type = other DNA
cattgtcctaagggctcgctcttcaggg

SEQ ID NO: 48140 - DNA, 28 bp, synthetic construct
  source 1..28: mol_type = other DNA
tagttaccctgaagagcgagcccttagg

SEQ ID NO: 48141 - DNA, 28 bp, synthetic construct
  source 1..28: mol_type = other DNA
taagggctcgctcttcagggtaactagg

SEQ ID NO: 48142 - DNA, 28 bp, synthetic construct
  source 1..28: mol_type = other DNA
aagggctcgctcttcagggtaactaggg

SEQ ID NO: 48143 - DNA, 28 bp, synthetic construct
  source 1..28: mol_type = other DNA
gtctgatcttccttctcagcatctgtgg

SEQ ID NO: 48144 - DNA, 28 bp, synthetic construct
  source 1..28: mol_type = other DNA
ccttctcagcatctgtggccttttgagg

SEQ ID NO: 48145 - DNA, 28 bp, synthetic construct
  source 1..28: mol_type = other DNA
cttctcagcatctgtggccttttgaggg

SEQ ID NO: 48146 - DNA, 28 bp, synthetic construct
  source 1..28: mol_type = other DNA
cagcatctgtggccttttgagggtctgg

SEQ ID NO: 48147 - DNA, 28 bp, synthetic construct
  source 1..28: mol_type = other DNA
agcatctgtggccttttgagggtctggg

SEQ ID NO: 48148 - DNA, 28 bp, synthetic construct
  source 1..28: mol_type = other DNA
ctgcatgtcatcccagaccctcaaaagg

SEQ ID NO: 48149 - DNA, 28 bp, synthetic construct
  source 1..28: mol_type = other DNA
ctttgtgggagtgggaggagcctacagg

SEQ ID NO: 48150 - DNA, 28 bp, synthetic construct
  source 1..28: mol_type = other DNA
taggctcctcccactcccacaaagcagg

SEQ ID NO: 48151 - DNA, 28 bp, synthetic construct
  source 1..28: mol_type = other DNA
gtgagacctgctttgtgggagtgggagg

SEQ ID NO: 48152 - DNA, 28 bp, synthetic construct
  source 1..28: mol_type = other DNA
aaggtgagacctgctttgtgggagtggg

SEQ ID NO: 48153 - DNA, 28 bp, synthetic construct
  source 1..28: mol_type = other DNA
gaaggtgagacctgctttgtgggagtgg

SEQ ID NO: 48154 - DNA, 28 bp, synthetic construct
  source 1..28: mol_type = other DNA
agagagaaggtgagacctgctttgtggg

SEQ ID NO: 48155 - DNA, 28 bp, synthetic construct
  source 1..28: mol_type = other DNA
cagagagaaggtgagacctgctttgtgg

SEQ ID NO: 48156 - DNA, 28 bp, synthetic construct
  source 1..28: mol_type = other DNA
caggcagagggtaagagcagagagaagg

SEQ ID NO: 48157 - DNA, 28 bp, synthetic construct
  source 1..28: mol_type = other DNA
ctgctcttaccctctgcctgcctcatgg

SEQ ID NO: 48158 - DNA, 28 bp, synthetic construct
  source 1..28: mol_type = other DNA
ctcttaccctctgcctgcctcatggtgg

SEQ ID NO: 48159 - DNA, 28 bp, synthetic construct
  source 1..28: mol_type = other DNA
taccctctgcctgcctcatggtggcagg

SEQ ID NO: 48160 - DNA, 28 bp, synthetic construct
  source 1..28: mol_type = other DNA
tgcctgccaccatgaggcaggcagaggg

SEQ ID NO: 48161 - DNA, 28 bp, synthetic construct
  source 1..28: mol_type = other DNA
ctgcctgccaccatgaggcaggcagagg

SEQ ID NO: 48162 - DNA, 28 bp, synthetic construct
  source 1..28: mol_type = other DNA
agggaactgcctgccaccatgaggcagg

SEQ ID NO: 48163 - DNA, 28 bp, synthetic construct
  source 1..28: mol_type = other DNA
gtggagggaactgcctgccaccatgagg

SEQ ID NO: 48164 - DNA, 28 bp, synthetic construct
  source 1..28: mol_type = other DNA
ttcttggtgggcagggggaggtggaggg

SEQ ID NO: 48165 - DNA, 28 bp, synthetic construct
  source 1..28: mol_type = other DNA
gttcttggtgggcagggggaggtggagg

SEQ ID NO: 48166 - DNA, 28 bp, synthetic construct
  source 1..28: mol_type = other DNA
attgttcttggtgggcagggggaggtgg

SEQ ID NO: 48167 - DNA, 28 bp, synthetic construct
  source 1..28: mol_type = other DNA
gtaattgttcttggtgggcagggggagg

SEQ ID NO: 48168 - DNA, 28 bp, synthetic construct
  source 1..28: mol_type = other DNA
gcagtaattgttcttggtgggcaggggg

SEQ ID NO: 48169 - DNA, 28 bp, synthetic construct
  source 1..28: mol_type = other DNA
tgcagtaattgttcttggtgggcagggg

SEQ ID NO: 48170 - DNA, 28 bp, synthetic construct
  source 1..28: mol_type = other DNA
ctgcagtaattgttcttggtgggcaggg

SEQ ID NO: 48171 - DNA, 28 bp, synthetic construct
  source 1..28: mol_type = other DNA
actgcagtaattgttcttggtgggcagg

SEQ ID NO: 48172 - DNA, 28 bp, synthetic construct
  source 1..28: mol_type = other DNA
agcgactgcagtaattgttcttggtggg

SEQ ID NO: 48173 - DNA, 28 bp, synthetic construct
  source 1..28: mol_type = other DNA
cagcgactgcagtaattgttcttggtgg

SEQ ID NO: 48174 - DNA, 28 bp, synthetic construct
  source 1..28: mol_type = other DNA
ctacagcgactgcagtaattgttcttgg

SEQ ID NO: 48175 - DNA, 28 bp, synthetic construct
  source 1..28: mol_type = other DNA
actgcagtcgctgtagcttgcagctcgg

SEQ ID NO: 48176 - DNA, 28 bp, synthetic construct
  source 1..28: mol_type = other DNA
cttgcagctcggctgtctcagtctctgg

SEQ ID NO: 48177 - DNA, 28 bp, synthetic construct
  source 1..28: mol_type = other DNA
gctcggctgtctcagtctctggcaaagg

SEQ ID NO: 48178 - DNA, 28 bp, synthetic construct
  source 1..28: mol_type = other DNA
tgtctcagtctctggcaaaggtgtttgg

SEQ ID NO: 48179 - DNA, 28 bp, synthetic construct
  source 1..28: mol_type = other DNA
tgagcttcaatgtgctcacggatgctgg

SEQ ID NO: 48180 - DNA, 28 bp, synthetic construct
  source 1..28: mol_type = other DNA
agcatccgtgagcacattgaagctcagg

SEQ ID NO: 48181 - DNA, 28 bp, synthetic construct
  source 1..28: mol_type = other DNA
ctggacctgagcttcaatgtgctcacgg

SEQ ID NO: 48182 - DNA, 28 bp, synthetic construct
  source 1..28: mol_type = other DNA
agcacattgaagctcaggtccagctcgg

SEQ ID NO: 48183 - DNA, 28 bp, synthetic construct
  source 1..28: mol_type = other DNA
attgaagctcaggtccagctcggtcagg

SEQ ID NO: 48184 - DNA, 28 bp, synthetic construct
  source 1..28: mol_type = other DNA
ttgaagctcaggtccagctcggtcaggg

SEQ ID NO: 48185 - DNA, 28 bp, synthetic construct
  source 1..28: mol_type = other DNA
gctcaggtccagctcggtcagggtctgg

SEQ ID NO: 48186 - DNA, 28 bp, synthetic construct
  source 1..28: mol_type = other DNA
aggtccagctcggtcagggtctggttgg

SEQ ID NO: 48187 - DNA, 28 bp, synthetic construct
  source 1..28: mol_type = other DNA
agagccaaccagaccctgaccgagctgg

SEQ ID NO: 48188 - DNA, 28 bp, synthetic construct
  source 1..28: mol_type = other DNA
agggtctggttggctctcagcccaaagg

SEQ ID NO: 48189 - DNA, 28 bp, synthetic construct
  source 1..28: mol_type = other DNA
ctggttggctctcagcccaaaggcaagg

SEQ ID NO: 48190 - DNA, 28 bp, synthetic construct
  source 1..28: mol_type = other DNA
tgaggactgcaaggaccttgcctttggg

SEQ ID NO: 48191 - DNA, 28 bp, synthetic construct
  source 1..28: mol_type = other DNA
ctgaggactgcaaggaccttgcctttgg

SEQ ID NO: 48192 - DNA, 28 bp, synthetic construct
  source 1..28: mol_type = other DNA
aaggtccttgcagtcctcagctgtgagg

SEQ ID NO: 48193 - DNA, 28 bp, synthetic construct
  source 1..28: mol_type = other DNA
tgtggcctcacagctgaggactgcaagg

SEQ ID NO: 48194 - DNA, 28 bp, synthetic construct
  source 1..28: mol_type = other DNA
ttggctggctgtggcctcacagctgagg

SEQ ID NO: 48195 - DNA, 28 bp, synthetic construct
  source 1..28: mol_type = other DNA
tgtgaggccacagccagccaacctgtgg

SEQ ID NO: 48196 - DNA, 28 bp, synthetic construct
  source 1..28: mol_type = other DNA
gtgtcttccacaggttggctggctgtgg

SEQ ID NO: 48197 - DNA, 28 bp, synthetic construct
  source 1..28: mol_type = other DNA
gggtgtgtgtcttccacaggttggctgg

SEQ ID NO: 48198 - DNA, 28 bp, synthetic construct
  source 1..28: mol_type = other DNA
ccatgggtgtgtgtcttccacaggttgg

SEQ ID NO: 48199 - DNA, 28 bp, synthetic construct
  source 1..28: mol_type = other DNA
aagaccatgggtgtgtgtcttccacagg

SEQ ID NO: 48200 - DNA, 28 bp, synthetic construct
  source 1..28: mol_type = other DNA
tggaagacacacacccatggtcttcagg

SEQ ID NO: 48201 - DNA, 28 bp, synthetic construct
  source 1..28: mol_type = other DNA
aacaggtgagtaacctgaagaccatggg

SEQ ID NO: 48202 - DNA, 28 bp, synthetic construct
  source 1..28: mol_type = other DNA
caacaggtgagtaacctgaagaccatgg

SEQ ID NO: 48203 - DNA, 28 bp, synthetic construct
  source 1..28: mol_type = other DNA
gcttatgggtgtctgttgaatcaacagg

SEQ ID NO: 48204 - DNA, 28 bp, synthetic construct
  source 1..28: mol_type = other DNA
tagtaggtgattaatggttgcttatggg

SEQ ID NO: 48205 - DNA, 28 bp, synthetic construct
  source 1..28: mol_type = other DNA
atagtaggtgattaatggttgcttatgg

SEQ ID NO: 48206 - DNA, 28 bp, synthetic construct
  source 1..28: mol_type = other DNA
aaccattaatcacctactatgcaccagg

SEQ ID NO: 48207 - DNA, 28 bp, synthetic construct
  source 1..28: mol_type = other DNA
ggcctggtgcatagtaggtgattaatgg

SEQ ID NO: 48208 - DNA, 28 bp, synthetic construct
  source 1..28: mol_type = other DNA
aatcacctactatgcaccaggcctgtgg

SEQ ID NO: 48209 - DNA, 28 bp, synthetic construct
  source 1..28: mol_type = other DNA
atcacctactatgcaccaggcctgtggg

SEQ ID NO: 48210 - DNA, 28 bp, synthetic construct
  source 1..28: mol_type = other DNA
ctggcccacaggcctggtgcatagtagg

SEQ ID NO: 48211 - DNA, 28 bp, synthetic construct
  source 1..28: mol_type = other DNA
ctactatgcaccaggcctgtgggccagg

SEQ ID NO: 48212 - DNA, 28 bp, synthetic construct
  source 1..28: mol_type = other DNA
tgcaccaggcctgtgggccaggcagagg

SEQ ID NO: 48213 - DNA, 28 bp, synthetic construct
  source 1..28: mol_type = other DNA
tagacctctgcctggcccacaggcctgg

SEQ ID NO: 48214 - DNA, 28 bp, synthetic construct
  source 1..28: mol_type = other DNA
ttttctagacctctgcctggcccacagg

SEQ ID NO: 48215 - DNA, 28 bp, synthetic construct
  source 1..28: mol_type = other DNA
atattcgttgaggccttctctggccggg

SEQ ID NO: 48216 - DNA, 28 bp, synthetic construct
  source 1..28: mol_type = other DNA
aatattcgttgaggccttctctggccgg

SEQ ID NO: 48217 - DNA, 28 bp, synthetic construct
  source 1..28: mol_type = other DNA
atcaaatattcgttgaggccttctctgg

SEQ ID NO: 48218 - DNA, 28 bp, synthetic construct
  source 1..28: mol_type = other DNA
ctttgtatttatcaaatattcgttgagg

SEQ ID NO: 48219 - DNA, 28 bp, synthetic construct
  source 1..28: mol_type = other DNA
aaggcagaagctgagtctgggctgaggg

SEQ ID NO: 48220 - DNA, 28 bp, synthetic construct
  source 1..28: mol_type = other DNA
caaggcagaagctgagtctgggctgagg

SEQ ID NO: 48221 - DNA, 28 bp, synthetic construct
  source 1..28: mol_type = other DNA
ctcagcccagactcagcttctgccttgg

SEQ ID NO: 48222 - DNA, 28 bp, synthetic construct
  source 1..28: mol_type = other DNA
gagatccaaggcagaagctgagtctggg

SEQ ID NO: 48223 - DNA, 28 bp, synthetic construct
  source 1..28: mol_type = other DNA
agagatccaaggcagaagctgagtctgg

SEQ ID NO: 48224 - DNA, 28 bp, synthetic construct
  source 1..28: mol_type = other DNA
gaagcagggatggggaagagatccaagg

SEQ ID NO: 48225 - DNA, 28 bp, synthetic construct
  source 1..28: mol_type = other DNA
tgggttctgttctgaagcagggatgggg

SEQ ID NO: 48226 - DNA, 28 bp, synthetic construct
  source 1..28: mol_type = other DNA
ctgggttctgttctgaagcagggatggg

SEQ ID NO: 48227 - DNA, 28 bp, synthetic construct
  source 1..28: mol_type = other DNA
ccatccctgcttcagaacagaacccagg

SEQ ID NO: 48228 - DNA, 28 bp, synthetic construct
  source 1..28: mol_type = other DNA
ctggcctgggttctgttctgaagcaggg

SEQ ID NO: 48229 - DNA, 28 bp, synthetic construct
  source 1..28: mol_type = other DNA
tctggcctgggttctgttctgaagcagg

SEQ ID NO: 48230 - DNA, 28 bp, synthetic construct
  source 1..28: mol_type = other DNA
acagaacccaggccagactcaccgcagg

SEQ ID NO: 48231 - DNA, 28 bp, synthetic construct
  source 1..28: mol_type = other DNA
cagaacccaggccagactcaccgcaggg

SEQ ID NO: 48232 - DNA, 28 bp, synthetic construct
  source 1..28: mol_type = other DNA
ggagaccctgcggtgagtctggcctggg

SEQ ID NO: 48233 - DNA, 28 bp, synthetic construct
  source 1..28: mol_type = other DNA
tggagaccctgcggtgagtctggcctgg

SEQ ID NO: 48234 - DNA, 28 bp, synthetic construct
  source 1..28: mol_type = other DNA
aggccagactcaccgcagggtctccagg

SEQ ID NO: 48235 - DNA, 28 bp, synthetic construct
  source 1..28: mol_type = other DNA
cctcctggagaccctgcggtgagtctgg

SEQ ID NO: 48236 - DNA, 28 bp, synthetic construct
  source 1..28: mol_type = other DNA
accgcagggtctccaggaggcagcgagg

SEQ ID NO: 48237 - DNA, 28 bp, synthetic construct
  source 1..28: mol_type = other DNA
ccctcgctgcctcctggagaccctgcgg

SEQ ID NO: 48238 - DNA, 28 bp, synthetic construct
  source 1..28: mol_type = other DNA
ctccaggaggcagcgagggcgtctcagg

SEQ ID NO: 48239 - DNA, 28 bp, synthetic construct
  source 1..28: mol_type = other DNA
tccaggaggcagcgagggcgtctcaggg

SEQ ID NO: 48240 - DNA, 28 bp, synthetic construct
  source 1..28: mol_type = other DNA
accctgagacgccctcgctgcctcctgg

SEQ ID NO: 48241 - DNA, 28 bp, synthetic construct
  source 1..28: mol_type = other DNA
cttacaaagactcttcactgcagagtgg

SEQ ID NO: 48242 - DNA, 28 bp, synthetic construct
  source 1..28: mol_type = other DNA
agagtggctcagcgagtttccacttagg

SEQ ID NO: 48243 - DNA, 28 bp, synthetic construct
  source 1..28: mol_type = other DNA
gtttccacttaggtccagctccttcagg

SEQ ID NO: 48244 - DNA, 28 bp, synthetic construct
  source 1..28: mol_type = other DNA
gaaacctgaaggagctggacctaagtgg

SEQ ID NO: 48245 - DNA, 28 bp, synthetic construct
  source 1..28: mol_type = other DNA
cttaggtccagctccttcaggtttctgg

SEQ ID NO: 48246 - DNA, 28 bp, synthetic construct
  source 1..28: mol_type = other DNA
aaggtcaccagaaacctgaaggagctgg

SEQ ID NO: 48247 - DNA, 28 bp, synthetic construct
  source 1..28: mol_type = other DNA
ctccttcaggtttctggtgaccttgagg

SEQ ID NO: 48248 - DNA, 28 bp, synthetic construct
  source 1..28: mol_type = other DNA
gtcctcaaggtcaccagaaacctgaagg

SEQ ID NO: 48249 - DNA, 28 bp, synthetic construct
  source 1..28: mol_type = other DNA
ttcaggtttctggtgaccttgaggacgg

SEQ ID NO: 48250 - DNA, 28 bp, synthetic construct
  source 1..28: mol_type = other DNA
tggcagattctcttctccgtcctcaagg

SEQ ID NO: 48251 - DNA, 28 bp, synthetic construct
  source 1..28: mol_type = other DNA
aggacggagaagagaatctgccaatagg

SEQ ID NO: 48252 - DNA, 28 bp, synthetic construct
  source 1..28: mol_type = other DNA
gaatctgccaataggcatctgtgactgg

SEQ ID NO: 48253 - DNA, 28 bp, synthetic construct
  source 1..28: mol_type = other DNA
aatctgccaataggcatctgtgactggg

SEQ ID NO: 48254 - DNA, 28 bp, synthetic construct
  source 1..28: mol_type = other DNA
gtgggtcccagtcacagatgcctattgg

SEQ ID NO: 48255 - DNA, 28 bp, synthetic construct
  source 1..28: mol_type = other DNA
tgtgactgggacccacctgaacctgagg

SEQ ID NO: 48256 - DNA, 28 bp, synthetic construct
  source 1..28: mol_type = other DNA
gtgactgggacccacctgaacctgaggg

SEQ ID NO: 48257 - DNA, 28 bp, synthetic construct
  source 1..28: mol_type = other DNA
tgactgggacccacctgaacctgagggg

SEQ ID NO: 48258 - DNA, 28 bp, synthetic construct
  source 1..28: mol_type = other DNA
gactgggacccacctgaacctgaggggg

SEQ ID NO: 48259 - DNA, 28 bp, synthetic construct
  source 1..28: mol_type = other DNA
ttctctctccccctcaggttcaggtggg

SEQ ID NO: 48260 - DNA, 28 bp, synthetic construct
  source 1..28: mol_type = other DNA
cttctctctccccctcaggttcaggtgg

SEQ ID NO: 48261 - DNA, 28 bp, synthetic construct
  source 1..28: mol_type = other DNA
cacctgaacctgagggggagagagaagg

SEQ ID NO: 48262 - DNA, 28 bp, synthetic construct
  source 1..28: mol_type = other DNA
gtccttctctctccccctcaggttcagg

SEQ ID NO: 48263 - DNA, 28 bp, synthetic construct
  source 1..28: mol_type = other DNA
gaacctgagggggagagagaaggacagg

SEQ ID NO: 48264 - DNA, 28 bp, synthetic construct
  source 1..28: mol_type = other DNA
tctcctgtccttctctctccccctcagg

SEQ ID NO: 48265 - DNA, 28 bp, synthetic construct
  source 1..28: mol_type = other DNA
aaggacaggagagatgtgatgtgtctgg

SEQ ID NO: 48266 - DNA, 28 bp, synthetic construct
  source 1..28: mol_type = other DNA
acaggagagatgtgatgtgtctggcagg

SEQ ID NO: 48267 - DNA, 28 bp, synthetic construct
  source 1..28: mol_type = other DNA
caggagagatgtgatgtgtctggcaggg

SEQ ID NO: 48268 - DNA, 28 bp, synthetic construct
  source 1..28: mol_type = other DNA
aggagagatgtgatgtgtctggcagggg

SEQ ID NO: 48269 - DNA, 28 bp, synthetic construct
  source 1..28: mol_type = other DNA
atgtgatgtgtctggcaggggtttgagg

SEQ ID NO: 48270 - DNA, 28 bp, synthetic construct
  source 1..28: mol_type = other DNA
ggtgcccagccctgcacaacacagttgg

SEQ ID NO: 48271 - DNA, 28 bp, synthetic construct
  source 1..28: mol_type = other DNA
gtgcccagccctgcacaacacagttggg

SEQ ID NO: 48272 - DNA, 28 bp, synthetic construct
  source 1..28: mol_type = other DNA
aagcccaactgtgttgtgcagggctggg

SEQ ID NO: 48273 - DNA, 28 bp, synthetic construct
  source 1..28: mol_type = other DNA
aaagcccaactgtgttgtgcagggctgg

SEQ ID NO: 48274 - DNA, 28 bp, synthetic construct
  source 1..28: mol_type = other DNA
ggacaaagcccaactgtgttgtgcaggg

SEQ ID NO: 48275 - DNA, 28 bp, synthetic construct
  source 1..28: mol_type = other DNA
gggacaaagcccaactgtgttgtgcagg

SEQ ID NO: 48276 - DNA, 28 bp, synthetic construct
  source 1..28: mol_type = other DNA
gttgggctttgtccccctgagcaccagg

SEQ ID NO: 48277 - DNA, 28 bp, synthetic construct
  source 1..28: mol_type = other DNA
tgtccccctgagcaccaggccacagcgg

SEQ ID NO: 48278 - DNA, 28 bp, synthetic construct
  source 1..28: mol_type = other DNA
gtccccctgagcaccaggccacagcggg

SEQ ID NO: 48279 - DNA, 28 bp, synthetic construct
  source 1..28: mol_type = other DNA
tacccgctgtggcctggtgctcaggggg

SEQ ID NO: 48280 - DNA, 28 bp, synthetic construct
  source 1..28: mol_type = other DNA
ctacccgctgtggcctggtgctcagggg

SEQ ID NO: 48281 - DNA, 28 bp, synthetic construct
  source 1..28: mol_type = other DNA
actacccgctgtggcctggtgctcaggg

SEQ ID NO: 48282 - DNA, 28 bp, synthetic construct
  source 1..28: mol_type = other DNA
cactacccgctgtggcctggtgctcagg

SEQ ID NO: 48283 - DNA, 28 bp, synthetic construct
  source 1..28: mol_type = other DNA
gggggtgggggtggctaaaggatcaggg

SEQ ID NO: 48284 - DNA, 28 bp, synthetic construct
  source 1..28: mol_type = other DNA
cgggggtgggggtggctaaaggatcagg

SEQ ID NO: 48285 - DNA, 28 bp, synthetic construct
  source 1..28: mol_type = other DNA
ctgatcctttagccacccccacccccgg

SEQ ID NO: 48286 - DNA, 28 bp, synthetic construct
  source 1..28: mol_type = other DNA
cctttagccacccccacccccggccagg

SEQ ID NO: 48287 - DNA, 28 bp, synthetic construct
  source 1..28: mol_type = other DNA
cactgagcctggccgggggtgggggtgg

SEQ ID NO: 48288 - DNA, 28 bp, synthetic construct
  source 1..28: mol_type = other DNA
gctcactgagcctggccgggggtggggg

SEQ ID NO: 48289 - DNA, 28 bp, synthetic construct
  source 1..28: mol_type = other DNA
tgctcactgagcctggccgggggtgggg

SEQ ID NO: 48290 - DNA, 28 bp, synthetic construct
  source 1..28: mol_type = other DNA
atgctcactgagcctggccgggggtggg

SEQ ID NO: 48291 - DNA, 28 bp, synthetic construct
  source 1..28: mol_type = other DNA
catgctcactgagcctggccgggggtgg

SEQ ID NO: 48292 - DNA, 28 bp, synthetic construct
  source 1..28: mol_type = other DNA
aggcatgctcactgagcctggccggggg

SEQ ID NO: 48293 - DNA, 28 bp, synthetic construct
  source 1..28: mol_type = other DNA
gaggcatgctcactgagcctggccgggg

SEQ ID NO: 48294 - DNA, 28 bp, synthetic construct
  source 1..28: mol_type = other DNA
agaggcatgctcactgagcctggccggg

SEQ ID NO: 48295 - DNA, 28 bp, synthetic construct
  source 1..28: mol_type = other DNA
cagaggcatgctcactgagcctggccgg

SEQ ID NO: 48296 - DNA, 28 bp, synthetic construct
  source 1..28: mol_type = other DNA
cggccaggctcagtgagcatgcctctgg

SEQ ID NO: 48297 - DNA, 28 bp, synthetic construct
  source 1..28: mol_type = other DNA
gcaccagaggcatgctcactgagcctgg

SEQ ID NO: 48298 - DNA, 28 bp, synthetic construct
  source 1..28: mol_type = other DNA
ctcagtgagcatgcctctggtgctcagg

SEQ ID NO: 48299 - DNA, 28 bp, synthetic construct
  source 1..28: mol_type = other DNA
gcatgcctctggtgctcaggtcactcgg

SEQ ID NO: 48300 - DNA, 28 bp, synthetic construct
  source 1..28: mol_type = other DNA
catgcctctggtgctcaggtcactcggg

SEQ ID NO: 48301 - DNA, 28 bp, synthetic construct
  source 1..28: mol_type = other DNA
taagcccgagtgacctgagcaccagagg

SEQ ID NO: 48302 - DNA, 28 bp, synthetic construct
  source 1..28: mol_type = other DNA
ctggtgctcaggtcactcgggcttatgg

SEQ ID NO: 48303 - DNA, 28 bp, synthetic construct
  source 1..28: mol_type = other DNA
gtcactcgggcttatggactgacagagg

SEQ ID NO: 48304 - DNA, 28 bp, synthetic construct
  source 1..28: mol_type = other DNA
tggactgacagaggagctgcagacatgg

SEQ ID NO: 48305 - DNA, 28 bp, synthetic construct
  source 1..28: mol_type = other DNA
ggactgacagaggagctgcagacatggg

SEQ ID NO: 48306 - DNA, 28 bp, synthetic construct
  source 1..28: mol_type = other DNA
ctgacagaggagctgcagacatgggtgg

SEQ ID NO: 48307 - DNA, 28 bp, synthetic construct
  source 1..28: mol_type = other DNA
agaggagctgcagacatgggtggtttgg

SEQ ID NO: 48308 - DNA, 28 bp, synthetic construct
  source 1..28: mol_type = other DNA
gaggagctgcagacatgggtggtttggg

SEQ ID NO: 48309 - DNA, 28 bp, synthetic construct
  source 1..28: mol_type = other DNA
agacatgggtggtttgggtactcacagg

SEQ ID NO: 48310 - DNA, 28 bp, synthetic construct
  source 1..28: mol_type = other DNA
ggtttgggtactcacaggactaccatgg

SEQ ID NO: 48311 - DNA, 28 bp, synthetic construct
  source 1..28: mol_type = other DNA
ttgggtactcacaggactaccatggtgg

SEQ ID NO: 48312 - DNA, 28 bp, synthetic construct
  source 1..28: mol_type = other DNA
tgggtactcacaggactaccatggtggg

SEQ ID NO: 48313 - DNA, 28 bp, synthetic construct
  source 1..28: mol_type = other DNA
gggtactcacaggactaccatggtgggg

SEQ ID NO: 48314 - DNA, 28 bp, synthetic construct
  source 1..28: mol_type = other DNA
cacagatcaacatggagccccaccatgg

SEQ ID NO: 48315 - DNA, 28 bp, synthetic construct
  source 1..28: mol_type = other DNA
tgagggcaggcagcacagatcaacatgg

SEQ ID NO: 48316 - DNA, 28 bp, synthetic construct
  source 1..28: mol_type = other DNA
gaagaagcttcagctgattgagggcagg

SEQ ID NO: 48317 - DNA, 28 bp, synthetic construct
  source 1..28: mol_type = other DNA
acgtgaagaagcttcagctgattgaggg

SEQ ID NO: 48318 - DNA, 28 bp, synthetic construct
  source 1..28: mol_type = other DNA
cacgtgaagaagcttcagctgattgagg

SEQ ID NO: 48319 - DNA, 28 bp, synthetic construct
  source 1..28: mol_type = other DNA
ctcaatcagctgaagcttcttcacgtgg

SEQ ID NO: 48320 - DNA, 28 bp, synthetic construct
  source 1..28: mol_type = other DNA
aatcagctgaagcttcttcacgtggcgg

SEQ ID NO: 48321 - DNA, 28 bp, synthetic construct
  source 1..28: mol_type = other DNA
atgggcatgtgtgtagaaacagacatgg

SEQ ID NO: 48322 - DNA, 28 bp, synthetic construct
  source 1..28: mol_type = other DNA
tacacacatgcccatttcttcgaaatgg

SEQ ID NO: 48323 - DNA, 28 bp, synthetic construct
  source 1..28: mol_type = other DNA
acacacatgcccatttcttcgaaatggg

SEQ ID NO: 48324 - DNA, 28 bp, synthetic construct
  source 1..28: mol_type = other DNA
aagtgatggcccatttcgaagaaatggg

SEQ ID NO: 48325 - DNA, 28 bp, synthetic construct
  source 1..28: mol_type = other DNA
caagtgatggcccatttcgaagaaatgg

SEQ ID NO: 48326 - DNA, 28 bp, synthetic construct
  source 1..28: mol_type = other DNA
ttcgaaatgggccatcacttgtgtcagg

SEQ ID NO: 48327 - DNA, 28 bp, synthetic construct
  source 1..28: mol_type = other DNA
aacaaaacgttcctgacacaagtgatgg

SEQ ID NO: 48328 - DNA, 28 bp, synthetic construct
  source 1..28: mol_type = other DNA
tttgttccgagtctcgtacaagcagtgg

SEQ ID NO: 48329 - DNA, 28 bp, synthetic construct
  source 1..28: mol_type = other DNA
gttccgagtctcgtacaagcagtggagg

SEQ ID NO: 48330 - DNA, 28 bp, synthetic construct
  source 1..28: mol_type = other DNA
ttccgagtctcgtacaagcagtggaggg

SEQ ID NO: 48331 - DNA, 28 bp, synthetic construct
  source 1..28: mol_type = other DNA
gtccctccactgcttgtacgagactcgg

SEQ ID NO: 48332 - DNA, 28 bp, synthetic construct
  source 1..28: mol_type = other DNA
agcagtggagggactccagagagtgtgg

SEQ ID NO: 48333 - DNA, 28 bp, synthetic construct
  source 1..28: mol_type = other DNA
cagctgctgctgcagccacactctctgg

SEQ ID NO: 48334 - DNA, 28 bp, synthetic construct
  source 1..28: mol_type = other DNA
agagtgtggctgcagcagcagctgcagg

SEQ ID NO: 48335 - DNA, 28 bp, synthetic construct
  source 1..28: mol_type = other DNA
gagtgtggctgcagcagcagctgcaggg

SEQ ID NO: 48336 - DNA, 28 bp, synthetic construct
  source 1..28: mol_type = other DNA
gtggctgcagcagcagctgcagggacgg

SEQ ID NO: 48337 - DNA, 28 bp, synthetic construct
  source 1..28: mol_type = other DNA
tggctgcagcagcagctgcagggacggg

SEQ ID NO: 48338 - DNA, 28 bp, synthetic construct
  source 1..28: mol_type = other DNA
ctgcagggacgggacccactgcatcagg

SEQ ID NO: 48339 - DNA, 28 bp, synthetic construct
  source 1..28: mol_type = other DNA
tctcaggggaggaacctgatgcagtggg

SEQ ID NO: 48340 - DNA, 28 bp, synthetic construct
  source 1..28: mol_type = other DNA
gtctcaggggaggaacctgatgcagtgg

SEQ ID NO: 48341 - DNA, 28 bp, synthetic construct
  source 1..28: mol_type = other DNA
catcaggttcctcccctgagacagccgg

SEQ ID NO: 48342 - DNA, 28 bp, synthetic construct
  source 1..28: mol_type = other DNA
ctttcactgccggctgtctcaggggagg

SEQ ID NO: 48343 - DNA, 28 bp, synthetic construct
  source 1..28: mol_type = other DNA
catctttcactgccggctgtctcagggg

SEQ ID NO: 48344 - DNA, 28 bp, synthetic construct
  source 1..28: mol_type = other DNA
acatctttcactgccggctgtctcaggg

SEQ ID NO: 48345 - DNA, 28 bp, synthetic construct
  source 1..28: mol_type = other DNA
aacatctttcactgccggctgtctcagg

SEQ ID NO: 48346 - DNA, 28 bp, synthetic construct
  source 1..28: mol_type = other DNA
agagatggagaacatctttcactgccgg

SEQ ID NO: 48347 - DNA, 28 bp, synthetic construct
  source 1..28: mol_type = other DNA
ttaagtgatgagggggagagagagatgg

SEQ ID NO: 48348 - DNA, 28 bp, synthetic construct
  source 1..28: mol_type = other DNA
ctctctctccccctcatcacttaacagg

SEQ ID NO: 48349 - DNA, 28 bp, synthetic construct
  source 1..28: mol_type = other DNA
ctattgggcctgttaagtgatgaggggg

SEQ ID NO: 48350 - DNA, 28 bp, synthetic construct
  source 1..28: mol_type = other DNA
cccctcatcacttaacaggcccaatagg

SEQ ID NO: 48351 - DNA, 28 bp, synthetic construct
  source 1..28: mol_type = other DNA
tcctattgggcctgttaagtgatgaggg

SEQ ID NO: 48352 - DNA, 28 bp, synthetic construct
  source 1..28: mol_type = other DNA
ttcctattgggcctgttaagtgatgagg

SEQ ID NO: 48353 - DNA, 28 bp, synthetic construct
  source 1..28: mol_type = other DNA
cttaacaggcccaataggaaacgtgtgg

SEQ ID NO: 48354 - DNA, 28 bp, synthetic construct
  source 1..28: mol_type = other DNA
gggcatcaaccacacgtttcctattggg

SEQ ID NO: 48355 - DNA, 28 bp, synthetic construct
  source 1..28: mol_type = other DNA
ggggcatcaaccacacgtttcctattgg

SEQ ID NO: 48356 - DNA, 28 bp, synthetic construct
  source 1..28: mol_type = other DNA
gaaacgtgtggttgatgccccaaacagg

SEQ ID NO: 48357 - DNA, 28 bp, synthetic construct
  source 1..28: mol_type = other DNA
gcatatggaatacatggcctgtttgggg

SEQ ID NO: 48358 - DNA, 28 bp, synthetic construct
  source 1..28: mol_type = other DNA
agcatatggaatacatggcctgtttggg

SEQ ID NO: 48359 - DNA, 28 bp, synthetic construct
  source 1..28: mol_type = other DNA
aagcatatggaatacatggcctgtttgg

SEQ ID NO: 48360 - DNA, 28 bp, synthetic construct
  source 1..28: mol_type = other DNA
agacgctagaagcatatggaatacatgg

SEQ ID NO: 48361 - DNA, 28 bp, synthetic construct
  source 1..28: mol_type = other DNA
atttggaaaagacgctagaagcatatgg

SEQ ID NO: 48362 - DNA, 28 bp, synthetic construct
  source 1..28: mol_type = other DNA
aaacattctaattgcatcatagatttgg

SEQ ID NO: 48363 - DNA, 28 bp, synthetic construct
  source 1..28: mol_type = other DNA
atgtcttggaggatgagaaggggagagg

SEQ ID NO: 48364 - DNA, 28 bp, synthetic construct
  source 1..28: mol_type = other DNA
ctccccttctcatcctccaagacatagg

SEQ ID NO: 48365 - DNA, 28 bp, synthetic construct
  source 1..28: mol_type = other DNA
gtcctatgtcttggaggatgagaagggg

SEQ ID NO: 48366 - DNA, 28 bp, synthetic construct
  source 1..28: mol_type = other DNA
tgtcctatgtcttggaggatgagaaggg

SEQ ID NO: 48367 - DNA, 28 bp, synthetic construct
  source 1..28: mol_type = other DNA
atgtcctatgtcttggaggatgagaagg

SEQ ID NO: 48368 - DNA, 28 bp, synthetic construct
  source 1..28: mol_type = other DNA
tttgcagcaatgtcctatgtcttggagg

SEQ ID NO: 48369 - DNA, 28 bp, synthetic construct
  source 1..28: mol_type = other DNA
ttctttgcagcaatgtcctatgtcttgg

SEQ ID NO: 48370 - DNA, 28 bp, synthetic construct
  source 1..28: mol_type = other DNA
ataggacattgctgcaaagaactcttgg

SEQ ID NO: 48371 - DNA, 28 bp, synthetic construct
  source 1..28: mol_type = other DNA
tgctgcaaagaactcttggaaacagagg

SEQ ID NO: 48372 - DNA, 28 bp, synthetic construct
  source 1..28: mol_type = other DNA
agaggtgaatgaagctgtagctcagagg

SEQ ID NO: 48373 - DNA, 28 bp, synthetic construct
  source 1..28: mol_type = other DNA
gaggtgaatgaagctgtagctcagaggg

SEQ ID NO: 48374 - DNA, 28 bp, synthetic construct
  source 1..28: mol_type = other DNA
tgaatgaagctgtagctcagagggatgg

SEQ ID NO: 48375 - DNA, 28 bp, synthetic construct
  source 1..28: mol_type = other DNA
gaatgaagctgtagctcagagggatggg

SEQ ID NO: 48376 - DNA, 28 bp, synthetic construct
  source 1..28: mol_type = other DNA
aatgaagctgtagctcagagggatgggg

SEQ ID NO: 48377 - DNA, 28 bp, synthetic construct
  source 1..28: mol_type = other DNA
tcttgaagaatacccatcttcaagaagg

SEQ ID NO: 48378 - DNA, 28 bp, synthetic construct
  source 1..28: mol_type = other DNA
tgaagaatacccatcttcaagaaggtgg

SEQ ID NO: 48379 - DNA, 28 bp, synthetic construct
  source 1..28: mol_type = other DNA
ccatcatctccaccttcttgaagatggg

SEQ ID NO: 48380 - DNA, 28 bp, synthetic construct
  source 1..28: mol_type = other DNA
gccatcatctccaccttcttgaagatgg

SEQ ID NO: 48381 - DNA, 28 bp, synthetic construct
  source 1..28: mol_type = other DNA
ggccccatctaacccatgcttcctgagg

SEQ ID NO: 48382 - DNA, 28 bp, synthetic construct
  source 1..28: mol_type = other DNA
gacctcaggaagcatgggttagatgggg

SEQ ID NO: 48383 - DNA, 28 bp, synthetic construct
  source 1..28: mol_type = other DNA
tgacctcaggaagcatgggttagatggg

SEQ ID NO: 48384 - DNA, 28 bp, synthetic construct
  source 1..28: mol_type = other DNA
atgacctcaggaagcatgggttagatgg

SEQ ID NO: 48385 - DNA, 28 bp, synthetic construct
  source 1..28: mol_type = other DNA
ctaacccatgcttcctgaggtcatctgg

SEQ ID NO: 48386 - DNA, 28 bp, synthetic construct
  source 1..28: mol_type = other DNA
cagtccagatgacctcaggaagcatggg

SEQ ID NO: 48387 - DNA, 28 bp, synthetic construct
  source 1..28: mol_type = other DNA
tcagtccagatgacctcaggaagcatgg

SEQ ID NO: 48388 - DNA, 28 bp, synthetic construct
  source 1..28: mol_type = other DNA
cttcctgaggtcatctggactgaaaagg

SEQ ID NO: 48389 - DNA, 28 bp, synthetic construct
  source 1..28: mol_type = other DNA
ttcctgaggtcatctggactgaaaaggg

SEQ ID NO: 48390 - DNA, 28 bp, synthetic construct
  source 1..28: mol_type = other DNA
gacccttttcagtccagatgacctcagg

SEQ ID NO: 48391 - DNA, 28 bp, synthetic construct
  source 1..28: mol_type = other DNA
ctgctctctggctgctgagggcatctgg

SEQ ID NO: 48392 - DNA, 28 bp, synthetic construct
  source 1..28: mol_type = other DNA
gatgccctcagcagccagagagcagagg

SEQ ID NO: 48393 - DNA, 28 bp, synthetic construct
  source 1..28: mol_type = other DNA
gagacctctgctctctggctgctgaggg

SEQ ID NO: 48394 - DNA, 28 bp, synthetic construct
  source 1..28: mol_type = other DNA
agagacctctgctctctggctgctgagg

SEQ ID NO: 48395 - DNA, 28 bp, synthetic construct
  source 1..28: mol_type = other DNA
agccagagagcagaggtctctgagctgg

SEQ ID NO: 48396 - DNA, 28 bp, synthetic construct
  source 1..28: mol_type = other DNA
gccagagagcagaggtctctgagctggg

SEQ ID NO: 48397 - DNA, 28 bp, synthetic construct
  source 1..28: mol_type = other DNA
ccccagctcagagacctctgctctctgg

SEQ ID NO: 48398 - DNA, 28 bp, synthetic construct
  source 1..28: mol_type = other DNA
agaggtctctgagctggggtcccaatgg

SEQ ID NO: 48399 - DNA, 28 bp, synthetic construct
  source 1..28: mol_type = other DNA
gagctggggtcccaatggctgagcttgg

SEQ ID NO: 48400 - DNA, 28 bp, synthetic construct
  source 1..28: mol_type = other DNA
tcccaatggctgagcttggagagcctgg

SEQ ID NO: 48401 - DNA, 28 bp, synthetic construct
  source 1..28: mol_type = other DNA
cccaatggctgagcttggagagcctggg

SEQ ID NO: 48402 - DNA, 28 bp, synthetic construct
  source 1..28: mol_type = other DNA
gcccaggctctccaagctcagccattgg

SEQ ID NO: 48403 - DNA, 28 bp, synthetic construct
  source 1..28: mol_type = other DNA
tggctgagcttggagagcctgggcaagg

SEQ ID NO: 48404 - DNA, 28 bp, synthetic construct
  source 1..28: mol_type = other DNA
agcctgggcaaggtaatgtagacagagg

SEQ ID NO: 48405 - DNA, 28 bp, synthetic construct
  source 1..28: mol_type = other DNA
gcctgggcaaggtaatgtagacagaggg

SEQ ID NO: 48406 - DNA, 28 bp, synthetic construct
  source 1..28: mol_type = other DNA
accctctgtctacattaccttgcccagg

SEQ ID NO: 48407 - DNA, 28 bp, synthetic construct
  source 1..28: mol_type = other DNA
gcaaggtaatgtagacagagggttgtgg

SEQ ID NO: 48408 - DNA, 28 bp, synthetic construct
  source 1..28: mol_type = other DNA
aggtaatgtagacagagggttgtggtgg

SEQ ID NO: 48409 - DNA, 28 bp, synthetic construct
  source 1..28: mol_type = other DNA
tgtagacagagggttgtggtggtcttgg

SEQ ID NO: 48410 - DNA, 28 bp, synthetic construct
  source 1..28: mol_type = other DNA
ttccttccgcttcatctgctgcatcagg

SEQ ID NO: 48411 - DNA, 28 bp, synthetic construct
  source 1..28: mol_type = other DNA
tgcctgatgcagcagatgaagcggaagg

SEQ ID NO: 48412 - DNA, 28 bp, synthetic construct
  source 1..28: mol_type = other DNA
cacttgcctgatgcagcagatgaagcgg

SEQ ID NO: 48413 - DNA, 28 bp, synthetic construct
  source 1..28: mol_type = other DNA
ttcatctgctgcatcaggcaagtgcagg

SEQ ID NO: 48414 - DNA, 28 bp, synthetic construct
  source 1..28: mol_type = other DNA
tgcatcaggcaagtgcaggccagccagg

SEQ ID NO: 48415 - DNA, 28 bp, synthetic construct
  source 1..28: mol_type = other DNA
caagtgcaggccagccaggacacccagg

SEQ ID NO: 48416 - DNA, 28 bp, synthetic construct
  source 1..28: mol_type = other DNA
aagtgcaggccagccaggacacccaggg

SEQ ID NO: 48417 - DNA, 28 bp, synthetic construct
  source 1..28: mol_type = other DNA
tgtcttgtgccctgggtgtcctggctgg

SEQ ID NO: 48418 - DNA, 28 bp, synthetic construct
  source 1..28: mol_type = other DNA
cctgtgtcttgtgccctgggtgtcctgg

SEQ ID NO: 48419 - DNA, 28 bp, synthetic construct
  source 1..28: mol_type = other DNA
caggacacccagggcacaagacacaggg

SEQ ID NO: 48420 - DNA, 28 bp, synthetic construct
  source 1..28: mol_type = other DNA
ctctgggccctgtgtcttgtgccctggg

SEQ ID NO: 48421 - DNA, 28 bp, synthetic construct
  source 1..28: mol_type = other DNA
gctctgggccctgtgtcttgtgccctgg

SEQ ID NO: 48422 - DNA, 28 bp, synthetic construct
  source 1..28: mol_type = other DNA
ttggtcaaatcaaacaaagagctctggg

SEQ ID NO: 48423 - DNA, 28 bp, synthetic construct
  source 1..28: mol_type = other DNA
gttggtcaaatcaaacaaagagctctgg

SEQ ID NO: 48424 - DNA, 28 bp, synthetic construct
  source 1..28: mol_type = other DNA
tctttgtttgatttgaccaacctaaagg

SEQ ID NO: 48425 - DNA, 28 bp, synthetic construct
  source 1..28: mol_type = other DNA
aggcaagcaattagagcctttaggttgg

SEQ ID NO: 48426 - DNA, 28 bp, synthetic construct
  source 1..28: mol_type = other DNA
tgaaaggcaagcaattagagcctttagg

SEQ ID NO: 48427 - DNA, 28 bp, synthetic construct
  source 1..28: mol_type = other DNA
tttctacagatatttcacagatgaaagg

SEQ ID NO: 48428 - DNA, 28 bp, synthetic construct
  source 1..28: mol_type = other DNA
tatctgtagaaatattccttcctgctgg

SEQ ID NO: 48429 - DNA, 28 bp, synthetic construct
  source 1..28: mol_type = other DNA
ctggggttctctgagtccagcaggaagg

SEQ ID NO: 48430 - DNA, 28 bp, synthetic construct
  source 1..28: mol_type = other DNA
cttcctgctggactcagagaaccccagg

SEQ ID NO: 48431 - DNA, 28 bp, synthetic construct
  source 1..28: mol_type = other DNA
ggtcctggggttctctgagtccagcagg

SEQ ID NO: 48432 - DNA, 28 bp, synthetic construct
  source 1..28: mol_type = other DNA
gcaggcacgttgggtagaggtcctgggg

SEQ ID NO: 48433 - DNA, 28 bp, synthetic construct
  source 1..28: mol_type = other DNA
agcaggcacgttgggtagaggtcctggg

SEQ ID NO: 48434 - DNA, 28 bp, synthetic construct
  source 1..28: mol_type = other DNA
gagcaggcacgttgggtagaggtcctgg

SEQ ID NO: 48435 - DNA, 28 bp, synthetic construct
  source 1..28: mol_type = other DNA
tctttggagcaggcacgttgggtagagg

SEQ ID NO: 48436 - DNA, 28 bp, synthetic construct
  source 1..28: mol_type = other DNA
ctacccaacgtgcctgctccaaagaagg

SEQ ID NO: 48437 - DNA, 28 bp, synthetic construct
  source 1..28: mol_type = other DNA
attccttctttggagcaggcacgttggg

SEQ ID NO: 48438 - DNA, 28 bp, synthetic construct
  source 1..28: mol_type = other DNA
cattccttctttggagcaggcacgttgg

SEQ ID NO: 48439 - DNA, 28 bp, synthetic construct
  source 1..28: mol_type = other DNA
acgtgcctgctccaaagaaggaatgagg

SEQ ID NO: 48440 - DNA, 28 bp, synthetic construct
  source 1..28: mol_type = other DNA
cagaacctcattccttctttggagcagg

SEQ ID NO: 48441 - DNA, 28 bp, synthetic construct
  source 1..28: mol_type = other DNA
gctctgcagaacctcattccttctttgg

SEQ ID NO: 48442 - DNA, 28 bp, synthetic construct
  source 1..28: mol_type = other DNA
gaaggaatgaggttctgcagagctgtgg

SEQ ID NO: 48443 - DNA, 28 bp, synthetic construct
  source 1..28: mol_type = other DNA
cagagctgtggtccgagccgtgatcagg

SEQ ID NO: 48444 - DNA, 28 bp, synthetic construct
  source 1..28: mol_type = other DNA
gctgtggtccgagccgtgatcaggaagg

SEQ ID NO: 48445 - DNA, 28 bp, synthetic construct
  source 1..28: mol_type = other DNA
cgaggcatccttcctgatcacggctcgg

SEQ ID NO: 48446 - DNA, 28 bp, synthetic construct
  source 1..28: mol_type = other DNA
cgagccgtgatcaggaaggatgcctcgg

SEQ ID NO: 48447 - DNA, 28 bp, synthetic construct
  source 1..28: mol_type = other DNA
gagccgtgatcaggaaggatgcctcggg

SEQ ID NO: 48448 - DNA, 28 bp, synthetic construct
  source 1..28: mol_type = other DNA
cttcccgaggcatccttcctgatcacgg

SEQ ID NO: 48449 - DNA, 28 bp, synthetic construct
  source 1..28: mol_type = other DNA
ttgctggggaaaactatacttcccgagg

SEQ ID NO: 48450 - DNA, 28 bp, synthetic construct
  source 1..28: mol_type = other DNA
ggatgcactgctgggcagtttgctgggg

SEQ ID NO: 48451 - DNA, 28 bp, synthetic construct
  source 1..28: mol_type = other DNA
cggatgcactgctgggcagtttgctggg

SEQ ID NO: 48452 - DNA, 28 bp, synthetic construct
  source 1..28: mol_type = other DNA
gcggatgcactgctgggcagtttgctgg

SEQ ID NO: 48453 - DNA, 28 bp, synthetic construct
  source 1..28: mol_type = other DNA
gcaaactgcccagcagtgcatccgccgg

SEQ ID NO: 48454 - DNA, 28 bp, synthetic construct
  source 1..28: mol_type = other DNA
tgcccagcagtgcatccgccggctgtgg

SEQ ID NO: 48455 - DNA, 28 bp, synthetic construct
  source 1..28: mol_type = other DNA
agccacagccggcggatgcactgctggg

SEQ ID NO: 48456 - DNA, 28 bp, synthetic construct
  source 1..28: mol_type = other DNA
cagccacagccggcggatgcactgctgg

SEQ ID NO: 48457 - DNA, 28 bp, synthetic construct
  source 1..28: mol_type = other DNA
cagcagtgcatccgccggctgtggctgg

SEQ ID NO: 48458 - DNA, 28 bp, synthetic construct
  source 1..28: mol_type = other DNA
ctgcactggagccagccacagccggcgg

SEQ ID NO: 48459 - DNA, 28 bp, synthetic construct
  source 1..28: mol_type = other DNA
tgtctgcactggagccagccacagccgg

SEQ ID NO: 48460 - DNA, 28 bp, synthetic construct
  source 1..28: mol_type = other DNA
tccagtgcagacagagctcagaactcgg

SEQ ID NO: 48461 - DNA, 28 bp, synthetic construct
  source 1..28: mol_type = other DNA
gccgagttctgagctctgtctgcactgg

SEQ ID NO: 48462 - DNA, 28 bp, synthetic construct
  source 1..28: mol_type = other DNA
aactcggctcctgcaagacccatcctgg

SEQ ID NO: 48463 - DNA, 28 bp, synthetic construct
  source 1..28: mol_type = other DNA
gtagatgagccaggatgggtcttgcagg

SEQ ID NO: 48464 - DNA, 28 bp, synthetic construct
  source 1..28: mol_type = other DNA
ctcgatggtgtagatgagccaggatggg

SEQ ID NO: 48465 - DNA, 28 bp, synthetic construct
  source 1..28: mol_type = other DNA
cctcgatggtgtagatgagccaggatgg

SEQ ID NO: 48466 - DNA, 28 bp, synthetic construct
  source 1..28: mol_type = other DNA
tcatcctcgatggtgtagatgagccagg

SEQ ID NO: 48467 - DNA, 28 bp, synthetic construct
  source 1..28: mol_type = other DNA
cagagcggctgctcttcatcctcgatgg

SEQ ID NO: 48468 - DNA, 28 bp, synthetic construct
  source 1..28: mol_type = other DNA
catcgaggatgaagagcagccgctctgg

SEQ ID NO: 48469 - DNA, 28 bp, synthetic construct
  source 1..28: mol_type = other DNA
gaagagcagccgctctggcctagacagg

SEQ ID NO: 48470 - DNA, 28 bp, synthetic construct
  source 1..28: mol_type = other DNA
tagacagatcctgtctaggccagagcgg

SEQ ID NO: 48471 - DNA, 28 bp, synthetic construct
  source 1..28: mol_type = other DNA
tctggcctagacaggatctgtctaatgg

SEQ ID NO: 48472 - DNA, 28 bp, synthetic construct
  source 1..28: mol_type = other DNA
ctggcctagacaggatctgtctaatggg

SEQ ID NO: 48473 - DNA, 28 bp, synthetic construct
  source 1..28: mol_type = other DNA
ggctcccattagacagatcctgtctagg

SEQ ID NO: 48474 - DNA, 28 bp, synthetic construct
  source 1..28: mol_type = other DNA
tagacaggatctgtctaatgggagccgg

SEQ ID NO: 48475 - DNA, 28 bp, synthetic construct
  source 1..28: mol_type = other DNA
aggatctgtctaatgggagccggagtgg

SEQ ID NO: 48476 - DNA, 28 bp, synthetic construct
  source 1..28: mol_type = other DNA
atcggaaaagatgggacagccactccgg

SEQ ID NO: 48477 - DNA, 28 bp, synthetic construct
  source 1..28: mol_type = other DNA
tctcgctgagctcatcggaaaagatggg

SEQ ID NO: 48478 - DNA, 28 bp, synthetic construct
  source 1..28: mol_type = other DNA
gtctcgctgagctcatcggaaaagatgg

SEQ ID NO: 48479 - DNA, 28 bp, synthetic construct
  source 1..28: mol_type = other DNA
aggtggtgagtctcgctgagctcatcgg

SEQ ID NO: 48480 - DNA, 28 bp, synthetic construct
  source 1..28: mol_type = other DNA
atgagctcagcgagactcaccaccttgg

SEQ ID NO: 48481 - DNA, 28 bp, synthetic construct
  source 1..28: mol_type = other DNA
ctcagcgagactcaccaccttggactgg

SEQ ID NO: 48482 - DNA, 28 bp, synthetic construct
  source 1..28: mol_type = other DNA
tcagcgagactcaccaccttggactggg

SEQ ID NO: 48483 - DNA, 28 bp, synthetic construct
  source 1..28: mol_type = other DNA
tgcagagagctggcccagtccaaggtgg

SEQ ID NO: 48484 - DNA, 28 bp, synthetic construct
  source 1..28: mol_type = other DNA
agctgcagagagctggcccagtccaagg

SEQ ID NO: 48485 - DNA, 28 bp, synthetic construct
  source 1..28: mol_type = other DNA
gtcttctacttcagctgcagagagctgg

SEQ ID NO: 48486 - DNA, 28 bp, synthetic construct
  source 1..28: mol_type = other DNA
tctgcagctgaagtagaagacatgctgg

SEQ ID NO: 48487 - DNA, 28 bp, synthetic construct
  source 1..28: mol_type = other DNA
gctgaagtagaagacatgctggaagcgg

SEQ ID NO: 48488 - DNA, 28 bp, synthetic construct
  source 1..28: mol_type = other DNA
atgctggaagcggtccccatacagctgg

SEQ ID NO: 48489 - DNA, 28 bp, synthetic construct
  source 1..28: mol_type = other DNA
tccccatacagctggcctctcccccagg

SEQ ID NO: 48490 - DNA, 28 bp, synthetic construct
  source 1..28: mol_type = other DNA
gcctgggggagaggccagctgtatgggg

SEQ ID NO: 48491 - DNA, 28 bp, synthetic construct
  source 1..28: mol_type = other DNA
agcctgggggagaggccagctgtatggg

SEQ ID NO: 48492 - DNA, 28 bp, synthetic construct
  source 1..28: mol_type = other DNA
aagcctgggggagaggccagctgtatgg

SEQ ID NO: 48493 - DNA, 28 bp, synthetic construct
  source 1..28: mol_type = other DNA
ggcaggtgaaggaagcctgggggagagg

SEQ ID NO: 48494 - DNA, 28 bp, synthetic construct
  source 1..28: mol_type = other DNA
ctcccccaggcttccttcacctgcctgg

SEQ ID NO: 48495 - DNA, 28 bp, synthetic construct
  source 1..28: mol_type = other DNA
ggccaggcaggtgaaggaagcctggggg

SEQ ID NO: 48496 - DNA, 28 bp, synthetic construct
  source 1..28: mol_type = other DNA
tggccaggcaggtgaaggaagcctgggg

SEQ ID NO: 48497 - DNA, 28 bp, synthetic construct
  source 1..28: mol_type = other DNA
ctggccaggcaggtgaaggaagcctggg

SEQ ID NO: 48498 - DNA, 28 bp, synthetic construct
  source 1..28: mol_type = other DNA
actggccaggcaggtgaaggaagcctgg

SEQ ID NO: 48499 - DNA, 28 bp, synthetic construct
  source 1..28: mol_type = other DNA
aagtcaacactggccaggcaggtgaagg

SEQ ID NO: 48500 - DNA, 28 bp, synthetic construct
  source 1..28: mol_type = other DNA
attgggaagtcaacactggccaggcagg

SEQ ID NO: 48501 - DNA, 28 bp, synthetic construct
  source 1..28: mol_type = other DNA
tggaattgggaagtcaacactggccagg

SEQ ID NO: 48502 - DNA, 28 bp, synthetic construct
  source 1..28: mol_type = other DNA
gctgctggaattgggaagtcaacactgg

SEQ ID NO: 48503 - DNA, 28 bp, synthetic construct
  source 1..28: mol_type = other DNA
catactgcagggggctgctggaattggg

SEQ ID NO: 48504 - DNA, 28 bp, synthetic construct
  source 1..28: mol_type = other DNA
tcatactgcagggggctgctggaattgg

SEQ ID NO: 48505 - DNA, 28 bp, synthetic construct
  source 1..28: mol_type = other DNA
gcatagtcatactgcagggggctgctgg

SEQ ID NO: 48506 - DNA, 28 bp, synthetic construct
  source 1..28: mol_type = other DNA
cagccccctgcagtatgactatgcgagg

SEQ ID NO: 48507 - DNA, 28 bp, synthetic construct
  source 1..28: mol_type = other DNA
gaacctcgcatagtcatactgcaggggg

SEQ ID NO: 48508 - DNA, 28 bp, synthetic construct
  source 1..28: mol_type = other DNA
agaacctcgcatagtcatactgcagggg

SEQ ID NO: 48509 - DNA, 28 bp, synthetic construct
  source 1..28: mol_type = other DNA
aagaacctcgcatagtcatactgcaggg

SEQ ID NO: 48510 - DNA, 28 bp, synthetic construct
  source 1..28: mol_type = other DNA
caagaacctcgcatagtcatactgcagg

SEQ ID NO: 48511 - DNA, 28 bp, synthetic construct
  source 1..28: mol_type = other DNA
ctgcagtatgactatgcgaggttcttgg

SEQ ID NO: 48512 - DNA, 28 bp, synthetic construct
  source 1..28: mol_type = other DNA
tgcagtatgactatgcgaggttcttggg

SEQ ID NO: 48513 - DNA, 28 bp, synthetic construct
  source 1..28: mol_type = other DNA
gactatgcgaggttcttgggtatccagg

SEQ ID NO: 48514 - DNA, 28 bp, synthetic construct
  source 1..28: mol_type = other DNA
tgcgaggttcttgggtatccaggcctgg

SEQ ID NO: 48515 - DNA, 28 bp, synthetic construct
  source 1..28: mol_type = other DNA
gcgaggttcttgggtatccaggcctggg

SEQ ID NO: 48516 - DNA, 28 bp, synthetic construct
  source 1..28: mol_type = other DNA
atcagagacttatttggcccaggcctgg

SEQ ID NO: 48517 - DNA, 28 bp, synthetic construct
  source 1..28: mol_type = other DNA
ttgagatcagagacttatttggcccagg

SEQ ID NO: 48518 - DNA, 28 bp, synthetic construct
  source 1..28: mol_type = other DNA
atttaattgagatcagagacttatttgg

SEQ ID NO: 48519 - DNA, 28 bp, synthetic construct
  source 1..28: mol_type = other DNA
gtcctcgattctcctccacataatcagg

SEQ ID NO: 48520 - DNA, 28 bp, synthetic construct
  source 1..28: mol_type = other DNA
ggcctgattatgtggaggagaatcgagg

SEQ ID NO: 48521 - DNA, 28 bp, synthetic construct
  source 1..28: mol_type = other DNA
aagagaagctggcctgattatgtggagg

SEQ ID NO: 48522 - DNA, 28 bp, synthetic construct
  source 1..28: mol_type = other DNA
gtcaagagaagctggcctgattatgtgg

SEQ ID NO: 48523 - DNA, 28 bp, synthetic construct
  source 1..28: mol_type = other DNA
ataatcaggccagcttctcttgaccagg

SEQ ID NO: 48524 - DNA, 28 bp, synthetic construct
  source 1..28: mol_type = other DNA
taatcaggccagcttctcttgaccaggg

SEQ ID NO: 48525 - DNA, 28 bp, synthetic construct
  source 1..28: mol_type = other DNA
aatcaggccagcttctcttgaccagggg

SEQ ID NO: 48526 - DNA, 28 bp, synthetic construct
  source 1..28: mol_type = other DNA
ccaagatcccctggtcaagagaagctgg

SEQ ID NO: 48527 - DNA, 28 bp, synthetic construct
  source 1..28: mol_type = other DNA
ctcttgaccaggggatcttggcttctgg

SEQ ID NO: 48528 - DNA, 28 bp, synthetic construct
  source 1..28: mol_type = other DNA
tcttgaccaggggatcttggcttctggg

SEQ ID NO: 48529 - DNA, 28 bp, synthetic construct
  source 1..28: mol_type = other DNA
cttgaccaggggatcttggcttctgggg

SEQ ID NO: 48530 - DNA, 28 bp, synthetic construct
  source 1..28: mol_type = other DNA
cctcaccccagaagccaagatcccctgg

SEQ ID NO: 48531 - DNA, 28 bp, synthetic construct
  source 1..28: mol_type = other DNA
tagaagtagcagctgtgtgaatttttgg

SEQ ID NO: 48532 - DNA, 28 bp, synthetic construct
  source 1..28: mol_type = other DNA
ttttggttaaaatcctcatttttccagg

SEQ ID NO: 48533 - DNA, 28 bp, synthetic construct
  source 1..28: mol_type = other DNA
tttggttaaaatcctcatttttccaggg

SEQ ID NO: 48534 - DNA, 28 bp, synthetic construct
  source 1..28: mol_type = other DNA
aaatcctcatttttccagggccatgtgg

SEQ ID NO: 48535 - DNA, 28 bp, synthetic construct
  source 1..28: mol_type = other DNA
tgttccacatggccctggaaaaatgagg

SEQ ID NO: 48536 - DNA, 28 bp, synthetic construct
  source 1..28: mol_type = other DNA
atttttccagggccatgtggaacagagg

SEQ ID NO: 48537 - DNA, 28 bp, synthetic construct
  source 1..28: mol_type = other DNA
agagagcctctgttccacatggccctgg

SEQ ID NO: 48538 - DNA, 28 bp, synthetic construct
  source 1..28: mol_type = other DNA
tgtgagagagagcctctgttccacatgg

SEQ ID NO: 48539 - DNA, 28 bp, synthetic construct
  source 1..28: mol_type = other DNA
tggaacagaggctctctctcacagaagg

SEQ ID NO: 48540 - DNA, 28 bp, synthetic construct
  source 1..28: mol_type = other DNA
ggctctctctcacagaaggctcccatgg

SEQ ID NO: 48541 - DNA, 28 bp, synthetic construct
  source 1..28: mol_type = other DNA
gctctctctcacagaaggctcccatggg

SEQ ID NO: 48542 - DNA, 28 bp, synthetic construct
  source 1..28: mol_type = other DNA
ctctctcacagaaggctcccatgggtgg

SEQ ID NO: 48543 - DNA, 28 bp, synthetic construct
  source 1..28: mol_type = other DNA
tctcacagaaggctcccatgggtggtgg

SEQ ID NO: 48544 - DNA, 28 bp, synthetic construct
  source 1..28: mol_type = other DNA
cacagaaggctcccatgggtggtggtgg

SEQ ID NO: 48545 - DNA, 28 bp, synthetic construct
  source 1..28: mol_type = other DNA
acagaaggctcccatgggtggtggtggg

SEQ ID NO: 48546 - DNA, 28 bp, synthetic construct
  source 1..28: mol_type = other DNA
cagaaggctcccatgggtggtggtgggg

SEQ ID NO: 48547 - DNA, 28 bp, synthetic construct
  source 1..28: mol_type = other DNA
ctcccatgggtggtggtggggctgtagg

SEQ ID NO: 48548 - DNA, 28 bp, synthetic construct
  source 1..28: mol_type = other DNA
agcctacagccccaccaccacccatggg

SEQ ID NO: 48549 - DNA, 28 bp, synthetic construct
  source 1..28: mol_type = other DNA
cagcctacagccccaccaccacccatgg

SEQ ID NO: 48550 - DNA, 28 bp, synthetic construct
  source 1..28: mol_type = other DNA
catgggtggtggtggggctgtaggctgg

SEQ ID NO: 48551 - DNA, 28 bp, synthetic construct
  source 1..28: mol_type = other DNA
ggggctgtaggctggtgtgcgcctgtgg

SEQ ID NO: 48552 - DNA, 28 bp, synthetic construct
  source 1..28: mol_type = other DNA
gggctgtaggctggtgtgcgcctgtggg

SEQ ID NO: 48553 - DNA, 28 bp, synthetic construct
  source 1..28: mol_type = other DNA
ggctgtaggctggtgtgcgcctgtgggg

SEQ ID NO: 48554 - DNA, 28 bp, synthetic construct
  source 1..28: mol_type = other DNA
gctgtaggctggtgtgcgcctgtggggg

SEQ ID NO: 48555 - DNA, 28 bp, synthetic construct
  source 1..28: mol_type = other DNA
gcagcggtggtaggaacgcccccacagg

SEQ ID NO: 48556 - DNA, 28 bp, synthetic construct
  source 1..28: mol_type = other DNA
ggggcgttcctaccaccgctgcccatgg

SEQ ID NO: 48557 - DNA, 28 bp, synthetic construct
  source 1..28: mol_type = other DNA
gggcgttcctaccaccgctgcccatggg

SEQ ID NO: 48558 - DNA, 28 bp, synthetic construct
  source 1..28: mol_type = other DNA
ggcgttcctaccaccgctgcccatgggg

SEQ ID NO: 48559 - DNA, 28 bp, synthetic construct
  source 1..28: mol_type = other DNA
gcgttcctaccaccgctgcccatggggg

SEQ ID NO: 48560 - DNA, 28 bp, synthetic construct
  source 1..28: mol_type = other DNA
gcaggcccccatgggcagcggtggtagg

SEQ ID NO: 48561 - DNA, 28 bp, synthetic construct
  source 1..28: mol_type = other DNA
aaaggcaggcccccatgggcagcggtgg

SEQ ID NO: 48562 - DNA, 28 bp, synthetic construct
  source 1..28: mol_type = other DNA
gagaaaggcaggcccccatgggcagcgg

SEQ ID NO: 48563 - DNA, 28 bp, synthetic construct
  source 1..28: mol_type = other DNA
aaatcagagaaaggcaggcccccatggg

SEQ ID NO: 48564 - DNA, 28 bp, synthetic construct
  source 1..28: mol_type = other DNA
gaaatcagagaaaggcaggcccccatgg

SEQ ID NO: 48565 - DNA, 28 bp, synthetic construct
  source 1..28: mol_type = other DNA
agagagagagaaatcagagaaaggcagg

SEQ ID NO: 48566 - DNA, 28 bp, synthetic construct
  source 1..28: mol_type = other DNA
aaagagagagagagaaatcagagaaagg

SEQ ID NO: 48567 - DNA, 28 bp, synthetic construct
  source 1..28: mol_type = other DNA
tctctctttctctgatttctaagtaagg

SEQ ID NO: 48568 - DNA, 28 bp, synthetic construct
  source 1..28: mol_type = other DNA
ctctctttctctgatttctaagtaaggg

SEQ ID NO: 48569 - DNA, 28 bp, synthetic construct
  source 1..28: mol_type = other DNA
tctttctctgatttctaagtaagggagg

SEQ ID NO: 48570 - DNA, 28 bp, synthetic construct
  source 1..28: mol_type = other DNA
ctttctctgatttctaagtaagggaggg

SEQ ID NO: 48571 - DNA, 28 bp, synthetic construct
  source 1..28: mol_type = other DNA
gatttctaagtaagggagggaaagaagg

SEQ ID NO: 48572 - DNA, 28 bp, synthetic construct
  source 1..28: mol_type = other DNA
taagggagggaaagaaggaacataaagg

SEQ ID NO: 48573 - DNA, 28 bp, synthetic construct
  source 1..28: mol_type = other DNA
aattaattaattaaacaactgttttagg

SEQ ID NO: 48574 - DNA, 28 bp, synthetic construct
  source 1..28: mol_type = other DNA
gacagcgcagtgtgtggcttggagtagg

SEQ ID NO: 48575 - DNA, 28 bp, synthetic construct
  source 1..28: mol_type = other DNA
tctgcagacagcgcagtgtgtggcttgg

SEQ ID NO: 48576 - DNA, 28 bp, synthetic construct
  source 1..28: mol_type = other DNA
cagtgtctgcagacagcgcagtgtgtgg

SEQ ID NO: 48577 - DNA, 28 bp, synthetic construct
  source 1..28: mol_type = other DNA
cacacactgcgctgtctgcagacactgg

SEQ ID NO: 48578 - DNA, 28 bp, synthetic construct
  source 1..28: mol_type = other DNA
aggttggcaggctaagcagaggttctgg

SEQ ID NO: 48579 - DNA, 28 bp, synthetic construct
  source 1..28: mol_type = other DNA
agaacctctgcttagcctgccaacctgg

SEQ ID NO: 48580 - DNA, 28 bp, synthetic construct
  source 1..28: mol_type = other DNA
gggaccaggttggcaggctaagcagagg

SEQ ID NO: 48581 - DNA, 28 bp, synthetic construct
  source 1..28: mol_type = other DNA
tgcttagcctgccaacctggtccccagg

SEQ ID NO: 48582 - DNA, 28 bp, synthetic construct
  source 1..28: mol_type = other DNA
gcttagcctgccaacctggtccccaggg

SEQ ID NO: 48583 - DNA, 28 bp, synthetic construct
  source 1..28: mol_type = other DNA
cttagcctgccaacctggtccccagggg

SEQ ID NO: 48584 - DNA, 28 bp, synthetic construct
  source 1..28: mol_type = other DNA
agagtcccctggggaccaggttggcagg

SEQ ID NO: 48585 - DNA, 28 bp, synthetic construct
  source 1..28: mol_type = other DNA
acaaagagtcccctggggaccaggttgg

SEQ ID NO: 48586 - DNA, 28 bp, synthetic construct
  source 1..28: mol_type = other DNA
atggacaaagagtcccctggggaccagg

SEQ ID NO: 48587 - DNA, 28 bp, synthetic construct
  source 1..28: mol_type = other DNA
aaatgtatggacaaagagtcccctgggg

SEQ ID NO: 48588 - DNA, 28 bp, synthetic construct
  source 1..28: mol_type = other DNA
caaatgtatggacaaagagtcccctggg

SEQ ID NO: 48589 - DNA, 28 bp, synthetic construct
  source 1..28: mol_type = other DNA
gcaaatgtatggacaaagagtcccctgg

SEQ ID NO: 48590 - DNA, 28 bp, synthetic construct
  source 1..28: mol_type = other DNA
tggtgaggtgggagaggcaaatgtatgg

SEQ ID NO: 48591 - DNA, 28 bp, synthetic construct
  source 1..28: mol_type = other DNA
gcctctcccacctcaccaccccgccagg

SEQ ID NO: 48592 - DNA, 28 bp, synthetic construct
  source 1..28: mol_type = other DNA
tcctggcggggtggtgaggtgggagagg

SEQ ID NO: 48593 - DNA, 28 bp, synthetic construct
  source 1..28: mol_type = other DNA
tgagctcctggcggggtggtgaggtggg

SEQ ID NO: 48594 - DNA, 28 bp, synthetic construct
  source 1..28: mol_type = other DNA
ctgagctcctggcggggtggtgaggtgg

SEQ ID NO: 48595 - DNA, 28 bp, synthetic construct
  source 1..28: mol_type = other DNA
ctactgagctcctggcggggtggtgagg

SEQ ID NO: 48596 - DNA, 28 bp, synthetic construct
  source 1..28: mol_type = other DNA
ctcaccaccccgccaggagctcagtagg

SEQ ID NO: 48597 - DNA, 28 bp, synthetic construct
  source 1..28: mol_type = other DNA
tcaccaccccgccaggagctcagtaggg

SEQ ID NO: 48598 - DNA, 28 bp, synthetic construct
  source 1..28: mol_type = other DNA
agaccctactgagctcctggcggggtgg

SEQ ID NO: 48599 - DNA, 28 bp, synthetic construct
  source 1..28: mol_type = other DNA
gtgagaccctactgagctcctggcgggg

SEQ ID NO: 48600 - DNA, 28 bp, synthetic construct
  source 1..28: mol_type = other DNA
ggtgagaccctactgagctcctggcggg

SEQ ID NO: 48601 - DNA, 28 bp, synthetic construct
  source 1..28: mol_type = other DNA
aggtgagaccctactgagctcctggcgg

SEQ ID NO: 48602 - DNA, 28 bp, synthetic construct
  source 1..28: mol_type = other DNA
cacaggtgagaccctactgagctcctgg

SEQ ID NO: 48603 - DNA, 28 bp, synthetic construct
  source 1..28: mol_type = other DNA
atgaaacgtcaggaatttactacacagg

SEQ ID NO: 48604 - DNA, 28 bp, synthetic construct
  source 1..28: mol_type = other DNA
agtaaattcctgacgtttcatccagagg

SEQ ID NO: 48605 - DNA, 28 bp, synthetic construct
  source 1..28: mol_type = other DNA
tcctgacgtttcatccagaggccattgg

SEQ ID NO: 48606 - DNA, 28 bp, synthetic construct
  source 1..28: mol_type = other DNA
cccaatggcctctggatgaaacgtcagg

SEQ ID NO: 48607 - DNA, 28 bp, synthetic construct
  source 1..28: mol_type = other DNA
tttcatccagaggccattgggtcccagg

SEQ ID NO: 48608 - DNA, 28 bp, synthetic construct
  source 1..28: mol_type = other DNA
gaggctcctgggacccaatggcctctgg

SEQ ID NO: 48609 - DNA, 28 bp, synthetic construct
  source 1..28: mol_type = other DNA
agagcaggaggctcctgggacccaatgg

SEQ ID NO: 48610 - DNA, 28 bp, synthetic construct
  source 1..28: mol_type = other DNA
tgggtcccaggagcctcctgctctctgg

SEQ ID NO: 48611 - DNA, 28 bp, synthetic construct
  source 1..28: mol_type = other DNA
gggtcccaggagcctcctgctctctggg

SEQ ID NO: 48612 - DNA, 28 bp, synthetic construct
  source 1..28: mol_type = other DNA
agcacccagagagcaggaggctcctggg

SEQ ID NO: 48613 - DNA, 28 bp, synthetic construct
  source 1..28: mol_type = other DNA
tagcacccagagagcaggaggctcctgg

SEQ ID NO: 48614 - DNA, 28 bp, synthetic construct
  source 1..28: mol_type = other DNA
aggagcctcctgctctctgggtgctagg

SEQ ID NO: 48615 - DNA, 28 bp, synthetic construct
  source 1..28: mol_type = other DNA
gcctcctgctctctgggtgctaggctgg

SEQ ID NO: 48616 - DNA, 28 bp, synthetic construct
  source 1..28: mol_type = other DNA
cccagcctagcacccagagagcaggagg

SEQ ID NO: 48617 - DNA, 28 bp, synthetic construct
  source 1..28: mol_type = other DNA
cagcccagcctagcacccagagagcagg

SEQ ID NO: 48618 - DNA, 28 bp, synthetic construct
  source 1..28: mol_type = other DNA
gctctctgggtgctaggctgggctgagg

SEQ ID NO: 48619 - DNA, 28 bp, synthetic construct
  source 1..28: mol_type = other DNA
ctctgggtgctaggctgggctgaggtgg

SEQ ID NO: 48620 - DNA, 28 bp, synthetic construct
  source 1..28: mol_type = other DNA
tctgggtgctaggctgggctgaggtggg

SEQ ID NO: 48621 - DNA, 28 bp, synthetic construct
  source 1..28: mol_type = other DNA
ctgggtgctaggctgggctgaggtgggg

SEQ ID NO: 48622 - DNA, 28 bp, synthetic construct
  source 1..28: mol_type = other DNA
gatccccagctccccagcactgctgtgg

SEQ ID NO: 48623 - DNA, 28 bp, synthetic construct
  source 1..28: mol_type = other DNA
catccacagcagtgctggggagctgggg

SEQ ID NO: 48624 - DNA, 28 bp, synthetic construct
  source 1..28: mol_type = other DNA
acatccacagcagtgctggggagctggg

SEQ ID NO: 48625 - DNA, 28 bp, synthetic construct
  source 1..28: mol_type = other DNA
cacatccacagcagtgctggggagctgg

SEQ ID NO: 48626 - DNA, 28 bp, synthetic construct
  source 1..28: mol_type = other DNA
cagctccccagcactgctgtggatgtgg

SEQ ID NO: 48627 - DNA, 28 bp, synthetic construct
  source 1..28: mol_type = other DNA
agctccccagcactgctgtggatgtggg

SEQ ID NO: 48628 - DNA, 28 bp, synthetic construct
  source 1..28: mol_type = other DNA
gctccccagcactgctgtggatgtgggg

SEQ ID NO: 48629 - DNA, 28 bp, synthetic construct
  source 1..28: mol_type = other DNA
ctccccagcactgctgtggatgtggggg

SEQ ID NO: 48630 - DNA, 28 bp, synthetic construct
  source 1..28: mol_type = other DNA
cgcccccacatccacagcagtgctgggg

SEQ ID NO: 48631 - DNA, 28 bp, synthetic construct
  source 1..28: mol_type = other DNA
acgcccccacatccacagcagtgctggg

SEQ ID NO: 48632 - DNA, 28 bp, synthetic construct
  source 1..28: mol_type = other DNA
aacgcccccacatccacagcagtgctgg

SEQ ID NO: 48633 - DNA, 28 bp, synthetic construct
  source 1..28: mol_type = other DNA
agcactgctgtggatgtgggggcgttgg

SEQ ID NO: 48634 - DNA, 28 bp, synthetic construct
  source 1..28: mol_type = other DNA
gcactgctgtggatgtgggggcgttggg

SEQ ID NO: 48635 - DNA, 28 bp, synthetic construct
  source 1..28: mol_type = other DNA
ggatgtgggggcgttgggtgactcctgg

SEQ ID NO: 48636 - DNA, 28 bp, synthetic construct
  source 1..28: mol_type = other DNA
tgggggcgttgggtgactcctggcttgg

SEQ ID NO: 48637 - DNA, 28 bp, synthetic construct
  source 1..28: mol_type = other DNA
gggtgactcctggcttggagactcatgg

SEQ ID NO: 48638 - DNA, 28 bp, synthetic construct
  source 1..28: mol_type = other DNA
actcctggcttggagactcatggtctgg

SEQ ID NO: 48639 - DNA, 28 bp, synthetic construct
  source 1..28: mol_type = other DNA
ctcctggcttggagactcatggtctggg

SEQ ID NO: 48640 - DNA, 28 bp, synthetic construct
  source 1..28: mol_type = other DNA
tcctggcttggagactcatggtctgggg

SEQ ID NO: 48641 - DNA, 28 bp, synthetic construct
  source 1..28: mol_type = other DNA
tccccagaccatgagtctccaagccagg

SEQ ID NO: 48642 - DNA, 28 bp, synthetic construct
  source 1..28: mol_type = other DNA
ttggagactcatggtctggggagcttgg

SEQ ID NO: 48643 - DNA, 28 bp, synthetic construct
  source 1..28: mol_type = other DNA
atggtctggggagcttggaagagcttgg

SEQ ID NO: 48644 - DNA, 28 bp, synthetic construct
  source 1..28: mol_type = other DNA
tggggagcttggaagagcttggtagagg

SEQ ID NO: 48645 - DNA, 28 bp, synthetic construct
  source 1..28: mol_type = other DNA
cttggaagagcttggtagaggagtgagg

SEQ ID NO: 48646 - DNA, 28 bp, synthetic construct
  source 1..28: mol_type = other DNA
ggtagaggagtgaggcagagatttctgg

SEQ ID NO: 48647 - DNA, 28 bp, synthetic construct
  source 1..28: mol_type = other DNA
gtagaggagtgaggcagagatttctggg

SEQ ID NO: 48648 - DNA, 28 bp, synthetic construct
  source 1..28: mol_type = other DNA
tagaggagtgaggcagagatttctgggg

SEQ ID NO: 48649 - DNA, 28 bp, synthetic construct
  source 1..28: mol_type = other DNA
agaggagtgaggcagagatttctggggg

SEQ ID NO: 48650 - DNA, 28 bp, synthetic construct
  source 1..28: mol_type = other DNA
gaggagtgaggcagagatttctgggggg

SEQ ID NO: 48651 - DNA, 28 bp, synthetic construct
  source 1..28: mol_type = other DNA
taaaagaaaataaatgttcagtaaatgg

SEQ ID NO: 48652 - DNA, 28 bp, synthetic construct
  source 1..28: mol_type = other DNA
atttactgaacatttattttcttttagg

SEQ ID NO: 48653 - DNA, 28 bp, synthetic construct
  source 1..28: mol_type = other DNA
aaactctcacaacagtcctgagagatgg

SEQ ID NO: 48654 - DNA, 28 bp, synthetic construct
  source 1..28: mol_type = other DNA
aactctcacaacagtcctgagagatggg

SEQ ID NO: 48655 - DNA, 28 bp, synthetic construct
  source 1..28: mol_type = other DNA
ataatattattaagacccatctctcagg

SEQ ID NO: 48656 - DNA, 28 bp, synthetic construct
  source 1..28: mol_type = other DNA
atgggggacagcagaggaaggatagggg

SEQ ID NO: 48657 - DNA, 28 bp, synthetic construct
  source 1..28: mol_type = other DNA
catgggggacagcagaggaaggataggg

SEQ ID NO: 48658 - DNA, 28 bp, synthetic construct
  source 1..28: mol_type = other DNA
acatgggggacagcagaggaaggatagg

SEQ ID NO: 48659 - DNA, 28 bp, synthetic construct
  source 1..28: mol_type = other DNA
tccttcctctgctgtcccccatgtcagg

SEQ ID NO: 48660 - DNA, 28 bp, synthetic construct
  source 1..28: mol_type = other DNA
acctgacatgggggacagcagaggaagg

SEQ ID NO: 48661 - DNA, 28 bp, synthetic construct
  source 1..28: mol_type = other DNA
ggggacctgacatgggggacagcagagg

SEQ ID NO: 48662 - DNA, 28 bp, synthetic construct
  source 1..28: mol_type = other DNA
gtctgtgcatggggacctgacatggggg

SEQ ID NO: 48663 - DNA, 28 bp, synthetic construct
  source 1..28: mol_type = other DNA
tgtctgtgcatggggacctgacatgggg

SEQ ID NO: 48664 - DNA, 28 bp, synthetic construct
  source 1..28: mol_type = other DNA
atgtctgtgcatggggacctgacatggg

SEQ ID NO: 48665 - DNA, 28 bp, synthetic construct
  source 1..28: mol_type = other DNA
catgtctgtgcatggggacctgacatgg

SEQ ID NO: 48666 - DNA, 28 bp, synthetic construct
  source 1..28: mol_type = other DNA
gtccccatgcacagacatgatcctctgg

SEQ ID NO: 48667 - DNA, 28 bp, synthetic construct
  source 1..28: mol_type = other DNA
tccccatgcacagacatgatcctctggg

SEQ ID NO: 48668 - DNA, 28 bp, synthetic construct
  source 1..28: mol_type = other DNA
acccagaggatcatgtctgtgcatgggg

SEQ ID NO: 48669 - DNA, 28 bp, synthetic construct
  source 1..28: mol_type = other DNA
cacccagaggatcatgtctgtgcatggg

SEQ ID NO: 48670 - DNA, 28 bp, synthetic construct
  source 1..28: mol_type = other DNA
ccatgcacagacatgatcctctgggtgg

SEQ ID NO: 48671 - DNA, 28 bp, synthetic construct
  source 1..28: mol_type = other DNA
catgcacagacatgatcctctgggtggg

SEQ ID NO: 48672 - DNA, 28 bp, synthetic construct
  source 1..28: mol_type = other DNA
atgcacagacatgatcctctgggtgggg

SEQ ID NO: 48673 - DNA, 28 bp, synthetic construct
  source 1..28: mol_type = other DNA
gaatcagctggtgggccccacccagagg

SEQ ID NO: 48674 - DNA, 28 bp, synthetic construct
  source 1..28: mol_type = other DNA
tgggtggagctgtgaatcagctggtggg

SEQ ID NO: 48675 - DNA, 28 bp, synthetic construct
  source 1..28: mol_type = other DNA
ctgggtggagctgtgaatcagctggtgg

SEQ ID NO: 48676 - DNA, 28 bp, synthetic construct
  source 1..28: mol_type = other DNA
caccagctgattcacagctccacccagg

SEQ ID NO: 48677 - DNA, 28 bp, synthetic construct
  source 1..28: mol_type = other DNA
accagctgattcacagctccacccaggg

SEQ ID NO: 48678 - DNA, 28 bp, synthetic construct
  source 1..28: mol_type = other DNA
gccctgggtggagctgtgaatcagctgg

SEQ ID NO: 48679 - DNA, 28 bp, synthetic construct
  source 1..28: mol_type = other DNA
gctgaggcaggctgacagccctgggtgg

SEQ ID NO: 48680 - DNA, 28 bp, synthetic construct
  source 1..28: mol_type = other DNA
cttgctgaggcaggctgacagccctggg

SEQ ID NO: 48681 - DNA, 28 bp, synthetic construct
  source 1..28: mol_type = other DNA
gcttgctgaggcaggctgacagccctgg

SEQ ID NO: 48682 - DNA, 28 bp, synthetic construct
  source 1..28: mol_type = other DNA
ctggagaggtgaggcttgctgaggcagg

SEQ ID NO: 48683 - DNA, 28 bp, synthetic construct
  source 1..28: mol_type = other DNA
gcctcagcaagcctcacctctccagcgg

SEQ ID NO: 48684 - DNA, 28 bp, synthetic construct
  source 1..28: mol_type = other DNA
gccgctggagaggtgaggcttgctgagg

SEQ ID NO: 48685 - DNA, 28 bp, synthetic construct
  source 1..28: mol_type = other DNA
acatctggacgccgctggagaggtgagg

SEQ ID NO: 48686 - DNA, 28 bp, synthetic construct
  source 1..28: mol_type = other DNA
ctgacacatctggacgccgctggagagg

SEQ ID NO: 48687 - DNA, 28 bp, synthetic construct
  source 1..28: mol_type = other DNA
ctctccagcggcgtccagatgtgtcagg

SEQ ID NO: 48688 - DNA, 28 bp, synthetic construct
  source 1..28: mol_type = other DNA
gctgcctgacacatctggacgccgctgg

SEQ ID NO: 48689 - DNA, 28 bp, synthetic construct
  source 1..28: mol_type = other DNA
ttttgagacagctgcctgacacatctgg

SEQ ID NO: 48690 - DNA, 28 bp, synthetic construct
  source 1..28: mol_type = other DNA
tctcaaaacccttctctctgagccctgg

SEQ ID NO: 48691 - DNA, 28 bp, synthetic construct
  source 1..28: mol_type = other DNA
ctcaaaacccttctctctgagccctggg

SEQ ID NO: 48692 - DNA, 28 bp, synthetic construct
  source 1..28: mol_type = other DNA
gggtgcacccagggctcagagagaaggg

SEQ ID NO: 48693 - DNA, 28 bp, synthetic construct
  source 1..28: mol_type = other DNA
ggggtgcacccagggctcagagagaagg

SEQ ID NO: 48694 - DNA, 28 bp, synthetic construct
  source 1..28: mol_type = other DNA
tctctgagccctgggtgcaccccgccgg

SEQ ID NO: 48695 - DNA, 28 bp, synthetic construct
  source 1..28: mol_type = other DNA
atgaattgccggcggggtgcacccaggg

SEQ ID NO: 48696 - DNA, 28 bp, synthetic construct
  source 1..28: mol_type = other DNA
catgaattgccggcggggtgcacccagg

SEQ ID NO: 48697 - DNA, 28 bp, synthetic construct
  source 1..28: mol_type = other DNA
ctgggtgcaccccgccggcaattcatgg

SEQ ID NO: 48698 - DNA, 28 bp, synthetic construct
  source 1..28: mol_type = other DNA
caccccgccggcaattcatggatccagg

SEQ ID NO: 48699 - DNA, 28 bp, synthetic construct
  source 1..28: mol_type = other DNA
accccgccggcaattcatggatccaggg

SEQ ID NO: 48700 - DNA, 28 bp, synthetic construct
  source 1..28: mol_type = other DNA
gccctggatccatgaattgccggcgggg

SEQ ID NO: 48701 - DNA, 28 bp, synthetic construct
  source 1..28: mol_type = other DNA
tgccctggatccatgaattgccggcggg

SEQ ID NO: 48702 - DNA, 28 bp, synthetic construct
  source 1..28: mol_type = other DNA
atgccctggatccatgaattgccggcgg

SEQ ID NO: 48703 - DNA, 28 bp, synthetic construct
  source 1..28: mol_type = other DNA
ctaatgccctggatccatgaattgccgg

SEQ ID NO: 48704 - DNA, 28 bp, synthetic construct
  source 1..28: mol_type = other DNA
tcatggatccagggcattagcactgcgg

SEQ ID NO: 48705 - DNA, 28 bp, synthetic construct
  source 1..28: mol_type = other DNA
tggatccagggcattagcactgcggtgg

SEQ ID NO: 48706 - DNA, 28 bp, synthetic construct
  source 1..28: mol_type = other DNA
atccagggcattagcactgcggtggagg

SEQ ID NO: 48707 - DNA, 28 bp, synthetic construct
  source 1..28: mol_type = other DNA
cacctccaccgcagtgctaatgccctgg

SEQ ID NO: 48708 - DNA, 28 bp, synthetic construct
  source 1..28: mol_type = other DNA
cagggcattagcactgcggtggaggtgg

SEQ ID NO: 48709 - DNA, 28 bp, synthetic construct
  source 1..28: mol_type = other DNA
agggcattagcactgcggtggaggtggg

SEQ ID NO: 48710 - DNA, 28 bp, synthetic construct
  source 1..28: mol_type = other DNA
cattagcactgcggtggaggtgggttgg

SEQ ID NO: 48711 - DNA, 28 bp, synthetic construct
  source 1..28: mol_type = other DNA
agcactgcggtggaggtgggttggctgg

SEQ ID NO: 48712 - DNA, 28 bp, synthetic construct
  source 1..28: mol_type = other DNA
gcactgcggtggaggtgggttggctggg

SEQ ID NO: 48713 - DNA, 28 bp, synthetic construct
  source 1..28: mol_type = other DNA
ggaggtgggttggctgggagaccccagg

SEQ ID NO: 48714 - DNA, 28 bp, synthetic construct
  source 1..28: mol_type = other DNA
ggtgggttggctgggagaccccaggtgg

SEQ ID NO: 48715 - DNA, 28 bp, synthetic construct
  source 1..28: mol_type = other DNA
gtgggttggctgggagaccccaggtggg

SEQ ID NO: 48716 - DNA, 28 bp, synthetic construct
  source 1..28: mol_type = other DNA
tgggttggctgggagaccccaggtgggg

SEQ ID NO: 48717 - DNA, 28 bp, synthetic construct
  source 1..28: mol_type = other DNA
tgggagaccccaggtggggttcacttgg

SEQ ID NO: 48718 - DNA, 28 bp, synthetic construct
  source 1..28: mol_type = other DNA
gggagaccccaggtggggttcacttggg

SEQ ID NO: 48719 - DNA, 28 bp, synthetic construct
  source 1..28: mol_type = other DNA
ctacagcccaagtgaaccccacctgggg

SEQ ID NO: 48720 - DNA, 28 bp, synthetic construct
  source 1..28: mol_type = other DNA
cctacagcccaagtgaaccccacctggg

SEQ ID NO: 48721 - DNA, 28 bp, synthetic construct
  source 1..28: mol_type = other DNA
ccctacagcccaagtgaaccccacctgg

SEQ ID NO: 48722 - DNA, 28 bp, synthetic construct
  source 1..28: mol_type = other DNA
caggtggggttcacttgggctgtagggg

SEQ ID NO: 48723 - DNA, 28 bp, synthetic construct
  source 1..28: mol_type = other DNA
ggttcacttgggctgtaggggaatgagg

SEQ ID NO: 48724 - DNA, 28 bp, synthetic construct
  source 1..28: mol_type = other DNA
gttcacttgggctgtaggggaatgaggg

SEQ ID NO: 48725 - DNA, 28 bp, synthetic construct
  source 1..28: mol_type = other DNA
tgggctgtaggggaatgagggagagtgg

SEQ ID NO: 48726 - DNA, 28 bp, synthetic construct
  source 1..28: mol_type = other DNA
aggggaatgagggagagtggcctacagg

SEQ ID NO: 48727 - DNA, 28 bp, synthetic construct
  source 1..28: mol_type = other DNA
agtggcctacaggaaagagacaaagagg

SEQ ID NO: 48728 - DNA, 28 bp, synthetic construct
  source 1..28: mol_type = other DNA
gcctacaggaaagagacaaagaggttgg

SEQ ID NO: 48729 - DNA, 28 bp, synthetic construct
  source 1..28: mol_type = other DNA
tccaacctctttgtctctttcctgtagg

SEQ ID NO: 48730 - DNA, 28 bp, synthetic construct
  source 1..28: mol_type = other DNA
gacaaagaggttggagacacatcagagg

SEQ ID NO: 48731 - DNA, 28 bp, synthetic construct
  source 1..28: mol_type = other DNA
acaaagaggttggagacacatcagaggg

SEQ ID NO: 48732 - DNA, 28 bp, synthetic construct
  source 1..28: mol_type = other DNA
caaagaggttggagacacatcagagggg

SEQ ID NO: 48733 - DNA, 28 bp, synthetic construct
  source 1..28: mol_type = other DNA
gaggttggagacacatcagaggggcagg

SEQ ID NO: 48734 - DNA, 28 bp, synthetic construct
  source 1..28: mol_type = other DNA
aggttggagacacatcagaggggcaggg

SEQ ID NO: 48735 - DNA, 28 bp, synthetic construct
  source 1..28: mol_type = other DNA
ggttggagacacatcagaggggcagggg

SEQ ID NO: 48736 - DNA, 28 bp, synthetic construct
  source 1..28: mol_type = other DNA
gagacacatcagaggggcaggggcaagg

SEQ ID NO: 48737 - DNA, 28 bp, synthetic construct
  source 1..28: mol_type = other DNA
atcagaggggcaggggcaaggtgccagg

SEQ ID NO: 48738 - DNA, 28 bp, synthetic construct
  source 1..28: mol_type = other DNA
tcagaggggcaggggcaaggtgccaggg

SEQ ID NO: 48739 - DNA, 28 bp, synthetic construct
  source 1..28: mol_type = other DNA
ggggcaaggtgccagggaactgagctgg

SEQ ID NO: 48740 - DNA, 28 bp, synthetic construct
  source 1..28: mol_type = other DNA
gagagaggagaccagctcagttccctgg

SEQ ID NO: 48741 - DNA, 28 bp, synthetic construct
  source 1..28: mol_type = other DNA
gctggtctcctctctcaaccaagagagg

SEQ ID NO: 48742 - DNA, 28 bp, synthetic construct
  source 1..28: mol_type = other DNA
tctcctctctcaaccaagagaggtcagg

SEQ ID NO: 48743 - DNA, 28 bp, synthetic construct
  source 1..28: mol_type = other DNA
tatcctgacctctcttggttgagagagg

SEQ ID NO: 48744 - DNA, 28 bp, synthetic construct
  source 1..28: mol_type = other DNA
ttcactggtgtatcctgacctctcttgg

SEQ ID NO: 48745 - DNA, 28 bp, synthetic construct
  source 1..28: mol_type = other DNA
cagttccatgtcactgctcagaggaagg

SEQ ID NO: 48746 - DNA, 28 bp, synthetic construct
  source 1..28: mol_type = other DNA
ccatgtcactgctcagaggaaggcctgg

SEQ ID NO: 48747 - DNA, 28 bp, synthetic construct
  source 1..28: mol_type = other DNA
gtcactgctcagaggaaggcctggcagg

SEQ ID NO: 48748 - DNA, 28 bp, synthetic construct
  source 1..28: mol_type = other DNA
tcactgctcagaggaaggcctggcaggg

SEQ ID NO: 48749 - DNA, 28 bp, synthetic construct
  source 1..28: mol_type = other DNA
ctgctcagaggaaggcctggcagggagg

SEQ ID NO: 48750 - DNA, 28 bp, synthetic construct
  source 1..28: mol_type = other DNA
tgctcagaggaaggcctggcagggaggg

SEQ ID NO: 48751 - DNA, 28 bp, synthetic construct
  source 1..28: mol_type = other DNA
ggaaggcctggcagggagggctcagtgg

SEQ ID NO: 48752 - DNA, 28 bp, synthetic construct
  source 1..28: mol_type = other DNA
aggcctggcagggagggctcagtggtgg

SEQ ID NO: 48753 - DNA, 28 bp, synthetic construct
  source 1..28: mol_type = other DNA
ggcctggcagggagggctcagtggtggg

SEQ ID NO: 48754 - DNA, 28 bp, synthetic construct
  source 1..28: mol_type = other DNA
gcctggcagggagggctcagtggtgggg

SEQ ID NO: 48755 - DNA, 28 bp, synthetic construct
  source 1..28: mol_type = other DNA
accccaccactgagccctccctgccagg

SEQ ID NO: 48756 - DNA, 28 bp, synthetic construct
  source 1..28: mol_type = other DNA
gagggctcagtggtggggtcccaagagg

SEQ ID NO: 48757 - DNA, 28 bp, synthetic construct
  source 1..28: mol_type = other DNA
agggctcagtggtggggtcccaagaggg

SEQ ID NO: 48758 - DNA, 28 bp, synthetic construct
  source 1..28: mol_type = other DNA
ctcagtggtggggtcccaagagggcagg

SEQ ID NO: 48759 - DNA, 28 bp, synthetic construct
  source 1..28: mol_type = other DNA
tcagtggtggggtcccaagagggcaggg

SEQ ID NO: 48760 - DNA, 28 bp, synthetic construct
  source 1..28: mol_type = other DNA
tggtggggtcccaagagggcagggcagg

SEQ ID NO: 48761 - DNA, 28 bp, synthetic construct
  source 1..28: mol_type = other DNA
gtcccaagagggcagggcaggcatgagg

SEQ ID NO: 48762 - DNA, 28 bp, synthetic construct
  source 1..28: mol_type = other DNA
tcccaagagggcagggcaggcatgaggg

SEQ ID NO: 48763 - DNA, 28 bp, synthetic construct
  source 1..28: mol_type = other DNA
gccctcatgcctgccctgccctcttggg

SEQ ID NO: 48764 - DNA, 28 bp, synthetic construct
  source 1..28: mol_type = other DNA
ggccctcatgcctgccctgccctcttgg

SEQ ID NO: 48765 - DNA, 28 bp, synthetic construct
  source 1..28: mol_type = other DNA
agagggcagggcaggcatgagggccagg

SEQ ID NO: 48766 - DNA, 28 bp, synthetic construct
  source 1..28: mol_type = other DNA
gagggcagggcaggcatgagggccaggg

SEQ ID NO: 48767 - DNA, 28 bp, synthetic construct
  source 1..28: mol_type = other DNA
agggcagggcaggcatgagggccagggg

SEQ ID NO: 48768 - DNA, 28 bp, synthetic construct
  source 1..28: mol_type = other DNA
ggcatgagggccaggggatgtcccgcgg

SEQ ID NO: 48769 - DNA, 28 bp, synthetic construct
  source 1..28: mol_type = other DNA
gcatgagggccaggggatgtcccgcggg

SEQ ID NO: 48770 - DNA, 28 bp, synthetic construct
  source 1..28: mol_type = other DNA
gggccaggggatgtcccgcgggcagtgg

SEQ ID NO: 48771 - DNA, 28 bp, synthetic construct
  source 1..28: mol_type = other DNA
ggccaggggatgtcccgcgggcagtggg

SEQ ID NO: 48772 - DNA, 28 bp, synthetic construct
  source 1..28: mol_type = other DNA
gccaggggatgtcccgcgggcagtgggg

SEQ ID NO: 48773 - DNA, 28 bp, synthetic construct
  source 1..28: mol_type = other DNA
accccactgcccgcgggacatcccctgg

SEQ ID NO: 48774 - DNA, 28 bp, synthetic construct
  source 1..28: mol_type = other DNA
gtggacagaggaccccactgcccgcggg

SEQ ID NO: 48775 - DNA, 28 bp, synthetic construct
  source 1..28: mol_type = other DNA
agtggacagaggaccccactgcccgcgg

SEQ ID NO: 48776 - DNA, 28 bp, synthetic construct
  source 1..28: mol_type = other DNA
caggaaggggcaggtgagtggacagagg

SEQ ID NO: 48777 - DNA, 28 bp, synthetic construct
  source 1..28: mol_type = other DNA
ctctgtccactcacctgccccttcctgg

SEQ ID NO: 48778 - DNA, 28 bp, synthetic construct
  source 1..28: mol_type = other DNA
tctgtccactcacctgccccttcctggg

SEQ ID NO: 48779 - DNA, 28 bp, synthetic construct
  source 1..28: mol_type = other DNA
ccaagcccaggaaggggcaggtgagtgg

SEQ ID NO: 48780 - DNA, 28 bp, synthetic construct
  source 1..28: mol_type = other DNA
cactcacctgccccttcctgggcttggg

SEQ ID NO: 48781 - DNA, 28 bp, synthetic construct
  source 1..28: mol_type = other DNA
tgtgcgcccaagcccaggaaggggcagg

SEQ ID NO: 48782 - DNA, 28 bp, synthetic construct
  source 1..28: mol_type = other DNA
tcactgtgcgcccaagcccaggaagggg

SEQ ID NO: 48783 - DNA, 28 bp, synthetic construct
  source 1..28: mol_type = other DNA
gtcactgtgcgcccaagcccaggaaggg

SEQ ID NO: 48784 - DNA, 28 bp, synthetic construct
  source 1..28: mol_type = other DNA
ggtcactgtgcgcccaagcccaggaagg

SEQ ID NO: 48785 - DNA, 28 bp, synthetic construct
  source 1..28: mol_type = other DNA
ctgaggtcactgtgcgcccaagcccagg

SEQ ID NO: 48786 - DNA, 28 bp, synthetic construct
  source 1..28: mol_type = other DNA
agtgacctcagccccatctgctcccagg

SEQ ID NO: 48787 - DNA, 28 bp, synthetic construct
  source 1..28: mol_type = other DNA
ccatacctgggagcagatggggctgagg

SEQ ID NO: 48788 - DNA, 28 bp, synthetic construct
  source 1..28: mol_type = other DNA
cagccccatctgctcccaggtatggagg

SEQ ID NO: 48789 - DNA, 28 bp, synthetic construct
  source 1..28: mol_type = other DNA
agccccatctgctcccaggtatggaggg

SEQ ID NO: 48790 - DNA, 28 bp, synthetic construct
  source 1..28: mol_type = other DNA
agccctccatacctgggagcagatgggg

SEQ ID NO: 48791 - DNA, 28 bp, synthetic construct
  source 1..28: mol_type = other DNA
tagccctccatacctgggagcagatggg

SEQ ID NO: 48792 - DNA, 28 bp, synthetic construct
  source 1..28: mol_type = other DNA
ctagccctccatacctgggagcagatgg

SEQ ID NO: 48793 - DNA, 28 bp, synthetic construct
  source 1..28: mol_type = other DNA
catctgctcccaggtatggagggctagg

SEQ ID NO: 48794 - DNA, 28 bp, synthetic construct
  source 1..28: mol_type = other DNA
tcccaggtatggagggctaggtcccagg

SEQ ID NO: 48795 - DNA, 28 bp, synthetic construct
  source 1..28: mol_type = other DNA
gcctgggacctagccctccatacctggg

SEQ ID NO: 48796 - DNA, 28 bp, synthetic construct
  source 1..28: mol_type = other DNA
ggcctgggacctagccctccatacctgg

SEQ ID NO: 48797 - DNA, 28 bp, synthetic construct
  source 1..28: mol_type = other DNA
gctcagtatggggagcagcgggcctggg

SEQ ID NO: 48798 - DNA, 28 bp, synthetic construct
  source 1..28: mol_type = other DNA
ggctcagtatggggagcagcgggcctgg

SEQ ID NO: 48799 - DNA, 28 bp, synthetic construct
  source 1..28: mol_type = other DNA
ctggtggctcagtatggggagcagcggg

SEQ ID NO: 48800 - DNA, 28 bp, synthetic construct
  source 1..28: mol_type = other DNA
cctggtggctcagtatggggagcagcgg

SEQ ID NO: 48801 - DNA, 28 bp, synthetic construct
  source 1..28: mol_type = other DNA
tccccatactgagccaccaggtacgagg

SEQ ID NO: 48802 - DNA, 28 bp, synthetic construct
  source 1..28: mol_type = other DNA
gcctcgtacctggtggctcagtatgggg

SEQ ID NO: 48803 - DNA, 28 bp, synthetic construct
  source 1..28: mol_type = other DNA
ggcctcgtacctggtggctcagtatggg

SEQ ID NO: 48804 - DNA, 28 bp, synthetic construct
  source 1..28: mol_type = other DNA
tggcctcgtacctggtggctcagtatgg

SEQ ID NO: 48805 - DNA, 28 bp, synthetic construct
  source 1..28: mol_type = other DNA
ggcatggaggtggcctcgtacctggtgg

SEQ ID NO: 48806 - DNA, 28 bp, synthetic construct
  source 1..28: mol_type = other DNA
agtggcatggaggtggcctcgtacctgg

SEQ ID NO: 48807 - DNA, 28 bp, synthetic construct
  source 1..28: mol_type = other DNA
ccagagaagacgagtggcatggaggtgg

SEQ ID NO: 48808 - DNA, 28 bp, synthetic construct
  source 1..28: mol_type = other DNA
cagccagagaagacgagtggcatggagg

SEQ ID NO: 48809 - DNA, 28 bp, synthetic construct
  source 1..28: mol_type = other DNA
gctcagccagagaagacgagtggcatgg

SEQ ID NO: 48810 - DNA, 28 bp, synthetic construct
  source 1..28: mol_type = other DNA
atgccactcgtcttctctggctgagcgg

SEQ ID NO: 48811 - DNA, 28 bp, synthetic construct
  source 1..28: mol_type = other DNA
tgccactcgtcttctctggctgagcggg

SEQ ID NO: 48812 - DNA, 28 bp, synthetic construct
  source 1..28: mol_type = other DNA
cacccgctcagccagagaagacgagtgg

SEQ ID NO: 48813 - DNA, 28 bp, synthetic construct
  source 1..28: mol_type = other DNA
gcgggtgtctcacccgaagagctcctgg

SEQ ID NO: 48814 - DNA, 28 bp, synthetic construct
  source 1..28: mol_type = other DNA
ataaagcgcactccaggagctcttcggg

SEQ ID NO: 48815 - DNA, 28 bp, synthetic construct
  source 1..28: mol_type = other DNA
aataaagcgcactccaggagctcttcgg

SEQ ID NO: 48816 - DNA, 28 bp, synthetic construct
  source 1..28: mol_type = other DNA
gaagagctcctggagtgcgctttattgg

SEQ ID NO: 48817 - DNA, 28 bp, synthetic construct
  source 1..28: mol_type = other DNA
tctgctcgccaataaagcgcactccagg

SEQ ID NO: 48818 - DNA, 28 bp, synthetic construct
  source 1..28: mol_type = other DNA
gtgcgctttattggcgagcagaagctgg

SEQ ID NO: 48819 - DNA, 28 bp, synthetic construct
  source 1..28: mol_type = other DNA
gaactccttcagctcctccttcttcagg

SEQ ID NO: 48820 - DNA, 28 bp, synthetic construct
  source 1..28: mol_type = other DNA
gagttcctgaagaaggaggagctgaagg

SEQ ID NO: 48821 - DNA, 28 bp, synthetic construct
  source 1..28: mol_type = other DNA
tgttacttggagttcctgaagaaggagg

SEQ ID NO: 48822 - DNA, 28 bp, synthetic construct
  source 1..28: mol_type = other DNA
tccttcttcaggaactccaagtaacagg

SEQ ID NO: 48823 - DNA, 28 bp, synthetic construct
  source 1..28: mol_type = other DNA
gcctgttacttggagttcctgaagaagg

SEQ ID NO: 48824 - DNA, 28 bp, synthetic construct
  source 1..28: mol_type = other DNA
cttcaggaactccaagtaacaggccagg

SEQ ID NO: 48825 - DNA, 28 bp, synthetic construct
  source 1..28: mol_type = other DNA
caggaactccaagtaacaggccaggcgg

SEQ ID NO: 48826 - DNA, 28 bp, synthetic construct
  source 1..28: mol_type = other DNA
tccaagtaacaggccaggcggccccagg

SEQ ID NO: 48827 - DNA, 28 bp, synthetic construct
  source 1..28: mol_type = other DNA
gcctggggccgcctggcctgttacttgg

SEQ ID NO: 48828 - DNA, 28 bp, synthetic construct
  source 1..28: mol_type = other DNA
atggctggcggagcctggggccgcctgg

SEQ ID NO: 48829 - DNA, 28 bp, synthetic construct
  source 1..28: mol_type = other DNA
ggacagagatggctggcggagcctgggg

SEQ ID NO: 48830 - DNA, 28 bp, synthetic construct
  source 1..28: mol_type = other DNA
gggacagagatggctggcggagcctggg

SEQ ID NO: 48831 - DNA, 28 bp, synthetic construct
  source 1..28: mol_type = other DNA
cgggacagagatggctggcggagcctgg

SEQ ID NO: 48832 - DNA, 28 bp, synthetic construct
  source 1..28: mol_type = other DNA
caggctccgccagccatctctgtcccgg

SEQ ID NO: 48833 - DNA, 28 bp, synthetic construct
  source 1..28: mol_type = other DNA
ttaactccgggacagagatggctggcgg

SEQ ID NO: 48834 - DNA, 28 bp, synthetic construct
  source 1..28: mol_type = other DNA
ctcttaactccgggacagagatggctgg

SEQ ID NO: 48835 - DNA, 28 bp, synthetic construct
  source 1..28: mol_type = other DNA
cagccatctctgtcccggagttaagagg

SEQ ID NO: 48836 - DNA, 28 bp, synthetic construct
  source 1..28: mol_type = other DNA
agccatctctgtcccggagttaagaggg

SEQ ID NO: 48837 - DNA, 28 bp, synthetic construct
  source 1..28: mol_type = other DNA
caccctcttaactccgggacagagatgg

SEQ ID NO: 48838 - DNA, 28 bp, synthetic construct
  source 1..28: mol_type = other DNA
tctgtcccggagttaagagggtgtctgg

SEQ ID NO: 48839 - DNA, 28 bp, synthetic construct
  source 1..28: mol_type = other DNA
ctgtcccggagttaagagggtgtctggg

SEQ ID NO: 48840 - DNA, 28 bp, synthetic construct
  source 1..28: mol_type = other DNA
tgtcccggagttaagagggtgtctgggg

SEQ ID NO: 48841 - DNA, 28 bp, synthetic construct
  source 1..28: mol_type = other DNA
gtcccggagttaagagggtgtctggggg

SEQ ID NO: 48842 - DNA, 28 bp, synthetic construct
  source 1..28: mol_type = other DNA
atcccccagacaccctcttaactccggg

SEQ ID NO: 48843 - DNA, 28 bp, synthetic construct
  source 1..28: mol_type = other DNA
catcccccagacaccctcttaactccgg

SEQ ID NO: 48844 - DNA, 28 bp, synthetic construct
  source 1..28: mol_type = other DNA
aagagggtgtctgggggatgttcccagg

SEQ ID NO: 48845 - DNA, 28 bp, synthetic construct
  source 1..28: mol_type = other DNA
agggtgtctgggggatgttcccaggtgg

SEQ ID NO: 48846 - DNA, 28 bp, synthetic construct
  source 1..28: mol_type = other DNA
gtctgggggatgttcccaggtggtgagg

SEQ ID NO: 48847 - DNA, 28 bp, synthetic construct
  source 1..28: mol_type = other DNA
tctgggggatgttcccaggtggtgaggg

SEQ ID NO: 48848 - DNA, 28 bp, synthetic construct
  source 1..28: mol_type = other DNA
gatgttcccaggtggtgagggtatcagg

SEQ ID NO: 48849 - DNA, 28 bp, synthetic construct
  source 1..28: mol_type = other DNA
ttcccaggtggtgagggtatcaggcagg

SEQ ID NO: 48850 - DNA, 28 bp, synthetic construct
  source 1..28: mol_type = other DNA
tgcctgcctgataccctcaccacctggg

SEQ ID NO: 48851 - DNA, 28 bp, synthetic construct
  source 1..28: mol_type = other DNA
ctgcctgcctgataccctcaccacctgg

SEQ ID NO: 48852 - DNA, 28 bp, synthetic construct
  source 1..28: mol_type = other DNA
cagagaacagtgctgtcctttgccttgg

SEQ ID NO: 48853 - DNA, 28 bp, synthetic construct
  source 1..28: mol_type = other DNA
taagagacggtaagagccaaggcaaagg

SEQ ID NO: 48854 - DNA, 28 bp, synthetic construct
  source 1..28: mol_type = other DNA
gctgaataagagacggtaagagccaagg

SEQ ID NO: 48855 - DNA, 28 bp, synthetic construct
  source 1..28: mol_type = other DNA
ctcttaccgtctcttattcagcattcgg

SEQ ID NO: 48856 - DNA, 28 bp, synthetic construct
  source 1..28: mol_type = other DNA
tgggttccgaatgctgaataagagacgg

SEQ ID NO: 48857 - DNA, 28 bp, synthetic construct
  source 1..28: mol_type = other DNA
ttcggaacccagttttataaatcccagg

SEQ ID NO: 48858 - DNA, 28 bp, synthetic construct
  source 1..28: mol_type = other DNA
tcggaacccagttttataaatcccaggg

SEQ ID NO: 48859 - DNA, 28 bp, synthetic construct
  source 1..28: mol_type = other DNA
taggtgccctgggatttataaaactggg

SEQ ID NO: 48860 - DNA, 28 bp, synthetic construct
  source 1..28: mol_type = other DNA
gtaggtgccctgggatttataaaactgg

SEQ ID NO: 48861 - DNA, 28 bp, synthetic construct
  source 1..28: mol_type = other DNA
atcggcgtctatctgtaggtgccctggg

SEQ ID NO: 48862 - DNA, 28 bp, synthetic construct
  source 1..28: mol_type = other DNA
tatcggcgtctatctgtaggtgccctgg

SEQ ID NO: 48863 - DNA, 28 bp, synthetic construct
  source 1..28: mol_type = other DNA
ggcacctacagatagacgccgatagagg

SEQ ID NO: 48864 - DNA, 28 bp, synthetic construct
  source 1..28: mol_type = other DNA
gcacctacagatagacgccgatagaggg

SEQ ID NO: 48865 - DNA, 28 bp, synthetic construct
  source 1..28: mol_type = other DNA
cacctacagatagacgccgatagagggg

SEQ ID NO: 48866 - DNA, 28 bp, synthetic construct
  source 1..28: mol_type = other DNA
acctacagatagacgccgatagaggggg

SEQ ID NO: 48867 - DNA, 28 bp, synthetic construct
  source 1..28: mol_type = other DNA
tccccctctatcggcgtctatctgtagg

SEQ ID NO: 48868 - DNA, 28 bp, synthetic construct
  source 1..28: mol_type = other DNA
cagatagacgccgatagagggggagtgg

SEQ ID NO: 48869 - DNA, 28 bp, synthetic construct
  source 1..28: mol_type = other DNA
tagacgccgatagagggggagtggtagg

SEQ ID NO: 48870 - DNA, 28 bp, synthetic construct
  source 1..28: mol_type = other DNA
gcttttcctaccactccccctctatcgg

SEQ ID NO: 48871 - DNA, 28 bp, synthetic construct
  source 1..28: mol_type = other DNA
tagagggggagtggtaggaaaagccagg

SEQ ID NO: 48872 - DNA, 28 bp, synthetic construct
  source 1..28: mol_type = other DNA
agagggggagtggtaggaaaagccaggg

SEQ ID NO: 48873 - DNA, 28 bp, synthetic construct
  source 1..28: mol_type = other DNA
gagggggagtggtaggaaaagccagggg

SEQ ID NO: 48874 - DNA, 28 bp, synthetic construct
  source 1..28: mol_type = other DNA
ggggagtggtaggaaaagccaggggagg

SEQ ID NO: 48875 - DNA, 28 bp, synthetic construct
  source 1..28: mol_type = other DNA
gggagtggtaggaaaagccaggggaggg

SEQ ID NO: 48876 - DNA, 28 bp, synthetic construct
  source 1..28: mol_type = other DNA
agtggtaggaaaagccaggggagggagg

SEQ ID NO: 48877 - DNA, 28 bp, synthetic construct
  source 1..28: mol_type = other DNA
aaagccaggggagggaggagcccagagg

SEQ ID NO: 48878 - DNA, 28 bp, synthetic construct
  source 1..28: mol_type = other DNA
aagccaggggagggaggagcccagaggg

SEQ ID NO: 48879 - DNA, 28 bp, synthetic construct
  source 1..28: mol_type = other DNA
agccaggggagggaggagcccagagggg

SEQ ID NO: 48880 - DNA, 28 bp, synthetic construct
  source 1..28: mol_type = other DNA
ggcccctctgggctcctccctcccctgg

SEQ ID NO: 48881 - DNA, 28 bp, synthetic construct
  source 1..28: mol_type = other DNA
gagcccagaggggcctgcaagacactgg

SEQ ID NO: 48882 - DNA, 28 bp, synthetic construct
  source 1..28: mol_type = other DNA
cttccagtgtcttgcaggcccctctggg

SEQ ID NO: 48883 - DNA, 28 bp, synthetic construct
  source 1..28: mol_type = other DNA
tcttccagtgtcttgcaggcccctctgg

SEQ ID NO: 48884 - DNA, 28 bp, synthetic construct
  source 1..28: mol_type = other DNA
cagctgacttcttccagtgtcttgcagg

SEQ ID NO: 48885 - DNA, 28 bp, synthetic construct
  source 1..28: mol_type = other DNA
aagacactggaagaagtcagctgatagg

SEQ ID NO: 48886 - DNA, 28 bp, synthetic construct
  source 1..28: mol_type = other DNA
agacactggaagaagtcagctgataggg

SEQ ID NO: 48887 - DNA, 28 bp, synthetic construct
  source 1..28: mol_type = other DNA
cactggaagaagtcagctgatagggagg

SEQ ID NO: 48888 - DNA, 28 bp, synthetic construct
  source 1..28: mol_type = other DNA
aagaagtcagctgatagggaggtcctgg

SEQ ID NO: 48889 - DNA, 28 bp, synthetic construct
  source 1..28: mol_type = other DNA
agaagtcagctgatagggaggtcctggg

SEQ ID NO: 48890 - DNA, 28 bp, synthetic construct
  source 1..28: mol_type = other DNA
gtcagctgatagggaggtcctgggatgg

SEQ ID NO: 48891 - DNA, 28 bp, synthetic construct
  source 1..28: mol_type = other DNA
tcagctgatagggaggtcctgggatggg

SEQ ID NO: 48892 - DNA, 28 bp, synthetic construct
  source 1..28: mol_type = other DNA
cagctgatagggaggtcctgggatgggg

SEQ ID NO: 48893 - DNA, 28 bp, synthetic construct
  source 1..28: mol_type = other DNA
atagggaggtcctgggatggggtccagg

SEQ ID NO: 48894 - DNA, 28 bp, synthetic construct
  source 1..28: mol_type = other DNA
tagggaggtcctgggatggggtccaggg

SEQ ID NO: 48895 - DNA, 28 bp, synthetic construct
  source 1..28: mol_type = other DNA
aggtcctgggatggggtccagggccagg

SEQ ID NO: 48896 - DNA, 28 bp, synthetic construct
  source 1..28: mol_type = other DNA
cctgggatggggtccagggccaggcagg

SEQ ID NO: 48897 - DNA, 28 bp, synthetic construct
  source 1..28: mol_type = other DNA
ctgggatggggtccagggccaggcaggg

SEQ ID NO: 48898 - DNA, 28 bp, synthetic construct
  source 1..28: mol_type = other DNA
ggatggggtccagggccaggcagggagg

SEQ ID NO: 48899 - DNA, 28 bp, synthetic construct
  source 1..28: mol_type = other DNA
gatggggtccagggccaggcagggaggg

SEQ ID NO: 48900 - DNA, 28 bp, synthetic construct
  source 1..28: mol_type = other DNA
ggtccagggccaggcagggagggtgagg

SEQ ID NO: 48901 - DNA, 28 bp, synthetic construct
  source 1..28: mol_type = other DNA
gtccagggccaggcagggagggtgaggg

SEQ ID NO: 48902 - DNA, 28 bp, synthetic construct
  source 1..28: mol_type = other DNA
caccctcaccctccctgcctggccctgg

SEQ ID NO: 48903 - DNA, 28 bp, synthetic construct
  source 1..28: mol_type = other DNA
gggccaggcagggagggtgagggtgagg

SEQ ID NO: 48904 - DNA, 28 bp, synthetic construct
  source 1..28: mol_type = other DNA
ggccaggcagggagggtgagggtgaggg

SEQ ID NO: 48905 - DNA, 28 bp, synthetic construct
  source 1..28: mol_type = other DNA
gccaggcagggagggtgagggtgagggg

SEQ ID NO: 48906 - DNA, 28 bp, synthetic construct
  source 1..28: mol_type = other DNA
tcccctcaccctcaccctccctgcctgg

SEQ ID NO: 48907 - DNA, 28 bp, synthetic construct
  source 1..28: mol_type = other DNA
gggagggtgagggtgaggggagatgtgg

SEQ ID NO: 48908 - DNA, 28 bp, synthetic construct
  source 1..28: mol_type = other DNA
gtgagggtgaggggagatgtggtgacgg

SEQ ID NO: 48909 - DNA, 28 bp, synthetic construct
  source 1..28: mol_type = other DNA
tgagggtgaggggagatgtggtgacggg

SEQ ID NO: 48910 - DNA, 28 bp, synthetic construct
  source 1..28: mol_type = other DNA
tgaggggagatgtggtgacgggagatgg

SEQ ID NO: 48911 - DNA, 28 bp, synthetic construct
  source 1..28: mol_type = other DNA
gaggggagatgtggtgacgggagatggg

SEQ ID NO: 48912 - DNA, 28 bp, synthetic construct
  source 1..28: mol_type = other DNA
aggggagatgtggtgacgggagatgggg

SEQ ID NO: 48913 - DNA, 28 bp, synthetic construct
  source 1..28: mol_type = other DNA
agatgtggtgacgggagatggggtgtgg

SEQ ID NO: 48914 - DNA, 28 bp, synthetic construct
  source 1..28: mol_type = other DNA
gatgtggtgacgggagatggggtgtggg

SEQ ID NO: 48915 - DNA, 28 bp, synthetic construct
  source 1..28: mol_type = other DNA
gtgttcctcagattcttccctctcctgg

SEQ ID NO: 48916 - DNA, 28 bp, synthetic construct
  source 1..28: mol_type = other DNA
tgttcctcagattcttccctctcctggg

SEQ ID NO: 48917 - DNA, 28 bp, synthetic construct
  source 1..28: mol_type = other DNA
aggacccaggagagggaagaatctgagg

SEQ ID NO: 48918 - DNA, 28 bp, synthetic construct
  source 1..28: mol_type = other DNA
tcagattcttccctctcctgggtcctgg

SEQ ID NO: 48919 - DNA, 28 bp, synthetic construct
  source 1..28: mol_type = other DNA
tctcaggagtccaggacccaggagaggg

SEQ ID NO: 48920 - DNA, 28 bp, synthetic construct
  source 1..28: mol_type = other DNA
atctcaggagtccaggacccaggagagg

SEQ ID NO: 48921 - DNA, 28 bp, synthetic construct
  source 1..28: mol_type = other DNA
ggttgatctcaggagtccaggacccagg

SEQ ID NO: 48922 - DNA, 28 bp, synthetic construct
  source 1..28: mol_type = other DNA
gctcaagggttgatctcaggagtccagg

SEQ ID NO: 48923 - DNA, 28 bp, synthetic construct
  source 1..28: mol_type = other DNA
tcctgagatcaacccttgagctgcaagg

SEQ ID NO: 48924 - DNA, 28 bp, synthetic construct
  source 1..28: mol_type = other DNA
gccttgcagctcaagggttgatctcagg

SEQ ID NO: 48925 - DNA, 28 bp, synthetic construct
  source 1..28: mol_type = other DNA
acccttgagctgcaaggctgagaagagg

SEQ ID NO: 48926 - DNA, 28 bp, synthetic construct
  source 1..28: mol_type = other DNA
acctcttctcagccttgcagctcaaggg

SEQ ID NO: 48927 - DNA, 28 bp, synthetic construct
  source 1..28: mol_type = other DNA
cacctcttctcagccttgcagctcaagg

SEQ ID NO: 48928 - DNA, 28 bp, synthetic construct
  source 1..28: mol_type = other DNA
cttgagctgcaaggctgagaagaggtgg

SEQ ID NO: 48929 - DNA, 28 bp, synthetic construct
  source 1..28: mol_type = other DNA
ttgagctgcaaggctgagaagaggtggg

SEQ ID NO: 48930 - DNA, 28 bp, synthetic construct
  source 1..28: mol_type = other DNA
tgagctgcaaggctgagaagaggtgggg

SEQ ID NO: 48931 - DNA, 28 bp, synthetic construct
  source 1..28: mol_type = other DNA
gctgcaaggctgagaagaggtggggtgg

SEQ ID NO: 48932 - DNA, 28 bp, synthetic construct
  source 1..28: mol_type = other DNA
ctgcaaggctgagaagaggtggggtggg

SEQ ID NO: 48933 - DNA, 28 bp, synthetic construct
  source 1..28: mol_type = other DNA
caaggctgagaagaggtggggtgggagg

SEQ ID NO: 48934 - DNA, 28 bp, synthetic construct
  source 1..28: mol_type = other DNA
ggtggggtgggaggagccgcagagcagg

SEQ ID NO: 48935 - DNA, 28 bp, synthetic construct
  source 1..28: mol_type = other DNA
gtggggtgggaggagccgcagagcaggg

SEQ ID NO: 48936 - DNA, 28 bp, synthetic construct
  source 1..28: mol_type = other DNA
gtgggaggagccgcagagcagggaatgg

SEQ ID NO: 48937 - DNA, 28 bp, synthetic construct
  source 1..28: mol_type = other DNA
tgggaggagccgcagagcagggaatggg

SEQ ID NO: 48938 - DNA, 28 bp, synthetic construct
  source 1..28: mol_type = other DNA
ttctgaaagcccattccctgctctgcgg

SEQ ID NO: 48939 - DNA, 28 bp, synthetic construct
  source 1..28: mol_type = other DNA
gggaatgggctttcagaacccagagtgg

SEQ ID NO: 48940 - DNA, 28 bp, synthetic construct
  source 1..28: mol_type = other DNA
gctttcagaacccagagtggagccccgg

SEQ ID NO: 48941 - DNA, 28 bp, synthetic construct
  source 1..28: mol_type = other DNA
ctttcagaacccagagtggagccccggg

SEQ ID NO: 48942 - DNA, 28 bp, synthetic construct
  source 1..28: mol_type = other DNA
aacccagagtggagccccgggctgctgg

SEQ ID NO: 48943 - DNA, 28 bp, synthetic construct
  source 1..28: mol_type = other DNA
agccagcagcccggggctccactctggg

SEQ ID NO: 48944 - DNA, 28 bp, synthetic construct
  source 1..28: mol_type = other DNA
gagccagcagcccggggctccactctgg

SEQ ID NO: 48945 - DNA, 28 bp, synthetic construct
  source 1..28: mol_type = other DNA
gtggagccccgggctgctggctcccagg

SEQ ID NO: 48946 - DNA, 28 bp, synthetic construct
  source 1..28: mol_type = other DNA
aagaaacctgggagccagcagcccgggg

SEQ ID NO: 48947 - DNA, 28 bp, synthetic construct
  source 1..28: mol_type = other DNA
gaagaaacctgggagccagcagcccggg

SEQ ID NO: 48948 - DNA, 28 bp, synthetic construct
  source 1..28: mol_type = other DNA
tgaagaaacctgggagccagcagcccgg

SEQ ID NO: 48949 - DNA, 28 bp, synthetic construct
  source 1..28: mol_type = other DNA
ctcccaggtttcttcagacctctccagg

SEQ ID NO: 48950 - DNA, 28 bp, synthetic construct
  source 1..28: mol_type = other DNA
ggcctggagaggtctgaagaaacctggg

SEQ ID NO: 48951 - DNA, 28 bp, synthetic construct
  source 1..28: mol_type = other DNA
gggcctggagaggtctgaagaaacctgg

SEQ ID NO: 48952 - DNA, 28 bp, synthetic construct
  source 1..28: mol_type = other DNA
ggtttcttcagacctctccaggccctgg

SEQ ID NO: 48953 - DNA, 28 bp, synthetic construct
  source 1..28: mol_type = other DNA
gtttcttcagacctctccaggccctggg

SEQ ID NO: 48954 - DNA, 28 bp, synthetic construct
  source 1..28: mol_type = other DNA
tttcttcagacctctccaggccctgggg

SEQ ID NO: 48955 - DNA, 28 bp, synthetic construct
  source 1..28: mol_type = other DNA
ctggctggtgccccagggcctggagagg

SEQ ID NO: 48956 - DNA, 28 bp, synthetic construct
  source 1..28: mol_type = other DNA
tcttgctggctggtgccccagggcctgg

SEQ ID NO: 48957 - DNA, 28 bp, synthetic construct
  source 1..28: mol_type = other DNA
gctgttcttgctggctggtgccccaggg

SEQ ID NO: 48958 - DNA, 28 bp, synthetic construct
  source 1..28: mol_type = other DNA
cgctgttcttgctggctggtgccccagg

SEQ ID NO: 48959 - DNA, 28 bp, synthetic construct
  source 1..28: mol_type = other DNA
ttgactaggcgctgttcttgctggctgg

SEQ ID NO: 48960 - DNA, 28 bp, synthetic construct
  source 1..28: mol_type = other DNA
cttgttgactaggcgctgttcttgctgg

SEQ ID NO: 48961 - DNA, 28 bp, synthetic construct
  source 1..28: mol_type = other DNA
agaacagcgcctagtcaacaagagcagg

SEQ ID NO: 48962 - DNA, 28 bp, synthetic construct
  source 1..28: mol_type = other DNA
cagcgcctagtcaacaagagcaggaagg

SEQ ID NO: 48963 - DNA, 28 bp, synthetic construct
  source 1..28: mol_type = other DNA
cgtttccttcctgctcttgttgactagg

SEQ ID NO: 48964 - DNA, 28 bp, synthetic construct
  source 1..28: mol_type = other DNA
agagcaggaaggaaacgtcacccagagg

SEQ ID NO: 48965 - DNA, 28 bp, synthetic construct
  source 1..28: mol_type = other DNA
aaacgtcacccagaggaaacccacaagg

SEQ ID NO: 48966 - DNA, 28 bp, synthetic construct
  source 1..28: mol_type = other DNA
aacgtcacccagaggaaacccacaaggg

SEQ ID NO: 48967 - DNA, 28 bp, synthetic construct
  source 1..28: mol_type = other DNA
acgtcacccagaggaaacccacaagggg

SEQ ID NO: 48968 - DNA, 28 bp, synthetic construct
  source 1..28: mol_type = other DNA
acccagaggaaacccacaaggggcgtgg

SEQ ID NO: 48969 - DNA, 28 bp, synthetic construct
  source 1..28: mol_type = other DNA
gccacgccccttgtgggtttcctctggg

SEQ ID NO: 48970 - DNA, 28 bp, synthetic construct
  source 1..28: mol_type = other DNA
ggccacgccccttgtgggtttcctctgg

SEQ ID NO: 48971 - DNA, 28 bp, synthetic construct
  source 1..28: mol_type = other DNA
gaggaaacccacaaggggcgtggccagg

SEQ ID NO: 48972 - DNA, 28 bp, synthetic construct
  source 1..28: mol_type = other DNA
aggaaacccacaaggggcgtggccaggg

SEQ ID NO: 48973 - DNA, 28 bp, synthetic construct
  source 1..28: mol_type = other DNA
ggaaacccacaaggggcgtggccagggg

SEQ ID NO: 48974 - DNA, 28 bp, synthetic construct
  source 1..28: mol_type = other DNA
gaaacccacaaggggcgtggccaggggg

SEQ ID NO: 48975 - DNA, 28 bp, synthetic construct
  source 1..28: mol_type = other DNA
cctaccccctggccacgccccttgtggg

SEQ ID NO: 48976 - DNA, 28 bp, synthetic construct
  source 1..28: mol_type = other DNA
tcctaccccctggccacgccccttgtgg

SEQ ID NO: 48977 - DNA, 28 bp, synthetic construct
  source 1..28: mol_type = other DNA
cgtggccagggggtaggatcaaaccagg

SEQ ID NO: 48978 - DNA, 28 bp, synthetic construct
  source 1..28: mol_type = other DNA
ccaggcctggtttgatcctaccccctgg

SEQ ID NO: 48979 - DNA, 28 bp, synthetic construct
  source 1..28: mol_type = other DNA
cagggggtaggatcaaaccaggcctggg

SEQ ID NO: 48980 - DNA, 28 bp, synthetic construct
  source 1..28: mol_type = other DNA
gggtaggatcaaaccaggcctgggtagg

SEQ ID NO: 48981 - DNA, 28 bp, synthetic construct
  source 1..28: mol_type = other DNA
actctgagtctggcctacccaggcctgg

SEQ ID NO: 48982 - DNA, 28 bp, synthetic construct
  source 1..28: mol_type = other DNA
ctgtgactctgagtctggcctacccagg

SEQ ID NO: 48983 - DNA, 28 bp, synthetic construct
  source 1..28: mol_type = other DNA
ccatctgaatctgtgactctgagtctgg

SEQ ID NO: 48984 - DNA, 28 bp, synthetic construct
  source 1..28: mol_type = other DNA
cagactcagagtcacagattcagatggg

SEQ ID NO: 48985 - DNA, 28 bp, synthetic construct
  source 1..28: mol_type = other DNA
gagtcacagattcagatgggccacatgg

SEQ ID NO: 48986 - DNA, 28 bp, synthetic construct
  source 1..28: mol_type = other DNA
ttcagatgggccacatggcatctatagg

SEQ ID NO: 48987 - DNA, 28 bp, synthetic construct
  source 1..28: mol_type = other DNA
agatgggccacatggcatctataggcgg

SEQ ID NO: 48988 - DNA, 28 bp, synthetic construct
  source 1..28: mol_type = other DNA
gccacatggcatctataggcggaccagg

SEQ ID NO: 48989 - DNA, 28 bp, synthetic construct
  source 1..28: mol_type = other DNA
tcctggtccgcctatagatgccatgtgg

SEQ ID NO: 48990 - DNA, 28 bp, synthetic construct
  source 1..28: mol_type = other DNA
gcatctataggcggaccaggagcacagg

SEQ ID NO: 48991 - DNA, 28 bp, synthetic construct
  source 1..28: mol_type = other DNA
gtcagctggtctgggcctgtgctcctgg

SEQ ID NO: 48992 - DNA, 28 bp, synthetic construct
  source 1..28: mol_type = other DNA
ggcccagaccagctgacgctgcagcagg

SEQ ID NO: 48993 - DNA, 28 bp, synthetic construct
  source 1..28: mol_type = other DNA
tacctgctgcagcgtcagctggtctggg

SEQ ID NO: 48994 - DNA, 28 bp, synthetic construct
  source 1..28: mol_type = other DNA
gtacctgctgcagcgtcagctggtctgg

SEQ ID NO: 48995 - DNA, 28 bp, synthetic construct
  source 1..28: mol_type = other DNA
gaccagctgacgctgcagcaggtacagg

SEQ ID NO: 48996 - DNA, 28 bp, synthetic construct
  source 1..28: mol_type = other DNA
ggcctgtacctgctgcagcgtcagctgg

SEQ ID NO: 48997 - DNA, 28 bp, synthetic construct
  source 1..28: mol_type = other DNA
agcaggtacaggcccatactaaacacgg

SEQ ID NO: 48998 - DNA, 28 bp, synthetic construct
  source 1..28: mol_type = other DNA
gaggtgcacacaccgtgtttagtatggg

SEQ ID NO: 48999 - DNA, 28 bp, synthetic construct
  source 1..28: mol_type = other DNA
ggaggtgcacacaccgtgtttagtatgg

SEQ ID NO: 49000 - DNA, 28 bp, synthetic construct
  source 1..28: mol_type = other DNA
taaacacggtgtgtgcacctccacatgg

SEQ ID NO: 49001 - DNA, 28 bp, synthetic construct
  source 1..28: mol_type = other DNA
aaacacggtgtgtgcacctccacatggg

SEQ ID NO: 49002 - DNA, 28 bp, synthetic construct
  source 1..28: mol_type = other DNA
atgggctggcggagtgcccatgtggagg

SEQ ID NO: 49003 - DNA, 28 bp, synthetic construct
  source 1..28: mol_type = other DNA
atgatgggctggcggagtgcccatgtgg

SEQ ID NO: 49004 - DNA, 28 bp, synthetic construct
  source 1..28: mol_type = other DNA
agacaggctctagatgatgggctggcgg

SEQ ID NO: 49005 - DNA, 28 bp, synthetic construct
  source 1..28: mol_type = other DNA
tgcagacaggctctagatgatgggctgg

SEQ ID NO: 49006 - DNA, 28 bp, synthetic construct
  source 1..28: mol_type = other DNA
gctctgcagacaggctctagatgatggg

SEQ ID NO: 49007 - DNA, 28 bp, synthetic construct
  source 1..28: mol_type = other DNA
ggctctgcagacaggctctagatgatgg

SEQ ID NO: 49008 - DNA, 28 bp, synthetic construct
  source 1..28: mol_type = other DNA
tcatctagagcctgtctgcagagccagg

SEQ ID NO: 49009 - DNA, 28 bp, synthetic construct
  source 1..28: mol_type = other DNA
gagtctgcatcctggctctgcagacagg

SEQ ID NO: 49010 - DNA, 28 bp, synthetic construct
  source 1..28: mol_type = other DNA
acaactgctcggagagtctgcatcctgg

SEQ ID NO: 49011 - DNA, 28 bp, synthetic construct
  source 1..28: mol_type = other DNA
ctccgagcagttgtgtctgcagcccagg

SEQ ID NO: 49012 - DNA, 28 bp, synthetic construct
  source 1..28: mol_type = other DNA
ggcctgggctgcagacacaactgctcgg

SEQ ID NO: 49013 - DNA, 28 bp, synthetic construct
  source 1..28: mol_type = other DNA
gtctgcagcccaggcccagcctctcagg

SEQ ID NO: 49014 - DNA, 28 bp, synthetic construct
  source 1..28: mol_type = other DNA
gcagcccaggcccagcctctcaggatgg

SEQ ID NO: 49015 - DNA, 28 bp, synthetic construct
  source 1..28: mol_type = other DNA
cagcccaggcccagcctctcaggatggg

SEQ ID NO: 49016 - DNA, 28 bp, synthetic construct
  source 1..28: mol_type = other DNA
cccaggcccagcctctcaggatgggtgg

SEQ ID NO: 49017 - DNA, 28 bp, synthetic construct
  source 1..28: mol_type = other DNA
cccacccatcctgagaggctgggcctgg

SEQ ID NO: 49018 - DNA, 28 bp, synthetic construct
  source 1..28: mol_type = other DNA
caggcccagcctctcaggatgggtgggg

SEQ ID NO: 49019 - DNA, 28 bp, synthetic construct
  source 1..28: mol_type = other DNA
ggggccccacccatcctgagaggctggg

SEQ ID NO: 49020 - DNA, 28 bp, synthetic construct
  source 1..28: mol_type = other DNA
gggggccccacccatcctgagaggctgg

SEQ ID NO: 49021 - DNA, 28 bp, synthetic construct
  source 1..28: mol_type = other DNA
cacagggggccccacccatcctgagagg

SEQ ID NO: 49022 - DNA, 28 bp, synthetic construct
  source 1..28: mol_type = other DNA
atgggtggggccccctgtgtctgcccgg

SEQ ID NO: 49023 - DNA, 28 bp, synthetic construct
  source 1..28: mol_type = other DNA
tgggtggggccccctgtgtctgcccggg

SEQ ID NO: 49024 - DNA, 28 bp, synthetic construct
  source 1..28: mol_type = other DNA
aaggagctgcccgggcagacacaggggg

SEQ ID NO: 49025 - DNA, 28 bp, synthetic construct
  source 1..28: mol_type = other DNA
taaggagctgcccgggcagacacagggg

SEQ ID NO: 49026 - DNA, 28 bp, synthetic construct
  source 1..28: mol_type = other DNA
ataaggagctgcccgggcagacacaggg

SEQ ID NO: 49027 - DNA, 28 bp, synthetic construct
  source 1..28: mol_type = other DNA
aataaggagctgcccgggcagacacagg

SEQ ID NO: 49028 - DNA, 28 bp, synthetic construct
  source 1..28: mol_type = other DNA
tgtgtctgcccgggcagctccttattgg

SEQ ID NO: 49029 - DNA, 28 bp, synthetic construct
  source 1..28: mol_type = other DNA
gtgtctgcccgggcagctccttattggg

SEQ ID NO: 49030 - DNA, 28 bp, synthetic construct
  source 1..28: mol_type = other DNA
aatgtttcccaataaggagctgcccggg

SEQ ID NO: 49031 - DNA, 28 bp, synthetic construct
  source 1..28: mol_type = other DNA
taatgtttcccaataaggagctgcccgg

SEQ ID NO: 49032 - DNA, 28 bp, synthetic construct
  source 1..28: mol_type = other DNA
gctccttattgggaaacattagaactgg

SEQ ID NO: 49033 - DNA, 28 bp, synthetic construct
  source 1..28: mol_type = other DNA
ctccttattgggaaacattagaactggg

SEQ ID NO: 49034 - DNA, 28 bp, synthetic construct
  source 1..28: mol_type = other DNA
ggcccagttctaatgtttcccaataagg

SEQ ID NO: 49035 - DNA, 28 bp, synthetic construct
  source 1..28: mol_type = other DNA
tattgggaaacattagaactgggccagg

SEQ ID NO: 49036 - DNA, 28 bp, synthetic construct
  source 1..28: mol_type = other DNA
attgggaaacattagaactgggccaggg

SEQ ID NO: 49037 - DNA, 28 bp, synthetic construct
  source 1..28: mol_type = other DNA
atgagaggctgggaaaaatgctccctgg

SEQ ID NO: 49038 - DNA, 28 bp, synthetic construct
  source 1..28: mol_type = other DNA
agggagcatttttcccagcctctcatgg

SEQ ID NO: 49039 - DNA, 28 bp, synthetic construct
  source 1..28: mol_type = other DNA
catttttcccagcctctcatggttttgg

SEQ ID NO: 49040 - DNA, 28 bp, synthetic construct
  source 1..28: mol_type = other DNA
atttttcccagcctctcatggttttggg

SEQ ID NO: 49041 - DNA, 28 bp, synthetic construct
  source 1..28: mol_type = other DNA
gaagctcccaaaaccatgagaggctggg

SEQ ID NO: 49042 - DNA, 28 bp, synthetic construct
  source 1..28: mol_type = other DNA
agaagctcccaaaaccatgagaggctgg

SEQ ID NO: 49043 - DNA, 28 bp, synthetic construct
  source 1..28: mol_type = other DNA
ctcaagaagctcccaaaaccatgagagg

SEQ ID NO: 49044 - DNA, 28 bp, synthetic construct
  source 1..28: mol_type = other DNA
gcactgcatgtcctgccatgctaccagg

SEQ ID NO: 49045 - DNA, 28 bp, synthetic construct
  source 1..28: mol_type = other DNA
cactgcatgtcctgccatgctaccaggg

SEQ ID NO: 49046 - DNA, 28 bp, synthetic construct
  source 1..28: mol_type = other DNA
actgcatgtcctgccatgctaccagggg

SEQ ID NO: 49047 - DNA, 28 bp, synthetic construct
  source 1..28: mol_type = other DNA
gctttagtgcccctggtagcatggcagg

SEQ ID NO: 49048 - DNA, 28 bp, synthetic construct
  source 1..28: mol_type = other DNA
acatgctttagtgcccctggtagcatgg

SEQ ID NO: 49049 - DNA, 28 bp, synthetic construct
  source 1..28: mol_type = other DNA
ccaggggcactaaagcatgtgtcccagg

SEQ ID NO: 49050 - DNA, 28 bp, synthetic construct
  source 1..28: mol_type = other DNA
gcactaaagcatgtgtcccaggcccagg

SEQ ID NO: 49051 - DNA, 28 bp, synthetic construct
  source 1..28: mol_type = other DNA
cactaaagcatgtgtcccaggcccaggg

SEQ ID NO: 49052 - DNA, 28 bp, synthetic construct
  source 1..28: mol_type = other DNA
actaaagcatgtgtcccaggcccagggg

SEQ ID NO: 49053 - DNA, 28 bp, synthetic construct
  source 1..28: mol_type = other DNA
ctaaagcatgtgtcccaggcccaggggg

SEQ ID NO: 49054 - DNA, 28 bp, synthetic construct
  source 1..28: mol_type = other DNA
agaaggcaaacagccccctgggcctggg

SEQ ID NO: 49055 - DNA, 28 bp, synthetic construct
  source 1..28: mol_type = other DNA
cagaaggcaaacagccccctgggcctgg

SEQ ID NO: 49056 - DNA, 28 bp, synthetic construct
  source 1..28: mol_type = other DNA
caggcccagggggctgtttgccttctgg

SEQ ID NO: 49057 - DNA, 28 bp, synthetic construct
  source 1..28: mol_type = other DNA
aggcccagggggctgtttgccttctggg

SEQ ID NO: 49058 - DNA, 28 bp, synthetic construct
  source 1..28: mol_type = other DNA
ctgcccagaaggcaaacagccccctggg

SEQ ID NO: 49059 - DNA, 28 bp, synthetic construct
  source 1..28: mol_type = other DNA
gctgcccagaaggcaaacagccccctgg

SEQ ID NO: 49060 - DNA, 28 bp, synthetic construct
  source 1..28: mol_type = other DNA
ccttctgggcagcccagcacttagctgg

SEQ ID NO: 49061 - DNA, 28 bp, synthetic construct
  source 1..28: mol_type = other DNA
tggaaatgttcaccagctaagtgctggg

SEQ ID NO: 49062 - DNA, 28 bp, synthetic construct
  source 1..28: mol_type = other DNA
gtggaaatgttcaccagctaagtgctgg

SEQ ID NO: 49063 - DNA, 28 bp, synthetic construct
  source 1..28: mol_type = other DNA
aggaaggggctgttctgctttcaggtgg

SEQ ID NO: 49064 - DNA, 28 bp, synthetic construct
  source 1..28: mol_type = other DNA
atgaggaaggggctgttctgctttcagg

SEQ ID NO: 49065 - DNA, 28 bp, synthetic construct
  source 1..28: mol_type = other DNA
cagccccttcctcattcctgcaagcagg

SEQ ID NO: 49066 - DNA, 28 bp, synthetic construct
  source 1..28: mol_type = other DNA
aggcctgcttgcaggaatgaggaagggg

SEQ ID NO: 49067 - DNA, 28 bp, synthetic construct
  source 1..28: mol_type = other DNA
gaggcctgcttgcaggaatgaggaaggg

SEQ ID NO: 49068 - DNA, 28 bp, synthetic construct
  source 1..28: mol_type = other DNA
cgaggcctgcttgcaggaatgaggaagg

SEQ ID NO: 49069 - DNA, 28 bp, synthetic construct
  source 1..28: mol_type = other DNA
cttcctcattcctgcaagcaggcctcgg

SEQ ID NO: 49070 - DNA, 28 bp, synthetic construct
  source 1..28: mol_type = other DNA
ttcctcattcctgcaagcaggcctcggg

SEQ ID NO: 49071 - DNA, 28 bp, synthetic construct
  source 1..28: mol_type = other DNA
tcctcattcctgcaagcaggcctcgggg

SEQ ID NO: 49072 - DNA, 28 bp, synthetic construct
  source 1..28: mol_type = other DNA
tccccgaggcctgcttgcaggaatgagg

SEQ ID NO: 49073 - DNA, 28 bp, synthetic construct
  source 1..28: mol_type = other DNA
tcctgcaagcaggcctcggggagccagg

SEQ ID NO: 49074 - DNA, 28 bp, synthetic construct
  source 1..28: mol_type = other DNA
ccctggctccccgaggcctgcttgcagg

SEQ ID NO: 49075 - DNA, 28 bp, synthetic construct
  source 1..28: mol_type = other DNA
ctgcaagcaggcctcggggagccagggg

SEQ ID NO: 49076 - DNA, 28 bp, synthetic construct
  source 1..28: mol_type = other DNA
gaggaagtctgcccctggctccccgagg

SEQ ID NO: 49077 - DNA, 28 bp, synthetic construct
  source 1..28: mol_type = other DNA
agccaggggcagacttcctctttcgtgg

SEQ ID NO: 49078 - DNA, 28 bp, synthetic construct
  source 1..28: mol_type = other DNA
ttccacgaaagaggaagtctgcccctgg

SEQ ID NO: 49079 - DNA, 28 bp, synthetic construct
  source 1..28: mol_type = other DNA
tggcatcttgcagattccacgaaagagg

SEQ ID NO: 49080 - DNA, 28 bp, synthetic construct
  source 1..28: mol_type = other DNA
gaatctgcaagatgccaatgacttcagg

SEQ ID NO: 49081 - DNA, 28 bp, synthetic construct
  source 1..28: mol_type = other DNA
gcaagatgccaatgacttcaggttgagg

SEQ ID NO: 49082 - DNA, 28 bp, synthetic construct
  source 1..28: mol_type = other DNA
atgtcattcctcaacctgaagtcattgg

SEQ ID NO: 49083 - DNA, 28 bp, synthetic construct
  source 1..28: mol_type = other DNA
tggtgtgttacatcagcaaatgagtagg

SEQ ID NO: 49084 - DNA, 28 bp, synthetic construct
  source 1..28: mol_type = other DNA
tcatttgctgatgtaacacaccaccagg

SEQ ID NO: 49085 - DNA, 28 bp, synthetic construct
  source 1..28: mol_type = other DNA
gatgtaacacaccaccaggaatttctgg

SEQ ID NO: 49086 - DNA, 28 bp, synthetic construct
  source 1..28: mol_type = other DNA
ccaccaggaatttctggagatgctttgg

SEQ ID NO: 49087 - DNA, 28 bp, synthetic construct
  source 1..28: mol_type = other DNA
aaaccaaagcatctccagaaattcctgg

SEQ ID NO: 49088 - DNA, 28 bp, synthetic construct
  source 1..28: mol_type = other DNA
tttctggagatgctttggtttcacttgg

SEQ ID NO: 49089 - DNA, 28 bp, synthetic construct
  source 1..28: mol_type = other DNA
ggagatgctttggtttcacttggactgg

SEQ ID NO: 49090 - DNA, 28 bp, synthetic construct
  source 1..28: mol_type = other DNA
ggtttcacttggactggcagagcccagg

SEQ ID NO: 49091 - DNA, 28 bp, synthetic construct
  source 1..28: mol_type = other DNA
ctggcagagcccaggcttcaacccacgg

SEQ ID NO: 49092 - DNA, 28 bp, synthetic construct
  source 1..28: mol_type = other DNA
cccaggcttcaacccacggcttgcttgg

SEQ ID NO: 49093 - DNA, 28 bp, synthetic construct
  source 1..28: mol_type = other DNA
tccaagcaagccgtgggttgaagcctgg

SEQ ID NO: 49094 - DNA, 28 bp, synthetic construct
  source 1..28: mol_type = other DNA
cttcaacccacggcttgcttggacaagg

SEQ ID NO: 49095 - DNA, 28 bp, synthetic construct
  source 1..28: mol_type = other DNA
aggagtccttgtccaagcaagccgtggg

SEQ ID NO: 49096 - DNA, 28 bp, synthetic construct
  source 1..28: mol_type = other DNA
aaggagtccttgtccaagcaagccgtgg

SEQ ID NO: 49097 - DNA, 28 bp, synthetic construct
  source 1..28: mol_type = other DNA
ctcaaagaaataaatcaggcacataagg

SEQ ID NO: 49098 - DNA, 28 bp, synthetic construct
  source 1..28: mol_type = other DNA
aaactgaggctcaaagaaataaatcagg

SEQ ID NO: 49099 - DNA, 28 bp, synthetic construct
  source 1..28: mol_type = other DNA
agcctcagtttgcccatctattaaatgg

SEQ ID NO: 49100 - DNA, 28 bp, synthetic construct
  source 1..28: mol_type = other DNA
gcctcagtttgcccatctattaaatggg

SEQ ID NO: 49101 - DNA, 28 bp, synthetic construct
  source 1..28: mol_type = other DNA
tcccatttaatagatgggcaaactgagg

SEQ ID NO: 49102 - DNA, 28 bp, synthetic construct
  source 1..28: mol_type = other DNA
gcccatctattaaatgggacatcatagg

SEQ ID NO: 49103 - DNA, 28 bp, synthetic construct
  source 1..28: mol_type = other DNA
acctatgatgtcccatttaatagatggg

SEQ ID NO: 49104 - DNA, 28 bp, synthetic construct
  source 1..28: mol_type = other DNA
aacctatgatgtcccatttaatagatgg

SEQ ID NO: 49105 - DNA, 28 bp, synthetic construct
  source 1..28: mol_type = other DNA
aatgggacatcataggtttaccaagagg

SEQ ID NO: 49106 - DNA, 28 bp, synthetic construct
  source 1..28: mol_type = other DNA
taccaagaggcttcaattcagcaaaagg

SEQ ID NO: 49107 - DNA, 28 bp, synthetic construct
  source 1..28: mol_type = other DNA
gaccttttgctgaattgaagcctcttgg

SEQ ID NO: 49108 - DNA, 28 bp, synthetic construct
  source 1..28: mol_type = other DNA
gtcttagagtctctctctctttcccagg

SEQ ID NO: 49109 - DNA, 28 bp, synthetic construct
  source 1..28: mol_type = other DNA
tagagtctctctctctttcccaggctgg

SEQ ID NO: 49110 - DNA, 28 bp, synthetic construct
  source 1..28: mol_type = other DNA
ctctctttcccaggctggagtgcagtgg

SEQ ID NO: 49111 - DNA, 28 bp, synthetic construct
  source 1..28: mol_type = other DNA
agatcttgccactgcactccagcctggg

SEQ ID NO: 49112 - DNA, 28 bp, synthetic construct
  source 1..28: mol_type = other DNA
gagatcttgccactgcactccagcctgg

SEQ ID NO: 49113 - DNA, 28 bp, synthetic construct
  source 1..28: mol_type = other DNA
aggctggagtgcagtggcaagatctcgg

SEQ ID NO: 49114 - DNA, 28 bp, synthetic construct
  source 1..28: mol_type = other DNA
ctcactgcaagctccctccacctcctgg

SEQ ID NO: 49115 - DNA, 28 bp, synthetic construct
  source 1..28: mol_type = other DNA
tcactgcaagctccctccacctcctggg

SEQ ID NO: 49116 - DNA, 28 bp, synthetic construct
  source 1..28: mol_type = other DNA
gaatcgctggaacccaggaggtggaggg

SEQ ID NO: 49117 - DNA, 28 bp, synthetic construct
  source 1..28: mol_type = other DNA
agaatcgctggaacccaggaggtggagg

SEQ ID NO: 49118 - DNA, 28 bp, synthetic construct
  source 1..28: mol_type = other DNA
aggagaatcgctggaacccaggaggtgg

SEQ ID NO: 49119 - DNA, 28 bp, synthetic construct
  source 1..28: mol_type = other DNA
tgcaggagaatcgctggaacccaggagg

SEQ ID NO: 49120 - DNA, 28 bp, synthetic construct
  source 1..28: mol_type = other DNA
tgatgcaggagaatcgctggaacccagg

SEQ ID NO: 49121 - DNA, 28 bp, synthetic construct
  source 1..28: mol_type = other DNA
agctgggctgatgcaggagaatcgctgg

SEQ ID NO: 49122 - DNA, 28 bp, synthetic construct
  source 1..28: mol_type = other DNA
attctcctgcatcagcccagcttcctgg

SEQ ID NO: 49123 - DNA, 28 bp, synthetic construct
  source 1..28: mol_type = other DNA
ttctcctgcatcagcccagcttcctggg

SEQ ID NO: 49124 - DNA, 28 bp, synthetic construct
  source 1..28: mol_type = other DNA
actgcccaggaagctgggctgatgcagg

SEQ ID NO: 49125 - DNA, 28 bp, synthetic construct
  source 1..28: mol_type = other DNA
gcatcagcccagcttcctgggcagttgg

SEQ ID NO: 49126 - DNA, 28 bp, synthetic construct
  source 1..28: mol_type = other DNA
catcagcccagcttcctgggcagttggg

SEQ ID NO: 49127 - DNA, 28 bp, synthetic construct
  source 1..28: mol_type = other DNA
tgtaatcccaactgcccaggaagctggg

SEQ ID NO: 49128 - DNA, 28 bp, synthetic construct
  source 1..28: mol_type = other DNA
ctgtaatcccaactgcccaggaagctgg

SEQ ID NO: 49129 - DNA, 28 bp, synthetic construct
  source 1..28: mol_type = other DNA
tgagtgactgtaatcccaactgcccagg

SEQ ID NO: 49130 - DNA, 28 bp, synthetic construct
  source 1..28: mol_type = other DNA
gattacagtcactcaccaccacgcctgg

SEQ ID NO: 49131 - DNA, 28 bp, synthetic construct
  source 1..28: mol_type = other DNA
atacaaaacaattagccaggcgtggtgg

SEQ ID NO: 49132 - DNA, 28 bp, synthetic construct
  source 1..28: mol_type = other DNA
aaaatacaaaacaattagccaggcgtgg

SEQ ID NO: 49133 - DNA, 28 bp, synthetic construct
  source 1..28: mol_type = other DNA
tactaaaaatacaaaacaattagccagg

SEQ ID NO: 49134 - DNA, 28 bp, synthetic construct
  source 1..28: mol_type = other DNA
aattgttttgtatttttagtagagatgg

SEQ ID NO: 49135 - DNA, 28 bp, synthetic construct
  source 1..28: mol_type = other DNA
attgttttgtatttttagtagagatggg

SEQ ID NO: 49136 - DNA, 28 bp, synthetic construct
  source 1..28: mol_type = other DNA
ttgttttgtatttttagtagagatgggg

SEQ ID NO: 49137 - DNA, 28 bp, synthetic construct
  source 1..28: mol_type = other DNA
tcaccatgttagccagtctgatccgagg

SEQ ID NO: 49138 - DNA, 28 bp, synthetic construct
  source 1..28: mol_type = other DNA
tcacctcggatcagactggctaacatgg

SEQ ID NO: 49139 - DNA, 28 bp, synthetic construct
  source 1..28: mol_type = other DNA
gtgggcggatcacctcggatcagactgg

SEQ ID NO: 49140 - DNA, 28 bp, synthetic construct
  source 1..28: mol_type = other DNA
ctgatccgaggtgatccgcccacttcgg

SEQ ID NO: 49141 - DNA, 28 bp, synthetic construct
  source 1..28: mol_type = other DNA
ggaggccgaagtgggcggatcacctcgg

SEQ ID NO: 49142 - DNA, 28 bp, synthetic construct
  source 1..28: mol_type = other DNA
caacatttcgggaggccgaagtgggcgg

SEQ ID NO: 49143 - DNA, 28 bp, synthetic construct
  source 1..28: mol_type = other DNA
cgcccacttcggcctcccgaaatgttgg

SEQ ID NO: 49144 - DNA, 28 bp, synthetic construct
  source 1..28: mol_type = other DNA
gcccacttcggcctcccgaaatgttggg

SEQ ID NO: 49145 - DNA, 28 bp, synthetic construct
  source 1..28: mol_type = other DNA
tcccaacatttcgggaggccgaagtggg

SEQ ID NO: 49146 - DNA, 28 bp, synthetic construct
  source 1..28: mol_type = other DNA
atcccaacatttcgggaggccgaagtgg

SEQ ID NO: 49147 - DNA, 28 bp, synthetic construct
  source 1..28: mol_type = other DNA
cggcctcccgaaatgttgggattacagg

SEQ ID NO: 49148 - DNA, 28 bp, synthetic construct
  source 1..28: mol_type = other DNA
acacctgtaatcccaacatttcgggagg

SEQ ID NO: 49149 - DNA, 28 bp, synthetic construct
  source 1..28: mol_type = other DNA
ctcacacctgtaatcccaacatttcggg

SEQ ID NO: 49150 - DNA, 28 bp, synthetic construct
  source 1..28: mol_type = other DNA
gctcacacctgtaatcccaacatttcgg

SEQ ID NO: 49151 - DNA, 28 bp, synthetic construct
  source 1..28: mol_type = other DNA
gattacaggtgtgagcctccgtgcctgg

SEQ ID NO: 49152 - DNA, 28 bp, synthetic construct
  source 1..28: mol_type = other DNA
taaaatttatttaggccaggcacggagg

SEQ ID NO: 49153 - DNA, 28 bp, synthetic construct
  source 1..28: mol_type = other DNA
ttataaaatttatttaggccaggcacgg

SEQ ID NO: 49154 - DNA, 28 bp, synthetic construct
  source 1..28: mol_type = other DNA
aacatttataaaatttatttaggccagg

SEQ ID NO: 49155 - DNA, 28 bp, synthetic construct
  source 1..28: mol_type = other DNA
aaactaacatttataaaatttatttagg

SEQ ID NO: 49156 - DNA, 28 bp, synthetic construct
  source 1..28: mol_type = other DNA
ttttataaatgttagttttaaaaaatgg

SEQ ID NO: 49157 - DNA, 28 bp, synthetic construct
  source 1..28: mol_type = other DNA
aaaaaatggctaataagcacattgtagg

SEQ ID NO: 49158 - DNA, 28 bp, synthetic construct
  source 1..28: mol_type = other DNA
attctaatatcagattgaccagaagtgg

SEQ ID NO: 49159 - DNA, 28 bp, synthetic construct
  source 1..28: mol_type = other DNA
ttttagcacagcacttttccacttctgg

SEQ ID NO: 49160 - DNA, 28 bp, synthetic construct
  source 1..28: mol_type = other DNA
aagtggaaaagtgctgtgctaaaagtgg

SEQ ID NO: 49161 - DNA, 28 bp, synthetic construct
  source 1..28: mol_type = other DNA
agtggaaaagtgctgtgctaaaagtggg

SEQ ID NO: 49162 - DNA, 28 bp, synthetic construct
  source 1..28: mol_type = other DNA
agtgctgtgctaaaagtgggatgatcgg

SEQ ID NO: 49163 - DNA, 28 bp, synthetic construct
  source 1..28: mol_type = other DNA
gtgctgtgctaaaagtgggatgatcggg

SEQ ID NO: 49164 - DNA, 28 bp, synthetic construct
  source 1..28: mol_type = other DNA
ctgtgctaaaagtgggatgatcgggagg

SEQ ID NO: 49165 - DNA, 28 bp, synthetic construct
  source 1..28: mol_type = other DNA
tcgggaggctctgagcactccgtgaagg

SEQ ID NO: 49166 - DNA, 28 bp, synthetic construct
  source 1..28: mol_type = other DNA
ctacatggagtctcacggtccttcacgg

SEQ ID NO: 49167 - DNA, 28 bp, synthetic construct
  source 1..28: mol_type = other DNA
tgaaggaccgtgagactccatgtagcgg

SEQ ID NO: 49168 - DNA, 28 bp, synthetic construct
  source 1..28: mol_type = other DNA
gaaggaccgtgagactccatgtagcggg

SEQ ID NO: 49169 - DNA, 28 bp, synthetic construct
  source 1..28: mol_type = other DNA
ggaccgtgagactccatgtagcgggagg

SEQ ID NO: 49170 - DNA, 28 bp, synthetic construct
  source 1..28: mol_type = other DNA
attcctcccgctacatggagtctcacgg

SEQ ID NO: 49171 - DNA, 28 bp, synthetic construct
  source 1..28: mol_type = other DNA
gtgagactccatgtagcgggaggaatgg

SEQ ID NO: 49172 - DNA, 28 bp, synthetic construct
  source 1..28: mol_type = other DNA
actccatgtagcgggaggaatggcctgg

SEQ ID NO: 49173 - DNA, 28 bp, synthetic construct
  source 1..28: mol_type = other DNA
cctccaggccattcctcccgctacatgg

SEQ ID NO: 49174 - DNA, 28 bp, synthetic construct
  source 1..28: mol_type = other DNA
tgtagcgggaggaatggcctggaggagg

SEQ ID NO: 49175 - DNA, 28 bp, synthetic construct
  source 1..28: mol_type = other DNA
gtagcgggaggaatggcctggaggaggg

SEQ ID NO: 49176 - DNA, 28 bp, synthetic construct
  source 1..28: mol_type = other DNA
aggaatggcctggaggagggctgtgtgg

SEQ ID NO: 49177 - DNA, 28 bp, synthetic construct
  source 1..28: mol_type = other DNA
ggaatggcctggaggagggctgtgtggg

SEQ ID NO: 49178 - DNA, 28 bp, synthetic construct
  source 1..28: mol_type = other DNA
aaaaaagcccacacagccctcctccagg

SEQ ID NO: 49179 - DNA, 28 bp, synthetic construct
  source 1..28: mol_type = other DNA
ttttcctcctcacaccagccagttctgg

SEQ ID NO: 49180 - DNA, 28 bp, synthetic construct
  source 1..28: mol_type = other DNA
ggtgccagaactggctggtgtgaggagg

SEQ ID NO: 49181 - DNA, 28 bp, synthetic construct
  source 1..28: mol_type = other DNA
gttggtgccagaactggctggtgtgagg

SEQ ID NO: 49182 - DNA, 28 bp, synthetic construct
  source 1..28: mol_type = other DNA
ctagagagttggtgccagaactggctgg

SEQ ID NO: 49183 - DNA, 28 bp, synthetic construct
  source 1..28: mol_type = other DNA
gtgtctagagagttggtgccagaactgg

SEQ ID NO: 49184 - DNA, 28 bp, synthetic construct
  source 1..28: mol_type = other DNA
tggcaccaactctctagacaccaactgg

SEQ ID NO: 49185 - DNA, 28 bp, synthetic construct
  source 1..28: mol_type = other DNA
ggacaccagttggtgtctagagagttgg

SEQ ID NO: 49186 - DNA, 28 bp, synthetic construct
  source 1..28: mol_type = other DNA
cagaattgcactgtaggacaccagttgg

SEQ ID NO: 49187 - DNA, 28 bp, synthetic construct
  source 1..28: mol_type = other DNA
gcagtcagtgtcagaattgcactgtagg

SEQ ID NO: 49188 - DNA, 28 bp, synthetic construct
  source 1..28: mol_type = other DNA
cagtgcaattctgacactgactgcctgg

SEQ ID NO: 49189 - DNA, 28 bp, synthetic construct
  source 1..28: mol_type = other DNA
aattctgacactgactgcctggagttgg

SEQ ID NO: 49190 - DNA, 28 bp, synthetic construct
  source 1..28: mol_type = other DNA
gcctggagttggcatcaaacctcacagg

SEQ ID NO: 49191 - DNA, 28 bp, synthetic construct
  source 1..28: mol_type = other DNA
acctgtgaggtttgatgccaactccagg

SEQ ID NO: 49192 - DNA, 28 bp, synthetic construct
  source 1..28: mol_type = other DNA
agttggcatcaaacctcacaggtttagg

SEQ ID NO: 49193 - DNA, 28 bp, synthetic construct
  source 1..28: mol_type = other DNA
gttggcatcaaacctcacaggtttaggg

SEQ ID NO: 49194 - DNA, 28 bp, synthetic construct
  source 1..28: mol_type = other DNA
tcttcactgaaaccctaaacctgtgagg

SEQ ID NO: 49195 - DNA, 28 bp, synthetic construct
  source 1..28: mol_type = other DNA
caggtttagggtttcagtgaagagctgg

SEQ ID NO: 49196 - DNA, 28 bp, synthetic construct
  source 1..28: mol_type = other DNA
ccatttgcaactggcatctgatatgagg

SEQ ID NO: 49197 - DNA, 28 bp, synthetic construct
  source 1..28: mol_type = other DNA
ctcatatcagatgccagttgcaaatggg

SEQ ID NO: 49198 - DNA, 28 bp, synthetic construct
  source 1..28: mol_type = other DNA
tcatatcagatgccagttgcaaatgggg

SEQ ID NO: 49199 - DNA, 28 bp, synthetic construct
  source 1..28: mol_type = other DNA
gtggtctgggcaccccatttgcaactgg

SEQ ID NO: 49200 - DNA, 28 bp, synthetic construct
  source 1..28: mol_type = other DNA
gttgcaaatggggtgcccagaccactgg

SEQ ID NO: 49201 - DNA, 28 bp, synthetic construct
  source 1..28: mol_type = other DNA
agtcagacagagatgccagtggtctggg

SEQ ID NO: 49202 - DNA, 28 bp, synthetic construct
  source 1..28: mol_type = other DNA
aagtcagacagagatgccagtggtctgg

SEQ ID NO: 49203 - DNA, 28 bp, synthetic construct
  source 1..28: mol_type = other DNA
tcaccaagtcagacagagatgccagtgg

SEQ ID NO: 49204 - DNA, 28 bp, synthetic construct
  source 1..28: mol_type = other DNA
cacctgcctcagcctcccaaagtcctgg

SEQ ID NO: 49205 - DNA, 28 bp, synthetic construct
  source 1..28: mol_type = other DNA
acctgcctcagcctcccaaagtcctggg

SEQ ID NO: 49206 - DNA, 28 bp, synthetic construct
  source 1..28: mol_type = other DNA
cagcctcccaaagtcctgggattacagg

SEQ ID NO: 49207 - DNA, 28 bp, synthetic construct
  source 1..28: mol_type = other DNA
gattacaggcatgagccaccctgtctgg

SEQ ID NO: 49208 - DNA, 28 bp, synthetic construct
  source 1..28: mol_type = other DNA
taaacaaataaaaggccagacagggtgg

SEQ ID NO: 49209 - DNA, 28 bp, synthetic construct
  source 1..28: mol_type = other DNA
aaataaacaaataaaaggccagacaggg

SEQ ID NO: 49210 - DNA, 28 bp, synthetic construct
  source 1..28: mol_type = other DNA
taaataaacaaataaaaggccagacagg

SEQ ID NO: 49211 - DNA, 28 bp, synthetic construct
  source 1..28: mol_type = other DNA
aaataaaaataaataaacaaataaaagg

SEQ ID NO: 49212 - DNA, 28 bp, synthetic construct
  source 1..28: mol_type = other DNA
atttttatttatttatttatttttgagg

SEQ ID NO: 49213 - DNA, 28 bp, synthetic construct
  source 1..28: mol_type = other DNA
tagatagacatggagaggcattgcgtgg

SEQ ID NO: 49214 - DNA, 28 bp, synthetic construct
  source 1..28: mol_type = other DNA
ggaactggggtagatagacatggagagg

SEQ ID NO: 49215 - DNA, 28 bp, synthetic construct
  source 1..28: mol_type = other DNA
agtcgggaactggggtagatagacatgg

SEQ ID NO: 49216 - DNA, 28 bp, synthetic construct
  source 1..28: mol_type = other DNA
atgtggtgctaggagtcgggaactgggg

SEQ ID NO: 49217 - DNA, 28 bp, synthetic construct
  source 1..28: mol_type = other DNA
gatgtggtgctaggagtcgggaactggg

SEQ ID NO: 49218 - DNA, 28 bp, synthetic construct
  source 1..28: mol_type = other DNA
agatgtggtgctaggagtcgggaactgg

SEQ ID NO: 49219 - DNA, 28 bp, synthetic construct
  source 1..28: mol_type = other DNA
agttcccgactcctagcaccacatctgg

SEQ ID NO: 49220 - DNA, 28 bp, synthetic construct
  source 1..28: mol_type = other DNA
tgtgccagatgtggtgctaggagtcggg

SEQ ID NO: 49221 - DNA, 28 bp, synthetic construct
  source 1..28: mol_type = other DNA
atgtgccagatgtggtgctaggagtcgg

SEQ ID NO: 49222 - DNA, 28 bp, synthetic construct
  source 1..28: mol_type = other DNA
cctagcaccacatctggcacatcatagg

SEQ ID NO: 49223 - DNA, 28 bp, synthetic construct
  source 1..28: mol_type = other DNA
agcaccacatctggcacatcataggtgg

SEQ ID NO: 49224 - DNA, 28 bp, synthetic construct
  source 1..28: mol_type = other DNA
ctgaccacctatgatgtgccagatgtgg

SEQ ID NO: 49225 - DNA, 28 bp, synthetic construct
  source 1..28: mol_type = other DNA
cacatcataggtggtcagcatttattgg

SEQ ID NO: 49226 - DNA, 28 bp, synthetic construct
  source 1..28: mol_type = other DNA
ggtcagcatttattggatgaatgaatgg

SEQ ID NO: 49227 - DNA, 28 bp, synthetic construct
  source 1..28: mol_type = other DNA
tgagtcttgaagtacgaatagaatttgg

SEQ ID NO: 49228 - DNA, 28 bp, synthetic construct
  source 1..28: mol_type = other DNA
gaagtacgaatagaatttggcgaagtgg

SEQ ID NO: 49229 - DNA, 28 bp, synthetic construct
  source 1..28: mol_type = other DNA
cgaatagaatttggcgaagtggacaagg

SEQ ID NO: 49230 - DNA, 28 bp, synthetic construct
  source 1..28: mol_type = other DNA
tagaatttggcgaagtggacaaggcagg

SEQ ID NO: 49231 - DNA, 28 bp, synthetic construct
  source 1..28: mol_type = other DNA
tggacaaggcaggaaatgtgtattcagg

SEQ ID NO: 49232 - DNA, 28 bp, synthetic construct
  source 1..28: mol_type = other DNA
ggcaggaaatgtgtattcaggcatgagg

SEQ ID NO: 49233 - DNA, 28 bp, synthetic construct
  source 1..28: mol_type = other DNA
caggcatgaggcttagcttgtgcatagg

SEQ ID NO: 49234 - DNA, 28 bp, synthetic construct
  source 1..28: mol_type = other DNA
aggcttagcttgtgcataggtagaaagg

SEQ ID NO: 49235 - DNA, 28 bp, synthetic construct
  source 1..28: mol_type = other DNA
ataggtagaaaggcatgaaaaaacatgg

SEQ ID NO: 49236 - DNA, 28 bp, synthetic construct
  source 1..28: mol_type = other DNA
ttctcgaatccacaaatagtaagagagg

SEQ ID NO: 49237 - DNA, 28 bp, synthetic construct
  source 1..28: mol_type = other DNA
tctcgaatccacaaatagtaagagaggg

SEQ ID NO: 49238 - DNA, 28 bp, synthetic construct
  source 1..28: mol_type = other DNA
cgacttagccctctcttactatttgtgg

SEQ ID NO: 49239 - DNA, 28 bp, synthetic construct
  source 1..28: mol_type = other DNA
agtaagagagggctaagtcgttgtgtgg

SEQ ID NO: 49240 - DNA, 28 bp, synthetic construct
  source 1..28: mol_type = other DNA
gtaagagagggctaagtcgttgtgtggg

SEQ ID NO: 49241 - DNA, 28 bp, synthetic construct
  source 1..28: mol_type = other DNA
taagagagggctaagtcgttgtgtgggg

SEQ ID NO: 49242 - DNA, 28 bp, synthetic construct
  source 1..28: mol_type = other DNA
aagagagggctaagtcgttgtgtggggg

SEQ ID NO: 49243 - DNA, 28 bp, synthetic construct
  source 1..28: mol_type = other DNA
agggctaagtcgttgtgtgggggagagg

SEQ ID NO: 49244 - DNA, 28 bp, synthetic construct
  source 1..28: mol_type = other DNA
ggggagaggagaaatgaagttcaaatgg

SEQ ID NO: 49245 - DNA, 28 bp, synthetic construct
  source 1..28: mol_type = other DNA
agaggagaaatgaagttcaaatggtagg

SEQ ID NO: 49246 - DNA, 28 bp, synthetic construct
  source 1..28: mol_type = other DNA
gaaatgaagttcaaatggtaggcaaagg

SEQ ID NO: 49247 - DNA, 28 bp, synthetic construct
  source 1..28: mol_type = other DNA
agttcaaatggtaggcaaaggtcagtgg

SEQ ID NO: 49248 - DNA, 28 bp, synthetic construct
  source 1..28: mol_type = other DNA
gttcaaatggtaggcaaaggtcagtggg

SEQ ID NO: 49249 - DNA, 28 bp, synthetic construct
  source 1..28: mol_type = other DNA
aatggtaggcaaaggtcagtgggcaagg

SEQ ID NO: 49250 - DNA, 28 bp, synthetic construct
  source 1..28: mol_type = other DNA
atggtaggcaaaggtcagtgggcaaggg

SEQ ID NO: 49251 - DNA, 28 bp, synthetic construct
  source 1..28: mol_type = other DNA
gaataaaattcaagtgcaatttacaagg

SEQ ID NO: 49252 - DNA, 28 bp, synthetic construct
  source 1..28: mol_type = other DNA
aaattgcacttgaattttattctttagg

SEQ ID NO: 49253 - DNA, 28 bp, synthetic construct
  source 1..28: mol_type = other DNA
acttgaattttattctttaggcaaaagg

SEQ ID NO: 49254 - DNA, 28 bp, synthetic construct
  source 1..28: mol_type = other DNA
ttctttaggcaaaaggaagagtttaagg

SEQ ID NO: 49255 - DNA, 28 bp, synthetic construct
  source 1..28: mol_type = other DNA
tctttaggcaaaaggaagagtttaaggg

SEQ ID NO: 49256 - DNA, 28 bp, synthetic construct
  source 1..28: mol_type = other DNA
gaagagtttaagggtttcaagaagaagg

SEQ ID NO: 49257 - DNA, 28 bp, synthetic construct
  source 1..28: mol_type = other DNA
gtttcaagaagaaggacacgaccagtgg

SEQ ID NO: 49258 - DNA, 28 bp, synthetic construct
  source 1..28: mol_type = other DNA
tttcaagaagaaggacacgaccagtggg

SEQ ID NO: 49259 - DNA, 28 bp, synthetic construct
  source 1..28: mol_type = other DNA
aagaaggacacgaccagtgggttttagg

SEQ ID NO: 49260 - DNA, 28 bp, synthetic construct
  source 1..28: mol_type = other DNA
tcagaatgatcttcctaaaacccactgg

SEQ ID NO: 49261 - DNA, 28 bp, synthetic construct
  source 1..28: mol_type = other DNA
gtgggttttaggaagatcattctgatgg

SEQ ID NO: 49262 - DNA, 28 bp, synthetic construct
  source 1..28: mol_type = other DNA
gaagatcattctgatggcctttcagagg

SEQ ID NO: 49263 - DNA, 28 bp, synthetic construct
  source 1..28: mol_type = other DNA
atcattctgatggcctttcagaggatgg

SEQ ID NO: 49264 - DNA, 28 bp, synthetic construct
  source 1..28: mol_type = other DNA
ctgatggcctttcagaggatggctgagg

SEQ ID NO: 49265 - DNA, 28 bp, synthetic construct
  source 1..28: mol_type = other DNA
tagctctcctcagccatcctctgaaagg

SEQ ID NO: 49266 - DNA, 28 bp, synthetic construct
  source 1..28: mol_type = other DNA
cagaggatggctgaggagagctagcagg

SEQ ID NO: 49267 - DNA, 28 bp, synthetic construct
  source 1..28: mol_type = other DNA
agaggatggctgaggagagctagcaggg

SEQ ID NO: 49268 - DNA, 28 bp, synthetic construct
  source 1..28: mol_type = other DNA
ggatggctgaggagagctagcagggagg

SEQ ID NO: 49269 - DNA, 28 bp, synthetic construct
  source 1..28: mol_type = other DNA
ggctgaggagagctagcagggaggcagg

SEQ ID NO: 49270 - DNA, 28 bp, synthetic construct
  source 1..28: mol_type = other DNA
gctgaggagagctagcagggaggcaggg

SEQ ID NO: 49271 - DNA, 28 bp, synthetic construct
  source 1..28: mol_type = other DNA
gaggagagctagcagggaggcagggagg

SEQ ID NO: 49272 - DNA, 28 bp, synthetic construct
  source 1..28: mol_type = other DNA
agcagggaggcagggaggtcgagtcagg

SEQ ID NO: 49273 - DNA, 28 bp, synthetic construct
  source 1..28: mol_type = other DNA
gcagggaggcagggaggtcgagtcaggg

SEQ ID NO: 49274 - DNA, 28 bp, synthetic construct
  source 1..28: mol_type = other DNA
cagggaggcagggaggtcgagtcagggg

SEQ ID NO: 49275 - DNA, 28 bp, synthetic construct
  source 1..28: mol_type = other DNA
gaggtcgagtcaggggattttgaccagg

SEQ ID NO: 49276 - DNA, 28 bp, synthetic construct
  source 1..28: mol_type = other DNA
cgagtcaggggattttgaccaggccagg

SEQ ID NO: 49277 - DNA, 28 bp, synthetic construct
  source 1..28: mol_type = other DNA
caggggattttgaccaggccaggttagg

SEQ ID NO: 49278 - DNA, 28 bp, synthetic construct
  source 1..28: mol_type = other DNA
tgaccaggccaggttaggtgctatgagg

SEQ ID NO: 49279 - DNA, 28 bp, synthetic construct
  source 1..28: mol_type = other DNA
gggcctcatagcacctaacctggcctgg

SEQ ID NO: 49280 - DNA, 28 bp, synthetic construct
  source 1..28: mol_type = other DNA
aggccaggttaggtgctatgaggcccgg

SEQ ID NO: 49281 - DNA, 28 bp, synthetic construct
  source 1..28: mol_type = other DNA
ggccaggttaggtgctatgaggcccggg

SEQ ID NO: 49282 - DNA, 28 bp, synthetic construct
  source 1..28: mol_type = other DNA
agcccgggcctcatagcacctaacctgg

SEQ ID NO: 49283 - DNA, 28 bp, synthetic construct
  source 1..28: mol_type = other DNA
gttaggtgctatgaggcccgggctttgg

SEQ ID NO: 49284 - DNA, 28 bp, synthetic construct
  source 1..28: mol_type = other DNA
gaggcccgggctttggagaagaaccagg

SEQ ID NO: 49285 - DNA, 28 bp, synthetic construct
  source 1..28: mol_type = other DNA
atttcctggttcttctccaaagcccggg

SEQ ID NO: 49286 - DNA, 28 bp, synthetic construct
  source 1..28: mol_type = other DNA
catttcctggttcttctccaaagcccgg

SEQ ID NO: 49287 - DNA, 28 bp, synthetic construct
  source 1..28: mol_type = other DNA
cgggctttggagaagaaccaggaaatgg

SEQ ID NO: 49288 - DNA, 28 bp, synthetic construct
  source 1..28: mol_type = other DNA
tggagaagaaccaggaaatggcaactgg

SEQ ID NO: 49289 - DNA, 28 bp, synthetic construct
  source 1..28: mol_type = other DNA
agaagaaccaggaaatggcaactggagg

SEQ ID NO: 49290 - DNA, 28 bp, synthetic construct
  source 1..28: mol_type = other DNA
tttcttgcctccagttgccatttcctgg

SEQ ID NO: 49291 - DNA, 28 bp, synthetic construct
  source 1..28: mol_type = other DNA
aggaaatggcaactggaggcaagaaagg

SEQ ID NO: 49292 - DNA, 28 bp, synthetic construct
  source 1..28: mol_type = other DNA
ggaaatggcaactggaggcaagaaaggg

SEQ ID NO: 49293 - DNA, 28 bp, synthetic construct
  source 1..28: mol_type = other DNA
gaaatggcaactggaggcaagaaagggg

SEQ ID NO: 49294 - DNA, 28 bp, synthetic construct
  source 1..28: mol_type = other DNA
gcaactggaggcaagaaaggggagaagg

SEQ ID NO: 49295 - DNA, 28 bp, synthetic construct
  source 1..28: mol_type = other DNA
caagaaaggggagaaggccaaagcctgg

SEQ ID NO: 49296 - DNA, 28 bp, synthetic construct
  source 1..28: mol_type = other DNA
aagaaaggggagaaggccaaagcctggg

SEQ ID NO: 49297 - DNA, 28 bp, synthetic construct
  source 1..28: mol_type = other DNA
ttaagtgttgatggttcccaggctttgg

SEQ ID NO: 49298 - DNA, 28 bp, synthetic construct
  source 1..28: mol_type = other DNA
ctgttcttaagtgttgatggttcccagg

SEQ ID NO: 49299 - DNA, 28 bp, synthetic construct
  source 1..28: mol_type = other DNA
attctttactgttcttaagtgttgatgg

SEQ ID NO: 49300 - DNA, 28 bp, synthetic construct
  source 1..28: mol_type = other DNA
gaataaacatctaaagagaacaagaagg

SEQ ID NO: 49301 - DNA, 28 bp, synthetic construct
  source 1..28: mol_type = other DNA
aacatctaaagagaacaagaaggaatgg

SEQ ID NO: 49302 - DNA, 28 bp, synthetic construct
  source 1..28: mol_type = other DNA
agaacaagaaggaatggccagaagaagg

SEQ ID NO: 49303 - DNA, 28 bp, synthetic construct
  source 1..28: mol_type = other DNA
aaggaatggccagaagaaggaaaacagg

SEQ ID NO: 49304 - DNA, 28 bp, synthetic construct
  source 1..28: mol_type = other DNA
cagttctttcctgttttccttcttctgg

SEQ ID NO: 49305 - DNA, 28 bp, synthetic construct
  source 1..28: mol_type = other DNA
gaagaaggaaaacaggaaagaactgagg

SEQ ID NO: 49306 - DNA, 28 bp, synthetic construct
  source 1..28: mol_type = other DNA
aggaaaacaggaaagaactgaggcgtgg

SEQ ID NO: 49307 - DNA, 28 bp, synthetic construct
  source 1..28: mol_type = other DNA
ggaaaacaggaaagaactgaggcgtggg

SEQ ID NO: 49308 - DNA, 28 bp, synthetic construct
  source 1..28: mol_type = other DNA
aggcgtgggagcgcaagagagagaatgg

SEQ ID NO: 49309 - DNA, 28 bp, synthetic construct
  source 1..28: mol_type = other DNA
gcgcaagagagagaatggttcgagaagg

SEQ ID NO: 49310 - DNA, 28 bp, synthetic construct
  source 1..28: mol_type = other DNA
aatggttcgagaaggaagcagtcacagg

SEQ ID NO: 49311 - DNA, 28 bp, synthetic construct
  source 1..28: mol_type = other DNA
gagaaggaagcagtcacaggtgtcaagg

SEQ ID NO: 49312 - DNA, 28 bp, synthetic construct
  source 1..28: mol_type = other DNA
aagcagtcacaggtgtcaaggccattgg

SEQ ID NO: 49313 - DNA, 28 bp, synthetic construct
  source 1..28: mol_type = other DNA
agcagtcacaggtgtcaaggccattggg

SEQ ID NO: 49314 - DNA, 28 bp, synthetic construct
  source 1..28: mol_type = other DNA
agtcacaggtgtcaaggccattgggagg

SEQ ID NO: 49315 - DNA, 28 bp, synthetic construct
  source 1..28: mol_type = other DNA
ggccattgggaggtcaagtgagataagg

SEQ ID NO: 49316 - DNA, 28 bp, synthetic construct
  source 1..28: mol_type = other DNA
gtccttatctcacttgacctcccaatgg

SEQ ID NO: 49317 - DNA, 28 bp, synthetic construct
  source 1..28: mol_type = other DNA
ggaggtcaagtgagataaggactgaagg

SEQ ID NO: 49318 - DNA, 28 bp, synthetic construct
  source 1..28: mol_type = other DNA
gataaggactgaaggtcccaccaattgg

SEQ ID NO: 49319 - DNA, 28 bp, synthetic construct
  source 1..28: mol_type = other DNA
ataaggactgaaggtcccaccaattggg

SEQ ID NO: 49320 - DNA, 28 bp, synthetic construct
  source 1..28: mol_type = other DNA
tgaaggtcccaccaattgggccatcagg

SEQ ID NO: 49321 - DNA, 28 bp, synthetic construct
  source 1..28: mol_type = other DNA
ctgtgctcctgatggcccaattggtggg

SEQ ID NO: 49322 - DNA, 28 bp, synthetic construct
  source 1..28: mol_type = other DNA
cctgtgctcctgatggcccaattggtgg

SEQ ID NO: 49323 - DNA, 28 bp, synthetic construct
  source 1..28: mol_type = other DNA
agtcctgtgctcctgatggcccaattgg

SEQ ID NO: 49324 - DNA, 28 bp, synthetic construct
  source 1..28: mol_type = other DNA
gtgctctcaagtcctgtgctcctgatgg

SEQ ID NO: 49325 - DNA, 28 bp, synthetic construct
  source 1..28: mol_type = other DNA
ggagcacaggacttgagagcacttctgg

SEQ ID NO: 49326 - DNA, 28 bp, synthetic construct
  source 1..28: mol_type = other DNA
gagcacaggacttgagagcacttctggg

SEQ ID NO: 49327 - DNA, 28 bp, synthetic construct
  source 1..28: mol_type = other DNA
cacaggacttgagagcacttctgggtgg

SEQ ID NO: 49328 - DNA, 28 bp, synthetic construct
  source 1..28: mol_type = other DNA
acaggacttgagagcacttctgggtggg

SEQ ID NO: 49329 - DNA, 28 bp, synthetic construct
  source 1..28: mol_type = other DNA
cttctgggtgggaacagacccagcctgg

SEQ ID NO: 49330 - DNA, 28 bp, synthetic construct
  source 1..28: mol_type = other DNA
ttctgggtgggaacagacccagcctggg

SEQ ID NO: 49331 - DNA, 28 bp, synthetic construct
  source 1..28: mol_type = other DNA
tctgggtgggaacagacccagcctgggg

SEQ ID NO: 49332 - DNA, 28 bp, synthetic construct
  source 1..28: mol_type = other DNA
ggtgggaacagacccagcctggggcagg

SEQ ID NO: 49333 - DNA, 28 bp, synthetic construct
  source 1..28: mol_type = other DNA
gtgggaacagacccagcctggggcaggg

SEQ ID NO: 49334 - DNA, 28 bp, synthetic construct
  source 1..28: mol_type = other DNA
acagacccagcctggggcagggctcagg

SEQ ID NO: 49335 - DNA, 28 bp, synthetic construct
  source 1..28: mol_type = other DNA
agaaacctgagccctgccccaggctggg

SEQ ID NO: 49336 - DNA, 28 bp, synthetic construct
  source 1..28: mol_type = other DNA
cagaaacctgagccctgccccaggctgg

SEQ ID NO: 49337 - DNA, 28 bp, synthetic construct
  source 1..28: mol_type = other DNA
ccatcagaaacctgagccctgccccagg

SEQ ID NO: 49338 - DNA, 28 bp, synthetic construct
  source 1..28: mol_type = other DNA
ctggggcagggctcaggtttctgatggg

SEQ ID NO: 49339 - DNA, 28 bp, synthetic construct
  source 1..28: mol_type = other DNA
gggctcaggtttctgatgggaattctgg

SEQ ID NO: 49340 - DNA, 28 bp, synthetic construct
  source 1..28: mol_type = other DNA
tcaggtttctgatgggaattctggaagg

SEQ ID NO: 49341 - DNA, 28 bp, synthetic construct
  source 1..28: mol_type = other DNA
caggtttctgatgggaattctggaaggg

SEQ ID NO: 49342 - DNA, 28 bp, synthetic construct
  source 1..28: mol_type = other DNA
ctggattgaagcatgttgaataaaaggg

SEQ ID NO: 49343 - DNA, 28 bp, synthetic construct
  source 1..28: mol_type = other DNA
cctggattgaagcatgttgaataaaagg

SEQ ID NO: 49344 - DNA, 28 bp, synthetic construct
  source 1..28: mol_type = other DNA
cttttattcaacatgcttcaatccaggg

SEQ ID NO: 49345 - DNA, 28 bp, synthetic construct
  source 1..28: mol_type = other DNA
ttttattcaacatgcttcaatccagggg

SEQ ID NO: 49346 - DNA, 28 bp, synthetic construct
  source 1..28: mol_type = other DNA
gctgtggtcagacttcgggggcccctgg

SEQ ID NO: 49347 - DNA, 28 bp, synthetic construct
  source 1..28: mol_type = other DNA
gagcattgctgtggtcagacttcggggg

SEQ ID NO: 49348 - DNA, 28 bp, synthetic construct
  source 1..28: mol_type = other DNA
ggagcattgctgtggtcagacttcgggg

SEQ ID NO: 49349 - DNA, 28 bp, synthetic construct
  source 1..28: mol_type = other DNA
tggagcattgctgtggtcagacttcggg

SEQ ID NO: 49350 - DNA, 28 bp, synthetic construct
  source 1..28: mol_type = other DNA
ttggagcattgctgtggtcagacttcgg

SEQ ID NO: 49351 - DNA, 28 bp, synthetic construct
  source 1..28: mol_type = other DNA
agacacatggtttggagcattgctgtgg

SEQ ID NO: 49352 - DNA, 28 bp, synthetic construct
  source 1..28: mol_type = other DNA
aatgctccaaaccatgtgtctttcctgg

SEQ ID NO: 49353 - DNA, 28 bp, synthetic construct
  source 1..28: mol_type = other DNA
cttaagccaggaaagacacatggtttgg

SEQ ID NO: 49354 - DNA, 28 bp, synthetic construct
  source 1..28: mol_type = other DNA
caaaccatgtgtctttcctggcttaagg

SEQ ID NO: 49355 - DNA, 28 bp, synthetic construct
  source 1..28: mol_type = other DNA
tgaaccttaagccaggaaagacacatgg

SEQ ID NO: 49356 - DNA, 28 bp, synthetic construct
  source 1..28: mol_type = other DNA
gaggagggcgactgaaccttaagccagg

SEQ ID NO: 49357 - DNA, 28 bp, synthetic construct
  source 1..28: mol_type = other DNA
cttaaggttcagtcgccctcctcagagg

SEQ ID NO: 49358 - DNA, 28 bp, synthetic construct
  source 1..28: mol_type = other DNA
ttaaggttcagtcgccctcctcagaggg

SEQ ID NO: 49359 - DNA, 28 bp, synthetic construct
  source 1..28: mol_type = other DNA
taaggttcagtcgccctcctcagagggg

SEQ ID NO: 49360 - DNA, 28 bp, synthetic construct
  source 1..28: mol_type = other DNA
tctttcataggctcccctctgaggaggg

SEQ ID NO: 49361 - DNA, 28 bp, synthetic construct
  source 1..28: mol_type = other DNA
ctctttcataggctcccctctgaggagg

SEQ ID NO: 49362 - DNA, 28 bp, synthetic construct
  source 1..28: mol_type = other DNA
gggctctttcataggctcccctctgagg

SEQ ID NO: 49363 - DNA, 28 bp, synthetic construct
  source 1..28: mol_type = other DNA
gaggggagcctatgaaagagcccagtgg

SEQ ID NO: 49364 - DNA, 28 bp, synthetic construct
  source 1..28: mol_type = other DNA
ctgacactccactgggctctttcatagg

SEQ ID NO: 49365 - DNA, 28 bp, synthetic construct
  source 1..28: mol_type = other DNA
ctatgaaagagcccagtggagtgtcagg

SEQ ID NO: 49366 - DNA, 28 bp, synthetic construct
  source 1..28: mol_type = other DNA
tatgaaagagcccagtggagtgtcaggg

SEQ ID NO: 49367 - DNA, 28 bp, synthetic construct
  source 1..28: mol_type = other DNA
ggactcaggaccctgacactccactggg

SEQ ID NO: 49368 - DNA, 28 bp, synthetic construct
  source 1..28: mol_type = other DNA
aggactcaggaccctgacactccactgg

SEQ ID NO: 49369 - DNA, 28 bp, synthetic construct
  source 1..28: mol_type = other DNA
agggacaggactaggactaggactcagg

SEQ ID NO: 49370 - DNA, 28 bp, synthetic construct
  source 1..28: mol_type = other DNA
aagtggcagggacaggactaggactagg

SEQ ID NO: 49371 - DNA, 28 bp, synthetic construct
  source 1..28: mol_type = other DNA
cctcacaagtggcagggacaggactagg

SEQ ID NO: 49372 - DNA, 28 bp, synthetic construct
  source 1..28: mol_type = other DNA
ctagtcctgtccctgccacttgtgaggg

SEQ ID NO: 49373 - DNA, 28 bp, synthetic construct
  source 1..28: mol_type = other DNA
aagttccctcacaagtggcagggacagg

SEQ ID NO: 49374 - DNA, 28 bp, synthetic construct
  source 1..28: mol_type = other DNA
tgtccctgccacttgtgagggaacttgg

SEQ ID NO: 49375 - DNA, 28 bp, synthetic construct
  source 1..28: mol_type = other DNA
gtccctgccacttgtgagggaacttggg

SEQ ID NO: 49376 - DNA, 28 bp, synthetic construct
  source 1..28: mol_type = other DNA
ggcccaagttccctcacaagtggcaggg

SEQ ID NO: 49377 - DNA, 28 bp, synthetic construct
  source 1..28: mol_type = other DNA
aggcccaagttccctcacaagtggcagg

SEQ ID NO: 49378 - DNA, 28 bp, synthetic construct
  source 1..28: mol_type = other DNA
actgaggcccaagttccctcacaagtgg

SEQ ID NO: 49379 - DNA, 28 bp, synthetic construct
  source 1..28: mol_type = other DNA
agggaacttgggcctcagtttctccagg

SEQ ID NO: 49380 - DNA, 28 bp, synthetic construct
  source 1..28: mol_type = other DNA
gaacttgggcctcagtttctccaggtgg

SEQ ID NO: 49381 - DNA, 28 bp, synthetic construct
  source 1..28: mol_type = other DNA
aacttgggcctcagtttctccaggtggg

SEQ ID NO: 49382 - DNA, 28 bp, synthetic construct
  source 1..28: mol_type = other DNA
ttgtggagcccacctggagaaactgagg

SEQ ID NO: 49383 - DNA, 28 bp, synthetic construct
  source 1..28: mol_type = other DNA
aagagaagcaattgtggagcccacctgg

SEQ ID NO: 49384 - DNA, 28 bp, synthetic construct
  source 1..28: mol_type = other DNA
ggctccacaattgcttctcttgatctgg

SEQ ID NO: 49385 - DNA, 28 bp, synthetic construct
  source 1..28: mol_type = other DNA
cagtccagatcaagagaagcaattgtgg

SEQ ID NO: 49386 - DNA, 28 bp, synthetic construct
  source 1..28: mol_type = other DNA
cttgatctggactgccccagtgcccagg

SEQ ID NO: 49387 - DNA, 28 bp, synthetic construct
  source 1..28: mol_type = other DNA
tgtcactcactgaacctgggcactgggg

SEQ ID NO: 49388 - DNA, 28 bp, synthetic construct
  source 1..28: mol_type = other DNA
gtgtcactcactgaacctgggcactggg

SEQ ID NO: 49389 - DNA, 28 bp, synthetic construct
  source 1..28: mol_type = other DNA
tgtgtcactcactgaacctgggcactgg

SEQ ID NO: 49390 - DNA, 28 bp, synthetic construct
  source 1..28: mol_type = other DNA
agtgcccaggttcagtgagtgacacagg

SEQ ID NO: 49391 - DNA, 28 bp, synthetic construct
  source 1..28: mol_type = other DNA
gctgcctgtgtcactcactgaacctggg

SEQ ID NO: 49392 - DNA, 28 bp, synthetic construct
  source 1..28: mol_type = other DNA
agctgcctgtgtcactcactgaacctgg

SEQ ID NO: 49393 - DNA, 28 bp, synthetic construct
  source 1..28: mol_type = other DNA
aggttcagtgagtgacacaggcagctgg

SEQ ID NO: 49394 - DNA, 28 bp, synthetic construct
  source 1..28: mol_type = other DNA
ggttcagtgagtgacacaggcagctggg

SEQ ID NO: 49395 - DNA, 28 bp, synthetic construct
  source 1..28: mol_type = other DNA
agctgggtttccacatcctctgacttgg

SEQ ID NO: 49396 - DNA, 28 bp, synthetic construct
  source 1..28: mol_type = other DNA
gctgggtttccacatcctctgacttggg

SEQ ID NO: 49397 - DNA, 28 bp, synthetic construct
  source 1..28: mol_type = other DNA
tgaagggaacccaagtcagaggatgtgg

SEQ ID NO: 49398 - DNA, 28 bp, synthetic construct
  source 1..28: mol_type = other DNA
aggcagtgaagggaacccaagtcagagg

SEQ ID NO: 49399 - DNA, 28 bp, synthetic construct
  source 1..28: mol_type = other DNA
gacttgggttcccttcactgcctccagg

SEQ ID NO: 49400 - DNA, 28 bp, synthetic construct
  source 1..28: mol_type = other DNA
tgggttcccttcactgcctccaggcagg

SEQ ID NO: 49401 - DNA, 28 bp, synthetic construct
  source 1..28: mol_type = other DNA
gggttcccttcactgcctccaggcaggg

SEQ ID NO: 49402 - DNA, 28 bp, synthetic construct
  source 1..28: mol_type = other DNA
ccgagccctgcctggaggcagtgaaggg

SEQ ID NO: 49403 - DNA, 28 bp, synthetic construct
  source 1..28: mol_type = other DNA
gccgagccctgcctggaggcagtgaagg

SEQ ID NO: 49404 - DNA, 28 bp, synthetic construct
  source 1..28: mol_type = other DNA
gggtggagggccgagccctgcctggagg

SEQ ID NO: 49405 - DNA, 28 bp, synthetic construct
  source 1..28: mol_type = other DNA
tgggggtggagggccgagccctgcctgg

SEQ ID NO: 49406 - DNA, 28 bp, synthetic construct
  source 1..28: mol_type = other DNA
cagggctcggccctccacccccaagtgg

SEQ ID NO: 49407 - DNA, 28 bp, synthetic construct
  source 1..28: mol_type = other DNA
acacaatgggccacttgggggtggaggg

SEQ ID NO: 49408 - DNA, 28 bp, synthetic construct
  source 1..28: mol_type = other DNA
cacacaatgggccacttgggggtggagg

SEQ ID NO: 49409 - DNA, 28 bp, synthetic construct
  source 1..28: mol_type = other DNA
gctcacacaatgggccacttgggggtgg

SEQ ID NO: 49410 - DNA, 28 bp, synthetic construct
  source 1..28: mol_type = other DNA
tgagctcacacaatgggccacttggggg

SEQ ID NO: 49411 - DNA, 28 bp, synthetic construct
  source 1..28: mol_type = other DNA
ctgagctcacacaatgggccacttgggg

SEQ ID NO: 49412 - DNA, 28 bp, synthetic construct
  source 1..28: mol_type = other DNA
actgagctcacacaatgggccacttggg

SEQ ID NO: 49413 - DNA, 28 bp, synthetic construct
  source 1..28: mol_type = other DNA
aactgagctcacacaatgggccacttgg

SEQ ID NO: 49414 - DNA, 28 bp, synthetic construct
  source 1..28: mol_type = other DNA
gcccattgtgtgagctcagtttcagtgg

SEQ ID NO: 49415 - DNA, 28 bp, synthetic construct
  source 1..28: mol_type = other DNA
cccactgaaactgagctcacacaatggg

SEQ ID NO: 49416 - DNA, 28 bp, synthetic construct
  source 1..28: mol_type = other DNA
ccattgtgtgagctcagtttcagtgggg

SEQ ID NO: 49417 - DNA, 28 bp, synthetic construct
  source 1..28: mol_type = other DNA
gctcagtttcagtggggacagaaactgg

SEQ ID NO: 49418 - DNA, 28 bp, synthetic construct
  source 1..28: mol_type = other DNA
ctcagtttcagtggggacagaaactggg

SEQ ID NO: 49419 - DNA, 28 bp, synthetic construct
  source 1..28: mol_type = other DNA
tggggacagaaactgggttgagaaaagg

SEQ ID NO: 49420 - DNA, 28 bp, synthetic construct
  source 1..28: mol_type = other DNA
ggggacagaaactgggttgagaaaaggg

SEQ ID NO: 49421 - DNA, 28 bp, synthetic construct
  source 1..28: mol_type = other DNA
ttacttggcattggcttggtgggatagg

SEQ ID NO: 49422 - DNA, 28 bp, synthetic construct
  source 1..28: mol_type = other DNA
actatttacttggcattggcttggtggg

SEQ ID NO: 49423 - DNA, 28 bp, synthetic construct
  source 1..28: mol_type = other DNA
cactatttacttggcattggcttggtgg

SEQ ID NO: 49424 - DNA, 28 bp, synthetic construct
  source 1..28: mol_type = other DNA
ctgcactatttacttggcattggcttgg

SEQ ID NO: 49425 - DNA, 28 bp, synthetic construct
  source 1..28: mol_type = other DNA
agatactgcactatttacttggcattgg

SEQ ID NO: 49426 - DNA, 28 bp, synthetic construct
  source 1..28: mol_type = other DNA
tacataagatactgcactatttacttgg

SEQ ID NO: 49427 - DNA, 28 bp, synthetic construct
  source 1..28: mol_type = other DNA
agcccttgccctgcccttccccatctgg

SEQ ID NO: 49428 - DNA, 28 bp, synthetic construct
  source 1..28: mol_type = other DNA
gcccttgccctgcccttccccatctggg

SEQ ID NO: 49429 - DNA, 28 bp, synthetic construct
  source 1..28: mol_type = other DNA
acccagatggggaagggcagggcaaggg

SEQ ID NO: 49430 - DNA, 28 bp, synthetic construct
  source 1..28: mol_type = other DNA
cacccagatggggaagggcagggcaagg

SEQ ID NO: 49431 - DNA, 28 bp, synthetic construct
  source 1..28: mol_type = other DNA
agcagcacccagatggggaagggcaggg

SEQ ID NO: 49432 - DNA, 28 bp, synthetic construct
  source 1..28: mol_type = other DNA
cagcagcacccagatggggaagggcagg

SEQ ID NO: 49433 - DNA, 28 bp, synthetic construct
  source 1..28: mol_type = other DNA
taggcagcagcacccagatggggaaggg

SEQ ID NO: 49434 - DNA, 28 bp, synthetic construct
  source 1..28: mol_type = other DNA
ctaggcagcagcacccagatggggaagg

SEQ ID NO: 49435 - DNA, 28 bp, synthetic construct
  source 1..28: mol_type = other DNA
tgctctaggcagcagcacccagatgggg

SEQ ID NO: 49436 - DNA, 28 bp, synthetic construct
  source 1..28: mol_type = other DNA
atgctctaggcagcagcacccagatggg

SEQ ID NO: 49437 - DNA, 28 bp, synthetic construct
  source 1..28: mol_type = other DNA
tatgctctaggcagcagcacccagatgg

SEQ ID NO: 49438 - DNA, 28 bp, synthetic construct
  source 1..28: mol_type = other DNA
ggtgctgctgcctagagcatataaaagg

SEQ ID NO: 49439 - DNA, 28 bp, synthetic construct
  source 1..28: mol_type = other DNA
cagcaaggtgccttttatatgctctagg

SEQ ID NO: 49440 - DNA, 28 bp, synthetic construct
  source 1..28: mol_type = other DNA
ctagagcatataaaaggcaccttgctgg

SEQ ID NO: 49441 - DNA, 28 bp, synthetic construct
  source 1..28: mol_type = other DNA
tagagcatataaaaggcaccttgctggg

SEQ ID NO: 49442 - DNA, 28 bp, synthetic construct
  source 1..28: mol_type = other DNA
gggctagtatgagacatgcccagcaagg

SEQ ID NO: 49443 - DNA, 28 bp, synthetic construct
  source 1..28: mol_type = other DNA
catactagcccaccagactcagagacgg

SEQ ID NO: 49444 - DNA, 28 bp, synthetic construct
  source 1..28: mol_type = other DNA
ctctggttccgtctctgagtctggtggg

SEQ ID NO: 49445 - DNA, 28 bp, synthetic construct
  source 1..28: mol_type = other DNA
tctctggttccgtctctgagtctggtgg

SEQ ID NO: 49446 - DNA, 28 bp, synthetic construct
  source 1..28: mol_type = other DNA
ccagactcagagacggaaccagagacgg

SEQ ID NO: 49447 - DNA, 28 bp, synthetic construct
  source 1..28: mol_type = other DNA
cagactcagagacggaaccagagacggg

SEQ ID NO: 49448 - DNA, 28 bp, synthetic construct
  source 1..28: mol_type = other DNA
ggagggggatgctctggcccgtctctgg

SEQ ID NO: 49449 - DNA, 28 bp, synthetic construct
  source 1..28: mol_type = other DNA
ttcatggtggaggagggggatgctctgg

SEQ ID NO: 49450 - DNA, 28 bp, synthetic construct
  source 1..28: mol_type = other DNA
acagcgagtttcatggtggaggaggggg

SEQ ID NO: 49451 - DNA, 28 bp, synthetic construct
  source 1..28: mol_type = other DNA
gacagcgagtttcatggtggaggagggg

SEQ ID NO: 49452 - DNA, 28 bp, synthetic construct
  source 1..28: mol_type = other DNA
tgacagcgagtttcatggtggaggaggg

SEQ ID NO: 49453 - DNA, 28 bp, synthetic construct
  source 1..28: mol_type = other DNA
gtgacagcgagtttcatggtggaggagg

SEQ ID NO: 49454 - DNA, 28 bp, synthetic construct
  source 1..28: mol_type = other DNA
agggtgacagcgagtttcatggtggagg

SEQ ID NO: 49455 - DNA, 28 bp, synthetic construct
  source 1..28: mol_type = other DNA
gtgagggtgacagcgagtttcatggtgg

SEQ ID NO: 49456 - DNA, 28 bp, synthetic construct
  source 1..28: mol_type = other DNA
agggtgagggtgacagcgagtttcatgg

SEQ ID NO: 49457 - DNA, 28 bp, synthetic construct
  source 1..28: mol_type = other DNA
atgaaactcgctgtcaccctcaccctgg

SEQ ID NO: 49458 - DNA, 28 bp, synthetic construct
  source 1..28: mol_type = other DNA
gctgtcaccctcaccctggtcacactgg

SEQ ID NO: 49459 - DNA, 28 bp, synthetic construct
  source 1..28: mol_type = other DNA
cagagagccagtgtgaccagggtgaggg

SEQ ID NO: 49460 - DNA, 28 bp, synthetic construct
  source 1..28: mol_type = other DNA
gcagagagccagtgtgaccagggtgagg

SEQ ID NO: 49461 - DNA, 28 bp, synthetic construct
  source 1..28: mol_type = other DNA
ctgcagcagagagccagtgtgaccaggg

SEQ ID NO: 49462 - DNA, 28 bp, synthetic construct
  source 1..28: mol_type = other DNA
gctgcagcagagagccagtgtgaccagg

SEQ ID NO: 49463 - DNA, 28 bp, synthetic construct
  source 1..28: mol_type = other DNA
tcacactggctctctgctgcagctccgg

SEQ ID NO: 49464 - DNA, 28 bp, synthetic construct
  source 1..28: mol_type = other DNA
gagggaagggtctctgagcactcaccgg

SEQ ID NO: 49465 - DNA, 28 bp, synthetic construct
  source 1..28: mol_type = other DNA
tgctcagagacccttccctccctcctgg

SEQ ID NO: 49466 - DNA, 28 bp, synthetic construct
  source 1..28: mol_type = other DNA
agacccttccctccctcctggacttagg

SEQ ID NO: 49467 - DNA, 28 bp, synthetic construct
  source 1..28: mol_type = other DNA
gttcctaagtccaggagggagggaaggg

SEQ ID NO: 49468 - DNA, 28 bp, synthetic construct
  source 1..28: mol_type = other DNA
agttcctaagtccaggagggagggaagg

SEQ ID NO: 49469 - DNA, 28 bp, synthetic construct
  source 1..28: mol_type = other DNA
tgagagttcctaagtccaggagggaggg

SEQ ID NO: 49470 - DNA, 28 bp, synthetic construct
  source 1..28: mol_type = other DNA
ctgagagttcctaagtccaggagggagg

SEQ ID NO: 49471 - DNA, 28 bp, synthetic construct
  source 1..28: mol_type = other DNA
ctccctcctggacttaggaactctcagg

SEQ ID NO: 49472 - DNA, 28 bp, synthetic construct
  source 1..28: mol_type = other DNA
gtcctgagagttcctaagtccaggaggg

SEQ ID NO: 49473 - DNA, 28 bp, synthetic construct
  source 1..28: mol_type = other DNA
ggtcctgagagttcctaagtccaggagg

SEQ ID NO: 49474 - DNA, 28 bp, synthetic construct
  source 1..28: mol_type = other DNA
gggggtcctgagagttcctaagtccagg

SEQ ID NO: 49475 - DNA, 28 bp, synthetic construct
  source 1..28: mol_type = other DNA
ggaccccccagttctgctcagaagaagg

SEQ ID NO: 49476 - DNA, 28 bp, synthetic construct
  source 1..28: mol_type = other DNA
actccttcttctgagcagaactgggggg

SEQ ID NO: 49477 - DNA, 28 bp, synthetic construct
  source 1..28: mol_type = other DNA
cactccttcttctgagcagaactggggg

SEQ ID NO: 49478 - DNA, 28 bp, synthetic construct
  source 1..28: mol_type = other DNA
tcactccttcttctgagcagaactgggg

SEQ ID NO: 49479 - DNA, 28 bp, synthetic construct
  source 1..28: mol_type = other DNA
ctcactccttcttctgagcagaactggg

SEQ ID NO: 49480 - DNA, 28 bp, synthetic construct
  source 1..28: mol_type = other DNA
gctcactccttcttctgagcagaactgg

SEQ ID NO: 49481 - DNA, 28 bp, synthetic construct
  source 1..28: mol_type = other DNA
aggagtgagctgcccattcctgctctgg

SEQ ID NO: 49482 - DNA, 28 bp, synthetic construct
  source 1..28: mol_type = other DNA
ctgcccattcctgctctggagctgctgg

SEQ ID NO: 49483 - DNA, 28 bp, synthetic construct
  source 1..28: mol_type = other DNA
tgcccattcctgctctggagctgctggg

SEQ ID NO: 49484 - DNA, 28 bp, synthetic construct
  source 1..28: mol_type = other DNA
ctcccagcagctccagagcaggaatggg

SEQ ID NO: 49485 - DNA, 28 bp, synthetic construct
  source 1..28: mol_type = other DNA
ccattcctgctctggagctgctgggagg

SEQ ID NO: 49486 - DNA, 28 bp, synthetic construct
  source 1..28: mol_type = other DNA
caggtcctcccagcagctccagagcagg

SEQ ID NO: 49487 - DNA, 28 bp, synthetic construct
  source 1..28: mol_type = other DNA
ctgctctggagctgctgggaggacctgg

SEQ ID NO: 49488 - DNA, 28 bp, synthetic construct
  source 1..28: mol_type = other DNA
tgctctggagctgctgggaggacctggg

SEQ ID NO: 49489 - DNA, 28 bp, synthetic construct
  source 1..28: mol_type = other DNA
tgaaaaggctgctatctctcgctgatgg

SEQ ID NO: 49490 - DNA, 28 bp, synthetic construct
  source 1..28: mol_type = other DNA
gaaaaggctgctatctctcgctgatggg

SEQ ID NO: 49491 - DNA, 28 bp, synthetic construct
  source 1..28: mol_type = other DNA
ggctgctatctctcgctgatgggcctgg

SEQ ID NO: 49492 - DNA, 28 bp, synthetic construct
  source 1..28: mol_type = other DNA
gctgatgggcctggctgtttgcatctgg

SEQ ID NO: 49493 - DNA, 28 bp, synthetic construct
  source 1..28: mol_type = other DNA
ctgatgggcctggctgtttgcatctggg

SEQ ID NO: 49494 - DNA, 28 bp, synthetic construct
  source 1..28: mol_type = other DNA
tgggtctgcccagatgcaaacagccagg

SEQ ID NO: 49495 - DNA, 28 bp, synthetic construct
  source 1..28: mol_type = other DNA
tttgcatctgggcagacccagccagagg

SEQ ID NO: 49496 - DNA, 28 bp, synthetic construct
  source 1..28: mol_type = other DNA
ttgcatctgggcagacccagccagaggg

SEQ ID NO: 49497 - DNA, 28 bp, synthetic construct
  source 1..28: mol_type = other DNA
gacccagccagagggctagccagcttgg

SEQ ID NO: 49498 - DNA, 28 bp, synthetic construct
  source 1..28: mol_type = other DNA
ttccaagctggctagccctctggctggg

SEQ ID NO: 49499 - DNA, 28 bp, synthetic construct
  source 1..28: mol_type = other DNA
tttccaagctggctagccctctggctgg

SEQ ID NO: 49500 - DNA, 28 bp, synthetic construct
  source 1..28: mol_type = other DNA
agccagagggctagccagcttggaaagg

SEQ ID NO: 49501 - DNA, 28 bp, synthetic construct
  source 1..28: mol_type = other DNA
gccagagggctagccagcttggaaaggg

SEQ ID NO: 49502 - DNA, 28 bp, synthetic construct
  source 1..28: mol_type = other DNA
ccagagggctagccagcttggaaagggg

SEQ ID NO: 49503 - DNA, 28 bp, synthetic construct
  source 1..28: mol_type = other DNA
gggctagccagcttggaaaggggcctgg

SEQ ID NO: 49504 - DNA, 28 bp, synthetic construct
  source 1..28: mol_type = other DNA
catgtctccaggcccctttccaagctgg

SEQ ID NO: 49505 - DNA, 28 bp, synthetic construct
  source 1..28: mol_type = other DNA
cagaggagagaaggcacatgtctccagg

SEQ ID NO: 49506 - DNA, 28 bp, synthetic construct
  source 1..28: mol_type = other DNA
cagaagctgcaacacagaggagagaagg

SEQ ID NO: 49507 - DNA, 28 bp, synthetic construct
  source 1..28: mol_type = other DNA
gatctctgcagaagctgcaacacagagg

SEQ ID NO: 49508 - DNA, 28 bp, synthetic construct
  source 1..28: mol_type = other DNA
ggtttcgatgacacgctgaaagctcggg

SEQ ID NO: 49509 - DNA, 28 bp, synthetic construct
  source 1..28: mol_type = other DNA
gggtttcgatgacacgctgaaagctcgg

SEQ ID NO: 49510 - DNA, 28 bp, synthetic construct
  source 1..28: mol_type = other DNA
cagcgtgtcatcgaaaccctcctcatgg

SEQ ID NO: 49511 - DNA, 28 bp, synthetic construct
  source 1..28: mol_type = other DNA
taactggagggtgtgtccatgaggaggg

SEQ ID NO: 49512 - DNA, 28 bp, synthetic construct
  source 1..28: mol_type = other DNA
ataactggagggtgtgtccatgaggagg

SEQ ID NO: 49513 - DNA, 28 bp, synthetic construct
  source 1..28: mol_type = other DNA
ctcataactggagggtgtgtccatgagg

SEQ ID NO: 49514 - DNA, 28 bp, synthetic construct
  source 1..28: mol_type = other DNA
ctcatggacacaccctccagttatgagg

SEQ ID NO: 49515 - DNA, 28 bp, synthetic construct
  source 1..28: mol_type = other DNA
acaccctccagttatgaggctgccatgg

SEQ ID NO: 49516 - DNA, 28 bp, synthetic construct
  source 1..28: mol_type = other DNA
gttccatggcagcctcataactggaggg

SEQ ID NO: 49517 - DNA, 28 bp, synthetic construct
  source 1..28: mol_type = other DNA
agttccatggcagcctcataactggagg

SEQ ID NO: 49518 - DNA, 28 bp, synthetic construct
  source 1..28: mol_type = other DNA
aaaagttccatggcagcctcataactgg

SEQ ID NO: 49519 - DNA, 28 bp, synthetic construct
  source 1..28: mol_type = other DNA
tcttgatcagggctgaaaagttccatgg

SEQ ID NO: 49520 - DNA, 28 bp, synthetic construct
  source 1..28: mol_type = other DNA
acttttcagccctgatcaagacatgagg

SEQ ID NO: 49521 - DNA, 28 bp, synthetic construct
  source 1..28: mol_type = other DNA
cttttcagccctgatcaagacatgaggg

SEQ ID NO: 49522 - DNA, 28 bp, synthetic construct
  source 1..28: mol_type = other DNA
ttcagccctgatcaagacatgagggagg

SEQ ID NO: 49523 - DNA, 28 bp, synthetic construct
  source 1..28: mol_type = other DNA
gccctgatcaagacatgagggaggcagg

SEQ ID NO: 49524 - DNA, 28 bp, synthetic construct
  source 1..28: mol_type = other DNA
ccctgcctccctcatgtcttgatcaggg

SEQ ID NO: 49525 - DNA, 28 bp, synthetic construct
  source 1..28: mol_type = other DNA
cccctgcctccctcatgtcttgatcagg

SEQ ID NO: 49526 - DNA, 28 bp, synthetic construct
  source 1..28: mol_type = other DNA
gaggcaggggctcagctgaagaagctgg

SEQ ID NO: 49527 - DNA, 28 bp, synthetic construct
  source 1..28: mol_type = other DNA
gcaggggctcagctgaagaagctggtgg

SEQ ID NO: 49528 - DNA, 28 bp, synthetic construct
  source 1..28: mol_type = other DNA
atgctttctctgggcttttgggggaggg

SEQ ID NO: 49529 - DNA, 28 bp, synthetic construct
  source 1..28: mol_type = other DNA
gatgctttctctgggcttttgggggagg

SEQ ID NO: 49530 - DNA, 28 bp, synthetic construct
  source 1..28: mol_type = other DNA
aatgatgctttctctgggcttttggggg

SEQ ID NO: 49531 - DNA, 28 bp, synthetic construct
  source 1..28: mol_type = other DNA
taatgatgctttctctgggcttttgggg

SEQ ID NO: 49532 - DNA, 28 bp, synthetic construct
  source 1..28: mol_type = other DNA
ttaatgatgctttctctgggcttttggg

SEQ ID NO: 49533 - DNA, 28 bp, synthetic construct
  source 1..28: mol_type = other DNA
cttaatgatgctttctctgggcttttgg

SEQ ID NO: 49534 - DNA, 28 bp, synthetic construct
  source 1..28: mol_type = other DNA
cccagagaaagcatcattaagctcatgg

SEQ ID NO: 49535 - DNA, 28 bp, synthetic construct
  source 1..28: mol_type = other DNA
accatgagcttaatgatgctttctctgg

SEQ ID NO: 49536 - DNA, 28 bp, synthetic construct
  source 1..28: mol_type = other DNA
gtaaccagcacctttcacgtcacactgg

SEQ ID NO: 49537 - DNA, 28 bp, synthetic construct
  source 1..28: mol_type = other DNA
ctaaccagtgtgacgtgaaaggtgctgg

SEQ ID NO: 49538 - DNA, 28 bp, synthetic construct
  source 1..28: mol_type = other DNA
cctttcacgtcacactggttagaagtgg

SEQ ID NO: 49539 - DNA, 28 bp, synthetic construct
  source 1..28: mol_type = other DNA
actggttagaagtggcttccccaagtgg

SEQ ID NO: 49540 - DNA, 28 bp, synthetic construct
  source 1..28: mol_type = other DNA
ctggttagaagtggcttccccaagtggg

SEQ ID NO: 49541 - DNA, 28 bp, synthetic construct
  source 1..28: mol_type = other DNA
tggttagaagtggcttccccaagtgggg

SEQ ID NO: 49542 - DNA, 28 bp, synthetic construct
  source 1..28: mol_type = other DNA
aagtggcttccccaagtggggctgcagg

SEQ ID NO: 49543 - DNA, 28 bp, synthetic construct
  source 1..28: mol_type = other DNA
tggggcaatcctgcagccccacttgggg

SEQ ID NO: 49544 - DNA, 28 bp, synthetic construct
  source 1..28: mol_type = other DNA
ctggggcaatcctgcagccccacttggg

SEQ ID NO: 49545 - DNA, 28 bp, synthetic construct
  source 1..28: mol_type = other DNA
actggggcaatcctgcagccccacttgg

SEQ ID NO: 49546 - DNA, 28 bp, synthetic construct
  source 1..28: mol_type = other DNA
ggattagaaacaggtctgaaaactgggg

SEQ ID NO: 49547 - DNA, 28 bp, synthetic construct
  source 1..28: mol_type = other DNA
tggattagaaacaggtctgaaaactggg

SEQ ID NO: 49548 - DNA, 28 bp, synthetic construct
  source 1..28: mol_type = other DNA
ctggattagaaacaggtctgaaaactgg

SEQ ID NO: 49549 - DNA, 28 bp, synthetic construct
  source 1..28: mol_type = other DNA
tttcagacctgtttctaatccagagagg

SEQ ID NO: 49550 - DNA, 28 bp, synthetic construct
  source 1..28: mol_type = other DNA
tgactctcctctctggattagaaacagg

SEQ ID NO: 49551 - DNA, 28 bp, synthetic construct
  source 1..28: mol_type = other DNA
acagtggcactgtgactctcctctctgg

SEQ ID NO: 49552 - DNA, 28 bp, synthetic construct
  source 1..28: mol_type = other DNA
ggagagtcacagtgccactgtccccagg

SEQ ID NO: 49553 - DNA, 28 bp, synthetic construct
  source 1..28: mol_type = other DNA
tcctcctagagttgactgcacctctcgg

SEQ ID NO: 49554 - DNA, 28 bp, synthetic construct
  source 1..28: mol_type = other DNA
accgagaggtgcagtcaactctaggagg

SEQ ID NO: 49555 - DNA, 28 bp, synthetic construct
  source 1..28: mol_type = other DNA
ttaaccgagaggtgcagtcaactctagg

SEQ ID NO: 49556 - DNA, 28 bp, synthetic construct
  source 1..28: mol_type = other DNA
cacagaaacttcaacattaaccgagagg

SEQ ID NO: 49557 - DNA, 28 bp, synthetic construct
  source 1..28: mol_type = other DNA
ctctcggttaatgttgaagtttctgtgg

SEQ ID NO: 49558 - DNA, 28 bp, synthetic construct
  source 1..28: mol_type = other DNA
acaacagtgaatgaattgcatagttagg

SEQ ID NO: 49559 - DNA, 28 bp, synthetic construct
  source 1..28: mol_type = other DNA
ctatgcaattcattcactgttgtattgg

SEQ ID NO: 49560 - DNA, 28 bp, synthetic construct
  source 1..28: mol_type = other DNA
tatgcaattcattcactgttgtattggg

SEQ ID NO: 49561 - DNA, 28 bp, synthetic construct
  source 1..28: mol_type = other DNA
ttctgtttctttgtctatttgttttagg

SEQ ID NO: 49562 - DNA, 28 bp, synthetic construct
  source 1..28: mol_type = other DNA
aaatgctaattacacagtgagctttggg

SEQ ID NO: 49563 - DNA, 28 bp, synthetic construct
  source 1..28: mol_type = other DNA
taaatgctaattacacagtgagctttgg

SEQ ID NO: 49564 - DNA, 28 bp, synthetic construct
  source 1..28: mol_type = other DNA
gcagcggcagaggctggagcagttgggg

SEQ ID NO: 49565 - DNA, 28 bp, synthetic construct
  source 1..28: mol_type = other DNA
ggcagcggcagaggctggagcagttggg

SEQ ID NO: 49566 - DNA, 28 bp, synthetic construct
  source 1..28: mol_type = other DNA
tggcagcggcagaggctggagcagttgg

SEQ ID NO: 49567 - DNA, 28 bp, synthetic construct
  source 1..28: mol_type = other DNA
ctcaaagcatggcagcggcagaggctgg

SEQ ID NO: 49568 - DNA, 28 bp, synthetic construct
  source 1..28: mol_type = other DNA
tggactcaaagcatggcagcggcagagg

SEQ ID NO: 49569 - DNA, 28 bp, synthetic construct
  source 1..28: mol_type = other DNA
tgggcgtggactcaaagcatggcagcgg

SEQ ID NO: 49570 - DNA, 28 bp, synthetic construct
  source 1..28: mol_type = other DNA
ggctggtgggcgtggactcaaagcatgg

SEQ ID NO: 49571 - DNA, 28 bp, synthetic construct
  source 1..28: mol_type = other DNA
ttgaagagagcaaggctggtgggcgtgg

SEQ ID NO: 49572 - DNA, 28 bp, synthetic construct
  source 1..28: mol_type = other DNA
gtttattgaagagagcaaggctggtggg

SEQ ID NO: 49573 - DNA, 28 bp, synthetic construct
  source 1..28: mol_type = other DNA
ggtttattgaagagagcaaggctggtgg

SEQ ID NO: 49574 - DNA, 28 bp, synthetic construct
  source 1..28: mol_type = other DNA
tgtggtttattgaagagagcaaggctgg

SEQ ID NO: 49575 - DNA, 28 bp, synthetic construct
  source 1..28: mol_type = other DNA
tgcttgtggtttattgaagagagcaagg

SEQ ID NO: 49576 - DNA, 28 bp, synthetic construct
  source 1..28: mol_type = other DNA
agggggcacaaaagtgagatgcttgtgg

SEQ ID NO: 49577 - RNA, 20 nt, synthetic construct
  source 1..20: mol_type = other RNA
gttctgatgcagcttccatg

SEQ ID NO: 49578 - RNA, 20 nt, synthetic construct
  source 1..20: mol_type = other RNA
tatggatcgcccaagagttg

SEQ ID NO: 49579 - RNA, 20 nt, synthetic construct
  source 1..20: mol_type = other RNA
tgtcatgctgaaccgcattg

SEQ ID NO: 49580 - RNA, 20 nt, synthetic construct
  source 1..20: mol_type = other RNA
ttgacatagaagaggcacaa

SEQ ID NO: 49581 - RNA, 20 nt, synthetic construct
  source 1..20: mol_type = other RNA
cttgtggcgctgaaaacgaa

SEQ ID NO: 49582 - RNA, 20 nt, synthetic construct
  source 1..20: mol_type = other RNA
gatggcttggtccatcacgt

SEQ ID NO: 49583 - RNA, 20 nt, synthetic construct
  source 1..20: mol_type = other RNA
cagcctctgatcattcccgg

SEQ ID NO: 49584 - RNA, 20 nt, synthetic construct
  source 1..20: mol_type = other RNA
cagcttaggagactcatcag

SEQ ID NO: 49585 - RNA, 20 nt, synthetic construct
  source 1..20: mol_type = other RNA
cctagcagtacataccacca

SEQ ID NO: 49586 - RNA, 20 nt, synthetic construct
  source 1..20: mol_type = other RNA
ctgagaacattagtgctacg

SEQ ID NO: 49587 - RNA, 20 nt, synthetic construct
  source 1..20: mol_type = other RNA
gtggataccatagccatcca

SEQ ID NO: 49588 - RNA, 20 nt, synthetic construct
  source 1..20: mol_type = other RNA
tatggctcgagtctaaggaa

SEQ ID NO: 49589 - RNA, 20 nt, synthetic construct
  source 1..20: mol_type = other RNA
gctacagaagtgcttcgaag

SEQ ID NO: 49590 - RNA, 20 nt, synthetic construct
  source 1..20: mol_type = other RNA
tgggcaagtataccacggtg

SEQ ID NO: 49591 - RNA, 20 nt, synthetic construct
  source 1..20: mol_type = other RNA
agcaacggcgaagacgcggg

SEQ ID NO: 49592 - RNA, 20 nt, synthetic construct
  source 1..20: mol_type = other RNA
aggaattacctgtaatcgag

SEQ ID NO: 49593 - RNA, 20 nt, synthetic construct
  source 1..20: mol_type = other RNA
agtacacatttgtacaagct

SEQ ID NO: 49594 - RNA, 20 nt, synthetic construct
  source 1..20: mol_type = other RNA
tctggccaaaagcatgagag

SEQ ID NO: 49595 - RNA, 20 nt, synthetic construct
  source 1..20: mol_type = other RNA
atattcaagatcgttctgtg

SEQ ID NO: 49596 - RNA, 20 nt, synthetic construct
  source 1..20: mol_type = other RNA
tatggggtaatccgttggat

SEQ ID NO: 49597 - RNA, 20 nt, synthetic construct
  source 1..20: mol_type = other RNA
atgtacaacaagatccctgt

SEQ ID NO: 49598 - RNA, 20 nt, synthetic construct
  source 1..20: mol_type = other RNA
ctgattgccatgaatctggc

SEQ ID NO: 49599 - RNA, 20 nt, synthetic construct
  source 1..20: mol_type = other RNA
gccaggttgaagggagccgt

SEQ ID NO: 49600 - RNA, 20 nt, synthetic construct
  source 1..20: mol_type = other RNA
tcggtcatcagcgtcagcaa

SEQ ID NO: 49601 - RNA, 20 nt, synthetic construct
  source 1..20: mol_type = other RNA
cgtgacgcgacctagcgagg

SEQ ID NO: 49602 - RNA, 20 nt, synthetic construct
  source 1..20: mol_type = other RNA
tctctgtgcggtatttgaag

SEQ ID NO: 49603 - RNA, 20 nt, synthetic construct
  source 1..20: mol_type = other RNA
caggcccaataggaaacgtg

SEQ ID NO: 49604 - RNA, 20 nt, synthetic construct
  source 1..20: mol_type = other RNA
gattatgtggaggagaatcg

SEQ ID NO: 49605 - RNA, 20 nt, synthetic construct
  source 1..20: mol_type = other RNA
atggcagcctcataactgga

SEQ ID NO: 49606 - RNA, 20 nt, synthetic construct
  source 1..20: mol_type = other RNA
tgtcatcgaaaccctcctca

SEQ ID NO: 49607 - RNA, 20 nt, synthetic construct
  source 1..20: mol_type = other RNA
gctcctacgcccaatcactg

SEQ ID NO: 49608 - RNA, 20 nt, synthetic construct
  source 1..20: mol_type = other RNA
acactgcgatcgcatcatcg

SEQ ID NO: 49609 - RNA, 20 nt, synthetic construct
  source 1..20: mol_type = other RNA
gtaaatacctccaaatcccg

SEQ ID NO: 49610 - RNA, 20 nt, synthetic construct
  source 1..20: mol_type = other RNA
tctcataaagatgaaaagcg

SEQ ID NO: 49611 - RNA, 20 nt, synthetic construct
  source 1..20: mol_type = other RNA
ggtaagaggcagttgacgtg

SEQ ID NO: 49612 - RNA, 20 nt, synthetic construct
  source 1..20: mol_type = other RNA
gagggtgtgagcagaaaagc

SEQ ID NO: 49613 - RNA, 20 nt, synthetic construct
  source 1..20: mol_type = other RNA
aatgcattctccacaccagg

SEQ ID NO: 49614 - RNA, 20 nt, synthetic construct
  source 1..20: mol_type = other RNA
accaacaagacccagcaccg

SEQ ID NO: 49615 - RNA, 20 nt, synthetic construct
  source 1..20: mol_type = other RNA
aatcctgctccaaaaaacca

SEQ ID NO: 49616 - RNA, 20 nt, synthetic construct
  source 1..20: mol_type = other RNA
aaaccttattgaaggtgagg

SEQ ID NO: 49617 - RNA, 20 nt, synthetic construct
  source 1..20: mol_type = other RNA
aacctacggcctattctcag

SEQ ID NO: 49618 - RNA, 20 nt, synthetic construct
  source 1..20: mol_type = other RNA
ataatttaaaaaggtcagag

SEQ ID NO: 49619 - RNA, 20 nt, synthetic construct
  source 1..20: mol_type = other RNA
ggactctgctgtaatggaca

SEQ ID NO: 49620 - RNA, 20 nt, synthetic construct
  source 1..20: mol_type = other RNA
aatgggctcgagacacatca

SEQ ID NO: 49621 - RNA, 20 nt, synthetic construct
  source 1..20: mol_type = other RNA
gaggcatactttctgcacag

SEQ ID NO: 49622 - RNA, 20 nt, synthetic construct
  source 1..20: mol_type = other RNA
tagttgatcaagaattttgg

SEQ ID NO: 49623 - RNA, 20 nt, synthetic construct
  source 1..20: mol_type = other RNA
taactcctgagagttgtcgg

SEQ ID NO: 49624 - RNA, 20 nt, synthetic construct
  source 1..20: mol_type = other RNA
cacacacttcatcataaggg

SEQ ID NO: 49625 - RNA, 20 nt, synthetic construct
  source 1..20: mol_type = other RNA
gctactcacagttgtccaca

SEQ ID NO: 49626 - RNA, 20 nt, synthetic construct
  source 1..20: mol_type = other RNA
gctttaaggagacttcatgg

SEQ ID NO: 49627 - RNA, 20 nt, synthetic construct
  source 1..20: mol_type = other RNA
tgcactgatgaattttgaca

SEQ ID NO: 49628 - RNA, 20 nt, synthetic construct
  source 1..20: mol_type = other RNA
aaagtaaactttacatccag

SEQ ID NO: 49629 - RNA, 20 nt, synthetic construct
  source 1..20: mol_type = other RNA
tgaaaatttcaatgtagttg

SEQ ID NO: 49630 - RNA, 20 nt, synthetic construct
  source 1..20: mol_type = other RNA
gggatagtcaggtaaacagt

SEQ ID NO: 49631 - RNA, 20 nt, synthetic construct
  source 1..20: mol_type = other RNA
aacctattctcactaagatg

SEQ ID NO: 49632 - RNA, 20 nt, synthetic construct
  source 1..20: mol_type = other RNA
acttgagtactctaacacag

SEQ ID NO: 49633 - RNA, 20 nt, synthetic construct
  source 1..20: mol_type = other RNA
actctaaaaagtgaaaatca

SEQ ID NO: 49634 - RNA, 20 nt, synthetic construct
  source 1..20: mol_type = other RNA
ggatgttacaagacagacag

SEQ ID NO: 49635 - RNA, 20 nt, synthetic construct
  source 1..20: mol_type = other RNA
aaacccacaagtacttacat

SEQ ID NO: 49636 - RNA, 20 nt, synthetic construct
  source 1..20: mol_type = other RNA
ctcaggccccgcacgatccg

SEQ ID NO: 49637 - RNA, 20 nt, synthetic construct
  source 1..20: mol_type = other RNA
gccaagccctgtcggccgtg
